European Patent Application EP 4 640 697 A1, published October 29, 2025. Title: COMPLEX AND USE THEREOF. Applicant: EPIGENIC THERAPEUTICS, INC. The sequence listing filed with the application follows.

SEQUENCE LISTING (365 sequences)

SEQ ID NO: 1 - protein, 1368 aa, synthetic construct
  REGION 1..1368: note = dCas9_H840A_D10A
MDKKYSIGLAIGTNSVGWAVITDEYKVPSKKFKVLGNTDRHSIKKNLIGALLFDSGETAEATRLKRTARRRYTRRKNRICYLQEIFSNEMAKVDDSFFHRLEESFLVEEDKKHERHPIFGNIVDEVAYHEKYPTIYHLRKKLVDSTDKADLRLIYLALAHMIKFRGHFLIEGDLNPDNSDVDKLFIQLVQTYNQLFEENPINASGVDAKAILSARLSKSRRLENLIAQLPGEKKNGLFGNLIALSLGLTPNFKSNFDLAEDAKLQLSKDTYDDDLDNLLAQIGDQYADLFLAAKNLSDAILLSDILRVNTEITKAPLSASMIKRYDEHHQDLTLLKALVRQQLPEKYKEIFFDQSKNGYAGYIDGGASQEEFYKFIKPILEKMDGTEELLVKLNREDLLRKQRTFDNGSIPHQIHLGELHAILRRQEDFYPFLKDNREKIEKILTFRIPYYVGPLARGNSRFAWMTRKSEETITPWNFEEVVDKGASAQSFIERMTNFDKNLPNEKVLPKHSLLYEYFTVYNELTKVKYVTEGMRKPAFLSGEQKKAIVDLLFKTNRKVTVKQLKEDYFKKIECFDSVEISGVEDRFNASLGTYHDLLKIIKDKDFLDNEENEDILEDIVLTLTLFEDREMIEERLKTYAHLFDDKVMKQLKRRRYTGWGRLSRKLINGIRDKQSGKTILDFLKSDGFANRNFMQLIHDDSLTFKEDIQKAQVSGQGDSLHEHIANLAGSPAIKKGILQTVKVVDELVKVMGRHKPENIVIEMARENQTTQKGQKNSRERMKRIEEGIKELGSQILKEHPVENTQLQNEKLYLYYLQNGRDMYVDQELDINRLSDYDVDAIVPQSFLKDDSIDNKVLTRSDKNRGKSDNVPSEEVVKKMKNYWRQLLNAKLITQRKFDNLTKAERGGLSELDKAGFIKRQLVETRQITKHVAQILDSRMNTKYDENDKLIREVKVITLKSKLVSDFRKDFQFYKVREINNYHHAHDAYLNAVVGTALIKKYPKLESEFVYGDYKVYDVRKMIAKSEQEIGKATAKYFFYSNIMNFFKTEITLANGEIRKRPLIETNGETGEIVWDKGRDFATVRKVLSMPQVNIVKKTEVQTGGFSKESILPKRNSDKLIARKKDWDPKKYGGFDSPTVAYSVLVVAKVEKGKSKKLKSVKELLGITIMERSSFEKNPIDFLEAKGYKEVKKDLIIKLPKYSLFELENGRKRMLASAGELQKGNELALPSKYVNFLYLASHYEKLKGSPEDNEQKQLFVEQHKHYLDEIIEQISEFSKRVILADANLDKVLSAYNKHRDKPIREQAENIIHLFTLTNLGAPAAFKYFDTTIDRKRYTSTKEVLDATLIHQSITGLYETRIDLSQLGGD

SEQ ID NO: 2 - protein, 1368 aa, synthetic construct
  REGION 1..1368: note = nCas9_D10A
MDKKYSIGLAIGTNSVGWAVITDEYKVPSKKFKVLGNTDRHSIKKNLIGALLFDSGETAEATRLKRTARRRYTRRKNRICYLQEIFSNEMAKVDDSFFHRLEESFLVEEDKKHERHPIFGNIVDEVAYHEKYPTIYHLRKKLVDSTDKADLRLIYLALAHMIKFRGHFLIEGDLNPDNSDVDKLFIQLVQTYNQLFEENPINASGVDAKAILSARLSKSRRLENLIAQLPGEKKNGLFGNLIALSLGLTPNFKSNFDLAEDAKLQLSKDTYDDDLDNLLAQIGDQYADLFLAAKNLSDAILLSDILRVNTEITKAPLSASMIKRYDEHHQDLTLLKALVRQQLPEKYKEIFFDQSKNGYAGYIDGGASQEEFYKFIKPILEKMDGTEELLVKLNREDLLRKQRTFDNGSIPHQIHLGELHAILRRQEDFYPFLKDNREKIEKILTFRIPYYVGPLARGNSRFAWMTRKSEETITPWNFEEVVDKGASAQSFIERMTNFDKNLPNEKVLPKHSLLYEYFTVYNELTKVKYVTEGMRKPAFLSGEQKKAIVDLLFKTNRKVTVKQLKEDYFKKIECFDSVEISGVEDRFNASLGTYHDLLKIIKDKDFLDNEENEDILEDIVLTLTLFEDREMIEERLKTYAHLFDDKVMKQLKRRRYTGWGRLSRKLINGIRDKQSGKTILDFLKSDGFANRNFMQLIHDDSLTFKEDIQKAQVSGQGDSLHEHIANLAGSPAIKKGILQTVKVVDELVKVMGRHKPENIVIEMARENQTTQKGQKNSRERMKRIEEGIKELGSQILKEHPVENTQLQNEKLYLYYLQNGRDMYVDQELDINRLSDYDVHHIVPQSFLKDDSIDNKVLTRSDKNRGKSDNVPSEEVVKKMKNYWRQLLNAKLITQRKFDNLTKAERGGLSELDKAGFIKRQLVETRQITKHVAQILDSRMNTKYDENDKLIREVKVITLKSKLVSDFRKDFQFYKVREINNYHHAHDAYLNAVVGTALIKKYPKLESEFVYGDYKVYDVRKMIAKSEQEIGKATAKYFFYSNIMNFFKTEITLANGEIRKRPLIETNGETGEIVWDKGRDFATVRKVLSMPQVNIVKKTEVQTGGFSKESILPKRNSDKLIARKKDWDPKKYGGFDSPTVAYSVLVVAKVEKGKSKKLKSVKELLGITIMERSSFEKNPIDFLEAKGYKEVKKDLIIKLPKYSLFELENGRKRMLASAGELQKGNELALPSKYVNFLYLASHYEKLKGSPEDNEQKQLFVEQHKHYLDEIIEQISEFSKRVILADANLDKVLSAYNKHRDKPIREQAENIIHLFTLTNLGAPAAFKYFDTTIDRKRYTSTKEVLDATLIHQSITGLYETRIDLSQLGGD

SEQ ID NO: 3 - protein, 1368 aa, synthetic construct
  REGION 1..1368: note = nCas9_H839A
MDKKYSIGLDIGTNSVGWAVITDEYKVPSKKFKVLGNTDRHSIKKNLIGALLFDSGETAEATRLKRTARRRYTRRKNRICYLQEIFSNEMAKVDDSFFHRLEESFLVEEDKKHERHPIFGNIVDEVAYHEKYPTIYHLRKKLVDSTDKADLRLIYLALAHMIKFRGHFLIEGDLNPDNSDVDKLFIQLVQTYNQLFEENPINASGVDAKAILSARLSKSRRLENLIAQLPGEKKNGLFGNLIALSLGLTPNFKSNFDLAEDAKLQLSKDTYDDDLDNLLAQIGDQYADLFLAAKNLSDAILLSDILRVNTEITKAPLSASMIKRYDEHHQDLTLLKALVRQQLPEKYKEIFFDQSKNGYAGYIDGGASQEEFYKFIKPILEKMDGTEELLVKLNREDLLRKQRTFDNGSIPHQIHLGELHAILRRQEDFYPFLKDNREKIEKILTFRIPYYVGPLARGNSRFAWMTRKSEETITPWNFEEVVDKGASAQSFIERMTNFDKNLPNEKVLPKHSLLYEYFTVYNELTKVKYVTEGMRKPAFLSGEQKKAIVDLLFKTNRKVTVKQLKEDYFKKIECFDSVEISGVEDRFNASLGTYHDLLKIIKDKDFLDNEENEDILEDIVLTLTLFEDREMIEERLKTYAHLFDDKVMKQLKRRRYTGWGRLSRKLINGIRDKQSGKTILDFLKSDGFANRNFMQLIHDDSLTFKEDIQKAQVSGQGDSLHEHIANLAGSPAIKKGILQTVKVVDELVKVMGRHKPENIVIEMARENQTTQKGQKNSRERMKRIEEGIKELGSQILKEHPVENTQLQNEKLYLYYLQNGRDMYVDQELDINRLSDYDVAHIVPQSFLKDDSIDNKVLTRSDKNRGKSDNVPSEEVVKKMKNYWRQLLNAKLITQRKFDNLTKAERGGLSELDKAGFIKRQLVETRQITKHVAQILDSRMNTKYDENDKLIREVKVITLKSKLVSDFRKDFQFYKVREINNYHHAHDAYLNAVVGTALIKKYPKLESEFVYGDYKVYDVRKMIAKSEQEIGKATAKYFFYSNIMNFFKTEITLANGEIRKRPLIETNGETGEIVWDKGRDFATVRKVLSMPQVNIVKKTEVQTGGFSKESILPKRNSDKLIARKKDWDPKKYGGFDSPTVAYSVLVVAKVEKGKSKKLKSVKELLGITIMERSSFEKNPIDFLEAKGYKEVKKDLIIKLPKYSLFELENGRKRMLASAGELQKGNELALPSKYVNFLYLASHYEKLKGSPEDNEQKQLFVEQHKHYLDEIIEQISEFSKRVILADANLDKVLSAYNKHRDKPIREQAENIIHLFTLTNLGAPAAFKYFDTTIDRKRYTSTKEVLDATLIHQSITGLYETRIDLSQLGGD

SEQ ID NO: 4 - protein, 1368 aa, synthetic construct
  REGION 1..1368: note = nCas9_H840A
MDKKYSIGLDIGTNSVGWAVITDEYKVPSKKFKVLGNTDRHSIKKNLIGALLFDSGETAEATRLKRTARRRYTRRKNRICYLQEIFSNEMAKVDDSFFHRLEESFLVEEDKKHERHPIFGNIVDEVAYHEKYPTIYHLRKKLVDSTDKADLRLIYLALAHMIKFRGHFLIEGDLNPDNSDVDKLFIQLVQTYNQLFEENPINASGVDAKAILSARLSKSRRLENLIAQLPGEKKNGLFGNLIALSLGLTPNFKSNFDLAEDAKLQLSKDTYDDDLDNLLAQIGDQYADLFLAAKNLSDAILLSDILRVNTEITKAPLSASMIKRYDEHHQDLTLLKALVRQQLPEKYKEIFFDQSKNGYAGYIDGGASQEEFYKFIKPILEKMDGTEELLVKLNREDLLRKQRTFDNGSIPHQIHLGELHAILRRQEDFYPFLKDNREKIEKILTFRIPYYVGPLARGNSRFAWMTRKSEETITPWNFEEVVDKGASAQSFIERMTNFDKNLPNEKVLPKHSLLYEYFTVYNELTKVKYVTEGMRKPAFLSGEQKKAIVDLLFKTNRKVTVKQLKEDYFKKIECFDSVEISGVEDRFNASLGTYHDLLKIIKDKDFLDNEENEDILEDIVLTLTLFEDREMIEERLKTYAHLFDDKVMKQLKRRRYTGWGRLSRKLINGIRDKQSGKTILDFLKSDGFANRNFMQLIHDDSLTFKEDIQKAQVSGQGDSLHEHIANLAGSPAIKKGILQTVKVVDELVKVMGRHKPENIVIEMARENQTTQKGQKNSRERMKRIEEGIKELGSQILKEHPVENTQLQNEKLYLYYLQNGRDMYVDQELDINRLSDYDVHAIVPQSFLKDDSIDNKVLTRSDKNRGKSDNVPSEEVVKKMKNYWRQLLNAKLITQRKFDNLTKAERGGLSELDKAGFIKRQLVETRQITKHVAQILDSRMNTKYDENDKLIREVKVITLKSKLVSDFRKDFQFYKVREINNYHHAHDAYLNAVVGTALIKKYPKLESEFVYGDYKVYDVRKMIAKSEQEIGKATAKYFFYSNIMNFFKTEITLANGEIRKRPLIETNGETGEIVWDKGRDFATVRKVLSMPQVNIVKKTEVQTGGFSKESILPKRNSDKLIARKKDWDPKKYGGFDSPTVAYSVLVVAKVEKGKSKKLKSVKELLGITIMERSSFEKNPIDFLEAKGYKEVKKDLIIKLPKYSLFELENGRKRMLASAGELQKGNELALPSKYVNFLYLASHYEKLKGSPEDNEQKQLFVEQHKHYLDEIIEQISEFSKRVILADANLDKVLSAYNKHRDKPIREQAENIIHLFTLTNLGAPAAFKYFDTTIDRKRYTSTKEVLDATLIHQSITGLYETRIDLSQLGGD

SEQ ID NO: 5 - protein, 1368 aa, synthetic construct
  REGION 1..1368: note = nCas9_N863A
MDKKYSIGLDIGTNSVGWAVITDEYKVPSKKFKVLGNTDRHSIKKNLIGALLFDSGETAEATRLKRTARRRYTRRKNRICYLQEIFSNEMAKVDDSFFHRLEESFLVEEDKKHERHPIFGNIVDEVAYHEKYPTIYHLRKKLVDSTDKADLRLIYLALAHMIKFRGHFLIEGDLNPDNSDVDKLFIQLVQTYNQLFEENPINASGVDAKAILSARLSKSRRLENLIAQLPGEKKNGLFGNLIALSLGLTPNFKSNFDLAEDAKLQLSKDTYDDDLDNLLAQIGDQYADLFLAAKNLSDAILLSDILRVNTEITKAPLSASMIKRYDEHHQDLTLLKALVRQQLPEKYKEIFFDQSKNGYAGYIDGGASQEEFYKFIKPILEKMDGTEELLVKLNREDLLRKQRTFDNGSIPHQIHLGELHAILRRQEDFYPFLKDNREKIEKILTFRIPYYVGPLARGNSRFAWMTRKSEETITPWNFEEVVDKGASAQSFIERMTNFDKNLPNEKVLPKHSLLYEYFTVYNELTKVKYVTEGMRKPAFLSGEQKKAIVDLLFKTNRKVTVKQLKEDYFKKIECFDSVEISGVEDRFNASLGTYHDLLKIIKDKDFLDNEENEDILEDIVLTLTLFEDREMIEERLKTYAHLFDDKVMKQLKRRRYTGWGRLSRKLINGIRDKQSGKTILDFLKSDGFANRNFMQLIHDDSLTFKEDIQKAQVSGQGDSLHEHIANLAGSPAIKKGILQTVKVVDELVKVMGRHKPENIVIEMARENQTTQKGQKNSRERMKRIEEGIKELGSQILKEHPVENTQLQNEKLYLYYLQNGRDMYVDQELDINRLSDYDVHHIVPQSFLKDDSIDNKVLTRSDKARGKSDNVPSEEVVKKMKNYWRQLLNAKLITQRKFDNLTKAERGGLSELDKAGFIKRQLVETRQITKHVAQILDSRMNTKYDENDKLIREVKVITLKSKLVSDFRKDFQFYKVREINNYHHAHDAYLNAVVGTALIKKYPKLESEFVYGDYKVYDVRKMIAKSEQEIGKATAKYFFYSNIMNFFKTEITLANGEIRKRPLIETNGETGEIVWDKGRDFATVRKVLSMPQVNIVKKTEVQTGGFSKESILPKRNSDKLIARKKDWDPKKYGGFDSPTVAYSVLVVAKVEKGKSKKLKSVKELLGITIMERSSFEKNPIDFLEAKGYKEVKKDLIIKLPKYSLFELENGRKRMLASAGELQKGNELALPSKYVNFLYLASHYEKLKGSPEDNEQKQLFVEQHKHYLDEIIEQISEFSKRVILADANLDKVLSAYNKHRDKPIREQAENIIHLFTLTNLGAPAAFKYFDTTIDRKRYTSTKEVLDATLIHQSITGLYETRIDLSQLGGD

SEQ ID NO: 6 - protein, 1307 aa, synthetic construct
  REGION 1..1307: note = dCas12(AsCpf1
MTQFEGFTNLYQVSKTLRFELIPQGKTLKHIQEQGFIEEDKARNDHYKELKPIIDRIYKTYADQCLQLVQLDWENLSAAIDSYRKEKTEETRNALIEEQATYRNAIHDYFIGRTDNLTDAINKRHAEIYKGLFKAELFNGKVLKQLGTVTTTEHENALLRSFDKFTTYFSGFYENRKNVFSAEDISTAIPHRIVQDNFPKFKENCHIFTRLITAVPSLREHFENVKKAIGIFVSTSIEEVFSFPFYNQLLTQTQIDLYNQLLGGISREAGTEKIKGLNEVLNLAIQKNDETAHIIASLPHRFIPLFKQILSDRNTLSFILEEFKSDEEVIQSFCKYKTLLRNENVLETAEALFNELNSIDLTHIFISHKKLETISSALCDHWDTLRNALYERRISELTGKITKSAKEKVQRSLKHEDINLQEIISAAGKELSEAFKQKTSEILSHAHAALDQPLPTTLKKQEEKEILKSQLDSLLGLYHLLDWFAVDESNEVDPEFSARLTGIKLEMEPSLSFYNKARNYATKKPYSVEKFKLNFQMPTLASGWDVNKEKNNGAILFVKNGLYYLGIMPKQKGRYKALSFEPTEKTSEGFDKMYYDYFPDAAKMIPKCSTQLKAVTAHFQTHTTPILLSNNFIEPLEITKEIYDLNNPEKEPKKFQTAYAKKTGDQKGYREALCKWIDFTRDFLSKYTKTTSIDLSSLRPSSQYKDLGEYYAELNPLLYHISFQRIAEKEIMDAVETGKLYLFQIYNKDFAKGHHGKPNLHTLYWTGLFSPENLAKTSIKLNGQAELFYRPKSRMKRMAHRLGEKMLNKKLKDQKTPIPDTLYQELYDYVNHRLSHDLSDEARALLPNVITKEVSHEIIKDRRFTSDKFFFHVPITLNYQAANSPSKFNQRVNAYLKEHPETPIIGIARGERNLIYITVIDSTGKILEQRSLNTIQQFDYQKKLDNREKERVAARQAWSVVGTIKDLKQGYLSQVIHEIVDLMIHYQAVVVLENLNFGFKSKRTGIAEKAVYQQFEKMLIDKLNCLVLKDYPAEKVGGVLNPYQLTDQFTSFAKMGTQSGFLFYVPAPYTSKIDPLTGFVDPFVWKTIKNHESRKHFLEGFDFLHYDVKTGDFILHFKMNRNLSFQRGLPGFMPAWDIVFEKNETQFDAKGTPFIAGKRIVPVIENHRFTGRYRDLYPANELIALLEEKGIVFRDGSNILPKLLENDDSHAIDTMVALIRSVLQMRNSNAATGEDYINSPVRDLNGVCFDSRFQNPEWPMDADANGAYHIALKGQLLLNHLKESKDLKLQNGISNQDWLAYIQELRN

SEQ ID NO: 7 - protein, 1228 aa, synthetic construct
  REGION 1..1228: note = dCas12(LbCpf1
MSKLEKFTNCYSLSKTLRFKAIPVGKTQENIDNKRLLVEDEKRAEDYKGVKKLLDRYYLSFINDVLHSIKLKNLNNYISLFRKKTRTEKENKELENLEINLRKEIAKAFKGNEGYKSLFKKDIIETILPEFLDDKDEIALVNSFNGFTTAFTGFFDNRENMFSEEAKSTSIAFRCINENLTRYISNMDIFEKVDAIFDKHEVQEIKEKILNSDYDVEDFFEGEFFNFVLTQEGIDVYNAIIGGFVTESGEKIKGLNEYINLYNQKTKQKLPKFKPLYKQVLSDRESLSFYGEGYTSDEEVLEVFRNTLNKNSEIFSSIKKLEKLFKNFDEYSSAGIFVKNGPAISTISKDIFGEWNVIRDKWNAEYDDIHLKKKAVVTEKYEDDRRKSFKKIGSFSLEQLQEYADADLSVVEKLKEIIIQKVDEIYKVYGSSEKLFDADFVLEKSLKKNDAVVAIMKDLLDSVKSFENYIKAFFGEGKETNRDESFYGDFVLAYDILLKVDHIYDAIRNYVTQKPYSKDKFKLYFQNPQFMGGWDKDKETDYRATILRYGSKYYLAIMDKKYAKCLQKIDKDDVNGNYEKINYKLLPGPNKMLPKVFFSKKWMAYYNPSEDIQKIYKNGTFKKGDMFNLNDCHKLIDFFKDSISRYPKWSNAYDFNFSETEKYKDIAGFYREVEEQGYKVSFESASKKEVDKLVEEGKLYMFQIYNKDFSDKSHGTPNLHTMYFKLLFDENNHGQIRLSGGAELFMRRASLKKEELVVHPANSPIANKNPDNPKKTTTLSYDVYKDKRFSEDQYELHIPIAINKCPKNIFKINTEVRVLLKHDDNPYVIGIARGERNLLYIVVVDGKGNIVEQYSLNEIINNFNGIRIKTDYHSLLDKKEKERFEARQNWTSIENIKELKAGYISQVVHKICELVEKYDAVIALEDLNSGFKNSRVKVEKQVYQKFEKMLIDKLNYMVDKKSNPCATGGALKGYQITNKFESFKSMSTQNGFIFYIPAWLTSKIDPSTGFVNLLKTKYTSIADSKKFISSFDRIMYVPEEDLFEFALDYKNFSRTDADYIKKWKLYSYGNRIRIFRNPKKNNVFDWEEVCLTSAYKELFNKYGINYQQGDIRALLCEQSDKAFYSSFMALMSLMLQMRNSITGRTDVDFLISPVKNSDGIFYDSRNYEAQENAILPKNADANGAYNIARKVLWAIGQFKKAEDEKLDKVKIAISNKEWLEYAQTSVKH

SEQ ID NO: 8 - protein, 1228 aa, synthetic construct
  REGION 1..1228: note = dCas12a
MSKLEKFTNCYSLSKTLRFKAIPVGKTQENIDNKRLLVEDEKRAEDYKGVKKLLDRYYLSFINDVLHSIKLKNLNNYISLFRKKTRTEKENKELENLEINLRKEIAKAFKGNEGYKSLFKKDIIETILPEFLDDKDEIALVNSFNGFTTAFTGFFDNRENMFSEEAKSTSIAFRCINENLTRYISNMDIFEKVDAIFDKHEVQEIKEKILNSDYDVEDFFEGEFFNFVLTQEGIDVYNAIIGGFVTESGEKIKGLNEYINLYNQKTKQKLPKFKPLYKQVLSDRESLSFYGEGYTSDEEVLEVFRNTLNKNSEIFSSIKKLEKLFKNFDEYSSAGIFVKNGPAISTISKDIFGEWNVIRDKWNAEYDDIHLKKKAVVTEKYEDDRRKSFKKIGSFSLEQLQEYADADLSVVEKLKEIIIQKVDEIYKVYGSSEKLFDADFVLEKSLKKNDAVVAIMKDLLDSVKSFENYIKAFFGEGKETNRDESFYGDFVLAYDILLKVDHIYDAIRNYVTQKPYSKDKFKLYFQNPQFMGGWDKDKETDYRATILRYGSKYYLAIMDKKYAKCLQKIDKDDVNGNYEKINYKLLPGPNKMLPKVFFSKKWMAYYNPSEDIQKIYKNGTFKKGDMFNLNDCHKLIDFFKDSISRYPKWSNAYDFNFSETEKYKDIAGFYREVEEQGYKVSFESASKKEVDKLVEEGKLYMFQIYNKDFSDKSHGTPNLHTMYFKLLFDENNHGQIRLSGGAELFMRRASLKKEELVVHPANSPIANKNPDNPKKTTTLSYDVYKDKRFSEDQYELHIPIAINKCPKNIFKINTEVRVLLKHDDNPYVIGIARGERNLLYIVVVDGKGNIVEQYSLNEIINNFNGIRIKTDYHSLLDKKEKERFEARQNWTSIENIKELKAGYISQVVHKICELVEKYDAVIALADLNSGFKNSRVKVEKQVYQKFEKMLIDKLNYMVDKKSNPCATGGALKGYQITNKFESFKSMSTQNGFIFYIPAWLTSKIDPSTGFVNLLKTKYTSIADSKKFISSFDRIMYVPEEDLFEFALDYKNFSRTDADYIKKWKLYSYGNRIRIFRNPKKNNVFDWEEVCLTSAYKELFNKYGINYQQGDIRALLCEQSDKAFYSSFMALMSLMLQMRNSITGRTDVAFLISPVKNSDGIFYDSRNYEAQENAILPKNADANGAYNIARKVLWAIGQFKKAEDEKLDKVKIAISNKEWLEYAQTSVKH

SEQ ID NO: 9 - protein, 1011 aa, synthetic construct
  REGION 1..1011: note = dCas12i
MGITMSDTTFRPYKSKLNPNERKMPMVVDTMNWCDNACSVFFDLFVGLYGGVKIGDVTNFLTEKQDTTTDADLLCAINWFRAMPVSNPDAVVGPEQLVVRFRDYSGHNPSPMASMYLSAPVNPRYTWVDCRFLYQQMCQTLGANLDVDISTLVQTGLLPIQKDTQLNAYSFCSNVFGEGVKEDPSAKVTSYTAAANALSGATNPIITYEDYRQILSSAITNRPSRKGAKDILAADLDSTKTGVLPGNYVSQRIAMYQASAASKARGVVLPNRLRVKAYLQNLVGLNYICTTWAAPMLRAVGDIKSKNSNNYRFVGERLERQQEIDNLLAVSNIRSAQAILQQFRANESNQFYIKKRHIGKGLPSLYDMWDLMDEKEGIDNYIQSLKGDKTERLPIRELLQIIYPHRKSVSAELFLSAAELTDVEDRQNRCMVHPTVRGSLVINFGKSSTIFGAITPPDTLIKFRGEMVPAGQTGMIWFTMHLVDGGKWVKHHIPCHSSRYFEEIYAWKKDLPTLPFPRRSLYGYAIGNKISDTRKIDLRRKKASKQYLRTLENMTHNVEFDPTTQFMVDQELNVTITARVKKIPPVRDVPVGSRIMGLNKNQTIRDCYSIWERVEANTSGSFQHPVVQDVWLRLVADGHVTSTVNGPNGQIDQMSYSGPDVANCGNWMQERSNFITSVDDADQSIMKHFLWNNRVKLYAWNCVYAGTLMKAISKQMTTANRNLFRNEILSFVGGRFGCRLGSLAQVSLDLLRRMKSVISCYFSRNNAFTIEERSAFDKELMELFESLDNKMNNKRKEKVNRTLSSIFQVAKQHNVVRLVVTKNLQTPDANVRSVMNQRSVDWCARKIEEKIVDLGNVIGIYVDLVEALDLSHLDPFIYIAKGDVGKECQFDEVESSSLLPIHTSMFRDWHGLVNKGRTTTPIYHSALRSFASHYGLRFDDLARIKAAELAKMLPDQKVFIPHRGGRFFMSTYPVTSTSRPVSYDGRQRFLNSGDMVAPVNTMLRGFRRARS

SEQ ID NO: 10 - protein, 19 aa, synthetic construct
  REGION 1..19: note = GCN4
EELLSKNYHLENEVARLKK

SEQ ID NO: 11 - protein, 16 aa, synthetic construct
  REGION 1..16: note = GFP11
RDHMVLHEYVNAAGIT

SEQ ID NO: 12 - protein, 7 aa, synthetic construct
  REGION 1..7: note = peptide GVKESLV
GVLGSLV

SEQ ID NO: 13 - protein, 247 aa, synthetic construct
  REGION 1..247: note = scFv
MGPDIVMTQSPSSLSASVGDRVTITCRSSTGAVTTSNYASWVQEKPGKLFKGLIGGTNNRAPGVPSRFSGSLIGDKATLTISSLQPEDFATYFCALWYSNHWVFGQGTKVELKRGGGGSGGGGSGGGGSSGGGSEVKLLESGGGLVQPGGSLKLSCAVSGFSLTDYGVNWVRQAPGRGLEWIGVIWGDGITDYNSALKDRFIISKDNGKNTVYLQMSKVRSDDTALYYCVTGLFDYWGQGTLVTVSS

SEQ ID NO: 14 - protein, 213 aa, synthetic construct
  REGION 1..213: note = GFP1-10
SKGEELFTGVVPILVELDGDVNGHKFSVRGEGEGDATIGKLTLKFICTTGKLPVPWPTLVTTLTYGVQCFSRYPDHMKRHDFFKSAMPEGYVQERTISFKDDGKYKTRAVVKFEGDTLVNRIELKGTDFKEDGNILGHKLEYNFNSHNVYITADKQKNGIKANFTVRHNVEDGSVQLADHYQQNTPIGDGPVLLPDNHYLSTQTVLSKDPNEK

SEQ ID NO: 15 - protein, 238 aa, synthetic construct
  REGION 1..238: note = GFP
MSKGEELFTGVVPILVELDGDVNGHKFSVSGEGEGDATYGKLTLKFICTTGKLPVPWPTLVTTFSYGVQCFSRYPDHMKQHDFFKSAMPEGYVQERTIFFKDDGNYKTRAEVKFEGDTLVNRIELKGIDFKEDGNILGHKLEYNYNSHNVYIMADKQKNGIKVNFKIRHNIEDGSVQLADHYQQNTPIGDGPVLLPDNHYLSTQSALSKDPNEKRDHMVLLEFVTAAGITHGMDELYK

SEQ ID NO: 16 - protein, 233 aa, synthetic construct
  REGION 1..233: note = mCherry
MVSKGEEDNMAIIKEFMRFKVHMEGSVNGHEFEIEGEGEGRPYEGTQTAKLKVTKGGPLPFAWDILSPQFMYGSKAYVKHPADIPDYLKLSFPEGFKWERVMNFEDGGVVTVTQDSSLQDGEFIYKVKLRGTNFPSDGPVMQKKTMGWEASSERMYPEDGALKGEIKQRLKLKDGGHYDAEVKTTYKAKKPVQLPGAYNVNIKLDITSHNEDYTIVEQYERAEGRHSTGGMDE

SEQ ID NO: 17 - protein, 240 aa, synthetic construct
  REGION 1..240: note = eCFP
  SITE 240: note = misc_feature - Xaa =
MVSKGEELFTGVVPILVELDGDVNGHKFSVSGEGEGDATYGKLTLKFICTTGKLPVPWPTLVTTLTWGVQCFSRYPDHMKQHDFFKSAMPEGYVQERTIFFKDDGNYKTRAEVKFEGDTLVNRIELKGIDFKEDGNILGHKLEYNYISHNVYITADKQKNGIKANFKIRHNIEDGSVQLADHYQQNTPIGDGPVLLPDNHYLSTQSALSKDPNEKRDHMVLLEFVTAAGITLGMDELYKX

SEQ ID NO: 18 - protein, 239 aa, synthetic construct
  REGION 1..239: note = eYFP
MVSKGEELFTGVVPILVELDGDVNGHKFSVSGEGEGDATYGKLTLKFICTTGKLPVPWPTLVTTFGYGLQCFARYPDHMKQHDFFKSAMPEGYVQERTIFFKDDGNYKTRAEVKFEGDTLVNRIELKGIDFKEDGNILGHKLEYNYNSHNVYIMADKQKNGIKVNFKIRHNIEDGSVQLADHYQQNTPIGDGPVLLPDNHYLSYQSALSKDPNEKRDHMVLLEFVTAAGITLGMDELYK

SEQ ID NO: 19 - protein, 302 aa, synthetic construct
  REGION 1..302: note = DNMT3A-CD
MNHDQEFDPPKVYPPVPAEKRKPIRVLSLFDGIATGLLVLKDLGIQVDRYIASEVCEDSITVGMVRHQGKIMYVGDVRSVTQKHIQEWGPFDLVIGGSPCNDLSIVNPARKGLYEGTGRLFFEFYRLLHDARPKEGDDRPFFWLFENVVAMGVSDKRDISRFLESNPVMIDAKEVSAAHRARYFWGNLPGMNRPLASTVNDKLELQECLEHGRIAKFSKVRTITTRSNSIKQGKDQHFPVFMNEKEDILWCTEMERVFGFPVHYTDVSNMSRLARQRLLGRSWSVPVIRHLFAPLKEYFACV

SEQ ID NO: 20 - protein, 279 aa, synthetic construct
  REGION 1..279: note = DNMT3B
IRVLSLFDGIATGYLVLKELGIKVGKYVASEVCEESIAVGTVKHEGNIKYVNDVRNITKKNIEEWGPFDLVIGGSPCNDLSNVNPARKGLYEGTGRLFFEFYHLLNYSRPKEGDDRPFFWMFENVVAMKVGDKRDISRFLECNPVMIDAIKVSAAHRARYFWGNLPGMNRPVIASKNDKLELQDCLEYNRIAKLKKVQTITTKSNSIKQGKNQLFPVVMNGKEDVLWCTELERIFGFPVHYTDVSNMGRGARQKLLGRSWSVPVIRHLFAPLKDYFACE

SEQ ID NO: 21 - protein, 215 aa, synthetic construct
  REGION 1..215: note = DNMT3L-CD
MGPMEIYKTVSAWKRQPVRVLSLFRNIDKVLKSLGFLESGSGSGGGTLKYVEDVTNVVRRDVEKWGPFDLVYGSTQPLGSSCDRCPGWYMFQFHRILQYALPRQESQRPFFWIFMDNLLLTEDDQETTTRFLQTEAVTLQDVRGRDYQNAMRVWSNIPGLKSKHAPLTPKEEEYLQAQVRSRSKLDAPKVDLLVKNCLLPLREYFKYFSQNSLPL

SEQ ID NO: 22 - protein, 203 aa, synthetic construct
  REGION 1..203: note = hDNMT3L
MFETVPVWRRQPVRVLSLFEDIKKELTSLGFLESGSDPGQLKHVVDVTDTVRKDVEEWGPFDLVYGATPPLGHTCDRPPSWYLFQFHRLLQYARPKPGSPRPFFWMFVDNLVLNKEDLDVASRFLEMEPVTIPDVHGGSLQNAVRVWSNIPAIRSSRHWALVSEEELSLLAQNKQSSKLAAKWPTKLVKNCFLPLREYFKYFS

SEQ ID NO: 23 - protein, 461 aa, synthetic construct
  REGION 1..461: note = DNMT1
LRTLDVFSGCGGLSEGFHQAGISDTLWAIEMWDPAAQAFRLNNPGSTVFTEDCNILLKLVMAGETTNSRGQRLPQKGDVEMLCGGPPCQGFSGMNRFNSRTYSKFKNSLVVSFLSYCDYYRPRFFLLENVRNFVSFKRSMVLKLTLRCLVRMGYQCTFGVLQAGQYGVAQTRRRAIILAAAPGEKLPLFPEPLHVFAPRACQLSVVVDDKKFVSNITRLSSGPFRTITVRDTMSDLPEVRNGASALEISYNGEPQSWFQRQLRGAQYQPILRDHICKDMSALVAARMRHIPLAPGSDWRDLPNIEVRLSDGTMARKLRYTHHDRKNGRSSSGALRGVCSCVEAGKACDPAARQFNTLIPWCLPHTGNRHNHWAGLYGRLEWDGFFSTTVTNPEPMGKQGRVLHPEQHRVVSVRECARSQGFPDTYRLFGNILDKHRQVGNAVPPPLAKAIGLEIKLCMLAK

SEQ ID NO: 24 - protein, 279 aa, synthetic construct
  REGION 1..279: note = Dnmt3c(from mouse)
IRVLSLFDGIATGYLVLKELGIKVEKYIASEVCAESIAVGTVKHEGQIKYVDDIRNITKEHIDEWGPFDLVIGGSPCNDLSCVNPVRKGLFEGTGRLFFEFYRLLNYSCPEEEDDRPFFWMFENVVAMEVGDKRDISRFLECNPVMIDAIKVSAAHRARYFWGNLPGMNRPVMASKNDKLELQDCLEFSRTAKLKKVQTITTKSNSIRQGKNQLFPVVMNGKDDVLWCTELERIFGFPEHYTDVSNMGRGARQKLLGRSWSVPVIRHLFAPLKDHFACE

SEQ ID NO: 25 - protein, 62 aa, synthetic construct
  REGION 1..62: note = KRAB
RTLVTFKDVFVDFTREEWKLLDTAQQIVYRNVMLENYKNLVSLGYQLTKPDVILRLEKGEEP

SEQ ID NO: 26 - protein, 62 aa, synthetic construct
  REGION 1..62: note = Zim3
VTFEDVTVNFTQGEWQRLNPEQRNLYRDVMLENYSNLVSVGQGETTKPDVILRLEQGKEPWL

SEQ ID NO: 27 - protein, 61 aa, synthetic construct
  REGION 1..61: note = Znf680
LTFRDVAIEFSLEEWQCLDTAQRNLYRKVMFENYRNLVFLGIAVSKPHLITCLEQGKEPWN

SEQ ID NO: 28 - protein, 62 aa, synthetic construct
  REGION 1..62: note = Znf554
VTFEDVSMDFSQEEWELLEPAQKNLYREVMLENYRNVVSLEALKNQCTDVGIKEGPLSPAQT

SEQ ID NO: 29 - protein, 61 aa, synthetic construct
  REGION 1..61: note = Znf264
VTFDDVAVTFTKEEWGQLDLAQRTLYQEVMLENCGLLVSLGCPVPKAELICHLEHGQEPWT

SEQ ID NO: 30 - protein, 61 aa, synthetic construct
  REGION 1..61: note = Znf582
ELFRDVAIVFSQEEWQWLAPAQRDLYRDVMLETYSNLVSLGLAVSKPDVISFLEQGKEPWM

SEQ ID NO: 31 - protein, 61 aa, synthetic construct
  REGION 1..61: note = Znf324
MAFEDVAVYFSQEEWGLLDTAQRALYRRVMLDNFALVASLGLSTSRPRVVIQLERGEEPWV

SEQ ID NO: 32 - protein, 62 aa, synthetic construct
  REGION 1..62: note = Znf669
VAFEDVAVNFTQEEWALLDSSQKNLYREVMQETCRNLASVGSQWKDQNIEDHFEKPGKDIRN

SEQ ID NO: 33 - protein, 61 aa, synthetic construct
  REGION 1..61: note = Znf354a
LTFEDVAVLFTRDEWRKLAPSQRNLYRDVMLENYRNLVSLGLPFTKPKVISLLQQGEDPWE

SEQ ID NO: 34 - protein, 61 aa, synthetic construct
  REGION 1..61: note = Znf82
VMFSDVSIDFSPEEWEYLDLEQKDLYRDVMLENYSNLVSLGCFISKPDVISSLEQGKEPWK

SEQ ID NO: 35 - protein, 61 aa, synthetic construct
  REGION 1..61: note = Znf595
VTFRDVAIEFSPEEWKCLDPAQQNLYRDVMLENYRNLVSLGFVISNPDLVTCLEQIKEPCN

SEQ ID NO: 36 - protein, 61 aa, synthetic construct
  REGION 1..61: note = Znf419
VTFEDVAVYFSQEEWRLLDDAQRLLYRNVMLENFTLLASLGLASSKTHEITQLESWEEPFM

SEQ ID NO: 37 - protein, 61 aa, synthetic construct
  REGION 1..61: note = Znf566
VMFSDVSVDFSQEEWECLNDDQRDLYRDVMLENYSNLVSMGHSISKPNVISYLEQGKEPWL

SEQ ID NO: 38 - protein, 61 aa, synthetic construct
  REGION 1..61: note = Zim2
VTFEDVLVDFSPEELSSLSAAQRNLYREVMLENYRNLVSLGHQFSKPDIISRLEEEESYAM

SEQ ID NO: 39 - protein, 383 aa, synthetic construct
  REGION 1..383: note = EHMT2(G9A)
TGSAAIAEVLLNARCDLHAVNYHGDTPLHIAARESYHDCVLLFLSRGANPELRNKEGDTAWDLTPERSDVWFALQLNRKLRLGVGNRAIRTEKIICRDVARGYENVPIPCVNGVDGEPCPEDYKYISENCETSTMNIDRNITHLQHCTCVDDCSSSNCLCGQLSIRCWYDKDGRLLQEFNKIEPPLIFECNQACSCWRNCKNRVVQSGIKVRLQLYRTAKMGWGVRALQTIPQGTFICEYVGELISDAEADVREDDSYLFDLDNKDGEVYCIDARYYGNISRFINHLCDPNIIPVRVFMLHQDLRFPRIAFFSSRDIRTGEELGFDYGDRFWDIKSKYFTCQCGSEKCKHSAEAIALEQSRLARLDPHPELLPELGSLPPVNT

SEQ ID NO: 40 - protein, 411 aa, synthetic construct
  REGION 1..411: note = SUV39H1
AENLKGCSVCCKSSWNQLQDLCRLAKLSCPALGISKRNLYDFEVEYLCDYKKIREQEYYLVKWRGYPDSESTWEPRQNLKCVRILKQFHKDLERELLRRHHRSKTPRHLDPSLANYLVQKAKQRRALRRWEQELNAKRSHLGRITVENEVDLDGPPRAFVYINEYRVGEGITLNQVAVGCECQDCLWAPTGGCCPGASLHKFAYNDQGQVRLRAGLPIYECNSRCRCGYDCPNRVVQKGIRYDLCIFRTDDGRGWGVRTLEKIRKNSFVMEYVGEIITSEEAERRGQIYDRQGATYLFDLDYVEDVYTVDAAYYGNISHFVNHSCDPNLQVYNVFIDNLDERLPRIAFFATRTIRAGEELTFDYNMQVDPVDMESTRMDSNFGLAGLPGSPKKRVRIECKCGTESCRKYLF

SEQ ID NO: 41 - protein, 47 aa, synthetic construct
  REGION 1..47: note = ZFPM1(FOG)
SRRKQSNPRQIKRSLGDMEAREEVQLVGASHMEQKATAPEAPSPPSA

SEQ ID NO: 42 - protein, 834 aa, synthetic construct
  REGION 1..834: note = TRIM28(KAP1)
AASAAAASAAAASAASGSPGPGEGSAGGEKRSTAPSAAASASASAAASSPAGGGAEALELLEHCGVCRERLRPEREPRLLPCLHSACSACLGPAAPAAANSSGDGGAAGDGTVVDCPVCKQQCFSKDIVENYFMRDSGSKAATDAQDANQCCTSCEDNAPATSYCVECSEPLCETCVEAHQRVKYTKDHTVRSTGPAKSRDGERTVYCNVHKHEPLVLFCESCDTLTCRDCQLNAHKDHQYQFLEDAVRNQRKLLASLVKRLGDKHATLQKSTKEVRSSIRQVSDVQKRVQVDVKMAILQIMKELNKRGRVLVNDAQKVTEGQQERLERQHWTMTKIQKHQEHILRFASWALESDNNTALLLSKKLIYFQLHRALKMIVDPVEPHGEMKFQWDLNAWTKSAEAFGKIVAERPGTNSTGPAPMAPPRAPGPLSKQGSGSSQPMEVQEGYGFGSGDDPYSSAEPHVSGVKRSRSGEGEVSGLMRKVPRVSLERLDLDLTADSQPPVFKVFPGSTTEDYNLIVIERGAAAAATGQPGTAPAGTPGAPPLAGMAIVKEEETEAAIGAPPTATEGPETKPVLMALAEGPGAEGPRLASPSGSTSSGLEVVAPEGTSAPGGGPGTLDDSATICRVCQKPGDLVMCNQCEFCFHLDCHLPALQDVPGEEWSCSLCHVLPDLKEEDGSLSLDGADSTGVVAKLSPANQRKCERVLLALFCHEPCRPLHQLATDSTFSLDQPGGTLDLTLIRARLQEKLSPPYSSPQEFAQDVGRMFKQFNKLTEDKADVQSIIGLQRFFETRMNEAFGDTKFSAVLVEPPPMSLPGAGLSSQELSGGPGDGP

SEQ ID NO: 43 - protein, 745 aa, synthetic construct
  REGION 1..745: note = EZH2
GQTGKKSEKGPVCWRKRVKSEYMRLRQLKRFRRADEVKSMFSSNRQKILERTEILNQEWKQRRIQPVHILTSVSSLRGTRECSVTSDLDFPTQVIPLKTLNAVASVPIMYSWSPLQQNFMVEDETVLHNIPYMGDEVLDQDGTFIEELIKNYDGKVHGDRECGFINDEIFVELVNALGQYNDDDDDDDGDDPEEREEKQKDLEDHRDDKESRPPRKFPSDKIFEAISSMFPDKGTAEELKEKYKELTEQQLPGALPPECTPNIDGPNAKSVQREQSLHSFHTLFCRRCFKYDCFLHPFHATPNTYKRKNTETALDNKPCGPQCYQHLEGAKEFAAALTAERIKTPPKRPGGRRRGRLPNNSSRPSTPTINVLESKDTDSDREAGTETGGENNDKEEEEKKDETSSSSEANSRCQTPIKMKPNIEPPENVEWSGAEASMFRVLIGTYYDNFCAIARLIGTKTCRQVYEFRVKESSIIAPAPAEDVDTPPRKKKRKHRLWAAHCRKIQLKKDGSSNHVYNYQPCDHPRQPCDSSCPCVIAQNFCEKFCQCSSECQNRFPGCRCKAQCNTKQCPCYLAVRECDPDLCLTCGAADHWDSKNVSCKNCSIQRGSKKHLLLAPSDVAGWGIFIKDPVQKNEFISEYCGEIISQDEADRRGKVYDKYMCSFLFNLNNDFVVDATRKGNKIRFANHSVNPNCYAKVMMVNGDHRIGIFAKRAIQTGEELFFDYRYSQADALKYVGIEREMEIP

SEQ ID NO: 44 - protein, 219 aa, synthetic construct
  REGION 1..219: note = MXD1(SID FL)
AAAVRMNIQMLLEAADYLERREREAEHGYASMLPYNNKDRDALKRRNKSKKNNSSSRSTHNEMEKNRRAHLRLCLEKLKGLVPLGPESSRHTTLSLLTKAKLHIKKLEDCDRKAVHQIDQLQREQRHLKRQLEKLGIERIRMDSIGSTVSSERSDSDREIDVDVESTDYLTGDLDWSSSSVSDSDERGSMQSLGSDEGYSSTSIKRIKLQDSHKACLGL

SEQ ID NO: 45 - protein, 29 aa, synthetic construct
  REGION 1..29: note = SID
MNIQMLLEAADYLERREREAEHGYASMLP

SEQ ID NO: 46 - protein, 875 aa, synthetic construct
  REGION 1..875: note = LSD1(KDMA1)
LSGKKAAAAAAAAAAAATGTEAGPGTAGGSENGSEVAAQPAGLSGPAEVGPGAVGERTPRKKEPPRASPPGGLAEPPGSAGPQAGPTVVPGSATPMETGIAETPEGRRTSRRKRAKVEYREMDESLANLSEDEYYSEEERNAKAEKEKKLPPPPPQAPPEEENESEPEEPSGQAGGLQDDSSGGYGDGQASGVEGAAFQSRLPHDRMTSQEAACFPDIISGPQQTQKVFLFIRNRTLQLWLDNPKIQLTFEATLQQLEAPYNSDTVLVHRVHSYLERHGLINFGIYKRIKPLPTKKTGKVIIIGSGVSGLAAARQLQSFGMDVTLLEARDRVGGRVATFRKGNYVADLGAMVVTGLGGNPMAVVSKQVNMELAKIKQKCPLYEANGQADTVKVPKEKDEMVEQEFNRLLEATSYLSHQLDFNVLNNKPVSLGQALEVVIQLQEKHVKDEQIEHWKKIVKTQEELKELLNKMVNLKEKIKELHQQYKEASEVKPPRDITAEFLVKSKHRDLTALCKEYDELAETQGKLEEKLQELEANPPSDVYLSSRDRQILDWHFANLEFANATPLSTLSLKHWDQDDDFEFTGSHLTVRNGYSCVPVALAEGLDIKLNTAVRQVRYTASGCEVIAVNTRSTSQTFIYKCDAVLCTLPLGVLKQQPPAVQFVPPLPEWKTSAVQRMGFGNLNKVVLCFDRVFWDPSVNLFGHVGSTTASRGELFLFWNLYKAPILLALVAGEAAGIMENISDDVIVGRCLAILKGIFGSSAVPQPKETVVSRWRADPWARGSYSYVAAGSSGNDYDLMAQPITPGPSIPGAPQPIPRLFFAGEHTIRNYPATVHGALLSGLREAGRIADQFLGAMYTLPRQATPGVPAQQSPSM

SEQ ID NO: 47 - protein, 190 aa, synthetic construct
  REGION 1..190: note = HP1a (long)
GKKTKRTADSSSSEDEEEYVVEKVLDRRVVKGQVEYLLKWKGFSEEHNTWEPEKNLDCPELISEFMKKYKKMKEGENNKPREKSESNKRKSNFSNSADDIKSKKKREQSNDIARGFERGLEPEKIIGATDSCGDLMFLMKWKDTDEADLVLAKEANVKCPQIVIAFYEERLTWHAYPEDAENKEKETAKS

SEQ ID NO: 48 - protein, 119 aa, synthetic construct
  REGION 1..119: note = HP1a (short)
MKEGENNKPREKSESNKRKSNFSNSADDIKSKKKREQSNDIARGFERGLEPEKIIGATDSCGDLMFLMKWKDTDEADLVLAKEANVKCPQIVIAFYEERLTWHAYPEDAENKEKETAKS

SEQ ID NO: 49 - protein, 427 aa, synthetic construct
  REGION 1..427: note = HDAC3
AKTVAYFYDPDVGNFHYGAGHPMKPHRLALTHSLVLHYGLYKKMIVFKPYQASQHDMCRFHSEDYIDFLQRVSPTNMQGFTKSLNAFNVGDDCPVFPGLFEFCSRYTGASLQGATQLNNKICDIAINWAGGLHHAKKFEASGFCYVNDIVIGILELLKYHPRVLYIDIDIHHGDGVQEAFYLTDRVMTVSFHKYGNYFFPGTGDMYEVGAESGRYYCLNVPLRDGIDDQSYKHLFQPVINQVVDFYQPTCIVLQCGADSLGCDRLGCFNLSIRGHGECVEYVKSFNIPLLVLGGGGYTVRNVARCWTYETSLLVEEAISEELPYSEYFEYFAPDFTLHPDVSTRIENQNSRQYLDQIRQTIFENLKMLNHAPSVQIHDVPADLLTYDRTDEADAEERGPEENYSRPEAPNEFYDGDHDNDKESDVEI

SEQ ID NO: 50 - protein, 301 aa, synthetic construct
  REGION 1..301: note = hSIRT1
TILKDLLPETIPPPELDDMTLWQIVINILSEPPKRKKRKDINTIEDAVKLLQECKKIIVLTGAGVSVSCGIPDFRSRDGIYARLAVDFPDLPDPQAMFDIEYFRKDPRPFFKFAKEIYPGQFQPSLCHKFIALSDKEGKLLRNYTQNIDTLEQVAGIQRIIQCHGSFATASCLICKYKVDCEAVRGDIFNQVVPRCPRCPADEPLAIMKPEIVFFGENLPEQFHRAMKYDKDEVDLLIVIGSSLKVRPVALIPSSIPHEVPQILINREPLPHLHFDVELLGDCDVIINELCHRLGGEYAKL

SEQ ID NO: 51 - protein, 2502 aa, synthetic construct
  REGION 1..2502: note = 1st fusion_DNMT3ACD-DNMT3LCD-dCas9-10xGCN4
MNHDQEFDPPKVYPPVPAEKRKPIRVLSLFDGIATGLLVLKDLGIQVDRYIASEVCEDSITVGMVRHQGKIMYVGDVRSVTQKHIQEWGPFDLVIGGSPCNDLSIVNPARKGLYEGTGRLFFEFYRLLHDARPKEGDDRPFFWLFENVVAMGVSDKRDISRFLESNPVMIDAKEVSAAHRARYFWGNLPGMNRPLASTVNDKLELQECLEHGRIAKFSKVRTITTRSNSIKQGKDQHFPVFMNEKEDILWCTEMERVFGFPVHYTDVSNMSRLARQRLLGRSWSVPVIRHLFAPLKEYFACVSSGNSNANSRGPSFSSGLVPLSLRGSHMGPMEIYKTVSAWKRQPVRVLSLFRNIDKVLKSLGFLESGSGSGGGTLKYVEDVTNVVRRDVEKWGPFDLVYGSTQPLGSSCDRCPGWYMFQFHRILQYALPRQESQRPFFWIFMDNLLLTEDDQETTTRFLQTEAVTLQDVRGRDYQNAMRVWSNIPGLKSKHAPLTPKEEEYLQAQVRSRSKLDAPKVDLLVKNCLLPLREYFKYFSQNSLPLGGPSSGAPPPSGGSPAGSPTSTEEGTSESATPESGPGTSTEPSEGSAPGSPAGSPTSTEEGTSTEPSEGSAPGTSTEPSEPKKKRKVMDKKYSIGLAIGTNSVGWAVITDEYKVPSKKFKVLGNTDRHSIKKNLIGALLFDSGETAEATRLKRTARRRYTRRKNRICYLQEIFSNEMAKVDDSFFHRLEESFLVEEDKKHERHPIFGNIVDEVAYHEKYPTIYHLRKKLVDSTDKADLRLIYLALAHMIKFRGHFLIEGDLNPDNSDVDKLFIQLVQTYNQLFEENPINASGVDAKAILSARLSKSRRLENLIAQLPGEKKNGLFGNLIALSLGLTPNFKSNFDLAEDAKLQLSKDTYDDDLDNLLAQIGDQYADLFLAAKNLSDAILLSDILRVNTEITKAPLSASMIKRYDEHHQDLTLLKALVRQQLPEKYKEIFFDQSKNGYAGYIDGGASQEEFYKFIKPILEKMDGTEELLVKLNREDLLRKQRTFDNGSIPHQIHLGELHAILRRQEDFYPFLKDNREKIEKILTFRIPYYVGPLARGNSRFAWMTRKSEETITPWNFEEVVDKGASAQSFIERMTNFDKNLPNEKVLPKHSLLYEYFTVYNELTKVKYVTEGMRKPAFLSGEQKKAIVDLLFKTNRKVTVKQLKEDYFKKIECFDSVEISGVEDRFNASLGTYHDLLKIIKDKDFLDNEENEDILEDIVLTLTLFEDREMIEERLKTYAHLFDDKVMKQLKRRRYTGWGRLSRKLINGIRDKQSGKTILDFLKSDGFANRNFMQLIHDDSLTFKEDIQKAQVSGQGDSLHEHIANLAGSPAIKKGILQTVKVVDELVKVMGRHKPENIVIEMARENQTTQKGQKNSRERMKRIEEGIKELGSQILKEHPVENTQLQNEKLYLYYLQNGRDMYVDQELDINRLSDYDVDAIVPQSFLKDDSIDNKVLTRSDKNRGKSDNVPSEEVVKKMKNYWRQLLNAKLITQRKFDNLTKAERGGLSELDKAGFIKRQLVETRQITKHVAQILDSRMNTKYDENDKLIREVKVITLKSKLVSDFRKDFQFYKVREINNYHHAHDAYLNAVVGTALIKKYPKLESEFVYGDYKVYDVRKMIAKSEQEIGKATAKYFFYSNIMNFFKTEITLANGEIRKRPLIETNGETGEIVWDKGRDFATVRKVLSMPQVNIVKKTEVQTGGFSKESILPKRNSDKLIARKKDWDPKKYGGFDSPTVAYSVLVVAKVEKGKSKKLKSVKELLGITIMERSSFEKNPIDFLEAKGYKEVKKDLIIKLPKYSLFELENGRKRMLASAGELQKGNELALPSKYVNFLYLASHYEKLKGSPEDNEQKQLFVEQHKHYLDEIIEQISEFSKRVILADANLDKVLSAYNKHRDKPIREQAENIIHLFTLTNLGAPAAFKYFDTTIDRKRYTSTKEVLDATLIHQSITGLYETRIDLSQLGGDYPYDVPDYASLGSGSPKKKRKVEDPKKKRKVDGIGSGSNGSSGEELLSKNYHLENEVARLKKGSGSGGSGSGGSGSGSGGSGSGGSGSGEELLSKNYHLENEVARLKKGSGSGGSGSGGSGSGSGGSGSGGSGSGEELLSKNYHLENEVARLKKGSGSGGSGSGGSGSGSGGSGSGGSGSGEELLSKNYHLENEVARLKKGSGSGGSGSGGSGSGSGGSGSGGSGSGEELLSKNYHLENEVARLKKGSGSGGSGSGGSGSGSGGSGSGGSGSGEELLSKNYHLENEVARLKKGSGSGGSGSGGSGSGSGGSGSGGSGSGEELLSKNYHLENEVARLKKGSGSGGSGSGGSGSGSGGSGSGGSGSGEELLSKNYHLENEVARLKKGSGSGGSGSGGSGSGSGGSGSGGSGSGEELLSKNYHLENEVARLKKGSGSGGSGSGGSGSGSGGSGSGGSGSGEELLSKNYHLENEVARLKKGSGSGQRGSKRTADGSEFESPKKKRKV

SEQ ID NO: 52 - protein, 370 aa, synthetic construct
  REGION 1..370: note = 2nd fusion_scFv-KRAB
MGPDIVMTQSPSSLSASVGDRVTITCRSSTGAVTTSNYASWVQEKPGKLFKGLIGGTNNRAPGVPSRFSGSLIGDKATLTISSLQPEDFATYFCALWYSNHWVFGQGTKVELKRGGGGSGGGGSGGGGSSGGGSEVKLLESGGGLVQPGGSLKLSCAVSGFSLTDYGVNWVRQAPGRGLEWIGVIWGDGITDYNSALKDRFIISKDNGKNTVYLQMSKVRSDDTALYYCVTGLFDYWGQGTLVTVSSYPYDVPDYAGGGGGSGGGGSGGGGSGGGGSSLDPGGGGSGRTLVTFKDVFVDFTREEWKLLDTAQQIVYRNVMLENYKNLVSLGYQLTKPDVILRLEKGEEPGSGKRTADGSEFESPKKKRKV

SEQ ID NO: 53 - protein, 370 aa, synthetic construct
  REGION 1..370: note = 2nd fusion_scFv-Zim3
MGPDIVMTQSPSSLSASVGDRVTITCRSSTGAVTTSNYASWVQEKPGKLFKGLIGGTNNRAPGVPSRFSGSLIGDKATLTISSLQPEDFATYFCALWYSNHWVFGQGTKVELKRGGGGSGGGGSGGGGSSGGGSEVKLLESGGGLVQPGGSLKLSCAVSGFSLTDYGVNWVRQAPGRGLEWIGVIWGDGITDYNSALKDRFIISKDNGKNTVYLQMSKVRSDDTALYYCVTGLFDYWGQGTLVTVSSYPYDVPDYAGGGGGSGGGGSGGGGSGGGGSSLDPGGGGSGVTFEDVTVNFTQGEWQRLNPEQRNLYRDVMLENYSNLVSVGQGETTKPDVILRLEQGKEPWLGSGKRTADGSEFESPKKKRKV

SEQ ID NO: 54 - protein, 369 aa, synthetic construct
  REGION 1..369: note = 2nd fusion_scFv-Znf680
MGPDIVMTQSPSSLSASVGDRVTITCRSSTGAVTTSNYASWVQEKPGKLFKGLIGGTNNRAPGVPSRFSGSLIGDKATLTISSLQPEDFATYFCALWYSNHWVFGQGTKVELKRGGGGSGGGGSGGGGSSGGGSEVKLLESGGGLVQPGGSLKLSCAVSGFSLTDYGVNWVRQAPGRGLEWIGVIWGDGITDYNSALKDRFIISKDNGKNTVYLQMSKVRSDDTALYYCVTGLFDYWGQGTLVTVSSYPYDVPDYAGGGGGSGGGGSGGGGSGGGGSSLDPGGGGSGLTFRDVAIEFSLEEWQCLDTAQRNLYRKVMFENYRNLVFLGIAVSKPHLITCLEQGKEPWNGSGKRTADGSEFESPKKKRKV

SEQ ID NO: 55 - protein, 370 aa, synthetic construct
  REGION 1..370: note = 2nd fusion_scFv-Znf554
MGPDIVMTQSPSSLSASVGDRVTITCRSSTGAVTTSNYASWVQEKPGKLFKGLIGGTNNRAPGVPSRFSGSLIGDKATLTISSLQPEDFATYFCALWYSNHWVFGQGTKVELKRGGGGSGGGGSGGGGSSGGGSEVKLLESGGGLVQPGGSLKLSCAVSGFSLTDYGVNWVRQAPGRGLEWIGVIWGDGITDYNSALKDRFIISKDNGKNTVYLQMSKVRSDDTALYYCVTGLFDYWGQGTLVTVSSYPYDVPDYAGGGGGSGGGGSGGGGSGGGGSSLDPGGGGSGVTFEDVSMDFSQEEWELLEPAQKNLYREVMLENYRNVVSLEALKNQCTDVGIKEGPLSPAQTGSGKRTADGSEFESPKKKRKV

SEQ ID NO: 56 - protein, 369 aa, synthetic construct
  REGION 1..369: note = 2nd fusion_scFv-Znf264
MGPDIVMTQSPSSLSASVGDRVTITCRSSTGAVTTSNYASWVQEKPGKLFKGLIGGTNNRAPGVPSRFSGSLIGDKATLTISSLQPEDFATYFCALWYSNHWVFGQGTKVELKRGGGGSGGGGSGGGGSSGGGSEVKLLESGGGLVQPGGSLKLSCAVSGFSLTDYGVNWVRQAPGRGLEWIGVIWGDGITDYNSALKDRFIISKDNGKNTVYLQMSKVRSDDTALYYCVTGLFDYWGQGTLVTVSSYPYDVPDYAGGGGGSGGGGSGGGGSGGGGSSLDPGGGGSGVTFDDVAVTFTKEEWGQLDLAQRTLYQEVMLENCGLLVSLGCPVPKAELICHLEHGQEPWTGSGKRTADGSEFESPKKKRKV

SEQ ID NO: 57 - protein, 369 aa, synthetic construct
  REGION 1..369: note = 2nd fusion_scFv-Znf582
MGPDIVMTQSPSSLSASVGDRVTITCRSSTGAVTTSNYASWVQEKPGKLFKGLIGGTNNRAPGVPSRFSGSLIGDKATLTISSLQPEDFATYFCALWYSNHWVFGQGTKVELKRGGGGSGGGGSGGGGSSGGGSEVKLLESGGGLVQPGGSLKLSCAVSGFSLTDYGVNWVRQAPGRGLEWIGVIWGDGITDYNSALKDRFIISKDNGKNTVYLQMSKVRSDDTALYYCVTGLFDYWGQGTLVTVSSYPYDVPDYAGGGGGSGGGGSGGGGSGGGGSSLDPGGGGSGELFRDVAIVFSQEEWQWLAPAQRDLYRDVMLETYSNLVSLGLAVSKPDVISFLEQGKEPWMGSGKRTADGSEFESPKKKRKV

SEQ ID NO: 58 - protein, 369 aa, synthetic construct
  REGION 1..369: note = 2nd fusion_scFv-Znf324
MGPDIVMTQSPSSLSASVGDRVTITCRSSTGAVTTSNYASWVQEKPGKLFKGLIGGTNNRAPGVPSRFSGSLIGDKATLTISSLQPEDFATYFCALWYSNHWVFGQGTKVELKRGGGGSGGGGSGGGGSSGGGSEVKLLESGGGLVQPGGSLKLSCAVSGFSLTDYGVNWVRQAPGRGLEWIGVIWGDGITDYNSALKDRFIISKDNGKNTVYLQMSKVRSDDTALYYCVTGLFDYWGQGTLVTVSSYPYDVPDYAGGGGGSGGGGSGGGGSGGGGSSLDPGGGGSGMAFEDVAVYFSQEEWGLLDTAQRALYRRVMLDNFALVASLGLSTSRPRVVIQLERGEEPWVGSGKRTADGSEFESPKKKRKV

SEQ ID NO: 59 - protein, 370 aa, synthetic construct
  REGION 1..370: note = 2nd fusion_scFv-Znf669
MGPDIVMTQSPSSLSASVGDRVTITCRSSTGAVTTSNYASWVQEKPGKLFKGLIGGTNNRAPGVPSRFSGSLIGDKATLTISSLQPEDFATYFCALWYSNHWVFGQGTKVELKRGGGGSGGGGSGGGGSSGGGSEVKLLESGGGLVQPGGSLKLSCAVSGFSLTDYGVNWVRQAPGRGLEWIGVIWGDGITDYNSALKDRFIISKDNGKNTVYLQMSKVRSDDTALYYCVTGLFDYWGQGTLVTVSSYPYDVPDYAGGGGGSGGGGSGGGGSGGGGSSLDPGGGGSGVAFEDVAVNFTQEEWALLDSSQKNLYREVMQETCRNLASVGSQWKDQNIEDHFEKPGKDIRNGSGKRTADGSEFESPKKKRKV

SEQ ID NO: 60 - protein, 369 aa, synthetic construct
  REGION 1..369: note = 2nd fusion_scFv-Znf354a
MGPDIVMTQSPSSLSASVGDRVTITCRSSTGAVTTSNYASWVQEKPGKLFKGLIGGTNNRAPGVPSRFSGSLIGDKATLTISSLQPEDFATYFCALWYSNHWVFGQGTKVELKRGGGGSGGGGSGGGGSSGGGSEVKLLESGGGLVQPGGSLKLSCAVSGFSLTDYGVNWVRQAPGRGLEWIGVIWGDGITDYNSALKDRFIISKDNGKNTVYLQMSKVRSDDTALYYCVTGLFDYWGQGTLVTVSSYPYDVPDYAGGGGGSGGGGSGGGGSGGGGSSLDPGGGGSGLTFEDVAVLFTRDEWRKLAPSQRNLYRDVMLENYRNLVSLGLPFTKPKVISLLQQGEDPWEGSGKRTADGSEFESPKKKRKV

SEQ ID NO: 61 - protein, 369 aa, synthetic construct
  REGION 1..369: note = 2nd fusion_scFv-Znf82
MGPDIVMTQSPSSLSASVGDRVTITCRSSTGAVTTSNYASWVQEKPGKLFKGLIGGTNNRAPGVPSRFSGSLIGDKATLTISSLQPEDFATYFCALWYSNHWVFGQGTKVELKRGGGGSGGGGSGGGGSSGGGSEVKLLESGGGLVQPGGSLKLSCAVSGFSLTDYGVNWVRQAPGRGLEWIGVIWGDGITDYNSALKDRFIISKDNGKNTVYLQMSKVRSDDTALYYCVTGLFDYWGQGTLVTVSSYPYDVPDYAGGGGGSGGGGSGGGGSGGGGSSLDPGGGGSGVMFSDVSIDFSPEEWEYLDLEQKDLYRDVMLENYSNLVSLGCFISKPDVISSLEQGKEPWKGSGKRTADGSEFESPKKKRKV

SEQ ID NO: 62 - protein, 369 aa, synthetic construct
  REGION 1..369: note = 2nd fusion_scFv-Znf595
MGPDIVMTQSPSSLSASVGDRVTITCRSSTGAVTTSNYASWVQEKPGKLFKGLIGGTNNRAPGVPSRFSGSLIGDKATLTISSLQPEDFATYFCALWYSNHWVFGQGTKVELKRGGGGSGGGGSGGGGSSGGGSEVKLLESGGGLVQPGGSLKLSCAVSGFSLTDYGVNWVRQAPGRGLEWIGVIWGDGITDYNSALKDRFIISKDNGKNTVYLQMSKVRSDDTALYYCVTGLFDYWGQGTLVTVSSYPYDVPDYAGGGGGSGGGGSGGGGSGGGGSSLDPGGGGSGVTFRDVAIEFSPEEWKCLDPAQQNLYRDVMLENYRNLVSLGFVISNPDLVTCLEQIKEPCNGSGKRTADGSEFESPKKKRKV

SEQ ID NO: 63 - protein, 369 aa, synthetic construct
  REGION 1..369: note = 2nd fusion_scFv-Znf419
MGPDIVMTQSPSSLSASVGDRVTITCRSSTGAVTTSNYASWVQEKPGKLFKGLIGGTNNRAPGVPSRFSGSLIGDKATLTISSLQPEDFATYFCALWYSNHWVFGQGTKVELKRGGGGSGGGGSGGGGSSGGGSEVKLLESGGGLVQPGGSLKLSCAVSGFSLTDYGVNWVRQAPGRGLEWIGVIWGDGITDYNSALKDRFIISKDNGKNTVYLQMSKVRSDDTALYYCVTGLFDYWGQGTLVTVSSYPYDVPDYAGGGGGSGGGGSGGGGSGGGGSSLDPGGGGSGVTFEDVAVYFSQEEWRLLDDAQRLLYRNVMLENFTLLASLGLASSKTHEITQLESWEEPFMGSGKRTADGSEFESPKKKRKV

SEQ ID NO: 64 - protein, 369 aa, synthetic construct
  REGION 1..369: note = 2nd fusion_scFv-Znf566
MGPDIVMTQSPSSLSASVGDRVTITCRSSTGAVTTSNYASWVQEKPGKLFKGLIGGTNNRAPGVPSRFSGSLIGDKATLTISSLQPEDFATYFCALWYSNHWVFGQGTKVELKRGGGGSGGGGSGGGGSSGGGSEVKLLESGGGLVQPGGSLKLSCAVSGFSLTDYGVNWVRQAPGRGLEWIGVIWGDGITDYNSALKDRFIISKDNGKNTVYLQMSKVRSDDTALYYCVTGLFDYWGQGTLVTVSSYPYDVPDYAGGGGGSGGGGSGGGGSGGGGSSLDPGGGGSGVMFSDVSVDFSQEEWECLNDDQRDLYRDVMLENYSNLVSMGHSISKPNVISYLEQGKEPWLGSGKRTADGSEFESPKKKRKV

SEQ ID NO: 65 - protein, 369 aa, synthetic construct
  REGION 1..369: note = 2nd fusion_scFv-Zim2
MGPDIVMTQSPSSLSASVGDRVTITCRSSTGAVTTSNYASWVQEKPGKLFKGLIGGTNNRAPGVPSRFSGSLIGDKATLTISSLQPEDFATYFCALWYSNHWVFGQGTKVELKRGGGGSGGGGSGGGGSSGGGSEVKLLESGGGLVQPGGSLKLSCAVSGFSLTDYGVNWVRQAPGRGLEWIGVIWGDGITDYNSALKDRFIISKDNGKNTVYLQMSKVRSDDTALYYCVTGLFDYWGQGTLVTVSSYPYDVPDYAGGGGGSGGGGSGGGGSGGGGSSLDPGGGGSGVTFEDVLVDFSPEELSSLSAAQRNLYREVMLENYRNLVSLGHQFSKPDIISRLEEEESYAMGSGKRTADGSEFESPKKKRKV

SEQ ID NO: 66 - protein, 691 aa, synthetic construct
  REGION 1..691: note = 2nd fusion_scFv-EHMT2(G9A)
MGPDIVMTQSPSSLSASVGDRVTITCRSSTGAVTTSNYASWVQEKPGKLFKGLIGGTNNRAPGVPSRFSGSLIGDKATLTISSLQPEDFATYFCALWYSNHWVFGQGTKVELKRGGGGSGGGGSGGGGSSGGGSEVKLLESGGGLVQPGGSLKLSCAVSGFSLTDYGVNWVRQAPGRGLEWIGVIWGDGITDYNSALKDRFIISKDNGKNTVYLQMSKVRSDDTALYYCVTGLFDYWGQGTLVTVSSYPYDVPDYAGGGGGSGGGGSGGGGSGGGGSSLDPGGGGSGTGSAAIAEVLLNARCDLHAVNYHGDTPLHIAARESYHDCVLLFLSRGANPELRNKEGDTAWDLTPERSDVWFALQLNRKLRLGVGNRAIRTEKIICRDVARGYENVPIPCVNGVDGEPCPEDYKYISENCETSTMNIDRNITHLQHCTCVDDCSSSNCLCGQLSIRCWYDKDGRLLQEFNKIEPPLIFECNQACSCWRNCKNRVVQSGIKVRLQLYRTAKMGWGVRALQTIPQGTFICEYVGELISDAEADVREDDSYLFDLDNKDGEVYCIDARYYGNISRFINHLCDPNIIPVRVFMLHQDLRFPRIAFFSSRDIRTGEELGFDYGDRFWDIKSKYFTCQCGSEKCKHSAEAIALEQSRLARLDPHPELLPELGSLPPVNTGSGKRTADGSEFESPKKKRKV

SEQ ID NO: 67 - protein, 719 aa, synthetic construct
  REGION 1..719: note = 2nd fusion_scFv-SUV39H1
MGPDIVMTQSPSSLSASVGDRVTITCRSSTGAVTTSNYASWVQEKPGKLFKGLIGGTNNRAPGVPSRFSGSLIGDKATLTISSLQPEDFATYFCALWYSNHWVFGQGTKVELKRGGGGSGGGGSGGGGSSGGGSEVKLLESGGGLVQPGGSLKLSCAVSGFSLTDYGVNWVRQAPGRGLEWIGVIWGDGITDYNSALKDRFIISKDNGKNTVYLQMSKVRSDDTALYYCVTGLFDYWGQGTLVTVSSYPYDVPDYAGGGGGSGGGGSGGGGSGGGGSSLDPGGGGSGAENLKGCSVCCKSSWNQLQDLCRLAKLSCPALGISKRNLYDFEVEYLCDYKKIREQEYYLVKWRGYPDSESTWEPRQNLKCVRILKQFHKDLERELLRRHHRSKTPRHLDPSLANYLVQKAKQRRALRRWEQELNAKRSHLGRITVENEVDLDGPPRAFVYINEYRVGEGITLNQVAVGCECQDCLWAPTGGCCPGASLHKFAYNDQGQVRLRAGLPIYECNSRCRCGYDCPNRVVQKGIRYDLCIFRTDDGRGWGVRTLEKIRKNSFVMEYVGEIITSEEAERRGQIYDRQGATYLFDLDYVEDVYTVDAAYYGNISHFVNHSCDPNLQVYNVFIDNLDERLPRIAFFATRTIRAGEELTFDYNMQVDPVDMESTRMDSNFGLAGLPGSPKKRVRIECKCGTESCRKYLFGSGKRTADGSEFESPKKKRKV

SEQ ID NO: 68 - protein, 355 aa, synthetic construct
  REGION 1..355: note = 2nd fusion_scFv-ZFPM1(FOG)
MGPDIVMTQSPSSLSASVGDRVTITCRSSTGAVTTSNYASWVQEKPGKLFKGLIGGTNNRAPGVPSRFSGSLIGDKATLTISSLQPEDFATYFCALWYSNHWVFGQGTKVELKRGGGGSGGGGSGGGGSSGGGSEVKLLESGGGLVQPGGSLKLSCAVSGFSLTDYGVNWVRQAPGRGLEWIGVIWGDGITDYNSALKDRFIISKDNGKNTVYLQMSKVRSDDTALYYCVTGLFDYWGQGTLVTVSSYPYDVPDYAGGGGGSGGGGSGGGGSGGGGSSLDPGGGGSGSRRKQSNPRQIKRSLGDMEAREEVQLVGASHMEQKATAPEAPSPPSAGSGKRTADGSEFESPKKKRKV

SEQ ID NO: 69 - protein, 1142 aa, synthetic construct
  REGION 1..1142: note = 2nd fusion_scFv-TRIM28(KAP1)
MGPDIVMTQSPSSLSASVGDRVTITCRSSTGAVTTSNYASWVQEKPGKLFKGLIGGTNNRAPGVPSRFSGSLIGDKATLTISSLQPEDFATYFCALWYSNHWVFGQGTKVELKRGGGGSGGGGSGGGGSSGGGSEVKLLESGGGLVQPGGSLKLSCAVSGFSLTDYGVNWVRQAPGRGLEWIGVIWGDGITDYNSALKDRFIISKDNGKNTVYLQMSKVRSDDTALYYCVTGLFDYWGQGTLVTVSSYPYDVPDYAGGGGGSGGGGSGGGGSGGGGSSLDPGGGGSGAASAAAASAAAASAASGSPGPGEGSAGGEKRSTAPSAAASASASAAASSPAGGGAEALELLEHCGVCRERLRPEREPRLLPCLHSACSACLGPAAPAAANSSGDGGAAGDGTVVDCPVCKQQCFSKDIVENYFMRDSGSKAATDAQDANQCCTSCEDNAPATSYCVECSEPLCETCVEAHQRVKYTKDHTVRSTGPAKSRDGERTVYCNVHKHEPLVLFCESCDTLTCRDCQLNAHKDHQYQFLEDAVRNQRKLLASLVKRLGDKHATLQKSTKEVRSSIRQVSDVQKRVQVDVKMAILQIMKELNKRGRVLVNDAQKVTEGQQERLERQHWTMTKIQKHQEHILRFASWALESDNNTALLLSKKLIYFQLHRALKMIVDPVEPHGEMKFQWDLNAWTKSAEAFGKIVAERPGTNSTGPAPMAPPRAPGPLSKQGSGSSQPMEVQEGYGFGSGDDPYSSAEPHVSGVKRSRSGEGEVSGLMRKVPRVSLERLDLDLTADSQPPVFKVFPGSTTEDYNLIVIERGAAAAATGQPGTAPAGTPGAPPLAGMAIVKEEETEAAIGAPPTATEGPETKPVLMALAEGPGAEGPRLASPSGSTSSGLEVVAPEGTSAPGGGPGTLDDSATICRVCQKPGDLVMCNQCEFCFHLDCHLPALQDVPGEEWSCSLCHVLPDLKEEDGSLSLDGADSTGVVAKLSPANQRKCERVLLALFCHEPCRPLHQLATDSTFSLDQPGGTLDLTLIRARLQEKLSPPYSSPQEFAQDVGRMFKQFNKLTEDKADVQSIIGLQRFFETRMNEAFGDTKFSAVLVEPPPMSLPGAGLSSQELSGGPGDGPGSGKRTADGSEFESPKKKRKV

SEQ ID NO: 70 - protein, 1053 aa, synthetic construct
  REGION 1..1053: note = 2nd fusion_scFv-EZH2
MGPDIVMTQSPSSLSASVGDRVTITCRSSTGAVTTSNYASWVQEKPGKLFKGLIGGTNNRAPGVPSRFSGSLIGDKATLTISSLQPEDFATYFCALWYSNHWVFGQGTKVELKRGGGGSGGGGSGGGGSSGGGSEVKLLESGGGLVQPGGSLKLSCAVSGFSLTDYGVNWVRQAPGRGLEWIGVIWGDGITDYNSALKDRFIISKDNGKNTVYLQMSKVRSDDTALYYCVTGLFDYWGQGTLVTVSSYPYDVPDYAGGGGGSGGGGSGGGGSGGGGSSLDPGGGGSGGQTGKKSEKGPVCWRKRVKSEYMRLRQLKRFRRADEVKSMFSSNRQKILERTEILNQEWKQRRIQPVHILTSVSSLRGTRECSVTSDLDFPTQVIPLKTLNAVASVPIMYSWSPLQQNFMVEDETVLHNIPYMGDEVLDQDGTFIEELIKNYDGKVHGDRECGFINDEIFVELVNALGQYNDDDDDDDGDDPEEREEKQKDLEDHRDDKESRPPRKFPSDKIFEAISSMFPDKGTAEELKEKYKELTEQQLPGALPPECTPNIDGPNAKSVQREQSLHSFHTLFCRRCFKYDCFLHPFHATPNTYKRKNTETALDNKPCGPQCYQHLEGAKEFAAALTAERIKTPPKRPGGRRRGRLPNNSSRPSTPTINVLESKDTDSDREAGTETGGENNDKEEEEKKDETSSSSEANSRCQTPIKMKPNIEPPENVEWSGAEASMFRVLIGTYYDNFCAIARLIGTKTCRQVYEFRVKESSIIAPAPAEDVDTPPRKKKRKHRLWAAHCRKIQLKKDGSSNHVYNYQPCDHPRQPCDSSCPCVIAQNFCEKFCQCSSECQNRFPGCRCKAQCNTKQCPCYLAVRECDPDLCLTCGAADHWDSKNVSCKNCSIQRGSKKHLLLAPSDVAGWGIFIKDPVQKNEFISEYCGEIISQDEADRRGKVYDKYMCSFLFNLNNDFVVDATRKGNKIRFANHSVNPNCYAKVMMVNGDHRIGIFAKRAIQTGEELFFDYRYSQADALKYVGIEREMEIPGSGKRTADGSEFESPKKKRKV

SEQ ID NO: 71 - protein, 527 aa, synthetic construct
  REGION 1..527: note = 2nd fusion_scFv-MXD1(SID FL)
MGPDIVMTQSPSSLSASVGDRVTITCRSSTGAVTTSNYASWVQEKPGKLFKGLIGGTNNRAPGVPSRFSGSLIGDKATLTISSLQPEDFATYFCALWYSNHWVFGQGTKVELKRGGGGSGGGGSGGGGSSGGGSEVKLLESGGGLVQPGGSLKLSCAVSGFSLTDYGVNWVRQAPGRGLEWIGVIWGDGITDYNSALKDRFIISKDNGKNTVYLQMSKVRSDDTALYYCVTGLFDYWGQGTLVTVSSYPYDVPDYAGGGGGSGGGGSGGGGSGGGGSSLDPGGGGSGAAAVRMNIQMLLEAADYLERREREAEHGYASMLPYNNKDRDALKRRNKSKKNNSSSRSTHNEMEKNRRAHLRLCLEKLKGLVPLGPESSRHTTLSLLTKAKLHIKKLEDCDRKAVHQIDQLQREQRHLKRQLEKLGIERIRMDSIGSTVSSERSDSDREIDVDVESTDYLTGDLDWSSSSVSDSDERGSMQSLGSDEGYSSTSIKRIKLQDSHKACLGLGSGKRTADGSEFESPKKKRKV

SEQ ID NO: 72 - protein, 337 aa, synthetic construct
  REGION 1..337: note = 2nd fusion_scFv-SID
MGPDIVMTQSPSSLSASVGDRVTITCRSSTGAVTTSNYASWVQEKPGKLFKGLIGGTNNRAPGVPSRFSGSLIGDKATLTISSLQPEDFATYFCALWYSNHWVFGQGTKVELKRGGGGSGGGGSGGGGSSGGGSEVKLLESGGGLVQPGGSLKLSCAVSGFSLTDYGVNWVRQAPGRGLEWIGVIWGDGITDYNSALKDRFIISKDNGKNTVYLQMSKVRSDDTALYYCVTGLFDYWGQGTLVTVSSYPYDVPDYAGGGGGSGGGGSGGGGSGGGGSSLDPGGGGSGMNIQMLLEAADYLERREREAEHGYASMLPGSGKRTADGSEFESPKKKRKV

SEQ ID NO: 73 - protein, 1183 aa, synthetic construct
  REGION 1..1183: note = 2nd fusion_scFv-LSD1(KDMA1)
MGPDIVMTQSPSSLSASVGDRVTITCRSSTGAVTTSNYASWVQEKPGKLFKGLIGGTNNRAPGVPSRFSGSLIGDKATLTISSLQPEDFATYFCALWYSNHWVFGQGTKVELKRGGGGSGGGGSGGGGSSGGGSEVKLLESGGGLVQPGGSLKLSCAVSGFSLTDYGVNWVRQAPGRGLEWIGVIWGDGITDYNSALKDRFIISKDNGKNTVYLQMSKVRSDDTALYYCVTGLFDYWGQGTLVTVSSYPYDVPDYAGGGGGSGGGGSGGGGSGGGGSSLDPGGGGSGLSGKKAAAAAAAAAAAATGTEAGPGTAGGSENGSEVAAQPAGLSGPAEVGPGAVGERTPRKKEPPRASPPGGLAEPPGSAGPQAGPTVVPGSATPMETGIAETPEGRRTSRRKRAKVEYREMDESLANLSEDEYYSEEERNAKAEKEKKLPPPPPQAPPEEENESEPEEPSGQAGGLQDDSSGGYGDGQASGVEGAAFQSRLPHDRMTSQEAACFPDIISGPQQTQKVFLFIRNRTLQLWLDNPKIQLTFEATLQQLEAPYNSDTVLVHRVHSYLERHGLINFGIYKRIKPLPTKKTGKVIIIGSGVSGLAAARQLQSFGMDVTLLEARDRVGGRVATFRKGNYVADLGAMVVTGLGGNPMAVVSKQVNMELAKIKQKCPLYEANGQADTVKVPKEKDEMVEQEFNRLLEATSYLSHQLDFNVLNNKPVSLGQALEVVIQLQEKHVKDEQIEHWKKIVKTQEELKELLNKMVNLKEKIKELHQQYKEASEVKPPRDITAEFLVKSKHRDLTALCKEYDELAETQGKLEEKLQELEANPPSDVYLSSRDRQILDWHFANLEFANATPLSTLSLKHWDQDDDFEFTGSHLTVRNGYSCVPVALAEGLDIKLNTAVRQVRYTASGCEVIAVNTRSTSQTFIYKCDAVLCTLPLGVLKQQPPAVQFVPPLPEWKTSAVQRMGFGNLNKVVLCFDRVFWDPSVNLFGHVGSTTASRGELFLFWNLYKAPILLALVAGEAAGIMENISDDVIVGRCLAILKGIFGSSAVPQPKETVVSRWRADPWARGSYSYVAAGSSGNDYDLMAQPITPGPSIPGAPQPIPRLFFAGEHTIRNYPATVHGALLSGLREAGRIADQFLGAMYTLPRQATPGVPAQQSPSMGSGKRTADGSEFESPKKKRKV

SEQ ID NO: 74 - protein, 498 aa, synthetic construct
  REGION 1..498: note = 2nd fusion_scFv-HP1a long
MGPDIVMTQSPSSLSASVGDRVTITCRSSTGAVTTSNYASWVQEKPGKLFKGLIGGTNNRAPGVPSRFSGSLIGDKATLTISSLQPEDFATYFCALWYSNHWVFGQGTKVELKRGGGGSGGGGSGGGGSSGGGSEVKLLESGGGLVQPGGSLKLSCAVSGFSLTDYGVNWVRQAPGRGLEWIGVIWGDGITDYNSALKDRFIISKDNGKNTVYLQMSKVRSDDTALYYCVTGLFDYWGQGTLVTVSSYPYDVPDYAGGGGGSGGGGSGGGGSGGGGSSLDPGGGGSGGKKTKRTADSSSSEDEEEYVVEKVLDRRVVKGQVEYLLKWKGFSEEHNTWEPEKNLDCPELISEFMKKYKKMKEGENNKPREKSESNKRKSNFSNSADDIKSKKKREQSNDIARGFERGLEPEKIIGATDSCGDLMFLMKWKDTDEADLVLAKEANVKCPQIVIAFYEERLTWHAYPEDAENKEKETAKSGSGKRTADGSEFESPKKKRKV

SEQ ID NO: 75 - protein, 427 aa, synthetic construct
  REGION 1..427: note = 2nd fusion_scFv-HP1a short
MGPDIVMTQSPSSLSASVGDRVTITCRSSTGAVTTSNYASWVQEKPGKLFKGLIGGTNNRAPGVPSRFSGSLIGDKATLTISSLQPEDFATYFCALWYSNHWVFGQGTKVELKRGGGGSGGGGSGGGGSSGGGSEVKLLESGGGLVQPGGSLKLSCAVSGFSLTDYGVNWVRQAPGRGLEWIGVIWGDGITDYNSALKDRFIISKDNGKNTVYLQMSKVRSDDTALYYCVTGLFDYWGQGTLVTVSSYPYDVPDYAGGGGGSGGGGSGGGGSGGGGSSLDPGGGGSGMKEGENNKPREKSESNKRKSNFSNSADDIKSKKKREQSNDIARGFERGLEPEKIIGATDSCGDLMFLMKWKDTDEADLVLAKEANVKCPQIVIAFYEERLTWHAYPEDAENKEKETAKSGSGKRTADGSEFESPKKKRKV

SEQ ID NO: 76 - protein, 735 aa, synthetic construct
  REGION 1..735: note = 2nd fusion_scFv-HDAC3
MGPDIVMTQSPSSLSASVGDRVTITCRSSTGAVTTSNYASWVQEKPGKLFKGLIGGTNNRAPGVPSRFSGSLIGDKATLTISSLQPEDFATYFCALWYSNHWVFGQGTKVELKRGGGGSGGGGSGGGGSSGGGSEVKLLESGGGLVQPGGSLKLSCAVSGFSLTDYGVNWVRQAPGRGLEWIGVIWGDGITDYNSALKDRFIISKDNGKNTVYLQMSKVRSDDTALYYCVTGLFDYWGQGTLVTVSSYPYDVPDYAGGGGGSGGGGSGGGGSGGGGSSLDPGGGGSGAKTVAYFYDPDVGNFHYGAGHPMKPHRLALTHSLVLHYGLYKKMIVFKPYQASQHDMCRFHSEDYIDFLQRVSPTNMQGFTKSLNAFNVGDDCPVFPGLFEFCSRYTGASLQGATQLNNKICDIAINWAGGLHHAKKFEASGFCYVNDIVIGILELLKYHPRVLYIDIDIHHGDGVQEAFYLTDRVMTVSFHKYGNYFFPGTGDMYEVGAESGRYYCLNVPLRDGIDDQSYKHLFQPVINQVVDFYQPTCIVLQCGADSLGCDRLGCFNLSIRGHGECVEYVKSFNIPLLVLGGGGYTVRNVARCWTYETSLLVEEAISEELPYSEYFEYFAPDFTLHPDVSTRIENQNSRQYLDQIRQTIFENLKMLNHAPSVQIHDVPADLLTYDRTDEADAEERGPEENYSRPEAPNEFYDGDHDNDKESDVEIGSGKRTADGSEFESPKKKRKV

SEQ ID NO: 77 - protein, 1725 aa, synthetic construct
  REGION 1..1725: note = V1 fusion_3xGCN4-dCas9-3xGCN4
  SITE 1725: note = misc_feature - Xaa =
MPAAKRVKLDGSEELLSKNYHLENEVARLKKGSGSGGSGSGGSGSGSGGSGSGGSGSGEELLSKNYHLENEVARLKKGSGSGGSGSGGSGSGSGGSGSGGSGSGEELLSKNYHLENEVARLKKGSGSGGSGSGGSGSGSGGSGSGGSGSGPKKKRKVMDKKYSIGLAIGTNSVGWAVITDEYKVPSKKFKVLGNTDRHSIKKNLIGALLFDSGETAEATRLKRTARRRYTRRKNRICYLQEIFSNEMAKVDDSFFHRLEESFLVEEDKKHERHPIFGNIVDEVAYHEKYPTIYHLRKKLVDSTDKADLRLIYLALAHMIKFRGHFLIEGDLNPDNSDVDKLFIQLVQTYNQLFEENPINASGVDAKAILSARLSKSRRLENLIAQLPGEKKNGLFGNLIALSLGLTPNFKSNFDLAEDAKLQLSKDTYDDDLDNLLAQIGDQYADLFLAAKNLSDAILLSDILRVNTEITKAPLSASMIKRYDEHHQDLTLLKALVRQQLPEKYKEIFFDQSKNGYAGYIDGGASQEEFYKFIKPILEKMDGTEELLVKLNREDLLRKQRTFDNGSIPHQIHLGELHAILRRQEDFYPFLKDNREKIEKILTFRIPYYVGPLARGNSRFAWMTRKSEETITPWNFEEVVDKGASAQSFIERMTNFDKNLPNEKVLPKHSLLYEYFTVYNELTKVKYVTEGMRKPAFLSGEQKKAIVDLLFKTNRKVTVKQLKEDYFKKIECFDSVEISGVEDRFNASLGTYHDLLKIIKDKDFLDNEENEDILEDIVLTLTLFEDREMIEERLKTYAHLFDDKVMKQLKRRRYTGWGRLSRKLINGIRDKQSGKTILDFLKSDGFANRNFMQLIHDDSLTFKEDIQKAQVSGQGDSLHEHIANLAGSPAIKKGILQTVKVVDELVKVMGRHKPENIVIEMARENQTTQKGQKNSRERMKRIEEGIKELGSQILKEHPVENTQLQNEKLYLYYLQNGRDMYVDQELDINRLSDYDVDAIVPQSFLKDDSIDNKVLTRSDKNRGKSDNVPSEEVVKKMKNYWRQLLNAKLITQRKFDNLTKAERGGLSELDKAGFIKRQLVETRQITKHVAQILDSRMNTKYDENDKLIREVKVITLKSKLVSDFRKDFQFYKVREINNYHHAHDAYLNAVVGTALIKKYPKLESEFVYGDYKVYDVRKMIAKSEQEIGKATAKYFFYSNIMNFFKTEITLANGEIRKRPLIETNGETGEIVWDKGRDFATVRKVLSMPQVNIVKKTEVQTGGFSKESILPKRNSDKLIARKKDWDPKKYGGFDSPTVAYSVLVVAKVEKGKSKKLKSVKELLGITIMERSSFEKNPIDFLEAKGYKEVKKDLIIKLPKYSLFELENGRKRMLASAGELQKGNELALPSKYVNFLYLASHYEKLKGSPEDNEQKQLFVEQHKHYLDEIIEQISEFSKRVILADANLDKVLSAYNKHRDKPIREQAENIIHLFTLTNLGAPAAFKYFDTTIDRKRYTSTKEVLDATLIHQSITGLYETRIDLSQLGGDAYPYDVPDYASLGSGSPKKKRKVEDPKKKRKVDGSGSETPGTSGGSGSGSGGSGSGGSGSGEELLSKNYHLENEVARLKKGSGSGGSGSGGSGSGSGGSGSGGSGSGEELLSKNYHLENEVARLKKGSGSGGSGSGGSGSGSGGSGSGGSGSGEELLSKNYHLENEVARLKKGSGSGQRGSKRTADGSEFESPKKKRKVX

SEQ ID NO: 78 - protein, 360 aa, synthetic construct
  REGION 1..360: note = V2 fusion_scFv-KRAB
  SITE 360: note = misc_feature - Xaa =
MPAAKRVKLDGSGPDIVMTQSPSSLSASVGDRVTITCRSSTGAVTTSNYASWVQEKPGKLFKGLIGGTNNRAPGVPSRFSGSLIGDKATLTISSLQPEDFATYFCALWYSNHWVFGQGTKVELKRGGGGSGGGGSGGGGSSGGGSEVKLLESGGGLVQPGGSLKLSCAVSGFSLTDYGVNWVRQAPGRGLEWIGVIWGDGITDYNSALKDRFIISKDNGKNTVYLQMSKVRSDDTALYYCVTGLFDYWGQGTLVTVSSYPYDVPDYAGGGGGSGGGGSGGGGSGGGGSLDPGGGGSGRTLVTFKDVFVDFTREEWKLLDTAQQIVYRNVMLENYKNLVSLGYQLTKPDVILRLEKGEEPX

SEQ ID NO: 79 - protein, 2137 aa, synthetic construct
  REGION 1..2137: note = V3 fusion_D3a-D3l-dCas9-1xGCN4
  SITE 2137: note = misc_feature - Xaa =
MPAAKRVKLDGSNHDQEFDPPKVYPPVPAEKRKPIRVLSLFDGIATGLLVLKDLGIQVDRYIASEVCEDSITVGMVRHQGKIMYVGDVRSVTQKHIQEWGPFDLVIGGSPCNDLSIVNPARKGLYEGTGRLFFEFYRLLHDARPKEGDDRPFFWLFENVVAMGVSDKRDISRFLESNPVMIDAKEVSAAHRARYFWGNLPGMNRPLASTVNDKLELQECLEHGRIAKFSKVRTITTRSNSIKQGKDQHFPVFMNEKEDILWCTEMERVFGFPVHYTDVSNMSRLARQRLLGRSWSVPVIRHLFAPLKEYFACVSSGNSNANSRGPSFSSGLVPLSLRGSHMGPMEIYKTVSAWKRQPVRVLSLFRNIDKVLKSLGFLESGSGSGGGTLKYVEDVTNVVRRDVEKWGPFDLVYGSTQPLGSSCDRCPGWYMFQFHRILQYALPRQESQRPFFWIFMDNLLLTEDDQETTTRFLQTEAVTLQDVRGRDYQNAMRVWSNIPGLKSKHAPLTPKEEEYLQAQVRSRSKLDAPKVDLLVKNCLLPLREYFKYFSQNSLPLGGPSSGAPPPSGGSPAGSPTSTEEGTSESATPESGPGTSTEPSEGSAPGSPAGSPTSTEEGTSTEPSEGSAPGTSTEPSEPKKKRKVMDKKYSIGLAIGTNSVGWAVITDEYKVPSKKFKVLGNTDRHSIKKNLIGALLFDSGETAEATRLKRTARRRYTRRKNRICYLQEIFSNEMAKVDDSFFHRLEESFLVEEDKKHERHPIFGNIVDEVAYHEKYPTIYHLRKKLVDSTDKADLRLIYLALAHMIKFRGHFLIEGDLNPDNSDVDKLFIQLVQTYNQLFEENPINASGVDAKAILSARLSKSRRLENLIAQLPGEKKNGLFGNLIALSLGLTPNFKSNFDLAEDAKLQLSKDTYDDDLDNLLAQIGDQYADLFLAAKNLSDAILLSDILRVNTEITKAPLSASMIKRYDEHHQDLTLLKALVRQQLPEKYKEIFFDQSKNGYAGYIDGGASQEEFYKFIKPILEKMDGTEELLVKLNREDLLRKQRTFDNGSIPHQIHLGELHAILRRQEDFYPFLKDNREKIEKILTFRIPYYVGPLARGNSRFAWMTRKSEETITPWNFEEVVDKGASAQSFIERMTNFDKNLPNEKVLPKHSLLYEYFTVYNELTKVKYVTEGMRKPAFLSGEQKKAIVDLLFKTNRKVTVKQLKEDYFKKIECFDSVEISGVEDRFNASLGTYHDLLKIIKDKDFLDNEENEDILEDIVLTLTLFEDREMIEERLKTYAHLFDDKVMKQLKRRRYTGWGRLSRKLINGIRDKQSGKTILDFLKSDGFANRNFMQLIHDDSLTFKEDIQKAQVSGQGDSLHEHIANLAGSPAIKKGILQTVKVVDELVKVMGRHKPENIVIEMARENQTTQKGQKNSRERMKRIEEGIKELGSQILKEHPVENTQLQNEKLYLYYLQNGRDMYVDQELDINRLSDYDVDAIVPQSFLKDDSIDNKVLTRSDKNRGKSDNVPSEEVVKKMKNYWRQLLNAKLITQRKFDNLTKAERGGLSELDKAGFIKRQLVETRQITKHVAQILDSRMNTKYDENDKLIREVKVITLKSKLVSDFRKDFQFYKVREINNYHHAHDAYLNAVVGTALIKKYPKLESEFVYGDYKVYDVRKMIAKSEQEIGKATAKYFFYSNIMNFFKTEITLANGEIRKRPLIETNGETGEIVWDKGRDFATVRKVLSMPQVNIVKKTEVQTGGFSKESILPKRNSDKLIARKKDWDPKKYGGFDSPTVAYSVLVVAKVEKGKSKKLKSVKELLGITIMERSSFEKNPIDFLEAKGYKEVKKDLIIKLPKYSLFELENGRKRMLASAGELQKGNELALPSKYVNFLYLASHYEKLKGSPEDNEQKQLFVEQHKHYLDEIIEQISEFSKRVILADANLDKVLSAYNKHRDKPIREQAENIIHLFTLTNLGAPAAFKYFDTTIDRKRYTSTKEVLDATLIHQSITGLYETRIDLSQLGGDAYPYDVPDYASLGSGSPKKKRKVEDPKKKRKVDGIGSGSNGSSGEELLSKNYHLENEVARLKKGSGSGGSGSGGSGSGSGGSGSGGSGSGEELLSKNYHGSGSGQRGSKRTADGSEFESPKKKRKVX

SEQ ID NO: 80 - protein, 2147 aa, synthetic construct
  REGION 1..2147: note = V4 fusion_D3a-D3l-dCas9-2xGCN4
  SITE 2147: note = misc_feature - Xaa =
MPAAKRVKLDGSNHDQEFDPPKVYPPVPAEKRKPIRVLSLFDGIATGLLVLKDLGIQVDRYIASEVCEDSITVGMVRHQGKIMYVGDVRSVTQKHIQEWGPFDLVIGGSPCNDLSIVNPARKGLYEGTGRLFFEFYRLLHDARPKEGDDRPFFWLFENVVAMGVSDKRDISRFLESNPVMIDAKEVSAAHRARYFWGNLPGMNRPLASTVNDKLELQECLEHGRIAKFSKVRTITTRSNSIKQGKDQHFPVFMNEKEDILWCTEMERVFGFPVHYTDVSNMSRLARQRLLGRSWSVPVIRHLFAPLKEYFACVSSGNSNANSRGPSFSSGLVPLSLRGSHMGPMEIYKTVSAWKRQPVRVLSLFRNIDKVLKSLGFLESGSGSGGGTLKYVEDVTNVVRRDVEKWGPFDLVYGSTQPLGSSCDRCPGWYMFQFHRILQYALPRQESQRPFFWIFMDNLLLTEDDQETTTRFLQTEAVTLQDVRGRDYQNAMRVWSNIPGLKSKHAPLTPKEEEYLQAQVRSRSKLDAPKVDLLVKNCLLPLREYFKYFSQNSLPLGGPSSGAPPPSGGSPAGSPTSTEEGTSESATPESGPGTSTEPSEGSAPGSPAGSPTSTEEGTSTEPSEGSAPGTSTEPSEPKKKRKVMDKKYSIGLAIGTNSVGWAVITDEYKVPSKKFKVLGNTDRHSIKKNLIGALLFDSGETAEATRLKRTARRRYTRRKNRICYLQEIFSNEMAKVDDSFFHRLEESFLVEEDKKHERHPIFGNIVDEVAYHEKYPTIYHLRKKLVDSTDKADLRLIYLALAHMIKFRGHFLIEGDLNPDNSDVDKLFIQLVQTYNQLFEENPINASGVDAKAILSARLSKSRRLENLIAQLPGEKKNGLFGNLIALSLGLTPNFKSNFDLAEDAKLQLSKDTYDDDLDNLLAQIGDQYADLFLAAKNLSDAILLSDILRVNTEITKAPLSASMIKRYDEHHQDLTLLKALVRQQLPEKYKEIFFDQSKNGYAGYIDGGASQEEFYKFIKPILEKMDGTEELLVKLNREDLLRKQRTFDNGSIPHQIHLGELHAILRRQEDFYPFLKDNREKIEKILTFRIPYYVGPLARGNSRFAWMTRKSEETITPWNFEEVVDKGASAQSFIERMTNFDKNLPNEKVLPKHSLLYEYFTVYNELTKVKYVTEGMRKPAFLSGEQKKAIVDLLFKTNRKVTVKQLKEDYFKKIECFDSVEISGVEDRFNASLGTYHDLLKIIKDKDFLDNEENEDILEDIVLTLTLFEDREMIEERLKTYAHLFDDKVMKQLKRRRYTGWGRLSRKLINGIRDKQSGKTILDFLKSDGFANRNFMQLIHDDSLTFKEDIQKAQVSGQGDSLHEHIANLAGSPAIKKGILQTVKVVDELVKVMGRHKPENIVIEMARENQTTQKGQKNSRERMKRIEEGIKELGSQILKEHPVENTQLQNEKLYLYYLQNGRDMYVDQELDINRLSDYDVDAIVPQSFLKDDSIDNKVLTRSDKNRGKSDNVPSEEVVKKMKNYWRQLLNAKLITQRKFDNLTKAERGGLSELDKAGFIKRQLVETRQITKHVAQILDSRMNTKYDENDKLIREVKVITLKSKLVSDFRKDFQFYKVREINNYHHAHDAYLNAVVGTALIKKYPKLESEFVYGDYKVYDVRKMIAKSEQEIGKATAKYFFYSNIMNFFKTEITLANGEIRKRPLIETNGETGEIVWDKGRDFATVRKVLSMPQVNIVKKTEVQTGGFSKESILPKRNSDKLIARKKDWDPKKYGGFDSPTVAYSVLVVAKVEKGKSKKLKSVKELLGITIMERSSFEKNPIDFLEAKGYKEVKKDLIIKLPKYSLFELENGRKRMLASAGELQKGNELALPSKYVNFLYLASHYEKLKGSPEDNEQKQLFVEQHKHYLDEIIEQISEFSKRVILADANLDKVLSAYNKHRDKPIREQAENIIHLFTLTNLGAPAAFKYFDTTIDRKRYTSTKEVLDATLIHQSITGLYETRIDLSQLGGDAYPYDVPDYASLGSGSPKKKRKVEDPKKKRKVDGIGSGSNGSSGEELLSKNYHLENEVARLKKGSGSGGSGSGGSGSGSGGSGSGGSGSGEELLSKNYHLENEVARLKKGSGSGQRGSKRTADGSEFESPKKKRKVX

SEQ ID NO: 81 - protein, 2239 aa, synthetic construct
  REGION 1..2239: note = V5 fusion_D3a-D3l-dCas9-4xGCN4
  SITE 2239: note = misc_feature - Xaa =
MPAAKRVKLDGSNHDQEFDPPKVYPPVPAEKRKPIRVLSLFDGIATGLLVLKDLGIQVDRYIASEVCEDSITVGMVRHQGKIMYVGDVRSVTQKHIQEWGPFDLVIGGSPCNDLSIVNPARKGLYEGTGRLFFEFYRLLHDARPKEGDDRPFFWLFENVVAMGVSDKRDISRFLESNPVMIDAKEVSAAHRARYFWGNLPGMNRPLASTVNDKLELQECLEHGRIAKFSKVRTITTRSNSIKQGKDQHFPVFMNEKEDILWCTEMERVFGFPVHYTDVSNMSRLARQRLLGRSWSVPVIRHLFAPLKEYFACVSSGNSNANSRGPSFSSGLVPLSLRGSHMGPMEIYKTVSAWKRQPVRVLSLFRNIDKVLKSLGFLESGSGSGGGTLKYVEDVTNVVRRDVEKWGPFDLVYGSTQPLGSSCDRCPGWYMFQFHRILQYALPRQESQRPFFWIFMDNLLLTEDDQETTTRFLQTEAVTLQDVRGRDYQNAMRVWSNIPGLKSKHAPLTPKEEEYLQAQVRSRSKLDAPKVDLLVKNCLLPLREYFKYFSQNSLPLGGPSSGAPPPSGGSPAGSPTSTEEGTSESATPESGPGTSTEPSEGSAPGSPAGSPTSTEEGTSTEPSEGSAPGTSTEPSEPKKKRKVMDKKYSIGLAIGTNSVGWAVITDEYKVPSKKFKVLGNTDRHSIKKNLIGALLFDSGETAEATRLKRTARRRYTRRKNRICYLQEIFSNEMAKVDDSFFHRLEESFLVEEDKKHERHPIFGNIVDEVAYHEKYPTIYHLRKKLVDSTDKADLRLIYLALAHMIKFRGHFLIEGDLNPDNSDVDKLFIQLVQTYNQLFEENPINASGVDAKAILSARLSKSRRLENLIAQLPGEKKNGLFGNLIALSLGLTPNFKSNFDLAEDAKLQLSKDTYDDDLDNLLAQIGDQYADLFLAAKNLSDAILLSDILRVNTEITKAPLSASMIKRYDEHHQDLTLLKALVRQQLPEKYKEIFFDQSKNGYAGYIDGGASQEEFYKFIKPILEKMDGTEELLVKLNREDLLRKQRTFDNGSIPHQIHLGELHAILRRQEDFYPFLKDNREKIEKILTFRIPYYVGPLARGNSRFAWMTRKSEETITPWNFEEVVDKGASAQSFIERMTNFDKNLPNEKVLPKHSLLYEYFTVYNELTKVKYVTEGMRKPAFLSGEQKKAIVDLLFKTNRKVTVKQLKEDYFKKIECFDSVEISGVEDRFNASLGTYHDLLKIIKDKDFLDNEENEDILEDIVLTLTLFEDREMIEERLKTYAHLFDDKVMKQLKRRRYTGWGRLSRKLINGIRDKQSGKTILDFLKSDGFANRNFMQLIHDDSLTFKEDIQKAQVSGQGDSLHEHIANLAGSPAIKKGILQTVKVVDELVKVMGRHKPENIVIEMARENQTTQKGQKNSRERMKRIEEGIKELGSQILKEHPVENTQLQNEKLYLYYLQNGRDMYVDQELDINRLSDYDVDAIVPQSFLKDDSIDNKVLTRSDKNRGKSDNVPSEEVVKKMKNYWRQLLNAKLITQRKFDNLTKAERGGLSELDKAGFIKRQLVETRQITKHVAQILDSRMNTKYDENDKLIREVKVITLKSKLVSDFRKDFQFYKVREINNYHHAHDAYLNAVVGTALIKKYPKLESEFVYGDYKVYDVRKMIAKSEQEIGKATAKYFFYSNIMNFFKTEITLANGEIRKRPLIETNGETGEIVWDKGRDFATVRKVLSMPQVNIVKKTEVQTGGFSKESILPKRNSDKLIARKKDWDPKKYGGFDSPTVAYSVLVVAKVEKGKSKKLKSVKELLGITIMERSSFEKNPIDFLEAKGYKEVKKDLIIKLPKYSLFELENGRKRMLASAGELQKGNELALPSKYVNFLYLASHYEKLKGSPEDNEQKQLFVEQHKHYLDEIIEQISEFSKRVILADANLDKVLSAYNKHRDKPIREQAENIIHLFTLTNLGAPAAFKYFDTTIDRKRYTSTKEVLDATLIHQSITGLYETRIDLSQLGGDAYPYDVPDYASLGSGSPKKKRKVEDPKKKRKVDGIGSGSNGSSGEELLSKNYHLENEVARLKKGSGSGGSGSGGSGSGSGGSGSGGSGSGEELLSKNYHLENEVARLKKGSGSGGSGSGGSGSGSGGSGSGGSGSGEELLSKNYHLENEVARLKKGSGSGGSGSGGSGSGSGGSGSGGSGSGEELLSKNYHLENEVARLKKGSGSGQRGSKRTADGSEFESPKKKRKVX

SEQ ID NO: 82 - protein, 2515 aa, synthetic construct
  REGION 1..2515: note = V6 fusion_D3a-D3l-dCas9-10xGCN4
  SITE 2515: note = misc_feature - Xaa =
MPAAKRVKLDGSNHDQEFDPPKVYPPVPAEKRKPIRVLSLFDGIATGLLVLKDLGIQVDRYIASEVCEDSITVGMVRHQGKIMYVGDVRSVTQKHIQEWGPFDLVIGGSPCNDLSIVNPARKGLYEGTGRLFFEFYRLLHDARPKEGDDRPFFWLFENVVAMGVSDKRDISRFLESNPVMIDAKEVSAAHRARYFWGNLPGMNRPLASTVNDKLELQECLEHGRIAKFSKVRTITTRSNSIKQGKDQHFPVFMNEKEDILWCTEMERVFGFPVHYTDVSNMSRLARQRLLGRSWSVPVIRHLFAPLKEYFACVSSGNSNANSRGPSFSSGLVPLSLRGSHMGPMEIYKTVSAWKRQPVRVLSLFRNIDKVLKSLGFLESGSGSGGGTLKYVEDVTNVVRRDVEKWGPFDLVYGSTQPLGSSCDRCPGWYMFQFHRILQYALPRQESQRPFFWIFMDNLLLTEDDQETTTRFLQTEAVTLQDVRGRDYQNAMRVWSNIPGLKSKHAPLTPKEEEYLQAQVRSRSKLDAPKVDLLVKNCLLPLREYFKYFSQNSLPLGGPSSGAPPPSGGSPAGSPTSTEEGTSESATPESGPGTSTEPSEGSAPGSPAGSPTSTEEGTSTEPSEGSAPGTSTEPSEPKKKRKVMDKKYSIGLAIGTNSVGWAVITDEYKVPSKKFKVLGNTDRHSIKKNLIGALLFDSGETAEATRLKRTARRRYTRRKNRICYLQEIFSNEMAKVDDSFFHRLEESFLVEEDKKHERHPIFGNIVDEVAYHEKYPTIYHLRKKLVDSTDKADLRLIYLALAHMIKFRGHFLIEGDLNPDNSDVDKLFIQLVQTYNQLFEENPINASGVDAKAILSARLSKSRRLENLIAQLPGEKKNGLFGNLIALSLGLTPNFKSNFDLAEDAKLQLSKDTYDDDLDNLLAQIGDQYADLFLAAKNLSDAILLSDILRVNTEITKAPLSASMIKRYDEHHQDLTLLKALVRQQLPEKYKEIFFDQSKNGYAGYIDGGASQEEFYKFIKPILEKMDGTEELLVKLNREDLLRKQRTFDNGSIPHQIHLGELHAILRRQEDFYPFLKDNREKIEKILTFRIPYYVGPLARGNSRFAWMTRKSEETITPWNFEEVVDKGASAQSFIERMTNFDKNLPNEKVLPKHSLLYEYFTVYNELTKVKYVTEGMRKPAFLSGEQKKAIVDLLFKTNRKVTVKQLKEDYFKKIECFDSVEISGVEDRFNASLGTYHDLLKIIKDKDFLDNEENEDILEDIVLTLTLFEDREMIEERLKTYAHLFDDKVMKQLKRRRYTGWGRLSRKLINGIRDKQSGKTILDFLKSDGFANRNFMQLIHDDSLTFKEDIQKAQVSGQGDSLHEHIANLAGSPAIKKGILQTVKVVDELVKVMGRHKPENIVIEMARENQTTQKGQKNSRERMKRIEEGIKELGSQILKEHPVENTQLQNEKLYLYYLQNGRDMYVDQELDINRLSDYDVDAIVPQSFLKDDSIDNKVLTRSDKNRGKSDNVPSEEVVKKMKNYWRQLLNAKLITQRKFDNLTKAERGGLSELDKAGFIKRQLVETRQITKHVAQILDSRMNTKYDENDKLIREVKVITLKSKLVSDFRKDFQFYKVREINNYHHAHDAYLNAVVGTALIKKYPKLESEFVYGDYKVYDVRKMIAKSEQEIGKATAKYFFYSNIMNFFKTEITLANGEIRKRPLIETNGETGEIVWDKGRDFATVRKVLSMPQVNIVKKTEVQTGGFSKESILPKRNSDKLIARKKDWDPKKYGGFDSPTVAYSVLVVAKVEKGKSKKLKSVKELLGITIMERSSFEKNPIDFLEAKGYKEVKKDLIIKLPKYSLFELENGRKRMLASAGELQKGNELALPSKYVNFLYLASHYEKLKGSPEDNEQKQLFVEQHKHYLDEIIEQISEFSKRVILADANLDKVLSAYNKHRDKPIREQAENIIHLFTLTNLGAPAAFKYFDTTIDRKRYTSTKEVLDATLIHQSITGLYETRIDLSQLGGDAYPYDVPDYASLGSGSPKKKRKVEDPKKKRKVDGIGSGSNGSSGEELLSKNYHLENEVARLKKGSGSGGSGSGGSGSGSGGSGSGGSGSGEELLSKNYHLENEVARLKKGSGSGGSGSGGSGSGSGGSGSGGSGSGEELLSKNYHLENEVARLKKGSGSGGSGSGGSGSGSGGSGSGGSGSGEELLSKNYHLENEVARLKKGSGSGGSGSGGSGSGSGGSGSGGSGSGEELLSKNYHLENEVARLKKGSGSGGSGSGGSGSGSGGSGSGGSGSGEELLSKNYHLENEVARLKKGSGSGGSGSGGSGSGSGGSGSGGSGSGEELLSKNYHLENEVARLKKGSGSGGSGSGGSGSGSGGSGSGGSGSGEELLSKNYHLENEVARLKKGSGSGGSGSGGSGSGSGGSGSGGSGSGEELLSKNYHLENEVARLKKGSGSGGSGSGGSGSGSGGSGSGGSGSGEELLSKNYHLENEVARLKKGSGSGQRGSKRTADGSEFESPKKKRKVX

SEQ ID NO: 83 - protein, 912 aa, synthetic construct
  REGION 1..912: note = V7 fusion_D3a-D3l-scFv
  SITE 912: note = misc_feature - Xaa =
MPAAKRVKLDGSNHDQEFDPPKVYPPVPAEKRKPIRVLSLFDGIATGLLVLKDLGIQVDRYIASEVCEDSITVGMVRHQGKIMYVGDVRSVTQKHIQEWGPFDLVIGGSPCNDLSIVNPARKGLYEGTGRLFFEFYRLLHDARPKEGDDRPFFWLFENVVAMGVSDKRDISRFLESNPVMIDAKEVSAAHRARYFWGNLPGMNRPLASTVNDKLELQECLEHGRIAKFSKVRTITTRSNSIKQGKDQHFPVFMNEKEDILWCTEMERVFGFPVHYTDVSNMSRLARQRLLGRSWSVPVIRHLFAPLKEYFACVSSGNSNANSRGPSFSSGLVPLSLRGSHMGPMEIYKTVSAWKRQPVRVLSLFRNIDKVLKSLGFLESGSGSGGGTLKYVEDVTNVVRRDVEKWGPFDLVYGSTQPLGSSCDRCPGWYMFQFHRILQYALPRQESQRPFFWIFMDNLLLTEDDQETTTRFLQTEAVTLQDVRGRDYQNAMRVWSNIPGLKSKHAPLTPKEEEYLQAQVRSRSKLDAPKVDLLVKNCLLPLREYFKYFSQNSLPLGGPSSGAPPPSGGSPAGSPTSTEEGTSESATPESGPGTSTEPSEGSAPGSPAGSPTSTEEGTSTEPSEGSAPGTSTEPSEGPDIVMTQSPSSLSASVGDRVTITCRSSTGAVTTSNYASWVQEKPGKLFKGLIGGTNNRAPGVPSRFSGSLIGDKATLTISSLQPEDFATYFCALWYSNHWVFGQGTKVELKRGGGGSGGGGSGGGGSSGGGSEVKLLESGGGLVQPGGSLKLSCAVSGFSLTDYGVNWVRQAPGRGLEWIGVIWGDGITDYNSALKDRFIISKDNGKNTVYLQMSKVRSDDTALYYCVTGLFDYWGQGTLVTVSSYPYDVPDYAGGGGGSGGGGSGGGGSGGGGSX

SEQ ID NO: 84 - protein, 1638 aa, synthetic construct
  REGION 1..1638: note = V8 fusion_3xGCN4-dCas9-KRAB
  SITE 1638: note = misc_feature - Xaa =
MPAAKRVKLDGSEELLSKNYHLENEVARLKKGSGSGGSGSGGSGSGSGGSGSGGSGSGEELLSKNYHLENEVARLKKGSGSGGSGSGGSGSGSGGSGSGGSGSGEELLSKNYHLENEVARLKKGSGSGGSGSGGSGSGSGGSGSGGSGSGPKKKRKVMDKKYSIGLAIGTNSVGWAVITDEYKVPSKKFKVLGNTDRHSIKKNLIGALLFDSGETAEATRLKRTARRRYTRRKNRICYLQEIFSNEMAKVDDSFFHRLEESFLVEEDKKHERHPIFGNIVDEVAYHEKYPTIYHLRKKLVDSTDKADLRLIYLALAHMIKFRGHFLIEGDLNPDNSDVDKLFIQLVQTYNQLFEENPINASGVDAKAILSARLSKSRRLENLIAQLPGEKKNGLFGNLIALSLGLTPNFKSNFDLAEDAKLQLSKDTYDDDLDNLLAQIGDQYADLFLAAKNLSDAILLSDILRVNTEITKAPLSASMIKRYDEHHQDLTLLKALVRQQLPEKYKEIFFDQSKNGYAGYIDGGASQEEFYKFIKPILEKMDGTEELLVKLNREDLLRKQRTFDNGSIPHQIHLGELHAILRRQEDFYPFLKDNREKIEKILTFRIPYYVGPLARGNSRFAWMTRKSEETITPWNFEEVVDKGASAQSFIERMTNFDKNLPNEKVLPKHSLLYEYFTVYNELTKVKYVTEGMRKPAFLSGEQKKAIVDLLFKTNRKVTVKQLKEDYFKKIECFDSVEISGVEDRFNASLGTYHDLLKIIKDKDFLDNEENEDILEDIVLTLTLFEDREMIEERLKTYAHLFDDKVMKQLKRRRYTGWGRLSRKLINGIRDKQSGKTILDFLKSDGFANRNFMQLIHDDSLTFKEDIQKAQVSGQGDSLHEHIANLAGSPAIKKGILQTVKVVDELVKVMGRHKPENIVIEMARENQTTQKGQKNSRERMKRIEEGIKELGSQILKEHPVENTQLQNEKLYLYYLQNGRDMYVDQELDINRLSDYDVDAIVPQSFLKDDSIDNKVLTRSDKNRGKSDNVPSEEVVKKMKNYWRQLLNAKLITQRKFDNLTKAERGGLSELDKAGFIKRQLVETRQITKHVAQILDSRMNTKYDENDKLIREVKVITLKSKLVSDFRKDFQFYKVREINNYHHAHDAYLNAVVGTALIKKYPKLESEFVYGDYKVYDVRKMIAKSEQEIGKATAKYFFYSNIMNFFKTEITLANGEIRKRPLIETNGETGEIVWDKGRDFATVRKVLSMPQVNIVKKTEVQTGGFSKESILPKRNSDKLIARKKDWDPKKYGGFDSPTVAYSVLVVAKVEKGKSKKLKSVKELLGITIMERSSFEKNPIDFLEAKGYKEVKKDLIIKLPKYSLFELENGRKRMLASAGELQKGNELALPSKYVNFLYLASHYEKLKGSPEDNEQKQLFVEQHKHYLDEIIEQISEFSKRVILADANLDKVLSAYNKHRDKPIREQAENIIHLFTLTNLGAPAAFKYFDTTIDRKRYTSTKEVLDATLIHQSITGLYETRIDLSQLGGDAYPYDVPDYASLGSGSPKKKRKVEDPKKKRKVDGSGSETPGTSESATPESRTLVTFKDVFVDFTREEWKLLDTAQQIVYRNVMLENYKNLVSLGYQLTKPDVILRLEKGEEPX

SEQ ID NO: 85 - protein, 297 aa, synthetic construct
  REGION 1..297: note = V9 fusion_GFP1-10-KRAB
  SITE 297: note = misc_feature - Xaa =
MPAAKRVKLDGSSKGEELFTGVVPILVELDGDVNGHKFSVRGEGEGDATIGKLTLKFICTTGKLPVPWPTLVTTLTYGVQCFSRYPDHMKRHDFFKSAMPEGYVQERTISFKDDGKYKTRAVVKFEGDTLVNRIELKGTDFKEDGNILGHKLEYNFNSHNVYITADKQKNGIKANFTVRHNVEDGSVQLADHYQQNTPIGDGPVLLPDNHYLSTQTVLSKDPNEKLDPGGGGSGRTLVTFKDVFVDFTREEWKLLDTAQQIVYRNVMLENYKNLVSLGYQLTKPDVILRLEKGEEPX

SEQ ID NO: 86 - protein, 2123 aa, synthetic construct
  REGION 1..2123: note = V10 fusion_D3a-D3l-dCas9-1xGFP11
  SITE 2123: note = misc_feature - Xaa =
MPAAKRVKLDGSNHDQEFDPPKVYPPVPAEKRKPIRVLSLFDGIATGLLVLKDLGIQVDRYIASEVCEDSITVGMVRHQGKIMYVGDVRSVTQKHIQEWGPFDLVIGGSPCNDLSIVNPARKGLYEGTGRLFFEFYRLLHDARPKEGDDRPFFWLFENVVAMGVSDKRDISRFLESNPVMIDAKEVSAAHRARYFWGNLPGMNRPLASTVNDKLELQECLEHGRIAKFSKVRTITTRSNSIKQGKDQHFPVFMNEKEDILWCTEMERVFGFPVHYTDVSNMSRLARQRLLGRSWSVPVIRHLFAPLKEYFACVSSGNSNANSRGPSFSSGLVPLSLRGSHMGPMEIYKTVSAWKRQPVRVLSLFRNIDKVLKSLGFLESGSGSGGGTLKYVEDVTNVVRRDVEKWGPFDLVYGSTQPLGSSCDRCPGWYMFQFHRILQYALPRQESQRPFFWIFMDNLLLTEDDQETTTRFLQTEAVTLQDVRGRDYQNAMRVWSNIPGLKSKHAPLTPKEEEYLQAQVRSRSKLDAPKVDLLVKNCLLPLREYFKYFSQNSLPLGGPSSGAPPPSGGSPAGSPTSTEEGTSESATPESGPGTSTEPSEGSAPGSPAGSPTSTEEGTSTEPSEGSAPGTSTEPSEPKKKRKVMDKKYSIGLAIGTNSVGWAVITDEYKVPSKKFKVLGNTDRHSIKKNLIGALLFDSGETAEATRLKRTARRRYTRRKNRICYLQEIFSNEMAKVDDSFFHRLEESFLVEEDKKHERHPIFGNIVDEVAYHEKYPTIYHLRKKLVDSTDKADLRLIYLALAHMIKFRGHFLIEGDLNPDNSDVDKLFIQLVQTYNQLFEENPINASGVDAKAILSARLSKSRRLENLIAQLPGEKKNGLFGNLIALSLGLTPNFKSNFDLAEDAKLQLSKDTYDDDLDNLLAQIGDQYADLFLAAKNLSDAILLSDILRVNTEITKAPLSASMIKRYDEHHQDLTLLKALVRQQLPEKYKEIFFDQSKNGYAGYIDGGASQEEFYKFIKPILEKMDGTEELLVKLNREDLLRKQRTFDNGSIPHQIHLGELHAILRRQEDFYPFLKDNREKIEKILTFRIPYYVGPLARGNSRFAWMTRKSEETITPWNFEEVVDKGASAQSFIERMTNFDKNLPNEKVLPKHSLLYEYFTVYNELTKVKYVTEGMRKPAFLSGEQKKAIVDLLFKTNRKVTVKQLKEDYFKKIECFDSVEISGVEDRFNASLGTYHDLLKIIKDKDFLDNEENEDILEDIVLTLTLFEDREMIEERLKTYAHLFDDKVMKQLKRRRYTGWGRLSRKLINGIRDKQSGKTILDFLKSDGFANRNFMQLIHDDSLTFKEDIQKAQVSGQGDSLHEHIANLAGSPAIKKGILQTVKVVDELVKVMGRHKPENIVIEMARENQTTQKGQKNSRERMKRIEEGIKELGSQILKEHPVENTQLQNEKLYLYYLQNGRDMYVDQELDINRLSDYDVDAIVPQSFLKDDSIDNKVLTRSDKNRGKSDNVPSEEVVKKMKNYWRQLLNAKLITQRKFDNLTKAERGGLSELDKAGFIKRQLVETRQITKHVAQILDSRMNTKYDENDKLIREVKVITLKSKLVSDFRKDFQFYKVREINNYHHAHDAYLNAVVGTALIKKYPKLESEFVYGDYKVYDVRKMIAKSEQEIGKATAKYFFYSNIMNFFKTEITLANGEIRKRPLIETNGETGEIVWDKGRDFATVRKVLSMPQVNIVKKTEVQTGGFSKESILPKRNSDKLIARKKDWDPKKYGGFDSPTVAYSVLVVAKVEKGKSKKLKSVKELLGITIMERSSFEKNPIDFLEAKGYKEVKKDLIIKLPKYSLFELENGRKRMLASAGELQKGNELALPSKYVNFLYLASHYEKLKGSPEDNEQKQLFVEQHKHYLDEIIEQISEFSKRVILADANLDKVLSAYNKHRDKPIREQAENIIHLFTLTNLGAPAAFKYFDTTIDRKRYTSTKEVLDATLIHQSITGLYETRIDLSQLGGDAYPYDVPDYASLGSGSPKKKRKVEDPKKKRKVDGSGSETPGTSESATPESGSGSNGSSGSMRDHMVLHEYVNAAGITGGSGGAAARSGSGQRGSKRTADGSEFESPKKKRKVX

SEQ ID NO: 87 - protein, 2244 aa, synthetic construct
  REGION 1..2244: note = V11 fusion_D3a-D3l-dCas9-8xGFP11
  SITE 2244: note = misc_feature - Xaa =
MPAAKRVKLDGSNHDQEFDPPKVYPPVPAEKRKPIRVLSLFDGIATGLLVLKDLGIQVDRYIASEVCEDSITVGMVRHQGKIMYVGDVRSVTQKHIQEWGPFDLVIGGSPCNDLSIVNPARKGLYEGTGRLFFEFYRLLHDARPKEGDDRPFFWLFENVVAMGVSDKRDISRFLESNPVMIDAKEVSAAHRARYFWGNLPGMNRPLASTVNDKLELQECLEHGRIAKFSKVRTITTRSNSIKQGKDQHFPVFMNEKEDILWCTEMERVFGFPVHYTDVSNMSRLARQRLLGRSWSVPVIRHLFAPLKEYFACVSSGNSNANSRGPSFSSGLVPLSLRGSHMGPMEIYKTVSAWKRQPVRVLSLFRNIDKVLKSLGFLESGSGSGGGTLKYVEDVTNVVRRDVEKWGPFDLVYGSTQPLGSSCDRCPGWYMFQFHRILQYALPRQESQRPFFWIFMDNLLLTEDDQETTTRFLQTEAVTLQDVRGRDYQNAMRVWSNIPGLKSKHAPLTPKEEEYLQAQVRSRSKLDAPKVDLLVKNCLLPLREYFKYFSQNSLPLGGPSSGAPPPSGGSPAGSPTSTEEGTSESATPESGPGTSTEPSEGSAPGSPAGSPTSTEEGTSTEPSEGSAPGTSTEPSEPKKKRKVMDKKYSIGLAIGTNSVGWAVITDEYKVPSKKFKVLGNTDRHSIKKNLIGALLFDSGETAEATRLKRTARRRYTRRKNRICYLQEIFSNEMAKVDDSFFHRLEESFLVEEDKKHERHPIFGNIVDEVAYHEKYPTIYHLRKKLVDSTDKADLRLIYLALAHMIKFRGHFLIEGDLNPDNSDVDKLFIQLVQTYNQLFEENPINASGVDAKAILSARLSKSRRLENLIAQLPGEKKNGLFGNLIALSLGLTPNFKSNFDLAEDAKLQLSKDTYDDDLDNLLAQIGDQYADLFLAAKNLSDAILLSDILRVNTEITKAPLSASMIKRYDEHHQDLTLLKALVRQQLPEKYKEIFFDQSKNGYAGYIDGGASQEEFYKFIKPILEKMDGTEELLVKLNREDLLRKQRTFDNGSIPHQIHLGELHAILRRQEDFYPFLKDNREKIEKILTFRIPYYVGPLARGNSRFAWMTRKSEETITPWNFEEVVDKGASAQSFIERMTNFDKNLPNEKVLPKHSLLYEYFTVYNELTKVKYVTEGMRKPAFLSGEQKKAIVDLLFKTNRKVTVKQLKEDYFKKIECFDSVEISGVEDRFNASLGTYHDLLKIIKDKDFLDNEENEDILEDIVLTLTLFEDREMIEERLKTYAHLFDDKVMKQLKRRRYTGWGRLSRKLINGIRDKQSGKTILDFLKSDGFANRNFMQLIHDDSLTFKEDIQKAQVSGQGDSLHEHIANLAGSPAIKKGILQTVKVVDELVKVMGRHKPENIVIEMARENQTTQKGQKNSRERMKRIEEGIKELGSQILKEHPVENTQLQNEKLYLYYLQNGRDMYVDQELDINRLSDYDVDAIVPQSFLKDDSIDNKVLTRSDKNRGKSDNVPSEEVVKKMKNYWRQLLNAKLITQRKFDNLTKAERGGLSELDKAGFIKRQLVETRQITKHVAQILDSRMNTKYDENDKLIREVKVITLKSKLVSDFRKDFQFYKVREINNYHHAHDAYLNAVVGTALIKKYPKLESEFVYGDYKVYDVRKMIAKSEQEIGKATAKYFFYSNIMNFFKTEITLANGEIRKRPLIETNGETGEIVWDKGRDFATVRKVLSMPQVNIVKKTEVQTGGFSKESILPKRNSDKLIARKKDWDPKKYGGFDSPTVAYSVLVVAKVEKGKSKKLKSVKELLGITIMERSSFEKNPIDFLEAKGYKEVKKDLIIKLPKYSLFELENGRKRMLASAGELQKGNELALPSKYVNFLYLASHYEKLKGSPEDNEQKQLFVEQHKHYLDEIIEQISEFSKRVILADANLDKVLSAYNKHRDKPIREQAENIIHLFTLTNLGAPAAFKYFDTTIDRKRYTSTKEVLDATLIHQSITGLYETRIDLSQLGGDAYPYDVPDYASLGSGSPKKKRKVEDPKKKRKVDGSGSETPGTSESATPESGSGSNGSSGSMRDHMVLHEYVNAAGITGGSGGRDHMVLHEYVNAAGITGGSGGRDHMVLHEYVNAAGITGGSGGRDHMVLHEYVNAAGITGGSGGRDHMVLHEYVNAAGITGGSGGRDHMVLHEYVNAAGITGGSGGRDHMVLHEYVNAAGITAAARSGSGQRGSKRTADGSEFESPKKKRKVX

SEQ ID NO: 88 - protein, 2125 aa, synthetic construct
  REGION 1..2125: note = (from V15)_D3a-hD3l-dCas9-1xGCN4
  SITE 2125: note = misc_feature - Xaa =
MPAAKRVKLDGSNHDQEFDPPKVYPPVPAEKRKPIRVLSLFDGIATGLLVLKDLGIQVDRYIASEVCEDSITVGMVRHQGKIMYVGDVRSVTQKHIQEWGPFDLVIGGSPCNDLSIVNPARKGLYEGTGRLFFEFYRLLHDARPKEGDDRPFFWLFENVVAMGVSDKRDISRFLESNPVMIDAKEVSAAHRARYFWGNLPGMNRPLASTVNDKLELQECLEHGRIAKFSKVRTITTRSNSIKQGKDQHFPVFMNEKEDILWCTEMERVFGFPVHYTDVSNMSRLARQRLLGRSWSVPVIRHLFAPLKEYFACVSSGNSNANSRGPSFSSGLVPLSLRGSHMFETVPVWRRQPVRVLSLFEDIKKELTSLGFLESGSDPGQLKHVVDVTDTVRKDVEEWGPFDLVYGATPPLGHTCDRPPSWYLFQFHRLLQYARPKPGSPRPFFWMFVDNLVLNKEDLDVASRFLEMEPVTIPDVHGGSLQNAVRVWSNIPAIRSSRHWALVSEEELSLLAQNKQSSKLAAKWPTKLVKNCFLPLREYFKYFSGGPSSGAPPPSGGSPAGSPTSTEEGTSESATPESGPGTSTEPSEGSAPGSPAGSPTSTEEGTSTEPSEGSAPGTSTEPSEPKKKRKVMDKKYSIGLAIGTNSVGWAVITDEYKVPSKKFKVLGNTDRHSIKKNLIGALLFDSGETAEATRLKRTARRRYTRRKNRICYLQEIFSNEMAKVDDSFFHRLEESFLVEEDKKHERHPIFGNIVDEVAYHEKYPTIYHLRKKLVDSTDKADLRLIYLALAHMIKFRGHFLIEGDLNPDNSDVDKLFIQLVQTYNQLFEENPINASGVDAKAILSARLSKSRRLENLIAQLPGEKKNGLFGNLIALSLGLTPNFKSNFDLAEDAKLQLSKDTYDDDLDNLLAQIGDQYADLFLAAKNLSDAILLSDILRVNTEITKAPLSASMIKRYDEHHQDLTLLKALVRQQLPEKYKEIFFDQSKNGYAGYIDGGASQEEFYKFIKPILEKMDGTEELLVKLNREDLLRKQRTFDNGSIPHQIHLGELHAILRRQEDFYPFLKDNREKIEKILTFRIPYYVGPLARGNSRFAWMTRKSEETITPWNFEEVVDKGASAQSFIERMTNFDKNLPNEKVLPKHSLLYEYFTVYNELTKVKYVTEGMRKPAFLSGEQKKAIVDLLFKTNRKVTVKQLKEDYFKKIECFDSVEISGVEDRFNASLGTYHDLLKIIKDKDFLDNEENEDILEDIVLTLTLFEDREMIEERLKTYAHLFDDKVMKQLKRRRYTGWGRLSRKLINGIRDKQSGKTILDFLKSDGFANRNFMQLIHDDSLTFKEDIQKAQVSGQGDSLHEHIANLAGSPAIKKGILQTVKVVDELVKVMGRHKPENIVIEMARENQTTQKGQKNSRERMKRIEEGIKELGSQILKEHPVENTQLQNEKLYLYYLQNGRDMYVDQELDINRLSDYDVDAIVPQSFLKDDSIDNKVLTRSDKNRGKSDNVPSEEVVKKMKNYWRQLLNAKLITQRKFDNLTKAERGGLSELDKAGFIKRQLVETRQITKHVAQILDSRMNTKYDENDKLIREVKVITLKSKLVSDFRKDFQFYKVREINNYHHAHDAYLNAVVGTALIKKYPKLESEFVYGDYKVYDVRKMIAKSEQEIGKATAKYFFYSNIMNFFKTEITLANGEIRKRPLIETNGETGEIVWDKGRDFATVRKVLSMPQVNIVKKTEVQTGGFSKESILPKRNSDKLIARKKDWDPKKYGGFDSPTVAYSVLVVAKVEKGKSKKLKSVKELLGITIMERSSFEKNPIDFLEAKGYKEVKKDLIIKLPKYSLFELENGRKRMLASAGELQKGNELALPSKYVNFLYLASHYEKLKGSPEDNEQKQLFVEQHKHYLDEIIEQISEFSKRVILADANLDKVLSAYNKHRDKPIREQAENIIHLFTLTNLGAPAAFKYFDTTIDRKRYTSTKEVLDATLIHQSITGLYETRIDLSQLGGDAYPYDVPDYASLGSGSPKKKRKVEDPKKKRKVDGIGSGSNGSSGEELLSKNYHLENEVARLKKGSGSGGSGSGGSGSGSGGSGSGGSGSGEELLSKNYHGSGSGQRGSKRTADGSEFESPKKKRKVX

SEQ ID NO: 89 - protein, 2135 aa, synthetic construct
  REGION 1..2135: note = (from V16)_D3a-hD3l-dCas9-2xGCN4
  SITE 2135: note = misc_feature - Xaa =
MPAAKRVKLDGSNHDQEFDPPKVYPPVPAEKRKPIRVLSLFDGIATGLLVLKDLGIQVDRYIASEVCEDSITVGMVRHQGKIMYVGDVRSVTQKHIQEWGPFDLVIGGSPCNDLSIVNPARKGLYEGTGRLFFEFYRLLHDARPKEGDDRPFFWLFENVVAMGVSDKRDISRFLESNPVMIDAKEVSAAHRARYFWGNLPGMNRPLASTVNDKLELQECLEHGRIAKFSKVRTITTRSNSIKQGKDQHFPVFMNEKEDILWCTEMERVFGFPVHYTDVSNMSRLARQRLLGRSWSVPVIRHLFAPLKEYFACVSSGNSNANSRGPSFSSGLVPLSLRGSHMFETVPVWRRQPVRVLSLFEDIKKELTSLGFLESGSDPGQLKHVVDVTDTVRKDVEEWGPFDLVYGATPPLGHTCDRPPSWYLFQFHRLLQYARPKPGSPRPFFWMFVDNLVLNKEDLDVASRFLEMEPVTIPDVHGGSLQNAVRVWSNIPAIRSSRHWALVSEEELSLLAQNKQSSKLAAKWPTKLVKNCFLPLREYFKYFSGGPSSGAPPPSGGSPAGSPTSTEEGTSESATPESGPGTSTEPSEGSAPGSPAGSPTSTEEGTSTEPSEGSAPGTSTEPSEPKKKRKVMDKKYSIGLAIGTNSVGWAVITDEYKVPSKKFKVLGNTDRHSIKKNLIGALLFDSGETAEATRLKRTARRRYTRRKNRICYLQEIFSNEMAKVDDSFFHRLEESFLVEEDKKHERHPIFGNIVDEVAYHEKYPTIYHLRKKLVDSTDKADLRLIYLALAHMIKFRGHFLIEGDLNPDNSDVDKLFIQLVQTYNQLFEENPINASGVDAKAILSARLSKSRRLENLIAQLPGEKKNGLFGNLIALSLGLTPNFKSNFDLAEDAKLQLSKDTYDDDLDNLLAQIGDQYADLFLAAKNLSDAILLSDILRVNTEITKAPLSASMIKRYDEHHQDLTLLKALVRQQLPEKYKEIFFDQSKNGYAGYIDGGASQEEFYKFIKPILEKMDGTEELLVKLNREDLLRKQRTFDNGSIPHQIHLGELHAILRRQEDFYPFLKDNREKIEKILTFRIPYYVGPLARGNSRFAWMTRKSEETITPWNFEEVVDKGASAQSFIERMTNFDKNLPNEKVLPKHSLLYEYFTVYNELTKVKYVTEGMRKPAFLSGEQKKAIVDLLFKTNRKVTVKQLKEDYFKKIECFDSVEISGVEDRFNASLGTYHDLLKIIKDKDFLDNEENEDILEDIVLTLTLFEDREMIEERLKTYAHLFDDKVMKQLKRRRYTGWGRLSRKLINGIRDKQSGKTILDFLKSDGFANRNFMQLIHDDSLTFKEDIQKAQVSGQGDSLHEHIANLAGSPAIKKGILQTVKVVDELVKVMGRHKPENIVIEMARENQTTQKGQKNSRERMKRIEEGIKELGSQILKEHPVENTQLQNEKLYLYYLQNGRDMYVDQELDINRLSDYDVDAIVPQSFLKDDSIDNKVLTRSDKNRGKSDNVPSEEVVKKMKNYWRQLLNAKLITQRKFDNLTKAERGGLSELDKAGFIKRQLVETRQITKHVAQILDSRMNTKYDENDKLIREVKVITLKSKLVSDFRKDFQFYKVREINNYHHAHDAYLNAVVGTALIKKYPKLESEFVYGDYKVYDVRKMIAKSEQEIGKATAKYFFYSNIMNFFKTEITLANGEIRKRPLIETNGETGEIVWDKGRDFATVRKVLSMPQVNIVKKTEVQTGGFSKESILPKRNSDKLIARKKDWDPKKYGGFDSPTVAYSVLVVAKVEKGKSKKLKSVKELLGITIMERSSFEKNPIDFLEAKGYKEVKKDLIIKLPKYSLFELENGRKRMLASAGELQKGNELALPSKYVNFLYLASHYEKLKGSPEDNEQKQLFVEQHKHYLDEIIEQISEFSKRVILADANLDKVLSAYNKHRDKPIREQAENIIHLFTLTNLGAPAAFKYFDTTIDRKRYTSTKEVLDATLIHQSITGLYETRIDLSQLGGDAYPYDVPDYASLGSGSPKKKRKVEDPKKKRKVDGIGSGSNGSSGEELLSKNYHLENEVARLKKGSGSGGSGSGGSGSGSGGSGSGGSGSGEELLSKNYHLENEVARLKKGSGSGQRGSKRTADGSEFESPKKKRKVX

SEQ ID NO: 90 - protein, 2503 aa, synthetic construct
  REGION 1..2503: note = (from V17)_D3a-hD3l-dCas9-10xGCN4
  SITE 2503: note = misc_feature - Xaa =
MPAAKRVKLDGSNHDQEFDPPKVYPPVPAEKRKPIRVLSLFDGIATGLLVLKDLGIQVDRYIASEVCEDSITVGMVRHQGKIMYVGDVRSVTQKHIQEWGPFDLVIGGSPCNDLSIVNPARKGLYEGTGRLFFEFYRLLHDARPKEGDDRPFFWLFENVVAMGVSDKRDISRFLESNPVMIDAKEVSAAHRARYFWGNLPGMNRPLASTVNDKLELQECLEHGRIAKFSKVRTITTRSNSIKQGKDQHFPVFMNEKEDILWCTEMERVFGFPVHYTDVSNMSRLARQRLLGRSWSVPVIRHLFAPLKEYFACVSSGNSNANSRGPSFSSGLVPLSLRGSHMFETVPVWRRQPVRVLSLFEDIKKELTSLGFLESGSDPGQLKHVVDVTDTVRKDVEEWGPFDLVYGATPPLGHTCDRPPSWYLFQFHRLLQYARPKPGSPRPFFWMFVDNLVLNKEDLDVASRFLEMEPVTIPDVHGGSLQNAVRVWSNIPAIRSSRHWALVSEEELSLLAQNKQSSKLAAKWPTKLVKNCFLPLREYFKYFSGGPSSGAPPPSGGSPAGSPTSTEEGTSESATPESGPGTSTEPSEGSAPGSPAGSPTSTEEGTSTEPSEGSAPGTSTEPSEPKKKRKVMDKKYSIGLAIGTNSVGWAVITDEYKVPSKKFKVLGNTDRHSIKKNLIGALLFDSGETAEATRLKRTARRRYTRRKNRICYLQEIFSNEMAKVDDSFFHRLEESFLVEEDKKHERHPIFGNIVDEVAYHEKYPTIYHLRKKLVDSTDKADLRLIYLALAHMIKFRGHFLIEGDLNPDNSDVDKLFIQLVQTYNQLFEENPINASGVDAKAILSARLSKSRRLENLIAQLPGEKKNGLFGNLIALSLGLTPNFKSNFDLAEDAKLQLSKDTYDDDLDNLLAQIGDQYADLFLAAKNLSDAILLSDILRVNTEITKAPLSASMIKRYDEHHQDLTLLKALVRQQLPEKYKEIFFDQSKNGYAGYIDGGASQEEFYKFIKPILEKMDGTEELLVKLNREDLLRKQRTFDNGSIPHQIHLGELHAILRRQEDFYPFLKDNREKIEKILTFRIPYYVGPLARGNSRFAWMTRKSEETITPWNFEEVVDKGASAQSFIERMTNFDKNLPNEKVLPKHSLLYEYFTVYNELTKVKYVTEGMRKPAFLSGEQKKAIVDLLFKTNRKVTVKQLKEDYFKKIECFDSVEISGVEDRFNASLGTYHDLLKIIKDKDFLDNEENEDILEDIVLTLTLFEDREMIEERLKTYAHLFDDKVMKQLKRRRYTGWGRLSRKLINGIRDKQSGKTILDFLKSDGFANRNFMQLIHDDSLTFKEDIQKAQVSGQGDSLHEHIANLAGSPAIKKGILQTVKVVDELVKVMGRHKPENIVIEMARENQTTQKGQKNSRERMKRIEEGIKELGSQILKEHPVENTQLQNEKLYLYYLQNGRDMYVDQELDINRLSDYDVDAIVPQSFLKDDSIDNKVLTRSDKNRGKSDNVPSEEVVKKMKNYWRQLLNAKLITQRKFDNLTKAERGGLSELDKAGFIKRQLVETRQITKHVAQILDSRMNTKYDENDKLIREVKVITLKSKLVSDFRKDFQFYKVREINNYHHAHDAYLNAVVGTALIKKYPKLESEFVYGDYKVYDVRKMIAKSEQEIGKATAKYFFYSNIMNFFKTEITLANGEIRKRPLIETNGETGEIVWDKGRDFATVRKVLSMPQVNIVKKTEVQTGGFSKESILPKRNSDKLIARKKDWDPKKYGGFDSPTVAYSVLVVAKVEKGKSKKLKSVKELLGITIMERSSFEKNPIDFLEAKGYKEVKKDLIIKLPKYSLFELENGRKRMLASAGELQKGNELALPSKYVNFLYLASHYEKLKGSPEDNEQKQLFVEQHKHYLDEIIEQISEFSKRVILADANLDKVLSAYNKHRDKPIREQAENIIHLFTLTNLGAPAAFKYFDTTIDRKRYTSTKEVLDATLIHQSITGLYETRIDLSQLGGDAYPYDVPDYASLGSGSPKKKRKVEDPKKKRKVDGIGSGSNGSSGEELLSKNYHLENEVARLKKGSGSGGSGSGGSGSGSGGSGSGGSGSGEELLSKNYHLENEVARLKKGSGSGGSGSGGSGSGSGGSGSGGSGSGEELLSKNYHLENEVARLKKGSGSGGSGSGGSGSGSGGSGSGGSGSGEELLSKNYHLENEVARLKKGSGSGGSGSGGSGSGSGGSGSGGSGSGEELLSKNYHLENEVARLKKGSGSGGSGSGGSGSGSGGSGSGGSGSGEELLSKNYHLENEVARLKKGSGSGGSGSGGSGSGSGGSGSGGSGSGEELLSKNYHLENEVARLKKGSGSGGSGSGGSGSGSGGSGSGGSGSGEELLSKNYHLENEVARLKKGSGSGGSGSGGSGSGSGGSGSGGSGSGEELLSKNYHLENEVARLKKGSGSGGSGSGGSGSGSGGSGSGGSGSGEELLSKNYHLENEVARLKKGSGSGQRGSKRTADGSEFESPKKKRKVX

SEQ ID NO: 91 - protein, 1985 aa, synthetic construct
  REGION 1..1985: note = (from V18)_D3a-hD3l-dCas912a-1xGCN4
  SITE 1985: note = misc_feature - Xaa =
MPAAKRVKLDGSNHDQEFDPPKVYPPVPAEKRKPIRVLSLFDGIATGLLVLKDLGIQVDRYIASEVCEDSITVGMVRHQGKIMYVGDVRSVTQKHIQEWGPFDLVIGGSPCNDLSIVNPARKGLYEGTGRLFFEFYRLLHDARPKEGDDRPFFWLFENVVAMGVSDKRDISRFLESNPVMIDAKEVSAAHRARYFWGNLPGMNRPLASTVNDKLELQECLEHGRIAKFSKVRTITTRSNSIKQGKDQHFPVFMNEKEDILWCTEMERVFGFPVHYTDVSNMSRLARQRLLGRSWSVPVIRHLFAPLKEYFACVSSGNSNANSRGPSFSSGLVPLSLRGSHMFETVPVWRRQPVRVLSLFEDIKKELTSLGFLESGSDPGQLKHVVDVTDTVRKDVEEWGPFDLVYGATPPLGHTCDRPPSWYLFQFHRLLQYARPKPGSPRPFFWMFVDNLVLNKEDLDVASRFLEMEPVTIPDVHGGSLQNAVRVWSNIPAIRSSRHWALVSEEELSLLAQNKQSSKLAAKWPTKLVKNCFLPLREYFKYFSGGPSSGAPPPSGGSPAGSPTSTEEGTSESATPESGPGTSTEPSEGSAPGSPAGSPTSTEEGTSTEPSEGSAPGTSTEPSEPKKKRKVMSKLEKFTNCYSLSKTLRFKAIPVGKTQENIDNKRLLVEDEKRAEDYKGVKKLLDRYYLSFINDVLHSIKLKNLNNYISLFRKKTRTEKENKELENLEINLRKEIAKAFKGNEGYKSLFKKDIIETILPEFLDDKDEIALVNSFNGFTTAFTGFFDNRENMFSEEAKSTSIAFRCINENLTRYISNMDIFEKVDAIFDKHEVQEIKEKILNSDYDVEDFFEGEFFNFVLTQEGIDVYNAIIGGFVTESGEKIKGLNEYINLYNQKTKQKLPKFKPLYKQVLSDRESLSFYGEGYTSDEEVLEVFRNTLNKNSEIFSSIKKLEKLFKNFDEYSSAGIFVKNGPAISTISKDIFGEWNVIRDKWNAEYDDIHLKKKAVVTEKYEDDRRKSFKKIGSFSLEQLQEYADADLSVVEKLKEIIIQKVDEIYKVYGSSEKLFDADFVLEKSLKKNDAVVAIMKDLLDSVKSFENYIKAFFGEGKETNRDESFYGDFVLAYDILLKVDHIYDAIRNYVTQKPYSKDKFKLYFQNPQFMGGWDKDKETDYRATILRYGSKYYLAIMDKKYAKCLQKIDKDDVNGNYEKINYKLLPGPNKMLPKVFFSKKWMAYYNPSEDIQKIYKNGTFKKGDMFNLNDCHKLIDFFKDSISRYPKWSNAYDFNFSETEKYKDIAGFYREVEEQGYKVSFESASKKEVDKLVEEGKLYMFQIYNKDFSDKSHGTPNLHTMYFKLLFDENNHGQIRLSGGAELFMRRASLKKEELVVHPANSPIANKNPDNPKKTTTLSYDVYKDKRFSEDQYELHIPIAINKCPKNIFKINTEVRVLLKHDDNPYVIGIARGERNLLYIVVVDGKGNIVEQYSLNEIINNFNGIRIKTDYHSLLDKKEKERFEARQNWTSIENIKELKAGYISQVVHKICELVEKYDAVIALADLNSGFKNSRVKVEKQVYQKFEKMLIDKLNYMVDKKSNPCATGGALKGYQITNKFESFKSMSTQNGFIFYIPAWLTSKIDPSTGFVNLLKTKYTSIADSKKFISSFDRIMYVPEEDLFEFALDYKNFSRTDADYIKKWKLYSYGNRIRIFRNPKKNNVFDWEEVCLTSAYKELFNKYGINYQQGDIRALLCEQSDKAFYSSFMALMSLMLQMRNSITGRTDVAFLISPVKNSDGIFYDSRNYEAQENAILPKNADANGAYNIARKVLWAIGQFKKAEDEKLDKVKIAISNKEWLEYAQTSVKHAYPYDVPDYASLGSGSPKKKRKVEDPKKKRKVDGIGSGSNGSSGEELLSKNYHLENEVARLKKGSGSGGSGSGGSGSGSGGSGSGGSGSGEELLSKNYHGSGSGQRGSKRTADGSEFESPKKKRKVX

SEQ ID NO: 92 - protein, 1768 aa, synthetic construct
  REGION 1..1768: note = (from V19)_D3a-hD3l-dCas12i-1xGCN4
  SITE 1768: note = misc_feature - Xaa =
MPAAKRVKLDGSNHDQEFDPPKVYPPVPAEKRKPIRVLSLFDGIATGLLVLKDLGIQVDRYIASEVCEDSITVGMVRHQGKIMYVGDVRSVTQKHIQEWGPFDLVIGGSPCNDLSIVNPARKGLYEGTGRLFFEFYRLLHDARPKEGDDRPFFWLFENVVAMGVSDKRDISRFLESNPVMIDAKEVSAAHRARYFWGNLPGMNRPLASTVNDKLELQECLEHGRIAKFSKVRTITTRSNSIKQGKDQHFPVFMNEKEDILWCTEMERVFGFPVHYTDVSNMSRLARQRLLGRSWSVPVIRHLFAPLKEYFACVSSGNSNANSRGPSFSSGLVPLSLRGSHMFETVPVWRRQPVRVLSLFEDIKKELTSLGFLESGSDPGQLKHVVDVTDTVRKDVEEWGPFDLVYGATPPLGHTCDRPPSWYLFQFHRLLQYARPKPGSPRPFFWMFVDNLVLNKEDLDVASRFLEMEPVTIPDVHGGSLQNAVRVWSNIPAIRSSRHWALVSEEELSLLAQNKQSSKLAAKWPTKLVKNCFLPLREYFKYFSGGPSSGAPPPSGGSPAGSPTSTEEGTSESATPESGPGTSTEPSEGSAPGSPAGSPTSTEEGTSTEPSEGSAPGTSTEPSEPKKKRKVMGITMSDTTFRPYKSKLNPNERKMPMVVDTMNWCDNACSVFFDLFVGLYGGVKIGDVTNFLTEKQDTTTDADLLCAINWFRAMPVSNPDAVVGPEQLVVRFRDYSGHNPSPMASMYLSAPVNPRYTWVDCRFLYQQMCQTLGANLDVDISTLVQTGLLPIQKDTQLNAYSFCSNVFGEGVKEDPSAKVTSYTAAANALSGATNPIITYEDYRQILSSAITNRPSRKGAKDILAADLDSTKTGVLPGNYVSQRIAMYQASAASKARGVVLPNRLRVKAYLQNLVGLNYICTTWAAPMLRAVGDIKSKNSNNYRFVGERLERQQEIDNLLAVSNIRSAQAILQQFRANESNQFYIKKRHIGKGLPSLYDMWDLMDEKEGIDNYIQSLKGDKTERLPIRELLQIIYPHRKSVSAELFLSAAELTDVEDRQNRCMVHPTVRGSLVINFGKSSTIFGAITPPDTLIKFRGEMVPAGQTGMIWFTMHLVDGGKWVKHHIPCHSSRYFEEIYAWKKDLPTLPFPRRSLYGYAIGNKISDTRKIDLRRKKASKQYLRTLENMTHNVEFDPTTQFMVDQELNVTITARVKKIPPVRDVPVGSRIMGLNKNQTIRDCYSIWERVEANTSGSFQHPVVQDVWLRLVADGHVTSTVNGPNGQIDQMSYSGPDVANCGNWMQERSNFITSVDDADQSIMKHFLWNNRVKLYAWNCVYAGTLMKAISKQMTTANRNLFRNEILSFVGGRFGCRLGSLAQVSLDLLRRMKSVISCYFSRNNAFTIEERSAFDKELMELFESLDNKMNNKRKEKVNRTLSSIFQVAKQHNVVRLVVTKNLQTPDANVRSVMNQRSVDWCARKIEEKIVDLGNVIGIYVDLVEALDLSHLDPFIYIAKGDVGKECQFDEVESSSLLPIHTSMFRDWHGLVNKGRTTTPIYHSALRSFASHYGLRFDDLARIKAAELAKMLPDQKVFIPHRGGRFFMSTYPVTSTSRPVSYDGRQRFLNSGDMVAPVNTMLRGFRRARSAYPYDVPDYASLGSGSPKKKRKVEDPKKKRKVDGIGSGSNGSSGEELLSKNYHLENEVARLKKGSGSGGSGSGGSGSGSGGSGSGGSGSGEELLSKNYHGSGSGQRGSKRTADGSEFESPKKKRKVX

SEQ ID NO: 93 - protein, 358 aa, synthetic construct
  REGION 1..358: note = (from V20)_KRAB-scFv
  SITE 358: note = misc_feature - Xaa =
MPAAKRVKLDGSRTLVTFKDVFVDFTREEWKLLDTAQQIVYRNVMLENYKNLVSLGYQLTKPDVILRLEKGEEPGSGMGPDIVMTQSPSSLSASVGDRVTITCRSSTGAVTTSNYASWVQEKPGKLFKGLIGGTNNRAPGVPSRFSGSLIGDKATLTISSLQPEDFATYFCALWYSNHWVFGQGTKVELKRGGGGSGGGGSGGGGSSGGGSEVKLLESGGGLVQPGGSLKLSCAVSGFSLTDYGVNWVRQAPGRGLEWIGVIWGDGITDYNSALKDRFIISKDNGKNTVYLQMSKVRSDDTALYYCVTGLFDYWGQGTLVTVSSYPYDVPDYAGGGGGSGGGGSGGGGSGGGGSGSGX

SEQ ID NO: 94 - protein, 1554 aa, synthetic construct
  REGION 1..1554: note = (from V22)_1xGCN4-dCas9-KRAB
  SITE 1554: note = misc_feature - Xaa =
MPAAKRVKLDGSGSGGSGSGEELLSKNYHLENEVARLKKGSGSGGSGSGGSGSGSGGSGSGGSGSGPKKKRKVMDKKYSIGLAIGTNSVGWAVITDEYKVPSKKFKVLGNTDRHSIKKNLIGALLFDSGETAEATRLKRTARRRYTRRKNRICYLQEIFSNEMAKVDDSFFHRLEESFLVEEDKKHERHPIFGNIVDEVAYHEKYPTIYHLRKKLVDSTDKADLRLIYLALAHMIKFRGHFLIEGDLNPDNSDVDKLFIQLVQTYNQLFEENPINASGVDAKAILSARLSKSRRLENLIAQLPGEKKNGLFGNLIALSLGLTPNFKSNFDLAEDAKLQLSKDTYDDDLDNLLAQIGDQYADLFLAAKNLSDAILLSDILRVNTEITKAPLSASMIKRYDEHHQDLTLLKALVRQQLPEKYKEIFFDQSKNGYAGYIDGGASQEEFYKFIKPILEKMDGTEELLVKLNREDLLRKQRTFDNGSIPHQIHLGELHAILRRQEDFYPFLKDNREKIEKILTFRIPYYVGPLARGNSRFAWMTRKSEETITPWNFEEVVDKGASAQSFIERMTNFDKNLPNEKVLPKHSLLYEYFTVYNELTKVKYVTEGMRKPAFLSGEQKKAIVDLLFKTNRKVTVKQLKEDYFKKIECFDSVEISGVEDRFNASLGTYHDLLKIIKDKDFLDNEENEDILEDIVLTLTLFEDREMIEERLKTYAHLFDDKVMKQLKRRRYTGWGRLSRKLINGIRDKQSGKTILDFLKSDGFANRNFMQLIHDDSLTFKEDIQKAQVSGQGDSLHEHIANLAGSPAIKKGILQTVKVVDELVKVMGRHKPENIVIEMARENQTTQKGQKNSRERMKRIEEGIKELGSQILKEHPVENTQLQNEKLYLYYLQNGRDMYVDQELDINRLSDYDVDAIVPQSFLKDDSIDNKVLTRSDKNRGKSDNVPSEEVVKKMKNYWRQLLNAKLITQRKFDNLTKAERGGLSELDKAGFIKRQLVETRQITKHVAQILDSRMNTKYDENDKLIREVKVITLKSKLVSDFRKDFQFYKVREINNYHHAHDAYLNAVVGTALIKKYPKLESEFVYGDYKVYDVRKMIAKSEQEIGKATAKYFFYSNIMNFFKTEITLANGEIRKRPLIETNGETGEIVWDKGRDFATVRKVLSMPQVNIVKKTEVQTGGFSKESILPKRNSDKLIARKKDWDPKKYGGFDSPTVAYSVLVVAKVEKGKSKKLKSVKELLGITIMERSSFEKNPIDFLEAKGYKEVKKDLIIKLPKYSLFELENGRKRMLASAGELQKGNELALPSKYVNFLYLASHYEKLKGSPEDNEQKQLFVEQHKHYLDEIIEQISEFSKRVILADANLDKVLSAYNKHRDKPIREQAENIIHLFTLTNLGAPAAFKYFDTTIDRKRYTSTKEVLDATLIHQSITGLYETRIDLSQLGGDAYPYDVPDYASLGSGSPKKKRKVEDPKKKRKVDGSGSETPGTSESATPESRTLVTFKDVFVDFTREEWKLLDTAQQIVYRNVMLENYKNLVSLGYQLTKPDVILRLEKGEEPX

SEQ ID NO: 95 - protein, 1592 aa, synthetic construct
  REGION 1..1592: note = (from V23)_2xGCN4-dCas9-KRAB
  SITE 1592: note = misc_feature - Xaa =
MPAAKRVKLDGSEELLSKNYHLENEVARLKKGSGSGGSGSGGSGSGSGGSGSGGSGSGEELLSKNYHLENEVARLKKGSGSGGSGSGGSGSGSGGSGSGGSGSGPKKKRKVMDKKYSIGLAIGTNSVGWAVITDEYKVPSKKFKVLGNTDRHSIKKNLIGALLFDSGETAEATRLKRTARRRYTRRKNRICYLQEIFSNEMAKVDDSFFHRLEESFLVEEDKKHERHPIFGNIVDEVAYHEKYPTIYHLRKKLVDSTDKADLRLIYLALAHMIKFRGHFLIEGDLNPDNSDVDKLFIQLVQTYNQLFEENPINASGVDAKAILSARLSKSRRLENLIAQLPGEKKNGLFGNLIALSLGLTPNFKSNFDLAEDAKLQLSKDTYDDDLDNLLAQIGDQYADLFLAAKNLSDAILLSDILRVNTEITKAPLSASMIKRYDEHHQDLTLLKALVRQQLPEKYKEIFFDQSKNGYAGYIDGGASQEEFYKFIKPILEKMDGTEELLVKLNREDLLRKQRTFDNGSIPHQIHLGELHAILRRQEDFYPFLKDNREKIEKILTFRIPYYVGPLARGNSRFAWMTRKSEETITPWNFEEVVDKGASAQSFIERMTNFDKNLPNEKVLPKHSLLYEYFTVYNELTKVKYVTEGMRKPAFLSGEQKKAIVDLLFKTNRKVTVKQLKEDYFKKIECFDSVEISGVEDRFNASLGTYHDLLKIIKDKDFLDNEENEDILEDIVLTLTLFEDREMIEERLKTYAHLFDDKVMKQLKRRRYTGWGRLSRKLINGIRDKQSGKTILDFLKSDGFANRNFMQLIHDDSLTFKEDIQKAQVSGQGDSLHEHIANLAGSPAIKKGILQTVKVVDELVKVMGRHKPENIVIEMARENQTTQKGQKNSRERMKRIEEGIKELGSQILKEHPVENTQLQNEKLYLYYLQNGRDMYVDQELDINRLSDYDVDAIVPQSFLKDDSIDNKVLTRSDKNRGKSDNVPSEEVVKKMKNYWRQLLNAKLITQRKFDNLTKAERGGLSELDKAGFIKRQLVETRQITKHVAQILDSRMNTKYDENDKLIREVKVITLKSKLVSDFRKDFQFYKVREINNYHHAHDAYLNAVVGTALIKKYPKLESEFVYGDYKVYDVRKMIAKSEQEIGKATAKYFFYSNIMNFFKTEITLANGEIRKRPLIETNGETGEIVWDKGRDFATVRKVLSMPQVNIVKKTEVQTGGFSKESILPKRNSDKLIARKKDWDPKKYGGFDSPTVAYSVLVVAKVEKGKSKKLKSVKELLGITIMERSSFEKNPIDFLEAKGYKEVKKDLIIKLPKYSLFELENGRKRMLASAGELQKGNELALPSKYVNFLYLASHYEKLKGSPEDNEQKQLFVEQHKHYLDEIIEQISEFSKRVILADANLDKVLSAYNKHRDKPIREQAENIIHLFTLTNLGAPAAFKYFDTTIDRKRYTSTKEVLDATLIHQSITGLYETRIDLSQLGGDAYPYDVPDYASLGSGSPKKKRKVEDPKKKRKVDGSGSETPGTSESATPESRTLVTFKDVFVDFTREEWKLLDTAQQIVYRNVMLENYKNLVSLGYQLTKPDVILRLEKGEEPX

SEQ ID NO: 96 - protein, 1730 aa, synthetic construct
  REGION 1..1730: note = (from V25)_5xGCN4-dCas9-KRAB
  SITE 1730: note = misc_feature - Xaa =
MPAAKRVKLDGSEELLSKNYHLENEVARLKKGSGSGGSGSGGSGSGSGGSGSGGSGSGEELLSKNYHLENEVARLKKGSGSGGSGSGGSGSGSGGSGSGGSGSGEELLSKNYHLENEVARLKKGSGSGGSGSGGSGSGSGGSGSGGSGSGEELLSKNYHLENEVARLKKGSGSGGSGSGGSGSGSGGSGSGGSGSGEELLSKNYHLENEVARLKKGSGSGGSGSGGSGSGSGGSGSGGSGSGPKKKRKVMDKKYSIGLAIGTNSVGWAVITDEYKVPSKKFKVLGNTDRHSIKKNLIGALLFDSGETAEATRLKRTARRRYTRRKNRICYLQEIFSNEMAKVDDSFFHRLEESFLVEEDKKHERHPIFGNIVDEVAYHEKYPTIYHLRKKLVDSTDKADLRLIYLALAHMIKFRGHFLIEGDLNPDNSDVDKLFIQLVQTYNQLFEENPINASGVDAKAILSARLSKSRRLENLIAQLPGEKKNGLFGNLIALSLGLTPNFKSNFDLAEDAKLQLSKDTYDDDLDNLLAQIGDQYADLFLAAKNLSDAILLSDILRVNTEITKAPLSASMIKRYDEHHQDLTLLKALVRQQLPEKYKEIFFDQSKNGYAGYIDGGASQEEFYKFIKPILEKMDGTEELLVKLNREDLLRKQRTFDNGSIPHQIHLGELHAILRRQEDFYPFLKDNREKIEKILTFRIPYYVGPLARGNSRFAWMTRKSEETITPWNFEEVVDKGASAQSFIERMTNFDKNLPNEKVLPKHSLLYEYFTVYNELTKVKYVTEGMRKPAFLSGEQKKAIVDLLFKTNRKVTVKQLKEDYFKKIECFDSVEISGVEDRFNASLGTYHDLLKIIKDKDFLDNEENEDILEDIVLTLTLFEDREMIEERLKTYAHLFDDKVMKQLKRRRYTGWGRLSRKLINGIRDKQSGKTILDFLKSDGFANRNFMQLIHDDSLTFKEDIQKAQVSGQGDSLHEHIANLAGSPAIKKGILQTVKVVDELVKVMGRHKPENIVIEMARENQTTQKGQKNSRERMKRIEEGIKELGSQILKEHPVENTQLQNEKLYLYYLQNGRDMYVDQELDINRLSDYDVDAIVPQSFLKDDSIDNKVLTRSDKNRGKSDNVPSEEVVKKMKNYWRQLLNAKLITQRKFDNLTKAERGGLSELDKAGFIKRQLVETRQITKHVAQILDSRMNTKYDENDKLIREVKVITLKSKLVSDFRKDFQFYKVREINNYHHAHDAYLNAVVGTALIKKYPKLESEFVYGDYKVYDVRKMIAKSEQEIGKATAKYFFYSNIMNFFKTEITLANGEIRKRPLIETNGETGEIVWDKGRDFATVRKVLSMPQVNIVKKTEVQTGGFSKESILPKRNSDKLIARKKDWDPKKYGGFDSPTVAYSVLVVAKVEKGKSKKLKSVKELLGITIMERSSFEKNPIDFLEAKGYKEVKKDLIIKLPKYSLFELENGRKRMLASAGELQKGNELALPSKYVNFLYLASHYEKLKGSPEDNEQKQLFVEQHKHYLDEIIEQISEFSKRVILADANLDKVLSAYNKHRDKPIREQAENIIHLFTLTNLGAPAAFKYFDTTIDRKRYTSTKEVLDATLIHQSITGLYETRIDLSQLGGDAYPYDVPDYASLGSGSPKKKRKVEDPKKKRKVDGSGSETPGTSESATPESRTLVTFKDVFVDFTREEWKLLDTAQQIVYRNVMLENYKNLVSLGYQLTKPDVILRLEKGEEPX

SEQ ID NO: 97 - protein, 913 aa, synthetic construct
  REGION 1..913: note = (from V26)_D3a-hD3l-scFv
  SITE 913: note = misc_feature - Xaa =
MPAAKRVKLDGSNHDQEFDPPKVYPPVPAEKRKPIRVLSLFDGIATGLLVLKDLGIQVDRYIASEVCEDSITVGMVRHQGKIMYVGDVRSVTQKHIQEWGPFDLVIGGSPCNDLSIVNPARKGLYEGTGRLFFEFYRLLHDARPKEGDDRPFFWLFENVVAMGVSDKRDISRFLESNPVMIDAKEVSAAHRARYFWGNLPGMNRPLASTVNDKLELQECLEHGRIAKFSKVRTITTRSNSIKQGKDQHFPVFMNEKEDILWCTEMERVFGFPVHYTDVSNMSRLARQRLLGRSWSVPVIRHLFAPLKEYFACVSSGNSNANSRGPSFSSGLVPLSLRGSHMFETVPVWRRQPVRVLSLFEDIKKELTSLGFLESGSDPGQLKHVVDVTDTVRKDVEEWGPFDLVYGATPPLGHTCDRPPSWYLFQFHRLLQYARPKPGSPRPFFWMFVDNLVLNKEDLDVASRFLEMEPVTIPDVHGGSLQNAVRVWSNIPAIRSSRHWALVSEEELSLLAQNKQSSKLAAKWPTKLVKNCFLPLREYFKYFSGGPSSGAPPPSGGSPAGSPTSTEEGTSESATPESGPGTSTEPSEGSAPGSPAGSPTSTEEGTSTEPSEGSAPGTSTEPSEPKKKRKVPSEGPDIVMTQSPSSLSASVGDRVTITCRSSTGAVTTSNYASWVQEKPGKLFKGLIGGTNNRAPGVPSRFSGSLIGDKATLTISSLQPEDFATYFCALWYSNHWVFGQGTKVELKRGGGGSGGGGSGGGGSSGGGSEVKLLESGGGLVQPGGSLKLSCAVSGFSLTDYGVNWVRQAPGRGLEWIGVIWGDGITDYNSALKDRFIISKDNGKNTVYLQMSKVRSDDTALYYCVTGLFDYWGQGTLVTVSSYPYDVPDYAGGGGGSGGGGSGGGGSGGGGSGSGX

SEQ ID NO: 98 - protein, 1678 aa, synthetic construct
  REGION 1..1678: note = (from V26)_3xGCN4-dCas9-ZIM3
  SITE 1678: note = misc_feature - Xaa =
MPAAKRVKLDGSEELLSKNYHLENEVARLKKGSGSGGSGSGGSGSGSGGSGSGGSGSGEELLSKNYHLENEVARLKKGSGSGGSGSGGSGSGSGGSGSGGSGSGEELLSKNYHLENEVARLKKGSGSGGSGSGGSGSGSGGSGSGGSGSGPKKKRKVMDKKYSIGLAIGTNSVGWAVITDEYKVPSKKFKVLGNTDRHSIKKNLIGALLFDSGETAEATRLKRTARRRYTRRKNRICYLQEIFSNEMAKVDDSFFHRLEESFLVEEDKKHERHPIFGNIVDEVAYHEKYPTIYHLRKKLVDSTDKADLRLIYLALAHMIKFRGHFLIEGDLNPDNSDVDKLFIQLVQTYNQLFEENPINASGVDAKAILSARLSKSRRLENLIAQLPGEKKNGLFGNLIALSLGLTPNFKSNFDLAEDAKLQLSKDTYDDDLDNLLAQIGDQYADLFLAAKNLSDAILLSDILRVNTEITKAPLSASMIKRYDEHHQDLTLLKALVRQQLPEKYKEIFFDQSKNGYAGYIDGGASQEEFYKFIKPILEKMDGTEELLVKLNREDLLRKQRTFDNGSIPHQIHLGELHAILRRQEDFYPFLKDNREKIEKILTFRIPYYVGPLARGNSRFAWMTRKSEETITPWNFEEVVDKGASAQSFIERMTNFDKNLPNEKVLPKHSLLYEYFTVYNELTKVKYVTEGMRKPAFLSGEQKKAIVDLLFKTNRKVTVKQLKEDYFKKIECFDSVEISGVEDRFNASLGTYHDLLKIIKDKDFLDNEENEDILEDIVLTLTLFEDREMIEERLKTYAHLFDDKVMKQLKRRRYTGWGRLSRKLINGIRDKQSGKTILDFLKSDGFANRNFMQLIHDDSLTFKEDIQKAQVSGQGDSLHEHIANLAGSPAIKKGILQTVKVVDELVKVMGRHKPENIVIEMARENQTTQKGQKNSRERMKRIEEGIKELGSQILKEHPVENTQLQNEKLYLYYLQNGRDMYVDQELDINRLSDYDVDAIVPQSFLKDDSIDNKVLTRSDKNRGKSDNVPSEEVVKKMKNYWRQLLNAKLITQRKFDNLTKAERGGLSELDKAGFIKRQLVETRQITKHVAQILDSRMNTKYDENDKLIREVKVITLKSKLVSDFRKDFQFYKVREINNYHHAHDAYLNAVVGTALIKKYPKLESEFVYGDYKVYDVRKMIAKSEQEIGKATAKYFFYSNIMNFFKTEITLANGEIRKRPLIETNGETGEIVWDKGRDFATVRKVLSMPQVNIVKKTEVQTGGFSKESILPKRNSDKLIARKKDWDPKKYGGFDSPTVAYSVLVVAKVEKGKSKKLKSVKELLGITIMERSSFEKNPIDFLEAKGYKEVKKDLIIKLPKYSLFELENGRKRMLASAGELQKGNELALPSKYVNFLYLASHYEKLKGSPEDNEQKQLFVEQHKHYLDEIIEQISEFSKRVILADANLDKVLSAYNKHRDKPIREQAENIIHLFTLTNLGAPAAFKYFDTTIDRKRYTSTKEVLDATLIHQSITGLYETRIDLSQLGGDAYPYDVPDYASLGSGSPKKKRKVEDPKKKRKVDGSGSETPGTSESATPESMNNSQGRVTFEDVTVNFTQGEWQRLNPEQRNLYRDVMLENYSNLVSVGQGETTKPDVILRLEQGKEPWLEEEEVLGSGRAEKNGDIGGQIWKPKDVKESLLEX

SEQ ID NO: 99 - protein, 1536 aa, synthetic construct
  REGION 1..1536: note = (from V28)_3xGCN4-dCas12a-ZIM3
  SITE 1536: note = misc_feature - Xaa =
MPAAKRVKLDGSEELLSKNYHLENEVARLKKGSGSGGSGSGGSGSGSGGSGSGGSGSGEELLSKNYHLENEVARLKKGSGSGGSGSGGSGSGSGGSGSGGSGSGEELLSKNYHLENEVARLKKGSGSGGSGSGGSGSGSGGSGSGGSGSGPKKKRKVMSKLEKFTNCYSLSKTLRFKAIPVGKTQENIDNKRLLVEDEKRAEDYKGVKKLLDRYYLSFINDVLHSIKLKNLNNYISLFRKKTRTEKENKELENLEINLRKEIAKAFKGNEGYKSLFKKDIIETILPEFLDDKDEIALVNSFNGFTTAFTGFFDNRENMFSEEAKSTSIAFRCINENLTRYISNMDIFEKVDAIFDKHEVQEIKEKILNSDYDVEDFFEGEFFNFVLTQEGIDVYNAIIGGFVTESGEKIKGLNEYINLYNQKTKQKLPKFKPLYKQVLSDRESLSFYGEGYTSDEEVLEVFRNTLNKNSEIFSSIKKLEKLFKNFDEYSSAGIFVKNGPAISTISKDIFGEWNVIRDKWNAEYDDIHLKKKAVVTEKYEDDRRKSFKKIGSFSLEQLQEYADADLSVVEKLKEIIIQKVDEIYKVYGSSEKLFDADFVLEKSLKKNDAVVAIMKDLLDSVKSFENYIKAFFGEGKETNRDESFYGDFVLAYDILLKVDHIYDAIRNYVTQKPYSKDKFKLYFQNPQFMGGWDKDKETDYRATILRYGSKYYLAIMDKKYAKCLQKIDKDDVNGNYEKINYKLLPGPNKMLPKVFFSKKWMAYYNPSEDIQKIYKNGTFKKGDMFNLNDCHKLIDFFKDSISRYPKWSNAYDFNFSETEKYKDIAGFYREVEEQGYKVSFESASKKEVDKLVEEGKLYMFQIYNKDFSDKSHGTPNLHTMYFKLLFDENNHGQIRLSGGAELFMRRASLKKEELVVHPANSPIANKNPDNPKKTTTLSYDVYKDKRFSEDQYELHIPIAINKCPKNIFKINTEVRVLLKHDDNPYVIGIARGERNLLYIVVVDGKGNIVEQYSLNEIINNFNGIRIKTDYHSLLDKKEKERFEARQNWTSIENIKELKAGYISQVVHKICELVEKYDAVIALADLNSGFKNSRVKVEKQVYQKFEKMLIDKLNYMVDKKSNPCATGGALKGYQITNKFESFKSMSTQNGFIFYIPAWLTSKIDPSTGFVNLLKTKYTSIADSKKFISSFDRIMYVPEEDLFEFALDYKNFSRTDADYIKKWKLYSYGNRIRIFRNPKKNNVFDWEEVCLTSAYKELFNKYGINYQQGDIRALLCEQSDKAFYSSFMALMSLMLQMRNSITGRTDVAFLISPVKNSDGIFYDSRNYEAQENAILPKNADANGAYNIARKVLWAIGQFKKAEDEKLDKVKIAISNKEWLEYAQTSVKHAYPYDVPDYASLGSGSPKKKRKVEDPKKKRKVDGSGSETPGTSESATPESMNNSQGRVTFEDVTVNFTQGEWQRLNPEQRNLYRDVMLENYSNLVSVGQGETTKPDVILRLEQGKEPWLEEEEVLGSGRAEKNGDIGGQIWKPKDVKESLX

SEQ ID NO: 100 - protein, 1319 aa, synthetic construct
  REGION 1..1319: note = (from V29)_3xGCN4-dCas12i-ZIM3
  SITE 1319: note = misc_feature - Xaa =
MPAAKRVKLDGSEELLSKNYHLENEVARLKKGSGSGGSGSGGSGSGSGGSGSGGSGSGEELLSKNYHLENEVARLKKGSGSGGSGSGGSGSGSGGSGSGGSGSGEELLSKNYHLENEVARLKKGSGSGGSGSGGSGSGSGGSGSGGSGSGPKKKRKVMGITMSDTTFRPYKSKLNPNERKMPMVVDTMNWCDNACSVFFDLFVGLYGGVKIGDVTNFLTEKQDTTTDADLLCAINWFRAMPVSNPDAVVGPEQLVVRFRDYSGHNPSPMASMYLSAPVNPRYTWVDCRFLYQQMCQTLGANLDVDISTLVQTGLLPIQKDTQLNAYSFCSNVFGEGVKEDPSAKVTSYTAAANALSGATNPIITYEDYRQILSSAITNRPSRKGAKDILAADLDSTKTGVLPGNYVSQRIAMYQASAASKARGVVLPNRLRVKAYLQNLVGLNYICTTWAAPMLRAVGDIKSKNSNNYRFVGERLERQQEIDNLLAVSNIRSAQAILQQFRANESNQFYIKKRHIGKGLPSLYDMWDLMDEKEGIDNYIQSLKGDKTERLPIRELLQIIYPHRKSVSAELFLSAAELTDVEDRQNRCMVHPTVRGSLVINFGKSSTIFGAITPPDTLIKFRGEMVPAGQTGMIWFTMHLVDGGKWVKHHIPCHSSRYFEEIYAWKKDLPTLPFPRRSLYGYAIGNKISDTRKIDLRRKKASKQYLRTLENMTHNVEFDPTTQFMVDQELNVTITARVKKIPPVRDVPVGSRIMGLNKNQTIRDCYSIWERVEANTSGSFQHPVVQDVWLRLVADGHVTSTVNGPNGQIDQMSYSGPDVANCGNWMQERSNFITSVDDADQSIMKHFLWNNRVKLYAWNCVYAGTLMKAISKQMTTANRNLFRNEILSFVGGRFGCRLGSLAQVSLDLLRRMKSVISCYFSRNNAFTIEERSAFDKELMELFESLDNKMNNKRKEKVNRTLSSIFQVAKQHNVVRLVVTKNLQTPDANVRSVMNQRSVDWCARKIEEKIVDLGNVIGIYVDLVEALDLSHLDPFIYIAKGDVGKECQFDEVESSSLLPIHTSMFRDWHGLVNKGRTTTPIYHSALRSFASHYGLRFDDLARIKAAELAKMLPDQKVFIPHRGGRFFMSTYPVTSTSRPVSYDGRQRFLNSGDMVAPVNTMLRGFRRARSAYPYDVPDYASLGSGSPKKKRKVEDPKKKRKVDGSGSETPGTSESATPESMNNSQGRVTFEDVTVNFTQGEWQRLNPEQRNLYRDVMLENYSNLVSVGQGETTKPDVILRLEQGKEPWLEEEEVLGSGRAEKNGDIGGQIWKPKDVKESLX

SEQ ID NO: 101 - protein, 1976 aa, synthetic construct
  REGION 1..1976: note = (from V30)_10xGCN4-dCas9-ZIM3
  SITE 1976: note = misc_feature - Xaa =
MPAAKRVKLDGSEELLSKNYHLENEVARLKKGSGSGGSGSGGSGSGSGGSGSGGSGSGEELLSKNYHLENEVARLKKGSGSGGSGSGGSGSGSGGSGSGGSGSGEELLSKNYHLENEVARLKKGSGSGGSGSGGSGSGSGGSGSGGSGSGEELLSKNYHLENEVARLKKGSGSGGSGSGGSGSGSGGSGSGGSGSGEELLSKNYHLENEVARLKKGSGSGGSGSGGSGSGSGGSGSGGSGSGEELLSKNYHLENEVARLKKGSGSGGSGSGGSGSGSGGSGSGGSGSGEELLSKNYHLENEVARLKKGSGSGGSGSGGSGSGSGGSGSGGSGSGEELLSKNYHLENEVARLKKGSGSGGSGSGGSGSGSGGSGSGGSGSGEELLSKNYHLENEVARLKKGSGSGGSGSGGSGSGSGGSGSGGSGSGEELLSKNYHLENEVARLKKGSGSGPKKKRKVMDKKYSIGLAIGTNSVGWAVITDEYKVPSKKFKVLGNTDRHSIKKNLIGALLFDSGETAEATRLKRTARRRYTRRKNRICYLQEIFSNEMAKVDDSFFHRLEESFLVEEDKKHERHPIFGNIVDEVAYHEKYPTIYHLRKKLVDSTDKADLRLIYLALAHMIKFRGHFLIEGDLNPDNSDVDKLFIQLVQTYNQLFEENPINASGVDAKAILSARLSKSRRLENLIAQLPGEKKNGLFGNLIALSLGLTPNFKSNFDLAEDAKLQLSKDTYDDDLDNLLAQIGDQYADLFLAAKNLSDAILLSDILRVNTEITKAPLSASMIKRYDEHHQDLTLLKALVRQQLPEKYKEIFFDQSKNGYAGYIDGGASQEEFYKFIKPILEKMDGTEELLVKLNREDLLRKQRTFDNGSIPHQIHLGELHAILRRQEDFYPFLKDNREKIEKILTFRIPYYVGPLARGNSRFAWMTRKSEETITPWNFEEVVDKGASAQSFIERMTNFDKNLPNEKVLPKHSLLYEYFTVYNELTKVKYVTEGMRKPAFLSGEQKKAIVDLLFKTNRKVTVKQLKEDYFKKIECFDSVEISGVEDRFNASLGTYHDLLKIIKDKDFLDNEENEDILEDIVLTLTLFEDREMIEERLKTYAHLFDDKVMKQLKRRRYTGWGRLSRKLINGIRDKQSGKTILDFLKSDGFANRNFMQLIHDDSLTFKEDIQKAQVSGQGDSLHEHIANLAGSPAIKKGILQTVKVVDELVKVMGRHKPENIVIEMARENQTTQKGQKNSRERMKRIEEGIKELGSQILKEHPVENTQLQNEKLYLYYLQNGRDMYVDQELDINRLSDYDVDAIVPQSFLKDDSIDNKVLTRSDKNRGKSDNVPSEEVVKKMKNYWRQLLNAKLITQRKFDNLTKAERGGLSELDKAGFIKRQLVETRQITKHVAQILDSRMNTKYDENDKLIREVKVITLKSKLVSDFRKDFQFYKVREINNYHHAHDAYLNAVVGTALIKKYPKLESEFVYGDYKVYDVRKMIAKSEQEIGKATAKYFFYSNIMNFFKTEITLANGEIRKRPLIETNGETGEIVWDKGRDFATVRKVLSMPQVNIVKKTEVQTGGFSKESILPKRNSDKLIARKKDWDPKKYGGFDSPTVAYSVLVVAKVEKGKSKKLKSVKELLGITIMERSSFEKNPIDFLEAKGYKEVKKDLIIKLPKYSLFELENGRKRMLASAGELQKGNELALPSKYVNFLYLASHYEKLKGSPEDNEQKQLFVEQHKHYLDEIIEQISEFSKRVILADANLDKVLSAYNKHRDKPIREQAENIIHLFTLTNLGAPAAFKYFDTTIDRKRYTSTKEVLDATLIHQSITGLYETRIDLSQLGGDAYPYDVPDYASLGSGSPKKKRKVEDPKKKRKVDGSGSETPGTSESATPESMNNSQGRVTFEDVTVNFTQGEWQRLNPEQRNLYRDVMLENYSNLVSVGQGETTKPDVILRLEQGKEPWLEEEEVLGSGRAEKNGDIGGQIWKPKDVKESLX

SEQ ID NO: 102 - protein, 828 aa, synthetic construct
  REGION 1..828: note = (from V31)_scFv-hD3l-D3a
  SITE 828: note = misc_feature - Xaa =
MPAAKRVKLDGSGPDIVMTQSPSSLSASVGDRVTITCRSSTGAVTTSNYASWVQEKPGKLFKGLIGGTNNRAPGVPSRFSGSLIGDKATLTISSLQPEDFATYFCALWYSNHWVFGQGTKVELKRGGGGSGGGGSGGGGSSGGGSEVKLLESGGGLVQPGGSLKLSCAVSGFSLTDYGVNWVRQAPGRGLEWIGVIWGDGITDYNSALKDRFIISKDNGKNTVYLQMSKVRSDDTALYYCVTGLFDYWGQGTLVTVSSYPYDVPDYAGGGGGSGGGGSGGGGSGGGGSMFETVPVWRRQPVRVLSLFEDIKKELTSLGFLESGSDPGQLKHVVDVTDTVRKDVEEWGPFDLVYGATPPLGHTCDRPPSWYLFQFHRLLQYARPKPGSPRPFFWMFVDNLVLNKEDLDVASRFLEMEPVTIPDVHGGSLQNAVRVWSNIPAIRSSRHWALVSEEELSLLAQNKQSSKLAAKWPTKLVKNCFLPLREYFKYFSTELTSSLSSGNSNANSRGPSFSSGLVPLSLRGSHMNHDQEFDPPKVYPPVPAEKRKPIRVLSLFDGIATGLLVLKDLGIQVDRYIASEVCEDSITVGMVRHQGKIMYVGDVRSVTQKHIQEWGPFDLVIGGSPCNDLSIVNPARKGLYEGTGRLFFEFYRLLHDARPKEGDDRPFFWLFENVVAMGVSDKRDISRFLESNPVMIDAKEVSAAHRARYFWGNLPGMNRPLASTVNDKLELQECLEHGRIAKFSKVRTITTRSNSIKQGKDQHFPVFMNEKEDILWCTEMERVFGFPVHYTDVSNMSRLARQRLLGRSWSVPVIRHLFAPLKEYFACVX

SEQ ID NO: 103 - protein, 159 aa, synthetic construct
  REGION 1..159: note = (from V32)_1xGCN4-ZIM3
  SITE 159: note = misc_feature - Xaa =
MPAAKRVKLDGSEELLSKNYHLENEVARLKKGSGSGGSGSGGSGSGSGGSGSGGSGSGMNNSQGRVTFEDVTVNFTQGEWQRLNPEQRNLYRDVMLENYSNLVSVGQGETTKPDVILRLEQGKEPWLEEEEVLGSGRAEKNGDIGGQIWKPKDVKESLX

SEQ ID NO: 104 - protein, 2314 aa, synthetic construct
  REGION 1..2314: note = (from V32)_D3a-hD3l-dCas9-scFv
  SITE 2314: note = misc_feature - Xaa =
MPAAKRVKLDGSNHDQEFDPPKVYPPVPAEKRKPIRVLSLFDGIATGLLVLKDLGIQVDRYIASEVCEDSITVGMVRHQGKIMYVGDVRSVTQKHIQEWGPFDLVIGGSPCNDLSIVNPARKGLYEGTGRLFFEFYRLLHDARPKEGDDRPFFWLFENVVAMGVSDKRDISRFLESNPVMIDAKEVSAAHRARYFWGNLPGMNRPLASTVNDKLELQECLEHGRIAKFSKVRTITTRSNSIKQGKDQHFPVFMNEKEDILWCTEMERVFGFPVHYTDVSNMSRLARQRLLGRSWSVPVIRHLFAPLKEYFACVSSGNSNANSRGPSFSSGLVPLSLRGSHMFETVPVWRRQPVRVLSLFEDIKKELTSLGFLESGSDPGQLKHVVDVTDTVRKDVEEWGPFDLVYGATPPLGHTCDRPPSWYLFQFHRLLQYARPKPGSPRPFFWMFVDNLVLNKEDLDVASRFLEMEPVTIPDVHGGSLQNAVRVWSNIPAIRSSRHWALVSEEELSLLAQNKQSSKLAAKWPTKLVKNCFLPLREYFKYFSGGPSSGAPPPSGGSPAGSPTSTEEGTSESATPESGPGTSTEPSEGSAPGSPAGSPTSTEEGTSTEPSEGSAPGTSTEPSEPKKKRKVMDKKYSIGLAIGTNSVGWAVITDEYKVPSKKFKVLGNTDRHSIKKNLIGALLFDSGETAEATRLKRTARRRYTRRKNRICYLQEIFSNEMAKVDDSFFHRLEESFLVEEDKKHERHPIFGNIVDEVAYHEKYPTIYHLRKKLVDSTDKADLRLIYLALAHMIKFRGHFLIEGDLNPDNSDVDKLFIQLVQTYNQLFEENPINASGVDAKAILSARLSKSRRLENLIAQLPGEKKNGLFGNLIALSLGLTPNFKSNFDLAEDAKLQLSKDTYDDDLDNLLAQIGDQYADLFLAAKNLSDAILLSDILRVNTEITKAPLSASMIKRYDEHHQDLTLLKALVRQQLPEKYKEIFFDQSKNGYAGYIDGGASQEEFYKFIKPILEKMDGTEELLVKLNREDLLRKQRTFDNGSIPHQIHLGELHAILRRQEDFYPFLKDNREKIEKILTFRIPYYVGPLARGNSRFAWMTRKSEETITPWNFEEVVDKGASAQSFIERMTNFDKNLPNEKVLPKHSLLYEYFTVYNELTKVKYVTEGMRKPAFLSGEQKKAIVDLLFKTNRKVTVKQLKEDYFKKIECFDSVEISGVEDRFNASLGTYHDLLKIIKDKDFLDNEENEDILEDIVLTLTLFEDREMIEERLKTYAHLFDDKVMKQLKRRRYTGWGRLSRKLINGIRDKQSGKTILDFLKSDGFANRNFMQLIHDDSLTFKEDIQKAQVSGQGDSLHEHIANLAGSPAIKKGILQTVKVVDELVKVMGRHKPENIVIEMARENQTTQKGQKNSRERMKRIEEGIKELGSQILKEHPVENTQLQNEKLYLYYLQNGRDMYVDQELDINRLSDYDVDAIVPQSFLKDDSIDNKVLTRSDKNRGKSDNVPSEEVVKKMKNYWRQLLNAKLITQRKFDNLTKAERGGLSELDKAGFIKRQLVETRQITKHVAQILDSRMNTKYDENDKLIREVKVITLKSKLVSDFRKDFQFYKVREINNYHHAHDAYLNAVVGTALIKKYPKLESEFVYGDYKVYDVRKMIAKSEQEIGKATAKYFFYSNIMNFFKTEITLANGEIRKRPLIETNGETGEIVWDKGRDFATVRKVLSMPQVNIVKKTEVQTGGFSKESILPKRNSDKLIARKKDWDPKKYGGFDSPTVAYSVLVVAKVEKGKSKKLKSVKELLGITIMERSSFEKNPIDFLEAKGYKEVKKDLIIKLPKYSLFELENGRKRMLASAGELQKGNELALPSKYVNFLYLASHYEKLKGSPEDNEQKQLFVEQHKHYLDEIIEQISEFSKRVILADANLDKVLSAYNKHRDKPIREQAENIIHLFTLTNLGAPAAFKYFDTTIDRKRYTSTKEVLDATLIHQSITGLYETRIDLSQLGGDAYPYDVPDYASLGSGSPKKKRKVEDPKKKRKVDGIGSGSGPDIVMTQSPSSLSASVGDRVTITCRSSTGAVTTSNYASWVQEKPGKLFKGLIGGTNNRAPGVPSRFSGSLIGDKATLTISSLQPEDFATYFCALWYSNHWVFGQGTKVELKRGGGGSGGGGSGGGGSSGGGSEVKLLESGGGLVQPGGSLKLSCAVSGFSLTDYGVNWVRQAPGRGLEWIGVIWGDGITDYNSALKDRFIISKDNGKNTVYLQMSKVRSDDTALYYCVTGLFDYWGQGTLVTVSSYPYDVPDYAGGGGGSGGGGSGGGGSGGGGSX

SEQ ID NO: 105 - protein, 128 aa, synthetic construct
  REGION 1..128: note = (from V33)_KRAB-1xGCN4
  SITE 128: note = misc_feature - Xaa =
MPAAKRVKLDGSRTLVTFKDVFVDFTREEWKLLDTAQQIVYRNVMLENYKNLVSLGYQLTKPDVILRLEKGEEPGSGMEELLSKNYHLENEVARLKKGSGSGGSGSGGSGSGSGGSGSGGSGSGGSGX

SEQ ID NO: 106 - protein, 667 aa, synthetic construct
  REGION 1..667: note = (from V34)_D3a-D3l-1xGCN4
  SITE 667: note = misc_feature - Xaa =
MPAAKRVKLDGSNHDQEFDPPKVYPPVPAEKRKPIRVLSLFDGIATGLLVLKDLGIQVDRYIASEVCEDSITVGMVRHQGKIMYVGDVRSVTQKHIQEWGPFDLVIGGSPCNDLSIVNPARKGLYEGTGRLFFEFYRLLHDARPKEGDDRPFFWLFENVVAMGVSDKRDISRFLESNPVMIDAKEVSAAHRARYFWGNLPGMNRPLASTVNDKLELQECLEHGRIAKFSKVRTITTRSNSIKQGKDQHFPVFMNEKEDILWCTEMERVFGFPVHYTDVSNMSRLARQRLLGRSWSVPVIRHLFAPLKEYFACVSSGNSNANSRGPSFSSGLVPLSLRGSHMGPMEIYKTVSAWKRQPVRVLSLFRNIDKVLKSLGFLESGSGSGGGTLKYVEDVTNVVRRDVEKWGPFDLVYGSTQPLGSSCDRCPGWYMFQFHRILQYALPRQESQRPFFWIFMDNLLLTEDDQETTTRFLQTEAVTLQDVRGRDYQNAMRVWSNIPGLKSKHAPLTPKEEEYLQAQVRSRSKLDAPKVDLLVKNCLLPLREYFKYFSQNSLPLGGPSSGAPPPSGGSPAGSPTSTEEGTSESATGSGSGGSGSGGSGSGSGGSGSGGSGSGEELLSKNYHLENEVARLKKGSGSGGSGSGGSGSGSGGSGSGGSGSGPKKKRKVX

SEQ ID NO: 107 - protein, 1779 aa, synthetic construct
  REGION 1..1779: note = (from V34)_scFv-dCas9-KRAB
  SITE 1779: note = misc_feature - Xaa =
MPAAKRVKLDGSGPDIVMTQSPSSLSASVGDRVTITCRSSTGAVTTSNYASWVQEKPGKLFKGLIGGTNNRAPGVPSRFSGSLIGDKATLTISSLQPEDFATYFCALWYSNHWVFGQGTKVELKRGGGGSGGGGSGGGGSSGGGSEVKLLESGGGLVQPGGSLKLSCAVSGFSLTDYGVNWVRQAPGRGLEWIGVIWGDGITDYNSALKDRFIISKDNGKNTVYLQMSKVRSDDTALYYCVTGLFDYWGQGTLVTVSSYPYDVPDYAGGGGGSGGGGSGGGGSGGGGSGSGPKKKRKVMDKKYSIGLAIGTNSVGWAVITDEYKVPSKKFKVLGNTDRHSIKKNLIGALLFDSGETAEATRLKRTARRRYTRRKNRICYLQEIFSNEMAKVDDSFFHRLEESFLVEEDKKHERHPIFGNIVDEVAYHEKYPTIYHLRKKLVDSTDKADLRLIYLALAHMIKFRGHFLIEGDLNPDNSDVDKLFIQLVQTYNQLFEENPINASGVDAKAILSARLSKSRRLENLIAQLPGEKKNGLFGNLIALSLGLTPNFKSNFDLAEDAKLQLSKDTYDDDLDNLLAQIGDQYADLFLAAKNLSDAILLSDILRVNTEITKAPLSASMIKRYDEHHQDLTLLKALVRQQLPEKYKEIFFDQSKNGYAGYIDGGASQEEFYKFIKPILEKMDGTEELLVKLNREDLLRKQRTFDNGSIPHQIHLGELHAILRRQEDFYPFLKDNREKIEKILTFRIPYYVGPLARGNSRFAWMTRKSEETITPWNFEEVVDKGASAQSFIERMTNFDKNLPNEKVLPKHSLLYEYFTVYNELTKVKYVTEGMRKPAFLSGEQKKAIVDLLFKTNRKVTVKQLKEDYFKKIECFDSVEISGVEDRFNASLGTYHDLLKIIKDKDFLDNEENEDILEDIVLTLTLFEDREMIEERLKTYAHLFDDKVMKQLKRRRYTGWGRLSRKLINGIRDKQSGKTILDFLKSDGFANRNFMQLIHDDSLTFKEDIQKAQVSGQGDSLHEHIANLAGSPAIKKGILQTVKVVDELVKVMGRHKPENIVIEMARENQTTQKGQKNSRERMKRIEEGIKELGSQILKEHPVENTQLQNEKLYLYYLQNGRDMYVDQELDINRLSDYDVDAIVPQSFLKDDSIDNKVLTRSDKNRGKSDNVPSEEVVKKMKNYWRQLLNAKLITQRKFDNLTKAERGGLSELDKAGFIKRQLVETRQITKHVAQILDSRMNTKYDENDKLIREVKVITLKSKLVSDFRKDFQFYKVREINNYHHAHDAYLNAVVGTALIKKYPKLESEFVYGDYKVYDVRKMIAKSEQEIGKATAKYFFYSNIMNFFKTEITLANGEIRKRPLIETNGETGEIVWDKGRDFATVRKVLSMPQVNIVKKTEVQTGGFSKESILPKRNSDKLIARKKDWDPKKYGGFDSPTVAYSVLVVAKVEKGKSKKLKSVKELLGITIMERSSFEKNPIDFLEAKGYKEVKKDLIIKLPKYSLFELENGRKRMLASAGELQKGNELALPSKYVNFLYLASHYEKLKGSPEDNEQKQLFVEQHKHYLDEIIEQISEFSKRVILADANLDKVLSAYNKHRDKPIREQAENIIHLFTLTNLGAPAAFKYFDTTIDRKRYTSTKEVLDATLIHQSITGLYETRIDLSQLGGDAYPYDVPDYASLGSGSPKKKRKVEDPKKKRKVDGSGSETPGTSESATPESRTLVTFKDVFVDFTREEWKLLDTAQQIVYRNVMLENYKNLVSLGYQLTKPDVILRLEKGEEPX

SEQ ID NO: 108 - protein, 698 aa, synthetic construct
  REGION 1..698: note = (from V35)_1xGCN4-D3l-D3a
  SITE 698: note = misc_feature - Xaa =
MPAAKRVKLDGSGSGGSGSGEELLSKNYHLENEVARLKKGSGSGGSGSGGSGSGSGGSGSGGSGSGTPGTSEGGPSSGAPPPSGGSPAGSPTSTEEGTSESATPESGPGTSTEPSEGSAPGSPAGSPTSTEEGTSTEPSEGSAPGTSTEPSESATPESMFETVPVWRRQPVRVLSLFEDIKKELTSLGFLESGSDPGQLKHVVDVTDTVRKDVEEWGPFDLVYGATPPLGHTCDRPPSWYLFQFHRLLQYARPKPGSPRPFFWMFVDNLVLNKEDLDVASRFLEMEPVTIPDVHGGSLQNAVRVWSNIPAIRSSRHWALVSEEELSLLAQNKQSSKLAAKWPTKLVKNCFLPLREYFKYFSTELTSSLSSGNSNANSRGPSFSSGLVPLSLRGSHMNHDQEFDPPKVYPPVPAEKRKPIRVLSLFDGIATGLLVLKDLGIQVDRYIASEVCEDSITVGMVRHQGKIMYVGDVRSVTQKHIQEWGPFDLVIGGSPCNDLSIVNPARKGLYEGTGRLFFEFYRLLHDARPKEGDDRPFFWLFENVVAMGVSDKRDISRFLESNPVMIDAKEVSAAHRARYFWGNLPGMNRPLASTVNDKLELQECLEHGRIAKFSKVRTITTRSNSIKQGKDQHFPVFMNEKEDILWCTEMERVFGFPVHYTDVSNMSRLARQRLLGRSWSVPVIRHLFAPLKEYFACVX

SEQ ID NO: 109 - protein, 1911 aa, synthetic construct
  REGION 1..1911: note = (from V36)_scFv-dCas9-HP1a
  SITE 1911: note = misc_feature - Xaa =
MPAAKRVKLDGSGPDIVMTQSPSSLSASVGDRVTITCRSSTGAVTTSNYASWVQEKPGKLFKGLIGGTNNRAPGVPSRFSGSLIGDKATLTISSLQPEDFATYFCALWYSNHWVFGQGTKVELKRGGGGSGGGGSGGGGSSGGGSEVKLLESGGGLVQPGGSLKLSCAVSGFSLTDYGVNWVRQAPGRGLEWIGVIWGDGITDYNSALKDRFIISKDNGKNTVYLQMSKVRSDDTALYYCVTGLFDYWGQGTLVTVSSYPYDVPDYAGGGGGSGGGGSGGGGSGGGGSGSGPKKKRKVMDKKYSIGLAIGTNSVGWAVITDEYKVPSKKFKVLGNTDRHSIKKNLIGALLFDSGETAEATRLKRTARRRYTRRKNRICYLQEIFSNEMAKVDDSFFHRLEESFLVEEDKKHERHPIFGNIVDEVAYHEKYPTIYHLRKKLVDSTDKADLRLIYLALAHMIKFRGHFLIEGDLNPDNSDVDKLFIQLVQTYNQLFEENPINASGVDAKAILSARLSKSRRLENLIAQLPGEKKNGLFGNLIALSLGLTPNFKSNFDLAEDAKLQLSKDTYDDDLDNLLAQIGDQYADLFLAAKNLSDAILLSDILRVNTEITKAPLSASMIKRYDEHHQDLTLLKALVRQQLPEKYKEIFFDQSKNGYAGYIDGGASQEEFYKFIKPILEKMDGTEELLVKLNREDLLRKQRTFDNGSIPHQIHLGELHAILRRQEDFYPFLKDNREKIEKILTFRIPYYVGPLARGNSRFAWMTRKSEETITPWNFEEVVDKGASAQSFIERMTNFDKNLPNEKVLPKHSLLYEYFTVYNELTKVKYVTEGMRKPAFLSGEQKKAIVDLLFKTNRKVTVKQLKEDYFKKIECFDSVEISGVEDRFNASLGTYHDLLKIIKDKDFLDNEENEDILEDIVLTLTLFEDREMIEERLKTYAHLFDDKVMKQLKRRRYTGWGRLSRKLINGIRDKQSGKTILDFLKSDGFANRNFMQLIHDDSLTFKEDIQKAQVSGQGDSLHEHIANLAGSPAIKKGILQTVKVVDELVKVMGRHKPENIVIEMARENQTTQKGQKNSRERMKRIEEGIKELGSQILKEHPVENTQLQNEKLYLYYLQNGRDMYVDQELDINRLSDYDVDAIVPQSFLKDDSIDNKVLTRSDKNRGKSDNVPSEEVVKKMKNYWRQLLNAKLITQRKFDNLTKAERGGLSELDKAGFIKRQLVETRQITKHVAQILDSRMNTKYDENDKLIREVKVITLKSKLVSDFRKDFQFYKVREINNYHHAHDAYLNAVVGTALIKKYPKLESEFVYGDYKVYDVRKMIAKSEQEIGKATAKYFFYSNIMNFFKTEITLANGEIRKRPLIETNGETGEIVWDKGRDFATVRKVLSMPQVNIVKKTEVQTGGFSKESILPKRNSDKLIARKKDWDPKKYGGFDSPTVAYSVLVVAKVEKGKSKKLKSVKELLGITIMERSSFEKNPIDFLEAKGYKEVKKDLIIKLPKYSLFELENGRKRMLASAGELQKGNELALPSKYVNFLYLASHYEKLKGSPEDNEQKQLFVEQHKHYLDEIIEQISEFSKRVILADANLDKVLSAYNKHRDKPIREQAENIIHLFTLTNLGAPAAFKYFDTTIDRKRYTSTKEVLDATLIHQSITGLYETRIDLSQLGGDAYPYDVPDYASLGSGSPKKKRKVEDPKKKRKVDGSGSETPGTSESATPESRTLGKKTKRTADSSSSEDEEEYVVEKVLDRRVVKGQVEYLLKWKGFSEEHNTWEPEKNLDCPELISEFMKKYKKMKEGENNKPREKSESNKRKSNFSNSADDIKSKKKREQSNDIARGFERGLEPEKIIGATDSCGDLMFLMKWKDTDEADLVLAKEANVKCPQIVIAFYEERLTWHAYPEDAENKEKETAKSEX

SEQ ID NO: 110 - protein, 2243 aa, synthetic construct
  REGION 1..2243: note = (from V37)_D3a-D3l-dCas9-7xGFP11
  SITE 2243: note = misc_feature - Xaa =
PAAKRVKLDGSNHDQEFDPPKVYPPVPAEKRKPIRVLSLFDGIATGLLVLKDLGIQVDRYIASEVCEDSITVGMVRHQGKIMYVGDVRSVTQKHIQEWGPFDLVIGGSPCNDLSIVNPARKGLYEGTGRLFFEFYRLLHDARPKEGDDRPFFWLFENVVAMGVSDKRDISRFLESNPVMIDAKEVSAAHRARYFWGNLPGMNRPLASTVNDKLELQECLEHGRIAKFSKVRTITTRSNSIKQGKDQHFPVFMNEKEDILWCTEMERVFGFPVHYTDVSNMSRLARQRLLGRSWSVPVIRHLFAPLKEYFACVSSGNSNANSRGPSFSSGLVPLSLRGSHMGPMEIYKTVSAWKRQPVRVLSLFRNIDKVLKSLGFLESGSGSGGGTLKYVEDVTNVVRRDVEKWGPFDLVYGSTQPLGSSCDRCPGWYMFQFHRILQYALPRQESQRPFFWIFMDNLLLTEDDQETTTRFLQTEAVTLQDVRGRDYQNAMRVWSNIPGLKSKHAPLTPKEEEYLQAQVRSRSKLDAPKVDLLVKNCLLPLREYFKYFSQNSLPLGGPSSGAPPPSGGSPAGSPTSTEEGTSESATPESGPGTSTEPSEGSAPGSPAGSPTSTEEGTSTEPSEGSAPGTSTEPSEPKKKRKVMDKKYSIGLAIGTNSVGWAVITDEYKVPSKKFKVLGNTDRHSIKKNLIGALLFDSGETAEATRLKRTARRRYTRRKNRICYLQEIFSNEMAKVDDSFFHRLEESFLVEEDKKHERHPIFGNIVDEVAYHEKYPTIYHLRKKLVDSTDKADLRLIYLALAHMIKFRGHFLIEGDLNPDNSDVDKLFIQLVQTYNQLFEENPINASGVDAKAILSARLSKSRRLENLIAQLPGEKKNGLFGNLIALSLGLTPNFKSNFDLAEDAKLQLSKDTYDDDLDNLLAQIGDQYADLFLAAKNLSDAILLSDILRVNTEITKAPLSASMIKRYDEHHQDLTLLKALVRQQLPEKYKEIFFDQSKNGYAGYIDGGASQEEFYKFIKPILEKMDGTEELLVKLNREDLLRKQRTFDNGSIPHQIHLGELHAILRRQEDFYPFLKDNREKIEKILTFRIPYYVGPLARGNSRFAWMTRKSEETITPWNFEEVVDKGASAQSFIERMTNFDKNLPNEKVLPKHSLLYEYFTVYNELTKVKYVTEGMRKPAFLSGEQKKAIVDLLFKTNRKVTVKQLKEDYFKKIECFDSVEISGVEDRFNASLGTYHDLLKIIKDKDFLDNEENEDILEDIVLTLTLFEDREMIEERLKTYAHLFDDKVMKQLKRRRYTGWGRLSRKLINGIRDKQSGKTILDFLKSDGFANRNFMQLIHDDSLTFKEDIQKAQVSGQGDSLHEHIANLAGSPAIKKGILQTVKVVDELVKVMGRHKPENIVIEMARENQTTQKGQKNSRERMKRIEEGIKELGSQILKEHPVENTQLQNEKLYLYYLQNGRDMYVDQELDINRLSDYDVDAIVPQSFLKDDSIDNKVLTRSDKNRGKSDNVPSEEVVKKMKNYWRQLLNAKLITQRKFDNLTKAERGGLSELDKAGFIKRQLVETRQITKHVAQILDSRMNTKYDENDKLIREVKVITLKSKLVSDFRKDFQFYKVREINNYHHAHDAYLNAVVGTALIKKYPKLESEFVYGDYKVYDVRKMIAKSEQEIGKATAKYFFYSNIMNFFKTEITLANGEIRKRPLIETNGETGEIVWDKGRDFATVRKVLSMPQVNIVKKTEVQTGGFSKESILPKRNSDKLIARKKDWDPKKYGGFDSPTVAYSVLVVAKVEKGKSKKLKSVKELLGITIMERSSFEKNPIDFLEAKGYKEVKKDLIIKLPKYSLFELENGRKRMLASAGELQKGNELALPSKYVNFLYLASHYEKLKGSPEDNEQKQLFVEQHKHYLDEIIEQISEFSKRVILADANLDKVLSAYNKHRDKPIREQAENIIHLFTLTNLGAPAAFKYFDTTIDRKRYTSTKEVLDATLIHQSITGLYETRIDLSQLGGDAYPYDVPDYASLGSGSPKKKRKVEDPKKKRKVDGSGSETPGTSESATPESGSGSNGSSGSMRDHMVLHEYVNAAGITGGSGGRDHMVLHEYVNAAGITGGSGGRDHMVLHEYVNAAGITGGSGGRDHMVLHEYVNAAGITGGSGGRDHMVLHEYVNAAGITGGSGGRDHMVLHEYVNAAGITGGSGGRDHMVLHEYVNAAGITAAARSGSGQRGSKRTADGSEFESPKKKRKVX

SEQ ID NO: 111 - protein, 324 aa, synthetic construct
  REGION 1..324: note = (from v39)_GFP1-10-ZIM3
  SITE 324: note = misc_feature - Xaa =
MSKGEELFTGVVPILVELDGDVNGHKFSVRGEGEGDATIGKLTLKFICTTGKLPVPWPTLVTTLTYGVQCFSRYPDHMKRHDFFKSAMPEGYVQERTISFKDDGKYKTRAVVKFEGDTLVNRIELKGTDFKEDGNILGHKLEYNFNSHNVYITADKQKNGIKANFTVRHNVEDGSVQLADHYQQNTPIGDGPVLLPDNHYLSTQTVLSKDPNEKLDPGGGGSGMNNSQGRVTFEDVTVNFTQGEWQRLNPEQRNLYRDVMLENYSNLVSVGQGETTKPDVILRLEQGKEPWLEEEEVLGSGRAEKNGDIGGQIWKPKDVKESLX

SEQ ID NO: 112 - protein, 2106 aa, synthetic construct
  REGION 1..2106: note = (from V39)_D3a-hD3l-dCas9-1xGFP11
  SITE 2106: note = misc_feature - Xaa =
MPAAKRVKLDGSNHDQEFDPPKVYPPVPAEKRKPIRVLSLFDGIATGLLVLKDLGIQVDRYIASEVCEDSITVGMVRHQGKIMYVGDVRSVTQKHIQEWGPFDLVIGGSPCNDLSIVNPARKGLYEGTGRLFFEFYRLLHDARPKEGDDRPFFWLFENVVAMGVSDKRDISRFLESNPVMIDAKEVSAAHRARYFWGNLPGMNRPLASTVNDKLELQECLEHGRIAKFSKVRTITTRSNSIKQGKDQHFPVFMNEKEDILWCTEMERVFGFPVHYTDVSNMSRLARQRLLGRSWSVPVIRHLFAPLKEYFACVSSGNSNANSRGPSFSSGLVPLSLRGSHMFETVPVWRRQPVRVLSLFEDIKKELTSLGFLESGSDPGQLKHVVDVTDTVRKDVEEWGPFDLVYGATPPLGHTCDRPPSWYLFQFHRLLQYARPKPGSPRPFFWMFVDNLVLNKEDLDVASRFLEMEPVTIPDVHGGSLQNAVRVWSNIPAIRSSRHWALVSEEELSLLAQNKQSSKLAAKWPTKLVKNCFLPLREYFKYFSGGPSSGAPPPSGGSPAGSPTSTEEGTSESATPESGPGTSTEPSEGSAPGSPAGSPTSTEEGTSTEPSEGSAPGTSTEPSEPKKKRKVMDKKYSIGLAIGTNSVGWAVITDEYKVPSKKFKVLGNTDRHSIKKNLIGALLFDSGETAEATRLKRTARRRYTRRKNRICYLQEIFSNEMAKVDDSFFHRLEESFLVEEDKKHERHPIFGNIVDEVAYHEKYPTIYHLRKKLVDSTDKADLRLIYLALAHMIKFRGHFLIEGDLNPDNSDVDKLFIQLVQTYNQLFEENPINASGVDAKAILSARLSKSRRLENLIAQLPGEKKNGLFGNLIALSLGLTPNFKSNFDLAEDAKLQLSKDTYDDDLDNLLAQIGDQYADLFLAAKNLSDAILLSDILRVNTEITKAPLSASMIKRYDEHHQDLTLLKALVRQQLPEKYKEIFFDQSKNGYAGYIDGGASQEEFYKFIKPILEKMDGTEELLVKLNREDLLRKQRTFDNGSIPHQIHLGELHAILRRQEDFYPFLKDNREKIEKILTFRIPYYVGPLARGNSRFAWMTRKSEETITPWNFEEVVDKGASAQSFIERMTNFDKNLPNEKVLPKHSLLYEYFTVYNELTKVKYVTEGMRKPAFLSGEQKKAIVDLLFKTNRKVTVKQLKEDYFKKIECFDSVEISGVEDRFNASLGTYHDLLKIIKDKDFLDNEENEDILEDIVLTLTLFEDREMIEERLKTYAHLFDDKVMKQLKRRRYTGWGRLSRKLINGIRDKQSGKTILDFLKSDGFANRNFMQLIHDDSLTFKEDIQKAQVSGQGDSLHEHIANLAGSPAIKKGILQTVKVVDELVKVMGRHKPENIVIEMARENQTTQKGQKNSRERMKRIEEGIKELGSQILKEHPVENTQLQNEKLYLYYLQNGRDMYVDQELDINRLSDYDVDAIVPQSFLKDDSIDNKVLTRSDKNRGKSDNVPSEEVVKKMKNYWRQLLNAKLITQRKFDNLTKAERGGLSELDKAGFIKRQLVETRQITKHVAQILDSRMNTKYDENDKLIREVKVITLKSKLVSDFRKDFQFYKVREINNYHHAHDAYLNAVVGTALIKKYPKLESEFVYGDYKVYDVRKMIAKSEQEIGKATAKYFFYSNIMNFFKTEITLANGEIRKRPLIETNGETGEIVWDKGRDFATVRKVLSMPQVNIVKKTEVQTGGFSKESILPKRNSDKLIARKKDWDPKKYGGFDSPTVAYSVLVVAKVEKGKSKKLKSVKELLGITIMERSSFEKNPIDFLEAKGYKEVKKDLIIKLPKYSLFELENGRKRMLASAGELQKGNELALPSKYVNFLYLASHYEKLKGSPEDNEQKQLFVEQHKHYLDEIIEQISEFSKRVILADANLDKVLSAYNKHRDKPIREQAENIIHLFTLTNLGAPAAFKYFDTTIDRKRYTSTKEVLDATLIHQSITGLYETRIDLSQLGGDAYPYDVPDYASLGSGSPKKKRKVEDPKKKRKVDGSGSETPGTSESATPESGSGSNGSSGSMRDHMVLHEYVNAAGITAAARSGSGQRGSKRTADGSEFESPKKKRKVX

SEQ ID NO: 113 - protein, 706 aa, synthetic construct
  REGION 1..706: note = (from V40)_GFP1-10-HDAC1
  SITE 706: note = misc_feature - Xaa =
MSKGEELFTGVVPILVELDGDVNGHKFSVRGEGEGDATIGKLTLKFICTTGKLPVPWPTLVTTLTYGVQCFSRYPDHMKRHDFFKSAMPEGYVQERTISFKDDGKYKTRAVVKFEGDTLVNRIELKGTDFKEDGNILGHKLEYNFNSHNVYITADKQKNGIKANFTVRHNVEDGSVQLADHYQQNTPIGDGPVLLPDNHYLSTQTVLSKDPNEKLDPGGGGSGMAQTQGTRRKVCYYYDGDVGNYYYGQGHPMKPHRIRMTHNLLLNYGLYRKMEIYRPHKANAEEMTKYHSDDYIKFLRSIRPDNMSEYSKQMQRFNVGEDCPVFDGLFEFCQLSTGGSVASAVKLNKQQTDIAVNWAGGLHHAKKSEASGFCYVNDIVLAILELLKYHQRVLYIDIDIHHGDGVEEAFYTTDRVMTVSFHKYGEYFPGTGDLRDIGAGKGKYYAVNYPLRDGIDDESYEAIFKPVMSKVMEMFQPSAVVLQCGSDSLSGDRLGCFNLTIKGHAKCVEFVKSFNLPMLMLGGGGYTIRNVARCWTYETAVALDTEIPNELPYNDYFEYFGPDFKLHISPSNMTNQNTNEYLEKIKQRLFENLRMLPHAPGVQMQAIPEDAIPEESGDEDEDDPDKRISICSSDKRIACEEEFSDSEEEGEGGRKNSSNFKKAKRVKTEDEKEKDPEEKKEVTEEEKTKEEKPEAKGVKEEVKLAX

SEQ ID NO: 114 - protein, 1966 aa, synthetic construct
  REGION 1..1966: note = (from V41)_D3a-hD3l-dCas12a-1xGFP11
  SITE 1966: note = misc_feature - Xaa =
MPAAKRVKLDGSNHDQEFDPPKVYPPVPAEKRKPIRVLSLFDGIATGLLVLKDLGIQVDRYIASEVCEDSITVGMVRHQGKIMYVGDVRSVTQKHIQEWGPFDLVIGGSPCNDLSIVNPARKGLYEGTGRLFFEFYRLLHDARPKEGDDRPFFWLFENVVAMGVSDKRDISRFLESNPVMIDAKEVSAAHRARYFWGNLPGMNRPLASTVNDKLELQECLEHGRIAKFSKVRTITTRSNSIKQGKDQHFPVFMNEKEDILWCTEMERVFGFPVHYTDVSNMSRLARQRLLGRSWSVPVIRHLFAPLKEYFACVSSGNSNANSRGPSFSSGLVPLSLRGSHMFETVPVWRRQPVRVLSLFEDIKKELTSLGFLESGSDPGQLKHVVDVTDTVRKDVEEWGPFDLVYGATPPLGHTCDRPPSWYLFQFHRLLQYARPKPGSPRPFFWMFVDNLVLNKEDLDVASRFLEMEPVTIPDVHGGSLQNAVRVWSNIPAIRSSRHWALVSEEELSLLAQNKQSSKLAAKWPTKLVKNCFLPLREYFKYFSGGPSSGAPPPSGGSPAGSPTSTEEGTSESATPESGPGTSTEPSEGSAPGSPAGSPTSTEEGTSTEPSEGSAPGTSTEPSEPKKKRKVMSKLEKFTNCYSLSKTLRFKAIPVGKTQENIDNKRLLVEDEKRAEDYKGVKKLLDRYYLSFINDVLHSIKLKNLNNYISLFRKKTRTEKENKELENLEINLRKEIAKAFKGNEGYKSLFKKDIIETILPEFLDDKDEIALVNSFNGFTTAFTGFFDNRENMFSEEAKSTSIAFRCINENLTRYISNMDIFEKVDAIFDKHEVQEIKEKILNSDYDVEDFFEGEFFNFVLTQEGIDVYNAIIGGFVTESGEKIKGLNEYINLYNQKTKQKLPKFKPLYKQVLSDRESLSFYGEGYTSDEEVLEVFRNTLNKNSEIFSSIKKLEKLFKNFDEYSSAGIFVKNGPAISTISKDIFGEWNVIRDKWNAEYDDIHLKKKAVVTEKYEDDRRKSFKKIGSFSLEQLQEYADADLSVVEKLKEIIIQKVDEIYKVYGSSEKLFDADFVLEKSLKKNDAVVAIMKDLLDSVKSFENYIKAFFGEGKETNRDESFYGDFVLAYDILLKVDHIYDAIRNYVTQKPYSKDKFKLYFQNPQFMGGWDKDKETDYRATILRYGSKYYLAIMDKKYAKCLQKIDKDDVNGNYEKINYKLLPGPNKMLPKVFFSKKWMAYYNPSEDIQKIYKNGTFKKGDMFNLNDCHKLIDFFKDSISRYPKWSNAYDFNFSETEKYKDIAGFYREVEEQGYKVSFESASKKEVDKLVEEGKLYMFQIYNKDFSDKSHGTPNLHTMYFKLLFDENNHGQIRLSGGAELFMRRASLKKEELVVHPANSPIANKNPDNPKKTTTLSYDVYKDKRFSEDQYELHIPIAINKCPKNIFKINTEVRVLLKHDDNPYVIGIARGERNLLYIVVVDGKGNIVEQYSLNEIINNFNGIRIKTDYHSLLDKKEKERFEARQNWTSIENIKELKAGYISQVVHKICELVEKYDAVIALADLNSGFKNSRVKVEKQVYQKFEKMLIDKLNYMVDKKSNPCATGGALKGYQITNKFESFKSMSTQNGFIFYIPAWLTSKIDPSTGFVNLLKTKYTSIADSKKFISSFDRIMYVPEEDLFEFALDYKNFSRTDADYIKKWKLYSYGNRIRIFRNPKKNNVFDWEEVCLTSAYKELFNKYGINYQQGDIRALLCEQSDKAFYSSFMALMSLMLQMRNSITGRTDVAFLISPVKNSDGIFYDSRNYEAQENAILPKNADANGAYNIARKVLWAIGQFKKAEDEKLDKVKIAISNKEWLEYAQTSVKHAYPYDVPDYASLGSGSPKKKRKVEDPKKKRKVDGSGSETPGTSESATPESGSGSNGSSGSMRDHMVLHEYVNAAGITAAARSGSGQRGSKRTADGSEFESPKKKRKVX

SEQ ID NO: 115 - protein, 1749 aa, synthetic construct
  REGION 1..1749: note = (from V42)_D3a-hD3l-dCas12i-1xGFP11
  SITE 1749: note = misc_feature - Xaa =
MPAAKRVKLDGSNHDQEFDPPKVYPPVPAEKRKPIRVLSLFDGIATGLLVLKDLGIQVDRYIASEVCEDSITVGMVRHQGKIMYVGDVRSVTQKHIQEWGPFDLVIGGSPCNDLSIVNPARKGLYEGTGRLFFEFYRLLHDARPKEGDDRPFFWLFENVVAMGVSDKRDISRFLESNPVMIDAKEVSAAHRARYFWGNLPGMNRPLASTVNDKLELQECLEHGRIAKFSKVRTITTRSNSIKQGKDQHFPVFMNEKEDILWCTEMERVFGFPVHYTDVSNMSRLARQRLLGRSWSVPVIRHLFAPLKEYFACVSSGNSNANSRGPSFSSGLVPLSLRGSHMFETVPVWRRQPVRVLSLFEDIKKELTSLGFLESGSDPGQLKHVVDVTDTVRKDVEEWGPFDLVYGATPPLGHTCDRPPSWYLFQFHRLLQYARPKPGSPRPFFWMFVDNLVLNKEDLDVASRFLEMEPVTIPDVHGGSLQNAVRVWSNIPAIRSSRHWALVSEEELSLLAQNKQSSKLAAKWPTKLVKNCFLPLREYFKYFSGGPSSGAPPPSGGSPAGSPTSTEEGTSESATPESGPGTSTEPSEGSAPGSPAGSPTSTEEGTSTEPSEGSAPGTSTEPSEPKKKRKVMGITMSDTTFRPYKSKLNPNERKMPMVVDTMNWCDNACSVFFDLFVGLYGGVKIGDVTNFLTEKQDTTTDADLLCAINWFRAMPVSNPDAVVGPEQLVVRFRDYSGHNPSPMASMYLSAPVNPRYTWVDCRFLYQQMCQTLGANLDVDISTLVQTGLLPIQKDTQLNAYSFCSNVFGEGVKEDPSAKVTSYTAAANALSGATNPIITYEDYRQILSSAITNRPSRKGAKDILAADLDSTKTGVLPGNYVSQRIAMYQASAASKARGVVLPNRLRVKAYLQNLVGLNYICTTWAAPMLRAVGDIKSKNSNNYRFVGERLERQQEIDNLLAVSNIRSAQAILQQFRANESNQFYIKKRHIGKGLPSLYDMWDLMDEKEGIDNYIQSLKGDKTERLPIRELLQIIYPHRKSVSAELFLSAAELTDVEDRQNRCMVHPTVRGSLVINFGKSSTIFGAITPPDTLIKFRGEMVPAGQTGMIWFTMHLVDGGKWVKHHIPCHSSRYFEEIYAWKKDLPTLPFPRRSLYGYAIGNKISDTRKIDLRRKKASKQYLRTLENMTHNVEFDPTTQFMVDQELNVTITARVKKIPPVRDVPVGSRIMGLNKNQTIRDCYSIWERVEANTSGSFQHPVVQDVWLRLVADGHVTSTVNGPNGQIDQMSYSGPDVANCGNWMQERSNFITSVDDADQSIMKHFLWNNRVKLYAWNCVYAGTLMKAISKQMTTANRNLFRNEILSFVGGRFGCRLGSLAQVSLDLLRRMKSVISCYFSRNNAFTIEERSAFDKELMELFESLDNKMNNKRKEKVNRTLSSIFQVAKQHNVVRLVVTKNLQTPDANVRSVMNQRSVDWCARKIEEKIVDLGNVIGIYVDLVEALDLSHLDPFIYIAKGDVGKECQFDEVESSSLLPIHTSMFRDWHGLVNKGRTTTPIYHSALRSFASHYGLRFDDLARIKAAELAKMLPDQKVFIPHRGGRFFMSTYPVTSTSRPVSYDGRQRFLNSGDMVAPVNTMLRGFRRARSAYPYDVPDYASLGSGSPKKKRKVEDPKKKRKVDGSGSETPGTSESATPESGSGSNGSSGSMRDHMVLHEYVNAAGITAAARSGSGQRGSKRTADGSEFESPKKKRKVX

SEQ ID NO: 116 - protein, 801 aa, synthetic construct
  REGION 1..801: note = (from V43)_D3a-D3l-GFP1-10
  SITE 801: note = misc_feature - Xaa =
MPAAKRVKLDGSNHDQEFDPPKVYPPVPAEKRKPIRVLSLFDGIATGLLVLKDLGIQVDRYIASEVCEDSITVGMVRHQGKIMYVGDVRSVTQKHIQEWGPFDLVIGGSPCNDLSIVNPARKGLYEGTGRLFFEFYRLLHDARPKEGDDRPFFWLFENVVAMGVSDKRDISRFLESNPVMIDAKEVSAAHRARYFWGNLPGMNRPLASTVNDKLELQECLEHGRIAKFSKVRTITTRSNSIKQGKDQHFPVFMNEKEDILWCTEMERVFGFPVHYTDVSNMSRLARQRLLGRSWSVPVIRHLFAPLKEYFACVSSGNSNANSRGPSFSSGLVPLSLRGSHMGPMEIYKTVSAWKRQPVRVLSLFRNIDKVLKSLGFLESGSGSGGGTLKYVEDVTNVVRRDVEKWGPFDLVYGSTQPLGSSCDRCPGWYMFQFHRILQYALPRQESQRPFFWIFMDNLLLTEDDQETTTRFLQTEAVTLQDVRGRDYQNAMRVWSNIPGLKSKHAPLTPKEEEYLQAQVRSRSKLDAPKVDLLVKNCLLPLREYFKYFSQNSLPLGGPSSGAPPPSGGSPAGSPTSTEEGTSESATMSKGEELFTGVVPILVELDGDVNGHKFSVRGEGEGDATIGKLTLKFICTTGKLPVPWPTLVTTLTYGVQCFSRYPDHMKRHDFFKSAMPEGYVQERTISFKDDGKYKTRAVVKFEGDTLVNRIELKGTDFKEDGNILGHKLEYNFNSHNVYITADKQKNGIKANFTVRHNVEDGSVQLADHYQQNTPIGDGPVLLPDNHYLSTQTVLSKDPNEKX

SEQ ID NO: 117 - protein, 1562 aa, synthetic construct
  REGION 1..1562: note = (from V43)_1xGFP11-dCas9-KRAB
  SITE 1562: note = misc_feature - Xaa =
MPAAKRVKLDGSGPDIVIGSGGRDHMVLHEYVNAAGITAAARSGSGQRGSKRTADGSEFESPKKKRKVGGSGSGPKKKRKVMDKKYSIGLAIGTNSVGWAVITDEYKVPSKKFKVLGNTDRHSIKKNLIGALLFDSGETAEATRLKRTARRRYTRRKNRICYLQEIFSNEMAKVDDSFFHRLEESFLVEEDKKHERHPIFGNIVDEVAYHEKYPTIYHLRKKLVDSTDKADLRLIYLALAHMIKFRGHFLIEGDLNPDNSDVDKLFIQLVQTYNQLFEENPINASGVDAKAILSARLSKSRRLENLIAQLPGEKKNGLFGNLIALSLGLTPNFKSNFDLAEDAKLQLSKDTYDDDLDNLLAQIGDQYADLFLAAKNLSDAILLSDILRVNTEITKAPLSASMIKRYDEHHQDLTLLKALVRQQLPEKYKEIFFDQSKNGYAGYIDGGASQEEFYKFIKPILEKMDGTEELLVKLNREDLLRKQRTFDNGSIPHQIHLGELHAILRRQEDFYPFLKDNREKIEKILTFRIPYYVGPLARGNSRFAWMTRKSEETITPWNFEEVVDKGASAQSFIERMTNFDKNLPNEKVLPKHSLLYEYFTVYNELTKVKYVTEGMRKPAFLSGEQKKAIVDLLFKTNRKVTVKQLKEDYFKKIECFDSVEISGVEDRFNASLGTYHDLLKIIKDKDFLDNEENEDILEDIVLTLTLFEDREMIEERLKTYAHLFDDKVMKQLKRRRYTGWGRLSRKLINGIRDKQSGKTILDFLKSDGFANRNFMQLIHDDSLTFKEDIQKAQVSGQGDSLHEHIANLAGSPAIKKGILQTVKVVDELVKVMGRHKPENIVIEMARENQTTQKGQKNSRERMKRIEEGIKELGSQILKEHPVENTQLQNEKLYLYYLQNGRDMYVDQELDINRLSDYDVDAIVPQSFLKDDSIDNKVLTRSDKNRGKSDNVPSEEVVKKMKNYWRQLLNAKLITQRKFDNLTKAERGGLSELDKAGFIKRQLVETRQITKHVAQILDSRMNTKYDENDKLIREVKVITLKSKLVSDFRKDFQFYKVREINNYHHAHDAYLNAVVGTALIKKYPKLESEFVYGDYKVYDVRKMIAKSEQEIGKATAKYFFYSNIMNFFKTEITLANGEIRKRPLIETNGETGEIVWDKGRDFATVRKVLSMPQVNIVKKTEVQTGGFSKESILPKRNSDKLIARKKDWDPKKYGGFDSPTVAYSVLVVAKVEKGKSKKLKSVKELLGITIMERSSFEKNPIDFLEAKGYKEVKKDLIIKLPKYSLFELENGRKRMLASAGELQKGNELALPSKYVNFLYLASHYEKLKGSPEDNEQKQLFVEQHKHYLDEIIEQISEFSKRVILADANLDKVLSAYNKHRDKPIREQAENIIHLFTLTNLGAPAAFKYFDTTIDRKRYTSTKEVLDATLIHQSITGLYETRIDLSQLGGDAYPYDVPDYASLGSGSPKKKRKVEDPKKKRKVDGSGSETPGTSESATPESRTLVTFKDVFVDFTREEWKLLDTAQQIVYRNVMLENYKNLVSLGYQLTKPDVILRLEKGEEPX

SEQ ID NO: 118 - protein, 1717 aa, synthetic construct
  REGION 1..1717: note = (from V44)_7xGFP11-dCas9-ZIM3
  SITE 1717: note = misc_feature - Xaa =
MPAAKRVKLDGSMRDHMVLHEYVNAAGITGGSGGRDHMVLHEYVNAAGITGGSGGRDHMVLHEYVNAAGITGGSGGRDHMVLHEYVNAAGITGGSGGRDHMVLHEYVNAAGITGGSGGRDHMVLHEYVNAAGITGGSGGRDHMVLHEYVNAAGITAAARSGSGQRGSKRTADGSEFESPKKKRKVGGSGSGPKKKRKVMDKKYSIGLAIGTNSVGWAVITDEYKVPSKKFKVLGNTDRHSIKKNLIGALLFDSGETAEATRLKRTARRRYTRRKNRICYLQEIFSNEMAKVDDSFFHRLEESFLVEEDKKHERHPIFGNIVDEVAYHEKYPTIYHLRKKLVDSTDKADLRLIYLALAHMIKFRGHFLIEGDLNPDNSDVDKLFIQLVQTYNQLFEENPINASGVDAKAILSARLSKSRRLENLIAQLPGEKKNGLFGNLIALSLGLTPNFKSNFDLAEDAKLQLSKDTYDDDLDNLLAQIGDQYADLFLAAKNLSDAILLSDILRVNTEITKAPLSASMIKRYDEHHQDLTLLKALVRQQLPEKYKEIFFDQSKNGYAGYIDGGASQEEFYKFIKPILEKMDGTEELLVKLNREDLLRKQRTFDNGSIPHQIHLGELHAILRRQEDFYPFLKDNREKIEKILTFRIPYYVGPLARGNSRFAWMTRKSEETITPWNFEEVVDKGASAQSFIERMTNFDKNLPNEKVLPKHSLLYEYFTVYNELTKVKYVTEGMRKPAFLSGEQKKAIVDLLFKTNRKVTVKQLKEDYFKKIECFDSVEISGVEDRFNASLGTYHDLLKIIKDKDFLDNEENEDILEDIVLTLTLFEDREMIEERLKTYAHLFDDKVMKQLKRRRYTGWGRLSRKLINGIRDKQSGKTILDFLKSDGFANRNFMQLIHDDSLTFKEDIQKAQVSGQGDSLHEHIANLAGSPAIKKGILQTVKVVDELVKVMGRHKPENIVIEMARENQTTQKGQKNSRERMKRIEEGIKELGSQILKEHPVENTQLQNEKLYLYYLQNGRDMYVDQELDINRLSDYDVDAIVPQSFLKDDSIDNKVLTRSDKNRGKSDNVPSEEVVKKMKNYWRQLLNAKLITQRKFDNLTKAERGGLSELDKAGFIKRQLVETRQITKHVAQILDSRMNTKYDENDKLIREVKVITLKSKLVSDFRKDFQFYKVREINNYHHAHDAYLNAVVGTALIKKYPKLESEFVYGDYKVYDVRKMIAKSEQEIGKATAKYFFYSNIMNFFKTEITLANGEIRKRPLIETNGETGEIVWDKGRDFATVRKVLSMPQVNIVKKTEVQTGGFSKESILPKRNSDKLIARKKDWDPKKYGGFDSPTVAYSVLVVAKVEKGKSKKLKSVKELLGITIMERSSFEKNPIDFLEAKGYKEVKKDLIIKLPKYSLFELENGRKRMLASAGELQKGNELALPSKYVNFLYLASHYEKLKGSPEDNEQKQLFVEQHKHYLDEIIEQISEFSKRVILADANLDKVLSAYNKHRDKPIREQAENIIHLFTLTNLGAPAAFKYFDTTIDRKRYTSTKEVLDATLIHQSITGLYETRIDLSQLGGDAYPYDVPDYASLGSGSPKKKRKVEDPKKKRKVDGSGSETPGTSESATPESMNNSQGRVTFEDVTVNFTQGEWQRLNPEQRNLYRDVMLENYSNLVSVGQGETTKPDVILRLEQGKEPWLEEEEVLGSGRAEKNGDIGGQIWKPKDVKESLX

SEQ ID NO: 119 - protein, 848 aa, synthetic construct
  REGION 1..848: note = (from V44)_D3a-hD3l-GFP1-10
  SITE 848: note = misc_feature - Xaa =
MPAAKRVKLDGSNHDQEFDPPKVYPPVPAEKRKPIRVLSLFDGIATGLLVLKDLGIQVDRYIASEVCEDSITVGMVRHQGKIMYVGDVRSVTQKHIQEWGPFDLVIGGSPCNDLSIVNPARKGLYEGTGRLFFEFYRLLHDARPKEGDDRPFFWLFENVVAMGVSDKRDISRFLESNPVMIDAKEVSAAHRARYFWGNLPGMNRPLASTVNDKLELQECLEHGRIAKFSKVRTITTRSNSIKQGKDQHFPVFMNEKEDILWCTEMERVFGFPVHYTDVSNMSRLARQRLLGRSWSVPVIRHLFAPLKEYFACVSSGNSNANSRGPSFSSGLVPLSLRGSHMFETVPVWRRQPVRVLSLFEDIKKELTSLGFLESGSDPGQLKHVVDVTDTVRKDVEEWGPFDLVYGATPPLGHTCDRPPSWYLFQFHRLLQYARPKPGSPRPFFWMFVDNLVLNKEDLDVASRFLEMEPVTIPDVHGGSLQNAVRVWSNIPAIRSSRHWALVSEEELSLLAQNKQSSKLAAKWPTKLVKNCFLPLREYFKYFSGGPSSGAPPPSGGSPAGSPTSTEEGTSESATPESGPGTSTEPSEGSAPGSPAGSPTSTEEGTSTEPSEGSAPGTSTEPSEPKKKRKVPSEMSKGEELFTGVVPILVELDGDVNGHKFSVRGEGEGDATIGKLTLKFICTTGKLPVPWPTLVTTLTYGVQCFSRYPDHMKRHDFFKSAMPEGYVQERTISFKDDGKYKTRAVVKFEGDTLVNRIELKGTDFKEDGNILGHKLEYNFNSHNVYITADKQKNGIKANFTVRHNVEDGSVQLADHYQQNTPIGDGPVLLPDNHYLSTQTVLSKDPNEKX

SEQ ID NO: 120 - protein, 638 aa, synthetic construct
  REGION 1..638: note = (from V45)_D3a-D3l-1xGFP11
  SITE 638: note = misc_feature - Xaa =
MPAAKRVKLDGSNHDQEFDPPKVYPPVPAEKRKPIRVLSLFDGIATGLLVLKDLGIQVDRYIASEVCEDSITVGMVRHQGKIMYVGDVRSVTQKHIQEWGPFDLVIGGSPCNDLSIVNPARKGLYEGTGRLFFEFYRLLHDARPKEGDDRPFFWLFENVVAMGVSDKRDISRFLESNPVMIDAKEVSAAHRARYFWGNLPGMNRPLASTVNDKLELQECLEHGRIAKFSKVRTITTRSNSIKQGKDQHFPVFMNEKEDILWCTEMERVFGFPVHYTDVSNMSRLARQRLLGRSWSVPVIRHLFAPLKEYFACVSSGNSNANSRGPSFSSGLVPLSLRGSHMGPMEIYKTVSAWKRQPVRVLSLFRNIDKVLKSLGFLESGSGSGGGTLKYVEDVTNVVRRDVEKWGPFDLVYGSTQPLGSSCDRCPGWYMFQFHRILQYALPRQESQRPFFWIFMDNLLLTEDDQETTTRFLQTEAVTLQDVRGRDYQNAMRVWSNIPGLKSKHAPLTPKEEEYLQAQVRSRSKLDAPKVDLLVKNCLLPLREYFKYFSQNSLPLGGPSSGAPPPSGGSPAGSPTSTEEGTSESATGGSGGRDHMVLHEYVNAAGITAAARSGSGQRGSKRTADGSEFESPKKKRKVX

SEQ ID NO: 121 - protein, 1730 aa, synthetic construct
  REGION 1..1730: note = (from V45)_GFP1-10-dCas9-KRAB
  SITE 1730: note = misc_feature - Xaa =
MPAAKRVKLDGSGPDIVMSKGEELFTGVVPILVELDGDVNGHKFSVRGEGEGDATIGKLTLKFICTTGKLPVPWPTLVTTLTYGVQCFSRYPDHMKRHDFFKSAMPEGYVQERTISFKDDGKYKTRAVVKFEGDTLVNRIELKGTDFKEDGNILGHKLEYNFNSHNVYITADKQKNGIKANFTVRHNVEDGSVQLADHYQQNTPIGDGPVLLPDNHYLSTQTVLSKDPNEKLDPGGGGSGSGPKKKRKVMDKKYSIGLAIGTNSVGWAVITDEYKVPSKKFKVLGNTDRHSIKKNLIGALLFDSGETAEATRLKRTARRRYTRRKNRICYLQEIFSNEMAKVDDSFFHRLEESFLVEEDKKHERHPIFGNIVDEVAYHEKYPTIYHLRKKLVDSTDKADLRLIYLALAHMIKFRGHFLIEGDLNPDNSDVDKLFIQLVQTYNQLFEENPINASGVDAKAILSARLSKSRRLENLIAQLPGEKKNGLFGNLIALSLGLTPNFKSNFDLAEDAKLQLSKDTYDDDLDNLLAQIGDQYADLFLAAKNLSDAILLSDILRVNTEITKAPLSASMIKRYDEHHQDLTLLKALVRQQLPEKYKEIFFDQSKNGYAGYIDGGASQEEFYKFIKPILEKMDGTEELLVKLNREDLLRKQRTFDNGSIPHQIHLGELHAILRRQEDFYPFLKDNREKIEKILTFRIPYYVGPLARGNSRFAWMTRKSEETITPWNFEEVVDKGASAQSFIERMTNFDKNLPNEKVLPKHSLLYEYFTVYNELTKVKYVTEGMRKPAFLSGEQKKAIVDLLFKTNRKVTVKQLKEDYFKKIECFDSVEISGVEDRFNASLGTYHDLLKIIKDKDFLDNEENEDILEDIVLTLTLFEDREMIEERLKTYAHLFDDKVMKQLKRRRYTGWGRLSRKLINGIRDKQSGKTILDFLKSDGFANRNFMQLIHDDSLTFKEDIQKAQVSGQGDSLHEHIANLAGSPAIKKGILQTVKVVDELVKVMGRHKPENIVIEMARENQTTQKGQKNSRERMKRIEEGIKELGSQILKEHPVENTQLQNEKLYLYYLQNGRDMYVDQELDINRLSDYDVDAIVPQSFLKDDSIDNKVLTRSDKNRGKSDNVPSEEVVKKMKNYWRQLLNAKLITQRKFDNLTKAERGGLSELDKAGFIKRQLVETRQITKHVAQILDSRMNTKYDENDKLIREVKVITLKSKLVSDFRKDFQFYKVREINNYHHAHDAYLNAVVGTALIKKYPKLESEFVYGDYKVYDVRKMIAKSEQEIGKATAKYFFYSNIMNFFKTEITLANGEIRKRPLIETNGETGEIVWDKGRDFATVRKVLSMPQVNIVKKTEVQTGGFSKESILPKRNSDKLIARKKDWDPKKYGGFDSPTVAYSVLVVAKVEKGKSKKLKSVKELLGITIMERSSFEKNPIDFLEAKGYKEVKKDLIIKLPKYSLFELENGRKRMLASAGELQKGNELALPSKYVNFLYLASHYEKLKGSPEDNEQKQLFVEQHKHYLDEIIEQISEFSKRVILADANLDKVLSAYNKHRDKPIREQAENIIHLFTLTNLGAPAAFKYFDTTIDRKRYTSTKEVLDATLIHQSITGLYETRIDLSQLGGDAYPYDVPDYASLGSGSPKKKRKVEDPKKKRKVDGSGSETPGTSESATPESRTLVTFKDVFVDFTREEWKLLDTAQQIVYRNVMLENYKNLVSLGYQLTKPDVILRLEKGEEPX

SEQ ID NO: 122 - protein, 1785 aa, synthetic construct
  REGION 1..1785: note = (from V46)_10xGFP11-dCas9-ZIM3
  SITE 1785: note = misc_feature - Xaa =
MPAAKRVKLDGSMRDHMVLHEYVNAAGITGGSGGRDHMVLHEYVNAAGITGGSGGRDHMVLHEYVNAAGITGGSGGRDHMVLHEYVNAAGITGGSGGRDHMVLHEYVNAAGITGGSGGRDHMVLHEYVNAAGITGGSGGRDHMVLHEYVNAAGITAAAGGSGGRDHMVLHEYVNAAGITGGSGGRDHMVLHEYVNAAGITGGSGGRDHMVLHEYVNAAGITGGSGGRSGSGQRGSKRTADGSEFESPKKKRKVGGSGSGPKKKRKVMDKKYSIGLAIGTNSVGWAVITDEYKVPSKKFKVLGNTDRHSIKKNLIGALLFDSGETAEATRLKRTARRRYTRRKNRICYLQEIFSNEMAKVDDSFFHRLEESFLVEEDKKHERHPIFGNIVDEVAYHEKYPTIYHLRKKLVDSTDKADLRLIYLALAHMIKFRGHFLIEGDLNPDNSDVDKLFIQLVQTYNQLFEENPINASGVDAKAILSARLSKSRRLENLIAQLPGEKKNGLFGNLIALSLGLTPNFKSNFDLAEDAKLQLSKDTYDDDLDNLLAQIGDQYADLFLAAKNLSDAILLSDILRVNTEITKAPLSASMIKRYDEHHQDLTLLKALVRQQLPEKYKEIFFDQSKNGYAGYIDGGASQEEFYKFIKPILEKMDGTEELLVKLNREDLLRKQRTFDNGSIPHQIHLGELHAILRRQEDFYPFLKDNREKIEKILTFRIPYYVGPLARGNSRFAWMTRKSEETITPWNFEEVVDKGASAQSFIERMTNFDKNLPNEKVLPKHSLLYEYFTVYNELTKVKYVTEGMRKPAFLSGEQKKAIVDLLFKTNRKVTVKQLKEDYFKKIECFDSVEISGVEDRFNASLGTYHDLLKIIKDKDFLDNEENEDILEDIVLTLTLFEDREMIEERLKTYAHLFDDKVMKQLKRRRYTGWGRLSRKLINGIRDKQSGKTILDFLKSDGFANRNFMQLIHDDSLTFKEDIQKAQVSGQGDSLHEHIANLAGSPAIKKGILQTVKVVDELVKVMGRHKPENIVIEMARENQTTQKGQKNSRERMKRIEEGIKELGSQILKEHPVENTQLQNEKLYLYYLQNGRDMYVDQELDINRLSDYDVDAIVPQSFLKDDSIDNKVLTRSDKNRGKSDNVPSEEVVKKMKNYWRQLLNAKLITQRKFDNLTKAERGGLSELDKAGFIKRQLVETRQITKHVAQILDSRMNTKYDENDKLIREVKVITLKSKLVSDFRKDFQFYKVREINNYHHAHDAYLNAVVGTALIKKYPKLESEFVYGDYKVYDVRKMIAKSEQEIGKATAKYFFYSNIMNFFKTEITLANGEIRKRPLIETNGETGEIVWDKGRDFATVRKVLSMPQVNIVKKTEVQTGGFSKESILPKRNSDKLIARKKDWDPKKYGGFDSPTVAYSVLVVAKVEKGKSKKLKSVKELLGITIMERSSFEKNPIDFLEAKGYKEVKKDLIIKLPKYSLFELENGRKRMLASAGELQKGNELALPSKYVNFLYLASHYEKLKGSPEDNEQKQLFVEQHKHYLDEIIEQISEFSKRVILADANLDKVLSAYNKHRDKPIREQAENIIHLFTLTNLGAPAAFKYFDTTIDRKRYTSTKEVLDATLIHQSITGLYETRIDLSQLGGDAYPYDVPDYASLGSGSPKKKRKVEDPKKKRKVDGSGSETPGTSESATPESMNNSQGRVTFEDVTVNFTQGEWQRLNPEQRNLYRDVMLENYSNLVSVGQGETTKPDVILRLEQGKEPWLEEEEVLGSGRAEKNGDIGGQIWKPKDVKESLX

SEQ ID NO: 123 - protein, 398 aa, synthetic construct
  REGION 1..398: note = (from V47)scFv-ZIM3
MVPAAKRVKLDGSGPDIVMTQSPSSLSASVGDRVTITCRSSTGAVTTSNYASWVQEKPGKLFKGLIGGTNNRAPGVPSRFSGSLIGDKATLTISSLQPEDFATYFCALWYSNHWVFGQGTKVELKRGGGGSGGGGSGGGGSSGGGSEVKLLESGGGLVQPGGSLKLSCAVSGFSLTDYGVNWVRQAPGRGLEWIGVIWGDGITDYNSALKDRFIISKDNGKNTVYLQMSKVRSDDTALYYCVTGLFDYWGQGTLVTVSSYPYDVPDYAGGGGGSGGGGSGGGGSGGGGSLDPGGGGSGMNNSQGRVTFEDVTVNFTQGEWQRLNPEQRNLYRDVMLENYSNLVSVGQGETTKPDVILRLEQGKEPWLEEEEVLGSGRAEKNGDIGGQIWKPKDVKESL

SEQ ID NO: 124 - protein, 2126 aa, synthetic construct
  REGION 1..2126: note = (from V47)D3a-hD3l-dCas9-1xGCN4
  SITE 2126: note = misc_feature - Xaa =
MPAAKRVKLDGSNHDQEFDPPKVYPPVPAEKRKPIRVLSLFDGIATGLLVLKDLGIQVDRYIASEVCEDSITVGMVRHQGKIMYVGDVRSVTQKHIQEWGPFDLVIGGSPCNDLSIVNPARKGLYEGTGRLFFEFYRLLHDARPKEGDDRPFFWLFENVVAMGVSDKRDISRFLESNPVMIDAKEVSAAHRARYFWGNLPGMNRPLASTVNDKLELQECLEHGRIAKFSKVRTITTRSNSIKQGKDQHFPVFMNEKEDILWCTEMERVFGFPVHYTDVSNMSRLARQRLLGRSWSVPVIRHLFAPLKEYFACVSSGNSNANSRGPSFSSGLVPLSLRGSHMFETVPVWRRQPVRVLSLFEDIKKELTSLGFLESGSDPGQLKHVVDVTDTVRKDVEEWGPFDLVYGATPPLGHTCDRPPSWYLFQFHRLLQYARPKPGSPRPFFWMFVDNLVLNKEDLDVASRFLEMEPVTIPDVHGGSLQNAVRVWSNIPAIRSSRHWALVSEEELSLLAQNKQSSKLAAKWPTKLVKNCFLPLREYFKYFSGGPSSGAPPPSGGSPAGSPTSTEEGTSESATPESGPGTSTEPSEGSAPGSPAGSPTSTEEGTSTEPSEGSAPGTSTEPSEPKKKRKVGSDKKYSIGLAIGTNSVGWAVITDEYKVPSKKFKVLGNTDRHSIKKNLIGALLFDSGETAEATRLKRTARRRYTRRKNRICYLQEIFSNEMAKVDDSFFHRLEESFLVEEDKKHERHPIFGNIVDEVAYHEKYPTIYHLRKKLVDSTDKADLRLIYLALAHMIKFRGHFLIEGDLNPDNSDVDKLFIQLVQTYNQLFEENPINASGVDAKAILSARLSKSRRLENLIAQLPGEKKNGLFGNLIALSLGLTPNFKSNFDLAEDAKLQLSKDTYDDDLDNLLAQIGDQYADLFLAAKNLSDAILLSDILRVNTEITKAPLSASMIKRYDEHHQDLTLLKALVRQQLPEKYKEIFFDQSKNGYAGYIDGGASQEEFYKFIKPILEKMDGTEELLVKLNREDLLRKQRTFDNGSIPHQIHLGELHAILRRQEDFYPFLKDNREKIEKILTFRIPYYVGPLARGNSRFAWMTRKSEETITPWNFEEVVDKGASAQSFIERMTNFDKNLPNEKVLPKHSLLYEYFTVYNELTKVKYVTEGMRKPAFLSGEQKKAIVDLLFKTNRKVTVKQLKEDYFKKIECFDSVEISGVEDRFNASLGTYHDLLKIIKDKDFLDNEENEDILEDIVLTLTLFEDREMIEERLKTYAHLFDDKVMKQLKRRRYTGWGRLSRKLINGIRDKQSGKTILDFLKSDGFANRNFMQLIHDDSLTFKEDIQKAQVSGQGDSLHEHIANLAGSPAIKKGILQTVKVVDELVKVMGRHKPENIVIEMARENQTTQKGQKNSRERMKRIEEGIKELGSQILKEHPVENTQLQNEKLYLYYLQNGRDMYVDQELDINRLSDYDVDAIVPQSFLKDDSIDNKVLTRSDKNRGKSDNVPSEEVVKKMKNYWRQLLNAKLITQRKFDNLTKAERGGLSELDKAGFIKRQLVETRQITKHVAQILDSRMNTKYDENDKLIREVKVITLKSKLVSDFRKDFQFYKVREINNYHHAHDAYLNAVVGTALIKKYPKLESEFVYGDYKVYDVRKMIAKSEQEIGKATAKYFFYSNIMNFFKTEITLANGEIRKRPLIETNGETGEIVWDKGRDFATVRKVLSMPQVNIVKKTEVQTGGFSKESILPKRNSDKLIARKKDWDPKKYGGFDSPTVAYSVLVVAKVEKGKSKKLKSVKELLGITIMERSSFEKNPIDFLEAKGYKEVKKDLIIKLPKYSLFELENGRKRMLASAGELQKGNELALPSKYVNFLYLASHYEKLKGSPEDNEQKQLFVEQHKHYLDEIIEQISEFSKRVILADANLDKVLSAYNKHRDKPIREQAENIIHLFTLTNLGAPAAFKYFDTTIDRKRYTSTKEVLDATLIHQSITGLYETRIDLSQLGGDAYPYDVPDYASLGSGSPKKKRKVEDPKKKRKVDGIGSGSNGSSGEELLSKNYHLENEVARLKKGSGSGGSGSGGSGSGSGGSGSGGSGSGEELLSKNYHGSGSGQRGSKRTADGSEFESPKKKRKVX

SEQ ID NO: 125 - protein, 31 aa, synthetic construct
  REGION 1..31: note = linker1
GGGGGSGGGGSGGGGSGGGGSSLDPGGGGSG

SEQ ID NO: 126 - skipped

SEQ ID NO: 127 - protein, 27 aa, synthetic construct
  REGION 1..27: note = linker3
SSGNSNANSRGPSFSSGLVPLSLRGSH

SEQ ID NO: 128 - protein, 80 aa, synthetic construct
  REGION 1..80: note = linker4
GGPSSGAPPPSGGSPAGSPTSTEEGTSESATPESGPGTSTEPSEGSAPGSPAGSPTSTEEGTSTEPSEGSAPGTSTEPSE

SEQ ID NO: 129 - protein, 6 aa, synthetic construct
  REGION 1..6: note = linker5
SLGSGS

SEQ ID NO: 130 - protein, 12 aa, synthetic construct
  REGION 1..12: note = linker6
DGIGSGSNGSSG

SEQ ID NO: 131 - protein, 27 aa, synthetic construct
  REGION 1..27: note = linker7
GSGSGGSGSGGSGSGSGGSGSGGSGSG

SEQ ID NO: 132 - protein, 9 aa, synthetic construct
  REGION 1..9: note = linker8
GSGSGQRGS

SEQ ID NO: 133 - protein, 2517 aa, synthetic construct
  REGION 1..2517: note = V12_scFv-KRAB-2a-D3a-D3l-dCas9-1xGCN4
  SITE 2517: note = misc_feature - Xaa =
MGPDIVMTQSPSSLSASVGDRVTITCRSSTGAVTTSNYASWVQEKPGKLFKGLIGGTNNRAPGVPSRFSGSLIGDKATLTISSLQPEDFATYFCALWYSNHWVFGQGTKVELKRGGGGSGGGGSGGGGSSGGGSEVKLLESGGGLVQPGGSLKLSCAVSGFSLTDYGVNWVRQAPGRGLEWIGVIWGDGITDYNSALKDRFIISKDNGKNTVYLQMSKVRSDDTALYYCVTGLFDYWGQGTLVTVSSYPYDVPDYAGGGGGSGGGGSGGGGSGGGGSLDPGGGGSGRTLVTFKDVFVDFTREEWKLLDTAQQIVYRNVMLENYKNLVSLGYQLTKPDVILRLEKGEEPGSGKRTADGSEFESPKKKRKVGSGATNFSLLKQAGDVEENPGPMNHDQEFDPPKVYPPVPAEKRKPIRVLSLFDGIATGLLVLKDLGIQVDRYIASEVCEDSITVGMVRHQGKIMYVGDVRSVTQKHIQEWGPFDLVIGGSPCNDLSIVNPARKGLYEGTGRLFFEFYRLLHDARPKEGDDRPFFWLFENVVAMGVSDKRDISRFLESNPVMIDAKEVSAAHRARYFWGNLPGMNRPLASTVNDKLELQECLEHGRIAKFSKVRTITTRSNSIKQGKDQHFPVFMNEKEDILWCTEMERVFGFPVHYTDVSNMSRLARQRLLGRSWSVPVIRHLFAPLKEYFACVSSGNSNANSRGPSFSSGLVPLSLRGSHMGPMEIYKTVSAWKRQPVRVLSLFRNIDKVLKSLGFLESGSGSGGGTLKYVEDVTNVVRRDVEKWGPFDLVYGSTQPLGSSCDRCPGWYMFQFHRILQYALPRQESQRPFFWIFMDNLLLTEDDQETTTRFLQTEAVTLQDVRGRDYQNAMRVWSNIPGLKSKHAPLTPKEEEYLQAQVRSRSKLDAPKVDLLVKNCLLPLREYFKYFSQNSLPLGGPSSGAPPPSGGSPAGSPTSTEEGTSESATPESGPGTSTEPSEGSAPGSPAGSPTSTEEGTSTEPSEGSAPGTSTEPSEPKKKRKVMDKKYSIGLAIGTNSVGWAVITDEYKVPSKKFKVLGNTDRHSIKKNLIGALLFDSGETAEATRLKRTARRRYTRRKNRICYLQEIFSNEMAKVDDSFFHRLEESFLVEEDKKHERHPIFGNIVDEVAYHEKYPTIYHLRKKLVDSTDKADLRLIYLALAHMIKFRGHFLIEGDLNPDNSDVDKLFIQLVQTYNQLFEENPINASGVDAKAILSARLSKSRRLENLIAQLPGEKKNGLFGNLIALSLGLTPNFKSNFDLAEDAKLQLSKDTYDDDLDNLLAQIGDQYADLFLAAKNLSDAILLSDILRVNTEITKAPLSASMIKRYDEHHQDLTLLKALVRQQLPEKYKEIFFDQSKNGYAGYIDGGASQEEFYKFIKPILEKMDGTEELLVKLNREDLLRKQRTFDNGSIPHQIHLGELHAILRRQEDFYPFLKDNREKIEKILTFRIPYYVGPLARGNSRFAWMTRKSEETITPWNFEEVVDKGASAQSFIERMTNFDKNLPNEKVLPKHSLLYEYFTVYNELTKVKYVTEGMRKPAFLSGEQKKAIVDLLFKTNRKVTVKQLKEDYFKKIECFDSVEISGVEDRFNASLGTYHDLLKIIKDKDFLDNEENEDILEDIVLTLTLFEDREMIEERLKTYAHLFDDKVMKQLKRRRYTGWGRLSRKLINGIRDKQSGKTILDFLKSDGFANRNFMQLIHDDSLTFKEDIQKAQVSGQGDSLHEHIANLAGSPAIKKGILQTVKVVDELVKVMGRHKPENIVIEMARENQTTQKGQKNSRERMKRIEEGIKELGSQILKEHPVENTQLQNEKLYLYYLQNGRDMYVDQELDINRLSDYDVDAIVPQSFLKDDSIDNKVLTRSDKNRGKSDNVPSEEVVKKMKNYWRQLLNAKLITQRKFDNLTKAERGGLSELDKAGFIKRQLVETRQITKHVAQILDSRMNTKYDENDKLIREVKVITLKSKLVSDFRKDFQFYKVREINNYHHAHDAYLNAVVGTALIKKYPKLESEFVYGDYKVYDVRKMIAKSEQEIGKATAKYFFYSNIMNFFKTEITLANGEIRKRPLIETNGETGEIVWDKGRDFATVRKVLSMPQVNIVKKTEVQTGGFSKESILPKRNSDKLIARKKDWDPKKYGGFDSPTVAYSVLVVAKVEKGKSKKLKSVKELLGITIMERSSFEKNPIDFLEAKGYKEVKKDLIIKLPKYSLFELENGRKRMLASAGELQKGNELALPSKYVNFLYLASHYEKLKGSPEDNEQKQLFVEQHKHYLDEIIEQISEFSKRVILADANLDKVLSAYNKHRDKPIREQAENIIHLFTLTNLGAPAAFKYFDTTIDRKRYTSTKEVLDATLIHQSITGLYETRIDLSQLGGDAYPYDVPDYASLGSGSPKKKRKVEDPKKKRKVDGIGSGSNGSSGEELLSKNYHLENEVARLKKGSGSGGSGSGGSGSGSGGSGSGGSGSGEELLSKNYHGSGSGQRGSKRTADGSEFESPKKKRKVX

SEQ ID NO: 134 - protein, 2527 aa, synthetic construct
  REGION 1..2527: note = V13_scFv-KRAB-2a-D3a-D3l-dCas9-2xGCN4
  SITE 2527: note = misc_feature - Xaa =
MGPDIVMTQSPSSLSASVGDRVTITCRSSTGAVTTSNYASWVQEKPGKLFKGLIGGTNNRAPGVPSRFSGSLIGDKATLTISSLQPEDFATYFCALWYSNHWVFGQGTKVELKRGGGGSGGGGSGGGGSSGGGSEVKLLESGGGLVQPGGSLKLSCAVSGFSLTDYGVNWVRQAPGRGLEWIGVIWGDGITDYNSALKDRFIISKDNGKNTVYLQMSKVRSDDTALYYCVTGLFDYWGQGTLVTVSSYPYDVPDYAGGGGGSGGGGSGGGGSGGGGSLDPGGGGSGRTLVTFKDVFVDFTREEWKLLDTAQQIVYRNVMLENYKNLVSLGYQLTKPDVILRLEKGEEPGSGKRTADGSEFESPKKKRKVGSGATNFSLLKQAGDVEENPGPMNHDQEFDPPKVYPPVPAEKRKPIRVLSLFDGIATGLLVLKDLGIQVDRYIASEVCEDSITVGMVRHQGKIMYVGDVRSVTQKHIQEWGPFDLVIGGSPCNDLSIVNPARKGLYEGTGRLFFEFYRLLHDARPKEGDDRPFFWLFENVVAMGVSDKRDISRFLESNPVMIDAKEVSAAHRARYFWGNLPGMNRPLASTVNDKLELQECLEHGRIAKFSKVRTITTRSNSIKQGKDQHFPVFMNEKEDILWCTEMERVFGFPVHYTDVSNMSRLARQRLLGRSWSVPVIRHLFAPLKEYFACVSSGNSNANSRGPSFSSGLVPLSLRGSHMGPMEIYKTVSAWKRQPVRVLSLFRNIDKVLKSLGFLESGSGSGGGTLKYVEDVTNVVRRDVEKWGPFDLVYGSTQPLGSSCDRCPGWYMFQFHRILQYALPRQESQRPFFWIFMDNLLLTEDDQETTTRFLQTEAVTLQDVRGRDYQNAMRVWSNIPGLKSKHAPLTPKEEEYLQAQVRSRSKLDAPKVDLLVKNCLLPLREYFKYFSQNSLPLGGPSSGAPPPSGGSPAGSPTSTEEGTSESATPESGPGTSTEPSEGSAPGSPAGSPTSTEEGTSTEPSEGSAPGTSTEPSEPKKKRKVMDKKYSIGLAIGTNSVGWAVITDEYKVPSKKFKVLGNTDRHSIKKNLIGALLFDSGETAEATRLKRTARRRYTRRKNRICYLQEIFSNEMAKVDDSFFHRLEESFLVEEDKKHERHPIFGNIVDEVAYHEKYPTIYHLRKKLVDSTDKADLRLIYLALAHMIKFRGHFLIEGDLNPDNSDVDKLFIQLVQTYNQLFEENPINASGVDAKAILSARLSKSRRLENLIAQLPGEKKNGLFGNLIALSLGLTPNFKSNFDLAEDAKLQLSKDTYDDDLDNLLAQIGDQYADLFLAAKNLSDAILLSDILRVNTEITKAPLSASMIKRYDEHHQDLTLLKALVRQQLPEKYKEIFFDQSKNGYAGYIDGGASQEEFYKFIKPILEKMDGTEELLVKLNREDLLRKQRTFDNGSIPHQIHLGELHAILRRQEDFYPFLKDNREKIEKILTFRIPYYVGPLARGNSRFAWMTRKSEETITPWNFEEVVDKGASAQSFIERMTNFDKNLPNEKVLPKHSLLYEYFTVYNELTKVKYVTEGMRKPAFLSGEQKKAIVDLLFKTNRKVTVKQLKEDYFKKIECFDSVEISGVEDRFNASLGTYHDLLKIIKDKDFLDNEENEDILEDIVLTLTLFEDREMIEERLKTYAHLFDDKVMKQLKRRRYTGWGRLSRKLINGIRDKQSGKTILDFLKSDGFANRNFMQLIHDDSLTFKEDIQKAQVSGQGDSLHEHIANLAGSPAIKKGILQTVKVVDELVKVMGRHKPENIVIEMARENQTTQKGQKNSRERMKRIEEGIKELGSQILKEHPVENTQLQNEKLYLYYLQNGRDMYVDQELDINRLSDYDVDAIVPQSFLKDDSIDNKVLTRSDKNRGKSDNVPSEEVVKKMKNYWRQLLNAKLITQRKFDNLTKAERGGLSELDKAGFIKRQLVETRQITKHVAQILDSRMNTKYDENDKLIREVKVITLKSKLVSDFRKDFQFYKVREINNYHHAHDAYLNAVVGTALIKKYPKLESEFVYGDYKVYDVRKMIAKSEQEIGKATAKYFFYSNIMNFFKTEITLANGEIRKRPLIETNGETGEIVWDKGRDFATVRKVLSMPQVNIVKKTEVQTGGFSKESILPKRNSDKLIARKKDWDPKKYGGFDSPTVAYSVLVVAKVEKGKSKKLKSVKELLGITIMERSSFEKNPIDFLEAKGYKEVKKDLIIKLPKYSLFELENGRKRMLASAGELQKGNELALPSKYVNFLYLASHYEKLKGSPEDNEQKQLFVEQHKHYLDEIIEQISEFSKRVILADANLDKVLSAYNKHRDKPIREQAENIIHLFTLTNLGAPAAFKYFDTTIDRKRYTSTKEVLDATLIHQSITGLYETRIDLSQLGGDAYPYDVPDYASLGSGSPKKKRKVEDPKKKRKVDGIGSGSNGSSGEELLSKNYHLENEVARLKKGSGSGGSGSGGSGSGSGGSGSGGSGSGEELLSKNYHLENEVARLKKGSGSGQRGSKRTADGSEFESPKKKRKVX

SEQ ID NO: 135 - protein, 2895 aa, synthetic construct
  REGION 1..2895: note = V14_scFv-KRAB-2a-D3a-D3l-dCas9-10xGCN4
  SITE 2895: note = misc_feature - Xaa =
MGPDIVMTQSPSSLSASVGDRVTITCRSSTGAVTTSNYASWVQEKPGKLFKGLIGGTNNRAPGVPSRFSGSLIGDKATLTISSLQPEDFATYFCALWYSNHWVFGQGTKVELKRGGGGSGGGGSGGGGSSGGGSEVKLLESGGGLVQPGGSLKLSCAVSGFSLTDYGVNWVRQAPGRGLEWIGVIWGDGITDYNSALKDRFIISKDNGKNTVYLQMSKVRSDDTALYYCVTGLFDYWGQGTLVTVSSYPYDVPDYAGGGGGSGGGGSGGGGSGGGGSLDPGGGGSGRTLVTFKDVFVDFTREEWKLLDTAQQIVYRNVMLENYKNLVSLGYQLTKPDVILRLEKGEEPGSGKRTADGSEFESPKKKRKVGSGATNFSLLKQAGDVEENPGPMNHDQEFDPPKVYPPVPAEKRKPIRVLSLFDGIATGLLVLKDLGIQVDRYIASEVCEDSITVGMVRHQGKIMYVGDVRSVTQKHIQEWGPFDLVIGGSPCNDLSIVNPARKGLYEGTGRLFFEFYRLLHDARPKEGDDRPFFWLFENVVAMGVSDKRDISRFLESNPVMIDAKEVSAAHRARYFWGNLPGMNRPLASTVNDKLELQECLEHGRIAKFSKVRTITTRSNSIKQGKDQHFPVFMNEKEDILWCTEMERVFGFPVHYTDVSNMSRLARQRLLGRSWSVPVIRHLFAPLKEYFACVSSGNSNANSRGPSFSSGLVPLSLRGSHMGPMEIYKTVSAWKRQPVRVLSLFRNIDKVLKSLGFLESGSGSGGGTLKYVEDVTNVVRRDVEKWGPFDLVYGSTQPLGSSCDRCPGWYMFQFHRILQYALPRQESQRPFFWIFMDNLLLTEDDQETTTRFLQTEAVTLQDVRGRDYQNAMRVWSNIPGLKSKHAPLTPKEEEYLQAQVRSRSKLDAPKVDLLVKNCLLPLREYFKYFSQNSLPLGGPSSGAPPPSGGSPAGSPTSTEEGTSESATPESGPGTSTEPSEGSAPGSPAGSPTSTEEGTSTEPSEGSAPGTSTEPSEPKKKRKVMDKKYSIGLAIGTNSVGWAVITDEYKVPSKKFKVLGNTDRHSIKKNLIGALLFDSGETAEATRLKRTARRRYTRRKNRICYLQEIFSNEMAKVDDSFFHRLEESFLVEEDKKHERHPIFGNIVDEVAYHEKYPTIYHLRKKLVDSTDKADLRLIYLALAHMIKFRGHFLIEGDLNPDNSDVDKLFIQLVQTYNQLFEENPINASGVDAKAILSARLSKSRRLENLIAQLPGEKKNGLFGNLIALSLGLTPNFKSNFDLAEDAKLQLSKDTYDDDLDNLLAQIGDQYADLFLAAKNLSDAILLSDILRVNTEITKAPLSASMIKRYDEHHQDLTLLKALVRQQLPEKYKEIFFDQSKNGYAGYIDGGASQEEFYKFIKPILEKMDGTEELLVKLNREDLLRKQRTFDNGSIPHQIHLGELHAILRRQEDFYPFLKDNREKIEKILTFRIPYYVGPLARGNSRFAWMTRKSEETITPWNFEEVVDKGASAQSFIERMTNFDKNLPNEKVLPKHSLLYEYFTVYNELTKVKYVTEGMRKPAFLSGEQKKAIVDLLFKTNRKVTVKQLKEDYFKKIECFDSVEISGVEDRFNASLGTYHDLLKIIKDKDFLDNEENEDILEDIVLTLTLFEDREMIEERLKTYAHLFDDKVMKQLKRRRYTGWGRLSRKLINGIRDKQSGKTILDFLKSDGFANRNFMQLIHDDSLTFKEDIQKAQVSGQGDSLHEHIANLAGSPAIKKGILQTVKVVDELVKVMGRHKPENIVIEMARENQTTQKGQKNSRERMKRIEEGIKELGSQILKEHPVENTQLQNEKLYLYYLQNGRDMYVDQELDINRLSDYDVDAIVPQSFLKDDSIDNKVLTRSDKNRGKSDNVPSEEVVKKMKNYWRQLLNAKLITQRKFDNLTKAERGGLSELDKAGFIKRQLVETRQITKHVAQILDSRMNTKYDENDKLIREVKVITLKSKLVSDFRKDFQFYKVREINNYHHAHDAYLNAVVGTALIKKYPKLESEFVYGDYKVYDVRKMIAKSEQEIGKATAKYFFYSNIMNFFKTEITLANGEIRKRPLIETNGETGEIVWDKGRDFATVRKVLSMPQVNIVKKTEVQTGGFSKESILPKRNSDKLIARKKDWDPKKYGGFDSPTVAYSVLVVAKVEKGKSKKLKSVKELLGITIMERSSFEKNPIDFLEAKGYKEVKKDLIIKLPKYSLFELENGRKRMLASAGELQKGNELALPSKYVNFLYLASHYEKLKGSPEDNEQKQLFVEQHKHYLDEIIEQISEFSKRVILADANLDKVLSAYNKHRDKPIREQAENIIHLFTLTNLGAPAAFKYFDTTIDRKRYTSTKEVLDATLIHQSITGLYETRIDLSQLGGDAYPYDVPDYASLGSGSPKKKRKVEDPKKKRKVDGIGSGSNGSSGEELLSKNYHLENEVARLKKGSGSGGSGSGGSGSGSGGSGSGGSGSGEELLSKNYHLENEVARLKKGSGSGGSGSGGSGSGSGGSGSGGSGSGEELLSKNYHLENEVARLKKGSGSGGSGSGGSGSGSGGSGSGGSGSGEELLSKNYHLENEVARLKKGSGSGGSGSGGSGSGSGGSGSGGSGSGEELLSKNYHLENEVARLKKGSGSGGSGSGGSGSGSGGSGSGGSGSGEELLSKNYHLENEVARLKKGSGSGGSGSGGSGSGSGGSGSGGSGSGEELLSKNYHLENEVARLKKGSGSGGSGSGGSGSGSGGSGSGGSGSGEELLSKNYHLENEVARLKKGSGSGGSGSGGSGSGSGGSGSGGSGSGEELLSKNYHLENEVARLKKGSGSGGSGSGGSGSGSGGSGSGGSGSGEELLSKNYHLENEVARLKKGSGSGQRGSKRTADGSEFESPKKKRKVX

SEQ ID NO: 136 - protein, 2544 aa, synthetic construct
  REGION 1..2544: note = V15_scFv-ZIM3-2a-D3a-hD3L-dCas9-1xGCN4
  SITE 2544: note = misc_feature - Xaa =
MPAAKRVKLDGSGPDIVMTQSPSSLSASVGDRVTITCRSSTGAVTTSNYASWVQEKPGKLFKGLIGGTNNRAPGVPSRFSGSLIGDKATLTISSLQPEDFATYFCALWYSNHWVFGQGTKVELKRGGGGSGGGGSGGGGSSGGGSEVKLLESGGGLVQPGGSLKLSCAVSGFSLTDYGVNWVRQAPGRGLEWIGVIWGDGITDYNSALKDRFIISKDNGKNTVYLQMSKVRSDDTALYYCVTGLFDYWGQGTLVTVSSYPYDVPDYAGGGGGSGGGGSGGGGSGGGGSLDPGGGGSGMNNSQGRVTFEDVTVNFTQGEWQRLNPEQRNLYRDVMLENYSNLVSVGQGETTKPDVILRLEQGKEPWLEEEEVLGSGRAEKNGDIGGQIWKPKDVKESLGSGATNFSLLKQAGDVEENPGPMPAAKRVKLDGSNHDQEFDPPKVYPPVPAEKRKPIRVLSLFDGIATGLLVLKDLGIQVDRYIASEVCEDSITVGMVRHQGKIMYVGDVRSVTQKHIQEWGPFDLVIGGSPCNDLSIVNPARKGLYEGTGRLFFEFYRLLHDARPKEGDDRPFFWLFENVVAMGVSDKRDISRFLESNPVMIDAKEVSAAHRARYFWGNLPGMNRPLASTVNDKLELQECLEHGRIAKFSKVRTITTRSNSIKQGKDQHFPVFMNEKEDILWCTEMERVFGFPVHYTDVSNMSRLARQRLLGRSWSVPVIRHLFAPLKEYFACVSSGNSNANSRGPSFSSGLVPLSLRGSHMFETVPVWRRQPVRVLSLFEDIKKELTSLGFLESGSDPGQLKHVVDVTDTVRKDVEEWGPFDLVYGATPPLGHTCDRPPSWYLFQFHRLLQYARPKPGSPRPFFWMFVDNLVLNKEDLDVASRFLEMEPVTIPDVHGGSLQNAVRVWSNIPAIRSSRHWALVSEEELSLLAQNKQSSKLAAKWPTKLVKNCFLPLREYFKYFSGGPSSGAPPPSGGSPAGSPTSTEEGTSESATPESGPGTSTEPSEGSAPGSPAGSPTSTEEGTSTEPSEGSAPGTSTEPSEPKKKRKVMDKKYSIGLAIGTNSVGWAVITDEYKVPSKKFKVLGNTDRHSIKKNLIGALLFDSGETAEATRLKRTARRRYTRRKNRICYLQEIFSNEMAKVDDSFFHRLEESFLVEEDKKHERHPIFGNIVDEVAYHEKYPTIYHLRKKLVDSTDKADLRLIYLALAHMIKFRGHFLIEGDLNPDNSDVDKLFIQLVQTYNQLFEENPINASGVDAKAILSARLSKSRRLENLIAQLPGEKKNGLFGNLIALSLGLTPNFKSNFDLAEDAKLQLSKDTYDDDLDNLLAQIGDQYADLFLAAKNLSDAILLSDILRVNTEITKAPLSASMIKRYDEHHQDLTLLKALVRQQLPEKYKEIFFDQSKNGYAGYIDGGASQEEFYKFIKPILEKMDGTEELLVKLNREDLLRKQRTFDNGSIPHQIHLGELHAILRRQEDFYPFLKDNREKIEKILTFRIPYYVGPLARGNSRFAWMTRKSEETITPWNFEEVVDKGASAQSFIERMTNFDKNLPNEKVLPKHSLLYEYFTVYNELTKVKYVTEGMRKPAFLSGEQKKAIVDLLFKTNRKVTVKQLKEDYFKKIECFDSVEISGVEDRFNASLGTYHDLLKIIKDKDFLDNEENEDILEDIVLTLTLFEDREMIEERLKTYAHLFDDKVMKQLKRRRYTGWGRLSRKLINGIRDKQSGKTILDFLKSDGFANRNFMQLIHDDSLTFKEDIQKAQVSGQGDSLHEHIANLAGSPAIKKGILQTVKVVDELVKVMGRHKPENIVIEMARENQTTQKGQKNSRERMKRIEEGIKELGSQILKEHPVENTQLQNEKLYLYYLQNGRDMYVDQELDINRLSDYDVDAIVPQSFLKDDSIDNKVLTRSDKNRGKSDNVPSEEVVKKMKNYWRQLLNAKLITQRKFDNLTKAERGGLSELDKAGFIKRQLVETRQITKHVAQILDSRMNTKYDENDKLIREVKVITLKSKLVSDFRKDFQFYKVREINNYHHAHDAYLNAVVGTALIKKYPKLESEFVYGDYKVYDVRKMIAKSEQEIGKATAKYFFYSNIMNFFKTEITLANGEIRKRPLIETNGETGEIVWDKGRDFATVRKVLSMPQVNIVKKTEVQTGGFSKESILPKRNSDKLIARKKDWDPKKYGGFDSPTVAYSVLVVAKVEKGKSKKLKSVKELLGITIMERSSFEKNPIDFLEAKGYKEVKKDLIIKLPKYSLFELENGRKRMLASAGELQKGNELALPSKYVNFLYLASHYEKLKGSPEDNEQKQLFVEQHKHYLDEIIEQISEFSKRVILADANLDKVLSAYNKHRDKPIREQAENIIHLFTLTNLGAPAAFKYFDTTIDRKRYTSTKEVLDATLIHQSITGLYETRIDLSQLGGDAYPYDVPDYASLGSGSPKKKRKVEDPKKKRKVDGIGSGSNGSSGEELLSKNYHLENEVARLKKGSGSGGSGSGGSGSGSGGSGSGGSGSGEELLSKNYHGSGSGQRGSKRTADGSEFESPKKKRKVX

SEQ ID NO: 137 - protein, 2554 aa, synthetic construct
  REGION 1..2554: note = V16_scFv-ZIM3-2a-D3a-hD3L-dCas9-2xGCN4
  SITE 2554: note = misc_feature - Xaa =
MPAAKRVKLDGSGPDIVMTQSPSSLSASVGDRVTITCRSSTGAVTTSNYASWVQEKPGKLFKGLIGGTNNRAPGVPSRFSGSLIGDKATLTISSLQPEDFATYFCALWYSNHWVFGQGTKVELKRGGGGSGGGGSGGGGSSGGGSEVKLLESGGGLVQPGGSLKLSCAVSGFSLTDYGVNWVRQAPGRGLEWIGVIWGDGITDYNSALKDRFIISKDNGKNTVYLQMSKVRSDDTALYYCVTGLFDYWGQGTLVTVSSYPYDVPDYAGGGGGSGGGGSGGGGSGGGGSLDPGGGGSGMNNSQGRVTFEDVTVNFTQGEWQRLNPEQRNLYRDVMLENYSNLVSVGQGETTKPDVILRLEQGKEPWLEEEEVLGSGRAEKNGDIGGQIWKPKDVKESLGSGATNFSLLKQAGDVEENPGPMPAAKRVKLDGSNHDQEFDPPKVYPPVPAEKRKPIRVLSLFDGIATGLLVLKDLGIQVDRYIASEVCEDSITVGMVRHQGKIMYVGDVRSVTQKHIQEWGPFDLVIGGSPCNDLSIVNPARKGLYEGTGRLFFEFYRLLHDARPKEGDDRPFFWLFENVVAMGVSDKRDISRFLESNPVMIDAKEVSAAHRARYFWGNLPGMNRPLASTVNDKLELQECLEHGRIAKFSKVRTITTRSNSIKQGKDQHFPVFMNEKEDILWCTEMERVFGFPVHYTDVSNMSRLARQRLLGRSWSVPVIRHLFAPLKEYFACVSSGNSNANSRGPSFSSGLVPLSLRGSHMFETVPVWRRQPVRVLSLFEDIKKELTSLGFLESGSDPGQLKHVVDVTDTVRKDVEEWGPFDLVYGATPPLGHTCDRPPSWYLFQFHRLLQYARPKPGSPRPFFWMFVDNLVLNKEDLDVASRFLEMEPVTIPDVHGGSLQNAVRVWSNIPAIRSSRHWALVSEEELSLLAQNKQSSKLAAKWPTKLVKNCFLPLREYFKYFSGGPSSGAPPPSGGSPAGSPTSTEEGTSESATPESGPGTSTEPSEGSAPGSPAGSPTSTEEGTSTEPSEGSAPGTSTEPSEPKKKRKVMDKKYSIGLAIGTNSVGWAVITDEYKVPSKKFKVLGNTDRHSIKKNLIGALLFDSGETAEATRLKRTARRRYTRRKNRICYLQEIFSNEMAKVDDSFFHRLEESFLVEEDKKHERHPIFGNIVDEVAYHEKYPTIYHLRKKLVDSTDKADLRLIYLALAHMIKFRGHFLIEGDLNPDNSDVDKLFIQLVQTYNQLFEENPINASGVDAKAILSARLSKSRRLENLIAQLPGEKKNGLFGNLIALSLGLTPNFKSNFDLAEDAKLQLSKDTYDDDLDNLLAQIGDQYADLFLAAKNLSDAILLSDILRVNTEITKAPLSASMIKRYDEHHQDLTLLKALVRQQLPEKYKEIFFDQSKNGYAGYIDGGASQEEFYKFIKPILEKMDGTEELLVKLNREDLLRKQRTFDNGSIPHQIHLGELHAILRRQEDFYPFLKDNREKIEKILTFRIPYYVGPLARGNSRFAWMTRKSEETITPWNFEEVVDKGASAQSFIERMTNFDKNLPNEKVLPKHSLLYEYFTVYNELTKVKYVTEGMRKPAFLSGEQKKAIVDLLFKTNRKVTVKQLKEDYFKKIECFDSVEISGVEDRFNASLGTYHDLLKIIKDKDFLDNEENEDILEDIVLTLTLFEDREMIEERLKTYAHLFDDKVMKQLKRRRYTGWGRLSRKLINGIRDKQSGKTILDFLKSDGFANRNFMQLIHDDSLTFKEDIQKAQVSGQGDSLHEHIANLAGSPAIKKGILQTVKVVDELVKVMGRHKPENIVIEMARENQTTQKGQKNSRERMKRIEEGIKELGSQILKEHPVENTQLQNEKLYLYYLQNGRDMYVDQELDINRLSDYDVDAIVPQSFLKDDSIDNKVLTRSDKNRGKSDNVPSEEVVKKMKNYWRQLLNAKLITQRKFDNLTKAERGGLSELDKAGFIKRQLVETRQITKHVAQILDSRMNTKYDENDKLIREVKVITLKSKLVSDFRKDFQFYKVREINNYHHAHDAYLNAVVGTALIKKYPKLESEFVYGDYKVYDVRKMIAKSEQEIGKATAKYFFYSNIMNFFKTEITLANGEIRKRPLIETNGETGEIVWDKGRDFATVRKVLSMPQVNIVKKTEVQTGGFSKESILPKRNSDKLIARKKDWDPKKYGGFDSPTVAYSVLVVAKVEKGKSKKLKSVKELLGITIMERSSFEKNPIDFLEAKGYKEVKKDLIIKLPKYSLFELENGRKRMLASAGELQKGNELALPSKYVNFLYLASHYEKLKGSPEDNEQKQLFVEQHKHYLDEIIEQISEFSKRVILADANLDKVLSAYNKHRDKPIREQAENIIHLFTLTNLGAPAAFKYFDTTIDRKRYTSTKEVLDATLIHQSITGLYETRIDLSQLGGDAYPYDVPDYASLGSGSPKKKRKVEDPKKKRKVDGIGSGSNGSSGEELLSKNYHLENEVARLKKGSGSGGSGSGGSGSGSGGSGSGGSGSGEELLSKNYHLENEVARLKKGSGSGQRGSKRTADGSEFESPKKKRKVX

SEQ ID NO: 138 - protein, 2922 aa, synthetic construct
  REGION 1..2922: note = V17_scFv-ZIM3-2a-D3a-hD3L-dCas9-10xGCN4
  SITE 2922: note = misc_feature - Xaa =
MPAAKRVKLDGSGPDIVMTQSPSSLSASVGDRVTITCRSSTGAVTTSNYASWVQEKPGKLFKGLIGGTNNRAPGVPSRFSGSLIGDKATLTISSLQPEDFATYFCALWYSNHWVFGQGTKVELKRGGGGSGGGGSGGGGSSGGGSEVKLLESGGGLVQPGGSLKLSCAVSGFSLTDYGVNWVRQAPGRGLEWIGVIWGDGITDYNSALKDRFIISKDNGKNTVYLQMSKVRSDDTALYYCVTGLFDYWGQGTLVTVSSYPYDVPDYAGGGGGSGGGGSGGGGSGGGGSLDPGGGGSGMNNSQGRVTFEDVTVNFTQGEWQRLNPEQRNLYRDVMLENYSNLVSVGQGETTKPDVILRLEQGKEPWLEEEEVLGSGRAEKNGDIGGQIWKPKDVKESLGSGATNFSLLKQAGDVEENPGPMPAAKRVKLDGSNHDQEFDPPKVYPPVPAEKRKPIRVLSLFDGIATGLLVLKDLGIQVDRYIASEVCEDSITVGMVRHQGKIMYVGDVRSVTQKHIQEWGPFDLVIGGSPCNDLSIVNPARKGLYEGTGRLFFEFYRLLHDARPKEGDDRPFFWLFENVVAMGVSDKRDISRFLESNPVMIDAKEVSAAHRARYFWGNLPGMNRPLASTVNDKLELQECLEHGRIAKFSKVRTITTRSNSIKQGKDQHFPVFMNEKEDILWCTEMERVFGFPVHYTDVSNMSRLARQRLLGRSWSVPVIRHLFAPLKEYFACVSSGNSNANSRGPSFSSGLVPLSLRGSHMFETVPVWRRQPVRVLSLFEDIKKELTSLGFLESGSDPGQLKHVVDVTDTVRKDVEEWGPFDLVYGATPPLGHTCDRPPSWYLFQFHRLLQYARPKPGSPRPFFWMFVDNLVLNKEDLDVASRFLEMEPVTIPDVHGGSLQNAVRVWSNIPAIRSSRHWALVSEEELSLLAQNKQSSKLAAKWPTKLVKNCFLPLREYFKYFSGGPSSGAPPPSGGSPAGSPTSTEEGTSESATPESGPGTSTEPSEGSAPGSPAGSPTSTEEGTSTEPSEGSAPGTSTEPSEPKKKRKVMDKKYSIGLAIGTNSVGWAVITDEYKVPSKKFKVLGNTDRHSIKKNLIGALLFDSGETAEATRLKRTARRRYTRRKNRICYLQEIFSNEMAKVDDSFFHRLEESFLVEEDKKHERHPIFGNIVDEVAYHEKYPTIYHLRKKLVDSTDKADLRLIYLALAHMIKFRGHFLIEGDLNPDNSDVDKLFIQLVQTYNQLFEENPINASGVDAKAILSARLSKSRRLENLIAQLPGEKKNGLFGNLIALSLGLTPNFKSNFDLAEDAKLQLSKDTYDDDLDNLLAQIGDQYADLFLAAKNLSDAILLSDILRVNTEITKAPLSASMIKRYDEHHQDLTLLKALVRQQLPEKYKEIFFDQSKNGYAGYIDGGASQEEFYKFIKPILEKMDGTEELLVKLNREDLLRKQRTFDNGSIPHQIHLGELHAILRRQEDFYPFLKDNREKIEKILTFRIPYYVGPLARGNSRFAWMTRKSEETITPWNFEEVVDKGASAQSFIERMTNFDKNLPNEKVLPKHSLLYEYFTVYNELTKVKYVTEGMRKPAFLSGEQKKAIVDLLFKTNRKVTVKQLKEDYFKKIECFDSVEISGVEDRFNASLGTYHDLLKIIKDKDFLDNEENEDILEDIVLTLTLFEDREMIEERLKTYAHLFDDKVMKQLKRRRYTGWGRLSRKLINGIRDKQSGKTILDFLKSDGFANRNFMQLIHDDSLTFKEDIQKAQVSGQGDSLHEHIANLAGSPAIKKGILQTVKVVDELVKVMGRHKPENIVIEMARENQTTQKGQKNSRERMKRIEEGIKELGSQILKEHPVENTQLQNEKLYLYYLQNGRDMYVDQELDINRLSDYDVDAIVPQSFLKDDSIDNKVLTRSDKNRGKSDNVPSEEVVKKMKNYWRQLLNAKLITQRKFDNLTKAERGGLSELDKAGFIKRQLVETRQITKHVAQILDSRMNTKYDENDKLIREVKVITLKSKLVSDFRKDFQFYKVREINNYHHAHDAYLNAVVGTALIKKYPKLESEFVYGDYKVYDVRKMIAKSEQEIGKATAKYFFYSNIMNFFKTEITLANGEIRKRPLIETNGETGEIVWDKGRDFATVRKVLSMPQVNIVKKTEVQTGGFSKESILPKRNSDKLIARKKDWDPKKYGGFDSPTVAYSVLVVAKVEKGKSKKLKSVKELLGITIMERSSFEKNPIDFLEAKGYKEVKKDLIIKLPKYSLFELENGRKRMLASAGELQKGNELALPSKYVNFLYLASHYEKLKGSPEDNEQKQLFVEQHKHYLDEIIEQISEFSKRVILADANLDKVLSAYNKHRDKPIREQAENIIHLFTLTNLGAPAAFKYFDTTIDRKRYTSTKEVLDATLIHQSITGLYETRIDLSQLGGDAYPYDVPDYASLGSGSPKKKRKVEDPKKKRKVDGIGSGSNGSSGEELLSKNYHLENEVARLKKGSGSGGSGSGGSGSGSGGSGSGGSGSGEELLSKNYHLENEVARLKKGSGSGGSGSGGSGSGSGGSGSGGSGSGEELLSKNYHLENEVARLKKGSGSGGSGSGGSGSGSGGSGSGGSGSGEELLSKNYHLENEVARLKKGSGSGGSGSGGSGSGSGGSGSGGSGSGEELLSKNYHLENEVARLKKGSGSGGSGSGGSGSGSGGSGSGGSGSGEELLSKNYHLENEVARLKKGSGSGGSGSGGSGSGSGGSGSGGSGSGEELLSKNYHLENEVARLKKGSGSGGSGSGGSGSGSGGSGSGGSGSGEELLSKNYHLENEVARLKKGSGSGGSGSGGSGSGSGGSGSGGSGSGEELLSKNYHLENEVARLKKGSGSGGSGSGGSGSGSGGSGSGGSGSGEELLSKNYHLENEVARLKKGSGSGQRGSKRTADGSEFESPKKKRKVX

SEQ ID NO: 139 - protein, 2404 aa, synthetic construct
  REGION 1..2404: note = V18_scFv-ZIM3-2a-D3a-hD3L-dCas12a-1xGCN4
  SITE 2404: note = misc_feature - Xaa =
MPAAKRVKLDGSGPDIVMTQSPSSLSASVGDRVTITCRSSTGAVTTSNYASWVQEKPGKLFKGLIGGTNNRAPGVPSRFSGSLIGDKATLTISSLQPEDFATYFCALWYSNHWVFGQGTKVELKRGGGGSGGGGSGGGGSSGGGSEVKLLESGGGLVQPGGSLKLSCAVSGFSLTDYGVNWVRQAPGRGLEWIGVIWGDGITDYNSALKDRFIISKDNGKNTVYLQMSKVRSDDTALYYCVTGLFDYWGQGTLVTVSSYPYDVPDYAGGGGGSGGGGSGGGGSGGGGSLDPGGGGSGMNNSQGRVTFEDVTVNFTQGEWQRLNPEQRNLYRDVMLENYSNLVSVGQGETTKPDVILRLEQGKEPWLEEEEVLGSGRAEKNGDIGGQIWKPKDVKESLGSGATNFSLLKQAGDVEENPGPMPAAKRVKLDGSNHDQEFDPPKVYPPVPAEKRKPIRVLSLFDGIATGLLVLKDLGIQVDRYIASEVCEDSITVGMVRHQGKIMYVGDVRSVTQKHIQEWGPFDLVIGGSPCNDLSIVNPARKGLYEGTGRLFFEFYRLLHDARPKEGDDRPFFWLFENVVAMGVSDKRDISRFLESNPVMIDAKEVSAAHRARYFWGNLPGMNRPLASTVNDKLELQECLEHGRIAKFSKVRTITTRSNSIKQGKDQHFPVFMNEKEDILWCTEMERVFGFPVHYTDVSNMSRLARQRLLGRSWSVPVIRHLFAPLKEYFACVSSGNSNANSRGPSFSSGLVPLSLRGSHMFETVPVWRRQPVRVLSLFEDIKKELTSLGFLESGSDPGQLKHVVDVTDTVRKDVEEWGPFDLVYGATPPLGHTCDRPPSWYLFQFHRLLQYARPKPGSPRPFFWMFVDNLVLNKEDLDVASRFLEMEPVTIPDVHGGSLQNAVRVWSNIPAIRSSRHWALVSEEELSLLAQNKQSSKLAAKWPTKLVKNCFLPLREYFKYFSGGPSSGAPPPSGGSPAGSPTSTEEGTSESATPESGPGTSTEPSEGSAPGSPAGSPTSTEEGTSTEPSEGSAPGTSTEPSEPKKKRKVMSKLEKFTNCYSLSKTLRFKAIPVGKTQENIDNKRLLVEDEKRAEDYKGVKKLLDRYYLSFINDVLHSIKLKNLNNYISLFRKKTRTEKENKELENLEINLRKEIAKAFKGNEGYKSLFKKDIIETILPEFLDDKDEIALVNSFNGFTTAFTGFFDNRENMFSEEAKSTSIAFRCINENLTRYISNMDIFEKVDAIFDKHEVQEIKEKILNSDYDVEDFFEGEFFNFVLTQEGIDVYNAIIGGFVTESGEKIKGLNEYINLYNQKTKQKLPKFKPLYKQVLSDRESLSFYGEGYTSDEEVLEVFRNTLNKNSEIFSSIKKLEKLFKNFDEYSSAGIFVKNGPAISTISKDIFGEWNVIRDKWNAEYDDIHLKKKAVVTEKYEDDRRKSFKKIGSFSLEQLQEYADADLSVVEKLKEIIIQKVDEIYKVYGSSEKLFDADFVLEKSLKKNDAVVAIMKDLLDSVKSFENYIKAFFGEGKETNRDESFYGDFVLAYDILLKVDHIYDAIRNYVTQKPYSKDKFKLYFQNPQFMGGWDKDKETDYRATILRYGSKYYLAIMDKKYAKCLQKIDKDDVNGNYEKINYKLLPGPNKMLPKVFFSKKWMAYYNPSEDIQKIYKNGTFKKGDMFNLNDCHKLIDFFKDSISRYPKWSNAYDFNFSETEKYKDIAGFYREVEEQGYKVSFESASKKEVDKLVEEGKLYMFQIYNKDFSDKSHGTPNLHTMYFKLLFDENNHGQIRLSGGAELFMRRASLKKEELVVHPANSPIANKNPDNPKKTTTLSYDVYKDKRFSEDQYELHIPIAINKCPKNIFKINTEVRVLLKHDDNPYVIGIARGERNLLYIVVVDGKGNIVEQYSLNEIINNFNGIRIKTDYHSLLDKKEKERFEARQNWTSIENIKELKAGYISQVVHKICELVEKYDAVIALADLNSGFKNSRVKVEKQVYQKFEKMLIDKLNYMVDKKSNPCATGGALKGYQITNKFESFKSMSTQNGFIFYIPAWLTSKIDPSTGFVNLLKTKYTSIADSKKFISSFDRIMYVPEEDLFEFALDYKNFSRTDADYIKKWKLYSYGNRIRIFRNPKKNNVFDWEEVCLTSAYKELFNKYGINYQQGDIRALLCEQSDKAFYSSFMALMSLMLQMRNSITGRTDVAFLISPVKNSDGIFYDSRNYEAQENAILPKNADANGAYNIARKVLWAIGQFKKAEDEKLDKVKIAISNKEWLEYAQTSVKHAYPYDVPDYASLGSGSPKKKRKVEDPKKKRKVDGIGSGSNGSSGEELLSKNYHLENEVARLKKGSGSGGSGSGGSGSGSGGSGSGGSGSGEELLSKNYHGSGSGQRGSKRTADGSEFESPKKKRKVX

SEQ ID NO: 140 - protein, 2187 aa, synthetic construct
  REGION 1..2187: note = V19_scFv-ZIM3-2a-D3a-hD3L-dCas12i-1xGCN4
  SITE 2187: note = misc_feature - Xaa =
MPAAKRVKLDGSGPDIVMTQSPSSLSASVGDRVTITCRSSTGAVTTSNYASWVQEKPGKLFKGLIGGTNNRAPGVPSRFSGSLIGDKATLTISSLQPEDFATYFCALWYSNHWVFGQGTKVELKRGGGGSGGGGSGGGGSSGGGSEVKLLESGGGLVQPGGSLKLSCAVSGFSLTDYGVNWVRQAPGRGLEWIGVIWGDGITDYNSALKDRFIISKDNGKNTVYLQMSKVRSDDTALYYCVTGLFDYWGQGTLVTVSSYPYDVPDYAGGGGGSGGGGSGGGGSGGGGSLDPGGGGSGMNNSQGRVTFEDVTVNFTQGEWQRLNPEQRNLYRDVMLENYSNLVSVGQGETTKPDVILRLEQGKEPWLEEEEVLGSGRAEKNGDIGGQIWKPKDVKESLGSGATNFSLLKQAGDVEENPGPMPAAKRVKLDGSNHDQEFDPPKVYPPVPAEKRKPIRVLSLFDGIATGLLVLKDLGIQVDRYIASEVCEDSITVGMVRHQGKIMYVGDVRSVTQKHIQEWGPFDLVIGGSPCNDLSIVNPARKGLYEGTGRLFFEFYRLLHDARPKEGDDRPFFWLFENVVAMGVSDKRDISRFLESNPVMIDAKEVSAAHRARYFWGNLPGMNRPLASTVNDKLELQECLEHGRIAKFSKVRTITTRSNSIKQGKDQHFPVFMNEKEDILWCTEMERVFGFPVHYTDVSNMSRLARQRLLGRSWSVPVIRHLFAPLKEYFACVSSGNSNANSRGPSFSSGLVPLSLRGSHMFETVPVWRRQPVRVLSLFEDIKKELTSLGFLESGSDPGQLKHVVDVTDTVRKDVEEWGPFDLVYGATPPLGHTCDRPPSWYLFQFHRLLQYARPKPGSPRPFFWMFVDNLVLNKEDLDVASRFLEMEPVTIPDVHGGSLQNAVRVWSNIPAIRSSRHWALVSEEELSLLAQNKQSSKLAAKWPTKLVKNCFLPLREYFKYFSGGPSSGAPPPSGGSPAGSPTSTEEGTSESATPESGPGTSTEPSEGSAPGSPAGSPTSTEEGTSTEPSEGSAPGTSTEPSEPKKKRKVMGITMSDTTFRPYKSKLNPNERKMPMVVDTMNWCDNACSVFFDLFVGLYGGVKIGDVTNFLTEKQDTTTDADLLCAINWFRAMPVSNPDAVVGPEQLVVRFRDYSGHNPSPMASMYLSAPVNPRYTWVDCRFLYQQMCQTLGANLDVDISTLVQTGLLPIQKDTQLNAYSFCSNVFGEGVKEDPSAKVTSYTAAANALSGATNPIITYEDYRQILSSAITNRPSRKGAKDILAADLDSTKTGVLPGNYVSQRIAMYQASAASKARGVVLPNRLRVKAYLQNLVGLNYICTTWAAPMLRAVGDIKSKNSNNYRFVGERLERQQEIDNLLAVSNIRSAQAILQQFRANESNQFYIKKRHIGKGLPSLYDMWDLMDEKEGIDNYIQSLKGDKTERLPIRELLQIIYPHRKSVSAELFLSAAELTDVEDRQNRCMVHPTVRGSLVINFGKSSTIFGAITPPDTLIKFRGEMVPAGQTGMIWFTMHLVDGGKWVKHHIPCHSSRYFEEIYAWKKDLPTLPFPRRSLYGYAIGNKISDTRKIDLRRKKASKQYLRTLENMTHNVEFDPTTQFMVDQELNVTITARVKKIPPVRDVPVGSRIMGLNKNQTIRDCYSIWERVEANTSGSFQHPVVQDVWLRLVADGHVTSTVNGPNGQIDQMSYSGPDVANCGNWMQERSNFITSVDDADQSIMKHFLWNNRVKLYAWNCVYAGTLMKAISKQMTTANRNLFRNEILSFVGGRFGCRLGSLAQVSLDLLRRMKSVISCYFSRNNAFTIEERSAFDKELMELFESLDNKMNNKRKEKVNRTLSSIFQVAKQHNVVRLVVTKNLQTPDANVRSVMNQRSVDWCARKIEEKIVDLGNVIGIYVDLVEALDLSHLDPFIYIAKGDVGKECQFDEVESSSLLPIHTSMFRDWHGLVNKGRTTTPIYHSALRSFASHYGLRFDDLARIKAAELAKMLPDQKVFIPHRGGRFFMSTYPVTSTSRPVSYDGRQRFLNSGDMVAPVNTMLRGFRRARSAYPYDVPDYASLGSGSPKKKRKVEDPKKKRKVDGIGSGSNGSSGEELLSKNYHLENEVARLKKGSGSGGSGSGGSGSGSGGSGSGGSGSGEELLSKNYHGSGSGQRGSKRTADGSEFESPKKKRKVX

SEQ ID NO: 141 - protein, 2511 aa, synthetic construct
  REGION 1..2511: note = V20_KRAB-scFv-2a-D3a-D3l-dCas9-2xGCN4
  SITE 2511: note = misc_feature - Xaa =
MPAAKRVKLDGSRTLVTFKDVFVDFTREEWKLLDTAQQIVYRNVMLENYKNLVSLGYQLTKPDVILRLEKGEEPGSGMGPDIVMTQSPSSLSASVGDRVTITCRSSTGAVTTSNYASWVQEKPGKLFKGLIGGTNNRAPGVPSRFSGSLIGDKATLTISSLQPEDFATYFCALWYSNHWVFGQGTKVELKRGGGGSGGGGSGGGGSSGGGSEVKLLESGGGLVQPGGSLKLSCAVSGFSLTDYGVNWVRQAPGRGLEWIGVIWGDGITDYNSALKDRFIISKDNGKNTVYLQMSKVRSDDTALYYCVTGLFDYWGQGTLVTVSSYPYDVPDYAGGGGGSGGGGSGGGGSGGGGSGSGATNFSLLKQAGDVEENPGPMPAAKRVKLDGSNHDQEFDPPKVYPPVPAEKRKPIRVLSLFDGIATGLLVLKDLGIQVDRYIASEVCEDSITVGMVRHQGKIMYVGDVRSVTQKHIQEWGPFDLVIGGSPCNDLSIVNPARKGLYEGTGRLFFEFYRLLHDARPKEGDDRPFFWLFENVVAMGVSDKRDISRFLESNPVMIDAKEVSAAHRARYFWGNLPGMNRPLASTVNDKLELQECLEHGRIAKFSKVRTITTRSNSIKQGKDQHFPVFMNEKEDILWCTEMERVFGFPVHYTDVSNMSRLARQRLLGRSWSVPVIRHLFAPLKEYFACVSSGNSNANSRGPSFSSGLVPLSLRGSHMFETVPVWRRQPVRVLSLFEDIKKELTSLGFLESGSDPGQLKHVVDVTDTVRKDVEEWGPFDLVYGATPPLGHTCDRPPSWYLFQFHRLLQYARPKPGSPRPFFWMFVDNLVLNKEDLDVASRFLEMEPVTIPDVHGGSLQNAVRVWSNIPAIRSSRHWALVSEEELSLLAQNKQSSKLAAKWPTKLVKNCFLPLREYFKYFSGGPSSGAPPPSGGSPAGSPTSTEEGTSESATPESGPGTSTEPSEGSAPGSPAGSPTSTEEGTSTEPSEGSAPGTSTEPSEPKKKRKVMDKKYSIGLAIGTNSVGWAVITDEYKVPSKKFKVLGNTDRHSIKKNLIGALLFDSGETAEATRLKRTARRRYTRRKNRICYLQEIFSNEMAKVDDSFFHRLEESFLVEEDKKHERHPIFGNIVDEVAYHEKYPTIYHLRKKLVDSTDKADLRLIYLALAHMIKFRGHFLIEGDLNPDNSDVDKLFIQLVQTYNQLFEENPINASGVDAKAILSARLSKSRRLENLIAQLPGEKKNGLFGNLIALSLGLTPNFKSNFDLAEDAKLQLSKDTYDDDLDNLLAQIGDQYADLFLAAKNLSDAILLSDILRVNTEITKAPLSASMIKRYDEHHQDLTLLKALVRQQLPEKYKEIFFDQSKNGYAGYIDGGASQEEFYKFIKPILEKMDGTEELLVKLNREDLLRKQRTFDNGSIPHQIHLGELHAILRRQEDFYPFLKDNREKIEKILTFRIPYYVGPLARGNSRFAWMTRKSEETITPWNFEEVVDKGASAQSFIERMTNFDKNLPNEKVLPKHSLLYEYFTVYNELTKVKYVTEGMRKPAFLSGEQKKAIVDLLFKTNRKVTVKQLKEDYFKKIECFDSVEISGVEDRFNASLGTYHDLLKIIKDKDFLDNEENEDILEDIVLTLTLFEDREMIEERLKTYAHLFDDKVMKQLKRRRYTGWGRLSRKLINGIRDKQSGKTILDFLKSDGFANRNFMQLIHDDSLTFKEDIQKAQVSGQGDSLHEHIANLAGSPAIKKGILQTVKVVDELVKVMGRHKPENIVIEMARENQTTQKGQKNSRERMKRIEEGIKELGSQILKEHPVENTQLQNEKLYLYYLQNGRDMYVDQELDINRLSDYDVDAIVPQSFLKDDSIDNKVLTRSDKNRGKSDNVPSEEVVKKMKNYWRQLLNAKLITQRKFDNLTKAERGGLSELDKAGFIKRQLVETRQITKHVAQILDSRMNTKYDENDKLIREVKVITLKSKLVSDFRKDFQFYKVREINNYHHAHDAYLNAVVGTALIKKYPKLESEFVYGDYKVYDVRKMIAKSEQEIGKATAKYFFYSNIMNFFKTEITLANGEIRKRPLIETNGETGEIVWDKGRDFATVRKVLSMPQVNIVKKTEVQTGGFSKESILPKRNSDKLIARKKDWDPKKYGGFDSPTVAYSVLVVAKVEKGKSKKLKSVKELLGITIMERSSFEKNPIDFLEAKGYKEVKKDLIIKLPKYSLFELENGRKRMLASAGELQKGNELALPSKYVNFLYLASHYEKLKGSPEDNEQKQLFVEQHKHYLDEIIEQISEFSKRVILADANLDKVLSAYNKHRDKPIREQAENIIHLFTLTNLGAPAAFKYFDTTIDRKRYTSTKEVLDATLIHQSITGLYETRIDLSQLGGDAYPYDVPDYASLGSGSPKKKRKVEDPKKKRKVDGIGSGSNGSSGEELLSKNYHLENEVARLKKGSGSGGSGSGGSGSGSGGSGSGGSGSGEELLSKNYHLENEVARLKKGSGSGQRGSKRTADGSEFESPKKKRKVX

SEQ ID NO: 142 - protein, 2750 aa, synthetic construct
  REGION 1..2750: note = V21_hSIRT1-scFv-2a-D3a-D3l-dCas9-2xGCN4
  SITE 2750: note = misc_feature - Xaa =
MPAAKRVKLDGSTILKDLLPETIPPPELDDMTLWQIVINILSEPPKRKKRKDINTIEDAVKLLQECKKIIVLTGAGVSVSCGIPDFRSRDGIYARLAVDFPDLPDPQAMFDIEYFRKDPRPFFKFAKEIYPGQFQPSLCHKFIALSDKEGKLLRNYTQNIDTLEQVAGIQRIIQCHGSFATASCLICKYKVDCEAVRGDIFNQVVPRCPRCPADEPLAIMKPEIVFFGENLPEQFHRAMKYDKDEVDLLIVIGSSLKVRPVALIPSSIPHEVPQILINREPLPHLHFDVELLGDCDVIINELCHRLGGEYAKLGSGMGPDIVMTQSPSSLSASVGDRVTITCRSSTGAVTTSNYASWVQEKPGKLFKGLIGGTNNRAPGVPSRFSGSLIGDKATLTISSLQPEDFATYFCALWYSNHWVFGQGTKVELKRGGGGSGGGGSGGGGSSGGGSEVKLLESGGGLVQPGGSLKLSCAVSGFSLTDYGVNWVRQAPGRGLEWIGVIWGDGITDYNSALKDRFIISKDNGKNTVYLQMSKVRSDDTALYYCVTGLFDYWGQGTLVTVSSYPYDVPDYAGGGGGSGGGGSGGGGSGGGGSGSGATNFSLLKQAGDVEENPGPMPAAKRVKLDGSNHDQEFDPPKVYPPVPAEKRKPIRVLSLFDGIATGLLVLKDLGIQVDRYIASEVCEDSITVGMVRHQGKIMYVGDVRSVTQKHIQEWGPFDLVIGGSPCNDLSIVNPARKGLYEGTGRLFFEFYRLLHDARPKEGDDRPFFWLFENVVAMGVSDKRDISRFLESNPVMIDAKEVSAAHRARYFWGNLPGMNRPLASTVNDKLELQECLEHGRIAKFSKVRTITTRSNSIKQGKDQHFPVFMNEKEDILWCTEMERVFGFPVHYTDVSNMSRLARQRLLGRSWSVPVIRHLFAPLKEYFACVSSGNSNANSRGPSFSSGLVPLSLRGSHMFETVPVWRRQPVRVLSLFEDIKKELTSLGFLESGSDPGQLKHVVDVTDTVRKDVEEWGPFDLVYGATPPLGHTCDRPPSWYLFQFHRLLQYARPKPGSPRPFFWMFVDNLVLNKEDLDVASRFLEMEPVTIPDVHGGSLQNAVRVWSNIPAIRSSRHWALVSEEELSLLAQNKQSSKLAAKWPTKLVKNCFLPLREYFKYFSGGPSSGAPPPSGGSPAGSPTSTEEGTSESATPESGPGTSTEPSEGSAPGSPAGSPTSTEEGTSTEPSEGSAPGTSTEPSEPKKKRKVMDKKYSIGLAIGTNSVGWAVITDEYKVPSKKFKVLGNTDRHSIKKNLIGALLFDSGETAEATRLKRTARRRYTRRKNRICYLQEIFSNEMAKVDDSFFHRLEESFLVEEDKKHERHPIFGNIVDEVAYHEKYPTIYHLRKKLVDSTDKADLRLIYLALAHMIKFRGHFLIEGDLNPDNSDVDKLFIQLVQTYNQLFEENPINASGVDAKAILSARLSKSRRLENLIAQLPGEKKNGLFGNLIALSLGLTPNFKSNFDLAEDAKLQLSKDTYDDDLDNLLAQIGDQYADLFLAAKNLSDAILLSDILRVNTEITKAPLSASMIKRYDEHHQDLTLLKALVRQQLPEKYKEIFFDQSKNGYAGYIDGGASQEEFYKFIKPILEKMDGTEELLVKLNREDLLRKQRTFDNGSIPHQIHLGELHAILRRQEDFYPFLKDNREKIEKILTFRIPYYVGPLARGNSRFAWMTRKSEETITPWNFEEVVDKGASAQSFIERMTNFDKNLPNEKVLPKHSLLYEYFTVYNELTKVKYVTEGMRKPAFLSGEQKKAIVDLLFKTNRKVTVKQLKEDYFKKIECFDSVEISGVEDRFNASLGTYHDLLKIIKDKDFLDNEENEDILEDIVLTLTLFEDREMIEERLKTYAHLFDDKVMKQLKRRRYTGWGRLSRKLINGIRDKQSGKTILDFLKSDGFANRNFMQLIHDDSLTFKEDIQKAQVSGQGDSLHEHIANLAGSPAIKKGILQTVKVVDELVKVMGRHKPENIVIEMARENQTTQKGQKNSRERMKRIEEGIKELGSQILKEHPVENTQLQNEKLYLYYLQNGRDMYVDQELDINRLSDYDVDAIVPQSFLKDDSIDNKVLTRSDKNRGKSDNVPSEEVVKKMKNYWRQLLNAKLITQRKFDNLTKAERGGLSELDKAGFIKRQLVETRQITKHVAQILDSRMNTKYDENDKLIREVKVITLKSKLVSDFRKDFQFYKVREINNYHHAHDAYLNAVVGTALIKKYPKLESEFVYGDYKVYDVRKMIAKSEQEIGKATAKYFFYSNIMNFFKTEITLANGEIRKRPLIETNGETGEIVWDKGRDFATVRKVLSMPQVNIVKKTEVQTGGFSKESILPKRNSDKLIARKKDWDPKKYGGFDSPTVAYSVLVVAKVEKGKSKKLKSVKELLGITIMERSSFEKNPIDFLEAKGYKEVKKDLIIKLPKYSLFELENGRKRMLASAGELQKGNELALPSKYVNFLYLASHYEKLKGSPEDNEQKQLFVEQHKHYLDEIIEQISEFSKRVILADANLDKVLSAYNKHRDKPIREQAENIIHLFTLTNLGAPAAFKYFDTTIDRKRYTSTKEVLDATLIHQSITGLYETRIDLSQLGGDAYPYDVPDYASLGSGSPKKKRKVEDPKKKRKVDGIGSGSNGSSGEELLSKNYHLENEVARLKKGSGSGGSGSGGSGSGSGGSGSGGSGSGEELLSKNYHLENEVARLKKGSGSGQRGSKRTADGSEFESPKKKRKVX

SEQ ID NO: 143 - protein, 2487 aa, synthetic construct
  REGION 1..2487: note = V22_D3a-D3l-scFv-2a-1xGCN4-dCas9-KRAB
  SITE 2487: note = misc_feature - Xaa =
MPAAKRVKLDGSNHDQEFDPPKVYPPVPAEKRKPIRVLSLFDGIATGLLVLKDLGIQVDRYIASEVCEDSITVGMVRHQGKIMYVGDVRSVTQKHIQEWGPFDLVIGGSPCNDLSIVNPARKGLYEGTGRLFFEFYRLLHDARPKEGDDRPFFWLFENVVAMGVSDKRDISRFLESNPVMIDAKEVSAAHRARYFWGNLPGMNRPLASTVNDKLELQECLEHGRIAKFSKVRTITTRSNSIKQGKDQHFPVFMNEKEDILWCTEMERVFGFPVHYTDVSNMSRLARQRLLGRSWSVPVIRHLFAPLKEYFACVSSGNSNANSRGPSFSSGLVPLSLRGSHMGPMEIYKTVSAWKRQPVRVLSLFRNIDKVLKSLGFLESGSGSGGGTLKYVEDVTNVVRRDVEKWGPFDLVYGSTQPLGSSCDRCPGWYMFQFHRILQYALPRQESQRPFFWIFMDNLLLTEDDQETTTRFLQTEAVTLQDVRGRDYQNAMRVWSNIPGLKSKHAPLTPKEEEYLQAQVRSRSKLDAPKVDLLVKNCLLPLREYFKYFSQNSLPLGGPSSGAPPPSGGSPAGSPTSTEEGTSESATPESGPGTSTEPSEGSAPGSPAGSPTSTEEGTSTEPSEGSAPGTSTEPSEGPDIVMTQSPSSLSASVGDRVTITCRSSTGAVTTSNYASWVQEKPGKLFKGLIGGTNNRAPGVPSRFSGSLIGDKATLTISSLQPEDFATYFCALWYSNHWVFGQGTKVELKRGGGGSGGGGSGGGGSSGGGSEVKLLESGGGLVQPGGSLKLSCAVSGFSLTDYGVNWVRQAPGRGLEWIGVIWGDGITDYNSALKDRFIISKDNGKNTVYLQMSKVRSDDTALYYCVTGLFDYWGQGTLVTVSSYPYDVPDYAGGGGGSGGGGSGGGGSGGGGSGSGATNFSLLKQAGDVEENPGPMPAAKRVKLDGSGSGGSGSGEELLSKNYHLENEVARLKKGSGSGGSGSGGSGSGSGGSGSGGSGSGPKKKRKVMDKKYSIGLAIGTNSVGWAVITDEYKVPSKKFKVLGNTDRHSIKKNLIGALLFDSGETAEATRLKRTARRRYTRRKNRICYLQEIFSNEMAKVDDSFFHRLEESFLVEEDKKHERHPIFGNIVDEVAYHEKYPTIYHLRKKLVDSTDKADLRLIYLALAHMIKFRGHFLIEGDLNPDNSDVDKLFIQLVQTYNQLFEENPINASGVDAKAILSARLSKSRRLENLIAQLPGEKKNGLFGNLIALSLGLTPNFKSNFDLAEDAKLQLSKDTYDDDLDNLLAQIGDQYADLFLAAKNLSDAILLSDILRVNTEITKAPLSASMIKRYDEHHQDLTLLKALVRQQLPEKYKEIFFDQSKNGYAGYIDGGASQEEFYKFIKPILEKMDGTEELLVKLNREDLLRKQRTFDNGSIPHQIHLGELHAILRRQEDFYPFLKDNREKIEKILTFRIPYYVGPLARGNSRFAWMTRKSEETITPWNFEEVVDKGASAQSFIERMTNFDKNLPNEKVLPKHSLLYEYFTVYNELTKVKYVTEGMRKPAFLSGEQKKAIVDLLFKTNRKVTVKQLKEDYFKKIECFDSVEISGVEDRFNASLGTYHDLLKIIKDKDFLDNEENEDILEDIVLTLTLFEDREMIEERLKTYAHLFDDKVMKQLKRRRYTGWGRLSRKLINGIRDKQSGKTILDFLKSDGFANRNFMQLIHDDSLTFKEDIQKAQVSGQGDSLHEHIANLAGSPAIKKGILQTVKVVDELVKVMGRHKPENIVIEMARENQTTQKGQKNSRERMKRIEEGIKELGSQILKEHPVENTQLQNEKLYLYYLQNGRDMYVDQELDINRLSDYDVDAIVPQSFLKDDSIDNKVLTRSDKNRGKSDNVPSEEVVKKMKNYWRQLLNAKLITQRKFDNLTKAERGGLSELDKAGFIKRQLVETRQITKHVAQILDSRMNTKYDENDKLIREVKVITLKSKLVSDFRKDFQFYKVREINNYHHAHDAYLNAVVGTALIKKYPKLESEFVYGDYKVYDVRKMIAKSEQEIGKATAKYFFYSNIMNFFKTEITLANGEIRKRPLIETNGETGEIVWDKGRDFATVRKVLSMPQVNIVKKTEVQTGGFSKESILPKRNSDKLIARKKDWDPKKYGGFDSPTVAYSVLVVAKVEKGKSKKLKSVKELLGITIMERSSFEKNPIDFLEAKGYKEVKKDLIIKLPKYSLFELENGRKRMLASAGELQKGNELALPSKYVNFLYLASHYEKLKGSPEDNEQKQLFVEQHKHYLDEIIEQISEFSKRVILADANLDKVLSAYNKHRDKPIREQAENIIHLFTLTNLGAPAAFKYFDTTIDRKRYTSTKEVLDATLIHQSITGLYETRIDLSQLGGDAYPYDVPDYASLGSGSPKKKRKVEDPKKKRKVDGSGSETPGTSESATPESRTLVTFKDVFVDFTREEWKLLDTAQQIVYRNVMLENYKNLVSLGYQLTKPDVILRLEKGEEPX

SEQ ID NO: 144 - protein, 2525 aa, synthetic construct
  REGION 1..2525: note = V23_D3a-D3l-scFv-2a-2xGCN4-dCas9-KRAB
  SITE 2525: note = misc_feature - Xaa =
MPAAKRVKLDGSNHDQEFDPPKVYPPVPAEKRKPIRVLSLFDGIATGLLVLKDLGIQVDRYIASEVCEDSITVGMVRHQGKIMYVGDVRSVTQKHIQEWGPFDLVIGGSPCNDLSIVNPARKGLYEGTGRLFFEFYRLLHDARPKEGDDRPFFWLFENVVAMGVSDKRDISRFLESNPVMIDAKEVSAAHRARYFWGNLPGMNRPLASTVNDKLELQECLEHGRIAKFSKVRTITTRSNSIKQGKDQHFPVFMNEKEDILWCTEMERVFGFPVHYTDVSNMSRLARQRLLGRSWSVPVIRHLFAPLKEYFACVSSGNSNANSRGPSFSSGLVPLSLRGSHMGPMEIYKTVSAWKRQPVRVLSLFRNIDKVLKSLGFLESGSGSGGGTLKYVEDVTNVVRRDVEKWGPFDLVYGSTQPLGSSCDRCPGWYMFQFHRILQYALPRQESQRPFFWIFMDNLLLTEDDQETTTRFLQTEAVTLQDVRGRDYQNAMRVWSNIPGLKSKHAPLTPKEEEYLQAQVRSRSKLDAPKVDLLVKNCLLPLREYFKYFSQNSLPLGGPSSGAPPPSGGSPAGSPTSTEEGTSESATPESGPGTSTEPSEGSAPGSPAGSPTSTEEGTSTEPSEGSAPGTSTEPSEGPDIVMTQSPSSLSASVGDRVTITCRSSTGAVTTSNYASWVQEKPGKLFKGLIGGTNNRAPGVPSRFSGSLIGDKATLTISSLQPEDFATYFCALWYSNHWVFGQGTKVELKRGGGGSGGGGSGGGGSSGGGSEVKLLESGGGLVQPGGSLKLSCAVSGFSLTDYGVNWVRQAPGRGLEWIGVIWGDGITDYNSALKDRFIISKDNGKNTVYLQMSKVRSDDTALYYCVTGLFDYWGQGTLVTVSSYPYDVPDYAGGGGGSGGGGSGGGGSGGGGSGSGATNFSLLKQAGDVEENPGPMPAAKRVKLDGSEELLSKNYHLENEVARLKKGSGSGGSGSGGSGSGSGGSGSGGSGSGEELLSKNYHLENEVARLKKGSGSGGSGSGGSGSGSGGSGSGGSGSGPKKKRKVMDKKYSIGLAIGTNSVGWAVITDEYKVPSKKFKVLGNTDRHSIKKNLIGALLFDSGETAEATRLKRTARRRYTRRKNRICYLQEIFSNEMAKVDDSFFHRLEESFLVEEDKKHERHPIFGNIVDEVAYHEKYPTIYHLRKKLVDSTDKADLRLIYLALAHMIKFRGHFLIEGDLNPDNSDVDKLFIQLVQTYNQLFEENPINASGVDAKAILSARLSKSRRLENLIAQLPGEKKNGLFGNLIALSLGLTPNFKSNFDLAEDAKLQLSKDTYDDDLDNLLAQIGDQYADLFLAAKNLSDAILLSDILRVNTEITKAPLSASMIKRYDEHHQDLTLLKALVRQQLPEKYKEIFFDQSKNGYAGYIDGGASQEEFYKFIKPILEKMDGTEELLVKLNREDLLRKQRTFDNGSIPHQIHLGELHAILRRQEDFYPFLKDNREKIEKILTFRIPYYVGPLARGNSRFAWMTRKSEETITPWNFEEVVDKGASAQSFIERMTNFDKNLPNEKVLPKHSLLYEYFTVYNELTKVKYVTEGMRKPAFLSGEQKKAIVDLLFKTNRKVTVKQLKEDYFKKIECFDSVEISGVEDRFNASLGTYHDLLKIIKDKDFLDNEENEDILEDIVLTLTLFEDREMIEERLKTYAHLFDDKVMKQLKRRRYTGWGRLSRKLINGIRDKQSGKTILDFLKSDGFANRNFMQLIHDDSLTFKEDIQKAQVSGQGDSLHEHIANLAGSPAIKKGILQTVKVVDELVKVMGRHKPENIVIEMARENQTTQKGQKNSRERMKRIEEGIKELGSQILKEHPVENTQLQNEKLYLYYLQNGRDMYVDQELDINRLSDYDVDAIVPQSFLKDDSIDNKVLTRSDKNRGKSDNVPSEEVVKKMKNYWRQLLNAKLITQRKFDNLTKAERGGLSELDKAGFIKRQLVETRQITKHVAQILDSRMNTKYDENDKLIREVKVITLKSKLVSDFRKDFQFYKVREINNYHHAHDAYLNAVVGTALIKKYPKLESEFVYGDYKVYDVRKMIAKSEQEIGKATAKYFFYSNIMNFFKTEITLANGEIRKRPLIETNGETGEIVWDKGRDFATVRKVLSMPQVNIVKKTEVQTGGFSKESILPKRNSDKLIARKKDWDPKKYGGFDSPTVAYSVLVVAKVEKGKSKKLKSVKELLGITIMERSSFEKNPIDFLEAKGYKEVKKDLIIKLPKYSLFELENGRKRMLASAGELQKGNELALPSKYVNFLYLASHYEKLKGSPEDNEQKQLFVEQHKHYLDEIIEQISEFSKRVILADANLDKVLSAYNKHRDKPIREQAENIIHLFTLTNLGAPAAFKYFDTTIDRKRYTSTKEVLDATLIHQSITGLYETRIDLSQLGGDAYPYDVPDYASLGSGSPKKKRKVEDPKKKRKVDGSGSETPGTSESATPESRTLVTFKDVFVDFTREEWKLLDTAQQIVYRNVMLENYKNLVSLGYQLTKPDVILRLEKGEEPX

SEQ ID NO: 145 - protein, 2571 aa, synthetic construct
  REGION 1..2571: note = V24_D3a-D3l-scFv-2a-3xGCN4-dCas9-KRAB
  SITE 2571: note = misc_feature - Xaa =
MPAAKRVKLDGSNHDQEFDPPKVYPPVPAEKRKPIRVLSLFDGIATGLLVLKDLGIQVDRYIASEVCEDSITVGMVRHQGKIMYVGDVRSVTQKHIQEWGPFDLVIGGSPCNDLSIVNPARKGLYEGTGRLFFEFYRLLHDARPKEGDDRPFFWLFENVVAMGVSDKRDISRFLESNPVMIDAKEVSAAHRARYFWGNLPGMNRPLASTVNDKLELQECLEHGRIAKFSKVRTITTRSNSIKQGKDQHFPVFMNEKEDILWCTEMERVFGFPVHYTDVSNMSRLARQRLLGRSWSVPVIRHLFAPLKEYFACVSSGNSNANSRGPSFSSGLVPLSLRGSHMGPMEIYKTVSAWKRQPVRVLSLFRNIDKVLKSLGFLESGSGSGGGTLKYVEDVTNVVRRDVEKWGPFDLVYGSTQPLGSSCDRCPGWYMFQFHRILQYALPRQESQRPFFWIFMDNLLLTEDDQETTTRFLQTEAVTLQDVRGRDYQNAMRVWSNIPGLKSKHAPLTPKEEEYLQAQVRSRSKLDAPKVDLLVKNCLLPLREYFKYFSQNSLPLGGPSSGAPPPSGGSPAGSPTSTEEGTSESATPESGPGTSTEPSEGSAPGSPAGSPTSTEEGTSTEPSEGSAPGTSTEPSEGPDIVMTQSPSSLSASVGDRVTITCRSSTGAVTTSNYASWVQEKPGKLFKGLIGGTNNRAPGVPSRFSGSLIGDKATLTISSLQPEDFATYFCALWYSNHWVFGQGTKVELKRGGGGSGGGGSGGGGSSGGGSEVKLLESGGGLVQPGGSLKLSCAVSGFSLTDYGVNWVRQAPGRGLEWIGVIWGDGITDYNSALKDRFIISKDNGKNTVYLQMSKVRSDDTALYYCVTGLFDYWGQGTLVTVSSYPYDVPDYAGGGGGSGGGGSGGGGSGGGGSGSGATNFSLLKQAGDVEENPGPMPAAKRVKLDGSEELLSKNYHLENEVARLKKGSGSGGSGSGGSGSGSGGSGSGGSGSGEELLSKNYHLENEVARLKKGSGSGGSGSGGSGSGSGGSGSGGSGSGEELLSKNYHLENEVARLKKGSGSGGSGSGGSGSGSGGSGSGGSGSGPKKKRKVMDKKYSIGLAIGTNSVGWAVITDEYKVPSKKFKVLGNTDRHSIKKNLIGALLFDSGETAEATRLKRTARRRYTRRKNRICYLQEIFSNEMAKVDDSFFHRLEESFLVEEDKKHERHPIFGNIVDEVAYHEKYPTIYHLRKKLVDSTDKADLRLIYLALAHMIKFRGHFLIEGDLNPDNSDVDKLFIQLVQTYNQLFEENPINASGVDAKAILSARLSKSRRLENLIAQLPGEKKNGLFGNLIALSLGLTPNFKSNFDLAEDAKLQLSKDTYDDDLDNLLAQIGDQYADLFLAAKNLSDAILLSDILRVNTEITKAPLSASMIKRYDEHHQDLTLLKALVRQQLPEKYKEIFFDQSKNGYAGYIDGGASQEEFYKFIKPILEKMDGTEELLVKLNREDLLRKQRTFDNGSIPHQIHLGELHAILRRQEDFYPFLKDNREKIEKILTFRIPYYVGPLARGNSRFAWMTRKSEETITPWNFEEVVDKGASAQSFIERMTNFDKNLPNEKVLPKHSLLYEYFTVYNELTKVKYVTEGMRKPAFLSGEQKKAIVDLLFKTNRKVTVKQLKEDYFKKIECFDSVEISGVEDRFNASLGTYHDLLKIIKDKDFLDNEENEDILEDIVLTLTLFEDREMIEERLKTYAHLFDDKVMKQLKRRRYTGWGRLSRKLINGIRDKQSGKTILDFLKSDGFANRNFMQLIHDDSLTFKEDIQKAQVSGQGDSLHEHIANLAGSPAIKKGILQTVKVVDELVKVMGRHKPENIVIEMARENQTTQKGQKNSRERMKRIEEGIKELGSQILKEHPVENTQLQNEKLYLYYLQNGRDMYVDQELDINRLSDYDVDAIVPQSFLKDDSIDNKVLTRSDKNRGKSDNVPSEEVVKKMKNYWRQLLNAKLITQRKFDNLTKAERGGLSELDKAGFIKRQLVETRQITKHVAQILDSRMNTKYDENDKLIREVKVITLKSKLVSDFRKDFQFYKVREINNYHHAHDAYLNAVVGTALIKKYPKLESEFVYGDYKVYDVRKMIAKSEQEIGKATAKYFFYSNIMNFFKTEITLANGEIRKRPLIETNGETGEIVWDKGRDFATVRKVLSMPQVNIVKKTEVQTGGFSKESILPKRNSDKLIARKKDWDPKKYGGFDSPTVAYSVLVVAKVEKGKSKKLKSVKELLGITIMERSSFEKNPIDFLEAKGYKEVKKDLIIKLPKYSLFELENGRKRMLASAGELQKGNELALPSKYVNFLYLASHYEKLKGSPEDNEQKQLFVEQHKHYLDEIIEQISEFSKRVILADANLDKVLSAYNKHRDKPIREQAENIIHLFTLTNLGAPAAFKYFDTTIDRKRYTSTKEVLDATLIHQSITGLYETRIDLSQLGGDAYPYDVPDYASLGSGSPKKKRKVEDPKKKRKVDGSGSETPGTSESATPESRTLVTFKDVFVDFTREEWKLLDTAQQIVYRNVMLENYKNLVSLGYQLTKPDVILRLEKGEEPX

SEQ ID NO: 146 - protein, 2663 aa, synthetic construct
  REGION 1..2663: note = V25_D3a-D3l-scFv-2a-5xGCN4-dCas9-KRAB
  SITE 2663: note = misc_feature - Xaa =
MPAAKRVKLDGSNHDQEFDPPKVYPPVPAEKRKPIRVLSLFDGIATGLLVLKDLGIQVDRYIASEVCEDSITVGMVRHQGKIMYVGDVRSVTQKHIQEWGPFDLVIGGSPCNDLSIVNPARKGLYEGTGRLFFEFYRLLHDARPKEGDDRPFFWLFENVVAMGVSDKRDISRFLESNPVMIDAKEVSAAHRARYFWGNLPGMNRPLASTVNDKLELQECLEHGRIAKFSKVRTITTRSNSIKQGKDQHFPVFMNEKEDILWCTEMERVFGFPVHYTDVSNMSRLARQRLLGRSWSVPVIRHLFAPLKEYFACVSSGNSNANSRGPSFSSGLVPLSLRGSHMGPMEIYKTVSAWKRQPVRVLSLFRNIDKVLKSLGFLESGSGSGGGTLKYVEDVTNVVRRDVEKWGPFDLVYGSTQPLGSSCDRCPGWYMFQFHRILQYALPRQESQRPFFWIFMDNLLLTEDDQETTTRFLQTEAVTLQDVRGRDYQNAMRVWSNIPGLKSKHAPLTPKEEEYLQAQVRSRSKLDAPKVDLLVKNCLLPLREYFKYFSQNSLPLGGPSSGAPPPSGGSPAGSPTSTEEGTSESATPESGPGTSTEPSEGSAPGSPAGSPTSTEEGTSTEPSEGSAPGTSTEPSEGPDIVMTQSPSSLSASVGDRVTITCRSSTGAVTTSNYASWVQEKPGKLFKGLIGGTNNRAPGVPSRFSGSLIGDKATLTISSLQPEDFATYFCALWYSNHWVFGQGTKVELKRGGGGSGGGGSGGGGSSGGGSEVKLLESGGGLVQPGGSLKLSCAVSGFSLTDYGVNWVRQAPGRGLEWIGVIWGDGITDYNSALKDRFIISKDNGKNTVYLQMSKVRSDDTALYYCVTGLFDYWGQGTLVTVSSYPYDVPDYAGGGGGSGGGGSGGGGSGGGGSGSGATNFSLLKQAGDVEENPGPMPAAKRVKLDGSEELLSKNYHLENEVARLKKGSGSGGSGSGGSGSGSGGSGSGGSGSGEELLSKNYHLENEVARLKKGSGSGGSGSGGSGSGSGGSGSGGSGSGEELLSKNYHLENEVARLKKGSGSGGSGSGGSGSGSGGSGSGGSGSGEELLSKNYHLENEVARLKKGSGSGGSGSGGSGSGSGGSGSGGSGSGEELLSKNYHLENEVARLKKGSGSGGSGSGGSGSGSGGSGSGGSGSGPKKKRKVMDKKYSIGLAIGTNSVGWAVITDEYKVPSKKFKVLGNTDRHSIKKNLIGALLFDSGETAEATRLKRTARRRYTRRKNRICYLQEIFSNEMAKVDDSFFHRLEESFLVEEDKKHERHPIFGNIVDEVAYHEKYPTIYHLRKKLVDSTDKADLRLIYLALAHMIKFRGHFLIEGDLNPDNSDVDKLFIQLVQTYNQLFEENPINASGVDAKAILSARLSKSRRLENLIAQLPGEKKNGLFGNLIALSLGLTPNFKSNFDLAEDAKLQLSKDTYDDDLDNLLAQIGDQYADLFLAAKNLSDAILLSDILRVNTEITKAPLSASMIKRYDEHHQDLTLLKALVRQQLPEKYKEIFFDQSKNGYAGYIDGGASQEEFYKFIKPILEKMDGTEELLVKLNREDLLRKQRTFDNGSIPHQIHLGELHAILRRQEDFYPFLKDNREKIEKILTFRIPYYVGPLARGNSRFAWMTRKSEETITPWNFEEVVDKGASAQSFIERMTNFDKNLPNEKVLPKHSLLYEYFTVYNELTKVKYVTEGMRKPAFLSGEQKKAIVDLLFKTNRKVTVKQLKEDYFKKIECFDSVEISGVEDRFNASLGTYHDLLKIIKDKDFLDNEENEDILEDIVLTLTLFEDREMIEERLKTYAHLFDDKVMKQLKRRRYTGWGRLSRKLINGIRDKQSGKTILDFLKSDGFANRNFMQLIHDDSLTFKEDIQKAQVSGQGDSLHEHIANLAGSPAIKKGILQTVKVVDELVKVMGRHKPENIVIEMARENQTTQKGQKNSRERMKRIEEGIKELGSQILKEHPVENTQLQNEKLYLYYLQNGRDMYVDQELDINRLSDYDVDAIVPQSFLKDDSIDNKVLTRSDKNRGKSDNVPSEEVVKKMKNYWRQLLNAKLITQRKFDNLTKAERGGLSELDKAGFIKRQLVETRQITKHVAQILDSRMNTKYDENDKLIREVKVITLKSKLVSDFRKDFQFYKVREINNYHHAHDAYLNAVVGTALIKKYPKLESEFVYGDYKVYDVRKMIAKSEQEIGKATAKYFFYSNIMNFFKTEITLANGEIRKRPLIETNGETGEIVWDKGRDFATVRKVLSMPQVNIVKKTEVQTGGFSKESILPKRNSDKLIARKKDWDPKKYGGFDSPTVAYSVLVVAKVEKGKSKKLKSVKELLGITIMERSSFEKNPIDFLEAKGYKEVKKDLIIKLPKYSLFELENGRKRMLASAGELQKGNELALPSKYVNFLYLASHYEKLKGSPEDNEQKQLFVEQHKHYLDEIIEQISEFSKRVILADANLDKVLSAYNKHRDKPIREQAENIIHLFTLTNLGAPAAFKYFDTTIDRKRYTSTKEVLDATLIHQSITGLYETRIDLSQLGGDAYPYDVPDYASLGSGSPKKKRKVEDPKKKRKVDGSGSETPGTSESATPESRTLVTFKDVFVDFTREEWKLLDTAQQIVYRNVMLENYKNLVSLGYQLTKPDVILRLEKGEEPX

SEQ ID NO: 147 - protein, 2609 aa, synthetic construct
  REGION 1..2609: note = V26_D3a-hD3L-scFv-2a-3xGCN4-dCas9-ZIM3
  SITE 2609: note = misc_feature - Xaa =
MPAAKRVKLDGSNHDQEFDPPKVYPPVPAEKRKPIRVLSLFDGIATGLLVLKDLGIQVDRYIASEVCEDSITVGMVRHQGKIMYVGDVRSVTQKHIQEWGPFDLVIGGSPCNDLSIVNPARKGLYEGTGRLFFEFYRLLHDARPKEGDDRPFFWLFENVVAMGVSDKRDISRFLESNPVMIDAKEVSAAHRARYFWGNLPGMNRPLASTVNDKLELQECLEHGRIAKFSKVRTITTRSNSIKQGKDQHFPVFMNEKEDILWCTEMERVFGFPVHYTDVSNMSRLARQRLLGRSWSVPVIRHLFAPLKEYFACVSSGNSNANSRGPSFSSGLVPLSLRGSHMFETVPVWRRQPVRVLSLFEDIKKELTSLGFLESGSDPGQLKHVVDVTDTVRKDVEEWGPFDLVYGATPPLGHTCDRPPSWYLFQFHRLLQYARPKPGSPRPFFWMFVDNLVLNKEDLDVASRFLEMEPVTIPDVHGGSLQNAVRVWSNIPAIRSSRHWALVSEEELSLLAQNKQSSKLAAKWPTKLVKNCFLPLREYFKYFSGGPSSGAPPPSGGSPAGSPTSTEEGTSESATPESGPGTSTEPSEGSAPGSPAGSPTSTEEGTSTEPSEGSAPGTSTEPSEPKKKRKVPSEGPDIVMTQSPSSLSASVGDRVTITCRSSTGAVTTSNYASWVQEKPGKLFKGLIGGTNNRAPGVPSRFSGSLIGDKATLTISSLQPEDFATYFCALWYSNHWVFGQGTKVELKRGGGGSGGGGSGGGGSSGGGSEVKLLESGGGLVQPGGSLKLSCAVSGFSLTDYGVNWVRQAPGRGLEWIGVIWGDGITDYNSALKDRFIISKDNGKNTVYLQMSKVRSDDTALYYCVTGLFDYWGQGTLVTVSSYPYDVPDYAGGGGGSGGGGSGGGGSGGGGSGSGATNFSLLKQAGDVEENPGPMPAAKRVKLDGSEELLSKNYHLENEVARLKKGSGSGGSGSGGSGSGSGGSGSGGSGSGEELLSKNYHLENEVARLKKGSGSGGSGSGGSGSGSGGSGSGGSGSGEELLSKNYHLENEVARLKKGSGSGGSGSGGSGSGSGGSGSGGSGSGPKKKRKVMDKKYSIGLAIGTNSVGWAVITDEYKVPSKKFKVLGNTDRHSIKKNLIGALLFDSGETAEATRLKRTARRRYTRRKNRICYLQEIFSNEMAKVDDSFFHRLEESFLVEEDKKHERHPIFGNIVDEVAYHEKYPTIYHLRKKLVDSTDKADLRLIYLALAHMIKFRGHFLIEGDLNPDNSDVDKLFIQLVQTYNQLFEENPINASGVDAKAILSARLSKSRRLENLIAQLPGEKKNGLFGNLIALSLGLTPNFKSNFDLAEDAKLQLSKDTYDDDLDNLLAQIGDQYADLFLAAKNLSDAILLSDILRVNTEITKAPLSASMIKRYDEHHQDLTLLKALVRQQLPEKYKEIFFDQSKNGYAGYIDGGASQEEFYKFIKPILEKMDGTEELLVKLNREDLLRKQRTFDNGSIPHQIHLGELHAILRRQEDFYPFLKDNREKIEKILTFRIPYYVGPLARGNSRFAWMTRKSEETITPWNFEEVVDKGASAQSFIERMTNFDKNLPNEKVLPKHSLLYEYFTVYNELTKVKYVTEGMRKPAFLSGEQKKAIVDLLFKTNRKVTVKQLKEDYFKKIECFDSVEISGVEDRFNASLGTYHDLLKIIKDKDFLDNEENEDILEDIVLTLTLFEDREMIEERLKTYAHLFDDKVMKQLKRRRYTGWGRLSRKLINGIRDKQSGKTILDFLKSDGFANRNFMQLIHDDSLTFKEDIQKAQVSGQGDSLHEHIANLAGSPAIKKGILQTVKVVDELVKVMGRHKPENIVIEMARENQTTQKGQKNSRERMKRIEEGIKELGSQILKEHPVENTQLQNEKLYLYYLQNGRDMYVDQELDINRLSDYDVDAIVPQSFLKDDSIDNKVLTRSDKNRGKSDNVPSEEVVKKMKNYWRQLLNAKLITQRKFDNLTKAERGGLSELDKAGFIKRQLVETRQITKHVAQILDSRMNTKYDENDKLIREVKVITLKSKLVSDFRKDFQFYKVREINNYHHAHDAYLNAVVGTALIKKYPKLESEFVYGDYKVYDVRKMIAKSEQEIGKATAKYFFYSNIMNFFKTEITLANGEIRKRPLIETNGETGEIVWDKGRDFATVRKVLSMPQVNIVKKTEVQTGGFSKESILPKRNSDKLIARKKDWDPKKYGGFDSPTVAYSVLVVAKVEKGKSKKLKSVKELLGITIMERSSFEKNPIDFLEAKGYKEVKKDLIIKLPKYSLFELENGRKRMLASAGELQKGNELALPSKYVNFLYLASHYEKLKGSPEDNEQKQLFVEQHKHYLDEIIEQISEFSKRVILADANLDKVLSAYNKHRDKPIREQAENIIHLFTLTNLGAPAAFKYFDTTIDRKRYTSTKEVLDATLIHQSITGLYETRIDLSQLGGDAYPYDVPDYASLGSGSPKKKRKVEDPKKKRKVDGSGSETPGTSESATPESMNNSQGRVTFEDVTVNFTQGEWQRLNPEQRNLYRDVMLENYSNLVSVGQGETTKPDVILRLEQGKEPWLEEEEVLGSGRAEKNGDIGGQIWKPKDVKESLLEX

SEQ ID NO: 148 - protein, 2609 aa, synthetic construct
  REGION 1..2609: note = V27_3xGCN4-dCas9-ZIM3-2a-D3a-hD3L-scFv
  SITE 2609: note = misc_feature - Xaa =
MPAAKRVKLDGSEELLSKNYHLENEVARLKKGSGSGGSGSGGSGSGSGGSGSGGSGSGEELLSKNYHLENEVARLKKGSGSGGSGSGGSGSGSGGSGSGGSGSGEELLSKNYHLENEVARLKKGSGSGGSGSGGSGSGSGGSGSGGSGSGPKKKRKVMDKKYSIGLAIGTNSVGWAVITDEYKVPSKKFKVLGNTDRHSIKKNLIGALLFDSGETAEATRLKRTARRRYTRRKNRICYLQEIFSNEMAKVDDSFFHRLEESFLVEEDKKHERHPIFGNIVDEVAYHEKYPTIYHLRKKLVDSTDKADLRLIYLALAHMIKFRGHFLIEGDLNPDNSDVDKLFIQLVQTYNQLFEENPINASGVDAKAILSARLSKSRRLENLIAQLPGEKKNGLFGNLIALSLGLTPNFKSNFDLAEDAKLQLSKDTYDDDLDNLLAQIGDQYADLFLAAKNLSDAILLSDILRVNTEITKAPLSASMIKRYDEHHQDLTLLKALVRQQLPEKYKEIFFDQSKNGYAGYIDGGASQEEFYKFIKPILEKMDGTEELLVKLNREDLLRKQRTFDNGSIPHQIHLGELHAILRRQEDFYPFLKDNREKIEKILTFRIPYYVGPLARGNSRFAWMTRKSEETITPWNFEEVVDKGASAQSFIERMTNFDKNLPNEKVLPKHSLLYEYFTVYNELTKVKYVTEGMRKPAFLSGEQKKAIVDLLFKTNRKVTVKQLKEDYFKKIECFDSVEISGVEDRFNASLGTYHDLLKIIKDKDFLDNEENEDILEDIVLTLTLFEDREMIEERLKTYAHLFDDKVMKQLKRRRYTGWGRLSRKLINGIRDKQSGKTILDFLKSDGFANRNFMQLIHDDSLTFKEDIQKAQVSGQGDSLHEHIANLAGSPAIKKGILQTVKVVDELVKVMGRHKPENIVIEMARENQTTQKGQKNSRERMKRIEEGIKELGSQILKEHPVENTQLQNEKLYLYYLQNGRDMYVDQELDINRLSDYDVDAIVPQSFLKDDSIDNKVLTRSDKNRGKSDNVPSEEVVKKMKNYWRQLLNAKLITQRKFDNLTKAERGGLSELDKAGFIKRQLVETRQITKHVAQILDSRMNTKYDENDKLIREVKVITLKSKLVSDFRKDFQFYKVREINNYHHAHDAYLNAVVGTALIKKYPKLESEFVYGDYKVYDVRKMIAKSEQEIGKATAKYFFYSNIMNFFKTEITLANGEIRKRPLIETNGETGEIVWDKGRDFATVRKVLSMPQVNIVKKTEVQTGGFSKESILPKRNSDKLIARKKDWDPKKYGGFDSPTVAYSVLVVAKVEKGKSKKLKSVKELLGITIMERSSFEKNPIDFLEAKGYKEVKKDLIIKLPKYSLFELENGRKRMLASAGELQKGNELALPSKYVNFLYLASHYEKLKGSPEDNEQKQLFVEQHKHYLDEIIEQISEFSKRVILADANLDKVLSAYNKHRDKPIREQAENIIHLFTLTNLGAPAAFKYFDTTIDRKRYTSTKEVLDATLIHQSITGLYETRIDLSQLGGDAYPYDVPDYASLGSGSPKKKRKVEDPKKKRKVDGSGSETPGTSESATPESMNNSQGRVTFEDVTVNFTQGEWQRLNPEQRNLYRDVMLENYSNLVSVGQGETTKPDVILRLEQGKEPWLEEEEVLGSGRAEKNGDIGGQIWKPKDVKESLLEGSGATNFSLLKQAGDVEENPGPMPAAKRVKLDGSNHDQEFDPPKVYPPVPAEKRKPIRVLSLFDGIATGLLVLKDLGIQVDRYIASEVCEDSITVGMVRHQGKIMYVGDVRSVTQKHIQEWGPFDLVIGGSPCNDLSIVNPARKGLYEGTGRLFFEFYRLLHDARPKEGDDRPFFWLFENVVAMGVSDKRDISRFLESNPVMIDAKEVSAAHRARYFWGNLPGMNRPLASTVNDKLELQECLEHGRIAKFSKVRTITTRSNSIKQGKDQHFPVFMNEKEDILWCTEMERVFGFPVHYTDVSNMSRLARQRLLGRSWSVPVIRHLFAPLKEYFACVSSGNSNANSRGPSFSSGLVPLSLRGSHMFETVPVWRRQPVRVLSLFEDIKKELTSLGFLESGSDPGQLKHVVDVTDTVRKDVEEWGPFDLVYGATPPLGHTCDRPPSWYLFQFHRLLQYARPKPGSPRPFFWMFVDNLVLNKEDLDVASRFLEMEPVTIPDVHGGSLQNAVRVWSNIPAIRSSRHWALVSEEELSLLAQNKQSSKLAAKWPTKLVKNCFLPLREYFKYFSGGPSSGAPPPSGGSPAGSPTSTEEGTSESATPESGPGTSTEPSEGSAPGSPAGSPTSTEEGTSTEPSEGSAPGTSTEPSEPKKKRKVPSEGPDIVMTQSPSSLSASVGDRVTITCRSSTGAVTTSNYASWVQEKPGKLFKGLIGGTNNRAPGVPSRFSGSLIGDKATLTISSLQPEDFATYFCALWYSNHWVFGQGTKVELKRGGGGSGGGGSGGGGSSGGGSEVKLLESGGGLVQPGGSLKLSCAVSGFSLTDYGVNWVRQAPGRGLEWIGVIWGDGITDYNSALKDRFIISKDNGKNTVYLQMSKVRSDDTALYYCVTGLFDYWGQGTLVTVSSYPYDVPDYAGGGGGSGGGGSGGGGSGGGGSX

SEQ ID NO: 149 - protein, 2469 aa, synthetic construct
  REGION 1..2469: note = V28_3xGCN4-dCas12a-ZIM3-2a-D3a-hD3L-scFv
  SITE 2469: note = misc_feature - Xaa =
MPAAKRVKLDGSEELLSKNYHLENEVARLKKGSGSGGSGSGGSGSGSGGSGSGGSGSGEELLSKNYHLENEVARLKKGSGSGGSGSGGSGSGSGGSGSGGSGSGEELLSKNYHLENEVARLKKGSGSGGSGSGGSGSGSGGSGSGGSGSGPKKKRKVMSKLEKFTNCYSLSKTLRFKAIPVGKTQENIDNKRLLVEDEKRAEDYKGVKKLLDRYYLSFINDVLHSIKLKNLNNYISLFRKKTRTEKENKELENLEINLRKEIAKAFKGNEGYKSLFKKDIIETILPEFLDDKDEIALVNSFNGFTTAFTGFFDNRENMFSEEAKSTSIAFRCINENLTRYISNMDIFEKVDAIFDKHEVQEIKEKILNSDYDVEDFFEGEFFNFVLTQEGIDVYNAIIGGFVTESGEKIKGLNEYINLYNQKTKQKLPKFKPLYKQVLSDRESLSFYGEGYTSDEEVLEVFRNTLNKNSEIFSSIKKLEKLFKNFDEYSSAGIFVKNGPAISTISKDIFGEWNVIRDKWNAEYDDIHLKKKAVVTEKYEDDRRKSFKKIGSFSLEQLQEYADADLSVVEKLKEIIIQKVDEIYKVYGSSEKLFDADFVLEKSLKKNDAVVAIMKDLLDSVKSFENYIKAFFGEGKETNRDESFYGDFVLAYDILLKVDHIYDAIRNYVTQKPYSKDKFKLYFQNPQFMGGWDKDKETDYRATILRYGSKYYLAIMDKKYAKCLQKIDKDDVNGNYEKINYKLLPGPNKMLPKVFFSKKWMAYYNPSEDIQKIYKNGTFKKGDMFNLNDCHKLIDFFKDSISRYPKWSNAYDFNFSETEKYKDIAGFYREVEEQGYKVSFESASKKEVDKLVEEGKLYMFQIYNKDFSDKSHGTPNLHTMYFKLLFDENNHGQIRLSGGAELFMRRASLKKEELVVHPANSPIANKNPDNPKKTTTLSYDVYKDKRFSEDQYELHIPIAINKCPKNIFKINTEVRVLLKHDDNPYVIGIARGERNLLYIVVVDGKGNIVEQYSLNEIINNFNGIRIKTDYHSLLDKKEKERFEARQNWTSIENIKELKAGYISQVVHKICELVEKYDAVIALADLNSGFKNSRVKVEKQVYQKFEKMLIDKLNYMVDKKSNPCATGGALKGYQITNKFESFKSMSTQNGFIFYIPAWLTSKIDPSTGFVNLLKTKYTSIADSKKFISSFDRIMYVPEEDLFEFALDYKNFSRTDADYIKKWKLYSYGNRIRIFRNPKKNNVFDWEEVCLTSAYKELFNKYGINYQQGDIRALLCEQSDKAFYSSFMALMSLMLQMRNSITGRTDVAFLISPVKNSDGIFYDSRNYEAQENAILPKNADANGAYNIARKVLWAIGQFKKAEDEKLDKVKIAISNKEWLEYAQTSVKHAYPYDVPDYASLGSGSPKKKRKVEDPKKKRKVDGSGSETPGTSESATPESMNNSQGRVTFEDVTVNFTQGEWQRLNPEQRNLYRDVMLENYSNLVSVGQGETTKPDVILRLEQGKEPWLEEEEVLGSGRAEKNGDIGGQIWKPKDVKESLLEGSGATNFSLLKQAGDVEENPGPMPAAKRVKLDGSNHDQEFDPPKVYPPVPAEKRKPIRVLSLFDGIATGLLVLKDLGIQVDRYIASEVCEDSITVGMVRHQGKIMYVGDVRSVTQKHIQEWGPFDLVIGGSPCNDLSIVNPARKGLYEGTGRLFFEFYRLLHDARPKEGDDRPFFWLFENVVAMGVSDKRDISRFLESNPVMIDAKEVSAAHRARYFWGNLPGMNRPLASTVNDKLELQECLEHGRIAKFSKVRTITTRSNSIKQGKDQHFPVFMNEKEDILWCTEMERVFGFPVHYTDVSNMSRLARQRLLGRSWSVPVIRHLFAPLKEYFACVSSGNSNANSRGPSFSSGLVPLSLRGSHMFETVPVWRRQPVRVLSLFEDIKKELTSLGFLESGSDPGQLKHVVDVTDTVRKDVEEWGPFDLVYGATPPLGHTCDRPPSWYLFQFHRLLQYARPKPGSPRPFFWMFVDNLVLNKEDLDVASRFLEMEPVTIPDVHGGSLQNAVRVWSNIPAIRSSRHWALVSEEELSLLAQNKQSSKLAAKWPTKLVKNCFLPLREYFKYFSGGPSSGAPPPSGGSPAGSPTSTEEGTSESATPESGPGTSTEPSEGSAPGSPAGSPTSTEEGTSTEPSEGSAPGTSTEPSEPKKKRKVPSEGPDIVMTQSPSSLSASVGDRVTITCRSSTGAVTTSNYASWVQEKPGKLFKGLIGGTNNRAPGVPSRFSGSLIGDKATLTISSLQPEDFATYFCALWYSNHWVFGQGTKVELKRGGGGSGGGGSGGGGSSGGGSEVKLLESGGGLVQPGGSLKLSCAVSGFSLTDYGVNWVRQAPGRGLEWIGVIWGDGITDYNSALKDRFIISKDNGKNTVYLQMSKVRSDDTALYYCVTGLFDYWGQGTLVTVSSYPYDVPDYAGGGGGSGGGGSGGGGSGGGGSX

SEQ ID NO: 150 - protein, 2252 aa, synthetic construct
  REGION 1..2252: note = V29_3xGCN4-dCas12i-ZIM3-2a-D3a-hD3L-scFv
  SITE 2252: note = misc_feature - Xaa =
MPAAKRVKLDGSEELLSKNYHLENEVARLKKGSGSGGSGSGGSGSGSGGSGSGGSGSGEELLSKNYHLENEVARLKKGSGSGGSGSGGSGSGSGGSGSGGSGSGEELLSKNYHLENEVARLKKGSGSGGSGSGGSGSGSGGSGSGGSGSGPKKKRKVMGITMSDTTFRPYKSKLNPNERKMPMVVDTMNWCDNACSVFFDLFVGLYGGVKIGDVTNFLTEKQDTTTDADLLCAINWFRAMPVSNPDAVVGPEQLVVRFRDYSGHNPSPMASMYLSAPVNPRYTWVDCRFLYQQMCQTLGANLDVDISTLVQTGLLPIQKDTQLNAYSFCSNVFGEGVKEDPSAKVTSYTAAANALSGATNPIITYEDYRQILSSAITNRPSRKGAKDILAADLDSTKTGVLPGNYVSQRIAMYQASAASKARGVVLPNRLRVKAYLQNLVGLNYICTTWAAPMLRAVGDIKSKNSNNYRFVGERLERQQEIDNLLAVSNIRSAQAILQQFRANESNQFYIKKRHIGKGLPSLYDMWDLMDEKEGIDNYIQSLKGDKTERLPIRELLQIIYPHRKSVSAELFLSAAELTDVEDRQNRCMVHPTVRGSLVINFGKSSTIFGAITPPDTLIKFRGEMVPAGQTGMIWFTMHLVDGGKWVKHHIPCHSSRYFEEIYAWKKDLPTLPFPRRSLYGYAIGNKISDTRKIDLRRKKASKQYLRTLENMTHNVEFDPTTQFMVDQELNVTITARVKKIPPVRDVPVGSRIMGLNKNQTIRDCYSIWERVEANTSGSFQHPVVQDVWLRLVADGHVTSTVNGPNGQIDQMSYSGPDVANCGNWMQERSNFITSVDDADQSIMKHFLWNNRVKLYAWNCVYAGTLMKAISKQMTTANRNLFRNEILSFVGGRFGCRLGSLAQVSLDLLRRMKSVISCYFSRNNAFTIEERSAFDKELMELFESLDNKMNNKRKEKVNRTLSSIFQVAKQHNVVRLVVTKNLQTPDANVRSVMNQRSVDWCARKIEEKIVDLGNVIGIYVDLVEALDLSHLDPFIYIAKGDVGKECQFDEVESSSLLPIHTSMFRDWHGLVNKGRTTTPIYHSALRSFASHYGLRFDDLARIKAAELAKMLPDQKVFIPHRGGRFFMSTYPVTSTSRPVSYDGRQRFLNSGDMVAPVNTMLRGFRRARSAYPYDVPDYASLGSGSPKKKRKVEDPKKKRKVDGSGSETPGTSESATPESMNNSQGRVTFEDVTVNFTQGEWQRLNPEQRNLYRDVMLENYSNLVSVGQGETTKPDVILRLEQGKEPWLEEEEVLGSGRAEKNGDIGGQIWKPKDVKESLLEGSGATNFSLLKQAGDVEENPGPMPAAKRVKLDGSNHDQEFDPPKVYPPVPAEKRKPIRVLSLFDGIATGLLVLKDLGIQVDRYIASEVCEDSITVGMVRHQGKIMYVGDVRSVTQKHIQEWGPFDLVIGGSPCNDLSIVNPARKGLYEGTGRLFFEFYRLLHDARPKEGDDRPFFWLFENVVAMGVSDKRDISRFLESNPVMIDAKEVSAAHRARYFWGNLPGMNRPLASTVNDKLELQECLEHGRIAKFSKVRTITTRSNSIKQGKDQHFPVFMNEKEDILWCTEMERVFGFPVHYTDVSNMSRLARQRLLGRSWSVPVIRHLFAPLKEYFACVSSGNSNANSRGPSFSSGLVPLSLRGSHMFETVPVWRRQPVRVLSLFEDIKKELTSLGFLESGSDPGQLKHVVDVTDTVRKDVEEWGPFDLVYGATPPLGHTCDRPPSWYLFQFHRLLQYARPKPGSPRPFFWMFVDNLVLNKEDLDVASRFLEMEPVTIPDVHGGSLQNAVRVWSNIPAIRSSRHWALVSEEELSLLAQNKQSSKLAAKWPTKLVKNCFLPLREYFKYFSGGPSSGAPPPSGGSPAGSPTSTEEGTSESATPESGPGTSTEPSEGSAPGSPAGSPTSTEEGTSTEPSEGSAPGTSTEPSEPKKKRKVPSEGPDIVMTQSPSSLSASVGDRVTITCRSSTGAVTTSNYASWVQEKPGKLFKGLIGGTNNRAPGVPSRFSGSLIGDKATLTISSLQPEDFATYFCALWYSNHWVFGQGTKVELKRGGGGSGGGGSGGGGSSGGGSEVKLLESGGGLVQPGGSLKLSCAVSGFSLTDYGVNWVRQAPGRGLEWIGVIWGDGITDYNSALKDRFIISKDNGKNTVYLQMSKVRSDDTALYYCVTGLFDYWGQGTLVTVSSYPYDVPDYAGGGGGSGGGGSGGGGSGGGGSX

SEQ ID NO: 151 - protein, 2909 aa, synthetic construct
  REGION 1..2909: note = V30_10xGCN4-dCas9-ZIM3-2a-D3a-hD3L-scFv
  SITE 2909: note = misc_feature - Xaa =
MPAAKRVKLDGSEELLSKNYHLENEVARLKKGSGSGGSGSGGSGSGSGGSGSGGSGSGEELLSKNYHLENEVARLKKGSGSGGSGSGGSGSGSGGSGSGGSGSGEELLSKNYHLENEVARLKKGSGSGGSGSGGSGSGSGGSGSGGSGSGEELLSKNYHLENEVARLKKGSGSGGSGSGGSGSGSGGSGSGGSGSGEELLSKNYHLENEVARLKKGSGSGGSGSGGSGSGSGGSGSGGSGSGEELLSKNYHLENEVARLKKGSGSGGSGSGGSGSGSGGSGSGGSGSGEELLSKNYHLENEVARLKKGSGSGGSGSGGSGSGSGGSGSGGSGSGEELLSKNYHLENEVARLKKGSGSGGSGSGGSGSGSGGSGSGGSGSGEELLSKNYHLENEVARLKKGSGSGGSGSGGSGSGSGGSGSGGSGSGEELLSKNYHLENEVARLKKGSGSGPKKKRKVMDKKYSIGLAIGTNSVGWAVITDEYKVPSKKFKVLGNTDRHSIKKNLIGALLFDSGETAEATRLKRTARRRYTRRKNRICYLQEIFSNEMAKVDDSFFHRLEESFLVEEDKKHERHPIFGNIVDEVAYHEKYPTIYHLRKKLVDSTDKADLRLIYLALAHMIKFRGHFLIEGDLNPDNSDVDKLFIQLVQTYNQLFEENPINASGVDAKAILSARLSKSRRLENLIAQLPGEKKNGLFGNLIALSLGLTPNFKSNFDLAEDAKLQLSKDTYDDDLDNLLAQIGDQYADLFLAAKNLSDAILLSDILRVNTEITKAPLSASMIKRYDEHHQDLTLLKALVRQQLPEKYKEIFFDQSKNGYAGYIDGGASQEEFYKFIKPILEKMDGTEELLVKLNREDLLRKQRTFDNGSIPHQIHLGELHAILRRQEDFYPFLKDNREKIEKILTFRIPYYVGPLARGNSRFAWMTRKSEETITPWNFEEVVDKGASAQSFIERMTNFDKNLPNEKVLPKHSLLYEYFTVYNELTKVKYVTEGMRKPAFLSGEQKKAIVDLLFKTNRKVTVKQLKEDYFKKIECFDSVEISGVEDRFNASLGTYHDLLKIIKDKDFLDNEENEDILEDIVLTLTLFEDREMIEERLKTYAHLFDDKVMKQLKRRRYTGWGRLSRKLINGIRDKQSGKTILDFLKSDGFANRNFMQLIHDDSLTFKEDIQKAQVSGQGDSLHEHIANLAGSPAIKKGILQTVKVVDELVKVMGRHKPENIVIEMARENQTTQKGQKNSRERMKRIEEGIKELGSQILKEHPVENTQLQNEKLYLYYLQNGRDMYVDQELDINRLSDYDVDAIVPQSFLKDDSIDNKVLTRSDKNRGKSDNVPSEEVVKKMKNYWRQLLNAKLITQRKFDNLTKAERGGLSELDKAGFIKRQLVETRQITKHVAQILDSRMNTKYDENDKLIREVKVITLKSKLVSDFRKDFQFYKVREINNYHHAHDAYLNAVVGTALIKKYPKLESEFVYGDYKVYDVRKMIAKSEQEIGKATAKYFFYSNIMNFFKTEITLANGEIRKRPLIETNGETGEIVWDKGRDFATVRKVLSMPQVNIVKKTEVQTGGFSKESILPKRNSDKLIARKKDWDPKKYGGFDSPTVAYSVLVVAKVEKGKSKKLKSVKELLGITIMERSSFEKNPIDFLEAKGYKEVKKDLIIKLPKYSLFELENGRKRMLASAGELQKGNELALPSKYVNFLYLASHYEKLKGSPEDNEQKQLFVEQHKHYLDEIIEQISEFSKRVILADANLDKVLSAYNKHRDKPIREQAENIIHLFTLTNLGAPAAFKYFDTTIDRKRYTSTKEVLDATLIHQSITGLYETRIDLSQLGGDAYPYDVPDYASLGSGSPKKKRKVEDPKKKRKVDGSGSETPGTSESATPESMNNSQGRVTFEDVTVNFTQGEWQRLNPEQRNLYRDVMLENYSNLVSVGQGETTKPDVILRLEQGKEPWLEEEEVLGSGRAEKNGDIGGQIWKPKDVKESLLEGSGATNFSLLKQAGDVEENPGPMPAAKRVKLDGSNHDQEFDPPKVYPPVPAEKRKPIRVLSLFDGIATGLLVLKDLGIQVDRYIASEVCEDSITVGMVRHQGKIMYVGDVRSVTQKHIQEWGPFDLVIGGSPCNDLSIVNPARKGLYEGTGRLFFEFYRLLHDARPKEGDDRPFFWLFENVVAMGVSDKRDISRFLESNPVMIDAKEVSAAHRARYFWGNLPGMNRPLASTVNDKLELQECLEHGRIAKFSKVRTITTRSNSIKQGKDQHFPVFMNEKEDILWCTEMERVFGFPVHYTDVSNMSRLARQRLLGRSWSVPVIRHLFAPLKEYFACVSSGNSNANSRGPSFSSGLVPLSLRGSHMFETVPVWRRQPVRVLSLFEDIKKELTSLGFLESGSDPGQLKHVVDVTDTVRKDVEEWGPFDLVYGATPPLGHTCDRPPSWYLFQFHRLLQYARPKPGSPRPFFWMFVDNLVLNKEDLDVASRFLEMEPVTIPDVHGGSLQNAVRVWSNIPAIRSSRHWALVSEEELSLLAQNKQSSKLAAKWPTKLVKNCFLPLREYFKYFSGGPSSGAPPPSGGSPAGSPTSTEEGTSESATPESGPGTSTEPSEGSAPGSPAGSPTSTEEGTSTEPSEGSAPGTSTEPSEPKKKRKVPSEGPDIVMTQSPSSLSASVGDRVTITCRSSTGAVTTSNYASWVQEKPGKLFKGLIGGTNNRAPGVPSRFSGSLIGDKATLTISSLQPEDFATYFCALWYSNHWVFGQGTKVELKRGGGGSGGGGSGGGGSSGGGSEVKLLESGGGLVQPGGSLKLSCAVSGFSLTDYGVNWVRQAPGRGLEWIGVIWGDGITDYNSALKDRFIISKDNGKNTVYLQMSKVRSDDTALYYCVTGLFDYWGQGTLVTVSSYPYDVPDYAGGGGGSGGGGSGGGGSGGGGSX

SEQ ID NO: 152 - protein, 2487 aa, synthetic construct
  REGION 1..2487: note = V31_scFV-hD3L-D3a-2a-3xGCN4-dCas9-KRAB
  SITE 2487: note = misc_feature - Xaa =
MPAAKRVKLDGSGPDIVMTQSPSSLSASVGDRVTITCRSSTGAVTTSNYASWVQEKPGKLFKGLIGGTNNRAPGVPSRFSGSLIGDKATLTISSLQPEDFATYFCALWYSNHWVFGQGTKVELKRGGGGSGGGGSGGGGSSGGGSEVKLLESGGGLVQPGGSLKLSCAVSGFSLTDYGVNWVRQAPGRGLEWIGVIWGDGITDYNSALKDRFIISKDNGKNTVYLQMSKVRSDDTALYYCVTGLFDYWGQGTLVTVSSYPYDVPDYAGGGGGSGGGGSGGGGSGGGGSMFETVPVWRRQPVRVLSLFEDIKKELTSLGFLESGSDPGQLKHVVDVTDTVRKDVEEWGPFDLVYGATPPLGHTCDRPPSWYLFQFHRLLQYARPKPGSPRPFFWMFVDNLVLNKEDLDVASRFLEMEPVTIPDVHGGSLQNAVRVWSNIPAIRSSRHWALVSEEELSLLAQNKQSSKLAAKWPTKLVKNCFLPLREYFKYFSTELTSSLSSGNSNANSRGPSFSSGLVPLSLRGSHMNHDQEFDPPKVYPPVPAEKRKPIRVLSLFDGIATGLLVLKDLGIQVDRYIASEVCEDSITVGMVRHQGKIMYVGDVRSVTQKHIQEWGPFDLVIGGSPCNDLSIVNPARKGLYEGTGRLFFEFYRLLHDARPKEGDDRPFFWLFENVVAMGVSDKRDISRFLESNPVMIDAKEVSAAHRARYFWGNLPGMNRPLASTVNDKLELQECLEHGRIAKFSKVRTITTRSNSIKQGKDQHFPVFMNEKEDILWCTEMERVFGFPVHYTDVSNMSRLARQRLLGRSWSVPVIRHLFAPLKEYFACVGSGATNFSLLKQAGDVEENPGPMPAAKRVKLDGSEELLSKNYHLENEVARLKKGSGSGGSGSGGSGSGSGGSGSGGSGSGEELLSKNYHLENEVARLKKGSGSGGSGSGGSGSGSGGSGSGGSGSGEELLSKNYHLENEVARLKKGSGSGGSGSGGSGSGSGGSGSGGSGSGPKKKRKVMDKKYSIGLAIGTNSVGWAVITDEYKVPSKKFKVLGNTDRHSIKKNLIGALLFDSGETAEATRLKRTARRRYTRRKNRICYLQEIFSNEMAKVDDSFFHRLEESFLVEEDKKHERHPIFGNIVDEVAYHEKYPTIYHLRKKLVDSTDKADLRLIYLALAHMIKFRGHFLIEGDLNPDNSDVDKLFIQLVQTYNQLFEENPINASGVDAKAILSARLSKSRRLENLIAQLPGEKKNGLFGNLIALSLGLTPNFKSNFDLAEDAKLQLSKDTYDDDLDNLLAQIGDQYADLFLAAKNLSDAILLSDILRVNTEITKAPLSASMIKRYDEHHQDLTLLKALVRQQLPEKYKEIFFDQSKNGYAGYIDGGASQEEFYKFIKPILEKMDGTEELLVKLNREDLLRKQRTFDNGSIPHQIHLGELHAILRRQEDFYPFLKDNREKIEKILTFRIPYYVGPLARGNSRFAWMTRKSEETITPWNFEEVVDKGASAQSFIERMTNFDKNLPNEKVLPKHSLLYEYFTVYNELTKVKYVTEGMRKPAFLSGEQKKAIVDLLFKTNRKVTVKQLKEDYFKKIECFDSVEISGVEDRFNASLGTYHDLLKIIKDKDFLDNEENEDILEDIVLTLTLFEDREMIEERLKTYAHLFDDKVMKQLKRRRYTGWGRLSRKLINGIRDKQSGKTILDFLKSDGFANRNFMQLIHDDSLTFKEDIQKAQVSGQGDSLHEHIANLAGSPAIKKGILQTVKVVDELVKVMGRHKPENIVIEMARENQTTQKGQKNSRERMKRIEEGIKELGSQILKEHPVENTQLQNEKLYLYYLQNGRDMYVDQELDINRLSDYDVDAIVPQSFLKDDSIDNKVLTRSDKNRGKSDNVPSEEVVKKMKNYWRQLLNAKLITQRKFDNLTKAERGGLSELDKAGFIKRQLVETRQITKHVAQILDSRMNTKYDENDKLIREVKVITLKSKLVSDFRKDFQFYKVREINNYHHAHDAYLNAVVGTALIKKYPKLESEFVYGDYKVYDVRKMIAKSEQEIGKATAKYFFYSNIMNFFKTEITLANGEIRKRPLIETNGETGEIVWDKGRDFATVRKVLSMPQVNIVKKTEVQTGGFSKESILPKRNSDKLIARKKDWDPKKYGGFDSPTVAYSVLVVAKVEKGKSKKLKSVKELLGITIMERSSFEKNPIDFLEAKGYKEVKKDLIIKLPKYSLFELENGRKRMLASAGELQKGNELALPSKYVNFLYLASHYEKLKGSPEDNEQKQLFVEQHKHYLDEIIEQISEFSKRVILADANLDKVLSAYNKHRDKPIREQAENIIHLFTLTNLGAPAAFKYFDTTIDRKRYTSTKEVLDATLIHQSITGLYETRIDLSQLGGDAYPYDVPDYASLGSGSPKKKRKVEDPKKKRKVDGSGSETPGTSESATPESRTLVTFKDVFVDFTREEWKLLDTAQQIVYRNVMLENYKNLVSLGYQLTKPDVILRLEKGEEPX

SEQ ID NO: 153 - protein, 2494 aa, synthetic construct
  REGION 1..2494: note = V32_1xGCN4-ZIM3-2a-D3a-hD3L-dCas9-scFv
  SITE 2494: note = misc_feature - Xaa =
MPAAKRVKLDGSEELLSKNYHLENEVARLKKGSGSGGSGSGGSGSGSGGSGSGGSGSGMNNSQGRVTFEDVTVNFTQGEWQRLNPEQRNLYRDVMLENYSNLVSVGQGETTKPDVILRLEQGKEPWLEEEEVLGSGRAEKNGDIGGQIWKPKDVKESLGSGATNFSLLKQAGDVEENPGPMPAAKRVKLDGSNHDQEFDPPKVYPPVPAEKRKPIRVLSLFDGIATGLLVLKDLGIQVDRYIASEVCEDSITVGMVRHQGKIMYVGDVRSVTQKHIQEWGPFDLVIGGSPCNDLSIVNPARKGLYEGTGRLFFEFYRLLHDARPKEGDDRPFFWLFENVVAMGVSDKRDISRFLESNPVMIDAKEVSAAHRARYFWGNLPGMNRPLASTVNDKLELQECLEHGRIAKFSKVRTITTRSNSIKQGKDQHFPVFMNEKEDILWCTEMERVFGFPVHYTDVSNMSRLARQRLLGRSWSVPVIRHLFAPLKEYFACVSSGNSNANSRGPSFSSGLVPLSLRGSHMFETVPVWRRQPVRVLSLFEDIKKELTSLGFLESGSDPGQLKHVVDVTDTVRKDVEEWGPFDLVYGATPPLGHTCDRPPSWYLFQFHRLLQYARPKPGSPRPFFWMFVDNLVLNKEDLDVASRFLEMEPVTIPDVHGGSLQNAVRVWSNIPAIRSSRHWALVSEEELSLLAQNKQSSKLAAKWPTKLVKNCFLPLREYFKYFSGGPSSGAPPPSGGSPAGSPTSTEEGTSESATPESGPGTSTEPSEGSAPGSPAGSPTSTEEGTSTEPSEGSAPGTSTEPSEPKKKRKVMDKKYSIGLAIGTNSVGWAVITDEYKVPSKKFKVLGNTDRHSIKKNLIGALLFDSGETAEATRLKRTARRRYTRRKNRICYLQEIFSNEMAKVDDSFFHRLEESFLVEEDKKHERHPIFGNIVDEVAYHEKYPTIYHLRKKLVDSTDKADLRLIYLALAHMIKFRGHFLIEGDLNPDNSDVDKLFIQLVQTYNQLFEENPINASGVDAKAILSARLSKSRRLENLIAQLPGEKKNGLFGNLIALSLGLTPNFKSNFDLAEDAKLQLSKDTYDDDLDNLLAQIGDQYADLFLAAKNLSDAILLSDILRVNTEITKAPLSASMIKRYDEHHQDLTLLKALVRQQLPEKYKEIFFDQSKNGYAGYIDGGASQEEFYKFIKPILEKMDGTEELLVKLNREDLLRKQRTFDNGSIPHQIHLGELHAILRRQEDFYPFLKDNREKIEKILTFRIPYYVGPLARGNSRFAWMTRKSEETITPWNFEEVVDKGASAQSFIERMTNFDKNLPNEKVLPKHSLLYEYFTVYNELTKVKYVTEGMRKPAFLSGEQKKAIVDLLFKTNRKVTVKQLKEDYFKKIECFDSVEISGVEDRFNASLGTYHDLLKIIKDKDFLDNEENEDILEDIVLTLTLFEDREMIEERLKTYAHLFDDKVMKQLKRRRYTGWGRLSRKLINGIRDKQSGKTILDFLKSDGFANRNFMQLIHDDSLTFKEDIQKAQVSGQGDSLHEHIANLAGSPAIKKGILQTVKVVDELVKVMGRHKPENIVIEMARENQTTQKGQKNSRERMKRIEEGIKELGSQILKEHPVENTQLQNEKLYLYYLQNGRDMYVDQELDINRLSDYDVDAIVPQSFLKDDSIDNKVLTRSDKNRGKSDNVPSEEVVKKMKNYWRQLLNAKLITQRKFDNLTKAERGGLSELDKAGFIKRQLVETRQITKHVAQILDSRMNTKYDENDKLIREVKVITLKSKLVSDFRKDFQFYKVREINNYHHAHDAYLNAVVGTALIKKYPKLESEFVYGDYKVYDVRKMIAKSEQEIGKATAKYFFYSNIMNFFKTEITLANGEIRKRPLIETNGETGEIVWDKGRDFATVRKVLSMPQVNIVKKTEVQTGGFSKESILPKRNSDKLIARKKDWDPKKYGGFDSPTVAYSVLVVAKVEKGKSKKLKSVKELLGITIMERSSFEKNPIDFLEAKGYKEVKKDLIIKLPKYSLFELENGRKRMLASAGELQKGNELALPSKYVNFLYLASHYEKLKGSPEDNEQKQLFVEQHKHYLDEIIEQISEFSKRVILADANLDKVLSAYNKHRDKPIREQAENIIHLFTLTNLGAPAAFKYFDTTIDRKRYTSTKEVLDATLIHQSITGLYETRIDLSQLGGDAYPYDVPDYASLGSGSPKKKRKVEDPKKKRKVDGIGSGSGPDIVMTQSPSSLSASVGDRVTITCRSSTGAVTTSNYASWVQEKPGKLFKGLIGGTNNRAPGVPSRFSGSLIGDKATLTISSLQPEDFATYFCALWYSNHWVFGQGTKVELKRGGGGSGGGGSGGGGSSGGGSEVKLLESGGGLVQPGGSLKLSCAVSGFSLTDYGVNWVRQAPGRGLEWIGVIWGDGITDYNSALKDRFIISKDNGKNTVYLQMSKVRSDDTALYYCVTGLFDYWGQGTLVTVSSYPYDVPDYAGGGGGSGGGGSGGGGSGGGGSX

SEQ ID NO: 154 - protein, 2460 aa, synthetic construct
  REGION 1..2460: note = V33_KRAB-1xGCN4-2a-D3a-hD3l-dCas9-scFv
  SITE 2460: note = misc_feature - Xaa =
MPAAKRVKLDGSRTLVTFKDVFVDFTREEWKLLDTAQQIVYRNVMLENYKNLVSLGYQLTKPDVILRLEKGEEPGSGMEELLSKNYHLENEVARLKKGSGSGGSGSGGSGSGSGGSGSGGSGSGGSGATNFSLLKQAGDVEENPGPMPAAKRVKLDGSNHDQEFDPPKVYPPVPAEKRKPIRVLSLFDGIATGLLVLKDLGIQVDRYIASEVCEDSITVGMVRHQGKIMYVGDVRSVTQKHIQEWGPFDLVIGGSPCNDLSIVNPARKGLYEGTGRLFFEFYRLLHDARPKEGDDRPFFWLFENVVAMGVSDKRDISRFLESNPVMIDAKEVSAAHRARYFWGNLPGMNRPLASTVNDKLELQECLEHGRIAKFSKVRTITTRSNSIKQGKDQHFPVFMNEKEDILWCTEMERVFGFPVHYTDVSNMSRLARQRLLGRSWSVPVIRHLFAPLKEYFACVSSGNSNANSRGPSFSSGLVPLSLRGSHMFETVPVWRRQPVRVLSLFEDIKKELTSLGFLESGSDPGQLKHVVDVTDTVRKDVEEWGPFDLVYGATPPLGHTCDRPPSWYLFQFHRLLQYARPKPGSPRPFFWMFVDNLVLNKEDLDVASRFLEMEPVTIPDVHGGSLQNAVRVWSNIPAIRSSRHWALVSEEELSLLAQNKQSSKLAAKWPTKLVKNCFLPLREYFKYFSGGPSSGAPPPSGGSPAGSPTSTEEGTSESATPESGPGTSTEPSEGSAPGSPAGSPTSTEEGTSTEPSEGSAPGTSTEPSEPKKKRKVMDKKYSIGLAIGTNSVGWAVITDEYKVPSKKFKVLGNTDRHSIKKNLIGALLFDSGETAEATRLKRTARRRYTRRKNRICYLQEIFSNEMAKVDDSFFHRLEESFLVEEDKKHERHPIFGNIVDEVAYHEKYPTIYHLRKKLVDSTDKADLRLIYLALAHMIKFRGHFLIEGDLNPDNSDVDKLFIQLVQTYNQLFEENPINASGVDAKAILSARLSKSRRLENLIAQLPGEKKNGLFGNLIALSLGLTPNFKSNFDLAEDAKLQLSKDTYDDDLDNLLAQIGDQYADLFLAAKNLSDAILLSDILRVNTEITKAPLSASMIKRYDEHHQDLTLLKALVRQQLPEKYKEIFFDQSKNGYAGYIDGGASQEEFYKFIKPILEKMDGTEELLVKLNREDLLRKQRTFDNGSIPHQIHLGELHAILRRQEDFYPFLKDNREKIEKILTFRIPYYVGPLARGNSRFAWMTRKSEETITPWNFEEVVDKGASAQSFIERMTNFDKNLPNEKVLPKHSLLYEYFTVYNELTKVKYVTEGMRKPAFLSGEQKKAIVDLLFKTNRKVTVKQLKEDYFKKIECFDSVEISGVEDRFNASLGTYHDLLKIIKDKDFLDNEENEDILEDIVLTLTLFEDREMIEERLKTYAHLFDDKVMKQLKRRRYTGWGRLSRKLINGIRDKQSGKTILDFLKSDGFANRNFMQLIHDDSLTFKEDIQKAQVSGQGDSLHEHIANLAGSPAIKKGILQTVKVVDELVKVMGRHKPENIVIEMARENQTTQKGQKNSRERMKRIEEGIKELGSQILKEHPVENTQLQNEKLYLYYLQNGRDMYVDQELDINRLSDYDVDAIVPQSFLKDDSIDNKVLTRSDKNRGKSDNVPSEEVVKKMKNYWRQLLNAKLITQRKFDNLTKAERGGLSELDKAGFIKRQLVETRQITKHVAQILDSRMNTKYDENDKLIREVKVITLKSKLVSDFRKDFQFYKVREINNYHHAHDAYLNAVVGTALIKKYPKLESEFVYGDYKVYDVRKMIAKSEQEIGKATAKYFFYSNIMNFFKTEITLANGEIRKRPLIETNGETGEIVWDKGRDFATVRKVLSMPQVNIVKKTEVQTGGFSKESILPKRNSDKLIARKKDWDPKKYGGFDSPTVAYSVLVVAKVEKGKSKKLKSVKELLGITIMERSSFEKNPIDFLEAKGYKEVKKDLIIKLPKYSLFELENGRKRMLASAGELQKGNELALPSKYVNFLYLASHYEKLKGSPEDNEQKQLFVEQHKHYLDEIIEQISEFSKRVILADANLDKVLSAYNKHRDKPIREQAENIIHLFTLTNLGAPAAFKYFDTTIDRKRYTSTKEVLDATLIHQSITGLYETRIDLSQLGGDAYPYDVPDYASLGSGSPKKKRKVEDPKKKRKVDGIGSGSGPDIVMTQSPSSLSASVGDRVTITCRSSTGAVTTSNYASWVQEKPGKLFKGLIGGTNNRAPGVPSRFSGSLIGDKATLTISSLQPEDFATYFCALWYSNHWVFGQGTKVELKRGGGGSGGGGSGGGGSSGGGSEVKLLESGGGLVQPGGSLKLSCAVSGFSLTDYGVNWVRQAPGRGLEWIGVIWGDGITDYNSALKDRFIISKDNGKNTVYLQMSKVRSDDTALYYCVTGLFDYWGQGTLVTVSSYPYDVPDYAGGGGGSGGGGSGGGGSGGGGSX

SEQ ID NO: 155 - protein, 2467 aa, synthetic construct
  REGION 1..2467: note = V34_D3a-D3l-1xGCN4-2a-scFv-dCas9-KRAB
  SITE 2467: note = misc_feature - Xaa =
MPAAKRVKLDGSNHDQEFDPPKVYPPVPAEKRKPIRVLSLFDGIATGLLVLKDLGIQVDRYIASEVCEDSITVGMVRHQGKIMYVGDVRSVTQKHIQEWGPFDLVIGGSPCNDLSIVNPARKGLYEGTGRLFFEFYRLLHDARPKEGDDRPFFWLFENVVAMGVSDKRDISRFLESNPVMIDAKEVSAAHRARYFWGNLPGMNRPLASTVNDKLELQECLEHGRIAKFSKVRTITTRSNSIKQGKDQHFPVFMNEKEDILWCTEMERVFGFPVHYTDVSNMSRLARQRLLGRSWSVPVIRHLFAPLKEYFACVSSGNSNANSRGPSFSSGLVPLSLRGSHMGPMEIYKTVSAWKRQPVRVLSLFRNIDKVLKSLGFLESGSGSGGGTLKYVEDVTNVVRRDVEKWGPFDLVYGSTQPLGSSCDRCPGWYMFQFHRILQYALPRQESQRPFFWIFMDNLLLTEDDQETTTRFLQTEAVTLQDVRGRDYQNAMRVWSNIPGLKSKHAPLTPKEEEYLQAQVRSRSKLDAPKVDLLVKNCLLPLREYFKYFSQNSLPLGGPSSGAPPPSGGSPAGSPTSTEEGTSESATGSGSGGSGSGGSGSGSGGSGSGGSGSGEELLSKNYHLENEVARLKKGSGSGGSGSGGSGSGSGGSGSGGSGSGPKKKRKVGSGATNFSLLKQAGDVEENPGPMPAAKRVKLDGSGPDIVMTQSPSSLSASVGDRVTITCRSSTGAVTTSNYASWVQEKPGKLFKGLIGGTNNRAPGVPSRFSGSLIGDKATLTISSLQPEDFATYFCALWYSNHWVFGQGTKVELKRGGGGSGGGGSGGGGSSGGGSEVKLLESGGGLVQPGGSLKLSCAVSGFSLTDYGVNWVRQAPGRGLEWIGVIWGDGITDYNSALKDRFIISKDNGKNTVYLQMSKVRSDDTALYYCVTGLFDYWGQGTLVTVSSYPYDVPDYAGGGGGSGGGGSGGGGSGGGGSGSGPKKKRKVMDKKYSIGLAIGTNSVGWAVITDEYKVPSKKFKVLGNTDRHSIKKNLIGALLFDSGETAEATRLKRTARRRYTRRKNRICYLQEIFSNEMAKVDDSFFHRLEESFLVEEDKKHERHPIFGNIVDEVAYHEKYPTIYHLRKKLVDSTDKADLRLIYLALAHMIKFRGHFLIEGDLNPDNSDVDKLFIQLVQTYNQLFEENPINASGVDAKAILSARLSKSRRLENLIAQLPGEKKNGLFGNLIALSLGLTPNFKSNFDLAEDAKLQLSKDTYDDDLDNLLAQIGDQYADLFLAAKNLSDAILLSDILRVNTEITKAPLSASMIKRYDEHHQDLTLLKALVRQQLPEKYKEIFFDQSKNGYAGYIDGGASQEEFYKFIKPILEKMDGTEELLVKLNREDLLRKQRTFDNGSIPHQIHLGELHAILRRQEDFYPFLKDNREKIEKILTFRIPYYVGPLARGNSRFAWMTRKSEETITPWNFEEVVDKGASAQSFIERMTNFDKNLPNEKVLPKHSLLYEYFTVYNELTKVKYVTEGMRKPAFLSGEQKKAIVDLLFKTNRKVTVKQLKEDYFKKIECFDSVEISGVEDRFNASLGTYHDLLKIIKDKDFLDNEENEDILEDIVLTLTLFEDREMIEERLKTYAHLFDDKVMKQLKRRRYTGWGRLSRKLINGIRDKQSGKTILDFLKSDGFANRNFMQLIHDDSLTFKEDIQKAQVSGQGDSLHEHIANLAGSPAIKKGILQTVKVVDELVKVMGRHKPENIVIEMARENQTTQKGQKNSRERMKRIEEGIKELGSQILKEHPVENTQLQNEKLYLYYLQNGRDMYVDQELDINRLSDYDVDAIVPQSFLKDDSIDNKVLTRSDKNRGKSDNVPSEEVVKKMKNYWRQLLNAKLITQRKFDNLTKAERGGLSELDKAGFIKRQLVETRQITKHVAQILDSRMNTKYDENDKLIREVKVITLKSKLVSDFRKDFQFYKVREINNYHHAHDAYLNAVVGTALIKKYPKLESEFVYGDYKVYDVRKMIAKSEQEIGKATAKYFFYSNIMNFFKTEITLANGEIRKRPLIETNGETGEIVWDKGRDFATVRKVLSMPQVNIVKKTEVQTGGFSKESILPKRNSDKLIARKKDWDPKKYGGFDSPTVAYSVLVVAKVEKGKSKKLKSVKELLGITIMERSSFEKNPIDFLEAKGYKEVKKDLIIKLPKYSLFELENGRKRMLASAGELQKGNELALPSKYVNFLYLASHYEKLKGSPEDNEQKQLFVEQHKHYLDEIIEQISEFSKRVILADANLDKVLSAYNKHRDKPIREQAENIIHLFTLTNLGAPAAFKYFDTTIDRKRYTSTKEVLDATLIHQSITGLYETRIDLSQLGGDAYPYDVPDYASLGSGSPKKKRKVEDPKKKRKVDGSGSETPGTSESATPESRTLVTFKDVFVDFTREEWKLLDTAQQIVYRNVMLENYKNLVSLGYQLTKPDVILRLEKGEEPX

SEQ ID NO: 156 - protein, 2521 aa, synthetic construct
  REGION 1..2521: note = V35_scFv-dCas9-KRAB-2a-1xGCN4-D3l-D3a
  SITE 2521: note = misc_feature - Xaa =
MPAAKRVKLDGSGPDIVMTQSPSSLSASVGDRVTITCRSSTGAVTTSNYASWVQEKPGKLFKGLIGGTNNRAPGVPSRFSGSLIGDKATLTISSLQPEDFATYFCALWYSNHWVFGQGTKVELKRGGGGSGGGGSGGGGSSGGGSEVKLLESGGGLVQPGGSLKLSCAVSGFSLTDYGVNWVRQAPGRGLEWIGVIWGDGITDYNSALKDRFIISKDNGKNTVYLQMSKVRSDDTALYYCVTGLFDYWGQGTLVTVSSYPYDVPDYAGGGGGSGGGGSGGGGSGGGGSGSGPKKKRKVMDKKYSIGLAIGTNSVGWAVITDEYKVPSKKFKVLGNTDRHSIKKNLIGALLFDSGETAEATRLKRTARRRYTRRKNRICYLQEIFSNEMAKVDDSFFHRLEESFLVEEDKKHERHPIFGNIVDEVAYHEKYPTIYHLRKKLVDSTDKADLRLIYLALAHMIKFRGHFLIEGDLNPDNSDVDKLFIQLVQTYNQLFEENPINASGVDAKAILSARLSKSRRLENLIAQLPGEKKNGLFGNLIALSLGLTPNFKSNFDLAEDAKLQLSKDTYDDDLDNLLAQIGDQYADLFLAAKNLSDAILLSDILRVNTEITKAPLSASMIKRYDEHHQDLTLLKALVRQQLPEKYKEIFFDQSKNGYAGYIDGGASQEEFYKFIKPILEKMDGTEELLVKLNREDLLRKQRTFDNGSIPHQIHLGELHAILRRQEDFYPFLKDNREKIEKILTFRIPYYVGPLARGNSRFAWMTRKSEETITPWNFEEVVDKGASAQSFIERMTNFDKNLPNEKVLPKHSLLYEYFTVYNELTKVKYVTEGMRKPAFLSGEQKKAIVDLLFKTNRKVTVKQLKEDYFKKIECFDSVEISGVEDRFNASLGTYHDLLKIIKDKDFLDNEENEDILEDIVLTLTLFEDREMIEERLKTYAHLFDDKVMKQLKRRRYTGWGRLSRKLINGIRDKQSGKTILDFLKSDGFANRNFMQLIHDDSLTFKEDIQKAQVSGQGDSLHEHIANLAGSPAIKKGILQTVKVVDELVKVMGRHKPENIVIEMARENQTTQKGQKNSRERMKRIEEGIKELGSQILKEHPVENTQLQNEKLYLYYLQNGRDMYVDQELDINRLSDYDVDAIVPQSFLKDDSIDNKVLTRSDKNRGKSDNVPSEEVVKKMKNYWRQLLNAKLITQRKFDNLTKAERGGLSELDKAGFIKRQLVETRQITKHVAQILDSRMNTKYDENDKLIREVKVITLKSKLVSDFRKDFQFYKVREINNYHHAHDAYLNAVVGTALIKKYPKLESEFVYGDYKVYDVRKMIAKSEQEIGKATAKYFFYSNIMNFFKTEITLANGEIRKRPLIETNGETGEIVWDKGRDFATVRKVLSMPQVNIVKKTEVQTGGFSKESILPKRNSDKLIARKKDWDPKKYGGFDSPTVAYSVLVVAKVEKGKSKKLKSVKELLGITIMERSSFEKNPIDFLEAKGYKEVKKDLIIKLPKYSLFELENGRKRMLASAGELQKGNELALPSKYVNFLYLASHYEKLKGSPEDNEQKQLFVEQHKHYLDEIIEQISEFSKRVILADANLDKVLSAYNKHRDKPIREQAENIIHLFTLTNLGAPAAFKYFDTTIDRKRYTSTKEVLDATLIHQSITGLYETRIDLSQLGGDAYPYDVPDYASLGSGSPKKKRKVEDPKKKRKVDGSGSETPGTSESATPESRTLVTFKDVFVDFTREEWKLLDTAQQIVYRNVMLENYKNLVSLGYQLTKPDVILRLEKGEEPGSGATNFSLLKQAGDVEENPGPMPAAKRVKLDGSGSGGSGSGEELLSKNYHLENEVARLKKGSGSGGSGSGGSGSGSGGSGSGGSGSGTPGTSEGGPSSGAPPPSGGSPAGSPTSTEEGTSESATPESGPGTSTEPSEGSAPGSPAGSPTSTEEGTSTEPSEGSAPGTSTEPSESATPESMFETVPVWRRQPVRVLSLFEDIKKELTSLGFLESGSDPGQLKHVVDVTDTVRKDVEEWGPFDLVYGATPPLGHTCDRPPSWYLFQFHRLLQYARPKPGSPRPFFWMFVDNLVLNKEDLDVASRFLEMEPVTIPDVHGGSLQNAVRVWSNIPAIRSSRHWALVSEEELSLLAQNKQSSKLAAKWPTKLVKNCFLPLREYFKYFSTELTSSLSSGNSNANSRGPSFSSGLVPLSLRGSHMNHDQEFDPPKVYPPVPAEKRKPIRVLSLFDGIATGLLVLKDLGIQVDRYIASEVCEDSITVGMVRHQGKIMYVGDVRSVTQKHIQEWGPFDLVIGGSPCNDLSIVNPARKGLYEGTGRLFFEFYRLLHDARPKEGDDRPFFWLFENVVAMGVSDKRDISRFLESNPVMIDAKEVSAAHRARYFWGNLPGMNRPLASTVNDKLELQECLEHGRIAKFSKVRTITTRSNSIKQGKDQHFPVFMNEKEDILWCTEMERVFGFPVHYTDVSNMSRLARQRLLGRSWSVPVIRHLFAPLKEYFACVLEATNFSLLKQAGDVEENPGPMHX

SEQ ID NO: 157 - protein, 2653 aa, synthetic construct
  REGION 1..2653: note = V36_scFv-dCas9-HP1a-2a-1xGCN4-D3l-D3a
  SITE 2653: note = misc_feature - Xaa =
MPAAKRVKLDGSGPDIVMTQSPSSLSASVGDRVTITCRSSTGAVTTSNYASWVQEKPGKLFKGLIGGTNNRAPGVPSRFSGSLIGDKATLTISSLQPEDFATYFCALWYSNHWVFGQGTKVELKRGGGGSGGGGSGGGGSSGGGSEVKLLESGGGLVQPGGSLKLSCAVSGFSLTDYGVNWVRQAPGRGLEWIGVIWGDGITDYNSALKDRFIISKDNGKNTVYLQMSKVRSDDTALYYCVTGLFDYWGQGTLVTVSSYPYDVPDYAGGGGGSGGGGSGGGGSGGGGSGSGPKKKRKVMDKKYSIGLAIGTNSVGWAVITDEYKVPSKKFKVLGNTDRHSIKKNLIGALLFDSGETAEATRLKRTARRRYTRRKNRICYLQEIFSNEMAKVDDSFFHRLEESFLVEEDKKHERHPIFGNIVDEVAYHEKYPTIYHLRKKLVDSTDKADLRLIYLALAHMIKFRGHFLIEGDLNPDNSDVDKLFIQLVQTYNQLFEENPINASGVDAKAILSARLSKSRRLENLIAQLPGEKKNGLFGNLIALSLGLTPNFKSNFDLAEDAKLQLSKDTYDDDLDNLLAQIGDQYADLFLAAKNLSDAILLSDILRVNTEITKAPLSASMIKRYDEHHQDLTLLKALVRQQLPEKYKEIFFDQSKNGYAGYIDGGASQEEFYKFIKPILEKMDGTEELLVKLNREDLLRKQRTFDNGSIPHQIHLGELHAILRRQEDFYPFLKDNREKIEKILTFRIPYYVGPLARGNSRFAWMTRKSEETITPWNFEEVVDKGASAQSFIERMTNFDKNLPNEKVLPKHSLLYEYFTVYNELTKVKYVTEGMRKPAFLSGEQKKAIVDLLFKTNRKVTVKQLKEDYFKKIECFDSVEISGVEDRFNASLGTYHDLLKIIKDKDFLDNEENEDILEDIVLTLTLFEDREMIEERLKTYAHLFDDKVMKQLKRRRYTGWGRLSRKLINGIRDKQSGKTILDFLKSDGFANRNFMQLIHDDSLTFKEDIQKAQVSGQGDSLHEHIANLAGSPAIKKGILQTVKVVDELVKVMGRHKPENIVIEMARENQTTQKGQKNSRERMKRIEEGIKELGSQILKEHPVENTQLQNEKLYLYYLQNGRDMYVDQELDINRLSDYDVDAIVPQSFLKDDSIDNKVLTRSDKNRGKSDNVPSEEVVKKMKNYWRQLLNAKLITQRKFDNLTKAERGGLSELDKAGFIKRQLVETRQITKHVAQILDSRMNTKYDENDKLIREVKVITLKSKLVSDFRKDFQFYKVREINNYHHAHDAYLNAVVGTALIKKYPKLESEFVYGDYKVYDVRKMIAKSEQEIGKATAKYFFYSNIMNFFKTEITLANGEIRKRPLIETNGETGEIVWDKGRDFATVRKVLSMPQVNIVKKTEVQTGGFSKESILPKRNSDKLIARKKDWDPKKYGGFDSPTVAYSVLVVAKVEKGKSKKLKSVKELLGITIMERSSFEKNPIDFLEAKGYKEVKKDLIIKLPKYSLFELENGRKRMLASAGELQKGNELALPSKYVNFLYLASHYEKLKGSPEDNEQKQLFVEQHKHYLDEIIEQISEFSKRVILADANLDKVLSAYNKHRDKPIREQAENIIHLFTLTNLGAPAAFKYFDTTIDRKRYTSTKEVLDATLIHQSITGLYETRIDLSQLGGDAYPYDVPDYASLGSGSPKKKRKVEDPKKKRKVDGSGSETPGTSESATPESRTLGKKTKRTADSSSSEDEEEYVVEKVLDRRVVKGQVEYLLKWKGFSEEHNTWEPEKNLDCPELISEFMKKYKKMKEGENNKPREKSESNKRKSNFSNSADDIKSKKKREQSNDIARGFERGLEPEKIIGATDSCGDLMFLMKWKDTDEADLVLAKEANVKCPQIVIAFYEERLTWHAYPEDAENKEKETAKSEGSGATNFSLLKQAGDVEENPGPMPAAKRVKLDGSGSGGSGSGEELLSKNYHLENEVARLKKGSGSGGSGSGGSGSGSGGSGSGGSGSGTPGTSEGGPSSGAPPPSGGSPAGSPTSTEEGTSESATPESGPGTSTEPSEGSAPGSPAGSPTSTEEGTSTEPSEGSAPGTSTEPSESATPESMFETVPVWRRQPVRVLSLFEDIKKELTSLGFLESGSDPGQLKHVVDVTDTVRKDVEEWGPFDLVYGATPPLGHTCDRPPSWYLFQFHRLLQYARPKPGSPRPFFWMFVDNLVLNKEDLDVASRFLEMEPVTIPDVHGGSLQNAVRVWSNIPAIRSSRHWALVSEEELSLLAQNKQSSKLAAKWPTKLVKNCFLPLREYFKYFSTELTSSLSSGNSNANSRGPSFSSGLVPLSLRGSHMNHDQEFDPPKVYPPVPAEKRKPIRVLSLFDGIATGLLVLKDLGIQVDRYIASEVCEDSITVGMVRHQGKIMYVGDVRSVTQKHIQEWGPFDLVIGGSPCNDLSIVNPARKGLYEGTGRLFFEFYRLLHDARPKEGDDRPFFWLFENVVAMGVSDKRDISRFLESNPVMIDAKEVSAAHRARYFWGNLPGMNRPLASTVNDKLELQECLEHGRIAKFSKVRTITTRSNSIKQGKDQHFPVFMNEKEDILWCTEMERVFGFPVHYTDVSNMSRLARQRLLGRSWSVPVIRHLFAPLKEYFACVLEATNFSLLKQAGDVEENPGPMHX

SEQ ID NO: 158 - protein, 2571 aa, synthetic construct
  REGION 1..2571: note = V37_GFP1-10-KRAB-2a-D3a-D3l-dCas9-7xGFP11
  SITE 2571: note = misc_feature - Xaa =
MSKGEELFTGVVPILVELDGDVNGHKFSVRGEGEGDATIGKLTLKFICTTGKLPVPWPTLVTTLTYGVQCFSRYPDHMKRHDFFKSAMPEGYVQERTISFKDDGKYKTRAVVKFEGDTLVNRIELKGTDFKEDGNILGHKLEYNFNSHNVYITADKQKNGIKANFTVRHNVEDGSVQLADHYQQNTPIGDGPVLLPDNHYLSTQTVLSKDPNEKLDPGGGGSGRTLVTFKDVFVDFTREEWKLLDTAQQIVYRNVMLENYKNLVSLGYQLTKPDVILRLEKGEEPGSGKRTADGSEFESPKKKRKVGSGATNFSLLKQAGDVEENPGPPAAKRVKLDGSNHDQEFDPPKVYPPVPAEKRKPIRVLSLFDGIATGLLVLKDLGIQVDRYIASEVCEDSITVGMVRHQGKIMYVGDVRSVTQKHIQEWGPFDLVIGGSPCNDLSIVNPARKGLYEGTGRLFFEFYRLLHDARPKEGDDRPFFWLFENVVAMGVSDKRDISRFLESNPVMIDAKEVSAAHRARYFWGNLPGMNRPLASTVNDKLELQECLEHGRIAKFSKVRTITTRSNSIKQGKDQHFPVFMNEKEDILWCTEMERVFGFPVHYTDVSNMSRLARQRLLGRSWSVPVIRHLFAPLKEYFACVSSGNSNANSRGPSFSSGLVPLSLRGSHMGPMEIYKTVSAWKRQPVRVLSLFRNIDKVLKSLGFLESGSGSGGGTLKYVEDVTNVVRRDVEKWGPFDLVYGSTQPLGSSCDRCPGWYMFQFHRILQYALPRQESQRPFFWIFMDNLLLTEDDQETTTRFLQTEAVTLQDVRGRDYQNAMRVWSNIPGLKSKHAPLTPKEEEYLQAQVRSRSKLDAPKVDLLVKNCLLPLREYFKYFSQNSLPLGGPSSGAPPPSGGSPAGSPTSTEEGTSESATPESGPGTSTEPSEGSAPGSPAGSPTSTEEGTSTEPSEGSAPGTSTEPSEPKKKRKVMDKKYSIGLAIGTNSVGWAVITDEYKVPSKKFKVLGNTDRHSIKKNLIGALLFDSGETAEATRLKRTARRRYTRRKNRICYLQEIFSNEMAKVDDSFFHRLEESFLVEEDKKHERHPIFGNIVDEVAYHEKYPTIYHLRKKLVDSTDKADLRLIYLALAHMIKFRGHFLIEGDLNPDNSDVDKLFIQLVQTYNQLFEENPINASGVDAKAILSARLSKSRRLENLIAQLPGEKKNGLFGNLIALSLGLTPNFKSNFDLAEDAKLQLSKDTYDDDLDNLLAQIGDQYADLFLAAKNLSDAILLSDILRVNTEITKAPLSASMIKRYDEHHQDLTLLKALVRQQLPEKYKEIFFDQSKNGYAGYIDGGASQEEFYKFIKPILEKMDGTEELLVKLNREDLLRKQRTFDNGSIPHQIHLGELHAILRRQEDFYPFLKDNREKIEKILTFRIPYYVGPLARGNSRFAWMTRKSEETITPWNFEEVVDKGASAQSFIERMTNFDKNLPNEKVLPKHSLLYEYFTVYNELTKVKYVTEGMRKPAFLSGEQKKAIVDLLFKTNRKVTVKQLKEDYFKKIECFDSVEISGVEDRFNASLGTYHDLLKIIKDKDFLDNEENEDILEDIVLTLTLFEDREMIEERLKTYAHLFDDKVMKQLKRRRYTGWGRLSRKLINGIRDKQSGKTILDFLKSDGFANRNFMQLIHDDSLTFKEDIQKAQVSGQGDSLHEHIANLAGSPAIKKGILQTVKVVDELVKVMGRHKPENIVIEMARENQTTQKGQKNSRERMKRIEEGIKELGSQILKEHPVENTQLQNEKLYLYYLQNGRDMYVDQELDINRLSDYDVDAIVPQSFLKDDSIDNKVLTRSDKNRGKSDNVPSEEVVKKMKNYWRQLLNAKLITQRKFDNLTKAERGGLSELDKAGFIKRQLVETRQITKHVAQILDSRMNTKYDENDKLIREVKVITLKSKLVSDFRKDFQFYKVREINNYHHAHDAYLNAVVGTALIKKYPKLESEFVYGDYKVYDVRKMIAKSEQEIGKATAKYFFYSNIMNFFKTEITLANGEIRKRPLIETNGETGEIVWDKGRDFATVRKVLSMPQVNIVKKTEVQTGGFSKESILPKRNSDKLIARKKDWDPKKYGGFDSPTVAYSVLVVAKVEKGKSKKLKSVKELLGITIMERSSFEKNPIDFLEAKGYKEVKKDLIIKLPKYSLFELENGRKRMLASAGELQKGNELALPSKYVNFLYLASHYEKLKGSPEDNEQKQLFVEQHKHYLDEIIEQISEFSKRVILADANLDKVLSAYNKHRDKPIREQAENIIHLFTLTNLGAPAAFKYFDTTIDRKRYTSTKEVLDATLIHQSITGLYETRIDLSQLGGDAYPYDVPDYASLGSGSPKKKRKVEDPKKKRKVDGSGSETPGTSESATPESGSGSNGSSGSMRDHMVLHEYVNAAGITGGSGGRDHMVLHEYVNAAGITGGSGGRDHMVLHEYVNAAGITGGSGGRDHMVLHEYVNAAGITGGSGGRDHMVLHEYVNAAGITGGSGGRDHMVLHEYVNAAGITGGSGGRDHMVLHEYVNAAGITAAARSGSGQRGSKRTADGSEFESPKKKRKVX

SEQ ID NO: 159 - protein, 2445 aa, synthetic construct
  REGION 1..2445: note = V38_GFP1-10-KRAB-2a-D3a-D3l-dCas9-1xGFP11
  SITE 2445: note = misc_feature - Xaa =
MSKGEELFTGVVPILVELDGDVNGHKFSVRGEGEGDATIGKLTLKFICTTGKLPVPWPTLVTTLTYGVQCFSRYPDHMKRHDFFKSAMPEGYVQERTISFKDDGKYKTRAVVKFEGDTLVNRIELKGTDFKEDGNILGHKLEYNFNSHNVYITADKQKNGIKANFTVRHNVEDGSVQLADHYQQNTPIGDGPVLLPDNHYLSTQTVLSKDPNEKLDPGGGGSGRTLVTFKDVFVDFTREEWKLLDTAQQIVYRNVMLENYKNLVSLGYQLTKPDVILRLEKGEEPGSGKRTADGSEFESPKKKRKVGSGATNFSLLKQAGDVEENPGPPAAKRVKLDGSNHDQEFDPPKVYPPVPAEKRKPIRVLSLFDGIATGLLVLKDLGIQVDRYIASEVCEDSITVGMVRHQGKIMYVGDVRSVTQKHIQEWGPFDLVIGGSPCNDLSIVNPARKGLYEGTGRLFFEFYRLLHDARPKEGDDRPFFWLFENVVAMGVSDKRDISRFLESNPVMIDAKEVSAAHRARYFWGNLPGMNRPLASTVNDKLELQECLEHGRIAKFSKVRTITTRSNSIKQGKDQHFPVFMNEKEDILWCTEMERVFGFPVHYTDVSNMSRLARQRLLGRSWSVPVIRHLFAPLKEYFACVSSGNSNANSRGPSFSSGLVPLSLRGSHMGPMEIYKTVSAWKRQPVRVLSLFRNIDKVLKSLGFLESGSGSGGGTLKYVEDVTNVVRRDVEKWGPFDLVYGSTQPLGSSCDRCPGWYMFQFHRILQYALPRQESQRPFFWIFMDNLLLTEDDQETTTRFLQTEAVTLQDVRGRDYQNAMRVWSNIPGLKSKHAPLTPKEEEYLQAQVRSRSKLDAPKVDLLVKNCLLPLREYFKYFSQNSLPLGGPSSGAPPPSGGSPAGSPTSTEEGTSESATPESGPGTSTEPSEGSAPGSPAGSPTSTEEGTSTEPSEGSAPGTSTEPSEPKKKRKVMDKKYSIGLAIGTNSVGWAVITDEYKVPSKKFKVLGNTDRHSIKKNLIGALLFDSGETAEATRLKRTARRRYTRRKNRICYLQEIFSNEMAKVDDSFFHRLEESFLVEEDKKHERHPIFGNIVDEVAYHEKYPTIYHLRKKLVDSTDKADLRLIYLALAHMIKFRGHFLIEGDLNPDNSDVDKLFIQLVQTYNQLFEENPINASGVDAKAILSARLSKSRRLENLIAQLPGEKKNGLFGNLIALSLGLTPNFKSNFDLAEDAKLQLSKDTYDDDLDNLLAQIGDQYADLFLAAKNLSDAILLSDILRVNTEITKAPLSASMIKRYDEHHQDLTLLKALVRQQLPEKYKEIFFDQSKNGYAGYIDGGASQEEFYKFIKPILEKMDGTEELLVKLNREDLLRKQRTFDNGSIPHQIHLGELHAILRRQEDFYPFLKDNREKIEKILTFRIPYYVGPLARGNSRFAWMTRKSEETITPWNFEEVVDKGASAQSFIERMTNFDKNLPNEKVLPKHSLLYEYFTVYNELTKVKYVTEGMRKPAFLSGEQKKAIVDLLFKTNRKVTVKQLKEDYFKKIECFDSVEISGVEDRFNASLGTYHDLLKIIKDKDFLDNEENEDILEDIVLTLTLFEDREMIEERLKTYAHLFDDKVMKQLKRRRYTGWGRLSRKLINGIRDKQSGKTILDFLKSDGFANRNFMQLIHDDSLTFKEDIQKAQVSGQGDSLHEHIANLAGSPAIKKGILQTVKVVDELVKVMGRHKPENIVIEMARENQTTQKGQKNSRERMKRIEEGIKELGSQILKEHPVENTQLQNEKLYLYYLQNGRDMYVDQELDINRLSDYDVDAIVPQSFLKDDSIDNKVLTRSDKNRGKSDNVPSEEVVKKMKNYWRQLLNAKLITQRKFDNLTKAERGGLSELDKAGFIKRQLVETRQITKHVAQILDSRMNTKYDENDKLIREVKVITLKSKLVSDFRKDFQFYKVREINNYHHAHDAYLNAVVGTALIKKYPKLESEFVYGDYKVYDVRKMIAKSEQEIGKATAKYFFYSNIMNFFKTEITLANGEIRKRPLIETNGETGEIVWDKGRDFATVRKVLSMPQVNIVKKTEVQTGGFSKESILPKRNSDKLIARKKDWDPKKYGGFDSPTVAYSVLVVAKVEKGKSKKLKSVKELLGITIMERSSFEKNPIDFLEAKGYKEVKKDLIIKLPKYSLFELENGRKRMLASAGELQKGNELALPSKYVNFLYLASHYEKLKGSPEDNEQKQLFVEQHKHYLDEIIEQISEFSKRVILADANLDKVLSAYNKHRDKPIREQAENIIHLFTLTNLGAPAAFKYFDTTIDRKRYTSTKEVLDATLIHQSITGLYETRIDLSQLGGDAYPYDVPDYASLGSGSPKKKRKVEDPKKKRKVDGSGSETPGTSESATPESGSGSNGSSGSMRDHMVLHEYVNAAGITAAARSGSGQRGSKRTADGSEFESPKKKRKVX

SEQ ID NO: 160 - protein, 2451 aa, synthetic construct
  REGION 1..2451: note = V39_GFP1-10-ZIM3-2a-D3a-hD3L-dCas9-1xGFP11
  SITE 2451: note = misc_feature - Xaa =
MSKGEELFTGVVPILVELDGDVNGHKFSVRGEGEGDATIGKLTLKFICTTGKLPVPWPTLVTTLTYGVQCFSRYPDHMKRHDFFKSAMPEGYVQERTISFKDDGKYKTRAVVKFEGDTLVNRIELKGTDFKEDGNILGHKLEYNFNSHNVYITADKQKNGIKANFTVRHNVEDGSVQLADHYQQNTPIGDGPVLLPDNHYLSTQTVLSKDPNEKLDPGGGGSGMNNSQGRVTFEDVTVNFTQGEWQRLNPEQRNLYRDVMLENYSNLVSVGQGETTKPDVILRLEQGKEPWLEEEEVLGSGRAEKNGDIGGQIWKPKDVKESLGSGATNFSLLKQAGDVEENPGPMPAAKRVKLDGSNHDQEFDPPKVYPPVPAEKRKPIRVLSLFDGIATGLLVLKDLGIQVDRYIASEVCEDSITVGMVRHQGKIMYVGDVRSVTQKHIQEWGPFDLVIGGSPCNDLSIVNPARKGLYEGTGRLFFEFYRLLHDARPKEGDDRPFFWLFENVVAMGVSDKRDISRFLESNPVMIDAKEVSAAHRARYFWGNLPGMNRPLASTVNDKLELQECLEHGRIAKFSKVRTITTRSNSIKQGKDQHFPVFMNEKEDILWCTEMERVFGFPVHYTDVSNMSRLARQRLLGRSWSVPVIRHLFAPLKEYFACVSSGNSNANSRGPSFSSGLVPLSLRGSHMFETVPVWRRQPVRVLSLFEDIKKELTSLGFLESGSDPGQLKHVVDVTDTVRKDVEEWGPFDLVYGATPPLGHTCDRPPSWYLFQFHRLLQYARPKPGSPRPFFWMFVDNLVLNKEDLDVASRFLEMEPVTIPDVHGGSLQNAVRVWSNIPAIRSSRHWALVSEEELSLLAQNKQSSKLAAKWPTKLVKNCFLPLREYFKYFSGGPSSGAPPPSGGSPAGSPTSTEEGTSESATPESGPGTSTEPSEGSAPGSPAGSPTSTEEGTSTEPSEGSAPGTSTEPSEPKKKRKVMDKKYSIGLAIGTNSVGWAVITDEYKVPSKKFKVLGNTDRHSIKKNLIGALLFDSGETAEATRLKRTARRRYTRRKNRICYLQEIFSNEMAKVDDSFFHRLEESFLVEEDKKHERHPIFGNIVDEVAYHEKYPTIYHLRKKLVDSTDKADLRLIYLALAHMIKFRGHFLIEGDLNPDNSDVDKLFIQLVQTYNQLFEENPINASGVDAKAILSARLSKSRRLENLIAQLPGEKKNGLFGNLIALSLGLTPNFKSNFDLAEDAKLQLSKDTYDDDLDNLLAQIGDQYADLFLAAKNLSDAILLSDILRVNTEITKAPLSASMIKRYDEHHQDLTLLKALVRQQLPEKYKEIFFDQSKNGYAGYIDGGASQEEFYKFIKPILEKMDGTEELLVKLNREDLLRKQRTFDNGSIPHQIHLGELHAILRRQEDFYPFLKDNREKIEKILTFRIPYYVGPLARGNSRFAWMTRKSEETITPWNFEEVVDKGASAQSFIERMTNFDKNLPNEKVLPKHSLLYEYFTVYNELTKVKYVTEGMRKPAFLSGEQKKAIVDLLFKTNRKVTVKQLKEDYFKKIECFDSVEISGVEDRFNASLGTYHDLLKIIKDKDFLDNEENEDILEDIVLTLTLFEDREMIEERLKTYAHLFDDKVMKQLKRRRYTGWGRLSRKLINGIRDKQSGKTILDFLKSDGFANRNFMQLIHDDSLTFKEDIQKAQVSGQGDSLHEHIANLAGSPAIKKGILQTVKVVDELVKVMGRHKPENIVIEMARENQTTQKGQKNSRERMKRIEEGIKELGSQILKEHPVENTQLQNEKLYLYYLQNGRDMYVDQELDINRLSDYDVDAIVPQSFLKDDSIDNKVLTRSDKNRGKSDNVPSEEVVKKMKNYWRQLLNAKLITQRKFDNLTKAERGGLSELDKAGFIKRQLVETRQITKHVAQILDSRMNTKYDENDKLIREVKVITLKSKLVSDFRKDFQFYKVREINNYHHAHDAYLNAVVGTALIKKYPKLESEFVYGDYKVYDVRKMIAKSEQEIGKATAKYFFYSNIMNFFKTEITLANGEIRKRPLIETNGETGEIVWDKGRDFATVRKVLSMPQVNIVKKTEVQTGGFSKESILPKRNSDKLIARKKDWDPKKYGGFDSPTVAYSVLVVAKVEKGKSKKLKSVKELLGITIMERSSFEKNPIDFLEAKGYKEVKKDLIIKLPKYSLFELENGRKRMLASAGELQKGNELALPSKYVNFLYLASHYEKLKGSPEDNEQKQLFVEQHKHYLDEIIEQISEFSKRVILADANLDKVLSAYNKHRDKPIREQAENIIHLFTLTNLGAPAAFKYFDTTIDRKRYTSTKEVLDATLIHQSITGLYETRIDLSQLGGDAYPYDVPDYASLGSGSPKKKRKVEDPKKKRKVDGSGSETPGTSESATPESGSGSNGSSGSMRDHMVLHEYVNAAGITAAARSGSGQRGSKRTADGSEFESPKKKRKVX

SEQ ID NO: 161 - protein, 2833 aa, synthetic construct
  REGION 1..2833: note = V40_GFP1-10-HDAC1-2a-D3a-hD3L-dCas9-1xGFP11
  SITE 2833: note = misc_feature - Xaa =
MSKGEELFTGVVPILVELDGDVNGHKFSVRGEGEGDATIGKLTLKFICTTGKLPVPWPTLVTTLTYGVQCFSRYPDHMKRHDFFKSAMPEGYVQERTISFKDDGKYKTRAVVKFEGDTLVNRIELKGTDFKEDGNILGHKLEYNFNSHNVYITADKQKNGIKANFTVRHNVEDGSVQLADHYQQNTPIGDGPVLLPDNHYLSTQTVLSKDPNEKLDPGGGGSGMAQTQGTRRKVCYYYDGDVGNYYYGQGHPMKPHRIRMTHNLLLNYGLYRKMEIYRPHKANAEEMTKYHSDDYIKFLRSIRPDNMSEYSKQMQRFNVGEDCPVFDGLFEFCQLSTGGSVASAVKLNKQQTDIAVNWAGGLHHAKKSEASGFCYVNDIVLAILELLKYHQRVLYIDIDIHHGDGVEEAFYTTDRVMTVSFHKYGEYFPGTGDLRDIGAGKGKYYAVNYPLRDGIDDESYEAIFKPVMSKVMEMFQPSAVVLQCGSDSLSGDRLGCFNLTIKGHAKCVEFVKSFNLPMLMLGGGGYTIRNVARCWTYETAVALDTEIPNELPYNDYFEYFGPDFKLHISPSNMTNQNTNEYLEKIKQRLFENLRMLPHAPGVQMQAIPEDAIPEESGDEDEDDPDKRISICSSDKRIACEEEFSDSEEEGEGGRKNSSNFKKAKRVKTEDEKEKDPEEKKEVTEEEKTKEEKPEAKGVKEEVKLAGSGATNFSLLKQAGDVEENPGPMPAAKRVKLDGSNHDQEFDPPKVYPPVPAEKRKPIRVLSLFDGIATGLLVLKDLGIQVDRYIASEVCEDSITVGMVRHQGKIMYVGDVRSVTQKHIQEWGPFDLVIGGSPCNDLSIVNPARKGLYEGTGRLFFEFYRLLHDARPKEGDDRPFFWLFENVVAMGVSDKRDISRFLESNPVMIDAKEVSAAHRARYFWGNLPGMNRPLASTVNDKLELQECLEHGRIAKFSKVRTITTRSNSIKQGKDQHFPVFMNEKEDILWCTEMERVFGFPVHYTDVSNMSRLARQRLLGRSWSVPVIRHLFAPLKEYFACVSSGNSNANSRGPSFSSGLVPLSLRGSHMFETVPVWRRQPVRVLSLFEDIKKELTSLGFLESGSDPGQLKHVVDVTDTVRKDVEEWGPFDLVYGATPPLGHTCDRPPSWYLFQFHRLLQYARPKPGSPRPFFWMFVDNLVLNKEDLDVASRFLEMEPVTIPDVHGGSLQNAVRVWSNIPAIRSSRHWALVSEEELSLLAQNKQSSKLAAKWPTKLVKNCFLPLREYFKYFSGGPSSGAPPPSGGSPAGSPTSTEEGTSESATPESGPGTSTEPSEGSAPGSPAGSPTSTEEGTSTEPSEGSAPGTSTEPSEPKKKRKVMDKKYSIGLAIGTNSVGWAVITDEYKVPSKKFKVLGNTDRHSIKKNLIGALLFDSGETAEATRLKRTARRRYTRRKNRICYLQEIFSNEMAKVDDSFFHRLEESFLVEEDKKHERHPIFGNIVDEVAYHEKYPTIYHLRKKLVDSTDKADLRLIYLALAHMIKFRGHFLIEGDLNPDNSDVDKLFIQLVQTYNQLFEENPINASGVDAKAILSARLSKSRRLENLIAQLPGEKKNGLFGNLIALSLGLTPNFKSNFDLAEDAKLQLSKDTYDDDLDNLLAQIGDQYADLFLAAKNLSDAILLSDILRVNTEITKAPLSASMIKRYDEHHQDLTLLKALVRQQLPEKYKEIFFDQSKNGYAGYIDGGASQEEFYKFIKPILEKMDGTEELLVKLNREDLLRKQRTFDNGSIPHQIHLGELHAILRRQEDFYPFLKDNREKIEKILTFRIPYYVGPLARGNSRFAWMTRKSEETITPWNFEEVVDKGASAQSFIERMTNFDKNLPNEKVLPKHSLLYEYFTVYNELTKVKYVTEGMRKPAFLSGEQKKAIVDLLFKTNRKVTVKQLKEDYFKKIECFDSVEISGVEDRFNASLGTYHDLLKIIKDKDFLDNEENEDILEDIVLTLTLFEDREMIEERLKTYAHLFDDKVMKQLKRRRYTGWGRLSRKLINGIRDKQSGKTILDFLKSDGFANRNFMQLIHDDSLTFKEDIQKAQVSGQGDSLHEHIANLAGSPAIKKGILQTVKVVDELVKVMGRHKPENIVIEMARENQTTQKGQKNSRERMKRIEEGIKELGSQILKEHPVENTQLQNEKLYLYYLQNGRDMYVDQELDINRLSDYDVDAIVPQSFLKDDSIDNKVLTRSDKNRGKSDNVPSEEVVKKMKNYWRQLLNAKLITQRKFDNLTKAERGGLSELDKAGFIKRQLVETRQITKHVAQILDSRMNTKYDENDKLIREVKVITLKSKLVSDFRKDFQFYKVREINNYHHAHDAYLNAVVGTALIKKYPKLESEFVYGDYKVYDVRKMIAKSEQEIGKATAKYFFYSNIMNFFKTEITLANGEIRKRPLIETNGETGEIVWDKGRDFATVRKVLSMPQVNIVKKTEVQTGGFSKESILPKRNSDKLIARKKDWDPKKYGGFDSPTVAYSVLVVAKVEKGKSKKLKSVKELLGITIMERSSFEKNPIDFLEAKGYKEVKKDLIIKLPKYSLFELENGRKRMLASAGELQKGNELALPSKYVNFLYLASHYEKLKGSPEDNEQKQLFVEQHKHYLDEIIEQISEFSKRVILADANLDKVLSAYNKHRDKPIREQAENIIHLFTLTNLGAPAAFKYFDTTIDRKRYTSTKEVLDATLIHQSITGLYETRIDLSQLGGDAYPYDVPDYASLGSGSPKKKRKVEDPKKKRKVDGSGSETPGTSESATPESGSGSNGSSGSMRDHMVLHEYVNAAGITAAARSGSGQRGSKRTADGSEFESPKKKRKVX

SEQ ID NO: 162 - protein, 2311 aa, synthetic construct
  REGION 1..2311: note = V41_GFP1-10-ZIM3-2a-D3a-hD3L-dCas12a-1xGFP11
  SITE 2311: note = misc_feature - Xaa =
MSKGEELFTGVVPILVELDGDVNGHKFSVRGEGEGDATIGKLTLKFICTTGKLPVPWPTLVTTLTYGVQCFSRYPDHMKRHDFFKSAMPEGYVQERTISFKDDGKYKTRAVVKFEGDTLVNRIELKGTDFKEDGNILGHKLEYNFNSHNVYITADKQKNGIKANFTVRHNVEDGSVQLADHYQQNTPIGDGPVLLPDNHYLSTQTVLSKDPNEKLDPGGGGSGMNNSQGRVTFEDVTVNFTQGEWQRLNPEQRNLYRDVMLENYSNLVSVGQGETTKPDVILRLEQGKEPWLEEEEVLGSGRAEKNGDIGGQIWKPKDVKESLGSGATNFSLLKQAGDVEENPGPMPAAKRVKLDGSNHDQEFDPPKVYPPVPAEKRKPIRVLSLFDGIATGLLVLKDLGIQVDRYIASEVCEDSITVGMVRHQGKIMYVGDVRSVTQKHIQEWGPFDLVIGGSPCNDLSIVNPARKGLYEGTGRLFFEFYRLLHDARPKEGDDRPFFWLFENVVAMGVSDKRDISRFLESNPVMIDAKEVSAAHRARYFWGNLPGMNRPLASTVNDKLELQECLEHGRIAKFSKVRTITTRSNSIKQGKDQHFPVFMNEKEDILWCTEMERVFGFPVHYTDVSNMSRLARQRLLGRSWSVPVIRHLFAPLKEYFACVSSGNSNANSRGPSFSSGLVPLSLRGSHMFETVPVWRRQPVRVLSLFEDIKKELTSLGFLESGSDPGQLKHVVDVTDTVRKDVEEWGPFDLVYGATPPLGHTCDRPPSWYLFQFHRLLQYARPKPGSPRPFFWMFVDNLVLNKEDLDVASRFLEMEPVTIPDVHGGSLQNAVRVWSNIPAIRSSRHWALVSEEELSLLAQNKQSSKLAAKWPTKLVKNCFLPLREYFKYFSGGPSSGAPPPSGGSPAGSPTSTEEGTSESATPESGPGTSTEPSEGSAPGSPAGSPTSTEEGTSTEPSEGSAPGTSTEPSEPKKKRKVMSKLEKFTNCYSLSKTLRFKAIPVGKTQENIDNKRLLVEDEKRAEDYKGVKKLLDRYYLSFINDVLHSIKLKNLNNYISLFRKKTRTEKENKELENLEINLRKEIAKAFKGNEGYKSLFKKDIIETILPEFLDDKDEIALVNSFNGFTTAFTGFFDNRENMFSEEAKSTSIAFRCINENLTRYISNMDIFEKVDAIFDKHEVQEIKEKILNSDYDVEDFFEGEFFNFVLTQEGIDVYNAIIGGFVTESGEKIKGLNEYINLYNQKTKQKLPKFKPLYKQVLSDRESLSFYGEGYTSDEEVLEVFRNTLNKNSEIFSSIKKLEKLFKNFDEYSSAGIFVKNGPAISTISKDIFGEWNVIRDKWNAEYDDIHLKKKAVVTEKYEDDRRKSFKKIGSFSLEQLQEYADADLSVVEKLKEIIIQKVDEIYKVYGSSEKLFDADFVLEKSLKKNDAVVAIMKDLLDSVKSFENYIKAFFGEGKETNRDESFYGDFVLAYDILLKVDHIYDAIRNYVTQKPYSKDKFKLYFQNPQFMGGWDKDKETDYRATILRYGSKYYLAIMDKKYAKCLQKIDKDDVNGNYEKINYKLLPGPNKMLPKVFFSKKWMAYYNPSEDIQKIYKNGTFKKGDMFNLNDCHKLIDFFKDSISRYPKWSNAYDFNFSETEKYKDIAGFYREVEEQGYKVSFESASKKEVDKLVEEGKLYMFQIYNKDFSDKSHGTPNLHTMYFKLLFDENNHGQIRLSGGAELFMRRASLKKEELVVHPANSPIANKNPDNPKKTTTLSYDVYKDKRFSEDQYELHIPIAINKCPKNIFKINTEVRVLLKHDDNPYVIGIARGERNLLYIVVVDGKGNIVEQYSLNEIINNFNGIRIKTDYHSLLDKKEKERFEARQNWTSIENIKELKAGYISQVVHKICELVEKYDAVIALADLNSGFKNSRVKVEKQVYQKFEKMLIDKLNYMVDKKSNPCATGGALKGYQITNKFESFKSMSTQNGFIFYIPAWLTSKIDPSTGFVNLLKTKYTSIADSKKFISSFDRIMYVPEEDLFEFALDYKNFSRTDADYIKKWKLYSYGNRIRIFRNPKKNNVFDWEEVCLTSAYKELFNKYGINYQQGDIRALLCEQSDKAFYSSFMALMSLMLQMRNSITGRTDVAFLISPVKNSDGIFYDSRNYEAQENAILPKNADANGAYNIARKVLWAIGQFKKAEDEKLDKVKIAISNKEWLEYAQTSVKHAYPYDVPDYASLGSGSPKKKRKVEDPKKKRKVDGSGSETPGTSESATPESGSGSNGSSGSMRDHMVLHEYVNAAGITAAARSGSGQRGSKRTADGSEFESPKKKRKVX

SEQ ID NO: 163 - protein, 2094 aa, synthetic construct
  REGION 1..2094: note = V42_GFP1-10-ZIM3-2a-D3a-hD3L-dCas12i-1xGFP11
  SITE 2094: note = misc_feature - Xaa =
MSKGEELFTGVVPILVELDGDVNGHKFSVRGEGEGDATIGKLTLKFICTTGKLPVPWPTLVTTLTYGVQCFSRYPDHMKRHDFFKSAMPEGYVQERTISFKDDGKYKTRAVVKFEGDTLVNRIELKGTDFKEDGNILGHKLEYNFNSHNVYITADKQKNGIKANFTVRHNVEDGSVQLADHYQQNTPIGDGPVLLPDNHYLSTQTVLSKDPNEKLDPGGGGSGMNNSQGRVTFEDVTVNFTQGEWQRLNPEQRNLYRDVMLENYSNLVSVGQGETTKPDVILRLEQGKEPWLEEEEVLGSGRAEKNGDIGGQIWKPKDVKESLGSGATNFSLLKQAGDVEENPGPMPAAKRVKLDGSNHDQEFDPPKVYPPVPAEKRKPIRVLSLFDGIATGLLVLKDLGIQVDRYIASEVCEDSITVGMVRHQGKIMYVGDVRSVTQKHIQEWGPFDLVIGGSPCNDLSIVNPARKGLYEGTGRLFFEFYRLLHDARPKEGDDRPFFWLFENVVAMGVSDKRDISRFLESNPVMIDAKEVSAAHRARYFWGNLPGMNRPLASTVNDKLELQECLEHGRIAKFSKVRTITTRSNSIKQGKDQHFPVFMNEKEDILWCTEMERVFGFPVHYTDVSNMSRLARQRLLGRSWSVPVIRHLFAPLKEYFACVSSGNSNANSRGPSFSSGLVPLSLRGSHMFETVPVWRRQPVRVLSLFEDIKKELTSLGFLESGSDPGQLKHVVDVTDTVRKDVEEWGPFDLVYGATPPLGHTCDRPPSWYLFQFHRLLQYARPKPGSPRPFFWMFVDNLVLNKEDLDVASRFLEMEPVTIPDVHGGSLQNAVRVWSNIPAIRSSRHWALVSEEELSLLAQNKQSSKLAAKWPTKLVKNCFLPLREYFKYFSGGPSSGAPPPSGGSPAGSPTSTEEGTSESATPESGPGTSTEPSEGSAPGSPAGSPTSTEEGTSTEPSEGSAPGTSTEPSEPKKKRKVMGITMSDTTFRPYKSKLNPNERKMPMVVDTMNWCDNACSVFFDLFVGLYGGVKIGDVTNFLTEKQDTTTDADLLCAINWFRAMPVSNPDAVVGPEQLVVRFRDYSGHNPSPMASMYLSAPVNPRYTWVDCRFLYQQMCQTLGANLDVDISTLVQTGLLPIQKDTQLNAYSFCSNVFGEGVKEDPSAKVTSYTAAANALSGATNPIITYEDYRQILSSAITNRPSRKGAKDILAADLDSTKTGVLPGNYVSQRIAMYQASAASKARGVVLPNRLRVKAYLQNLVGLNYICTTWAAPMLRAVGDIKSKNSNNYRFVGERLERQQEIDNLLAVSNIRSAQAILQQFRANESNQFYIKKRHIGKGLPSLYDMWDLMDEKEGIDNYIQSLKGDKTERLPIRELLQIIYPHRKSVSAELFLSAAELTDVEDRQNRCMVHPTVRGSLVINFGKSSTIFGAITPPDTLIKFRGEMVPAGQTGMIWFTMHLVDGGKWVKHHIPCHSSRYFEEIYAWKKDLPTLPFPRRSLYGYAIGNKISDTRKIDLRRKKASKQYLRTLENMTHNVEFDPTTQFMVDQELNVTITARVKKIPPVRDVPVGSRIMGLNKNQTIRDCYSIWERVEANTSGSFQHPVVQDVWLRLVADGHVTSTVNGPNGQIDQMSYSGPDVANCGNWMQERSNFITSVDDADQSIMKHFLWNNRVKLYAWNCVYAGTLMKAISKQMTTANRNLFRNEILSFVGGRFGCRLGSLAQVSLDLLRRMKSVISCYFSRNNAFTIEERSAFDKELMELFESLDNKMNNKRKEKVNRTLSSIFQVAKQHNVVRLVVTKNLQTPDANVRSVMNQRSVDWCARKIEEKIVDLGNVIGIYVDLVEALDLSHLDPFIYIAKGDVGKECQFDEVESSSLLPIHTSMFRDWHGLVNKGRTTTPIYHSALRSFASHYGLRFDDLARIKAAELAKMLPDQKVFIPHRGGRFFMSTYPVTSTSRPVSYDGRQRFLNSGDMVAPVNTMLRGFRRARSAYPYDVPDYASLGSGSPKKKRKVEDPKKKRKVDGSGSETPGTSESATPESGSGSNGSSGSMRDHMVLHEYVNAAGITAAARSGSGQRGSKRTADGSEFESPKKKRKVX

SEQ ID NO: 164 - protein, 2392 aa, synthetic construct
  REGION 1..2392: note = V43_D3a-D3l-GFP1-10-2a-1xGFP11-dCas9-KRAB
  SITE 2392: note = misc_feature - Xaa =
MPAAKRVKLDGSNHDQEFDPPKVYPPVPAEKRKPIRVLSLFDGIATGLLVLKDLGIQVDRYIASEVCEDSITVGMVRHQGKIMYVGDVRSVTQKHIQEWGPFDLVIGGSPCNDLSIVNPARKGLYEGTGRLFFEFYRLLHDARPKEGDDRPFFWLFENVVAMGVSDKRDISRFLESNPVMIDAKEVSAAHRARYFWGNLPGMNRPLASTVNDKLELQECLEHGRIAKFSKVRTITTRSNSIKQGKDQHFPVFMNEKEDILWCTEMERVFGFPVHYTDVSNMSRLARQRLLGRSWSVPVIRHLFAPLKEYFACVSSGNSNANSRGPSFSSGLVPLSLRGSHMGPMEIYKTVSAWKRQPVRVLSLFRNIDKVLKSLGFLESGSGSGGGTLKYVEDVTNVVRRDVEKWGPFDLVYGSTQPLGSSCDRCPGWYMFQFHRILQYALPRQESQRPFFWIFMDNLLLTEDDQETTTRFLQTEAVTLQDVRGRDYQNAMRVWSNIPGLKSKHAPLTPKEEEYLQAQVRSRSKLDAPKVDLLVKNCLLPLREYFKYFSQNSLPLGGPSSGAPPPSGGSPAGSPTSTEEGTSESATMSKGEELFTGVVPILVELDGDVNGHKFSVRGEGEGDATIGKLTLKFICTTGKLPVPWPTLVTTLTYGVQCFSRYPDHMKRHDFFKSAMPEGYVQERTISFKDDGKYKTRAVVKFEGDTLVNRIELKGTDFKEDGNILGHKLEYNFNSHNVYITADKQKNGIKANFTVRHNVEDGSVQLADHYQQNTPIGDGPVLLPDNHYLSTQTVLSKDPNEKLDPGGGGSGSGATNFSLLKQAGDVEENPGPMPAAKRVKLDGSGPDIVIGSGGRDHMVLHEYVNAAGITAAARSGSGQRGSKRTADGSEFESPKKKRKVGGSGSGPKKKRKVMDKKYSIGLAIGTNSVGWAVITDEYKVPSKKFKVLGNTDRHSIKKNLIGALLFDSGETAEATRLKRTARRRYTRRKNRICYLQEIFSNEMAKVDDSFFHRLEESFLVEEDKKHERHPIFGNIVDEVAYHEKYPTIYHLRKKLVDSTDKADLRLIYLALAHMIKFRGHFLIEGDLNPDNSDVDKLFIQLVQTYNQLFEENPINASGVDAKAILSARLSKSRRLENLIAQLPGEKKNGLFGNLIALSLGLTPNFKSNFDLAEDAKLQLSKDTYDDDLDNLLAQIGDQYADLFLAAKNLSDAILLSDILRVNTEITKAPLSASMIKRYDEHHQDLTLLKALVRQQLPEKYKEIFFDQSKNGYAGYIDGGASQEEFYKFIKPILEKMDGTEELLVKLNREDLLRKQRTFDNGSIPHQIHLGELHAILRRQEDFYPFLKDNREKIEKILTFRIPYYVGPLARGNSRFAWMTRKSEETITPWNFEEVVDKGASAQSFIERMTNFDKNLPNEKVLPKHSLLYEYFTVYNELTKVKYVTEGMRKPAFLSGEQKKAIVDLLFKTNRKVTVKQLKEDYFKKIECFDSVEISGVEDRFNASLGTYHDLLKIIKDKDFLDNEENEDILEDIVLTLTLFEDREMIEERLKTYAHLFDDKVMKQLKRRRYTGWGRLSRKLINGIRDKQSGKTILDFLKSDGFANRNFMQLIHDDSLTFKEDIQKAQVSGQGDSLHEHIANLAGSPAIKKGILQTVKVVDELVKVMGRHKPENIVIEMARENQTTQKGQKNSRERMKRIEEGIKELGSQILKEHPVENTQLQNEKLYLYYLQNGRDMYVDQELDINRLSDYDVDAIVPQSFLKDDSIDNKVLTRSDKNRGKSDNVPSEEVVKKMKNYWRQLLNAKLITQRKFDNLTKAERGGLSELDKAGFIKRQLVETRQITKHVAQILDSRMNTKYDENDKLIREVKVITLKSKLVSDFRKDFQFYKVREINNYHHAHDAYLNAVVGTALIKKYPKLESEFVYGDYKVYDVRKMIAKSEQEIGKATAKYFFYSNIMNFFKTEITLANGEIRKRPLIETNGETGEIVWDKGRDFATVRKVLSMPQVNIVKKTEVQTGGFSKESILPKRNSDKLIARKKDWDPKKYGGFDSPTVAYSVLVVAKVEKGKSKKLKSVKELLGITIMERSSFEKNPIDFLEAKGYKEVKKDLIIKLPKYSLFELENGRKRMLASAGELQKGNELALPSKYVNFLYLASHYEKLKGSPEDNEQKQLFVEQHKHYLDEIIEQISEFSKRVILADANLDKVLSAYNKHRDKPIREQAENIIHLFTLTNLGAPAAFKYFDTTIDRKRYTSTKEVLDATLIHQSITGLYETRIDLSQLGGDAYPYDVPDYASLGSGSPKKKRKVEDPKKKRKVDGSGSETPGTSESATPESRTLVTFKDVFVDFTREEWKLLDTAQQIVYRNVMLENYKNLVSLGYQLTKPDVILRLEKGEEPX

SEQ ID NO: 165 - protein, 2588 aa, synthetic construct
  REGION 1..2588: note = V44_7xGFP11-dCas9-ZIM3-2a-D3a-hD3L-GFP1-10
  SITE 2588: note = misc_feature - Xaa =
MPAAKRVKLDGSMRDHMVLHEYVNAAGITGGSGGRDHMVLHEYVNAAGITGGSGGRDHMVLHEYVNAAGITGGSGGRDHMVLHEYVNAAGITGGSGGRDHMVLHEYVNAAGITGGSGGRDHMVLHEYVNAAGITGGSGGRDHMVLHEYVNAAGITAAARSGSGQRGSKRTADGSEFESPKKKRKVGGSGSGPKKKRKVMDKKYSIGLAIGTNSVGWAVITDEYKVPSKKFKVLGNTDRHSIKKNLIGALLFDSGETAEATRLKRTARRRYTRRKNRICYLQEIFSNEMAKVDDSFFHRLEESFLVEEDKKHERHPIFGNIVDEVAYHEKYPTIYHLRKKLVDSTDKADLRLIYLALAHMIKFRGHFLIEGDLNPDNSDVDKLFIQLVQTYNQLFEENPINASGVDAKAILSARLSKSRRLENLIAQLPGEKKNGLFGNLIALSLGLTPNFKSNFDLAEDAKLQLSKDTYDDDLDNLLAQIGDQYADLFLAAKNLSDAILLSDILRVNTEITKAPLSASMIKRYDEHHQDLTLLKALVRQQLPEKYKEIFFDQSKNGYAGYIDGGASQEEFYKFIKPILEKMDGTEELLVKLNREDLLRKQRTFDNGSIPHQIHLGELHAILRRQEDFYPFLKDNREKIEKILTFRIPYYVGPLARGNSRFAWMTRKSEETITPWNFEEVVDKGASAQSFIERMTNFDKNLPNEKVLPKHSLLYEYFTVYNELTKVKYVTEGMRKPAFLSGEQKKAIVDLLFKTNRKVTVKQLKEDYFKKIECFDSVEISGVEDRFNASLGTYHDLLKIIKDKDFLDNEENEDILEDIVLTLTLFEDREMIEERLKTYAHLFDDKVMKQLKRRRYTGWGRLSRKLINGIRDKQSGKTILDFLKSDGFANRNFMQLIHDDSLTFKEDIQKAQVSGQGDSLHEHIANLAGSPAIKKGILQTVKVVDELVKVMGRHKPENIVIEMARENQTTQKGQKNSRERMKRIEEGIKELGSQILKEHPVENTQLQNEKLYLYYLQNGRDMYVDQELDINRLSDYDVDAIVPQSFLKDDSIDNKVLTRSDKNRGKSDNVPSEEVVKKMKNYWRQLLNAKLITQRKFDNLTKAERGGLSELDKAGFIKRQLVETRQITKHVAQILDSRMNTKYDENDKLIREVKVITLKSKLVSDFRKDFQFYKVREINNYHHAHDAYLNAVVGTALIKKYPKLESEFVYGDYKVYDVRKMIAKSEQEIGKATAKYFFYSNIMNFFKTEITLANGEIRKRPLIETNGETGEIVWDKGRDFATVRKVLSMPQVNIVKKTEVQTGGFSKESILPKRNSDKLIARKKDWDPKKYGGFDSPTVAYSVLVVAKVEKGKSKKLKSVKELLGITIMERSSFEKNPIDFLEAKGYKEVKKDLIIKLPKYSLFELENGRKRMLASAGELQKGNELALPSKYVNFLYLASHYEKLKGSPEDNEQKQLFVEQHKHYLDEIIEQISEFSKRVILADANLDKVLSAYNKHRDKPIREQAENIIHLFTLTNLGAPAAFKYFDTTIDRKRYTSTKEVLDATLIHQSITGLYETRIDLSQLGGDAYPYDVPDYASLGSGSPKKKRKVEDPKKKRKVDGSGSETPGTSESATPESMNNSQGRVTFEDVTVNFTQGEWQRLNPEQRNLYRDVMLENYSNLVSVGQGETTKPDVILRLEQGKEPWLEEEEVLGSGRAEKNGDIGGQIWKPKDVKESLLEGSGATNFSLLKQAGDVEENPGPMPAAKRVKLDGSNHDQEFDPPKVYPPVPAEKRKPIRVLSLFDGIATGLLVLKDLGIQVDRYIASEVCEDSITVGMVRHQGKIMYVGDVRSVTQKHIQEWGPFDLVIGGSPCNDLSIVNPARKGLYEGTGRLFFEFYRLLHDARPKEGDDRPFFWLFENVVAMGVSDKRDISRFLESNPVMIDAKEVSAAHRARYFWGNLPGMNRPLASTVNDKLELQECLEHGRIAKFSKVRTITTRSNSIKQGKDQHFPVFMNEKEDILWCTEMERVFGFPVHYTDVSNMSRLARQRLLGRSWSVPVIRHLFAPLKEYFACVSSGNSNANSRGPSFSSGLVPLSLRGSHMFETVPVWRRQPVRVLSLFEDIKKELTSLGFLESGSDPGQLKHVVDVTDTVRKDVEEWGPFDLVYGATPPLGHTCDRPPSWYLFQFHRLLQYARPKPGSPRPFFWMFVDNLVLNKEDLDVASRFLEMEPVTIPDVHGGSLQNAVRVWSNIPAIRSSRHWALVSEEELSLLAQNKQSSKLAAKWPTKLVKNCFLPLREYFKYFSGGPSSGAPPPSGGSPAGSPTSTEEGTSESATPESGPGTSTEPSEGSAPGSPAGSPTSTEEGTSTEPSEGSAPGTSTEPSEPKKKRKVPSEMSKGEELFTGVVPILVELDGDVNGHKFSVRGEGEGDATIGKLTLKFICTTGKLPVPWPTLVTTLTYGVQCFSRYPDHMKRHDFFKSAMPEGYVQERTISFKDDGKYKTRAVVKFEGDTLVNRIELKGTDFKEDGNILGHKLEYNFNSHNVYITADKQKNGIKANFTVRHNVEDGSVQLADHYQQNTPIGDGPVLLPDNHYLSTQTVLSKDPNEKX

SEQ ID NO: 166 - protein, 2389 aa, synthetic construct
  REGION 1..2389: note = V45_D3a-D3l-1xGFP11-2a-GFP1-10-dCas9-KRAB
  SITE 2389: note = misc_feature - Xaa =
MPAAKRVKLDGSNHDQEFDPPKVYPPVPAEKRKPIRVLSLFDGIATGLLVLKDLGIQVDRYIASEVCEDSITVGMVRHQGKIMYVGDVRSVTQKHIQEWGPFDLVIGGSPCNDLSIVNPARKGLYEGTGRLFFEFYRLLHDARPKEGDDRPFFWLFENVVAMGVSDKRDISRFLESNPVMIDAKEVSAAHRARYFWGNLPGMNRPLASTVNDKLELQECLEHGRIAKFSKVRTITTRSNSIKQGKDQHFPVFMNEKEDILWCTEMERVFGFPVHYTDVSNMSRLARQRLLGRSWSVPVIRHLFAPLKEYFACVSSGNSNANSRGPSFSSGLVPLSLRGSHMGPMEIYKTVSAWKRQPVRVLSLFRNIDKVLKSLGFLESGSGSGGGTLKYVEDVTNVVRRDVEKWGPFDLVYGSTQPLGSSCDRCPGWYMFQFHRILQYALPRQESQRPFFWIFMDNLLLTEDDQETTTRFLQTEAVTLQDVRGRDYQNAMRVWSNIPGLKSKHAPLTPKEEEYLQAQVRSRSKLDAPKVDLLVKNCLLPLREYFKYFSQNSLPLGGPSSGAPPPSGGSPAGSPTSTEEGTSESATGGSGGRDHMVLHEYVNAAGITAAARSGSGQRGSKRTADGSEFESPKKKRKVGSGATNFSLLKQAGDVEENPGPMPAAKRVKLDGSGPDIVMSKGEELFTGVVPILVELDGDVNGHKFSVRGEGEGDATIGKLTLKFICTTGKLPVPWPTLVTTLTYGVQCFSRYPDHMKRHDFFKSAMPEGYVQERTISFKDDGKYKTRAVVKFEGDTLVNRIELKGTDFKEDGNILGHKLEYNFNSHNVYITADKQKNGIKANFTVRHNVEDGSVQLADHYQQNTPIGDGPVLLPDNHYLSTQTVLSKDPNEKLDPGGGGSGSGPKKKRKVMDKKYSIGLAIGTNSVGWAVITDEYKVPSKKFKVLGNTDRHSIKKNLIGALLFDSGETAEATRLKRTARRRYTRRKNRICYLQEIFSNEMAKVDDSFFHRLEESFLVEEDKKHERHPIFGNIVDEVAYHEKYPTIYHLRKKLVDSTDKADLRLIYLALAHMIKFRGHFLIEGDLNPDNSDVDKLFIQLVQTYNQLFEENPINASGVDAKAILSARLSKSRRLENLIAQLPGEKKNGLFGNLIALSLGLTPNFKSNFDLAEDAKLQLSKDTYDDDLDNLLAQIGDQYADLFLAAKNLSDAILLSDILRVNTEITKAPLSASMIKRYDEHHQDLTLLKALVRQQLPEKYKEIFFDQSKNGYAGYIDGGASQEEFYKFIKPILEKMDGTEELLVKLNREDLLRKQRTFDNGSIPHQIHLGELHAILRRQEDFYPFLKDNREKIEKILTFRIPYYVGPLARGNSRFAWMTRKSEETITPWNFEEVVDKGASAQSFIERMTNFDKNLPNEKVLPKHSLLYEYFTVYNELTKVKYVTEGMRKPAFLSGEQKKAIVDLLFKTNRKVTVKQLKEDYFKKIECFDSVEISGVEDRFNASLGTYHDLLKIIKDKDFLDNEENEDILEDIVLTLTLFEDREMIEERLKTYAHLFDDKVMKQLKRRRYTGWGRLSRKLINGIRDKQSGKTILDFLKSDGFANRNFMQLIHDDSLTFKEDIQKAQVSGQGDSLHEHIANLAGSPAIKKGILQTVKVVDELVKVMGRHKPENIVIEMARENQTTQKGQKNSRERMKRIEEGIKELGSQILKEHPVENTQLQNEKLYLYYLQNGRDMYVDQELDINRLSDYDVDAIVPQSFLKDDSIDNKVLTRSDKNRGKSDNVPSEEVVKKMKNYWRQLLNAKLITQRKFDNLTKAERGGLSELDKAGFIKRQLVETRQITKHVAQILDSRMNTKYDENDKLIREVKVITLKSKLVSDFRKDFQFYKVREINNYHHAHDAYLNAVVGTALIKKYPKLESEFVYGDYKVYDVRKMIAKSEQEIGKATAKYFFYSNIMNFFKTEITLANGEIRKRPLIETNGETGEIVWDKGRDFATVRKVLSMPQVNIVKKTEVQTGGFSKESILPKRNSDKLIARKKDWDPKKYGGFDSPTVAYSVLVVAKVEKGKSKKLKSVKELLGITIMERSSFEKNPIDFLEAKGYKEVKKDLIIKLPKYSLFELENGRKRMLASAGELQKGNELALPSKYVNFLYLASHYEKLKGSPEDNEQKQLFVEQHKHYLDEIIEQISEFSKRVILADANLDKVLSAYNKHRDKPIREQAENIIHLFTLTNLGAPAAFKYFDTTIDRKRYTSTKEVLDATLIHQSITGLYETRIDLSQLGGDAYPYDVPDYASLGSGSPKKKRKVEDPKKKRKVDGSGSETPGTSESATPESRTLVTFKDVFVDFTREEWKLLDTAQQIVYRNVMLENYKNLVSLGYQLTKPDVILRLEKGEEPX

SEQ ID NO: 167 - protein, 2656 aa, synthetic construct
  REGION 1..2656: note = V46_10xGFP11-dCas9-ZIM3-2a-D3a-hD3L-GFP1-10
  SITE 2656: note = misc_feature - Xaa =
MPAAKRVKLDGSMRDHMVLHEYVNAAGITGGSGGRDHMVLHEYVNAAGITGGSGGRDHMVLHEYVNAAGITGGSGGRDHMVLHEYVNAAGITGGSGGRDHMVLHEYVNAAGITGGSGGRDHMVLHEYVNAAGITGGSGGRDHMVLHEYVNAAGITAAAGGSGGRDHMVLHEYVNAAGITGGSGGRDHMVLHEYVNAAGITGGSGGRDHMVLHEYVNAAGITGGSGGRSGSGQRGSKRTADGSEFESPKKKRKVGGSGSGPKKKRKVMDKKYSIGLAIGTNSVGWAVITDEYKVPSKKFKVLGNTDRHSIKKNLIGALLFDSGETAEATRLKRTARRRYTRRKNRICYLQEIFSNEMAKVDDSFFHRLEESFLVEEDKKHERHPIFGNIVDEVAYHEKYPTIYHLRKKLVDSTDKADLRLIYLALAHMIKFRGHFLIEGDLNPDNSDVDKLFIQLVQTYNQLFEENPINASGVDAKAILSARLSKSRRLENLIAQLPGEKKNGLFGNLIALSLGLTPNFKSNFDLAEDAKLQLSKDTYDDDLDNLLAQIGDQYADLFLAAKNLSDAILLSDILRVNTEITKAPLSASMIKRYDEHHQDLTLLKALVRQQLPEKYKEIFFDQSKNGYAGYIDGGASQEEFYKFIKPILEKMDGTEELLVKLNREDLLRKQRTFDNGSIPHQIHLGELHAILRRQEDFYPFLKDNREKIEKILTFRIPYYVGPLARGNSRFAWMTRKSEETITPWNFEEVVDKGASAQSFIERMTNFDKNLPNEKVLPKHSLLYEYFTVYNELTKVKYVTEGMRKPAFLSGEQKKAIVDLLFKTNRKVTVKQLKEDYFKKIECFDSVEISGVEDRFNASLGTYHDLLKIIKDKDFLDNEENEDILEDIVLTLTLFEDREMIEERLKTYAHLFDDKVMKQLKRRRYTGWGRLSRKLINGIRDKQSGKTILDFLKSDGFANRNFMQLIHDDSLTFKEDIQKAQVSGQGDSLHEHIANLAGSPAIKKGILQTVKVVDELVKVMGRHKPENIVIEMARENQTTQKGQKNSRERMKRIEEGIKELGSQILKEHPVENTQLQNEKLYLYYLQNGRDMYVDQELDINRLSDYDVDAIVPQSFLKDDSIDNKVLTRSDKNRGKSDNVPSEEVVKKMKNYWRQLLNAKLITQRKFDNLTKAERGGLSELDKAGFIKRQLVETRQITKHVAQILDSRMNTKYDENDKLIREVKVITLKSKLVSDFRKDFQFYKVREINNYHHAHDAYLNAVVGTALIKKYPKLESEFVYGDYKVYDVRKMIAKSEQEIGKATAKYFFYSNIMNFFKTEITLANGEIRKRPLIETNGETGEIVWDKGRDFATVRKVLSMPQVNIVKKTEVQTGGFSKESILPKRNSDKLIARKKDWDPKKYGGFDSPTVAYSVLVVAKVEKGKSKKLKSVKELLGITIMERSSFEKNPIDFLEAKGYKEVKKDLIIKLPKYSLFELENGRKRMLASAGELQKGNELALPSKYVNFLYLASHYEKLKGSPEDNEQKQLFVEQHKHYLDEIIEQISEFSKRVILADANLDKVLSAYNKHRDKPIREQAENIIHLFTLTNLGAPAAFKYFDTTIDRKRYTSTKEVLDATLIHQSITGLYETRIDLSQLGGDAYPYDVPDYASLGSGSPKKKRKVEDPKKKRKVDGSGSETPGTSESATPESMNNSQGRVTFEDVTVNFTQGEWQRLNPEQRNLYRDVMLENYSNLVSVGQGETTKPDVILRLEQGKEPWLEEEEVLGSGRAEKNGDIGGQIWKPKDVKESLLEGSGATNFSLLKQAGDVEENPGPMPAAKRVKLDGSNHDQEFDPPKVYPPVPAEKRKPIRVLSLFDGIATGLLVLKDLGIQVDRYIASEVCEDSITVGMVRHQGKIMYVGDVRSVTQKHIQEWGPFDLVIGGSPCNDLSIVNPARKGLYEGTGRLFFEFYRLLHDARPKEGDDRPFFWLFENVVAMGVSDKRDISRFLESNPVMIDAKEVSAAHRARYFWGNLPGMNRPLASTVNDKLELQECLEHGRIAKFSKVRTITTRSNSIKQGKDQHFPVFMNEKEDILWCTEMERVFGFPVHYTDVSNMSRLARQRLLGRSWSVPVIRHLFAPLKEYFACVSSGNSNANSRGPSFSSGLVPLSLRGSHMFETVPVWRRQPVRVLSLFEDIKKELTSLGFLESGSDPGQLKHVVDVTDTVRKDVEEWGPFDLVYGATPPLGHTCDRPPSWYLFQFHRLLQYARPKPGSPRPFFWMFVDNLVLNKEDLDVASRFLEMEPVTIPDVHGGSLQNAVRVWSNIPAIRSSRHWALVSEEELSLLAQNKQSSKLAAKWPTKLVKNCFLPLREYFKYFSGGPSSGAPPPSGGSPAGSPTSTEEGTSESATPESGPGTSTEPSEGSAPGSPAGSPTSTEEGTSTEPSEGSAPGTSTEPSEPKKKRKVPSEMSKGEELFTGVVPILVELDGDVNGHKFSVRGEGEGDATIGKLTLKFICTTGKLPVPWPTLVTTLTYGVQCFSRYPDHMKRHDFFKSAMPEGYVQERTISFKDDGKYKTRAVVKFEGDTLVNRIELKGTDFKEDGNILGHKLEYNFNSHNVYITADKQKNGIKANFTVRHNVEDGSVQLADHYQQNTPIGDGPVLLPDNHYLSTQTVLSKDPNEKX

SEQ ID NO: 168 - protein, 2546 aa, synthetic construct
  REGION 1..2546: note = V47_scFv-ZIM3-2a-D3a-hD3L-dCas9-1xGCN4
  SITE 2546: note = misc_feature - Xaa =
MVPAAKRVKLDGSGPDIVMTQSPSSLSASVGDRVTITCRSSTGAVTTSNYASWVQEKPGKLFKGLIGGTNNRAPGVPSRFSGSLIGDKATLTISSLQPEDFATYFCALWYSNHWVFGQGTKVELKRGGGGSGGGGSGGGGSSGGGSEVKLLESGGGLVQPGGSLKLSCAVSGFSLTDYGVNWVRQAPGRGLEWIGVIWGDGITDYNSALKDRFIISKDNGKNTVYLQMSKVRSDDTALYYCVTGLFDYWGQGTLVTVSSYPYDVPDYAGGGGGSGGGGSGGGGSGGGGSLDPGGGGSGMNNSQGRVTFEDVTVNFTQGEWQRLNPEQRNLYRDVMLENYSNLVSVGQGETTKPDVILRLEQGKEPWLEEEEVLGSGRAEKNGDIGGQIWKPKDVKESLGSGATNFSLLKQAGDVEENPGPMPAAKRVKLDGSNHDQEFDPPKVYPPVPAEKRKPIRVLSLFDGIATGLLVLKDLGIQVDRYIASEVCEDSITVGMVRHQGKIMYVGDVRSVTQKHIQEWGPFDLVIGGSPCNDLSIVNPARKGLYEGTGRLFFEFYRLLHDARPKEGDDRPFFWLFENVVAMGVSDKRDISRFLESNPVMIDAKEVSAAHRARYFWGNLPGMNRPLASTVNDKLELQECLEHGRIAKFSKVRTITTRSNSIKQGKDQHFPVFMNEKEDILWCTEMERVFGFPVHYTDVSNMSRLARQRLLGRSWSVPVIRHLFAPLKEYFACVSSGNSNANSRGPSFSSGLVPLSLRGSHMFETVPVWRRQPVRVLSLFEDIKKELTSLGFLESGSDPGQLKHVVDVTDTVRKDVEEWGPFDLVYGATPPLGHTCDRPPSWYLFQFHRLLQYARPKPGSPRPFFWMFVDNLVLNKEDLDVASRFLEMEPVTIPDVHGGSLQNAVRVWSNIPAIRSSRHWALVSEEELSLLAQNKQSSKLAAKWPTKLVKNCFLPLREYFKYFSGGPSSGAPPPSGGSPAGSPTSTEEGTSESATPESGPGTSTEPSEGSAPGSPAGSPTSTEEGTSTEPSEGSAPGTSTEPSEPKKKRKVGSDKKYSIGLAIGTNSVGWAVITDEYKVPSKKFKVLGNTDRHSIKKNLIGALLFDSGETAEATRLKRTARRRYTRRKNRICYLQEIFSNEMAKVDDSFFHRLEESFLVEEDKKHERHPIFGNIVDEVAYHEKYPTIYHLRKKLVDSTDKADLRLIYLALAHMIKFRGHFLIEGDLNPDNSDVDKLFIQLVQTYNQLFEENPINASGVDAKAILSARLSKSRRLENLIAQLPGEKKNGLFGNLIALSLGLTPNFKSNFDLAEDAKLQLSKDTYDDDLDNLLAQIGDQYADLFLAAKNLSDAILLSDILRVNTEITKAPLSASMIKRYDEHHQDLTLLKALVRQQLPEKYKEIFFDQSKNGYAGYIDGGASQEEFYKFIKPILEKMDGTEELLVKLNREDLLRKQRTFDNGSIPHQIHLGELHAILRRQEDFYPFLKDNREKIEKILTFRIPYYVGPLARGNSRFAWMTRKSEETITPWNFEEVVDKGASAQSFIERMTNFDKNLPNEKVLPKHSLLYEYFTVYNELTKVKYVTEGMRKPAFLSGEQKKAIVDLLFKTNRKVTVKQLKEDYFKKIECFDSVEISGVEDRFNASLGTYHDLLKIIKDKDFLDNEENEDILEDIVLTLTLFEDREMIEERLKTYAHLFDDKVMKQLKRRRYTGWGRLSRKLINGIRDKQSGKTILDFLKSDGFANRNFMQLIHDDSLTFKEDIQKAQVSGQGDSLHEHIANLAGSPAIKKGILQTVKVVDELVKVMGRHKPENIVIEMARENQTTQKGQKNSRERMKRIEEGIKELGSQILKEHPVENTQLQNEKLYLYYLQNGRDMYVDQELDINRLSDYDVDAIVPQSFLKDDSIDNKVLTRSDKNRGKSDNVPSEEVVKKMKNYWRQLLNAKLITQRKFDNLTKAERGGLSELDKAGFIKRQLVETRQITKHVAQILDSRMNTKYDENDKLIREVKVITLKSKLVSDFRKDFQFYKVREINNYHHAHDAYLNAVVGTALIKKYPKLESEFVYGDYKVYDVRKMIAKSEQEIGKATAKYFFYSNIMNFFKTEITLANGEIRKRPLIETNGETGEIVWDKGRDFATVRKVLSMPQVNIVKKTEVQTGGFSKESILPKRNSDKLIARKKDWDPKKYGGFDSPTVAYSVLVVAKVEKGKSKKLKSVKELLGITIMERSSFEKNPIDFLEAKGYKEVKKDLIIKLPKYSLFELENGRKRMLASAGELQKGNELALPSKYVNFLYLASHYEKLKGSPEDNEQKQLFVEQHKHYLDEIIEQISEFSKRVILADANLDKVLSAYNKHRDKPIREQAENIIHLFTLTNLGAPAAFKYFDTTIDRKRYTSTKEVLDATLIHQSITGLYETRIDLSQLGGDAYPYDVPDYASLGSGSPKKKRKVEDPKKKRKVDGIGSGSNGSSGEELLSKNYHLENEVARLKKGSGSGGSGSGGSGSGSGGSGSGGSGSGEELLSKNYHGSGSGQRGSKRTADGSEFESPKKKRKVX

SEQ ID NO: 169 - DNA, 7509 bp, synthetic construct
  misc_feature 1..7509: note = DNA of 1st fusion_DNMT3ACD-DNMT3LCD-dCas9-10*GCN4
  source 1..7509: mol_type = other DNA
atgaaccatgaccaggaatttgaccccccaaaggtttacccacctgtgccagctgagaagaggaagcccatccgcgtgctgtctctctttgatgggattgctacagggctcctggtgctgaaggacctgggcatccaagtggaccgctacattgcctccgaggtgtgtgaggactccatcacggtgggcatggtgcggcaccagggaaagatcatgtacgtcggggacgtccgcagcgtcacacagaagcatatccaggagtggggcccattcgacctggtgattggaggcagtccctgcaatgacctctccattgtcaaccctgcccgcaagggactttatgagggtactggccgcctcttctttgagttctaccgcctcctgcatgatgcgcggcccaaggagggagatgatcgccccttcttctggctctttgagaatgtggtggccatgggcgttagtgacaagagggacatctcgcgatttcttgagtctaaccccgtgatgattgacgccaaagaagtgtctgctgcacacagggcccgttacttctggggtaaccttcctggcatgaacaggcctttggcatccactgtgaatgataagctggagctgcaagagtgtctggagcacggcagaatagccaagttcagcaaagtgaggaccattaccaccaggtcaaactctataaagcagggcaaagaccagcatttccccgtcttcatgaacgagaaggaggacatcctgtggtgcactgaaatggaaagggtgtttggcttccccgtccactacacagacgtctccaacatgagccgcttggcgaggcagagactgctgggccgatcgtggagcgtgccggtcatccgccacctcttcgctccgctgaaggaatattttgcttgtgtgtctagcggcaatagtaacgctaacagccgcgggccgagcttcagcagcggcctggtgccgttaagcttgcgcggcagccatatgggccctatggagatatacaagacagtgtctgcatggaagagacagccagtgcgggtactgagcctcttcagaaacatcgacaaggtactaaagagtttgggcttcttggaaagcggttctggttctgggggaggaacgctgaagtacgtggaagatgtcacaaatgtcgtgaggagagacgtggagaaatggggcccctttgacctggtgtacggctcgacgcagcccctaggcagctcttgtgatcgctgtcccggctggtacatgttccagttccaccggatcctgcagtatgcgctgcctcgccaggagagtcagcggcccttcttctggatattcatggacaatctgctgctgactgaggatgaccaagagacaactacccgcttccttcagacagaggctgtgaccctccaggatgtccgtggcagagactaccagaatgctatgcgggtgtggagcaacattccagggctgaagagcaagcatgcgcccctgaccccaaaggaagaagagtatctgcaagcccaagtcagaagcaggagcaagctggacgccccgaaagttgacctcctggtgaagaactgccttctcccgctgagagagtacttcaagtatttttctcaaaactcacttcctcttggagggccgagctctggcgcacccccaccaagtggagggtctcctgccgggtccccaacatctactgaagaaggcaccagcgaatccgcaacgcccgagtcaggccctggtacctccacagaaccatctgaaggtagtgcgcctggttccccagctggaagccctacttccaccgaagaaggcacgtcaaccgaaccaagtgaaggatctgcccctgggaccagcactgaaccatctgagccaaaaaagaagagaaaggtaatggacaagaagtacagcatcggcctggccatcggcaccaactctgtgggctgggccgtgatcaccgacgagtacaaggtgcccagcaagaaattcaaggtgctgggcaacaccgaccggcacagcatcaagaagaacctgatcggcgccctgctgttcgacagcggagaaacagccgaggccacccggctgaagagaaccgccagaagaagatacaccagacggaagaaccggatctgctatctgcaagagatcttcagcaacgagatggccaaggtggacgacagcttcttccacagactggaagagtccttcctggtggaagaggataagaagcacgagcggcaccccatcttcggcaacatcgtggacgaggtggcctaccacgagaagtaccccaccatctaccacctgagaaagaaactggtggacagcaccgacaaggccgacctgcggctgatctatctggccctggcccacatgatcaagttccggggccacttcctgatcgagggcgacctgaaccccgacaacagcgacgtggacaagctgttcatccagctggtgcagacctacaaccagctgttcgaggaaaaccccatcaacgccagcggcgtggacgccaaggccatcctgtctgccagactgagcaagagcagacggctggaaaatctgatcgcccagctgcccggcgagaagaagaatggcctgttcggcaacctgattgccctgagcctgggcctgacccccaacttcaagagcaacttcgacctggccgaggatgccaaactgcagctgagcaaggacacctacgacgacgacctggacaacctgctggcccagatcggcgaccagtacgccgacctgtttctggccgccaagaacctgtccgacgccatcctgctgagcgacatcctgagagtgaacaccgagatcaccaaggcccccctgagcgcctctatgatcaagagatacgacgagcaccaccaggacctgaccctgctgaaagctctcgtgcggcagcagctgcctgagaagtacaaagagattttcttcgaccagagcaagaacggctacgccggctacatcgatggcggagccagccaggaagagttctacaagttcatcaagcccatcctggaaaagatggacggcaccgaggaactgctcgtgaagctgaacagagaggacctgctgcggaagcagcggaccttcgacaacggcagcatcccccaccagatccacctgggagagctgcacgccattctgcggcggcaggaagatttttacccattcctgaaggacaaccgggaaaagatcgagaagatcctgaccttccgcatcccctactacgtgggccctctggccaggggaaacagcagattcgcctggatgaccagaaagagcgaggaaaccatcaccccctggaacttcgaggaagtggtggacaagggcgccagcgcccagagcttcatcgagcggatgaccaacttcgataagaacctgcccaacgagaaggtgctgcccaagcacagcctgctgtacgagtacttcaccgtgtacaacgagctgaccaaagtgaaatacgtgaccgagggaatgagaaagcccgccttcctgagcggcgagcagaaaaaagccatcgtggacctgctgttcaagaccaaccggaaagtgaccgtgaagcagctgaaagaggactacttcaagaaaatcgagtgcttcgactccgtggaaatctccggcgtggaagatcggttcaacgcctccctgggcacataccacgatctgctgaaaattatcaaggacaaggacttcctggacaatgaggaaaacgaggacattctggaagatatcgtgctgaccctgacactgtttgaggacagagagatgatcgaggaacggctgaaaacctatgcccacctgttcgacgacaaagtgatgaagcagctgaagcggcggagatacaccggctggggcaggctgagccggaagctgatcaacggcatccgggacaagcagtccggcaagacaatcctggatttcctgaagtccgacggcttcgccaacagaaacttcatgcagctgatccacgacgacagcctgacctttaaagaggacatccagaaagcccaggtgtccggccagggcgatagcctgcacgagcacattgccaatctggccggcagccccgccattaagaagggcatcctgcagacagtgaaggtggtggacgagctcgtgaaagtgatgggccggcacaagcccgagaacatcgtgatcgaaatggccagagagaaccagaccacccagaagggacagaagaacagccgcgagagaatgaagcggatcgaagagggcatcaaagagctgggcagccagatcctgaaagaacaccccgtggaaaacacccagctgcagaacgagaagctgtacctgtactacctgcagaatgggcgggatatgtacgtggaccaggaactggacatcaaccggctgtccgactacgatgtggacgctatcgtgcctcagagctttctgaaggacgactccatcgataacaaagtgctgactcggagcgacaagaaccggggcaagagcgacaacgtgccctccgaagaggtcgtgaagaagatgaagaactactggcgccagctgctgaatgccaagctgattacccagaggaagttcgacaatctgaccaaggccgagagaggcggcctgagcgaactggataaggccggcttcatcaagagacagctggtggaaacccggcagatcacaaagcacgtggcacagatcctggactcccggatgaacactaagtacgacgagaacgacaaactgatccgggaagtgaaagtgatcaccctgaagtccaagctggtgtccgatttccggaaggatttccagttttacaaagtgcgcgagatcaacaactaccaccacgcccacgacgcctacctgaacgccgtcgtgggaaccgccctgatcaaaaagtaccctaagctggaaagcgagttcgtgtacggcgactacaaggtgtacgacgtgcggaagatgatcgccaagagcgagcaggaaatcggcaaggctaccgccaagtacttcttctacagcaacatcatgaactttttcaagaccgagattaccctggccaacggcgagatccggaagcggcctctgatcgagacaaacggcgaaacaggcgagatcgtgtgggataagggccgggactttgccaccgtgcggaaagtgctgtctatgccccaagtgaatatcgtgaaaaagaccgaggtgcagacaggcggcttcagcaaagagtctatcctgcccaagaggaacagcgacaagctgatcgccagaaagaaggactgggaccctaagaagtacggcggcttcgacagccccaccgtggcctattctgtgctggtggtggccaaagtggaaaagggcaagtccaagaaactgaagagtgtgaaagagctgctggggatcaccatcatggaaagaagcagcttcgagaagaatcccatcgactttctggaagccaagggctacaaagaagtgaaaaaggacctgatcatcaagctgcctaagtactccctgttcgagctggaaaacggccggaagagaatgctggcctctgccggcgaactgcagaagggaaacgaactggccctgccctccaaatatgtgaacttcctgtacctggccagccactatgagaagctgaagggctcccccgaggataatgagcagaaacagctgtttgtggaacagcacaaacactacctggacgagatcatcgagcagatcagcgagttctccaagagagtgatcctggccgacgctaatctggacaaggtgctgagcgcctacaacaagcacagagacaagcctatcagagagcaggccgagaatatcatccacctgtttaccctgaccaatctgggagcccctgccgccttcaagtactttgacaccaccatcgaccggaagaggtacaccagcaccaaagaggtgctggacgccaccctgatccaccagagcatcaccggcctgtacgagacacggatcgacctgtctcagctgggaggcgacgcctatccctatgacgtgcccgattatgccagcctgggcagcggctcccccaagaaaaaacgcaaggtggaagatcctaagaaaaagcggaaagtggacggcattggtagtgggagcaacggcagcagcggagaggaactgctgagcaagaactaccacctggaaaacgaggtggccagactgaagaaaggctctggctctggcggaagcggttctggcggatcaggatctggaagtggcggctctggaagcggaggttctggatctggcgaagaactgctgtctaagaattatcacctcgagaacgaagtggctcggctcaagaaaggcagtggcagcggaggaagtggatccggcggtagtggtagtggaagcggcggatccggctcaggcggatctggttcaggggaagaactcctctccaaaaactaccatctcgagaatgaggtcgcccgcctgaaaaaaggatcaggttccggtggttctggcagcggtggttcaggctcaggcagcggcggtagcggtagcggtggaagcggaagcggagaagaacttctcagcaaaaattaccacttggagaatgaagttgcaagactcaaaaaaggttccggcagtggcggcagcggcagcggcggatctggtagtggatctggtggcagtggttcaggcggaagtggtagcggagaggaattgctctcaaagaactatcatttggagaacgaggttgcacgcttgaagaaaggcagcggatcaggcggatctggcagcggtggatctggttctggatccggcggctccggtagtggtggaagtggctctggggaagaattgcttagcaagaattatcatcttgaaaatgaggttgccaggcttaaaaaaggcagtggctccggcggatccggaagcggaggcagcggatctggatctggtggttcaggatctggcggttctggtagcggggaagaactgttgagtaaaaactatcaccttgagaacgaggtcgcaaggttgaaaaaaggatccggctctggcggctccggaagtggcggatctggctccggtagcggaggatcaggatccggcggaagcggatcaggcgaggaactgctttccaaaaattaccaccttgaaaacgaagtcgcccgcctcaagaaaggttctggcagcggaggctctggcagtggtggtagcggaagtggaagtggtggcagtggtagcggtggatctggaagcggcgaggaactcctgtcaaagaattaccatctcgaaaacgaggtcgcaaggctcaagaaaggctcaggatcaggcggctctggatccggcggttctggttccggctcaggtggaagtggatctggcggctcaggttccggcgaagaattgctttccaagaactaccatttggaaaatgaagtcgctcgtttgaagaaaggttcaggctccggccagcggggaagcaagcgcaccgccgatggttccgagttcgaaagccccaaaaaaaagcgcaaggtc

SEQ ID NO: 170 - DNA, 1107 bp, synthetic construct
  misc_feature 1..1107: note = DNA of 2nd fusion_scFv-KRAB
  source 1..1107: mol_type = other DNA
atgggccccgacatcgtgatgacccagagccccagcagcctgagcgccagcgtgggcgaccgcgtgaccatcacctgccgcagcagcaccggcgccgtgaccaccagcaactacgccagctgggtgcaggagaagcccggcaagctgttcaagggcctgatcggcggcaccaacaaccgcgcccccggcgtgcccagccgcttcagcggcagcctgatcggcgacaaggccaccctgaccatcagcagcctgcagcccgaggacttcgccacctacttctgcgccctgtggtacagcaaccactgggtgttcggccagggcaccaaggtggagctgaagcgcggcggcggcggcagcggcggcggcggcagcggcggcggcggcagcagcggcggcggcagcgaggtgaagctgctggagagcggcggcggcctggtgcagcccggcggcagcctgaagctgagctgcgccgtgagcggcttcagcctgaccgactacggcgtgaactgggtgcgccaggcccccggccgcggcctggagtggatcggcgtgatctggggcgacggcatcaccgactacaacagcgccctgaaggaccgcttcatcatcagcaaggacaacggcaagaacaccgtgtacctgcagatgagcaaggtgcgcagcgacgacaccgccctgtactactgcgtgaccggcctgttcgactactggggccagggcaccctggtgaccgtgagcagctacccatacgatgttccagattacgctggtggaggcggaggttctgggggaggaggtagtggcggtggtggttcaggaggcggcggaagcttggatccaggtggaggtggaagcggtcggacactggtgaccttcaaggatgtatttgtggacttcaccagggaggagtggaagctgctggacactgctcagcagatcgtgtacagaaatgtgatgctggagaactataagaacctggtttccttgggttatcagcttactaagccagatgtgatcctccggttggagaagggagaagagcccggaagcggaaagcgcaccgccgatggttccgagttcgaaagccccaaaaaaaagcgcaaggtc

SEQ ID NO: 171 - DNA, 1107 bp, synthetic construct
  misc_feature 1..1107: note = DNA of 2nd fusion_scFv-Zim3
  source 1..1107: mol_type = other DNA
atgggccccgacatcgtgatgacccagagccccagcagcctgagcgccagcgtgggcgaccgcgtgaccatcacctgccgcagcagcaccggcgccgtgaccaccagcaactacgccagctgggtgcaggagaagcccggcaagctgttcaagggcctgatcggcggcaccaacaaccgcgcccccggcgtgcccagccgcttcagcggcagcctgatcggcgacaaggccaccctgaccatcagcagcctgcagcccgaggacttcgccacctacttctgcgccctgtggtacagcaaccactgggtgttcggccagggcaccaaggtggagctgaagcgcggcggcggcggcagcggcggcggcggcagcggcggcggcggcagcagcggcggcggcagcgaggtgaagctgctggagagcggcggcggcctggtgcagcccggcggcagcctgaagctgagctgcgccgtgagcggcttcagcctgaccgactacggcgtgaactgggtgcgccaggcccccggccgcggcctggagtggatcggcgtgatctggggcgacggcatcaccgactacaacagcgccctgaaggaccgcttcatcatcagcaaggacaacggcaagaacaccgtgtacctgcagatgagcaaggtgcgcagcgacgacaccgccctgtactactgcgtgaccggcctgttcgactactggggccagggcaccctggtgaccgtgagcagctacccatacgatgttccagattacgctggtggaggcggaggttctgggggaggaggtagtggcggtggtggttcaggaggcggcggaagcttggatccaggtggaggtggaagcggtgtgaccttcgaggacgtgaccgtgaacttcacccaaggcgagtggcagagactgaaccccgagcagagaaacctgtaccgggacgtgatgctggaaaactacagcaacctggtgtccgtcggccagggcgagacaacaaagcctgacgtgatcctgcggctggaacagggcaaagaaccttggctgggaagcggaaagcgcaccgccgatggttccgagttcgaaagccccaaaaaaaagcgcaaggtc

SEQ ID NO: 172 - DNA, 1104 bp, synthetic construct
  misc_feature 1..1104: note = DNA of 2nd fusion_scFv-Znf680
  source 1..1104: mol_type = other DNA
atgggccccgacatcgtgatgacccagagccccagcagcctgagcgccagcgtgggcgaccgcgtgaccatcacctgccgcagcagcaccggcgccgtgaccaccagcaactacgccagctgggtgcaggagaagcccggcaagctgttcaagggcctgatcggcggcaccaacaaccgcgcccccggcgtgcccagccgcttcagcggcagcctgatcggcgacaaggccaccctgaccatcagcagcctgcagcccgaggacttcgccacctacttctgcgccctgtggtacagcaaccactgggtgttcggccagggcaccaaggtggagctgaagcgcggcggcggcggcagcggcggcggcggcagcggcggcggcggcagcagcggcggcggcagcgaggtgaagctgctggagagcggcggcggcctggtgcagcccggcggcagcctgaagctgagctgcgccgtgagcggcttcagcctgaccgactacggcgtgaactgggtgcgccaggcccccggccgcggcctggagtggatcggcgtgatctggggcgacggcatcaccgactacaacagcgccctgaaggaccgcttcatcatcagcaaggacaacggcaagaacaccgtgtacctgcagatgagcaaggtgcgcagcgacgacaccgccctgtactactgcgtgaccggcctgttcgactactggggccagggcaccctggtgaccgtgagcagctacccatacgatgttccagattacgctggtggaggcggaggttctgggggaggaggtagtggcggtggtggttcaggaggcggcggaagcttggatccaggtggaggtggaagcggtctgaccttcagagatgtggccatcgagttcagcctggaagagtggcagtgcctggacacagcccagcggaacctgtacagaaaagtgatgttcgagaactaccggaacctcgtgttcctgggaatcgccgtgtctaagccccacctgatcacctgtctcgagcaagggaaagaaccctggaacggaagcggaaagcgcaccgccgatggttccgagttcgaaagccccaaaaaaaagcgcaaggtc

SEQ ID NO: 173 - DNA, 1107 bp, synthetic construct
  misc_feature 1..1107: note = DNA of 2nd fusion_scFv-Znf554
  source 1..1107: mol_type = other DNA
atgggccccgacatcgtgatgacccagagccccagcagcctgagcgccagcgtgggcgaccgcgtgaccatcacctgccgcagcagcaccggcgccgtgaccaccagcaactacgccagctgggtgcaggagaagcccggcaagctgttcaagggcctgatcggcggcaccaacaaccgcgcccccggcgtgcccagccgcttcagcggcagcctgatcggcgacaaggccaccctgaccatcagcagcctgcagcccgaggacttcgccacctacttctgcgccctgtggtacagcaaccactgggtgttcggccagggcaccaaggtggagctgaagcgcggcggcggcggcagcggcggcggcggcagcggcggcggcggcagcagcggcggcggcagcgaggtgaagctgctggagagcggcggcggcctggtgcagcccggcggcagcctgaagctgagctgcgccgtgagcggcttcagcctgaccgactacggcgtgaactgggtgcgccaggcccccggccgcggcctggagtggatcggcgtgatctggggcgacggcatcaccgactacaacagcgccctgaaggaccgcttcatcatcagcaaggacaacggcaagaacaccgtgtacctgcagatgagcaaggtgcgcagcgacgacaccgccctgtactactgcgtgaccggcctgttcgactactggggccagggcaccctggtgaccgtgagcagctacccatacgatgttccagattacgctggtggaggcggaggttctgggggaggaggtagtggcggtggtggttcaggaggcggcggaagcttggatccaggtggaggtggaagcggtgtgacatttgaggatgtctccatggacttcagccaagaggaatgggagctgctggaacccgctcagaagaacctgtatagggaagtcatgctcgaaaattaccggaatgtggtgtccctggaagccctgaagaaccagtgtaccgacgtgggcatcaaagagggcccactgtctccagctcagaccggaagcggaaagcgcaccgccgatggttccgagttcgaaagccccaaaaaaaagcgcaaggtc

SEQ ID NO: 174 - DNA, 1104 bp, synthetic construct
  misc_feature 1..1104: note = DNA of 2nd fusion_scFv-Znf264
  source 1..1104: mol_type = other DNA
atgggccccgacatcgtgatgacccagagccccagcagcctgagcgccagcgtgggcgaccgcgtgaccatcacctgccgcagcagcaccggcgccgtgaccaccagcaactacgccagctgggtgcaggagaagcccggcaagctgttcaagggcctgatcggcggcaccaacaaccgcgcccccggcgtgcccagccgcttcagcggcagcctgatcggcgacaaggccaccctgaccatcagcagcctgcagcccgaggacttcgccacctacttctgcgccctgtggtacagcaaccactgggtgttcggccagggcaccaaggtggagctgaagcgcggcggcggcggcagcggcggcggcggcagcggcggcggcggcagcagcggcggcggcagcgaggtgaagctgctggagagcggcggcggcctggtgcagcccggcggcagcctgaagctgagctgcgccgtgagcggcttcagcctgaccgactacggcgtgaactgggtgcgccaggcccccggccgcggcctggagtggatcggcgtgatctggggcgacggcatcaccgactacaacagcgccctgaaggaccgcttcatcatcagcaaggacaacggcaagaacaccgtgtacctgcagatgagcaaggtgcgcagcgacgacaccgccctgtactactgcgtgaccggcctgttcgactactggggccagggcaccctggtgaccgtgagcagctacccatacgatgttccagattacgctggtggaggcggaggttctgggggaggaggtagtggcggtggtggttcaggaggcggcggaagcttggatccaggtggaggtggaagcggtgtgactttcgacgatgtggccgtgacctttaccaaagaagagtggggccagctggatctggcccagagaacactgtaccaagaagttatgctggagaactgcggcctgctggtgtctctgggatgtcctgtgcctaaggccgagctgatctgccacctggaacacggacaagagccttggaccggaagcggaaagcgcaccgccgatggttccgagttcgaaagccccaaaaaaaagcgcaaggtc

SEQ ID NO: 175 - DNA, 1104 bp, synthetic construct
  misc_feature 1..1104: note = DNA of 2nd fusion_scFv-Znf582
  source 1..1104: mol_type = other DNA
atgggccccgacatcgtgatgacccagagccccagcagcctgagcgccagcgtgggcgaccgcgtgaccatcacctgccgcagcagcaccggcgccgtgaccaccagcaactacgccagctgggtgcaggagaagcccggcaagctgttcaagggcctgatcggcggcaccaacaaccgcgcccccggcgtgcccagccgcttcagcggcagcctgatcggcgacaaggccaccctgaccatcagcagcctgcagcccgaggacttcgccacctacttctgcgccctgtggtacagcaaccactgggtgttcggccagggcaccaaggtggagctgaagcgcggcggcggcggcagcggcggcggcggcagcggcggcggcggcagcagcggcggcggcagcgaggtgaagctgctggagagcggcggcggcctggtgcagcccggcggcagcctgaagctgagctgcgccgtgagcggcttcagcctgaccgactacggcgtgaactgggtgcgccaggcccccggccgcggcctggagtggatcggcgtgatctggggcgacggcatcaccgactacaacagcgccctgaaggaccgcttcatcatcagcaaggacaacggcaagaacaccgtgtacctgcagatgagcaaggtgcgcagcgacgacaccgccctgtactactgcgtgaccggcctgttcgactactggggccagggcaccctggtgaccgtgagcagctacccatacgatgttccagattacgctggtggaggcggaggttctgggggaggaggtagtggcggtggtggttcaggaggcggcggaagcttggatccaggtggaggtggaagcggtgagctgttccgcgacgtggccattgtgttctctcaagaggaatggcagtggctggcccctgctcagagagatctctaccgcgacgttatgctggagacatactccaatctcgtgtccctcggcctggccgtgtccaaacctgatgtgatcagcttcctcgagcagggaaaagaaccttggatgggaagcggaaagcgcaccgccgatggttccgagttcgaaagccccaaaaaaaagcgcaaggtc

SEQ ID NO: 176 - DNA, 1104 bp, synthetic construct
  misc_feature 1..1104: note = DNA of 2nd fusion_scFv-Znf324
  source 1..1104: mol_type = other DNA
atgggccccgacatcgtgatgacccagagccccagcagcctgagcgccagcgtgggcgaccgcgtgaccatcacctgccgcagcagcaccggcgccgtgaccaccagcaactacgccagctgggtgcaggagaagcccggcaagctgttcaagggcctgatcggcggcaccaacaaccgcgcccccggcgtgcccagccgcttcagcggcagcctgatcggcgacaaggccaccctgaccatcagcagcctgcagcccgaggacttcgccacctacttctgcgccctgtggtacagcaaccactgggtgttcggccagggcaccaaggtggagctgaagcgcggcggcggcggcagcggcggcggcggcagcggcggcggcggcagcagcggcggcggcagcgaggtgaagctgctggagagcggcggcggcctggtgcagcccggcggcagcctgaagctgagctgcgccgtgagcggcttcagcctgaccgactacggcgtgaactgggtgcgccaggcccccggccgcggcctggagtggatcggcgtgatctggggcgacggcatcaccgactacaacagcgccctgaaggaccgcttcatcatcagcaaggacaacggcaagaacaccgtgtacctgcagatgagcaaggtgcgcagcgacgacaccgccctgtactactgcgtgaccggcctgttcgactactggggccagggcaccctggtgaccgtgagcagctacccatacgatgttccagattacgctggtggaggcggaggttctgggggaggaggtagtggcggtggtggttcaggaggcggcggaagcttggatccaggtggaggtggaagcggtatggcctttgaggacgtcgccgtgtatttttcccaagaagaatggggactgctcgacactgcccagagagccctgtatcgcagagtcatgctggacaacttcgccctggtggcctccctgggcctgtctacaagcagacccagagtggtcattcagctggaaagaggcgaggaaccctgggtcggaagcggaaagcgcaccgccgatggttccgagttcgaaagccccaaaaaaaagcgcaaggtc

SEQ ID NO: 177 - DNA, 1107 bp, synthetic construct
  misc_feature 1..1107: note = DNA of 2nd fusion_scFv-Znf669
  source 1..1107: mol_type = other DNA
atgggccccgacatcgtgatgacccagagccccagcagcctgagcgccagcgtgggcgaccgcgtgaccatcacctgccgcagcagcaccggcgccgtgaccaccagcaactacgccagctgggtgcaggagaagcccggcaagctgttcaagggcctgatcggcggcaccaacaaccgcgcccccggcgtgcccagccgcttcagcggcagcctgatcggcgacaaggccaccctgaccatcagcagcctgcagcccgaggacttcgccacctacttctgcgccctgtggtacagcaaccactgggtgttcggccagggcaccaaggtggagctgaagcgcggcggcggcggcagcggcggcggcggcagcggcggcggcggcagcagcggcggcggcagcgaggtgaagctgctggagagcggcggcggcctggtgcagcccggcggcagcctgaagctgagctgcgccgtgagcggcttcagcctgaccgactacggcgtgaactgggtgcgccaggcccccggccgcggcctggagtggatcggcgtgatctggggcgacggcatcaccgactacaacagcgccctgaaggaccgcttcatcatcagcaaggacaacggcaagaacaccgtgtacctgcagatgagcaaggtgcgcagcgacgacaccgccctgtactactgcgtgaccggcctgttcgactactggggccagggcaccctggtgaccgtgagcagctacccatacgatgttccagattacgctggtggaggcggaggttctgggggaggaggtagtggcggtggtggttcaggaggcggcggaagcttggatccaggtggaggtggaagcggtgtcgcctttgaagatgtggctgtgaatttcacccaagaagagtgggctctgctggacagcagccagaagaatctctaccgcgaagtgatgcaagagacatgccggaacctggcctctgtgggctctcagtggaaggaccagaacatcgaggaccacttcgagaagcccggcaaggacatcagaaacggaagcggaaagcgcaccgccgatggttccgagttcgaaagccccaaaaaaaagcgcaaggtc

SEQ ID NO: 178 - DNA, 1104 bp, synthetic construct
  misc_feature 1..1104: note = DNA of 2nd fusion_scFv-Znf354a
  source 1..1104: mol_type = other DNA
atgggccccgacatcgtgatgacccagagccccagcagcctgagcgccagcgtgggcgaccgcgtgaccatcacctgccgcagcagcaccggcgccgtgaccaccagcaactacgccagctgggtgcaggagaagcccggcaagctgttcaagggcctgatcggcggcaccaacaaccgcgcccccggcgtgcccagccgcttcagcggcagcctgatcggcgacaaggccaccctgaccatcagcagcctgcagcccgaggacttcgccacctacttctgcgccctgtggtacagcaaccactgggtgttcggccagggcaccaaggtggagctgaagcgcggcggcggcggcagcggcggcggcggcagcggcggcggcggcagcagcggcggcggcagcgaggtgaagctgctggagagcggcggcggcctggtgcagcccggcggcagcctgaagctgagctgcgccgtgagcggcttcagcctgaccgactacggcgtgaactgggtgcgccaggcccccggccgcggcctggagtggatcggcgtgatctggggcgacggcatcaccgactacaacagcgccctgaaggaccgcttcatcatcagcaaggacaacggcaagaacaccgtgtacctgcagatgagcaaggtgcgcagcgacgacaccgccctgtactactgcgtgaccggcctgttcgactactggggccagggcaccctggtgaccgtgagcagctacccatacgatgttccagattacgctggtggaggcggaggttctgggggaggaggtagtggcggtggtggttcaggaggcggcggaagcttggatccaggtggaggtggaagcggtctgacattcgaagatgtcgcagtgctgttcacccgggacgagtggaggaaactggctcccagccagcgcaatctgtatagagatgtgatgctggagaattacagaaatctcgtcagcctggggctgcccttcaccaagcctaaagtgatcagcctgctgcaacaaggcgaggatccttgggaaggaagcggaaagcgcaccgccgatggttccgagttcgaaagccccaaaaaaaagcgcaaggtc

SEQ ID NO: 179 - DNA, 1104 bp, synthetic construct
  misc_feature 1..1104: note = DNA of 2nd fusion_scFv-Znf82
  source 1..1104: mol_type = other DNA
atgggccccgacatcgtgatgacccagagccccagcagcctgagcgccagcgtgggcgaccgcgtgaccatcacctgccgcagcagcaccggcgccgtgaccaccagcaactacgccagctgggtgcaggagaagcccggcaagctgttcaagggcctgatcggcggcaccaacaaccgcgcccccggcgtgcccagccgcttcagcggcagcctgatcggcgacaaggccaccctgaccatcagcagcctgcagcccgaggacttcgccacctacttctgcgccctgtggtacagcaaccactgggtgttcggccagggcaccaaggtggagctgaagcgcggcggcggcggcagcggcggcggcggcagcggcggcggcggcagcagcggcggcggcagcgaggtgaagctgctggagagcggcggcggcctggtgcagcccggcggcagcctgaagctgagctgcgccgtgagcggcttcagcctgaccgactacggcgtgaactgggtgcgccaggcccccggccgcggcctggagtggatcggcgtgatctggggcgacggcatcaccgactacaacagcgccctgaaggaccgcttcatcatcagcaaggacaacggcaagaacaccgtgtacctgcagatgagcaaggtgcgcagcgacgacaccgccctgtactactgcgtgaccggcctgttcgactactggggccagggcaccctggtgaccgtgagcagctacccatacgatgttccagattacgctggtggaggcggaggttctgggggaggaggtagtggcggtggtggttcaggaggcggcggaagcttggatccaggtggaggtggaagcggtgttatgttctccgacgtgtccatcgactttagccccgaagagtgggagtatctggacctggaacagaaggatctgtatcgcgacgtgatgctcgagaattactctaacctggtgagcctgggctgcttcatcagcaagcccgatgtgatctctagcctggagcaaggcaaagagccatggaaaggaagcggaaagcgcaccgccgatggttccgagttcgaaagccccaaaaaaaagcgcaaggtc

SEQ ID NO: 180 - DNA, 1224 bp, synthetic construct
  misc_feature 1..1224: note = DNA of 2nd fusion_scFv-Znf595
  source 1..1224: mol_type = other DNA
atgggccccgacatcgtgatgacccagagccccagcagcctgagcgccagcgtgggcgaccgcgtgaccatcacctgccgcagcagcaccggcgccgtgaccaccagcaactacgccagctgggtgcaggagaagcccggcaagctgttcaagggcctgatcggcggcaccaacaaccgcgcccccggcgtgcccagccgcttcagcggcagcctgatcggcgacaaggccaccctgaccatcagcagcctgcagcccgaggacttcgccacctacttctgcgccctgtggtacagcaaccactgggtgttcggccagggcaccaaggtggagctgaagcgcggcggcggcggcagcggcggcggcggcagcggcggcggcggcagcagcggcggcggcagcgaggtgaagctgctggagagcggcggcggcctggtgcagcccggcggcagcctgaagctgagctgcgccgtgagcggcttcagcctgaccgactacggcgtgaactgggtgcgccaggcccccggccgcggcctggagtggatcggcgtgatctggggcgacggcatcaccgactacaacagcgccctgaaggaccgcttcatcatcagcaaggacaacggcaagaacaccgtgtacctgcagatgagcaaggtgcgcagcgacgacaccgccctgtactactgcgtgaccggcctgttcgactactggggccagggcaccctggtgaccgtgagcagctacccatacgatgttccagattacgctggtggaggcggaggttctgggggaggaggtagtggcggtggtggttcaggaggcggcggaagcttggatccaggtggaggtggaagcggtgtcaccttccgggacgtcgcaatcgaattcagccccgaggaatggaaatgtctggaccccgcacagcaaaacctctacagagatgtcatgctcgaaaactataggaacctggtctccctgggcttcgtgatcagcaaccctgatctcgtgacctgcctcgaacagatcaaagagccctgcaacgtcaccttccgggacgtcgcaatcgaattcagccccgaggaatggaaatgtctggaccccgcacagcaaaacctctacagagatgtcatgctcgaaaactataggaacctggtctccctgggcttcgtgatcagcaaccctgatctcgtgacctgcctcgaacagatcaaagagccctgcaac

SEQ ID NO: 181 - DNA, 1104 bp, synthetic construct
  misc_feature 1..1104: note = DNA of 2nd fusion_scFv-Znf419
  source 1..1104: mol_type = other DNA
atgggccccgacatcgtgatgacccagagccccagcagcctgagcgccagcgtgggcgaccgcgtgaccatcacctgccgcagcagcaccggcgccgtgaccaccagcaactacgccagctgggtgcaggagaagcccggcaagctgttcaagggcctgatcggcggcaccaacaaccgcgcccccggcgtgcccagccgcttcagcggcagcctgatcggcgacaaggccaccctgaccatcagcagcctgcagcccgaggacttcgccacctacttctgcgccctgtggtacagcaaccactgggtgttcggccagggcaccaaggtggagctgaagcgcggcggcggcggcagcggcggcggcggcagcggcggcggcggcagcagcggcggcggcagcgaggtgaagctgctggagagcggcggcggcctggtgcagcccggcggcagcctgaagctgagctgcgccgtgagcggcttcagcctgaccgactacggcgtgaactgggtgcgccaggcccccggccgcggcctggagtggatcggcgtgatctggggcgacggcatcaccgactacaacagcgccctgaaggaccgcttcatcatcagcaaggacaacggcaagaacaccgtgtacctgcagatgagcaaggtgcgcagcgacgacaccgccctgtactactgcgtgaccggcctgttcgactactggggccagggcaccctggtgaccgtgagcagctacccatacgatgttccagattacgctggtggaggcggaggttctgggggaggaggtagtggcggtggtggttcaggaggcggcggaagcttggatccaggtggaggtggaagcggtgttaccttcgaagatgttgccgtgtacttcagccaagaagagtggcggctgctggatgacgcccagagactgctgtatcggaatgttatgctcgaaaacttcaccctgctggcttccctgggactcgccagctctaagacccacgagattacccagctggaatcctgggaagaacccttcatgggaagcggaaagcgcaccgccgatggttccgagttcgaaagccccaaaaaaaagcgcaaggtc

SEQ ID NO: 182 - DNA, 1104 bp, synthetic construct
  misc_feature 1..1104: note = DNA of 2nd fusion_scFv-Znf566
  source 1..1104: mol_type = other DNA
atgggccccgacatcgtgatgacccagagccccagcagcctgagcgccagcgtgggcgaccgcgtgaccatcacctgccgcagcagcaccggcgccgtgaccaccagcaactacgccagctgggtgcaggagaagcccggcaagctgttcaagggcctgatcggcggcaccaacaaccgcgcccccggcgtgcccagccgcttcagcggcagcctgatcggcgacaaggccaccctgaccatcagcagcctgcagcccgaggacttcgccacctacttctgcgccctgtggtacagcaaccactgggtgttcggccagggcaccaaggtggagctgaagcgcggcggcggcggcagcggcggcggcggcagcggcggcggcggcagcagcggcggcggcagcgaggtgaagctgctggagagcggcggcggcctggtgcagcccggcggcagcctgaagctgagctgcgccgtgagcggcttcagcctgaccgactacggcgtgaactgggtgcgccaggcccccggccgcggcctggagtggatcggcgtgatctggggcgacggcatcaccgactacaacagcgccctgaaggaccgcttcatcatcagcaaggacaacggcaagaacaccgtgtacctgcagatgagcaaggtgcgcagcgacgacaccgccctgtactactgcgtgaccggcctgttcgactactggggccagggcaccctggtgaccgtgagcagctacccatacgatgttccagattacgctggtggaggcggaggttctgggggaggaggtagtggcggtggtggttcaggaggcggcggaagcttggatccaggtggaggtggaagcggtgtcatgttcagcgacgtgtccgtggactttagccaagaggaatgggaatgcctgaacgacgaccagcgggacctctatagggatgtcatgctcgagaactacagcaatctcgtttccatgggccacagcatctccaagccaaacgtcatcagctatctcgaacaaggcaaagagccctggctgggaagcggaaagcgcaccgccgatggttccgagttcgaaagccccaaaaaaaagcgcaaggtc

SEQ ID NO: 183 - DNA, 1104 bp, synthetic construct
  misc_feature 1..1104: note = DNA of 2nd fusion_scFv-Zim2
  source 1..1104: mol_type = other DNA
atgggccccgacatcgtgatgacccagagccccagcagcctgagcgccagcgtgggcgaccgcgtgaccatcacctgccgcagcagcaccggcgccgtgaccaccagcaactacgccagctgggtgcaggagaagcccggcaagctgttcaagggcctgatcggcggcaccaacaaccgcgcccccggcgtgcccagccgcttcagcggcagcctgatcggcgacaaggccaccctgaccatcagcagcctgcagcccgaggacttcgccacctacttctgcgccctgtggtacagcaaccactgggtgttcggccagggcaccaaggtggagctgaagcgcggcggcggcggcagcggcggcggcggcagcggcggcggcggcagcagcggcggcggcagcgaggtgaagctgctggagagcggcggcggcctggtgcagcccggcggcagcctgaagctgagctgcgccgtgagcggcttcagcctgaccgactacggcgtgaactgggtgcgccaggcccccggccgcggcctggagtggatcggcgtgatctggggcgacggcatcaccgactacaacagcgccctgaaggaccgcttcatcatcagcaaggacaacggcaagaacaccgtgtacctgcagatgagcaaggtgcgcagcgacgacaccgccctgtactactgcgtgaccggcctgttcgactactggggccagggcaccctggtgaccgtgagcagctacccatacgatgttccagattacgctggtggaggcggaggttctgggggaggaggtagtggcggtggtggttcaggaggcggcggaagcttggatccaggtggaggtggaagcggtgtcaccttcgaggatgtgctggtggatttcagccctgaggaactgagcagcctgtccgccgcacagagaaatctctatcgggaagtgatgctggagaactatcggaatctggtgtctctgggccaccagttcagcaagcctgacatcatcagcagactggaagaagaggaatcctacgccatgggaagcggaaagcgcaccgccgatggttccgagttcgaaagccccaaaaaaaagcgcaaggtc

SEQ ID NO: 184 - DNA, 2072 bp, synthetic construct
  misc_feature 1..2072: note = DNA of 2nd fusion_scFv-EHMT2(G9A)
  source 1..2072: mol_type = other DNA
atgggccccgacatcgtgatgacccagagccccagcagcctgagcgccagcgtgggcgaccgcgtgaccatcacctgccgcagcagcaccggcgccgtgaccaccagcaactacgccagctgggtgcaggagaagcccggcaagctgttcaagggcctgatcggcggcaccaacaaccgcgcccccggcgtgcccagccgcttcagcggcagcctgatcggcgacaaggccaccctgaccatcagcagcctgcagcccgaggacttcgccacctacttctgcgccctgtggtacagcaaccactgggtgttcggccagggcaccaaggtggagctgaagcgcggcggcggcggcagcggcggcggcggcagcggcggcggcggcagcagcggcggcggcagcgaggtgaagctgctggagagcggcggcggcctggtgcagcccggcggcagcctgaagctgagctgcgccgtgagcggcttcagcctgaccgactacggcgtgaactgggtgcgccaggcccccggccgcggcctggagtggatcggcgtgatctggggcgacggcatcaccgactacaacagcgccctgaaggaccgcttcatcatcagcaaggacaacggcaagaacaccgtgtacctgcagatgagcaaggtgcgcagcgacgacaccgccctgtactactgcgtgaccggcctgttcgactactggggccagggcaccctggtgaccgtgagcagctacccatacgatgttccagattacgctggtggaggcggaggttctgggggaggaggtagtggcggtggtggttcaggaggcggcggaagcttggatccaggtggaggtggaagcggttcacgggcagcgccgccatcgccgaagtccttctgaatgcgcgctgtgacctccatgctgtcaactaccatggggacacccccctgcacatcgcagctcgggagagctaccatgactgcgtgctgttattcctgtcacgtggggccaaccctgagctgcggaacaaagagggggacacagcatgggacctgactcccgagcgctccgacgtgtggtttgcgcttcaactcaaccgcaagctccgacttggggtgggaaatcgggccatccgcacagagaagatcatctgccgggacgtggctcggggctatgagaacgtgcccattccctgtgtcaacggtgtggatggggagccctgccctgaggattacaagtacatctcagagaactgcgagacgtccaccatgaacatcgatcgcaacatcacccacctgcagcactgcacgtgtgtggacgactgctctagctccaactgcctgtgcggccagctcagcatccggtgctggtatgacaaggatgggcgattgctccaggaatttaacaagattgagcctccgctgattttcgagtgtaaccaggcgtgctcatgctggagaaactgcaagaaccgggtcgtacagagtggcatcaaggtgcggctacagctctaccgaacagccaagatgggctggggggtccgcgccctgcagaccatcccacaggggaccttcatctgcgagtatgtcggggagctgatctctgatgctgaggctgatgtgagagaggatgattcttacctcttcgacttagacaacaaggatggagaggtgtactgcatagatgcccgttactatggcaacatcagccgcttcatcaaccacctgtgtgaccccaacatcattcccgtccgggtcttcatgctgcaccaagacctgcgatttccacgcatcgccttcttcagttcccgagacatccggactggggaggagctagggtttgactatggcgaccgcttctgggacatcaaaagcaaatatttcacctgccaatgtggctctgagaagtgcaagcactcagccgaagccattgccctggagcagagccgtctggcccgcctggacccacaccctgagctgctgcccgagctcggctccctgccccctgtcaacacaggaagcggaaagcgcaccgccgatggttccgagttcgaaagccccaaaaaaaagcgcaaggtc

SEQ ID NO: 185 - DNA, 2154 bp, synthetic construct
  misc_feature 1..2154: note = DNA of 2nd fusion_scFv-SUV39H1
  source 1..2154: mol_type = other DNA
atgggccccgacatcgtgatgacccagagccccagcagcctgagcgccagcgtgggcgaccgcgtgaccatcacctgccgcagcagcaccggcgccgtgaccaccagcaactacgccagctgggtgcaggagaagcccggcaagctgttcaagggcctgatcggcggcaccaacaaccgcgcccccggcgtgcccagccgcttcagcggcagcctgatcggcgacaaggccaccctgaccatcagcagcctgcagcccgaggacttcgccacctacttctgcgccctgtggtacagcaaccactgggtgttcggccagggcaccaaggtggagctgaagcgcggcggcggcggcagcggcggcggcggcagcggcggcggcggcagcagcggcggcggcagcgaggtgaagctgctggagagcggcggcggcctggtgcagcccggcggcagcctgaagctgagctgcgccgtgagcggcttcagcctgaccgactacggcgtgaactgggtgcgccaggcccccggccgcggcctggagtggatcggcgtgatctggggcgacggcatcaccgactacaacagcgccctgaaggaccgcttcatcatcagcaaggacaacggcaagaacaccgtgtacctgcagatgagcaaggtgcgcagcgacgacaccgccctgtactactgcgtgaccggcctgttcgactactggggccagggcaccctggtgaccgtgagcagctacccatacgatgttccagattacgctggtggaggcggaggttctgggggaggaggtagtggcggtggtggttcaggaggcggcggaagcttggatccaggtggaggtggaagcggtgcggaaaatttaaaaggctgcagcgtgtgttgcaagtcttcttggaatcagctgcaggacctgtgccgcctggccaagctctcctgccctgccctcggtatctctaagaggaacctctatgactttgaagtcgagtacctgtgcgattacaagaagatccgcgaacaggaatattacctggtgaaatggcgtggatatccagactcagagagcacctgggagccacggcagaatctcaagtgtgtgcgtatcctcaagcagttccacaaggacttagaaagggagctgctccggcggcaccaccggtcaaagaccccccggcacctggacccaagcttggccaactacctggtgcagaaggccaagcagaggcgggcgctccgtcgctgggagcaggagctcaatgccaagcgcagccatctgggacgcatcactgtagagaatgaggtggacctggacggccctccgcgggccttcgtgtacatcaatgagtaccgtgttggtgagggcatcaccctcaaccaggtggctgtgggctgcgagtgccaggactgtctgtgggcacccactggaggctgctgcccgggggcgtcactgcacaagtttgcctacaatgaccagggccaggtgcggcttcgagccgggctgcccatctacgagtgcaactcccgctgccgctgcggctatgactgcccaaatcgtgtggtacagaagggtatccgatatgacctctgcatcttccgcacggatgatgggcgtggctggggcgtccgcaccctggagaagattcgcaagaacagcttcgtcatggagtacgtgggagagatcattacctcagaggaggcagagcggcggggccagatctacgaccgtcagggcgccacctacctctttgacctggactacgtggaggacgtgtacaccgtggatgccgcctactatggcaacatctcccactttgtcaaccacagttgtgaccccaacctgcaggtgtacaacgtcttcatagacaaccttgacgagcggctgccccgcatcgctttctttgccacaagaaccatccgggcaggcgaggagctcacctttgattacaacatgcaagtggaccccgtggacatggagagcacccgcatggactccaactttggcctggctgggctccctggctcccctaagaagcgggtccgtattgaatgcaagtgtgggactgagtcctgccgcaaatacctcttcggaagcggaaagcgcaccgccgatggttccgagttcgaaagccccaaaaaaaagcgcaaggtc

SEQ ID NO: 186 - DNA, 1064 bp, synthetic construct
  misc_feature 1..1064: note = DNA of 2nd fusion_scFv-ZFPM1(FOG)
  source 1..1064: mol_type = other DNA
atgggccccgacatcgtgatgacccagagccccagcagcctgagcgccagcgtgggcgaccgcgtgaccatcacctgccgcagcagcaccggcgccgtgaccaccagcaactacgccagctgggtgcaggagaagcccggcaagctgttcaagggcctgatcggcggcaccaacaaccgcgcccccggcgtgcccagccgcttcagcggcagcctgatcggcgacaaggccaccctgaccatcagcagcctgcagcccgaggacttcgccacctacttctgcgccctgtggtacagcaaccactgggtgttcggccagggcaccaaggtggagctgaagcgcggcggcggcggcagcggcggcggcggcagcggcggcggcggcagcagcggcggcggcagcgaggtgaagctgctggagagcggcggcggcctggtgcagcccggcggcagcctgaagctgagctgcgccgtgagcggcttcagcctgaccgactacggcgtgaactgggtgcgccaggcccccggccgcggcctggagtggatcggcgtgatctggggcgacggcatcaccgactacaacagcgccctgaaggaccgcttcatcatcagcaaggacaacggcaagaacaccgtgtacctgcagatgagcaaggtgcgcagcgacgacaccgccctgtactactgcgtgaccggcctgttcgactactggggccagggcaccctggtgaccgtgagcagctacccatacgatgttccagattacgctggtggaggcggaggttctgggggaggaggtagtggcggtggtggttcaggaggcggcggaagcttggatccaggtggaggtggaagcggttccaggcggaaacagagcaacccccggcagatcaagcgttccctcggagacatggaggccagagaggaggtgcagttggtgggtgccagccacatggagcaaaaggccacggcacctgaagccccgagccctcccagcgcagaggaagcggaaagcgcaccgccgatggttccgagttcgaaagccccaaaaaaaagcgcaaggtc

SEQ ID NO: 187 - DNA, 3423 bp, synthetic construct
  misc_feature 1..3423: note = DNA of 2nd fusion_scFv-TRIM28(KAP1)
  source 1..3423: mol_type = other DNA
atgggccccgacatcgtgatgacccagagccccagcagcctgagcgccagcgtgggcgaccgcgtgaccatcacctgccgcagcagcaccggcgccgtgaccaccagcaactacgccagctgggtgcaggagaagcccggcaagctgttcaagggcctgatcggcggcaccaacaaccgcgcccccggcgtgcccagccgcttcagcggcagcctgatcggcgacaaggccaccctgaccatcagcagcctgcagcccgaggacttcgccacctacttctgcgccctgtggtacagcaaccactgggtgttcggccagggcaccaaggtggagctgaagcgcggcggcggcggcagcggcggcggcggcagcggcggcggcggcagcagcggcggcggcagcgaggtgaagctgctggagagcggcggcggcctggtgcagcccggcggcagcctgaagctgagctgcgccgtgagcggcttcagcctgaccgactacggcgtgaactgggtgcgccaggcccccggccgcggcctggagtggatcggcgtgatctggggcgacggcatcaccgactacaacagcgccctgaaggaccgcttcatcatcagcaaggacaacggcaagaacaccgtgtacctgcagatgagcaaggtgcgcagcgacgacaccgccctgtactactgcgtgaccggcctgttcgactactggggccagggcaccctggtgaccgtgagcagctacccatacgatgttccagattacgctggtggaggcggaggttctgggggaggaggtagtggcggtggtggttcaggaggcggcggaagcttggatccaggtggaggtggaagcggtgcggcctccgcggcggcagcctcggcagcagcggcctcggccgcctctggcagcccgggcccgggcgagggctccgctggcggcgaaaagcgctccaccgccccttcggccgcagcctcggcctctgcctcagccgcggcgtcgtcgcccgcggggggcggcgccgaggcgctggagctgctggagcactgcggcgtgtgcagagagcgcctgcgacccgagagggagccccgcctgctgccctgtttgcactcggcctgtagtgcctgcttagggcccgcggcccccgccgccgccaacagctcgggggacggcggggcggcgggcgacggcaccgtggtggactgtcccgtgtgcaagcaacagtgcttctccaaagacatcgtggagaattatttcatgcgtgatagtggcagcaaggctgccaccgacgcccaggatgcgaaccagtgctgcactagctgtgaggataatgccccagccaccagctactgtgtggagtgctcggagcctctgtgtgagacctgtgtagaggcgcaccagcgggtgaagtacaccaaggaccatactgtgcgctctactgggccagccaagtctcgggatggtgaacgtactgtctattgcaacgtacacaagcatgaaccccttgtgctgttttgtgagagctgtgatactctcacctgccgagactgccagctcaatgcccacaaggaccaccagtaccagttcttagaggatgcagtgaggaaccagcgcaagctcctggcctcactggtgaagcgccttggggacaaacatgcaacattgcagaagagcaccaaggaggttcgcagctcaatccgccaggtgtctgacgtacagaagcgtgtgcaagtggatgtcaagatggccatcctgcagatcatgaaggagctgaataagcggggccgtgtgctggtcaatgatgcccagaaggtgactgaggggcagcaggagcgcctggagcggcagcactggaccatgaccaagatccagaagcaccaggagcacattctgcgctttgcctcttgggctctggagagtgacaacaacacagcccttttgctttctaagaagttgatctacttccagctgcaccgggccctcaagatgattgtggatcccgtggagccacatggcgagatgaagtttcagtgggacctcaatgcctggaccaagagtgccgaggcctttggcaagattgtggcagagcgtcctggcactaactcaacaggccctgcacccatggcccctccaagagccccagggcccctgagcaagcagggctctggcagcagccagcccatggaggtgcaggaaggctatggctttgggtcaggagatgatccctactcaagtgcagagccccatgtgtcaggtgtgaaacggtcccgctcaggtgagggcgaggtgagcggccttatgcgcaaggtgccacgagtgagccttgaacgcctggacctggacctcacagctgacagccagccacccgtcttcaaggtcttcccaggcagtaccactgaggactacaaccttattgttattgaacgtggcgctgccgctgcagctaccggccagccagggactgcgcctgcaggaacccctggtgccccacccctggctggcatggccattgtcaaggaggaggagacggaggctgccattggagcccctcctactgccactgagggccctgagaccaaacctgtgcttatggctcttgcggagggtcctggtgctgagggtccccgcctggcctcacctagtggcagcaccagctcagggctggaggtggtggctcctgagggtacctcagccccaggtggtggcccgggaaccctggatgacagtgccaccatttgccgtgtctgccagaagccaggcgatctggttatgtgcaaccagtgtgagttttgtttccacctggactgtcacctgccggccctgcaggatgtaccaggggaggagtggagctgctcactctgccatgtgctccctgacctgaaggaggaggatggcagcctcagcctggatggtgcagacagcactggcgtggtggccaagctctcaccagccaaccagcggaaatgtgagcgtgtactgctggccctattctgtcacgaaccctgccgccccctgcatcagctggctaccgactccaccttctccctggaccagcccggtggcaccctggatctgaccctgatccgtgcccgcctccaggagaagttgtcacctccctacagctccccacaggagtttgcccaggatgtgggccgcatgttcaagcaattcaacaagttaactgaggacaaggcagacgtgcagtccatcatcggcctgcagcgcttcttcgagacgcgcatgaacgaggccttcggtgacaccaagttctctgctgtgctggtggagcccccgccgatgagcctgcctggtgctggcctgagttcccaggagctgtctggtggccctggtgatggccccggaagcggaaagcgcaccgccgatggttccgagttcgaaagccccaaaaaaaagcgcaaggtc

SEQ ID NO: 188 - DNA, 3156 bp, synthetic construct
  misc_feature 1..3156: note = DNA of 2nd fusion_scFv-EZH2
  source 1..3156: mol_type = other DNA
atgggccccgacatcgtgatgacccagagccccagcagcctgagcgccagcgtgggcgaccgcgtgaccatcacctgccgcagcagcaccggcgccgtgaccaccagcaactacgccagctgggtgcaggagaagcccggcaagctgttcaagggcctgatcggcggcaccaacaaccgcgcccccggcgtgcccagccgcttcagcggcagcctgatcggcgacaaggccaccctgaccatcagcagcctgcagcccgaggacttcgccacctacttctgcgccctgtggtacagcaaccactgggtgttcggccagggcaccaaggtggagctgaagcgcggcggcggcggcagcggcggcggcggcagcggcggcggcggcagcagcggcggcggcagcgaggtgaagctgctggagagcggcggcggcctggtgcagcccggcggcagcctgaagctgagctgcgccgtgagcggcttcagcctgaccgactacggcgtgaactgggtgcgccaggcccccggccgcggcctggagtggatcggcgtgatctggggcgacggcatcaccgactacaacagcgccctgaaggaccgcttcatcatcagcaaggacaacggcaagaacaccgtgtacctgcagatgagcaaggtgcgcagcgacgacaccgccctgtactactgcgtgaccggcctgttcgactactggggccagggcaccctggtgaccgtgagcagctacccatacgatgttccagattacgctggtggaggcggaggttctgggggaggaggtagtggcggtggtggttcaggaggcggcggaagcttggatccaggtggaggtggaagcggtggccagactgggaagaaatctgagaagggaccagtttgttggcggaagcgtgtaaaatcagagtacatgcgactgagacagctcaagaggttcagacgagctgatgaagtaaagagtatgtttagttccaatcgtcagaaaattttggaaagaacggaaatcttaaaccaagaatggaaacagcgaaggatacagcctgtgcacatcctgacttctgtgagctcattgcgcgggactagggagtgttcggtgaccagtgacttggattttccaacacaagtcatcccattaaagactctgaatgcagttgcttcagtacccataatgtattcttggtctcccctacagcagaattttatggtggaagatgaaactgttttacataacattccttatatgggagatgaagttttagatcaggatggtactttcattgaagaactaataaaaaattatgatgggaaagtacacggggatagagaatgtgggtttataaatgatgaaatttttgtggagttggtgaatgcccttggtcaatataatgatgatgacgatgatgatgatggagacgatcctgaagaaagagaagaaaagcagaaagatctggaggatcaccgagatgataaagaaagccgcccacctcggaaatttccttctgataaaatttttgaagccatttcctcaatgtttccagataagggcacagcagaagaactaaaggaaaaatataaagaactcaccgaacagcagctcccaggcgcacttcctcctgaatgtacccccaacatagatggaccaaatgctaaatctgttcagagagagcaaagcttacactcctttcatacgcttttctgtaggcgatgttttaaatatgactgcttcctacatccttttcatgcaacacccaacacttataagcggaagaacacagaaacagctctagacaacaaaccttgtggaccacagtgttaccagcatttggagggagcaaaggagtttgctgctgctctcaccgctgagcggataaagaccccaccaaaacgtccaggaggccgcagaagaggacggcttcccaataacagtagcaggcccagcacccccaccattaatgtgctggaatcaaaggatacagacagtgatagggaagcagggactgaaacggggggagagaacaatgataaagaagaagaagagaagaaagatgaaacttcgagctcctctgaagcaaattctcggtgtcaaacaccaataaagatgaagccaaatattgaacctcctgagaatgtggagtggagtggtgctgaagcctcaatgtttagagtcctcattggcacttactatgacaatttctgtgccattgctaggttaattgggaccaaaacatgtagacaggtgtatgagtttagagtcaaagaatctagcatcatagctccagctcccgctgaggatgtggatactcctccaaggaaaaagaagaggaaacaccggttgtgggctgcacactgcagaaagatacagctgaaaaaggacggctcctctaaccatgtttacaactatcaaccctgtgatcatccacggcagccttgtgacagttcgtgcccttgtgtgatagcacaaaatttttgtgaaaagttttgtcaatgtagttcagagtgtcaaaaccgctttccgggatgccgctgcaaagcacagtgcaacaccaagcagtgcccgtgctacctggctgtccgagagtgtgaccctgacctctgtcttacttgtggagccgctgaccattgggacagtaaaaatgtgtcctgcaagaactgcagtattcagcggggctccaaaaagcatctattgctggcaccatctgacgtggcaggctgggggatttttatcaaagatcctgtgcagaaaaatgaattcatctcagaatactgtggagagattatttctcaagatgaagctgacagaagagggaaagtgtatgataaatacatgtgcagctttctgttcaacttgaacaatgattttgtggtggatgcaacccgcaagggtaacaaaattcgttttgcaaatcattcggtaaatccaaactgctatgcaaaagttatgatggttaacggtgatcacaggataggtatttttgccaagagagccatccagactggcgaagagctgttttttgattacagatacagccaggctgatgccctgaagtatgtcggcatcgaaagagaaatggaaatccctggaagcggaaagcgcaccgccgatggttccgagttcgaaagccccaaaaaaaagcgcaaggtc

SEQ ID NO: 189 - DNA, 1578 bp, synthetic construct
  misc_feature 1..1578: note = DNA of 2nd fusion_scFv-MXD1(SID FL)
  source 1..1578: mol_type = other DNA
atgggccccgacatcgtgatgacccagagccccagcagcctgagcgccagcgtgggcgaccgcgtgaccatcacctgccgcagcagcaccggcgccgtgaccaccagcaactacgccagctgggtgcaggagaagcccggcaagctgttcaagggcctgatcggcggcaccaacaaccgcgcccccggcgtgcccagccgcttcagcggcagcctgatcggcgacaaggccaccctgaccatcagcagcctgcagcccgaggacttcgccacctacttctgcgccctgtggtacagcaaccactgggtgttcggccagggcaccaaggtggagctgaagcgcggcggcggcggcagcggcggcggcggcagcggcggcggcggcagcagcggcggcggcagcgaggtgaagctgctggagagcggcggcggcctggtgcagcccggcggcagcctgaagctgagctgcgccgtgagcggcttcagcctgaccgactacggcgtgaactgggtgcgccaggcccccggccgcggcctggagtggatcggcgtgatctggggcgacggcatcaccgactacaacagcgccctgaaggaccgcttcatcatcagcaaggacaacggcaagaacaccgtgtacctgcagatgagcaaggtgcgcagcgacgacaccgccctgtactactgcgtgaccggcctgttcgactactggggccagggcaccctggtgaccgtgagcagctacccatacgatgttccagattacgctggtggaggcggaggttctgggggaggaggtagtggcggtggtggttcaggaggcggcggaagcttggatccaggtggaggtggaagcggtgcggcggcggttcggatgaacatccagatgctgctggaggcggccgactatctggagcggcgggagagagaagctgaacatggttatgcctccatgttaccatacaataacaaggacagagatgccttaaaacggaggaacaaatccaaaaagaataacagcagtagcagatcaactcacaatgaaatggagaagaatagacgggctcatcttcgcttgtgcctggagaagttgaaggggctggtgccacttggacccgaatcaagtcgacacactacgttgagtttattaacaaaagccaaattgcacataaagaaacttgaagattgtgacagaaaagccgttcaccaaatcgaccagcttcagcgagagcagcgacacctgaagaggcagctggagaagctgggcattgagaggatccggatggacagcatcggctccaccgtctcctcggagcgctccgactccgacagggaaatcgacgttgacgtggagagcacggactatctcacaggtgatctggactggagcagcagcagtgtgagcgactctgacgagcggggcagcatgcagagcctcggcagtgatgagggctattccagcaccagcatcaagagaataaagctgcaggacagtcacaaggcgtgtcttggtctcggaagcggaaagcgcaccgccgatggttccgagttcgaaagccccaaaaaaaagcgcaaggtc

SEQ ID NO: 190 - DNA, 1008 bp, synthetic construct
  misc_feature 1..1008: note = DNA of 2nd fusion_scFv-SID
  source 1..1008: mol_type = other DNA
atgggccccgacatcgtgatgacccagagccccagcagcctgagcgccagcgtgggcgaccgcgtgaccatcacctgccgcagcagcaccggcgccgtgaccaccagcaactacgccagctgggtgcaggagaagcccggcaagctgttcaagggcctgatcggcggcaccaacaaccgcgcccccggcgtgcccagccgcttcagcggcagcctgatcggcgacaaggccaccctgaccatcagcagcctgcagcccgaggacttcgccacctacttctgcgccctgtggtacagcaaccactgggtgttcggccagggcaccaaggtggagctgaagcgcggcggcggcggcagcggcggcggcggcagcggcggcggcggcagcagcggcggcggcagcgaggtgaagctgctggagagcggcggcggcctggtgcagcccggcggcagcctgaagctgagctgcgccgtgagcggcttcagcctgaccgactacggcgtgaactgggtgcgccaggcccccggccgcggcctggagtggatcggcgtgatctggggcgacggcatcaccgactacaacagcgccctgaaggaccgcttcatcatcagcaaggacaacggcaagaacaccgtgtacctgcagatgagcaaggtgcgcagcgacgacaccgccctgtactactgcgtgaccggcctgttcgactactggggccagggcaccctggtgaccgtgagcagctacccatacgatgttccagattacgctggtggaggcggaggttctgggggaggaggtagtggcggtggtggttcaggaggcggcggaagcttggatccaggtggaggtggaagcggtatgaacatccagatgctgctggaggcggccgactatctggagcggcgggagagagaagctgaacatggttatgcctccatgttaccaggaagcggaaagcgcaccgccgatggttccgagttcgaaagccccaaaaaaaagcgcaaggtc

SEQ ID NO: 191 - DNA, 3546 bp, synthetic construct
  misc_feature 1..3546: note = DNA of 2nd fusion_scFv-LSD1(KDMA1)
  source 1..3546: mol_type = other DNA
atgggccccgacatcgtgatgacccagagccccagcagcctgagcgccagcgtgggcgaccgcgtgaccatcacctgccgcagcagcaccggcgccgtgaccaccagcaactacgccagctgggtgcaggagaagcccggcaagctgttcaagggcctgatcggcggcaccaacaaccgcgcccccggcgtgcccagccgcttcagcggcagcctgatcggcgacaaggccaccctgaccatcagcagcctgcagcccgaggacttcgccacctacttctgcgccctgtggtacagcaaccactgggtgttcggccagggcaccaaggtggagctgaagcgcggcggcggcggcagcggcggcggcggcagcggcggcggcggcagcagcggcggcggcagcgaggtgaagctgctggagagcggcggcggcctggtgcagcccggcggcagcctgaagctgagctgcgccgtgagcggcttcagcctgaccgactacggcgtgaactgggtgcgccaggcccccggccgcggcctggagtggatcggcgtgatctggggcgacggcatcaccgactacaacagcgccctgaaggaccgcttcatcatcagcaaggacaacggcaagaacaccgtgtacctgcagatgagcaaggtgcgcagcgacgacaccgccctgtactactgcgtgaccggcctgttcgactactggggccagggcaccctggtgaccgtgagcagctacccatacgatgttccagattacgctggtggaggcggaggttctgggggaggaggtagtggcggtggtggttcaggaggcggcggaagcttggatccaggtggaggtggaagcggtttatctgggaagaaggcggcagccgcggcggcggcggctgcagcggcagcaaccgggacggaggctggccctgggacagcaggcggctccgagaacgggtctgaggtggccgcgcagcccgcgggcctgtcgggcccagccgaggtcgggccgggggcggtgggggagcgcacaccccgcaagaaagagcctccgcgggcctcgccccccgggggcctggcggaaccgccggggtccgcagggcctcaggccggccctactgtcgtgcctgggtctgcgacccccatggaaactggaatagcagagactccggaggggcgtcggaccagccggcgcaagcgggcgaaggtagagtacagagagatggatgaaagcttggccaacctctcagaagatgagtattattcagaagaagagagaaatgccaaagcagagaaggaaaagaagcttcccccaccaccccctcaagccccacctgaggaagaaaatgaaagtgagcctgaagaaccatcggggcaagcaggaggacttcaagacgacagttctggagggtatggagacggccaagcatcaggtgtggagggcgcagctttccagagccgacttcctcatgaccggatgacttctcaagaagcagcctgttttccagatattatcagtggaccacaacagacccagaaggtttttcttttcattagaaaccgcacactgcagttgtggttggataatccaaagattcagctgacatttgaggctactctccaacaattagaagcaccttataacagtgatactgtgcttgtccaccgagttcacagttatttagagcgtcatggtcttatcaacttcggcatctataagaggataaaacccctaccaactaaaaagacaggaaaggtaattattataggctctggggtctcaggcttggcagcagctcgacagttacaaagttttggaatggatgtcacacttttggaagccagggatcgtgtgggtggacgagttgccacatttcgcaaaggaaactatgtagctgatcttggagccatggtggtaacaggtcttggagggaatcctatggctgtggtcagcaaacaagtaaatatggaactggccaagatcaagcaaaaatgcccactttatgaagccaacggacaagctgacactgtcaaggttcctaaagagaaagatgaaatggtagagcaagagtttaaccggttgctagaagctacatcttaccttagtcatcaactagacttcaatgtcctcaataataagcctgtgtcccttggccaggcattggaagttgtcattcagttacaagagaagcatgtcaaagatgagcagattgaacattggaagaagatagtgaaaactcaggaagaattgaaagaacttcttaataagatggtaaatttgaaagagaaaattaaagaactccatcagcaatacaaagaagcatctgaagtaaagccacccagagatattactgccgagttcttagtgaaaagcaaacacagggatctgaccgccctatgcaaggaatatgatgaattagctgaaacacaaggaaagctagaagaaaaacttcaggagttggaagcgaatcccccaagtgatgtatatctctcatcaagagacagacaaatacttgattggcattttgcaaatcttgaatttgctaatgccacacctctctcaactctctcccttaagcactgggatcaggatgatgactttgagttcactggcagccacctgacagtaaggaatggctactcgtgtgtgcctgtggctttagcagaaggcctagacattaaactgaatacagcagtgcgacaggttcgctacacggcttcaggatgtgaagtgatagctgtgaatacccgctccacgagtcaaacctttatttataaatgcgacgcagttctctgtacccttcccctgggtgtgctgaagcagcagccaccagccgttcagtttgtgccacctctccctgagtggaaaacatctgcagtccaaaggatgggatttggcaaccttaacaaggtggtgttgtgttttgatcgggtgttctgggatccaagtgtcaatttgttcgggcatgttggcagtacgactgccagcaggggtgagctcttcctcttctggaacctctataaagctccaatactgttggcactagtggcaggagaagctgctggtatcatggaaaacataagtgacgatgtgattgttggccgatgcctggccattctcaaagggatttttggtagcagtgcagtacctcagcccaaagaaactgtggtgtctcgttggcgtgctgatccctgggctcggggctcttattcctatgttgctgcaggatcatctggaaatgactatgatttaatggctcagccaatcactcctggcccctcgattccaggtgccccacagccgattccacgactcttctttgcgggagaacatacgatccgtaactacccagccacagtgcatggtgctctgctgagtgggctgcgagaagcgggaagaattgcagaccagtttttgggggccatgtatacgctgcctcgccaggccacaccaggtgttcctgcacagcagtccccaagcatgggaagcggaaagcgcaccgccgatggttccgagttcgaaagccccaaaaaaaagcgcaaggtc

SEQ ID NO: 192 - DNA, 1491 bp, synthetic construct
  misc_feature 1..1491: note = DNA of 2nd fusion_scFv-HP1a long
  source 1..1491: mol_type = other DNA
atgggccccgacatcgtgatgacccagagccccagcagcctgagcgccagcgtgggcgaccgcgtgaccatcacctgccgcagcagcaccggcgccgtgaccaccagcaactacgccagctgggtgcaggagaagcccggcaagctgttcaagggcctgatcggcggcaccaacaaccgcgcccccggcgtgcccagccgcttcagcggcagcctgatcggcgacaaggccaccctgaccatcagcagcctgcagcccgaggacttcgccacctacttctgcgccctgtggtacagcaaccactgggtgttcggccagggcaccaaggtggagctgaagcgcggcggcggcggcagcggcggcggcggcagcggcggcggcggcagcagcggcggcggcagcgaggtgaagctgctggagagcggcggcggcctggtgcagcccggcggcagcctgaagctgagctgcgccgtgagcggcttcagcctgaccgactacggcgtgaactgggtgcgccaggcccccggccgcggcctggagtggatcggcgtgatctggggcgacggcatcaccgactacaacagcgccctgaaggaccgcttcatcatcagcaaggacaacggcaagaacaccgtgtacctgcagatgagcaaggtgcgcagcgacgacaccgccctgtactactgcgtgaccggcctgttcgactactggggccagggcaccctggtgaccgtgagcagctacccatacgatgttccagattacgctggtggaggcggaggttctgggggaggaggtagtggcggtggtggttcaggaggcggcggaagcttggatccaggtggaggtggaagcggtggaaagaaaaccaagcggacagctgacagttcttcttcagaggatgaggaggagtatgttgtggagaaggtgctagacaggcgcgtggttaagggacaagtggaatatctactgaagtggaaaggcttttctgaggagcacaatacttgggaacctgagaaaaacttggattgccctgagctaatttctgaatttatgaaaaagtataagaagatgaaggagggtgaaaataataaacccagggagaagtcagaaagtaacaagaggaaatccaatttctcaaacagtgccgatgacatcaaatctaaaaaaaagagagagcagagcaatgatatcgctcggggctttgagagaggactggaaccagaaaagatcattggggcaacagattcctgtggtgatttaatgttcctaatgaaatggaaagacacagatgaagctgacctggttcttgcaaaagaagctaatgtgaaatgtccacaaattgtgatagcattttatgaagagagactgacatggcatgcatatcctgaggatgcggaaaacaaagagaaagaaacagcaaagagcggaagcggaaagcgcaccgccgatggttccgagttcgaaagccccaaaaaaaagcgcaaggtc

SEQ ID NO: 193 - DNA, 1278 bp, synthetic construct
  misc_feature 1..1278: note = DNA of 2nd fusion_scFv-HP1a short
  source 1..1278: mol_type = other DNA
atgggccccgacatcgtgatgacccagagccccagcagcctgagcgccagcgtgggcgaccgcgtgaccatcacctgccgcagcagcaccggcgccgtgaccaccagcaactacgccagctgggtgcaggagaagcccggcaagctgttcaagggcctgatcggcggcaccaacaaccgcgcccccggcgtgcccagccgcttcagcggcagcctgatcggcgacaaggccaccctgaccatcagcagcctgcagcccgaggacttcgccacctacttctgcgccctgtggtacagcaaccactgggtgttcggccagggcaccaaggtggagctgaagcgcggcggcggcggcagcggcggcggcggcagcggcggcggcggcagcagcggcggcggcagcgaggtgaagctgctggagagcggcggcggcctggtgcagcccggcggcagcctgaagctgagctgcgccgtgagcggcttcagcctgaccgactacggcgtgaactgggtgcgccaggcccccggccgcggcctggagtggatcggcgtgatctggggcgacggcatcaccgactacaacagcgccctgaaggaccgcttcatcatcagcaaggacaacggcaagaacaccgtgtacctgcagatgagcaaggtgcgcagcgacgacaccgccctgtactactgcgtgaccggcctgttcgactactggggccagggcaccctggtgaccgtgagcagctacccatacgatgttccagattacgctggtggaggcggaggttctgggggaggaggtagtggcggtggtggttcaggaggcggcggaagcttggatccaggtggaggtggaagcggtatgaaggagggtgaaaataataaacccagggagaagtcagaaagtaacaagaggaaatccaatttctcaaacagtgccgatgacatcaaatctaaaaaaaagagagagcagagcaatgatatcgctcggggctttgagagaggactggaaccagaaaagatcattggggcaacagattcctgtggtgatttaatgttcctaatgaaatggaaagacacagatgaagctgacctggttcttgcaaaagaagctaatgtgaaatgtccacaaattgtgatagcattttatgaagagagactgacatggcatgcatatcctgaggatgcggaaaacaaagagaaagaaacagcaaagagcggaagcggaaagcgcaccgccgatggttccgagttcgaaagccccaaaaaaaagcgcaaggtc

SEQ ID NO: 194 - DNA, 2202 bp, synthetic construct
  misc_feature 1..2202: note = DNA of 2nd fusion_scFv-HDAC3
  source 1..2202: mol_type = other DNA
atgggccccgacatcgtgatgacccagagccccagcagcctgagcgccagcgtgggcgaccgcgtgaccatcacctgccgcagcagcaccggcgccgtgaccaccagcaactacgccagctgggtgcaggagaagcccggcaagctgttcaagggcctgatcggcggcaccaacaaccgcgcccccggcgtgcccagccgcttcagcggcagcctgatcggcgacaaggccaccctgaccatcagcagcctgcagcccgaggacttcgccacctacttctgcgccctgtggtacagcaaccactgggtgttcggccagggcaccaaggtggagctgaagcgcggcggcggcggcagcggcggcggcggcagcggcggcggcggcagcagcggcggcggcagcgaggtgaagctgctggagagcggcggcggcctggtgcagcccggcggcagcctgaagctgagctgcgccgtgagcggcttcagcctgaccgactacggcgtgaactgggtgcgccaggcccccggccgcggcctggagtggatcggcgtgatctggggcgacggcatcaccgactacaacagcgccctgaaggaccgcttcatcatcagcaaggacaacggcaagaacaccgtgtacctgcagatgagcaaggtgcgcagcgacgacaccgccctgtactactgcgtgaccggcctgttcgactactggggccagggcaccctggtgaccgtgagcagctacccatacgatgttccagattacgctggtggaggcggaggttctgggggaggaggtagtggcggtggtggttcaggaggcggcggaagcttggatccaggtggaggtggaagcggtgccaagaccgtggcctatttctacgaccccgacgtgggcaacttccactacggagctggacaccctatgaagccccatcgcctggcattgacccatagcctggtcctgcattacggtctctataagaagatgatcgtcttcaagccataccaggcctcccaacatgacatgtgccgcttccactccgaggactacattgacttcctgcagagagtcagccccaccaatatgcaaggcttcaccaagagtcttaatgccttcaacgtaggcgatgactgcccagtgtttcccgggctctttgagttctgctcgcgttacacaggcgcatctctgcaaggagcaacccagctgaacaacaagatctgtgatattgccattaactgggctggtggtctgcaccatgccaagaagtttgaggcctctggcttctgctatgtcaacgacattgtgattggcatcctggagctgctcaagtaccaccctcgggtgctctacattgacattgacatccaccatggtgacggggttcaagaagctttctacctcactgaccgggtcatgacggtgtccttccacaaatacggaaattacttcttccctggcacaggtgacatgtatgaagtcggggcagagagtggccgctactactgtctgaacgtgcccctgcgggatggcattgatgaccagagttacaagcaccttttccagccggttatcaaccaggtagtggacttctaccaacccacgtgcattgtgctccagtgtggagctgactctctgggctgtgatcgattgggctgctttaacctcagcatccgagggcatggggaatgcgttgaatatgtcaagagcttcaatatccctctactcgtgctgggtggtggtggttatactgtccgaaatgttgcccgctgctggacatatgagacatcgctgctggtagaagaggccattagtgaggagcttccctatagtgaatacttcgagtactttgccccagacttcacacttcatccagatgtcagcacccgcatcgagaatcagaactcacgccagtatctggaccagatccgccagacaatctttgaaaacctgaagatgctgaaccatgcacctagtgtccagattcatgacgtgcctgcagacctcctgacctatgacaggactgatgaggctgatgcagaggagaggggtcctgaggagaactatagcaggccagaggcacccaatgagttctatgatggagaccatgacaatgacaaggaaagcgatgtggagattggaagcggaaagcgcaccgccgatggttccgagttcgaaagccccaaaaaaaagcgcaaggtc

SEQ ID NO: 195 - DNA, 8643 bp, synthetic construct
  misc_feature 1..8643: note = DNA of V1_3xGCN4-dCas9-3xGCN4
  source 1..8643: mol_type = other DNA
atcgtgctgaccctgacactgtttgaggacagagagatgatcgaggaacggctgaaaacctatgcccacctgttcgacgacaaagtgatgaagcagctgaagcggcggagatacaccggctggggcaggctgagccggaagctgatcaacggcatccgggacaagcagtccggcaagacaatcctggatttcctgaagtccgacggcttcgccaacagaaacttcatgcagctgatccacgacgacagcctgacctttaaagaggacatccagaaagcccaggtgtccggccagggcgatagcctgcacgagcacattgccaatctggccggcagccccgccattaagaagggcatcctgcagacagtgaaggtggtggacgagctcgtgaaagtgatgggccggcacaagcccgagaacatcgtgatcgaaatggccagagagaaccagaccacccagaagggacagaagaacagccgcgagagaatgaagcggatcgaagagggcatcaaagagctgggcagccagatcctgaaagaacaccccgtggaaaacacccagctgcagaacgagaagctgtacctgtactacctgcagaatgggcgggatatgtacgtggaccaggaactggacatcaaccggctgtccgactacgatgtggacgctatcgtgcctcagagctttctgaaggacgactccatcgataacaaagtgctgactcggagcgacaagaaccggggcaagagcgacaacgtgccctccgaagaggtcgtgaagaagatgaagaactactggcgccagctgctgaatgccaagctgattacccagaggaagttcgacaatctgaccaaggccgagagaggcggcctgagcgaactggataaggccggcttcatcaagagacagctggtggaaacccggcagatcacaaagcacgtggcacagatcctggactcccggatgaacactaagtacgacgagaacgacaaactgatccgggaagtgaaagtgatcaccctgaagtccaagctggtgtccgatttccggaaggatttccagttttacaaagtgcgcgagatcaacaactaccaccacgcccacgacgcctacctgaacgccgtcgtgggaaccgccctgatcaaaaagtaccctaagctggaaagcgagttcgtgtacggcgactacaaggtgtacgacgtgcggaagatgatcgccaagagcgagcaggaaatcggcaaggctaccgccaagtacttcttctacagcaacatcatgaactttttcaagaccgagattaccctggccaacggcgagatccggaagcggcctctgatcgagacaaacggcgaaacaggcgagatcgtgtgggataagggccgggactttgccaccgtgcggaaagtgctgtctatgccccaagtgaatatcgtgaaaaagaccgaggtgcagacaggcggcttcagcaaagagtctatcctgcccaagaggaacagcgacaagctgatcgccagaaagaaggactgggaccctaagaagtacggcggcttcgacagccccaccgtggcctattctgtgctggtggtggccaaagtggaaaagggcaagtccaagaaactgaagagtgtgaaagagctgctggggatcaccatcatggaaagaagcagcttcgagaagaatcccatcgactttctggaagccaagggctacaaagaagtgaaaaaggacctgatcatcaagctgcctaagtactccctgttcgagctggaaaacggccggaagagaatgctggcctctgccggcgaactgcagaagggaaacgaactggccctgccctccaaatatgtgaacttcctgtacctggccagccactatgagaagctgaagggctcccccgaggataatgagcagaaacagctgtttgtggaacagcacaaacactacctggacgagatcatcgagcagatcagcgagttctccaagagagtgatcctggccgacgctaatctggacaaggtgctgagcgcctacaacaagcacagagacaagcctatcagagagcaggccgagaatatcatccacctgtttaccctgaccaatctgggagcccctgccgccttcaagtactttgacaccaccatcgaccggaagaggtacaccagcaccaaagaggtgctggacgccaccctgatccaccagagcatcaccggcctgtacgagacacggatcgacctgtctcagctgggaggcgacgcctatccctatgacgtgcccgattatgccagcctgggcagcggctcccccaagaaaaaacgcaaggtggaagatcctaagaaaaagcggaaagtggacggcagcggcagcgagacccccggtaccagtggcggatctggctccggtagcggaggatcaggatccggcggaagcggatcaggcgaggaactgctttccaaaaattaccaccttgaaaacgaagtcgcccgcctcaagaaaggttctggcagcggaggctctggcagtggtggtagcggaagtggaagtggtggcagtggtagcggtggatctggaagcggcgaggaactcctgtcaaagaattaccatctcgaaaacgaggtcgcaaggctcaagaaaggctcaggatcaggcggctctggatccggcggttctggttccggctcaggtggaagtggatctggcggctcaggttccggcgaagaattgctttccaagaactaccatttggaaaatgaagtcgctcgtttgaagaaaggttcaggctccggccagcggggaagcaagcgcaccgccgatggttccgagttcgaaagccccaaaaaaaagcgcaaggtctgagatcccaagcacgcagcaatgcagctcaaaacgcttagcctagccacacccccacgggaaacagcagtgattaacctttagcaataaacgaaagtttaactaagctatactaaccccagggttggtcaatttcgtgccagccacaccctggtactgcatgcacgcaatgctagctgcccctttcccgtcctgggcaccccgagtctcccccgaccccgggtcccaggtatgctcccacctccacctgccccactcaccacctctgctagttccagacacctccgagacgaggaaaaaaaaaaaaaaaaaaaaaaaaaaaaaaaaaaaaaaaaaaaaaaaaaaaaaaaaaaaaaaaaaaaaaaaaaaaaaaaaaaaaaaaaaaaaaaaaaaaaaaaaaaaaaaaaaaaaaaaaaaaaaaaaaaaaaaaaaaaaaaaaaaaaaaaaaaaaaaaaaaaaaaaaaaaaaaaaaaaaaaaaaaaaaaaaaaaaaaaaaaaaaaaaaaaaaaaaaaaaaaaaaaaaaaaaaaaaaaaaaaaaaaaaaaaaaaaaaaaaaaaaaaaaaaaaaaaaaaaaaaaaaaaaaaaaaaaaaaaaaaaaaaaaaaaaaaaaaaaaaaaaaaaaaaaaaaaaaaaaaaaaaaaaaaaaaaaaaaaaaaaaaaaaaaaaaaaaaaaaaaaaaaaaaaaaaaccgtcttcaagctttctagaaattcactggccgtcgttttacaacgtcgtgactgggaaaaccctggcgttacccaacttaatcgccttgcagcacatccccctttcgccagctggcgtaatagcgaagaggcccgcaccgatcgcccttcccaacagttgcgcagcctgaatggcgaatggcgcctgatgcggtattttctccttacgcatctgtgcggtatttcacaccgcatatggtgcactctcagtacaatctgctctgatgccgcatagttaagccagccccgacacccgccaacacccgctgacgcgccctgacgggcttgtctgctcccggcatccgcttacagacaagctgtgaccgtctccgggagctgcatgtgtcagaggttttcaccgtcatcaccgaaacgcgcgagacgaaagggcctcgtgatacgcctatttttataggttaatgtcatgataataatggtttcttagacgtcaggtggcacttttcggggaaatgtgcgcggaacccctatttgtttatttttctaaatacattcaaatatgtatccgctcatgagacaataaccctgataaatgcttcaataatattgaaaaaggaagagtatgagtattcaacatttccgtgtcgcccttattcccttttttgcggcattttgccttcctgtttttgctcacccagaaacgctggtgaaagtaaaagatgctgaagatcagttgggtgcacgagtgggttacatcgaactggatctcaacagcggtaagatccttgagagttttcgccccgaagaacgttttccaatgatgagcacttttaaagttctgctatgtggcgcggtattatcccgtattgacgccgggcaagagcaactcggtcgccgcatacactattctcagaatgacttggttgagtactcaccagtcacagaaaagcatcttacggatggcatgacagtaagagaattatgcagtgctgccataaccatgagtgataacactgcggccaacttacttctgacaacgatcggaggaccgaaggagctaaccgcttttttgcacaacatgggggatcatgtaactcgccttgatcgttgggaaccggagctgaatgaagccataccaaacgacgagcgtgacaccacgatgcctgtagcaatggcaacaacgttgcgcaaactattaactggcgaactacttactctagcttcccggcaacaattaatagactggatggaggcggataaagttgcaggaccacttctgcgctcggcccttccggctggctggtttattgctgataaatctggagccggtgagcgtgggtctcgcggtatcattgcagcactggggccagatggtaagccctcccgtatcgtagttatctacacgacggggagtcaggcaactatggatgaacgaaatagacagatcgctgagataggtgcctcactgattaagcattggtaactgtcagaccaagtttactcatatatactttagattgatttaaaacttcatttttaatttaaaaggatctaggtgaagatcctttttgataatctcatgaccaaaatcccttaacgtgagttttcgttccactgagcgtcagaccccgtagaaaagatcaaaggatcttcttgagatcctttttttctgcgcgtaatctgctgcttgcaaacaaaaaaaccaccgctaccagcggtggtttgtttgccggatcaagagctaccaactctttttccgaaggtaactggcttcagcagagcgcagataccaaatactgttcttctagtgtagccgtagttaggccaccacttcaagaactctgtagcaccgcctacatacctcgctctgctaatcctgttaccagtggctgctgccagtggcgataagtcgtgtcttaccgggttggactcaagacgatagttaccggataaggcgcagcggtcgggctgaacggggggttcgtgcacacagcccagcttggagcgaacgacctacaccgaactgagatacctacagcgtgagctatgagaaagcgccacgcttcccgaagggagaaaggcggacaggtatccggtaagcggcagggtcggaacaggagagcgcacgagggagcttccagggggaaacgcctggtatctttatagtcctgtcgggtttcgccacctctgacttgagcgtcgatttttgtgatgctcgtcaggggggcggagcctatggaaaaacgccagcaacgcggcctttttacggttcctggccttttgctggccttttgctcacatgttctttcctgcgttatcccctgattctgtggataaccgtattaccgcctttgagtgagctgataccgctcgccgcagccgaacgaccgagcgcagcgagtcagtgagcgaggaagcggaagagcgcccaatacgcaaaccgcctctccccgcgcgttggccgattcattaatgcagctggcacgacaggtttcccgactggaaagcgggcagtgagcgcaacgcaattaatgtgagttagctcactcattaggcaccccaggctttacactttatgcttccggctcgtatgttgtgtggaattgtgagcggataacaatttcacacaggaaacagctatgaccatgattacgcctctagaaagctttaatacgactcactataaggactcactatttgttttcgcgcccagttgcaaaaagtgtcgacatttgcttctgacacaactgtgttcactagcaacctcaaacagacaccgccaccatgcctgctgctaagagagtgaaactggatggatccgaggaactgctgagcaagaactaccacctggaaaacgaggtggccagactgaagaaaggctctggctctggcggaagcggttctggcggatcaggatctggaagtggcggctctggaagcggaggttctggatctggcgaagaactgctgtctaagaattatcacctcgagaacgaagtggctcggctcaagaaaggcagtggcagcggaggaagtggatccggcggtagtggtagtggaagcggcggatccggctcaggcggatctggttcaggggaagaactcctctccaaaaactaccatctcgagaatgaggtcgcccgcctgaaaaaaggatcaggttccggtggttctggcagcggtggttcaggctcaggcagcggcggtagcggtagcggtggaagcggaagcggaccaaaaaagaagagaaaggtaatggacaagaagtacagcatcggcctggccatcggcaccaactctgtgggctgggccgtgatcaccgacgagtacaaggtgcccagcaagaaattcaaggtgctgggcaacaccgaccggcacagcatcaagaagaacctgatcggcgccctgctgttcgacagcggagaaacagccgaggccacccggctgaagagaaccgccagaagaagatacaccagacggaagaaccggatctgctatctgcaagagatcttcagcaacgagatggccaaggtggacgacagcttcttccacagactggaagagtccttcctggtggaagaggataagaagcacgagcggcaccccatcttcggcaacatcgtggacgaggtggcctaccacgagaagtaccccaccatctaccacctgagaaagaaactggtggacagcaccgacaaggccgacctgcggctgatctatctggccctggcccacatgatcaagttccggggccacttcctgatcgagggcgacctgaaccccgacaacagcgacgtggacaagctgttcatccagctggtgcagacctacaaccagctgttcgaggaaaaccccatcaacgccagcggcgtggacgccaaggccatcctgtctgccagactgagcaagagcagacggctggaaaatctgatcgcccagctgcccggcgagaagaagaatggcctgttcggcaacctgattgccctgagcctgggcctgacccccaacttcaagagcaacttcgacctggccgaggatgccaaactgcagctgagcaaggacacctacgacgacgacctggacaacctgctggcccagatcggcgaccagtacgccgacctgtttctggccgccaagaacctgtccgacgccatcctgctgagcgacatcctgagagtgaacaccgagatcaccaaggcccccctgagcgcctctatgatcaagagatacgacgagcaccaccaggacctgaccctgctgaaagctctcgtgcggcagcagctgcctgagaagtacaaagagattttcttcgaccagagcaagaacggctacgccggctacatcgatggcggagccagccaggaagagttctacaagttcatcaagcccatcctggaaaagatggacggcaccgaggaactgctcgtgaagctgaacagagaggacctgctgcggaagcagcggaccttcgacaacggcagcatcccccaccagatccacctgggagagctgcacgccattctgcggcggcaggaagatttttacccattcctgaaggacaaccgggaaaagatcgagaagatcctgaccttccgcatcccctactacgtgggccctctggccaggggaaacagcagattcgcctggatgaccagaaagagcgaggaaaccatcaccccctggaacttcgaggaagtggtggacaagggcgccagcgcccagagcttcatcgagcggatgaccaacttcgataagaacctgcccaacgagaaggtgctgcccaagcacagcctgctgtacgagtacttcaccgtgtacaacgagctgaccaaagtgaaatacgtgaccgagggaatgagaaagcccgccttcctgagcggcgagcagaaaaaagccatcgtggacctgctgttcaagaccaaccggaaagtgaccgtgaagcagctgaaagaggactacttcaagaaaatcgagtgcttcgactccgtggaaatctccggcgtggaagatcggttcaacgcctccctgggcacataccacgatctgctgaaaattatcaaggacaaggacttcctggacaatgaggaaaacgaggacattctggaagat

SEQ ID NO: 196 - DNA, 4357 bp, synthetic construct
  misc_feature 1..4357: note = DNA of V2_scFv-KRAB
  source 1..4357: mol_type = other DNA
gagatacctacagcgtgagctatgagaaagcgccacgcttcccgaagggagaaaggcggacaggtatccggtaagcggcagggtcggaacaggagagcgcacgagggagcttccagggggaaacgcctggtatctttatagtcctgtcgggtttcgccacctctgacttgagcgtcgatttttgtgatgctcgtcaggggggcggagcctatggaaaaacgccagcaacgcggcctttttacggttcctggccttttgctggccttttgctcacatgttctttcctgcgttatcccctgattctgtggataaccgtattaccgcctttgagtgagctgataccgctcgccgcagccgaacgaccgagcgcagcgagtcagtgagcgaggaagcggaagagcgcccaatacgcaaaccgcctctccccgcgcgttggccgattcattaatgcagctggcacgacaggtttcccgactggaaagcgggcagtgagcgcaacgcaattaatgtgagttagctcactcattaggcaccccaggctttacactttatgcttccggctcgtatgttgtgtggaattgtgagcggataacaatttcacacaggaaacagctatgaccatgattacgcctctagaaagctttaatacgactcactataaggactcactatttgttttcgcgcccagttgcaaaaagtgtcgacatttgcttctgacacaactgtgttcactagcaacctcaaacagacaccgccaccatgcctgctgctaagagagtgaaactggatggatccggccccgacatcgtgatgacccagagccccagcagcctgagcgccagcgtgggcgaccgcgtgaccatcacctgccgcagcagcaccggcgccgtgaccaccagcaactacgccagctgggtgcaggagaagcccggcaagctgttcaagggcctgatcggcggcaccaacaaccgcgcccccggcgtgcccagccgcttcagcggcagcctgatcggcgacaaggccaccctgaccatcagcagcctgcagcccgaggacttcgccacctacttctgcgccctgtggtacagcaaccactgggtgttcggccagggcaccaaggtggagctgaagcgcggcggcggcggcagcggcggcggcggcagcggcggcggcggcagcagcggcggcggcagcgaggtgaagctgctggagagcggcggcggcctggtgcagcccggcggcagcctgaagctgagctgcgccgtgagcggcttcagcctgaccgactacggcgtgaactgggtgcgccaggcccccggccgcggcctggagtggatcggcgtgatctggggcgacggcatcaccgactacaacagcgccctgaaggaccgcttcatcatcagcaaggacaacggcaagaacaccgtgtacctgcagatgagcaaggtgcgcagcgacgacaccgccctgtactactgcgtgaccggcctgttcgactactggggccagggcaccctggtgaccgtgagcagctacccatacgatgttccagattacgctggtggaggcggaggttctgggggaggaggtagtggcggtggtggttcaggaggcggcggaagcttggatccaggtggaggtggaagcggtcggacactggtgaccttcaaggatgtatttgtggacttcaccagggaggagtggaagctgctggacactgctcagcagatcgtgtacagaaatgtgatgctggagaactataagaacctggtttccttgggttatcagcttactaagccagatgtgatcctccggttggagaagggagaagagccctagtgagatcccaagcacgcagcaatgcagctcaaaacgcttagcctagccacacccccacgggaaacagcagtgattaacctttagcaataaacgaaagtttaactaagctatactaaccccagggttggtcaatttcgtgccagccacaccctggtactgcatgcacgcaatgctagctgcccctttcccgtcctgggcaccccgagtctcccccgaccccgggtcccaggtatgctcccacctccacctgccccactcaccacctctgctagttccagacacctccgagacgaggaaaaaaaaaaaaaaaaaaaaaaaaaaaaaaaaaaaaaaaaaaaaaaaaaaaaaaaaaaaaaaaaaaaaaaaaaaaaaaaaaaaaaaaaaaaaaaaaaaaaaaaaaaaaaaaaaaaaaaaaaaaaaaaaaaaaaaaaaaaaaaaaaaaaaaaaaaaaaaaaaaaaaaaaaaaaaaaaaaaaaaaaaaaaaaaaaaaaaaaaccgtcttcaagctttctagaaattcactggccgtcgttttacaacgtcgtgactgggaaaaccctggcgttacccaacttaatcgccttgcagcacatccccctttcgccagctggcgtaatagcgaagaggcccgcaccgatcgcccttcccaacagttgcgcagcctgaatggcgaatggcgcctgatgcggtattttctccttacgcatctgtgcggtatttcacaccgcatatggtgcactctcagtacaatctgctctgatgccgcatagttaagccagccccgacacccgccaacacccgctgacgcgccctgacgggcttgtctgctcccggcatccgcttacagacaagctgtgaccgtctccgggagctgcatgtgtcagaggttttcaccgtcatcaccgaaacgcgcgagacgaaagggcctcgtgatacgcctatttttataggttaatgtcatgataataatggtttcttagacgtcaggtggcacttttcggggaaatgtgcgcggaacccctatttgtttatttttctaaatacattcaaatatgtatccgctcatgagacaataaccctgataaatgcttcaataatattgaaaaaggaagagtatgagtattcaacatttccgtgtcgcccttattcccttttttgcggcattttgccttcctgtttttgctcacccagaaacgctggtgaaagtaaaagatgctgaagatcagttgggtgcacgagtgggttacatcgaactggatctcaacagcggtaagatccttgagagttttcgccccgaagaacgttttccaatgatgagcacttttaaagttctgctatgtggcgcggtattatcccgtattgacgccgggcaagagcaactcggtcgccgcatacactattctcagaatgacttggttgagtactcaccagtcacagaaaagcatcttacggatggcatgacagtaagagaattatgcagtgctgccataaccatgagtgataacactgcggccaacttacttctgacaacgatcggaggaccgaaggagctaaccgcttttttgcacaacatgggggatcatgtaactcgccttgatcgttgggaaccggagctgaatgaagccataccaaacgacgagcgtgacaccacgatgcctgtagcaatggcaacaacgttgcgcaaactattaactggcgaactacttactctagcttcccggcaacaattaatagactggatggaggcggataaagttgcaggaccacttctgcgctcggcccttccggctggctggtttattgctgataaatctggagccggtgagcgtgggtctcgcggtatcattgcagcactggggccagatggtaagccctcccgtatcgtagttatctacacgacggggagtcaggcaactatggatgaacgaaatagacagatcgctgagataggtgcctcactgattaagcattggtaactgtcagaccaagtttactcatatatactttagattgatttaaaacttcatttttaatttaaaaggatctaggtgaagatcctttttgataatctcatgaccaaaatcccttaacgtgagttttcgttccactgagcgtcagaccccgtagaaaagatcaaaggatcttcttgagatcctttttttctgcgcgtaatctgctgcttgcaaacaaaaaaaccaccgctaccagcggtggtttgtttgccggatcaagagctaccaactctttttccgaaggtaactggcttcagcagagcgcagataccaaatactgttcttctagtgtagccgtagttaggccaccacttcaagaactctgtagcaccgcctacatacctcgctctgctaatcctgttaccagtggctgctgccagtggcgataagtcgtgtcttaccgggttggactcaagacgatagttaccggataaggcgcagcggtcgggctgaacggggggttcgtgcacacagcccagcttggagcgaacgacctacaccgaact

SEQ ID NO: 197 - DNA, 9879 bp, synthetic construct
  misc_feature 1..9879: note = DNA of V3_D3a-D3l-dCas9-1xGCN4
  source 1..9879: mol_type = other DNA
tcatatatactttagattgatttaaaacttcatttttaatttaaaaggatctaggtgaagatcctttttgataatctcatgaccaaaatcccttaacgtgagttttcgttccactgagcgtcagaccccgtagaaaagatcaaaggatcttcttgagatcctttttttctgcgcgtaatctgctgcttgcaaacaaaaaaaccaccgctaccagcggtggtttgtttgccggatcaagagctaccaactctttttccgaaggtaactggcttcagcagagcgcagataccaaatactgttcttctagtgtagccgtagttaggccaccacttcaagaactctgtagcaccgcctacatacctcgctctgctaatcctgttaccagtggctgctgccagtggcgataagtcgtgtcttaccgggttggactcaagacgatagttaccggataaggcgcagcggtcgggctgaacggggggttcgtgcacacagcccagcttggagcgaacgacctacaccgaactgagatacctacagcgtgagctatgagaaagcgccacgcttcccgaagggagaaaggcggacaggtatccggtaagcggcagggtcggaacaggagagcgcacgagggagcttccagggggaaacgcctggtatctttatagtcctgtcgggtttcgccacctctgacttgagcgtcgatttttgtgatgctcgtcaggggggcggagcctatggaaaaacgccagcaacgcggcctttttacggttcctggccttttgctggccttttgctcacatgttctttcctgcgttatcccctgattctgtggataaccgtattaccgcctttgagtgagctgataccgctcgccgcagccgaacgaccgagcgcagcgagtcagtgagcgaggaagcggaagagcgcccaatacgcaaaccgcctctccccgcgcgttggccgattcattaatgcagctggcacgacaggtttcccgactggaaagcgggcagtgagcgcaacgcaattaatgtgagttagctcactcattaggcaccccaggctttacactttatgcttccggctcgtatgttgtgtggaattgtgagcggataacaatttcacacaggaaacagctatgaccatgattacgcctctagaaagctttaatacgactcactataaggactcactatttgttttcgcgcccagttgcaaaaagtgtcgacatttgcttctgacacaactgtgttcactagcaacctcaaacagacaccgccaccatgcctgctgctaagagagtgaaactggatggatccaaccatgaccaggaatttgaccccccaaaggtttacccacctgtgccagctgagaagaggaagcccatccgcgtgctgtctctctttgatgggattgctacagggctcctggtgctgaaggacctgggcatccaagtggaccgctacattgcctccgaggtgtgtgaggactccatcacggtgggcatggtgcggcaccagggaaagatcatgtacgtcggggacgtccgcagcgtcacacagaagcatatccaggagtggggcccattcgacctggtgattggaggcagtccctgcaatgacctctccattgtcaaccctgcccgcaagggactttatgagggtactggccgcctcttctttgagttctaccgcctcctgcatgatgcgcggcccaaggagggagatgatcgccccttcttctggctctttgagaatgtggtggccatgggcgttagtgacaagagggacatctcgcgatttcttgagtctaaccccgtgatgattgacgccaaagaagtgtctgctgcacacagggcccgttacttctggggtaaccttcctggcatgaacaggcctttggcatccactgtgaatgataagctggagctgcaagagtgtctggagcacggcagaatagccaagttcagcaaagtgaggaccattaccaccaggtcaaactctataaagcagggcaaagaccagcatttccccgtcttcatgaacgagaaggaggacatcctgtggtgcactgaaatggaaagggtgtttggcttccccgtccactacacagacgtctccaacatgagccgcttggcgaggcagagactgctgggccgatcgtggagcgtgccggtcatccgccacctcttcgctccgctgaaggaatattttgcttgtgtgtctagcggcaatagtaacgctaacagccgcgggccgagcttcagcagcggcctggtgccgttaagcttgcgcggcagccatatgggccctatggagatatacaagacagtgtctgcatggaagagacagccagtgcgggtactgagcctcttcagaaacatcgacaaggtactaaagagtttgggcttcttggaaagcggttctggttctgggggaggaacgctgaagtacgtggaagatgtcacaaatgtcgtgaggagagacgtggagaaatggggcccctttgacctggtgtacggctcgacgcagcccctaggcagctcttgtgatcgctgtcccggctggtacatgttccagttccaccggatcctgcagtatgcgctgcctcgccaggagagtcagcggcccttcttctggatattcatggacaatctgctgctgactgaggatgaccaagagacaactacccgcttccttcagacagaggctgtgaccctccaggatgtccgtggcagagactaccagaatgctatgcgggtgtggagcaacattccagggctgaagagcaagcatgcgcccctgaccccaaaggaagaagagtatctgcaagcccaagtcagaagcaggagcaagctggacgccccgaaagttgacctcctggtgaagaactgccttctcccgctgagagagtacttcaagtatttttctcaaaactcacttcctcttggagggccgagctctggcgcacccccaccaagtggagggtctcctgccgggtccccaacatctactgaagaaggcaccagcgaatccgcaacgcccgagtcaggccctggtacctccacagaaccatctgaaggtagtgcgcctggttccccagctggaagccctacttccaccgaagaaggcacgtcaaccgaaccaagtgaaggatctgcccctgggaccagcactgaaccatctgagccaaaaaagaagagaaaggtaatggacaagaagtacagcatcggcctggccatcggcaccaactctgtgggctgggccgtgatcaccgacgagtacaaggtgcccagcaagaaattcaaggtgctgggcaacaccgaccggcacagcatcaagaagaacctgatcggcgccctgctgttcgacagcggagaaacagccgaggccacccggctgaagagaaccgccagaagaagatacaccagacggaagaaccggatctgctatctgcaagagatcttcagcaacgagatggccaaggtggacgacagcttcttccacagactggaagagtccttcctggtggaagaggataagaagcacgagcggcaccccatcttcggcaacatcgtggacgaggtggcctaccacgagaagtaccccaccatctaccacctgagaaagaaactggtggacagcaccgacaaggccgacctgcggctgatctatctggccctggcccacatgatcaagttccggggccacttcctgatcgagggcgacctgaaccccgacaacagcgacgtggacaagctgttcatccagctggtgcagacctacaaccagctgttcgaggaaaaccccatcaacgccagcggcgtggacgccaaggccatcctgtctgccagactgagcaagagcagacggctggaaaatctgatcgcccagctgcccggcgagaagaagaatggcctgttcggcaacctgattgccctgagcctgggcctgacccccaacttcaagagcaacttcgacctggccgaggatgccaaactgcagctgagcaaggacacctacgacgacgacctggacaacctgctggcccagatcggcgaccagtacgccgacctgtttctggccgccaagaacctgtccgacgccatcctgctgagcgacatcctgagagtgaacaccgagatcaccaaggcccccctgagcgcctctatgatcaagagatacgacgagcaccaccaggacctgaccctgctgaaagctctcgtgcggcagcagctgcctgagaagtacaaagagattttcttcgaccagagcaagaacggctacgccggctacatcgatggcggagccagccaggaagagttctacaagttcatcaagcccatcctggaaaagatggacggcaccgaggaactgctcgtgaagctgaacagagaggacctgctgcggaagcagcggaccttcgacaacggcagcatcccccaccagatccacctgggagagctgcacgccattctgcggcggcaggaagatttttacccattcctgaaggacaaccgggaaaagatcgagaagatcctgaccttccgcatcccctactacgtgggccctctggccaggggaaacagcagattcgcctggatgaccagaaagagcgaggaaaccatcaccccctggaacttcgaggaagtggtggacaagggcgccagcgcccagagcttcatcgagcggatgaccaacttcgataagaacctgcccaacgagaaggtgctgcccaagcacagcctgctgtacgagtacttcaccgtgtacaacgagctgaccaaagtgaaatacgtgaccgagggaatgagaaagcccgccttcctgagcggcgagcagaaaaaagccatcgtggacctgctgttcaagaccaaccggaaagtgaccgtgaagcagctgaaagaggactacttcaagaaaatcgagtgcttcgactccgtggaaatctccggcgtggaagatcggttcaacgcctccctgggcacataccacgatctgctgaaaattatcaaggacaaggacttcctggacaatgaggaaaacgaggacattctggaagatatcgtgctgaccctgacactgtttgaggacagagagatgatcgaggaacggctgaaaacctatgcccacctgttcgacgacaaagtgatgaagcagctgaagcggcggagatacaccggctggggcaggctgagccggaagctgatcaacggcatccgggacaagcagtccggcaagacaatcctggatttcctgaagtccgacggcttcgccaacagaaacttcatgcagctgatccacgacgacagcctgacctttaaagaggacatccagaaagcccaggtgtccggccagggcgatagcctgcacgagcacattgccaatctggccggcagccccgccattaagaagggcatcctgcagacagtgaaggtggtggacgagctcgtgaaagtgatgggccggcacaagcccgagaacatcgtgatcgaaatggccagagagaaccagaccacccagaagggacagaagaacagccgcgagagaatgaagcggatcgaagagggcatcaaagagctgggcagccagatcctgaaagaacaccccgtggaaaacacccagctgcagaacgagaagctgtacctgtactacctgcagaatgggcgggatatgtacgtggaccaggaactggacatcaaccggctgtccgactacgatgtggacgctatcgtgcctcagagctttctgaaggacgactccatcgataacaaagtgctgactcggagcgacaagaaccggggcaagagcgacaacgtgccctccgaagaggtcgtgaagaagatgaagaactactggcgccagctgctgaatgccaagctgattacccagaggaagttcgacaatctgaccaaggccgagagaggcggcctgagcgaactggataaggccggcttcatcaagagacagctggtggaaacccggcagatcacaaagcacgtggcacagatcctggactcccggatgaacactaagtacgacgagaacgacaaactgatccgggaagtgaaagtgatcaccctgaagtccaagctggtgtccgatttccggaaggatttccagttttacaaagtgcgcgagatcaacaactaccaccacgcccacgacgcctacctgaacgccgtcgtgggaaccgccctgatcaaaaagtaccctaagctggaaagcgagttcgtgtacggcgactacaaggtgtacgacgtgcggaagatgatcgccaagagcgagcaggaaatcggcaaggctaccgccaagtacttcttctacagcaacatcatgaactttttcaagaccgagattaccctggccaacggcgagatccggaagcggcctctgatcgagacaaacggcgaaacaggcgagatcgtgtgggataagggccgggactttgccaccgtgcggaaagtgctgtctatgccccaagtgaatatcgtgaaaaagaccgaggtgcagacaggcggcttcagcaaagagtctatcctgcccaagaggaacagcgacaagctgatcgccagaaagaaggactgggaccctaagaagtacggcggcttcgacagccccaccgtggcctattctgtgctggtggtggccaaagtggaaaagggcaagtccaagaaactgaagagtgtgaaagagctgctggggatcaccatcatggaaagaagcagcttcgagaagaatcccatcgactttctggaagccaagggctacaaagaagtgaaaaaggacctgatcatcaagctgcctaagtactccctgttcgagctggaaaacggccggaagagaatgctggcctctgccggcgaactgcagaagggaaacgaactggccctgccctccaaatatgtgaacttcctgtacctggccagccactatgagaagctgaagggctcccccgaggataatgagcagaaacagctgtttgtggaacagcacaaacactacctggacgagatcatcgagcagatcagcgagttctccaagagagtgatcctggccgacgctaatctggacaaggtgctgagcgcctacaacaagcacagagacaagcctatcagagagcaggccgagaatatcatccacctgtttaccctgaccaatctgggagcccctgccgccttcaagtactttgacaccaccatcgaccggaagaggtacaccagcaccaaagaggtgctggacgccaccctgatccaccagagcatcaccggcctgtacgagacacggatcgacctgtctcagctgggaggcgacgcctatccctatgacgtgcccgattatgccagcctgggcagcggctcccccaagaaaaaacgcaaggtggaagatcctaagaaaaagcggaaagtggacggcattggtagtgggagcaacggcagcagcggagaggaactgctgagcaagaactaccacctggaaaacgaggtggccagactgaagaaaggctctggctctggcggaagcggttctggcggatcaggatctggaagtggcggctctggaagcggaggttctggatctggcgaagaactgctgtctaagaattatcacggttcaggctccggccagcggggaagcaagcgcaccgccgatggttccgagttcgaaagccccaaaaaaaagcgcaaggtctgagatcccaagcacgcagcaatgcagctcaaaacgcttagcctagccacacccccacgggaaacagcagtgattaacctttagcaataaacgaaagtttaactaagctatactaaccccagggttggtcaatttcgtgccagccacaccctggtactgcatgcacgcaatgctagctgcccctttcccgtcctgggcaccccgagtctcccccgaccccgggtcccaggtatgctcccacctccacctgccccactcaccacctctgctagttccagacacctccgagacgaggaaaaaaaaaaaaaaaaaaaaaaaaaaaaaaaaaaaaaaaaaaaaaaaaaaaaaaaaaaaaaaaaaaaaaaaaaaaaaaaaaaaaaaaaaaaaaaaaaaaaaaaaaaaaaaaaaaaaaaaaaaaaaaaaaaaaaaaaaaaaaaaaaaaaaaaaaaaaaaaaaaaaaaaaaaaaaaaaaaaaaaaaaaaaaaaaaaaaaaaaaaaaaaaaaaaaaaaaaaaaaaaaaaaaaaaaaaaaaaaaaaaaaaaaaaaaaaaaaaaaaaaaaaaaaaaaaaaaaaaaaaaaaaaaaaaaaaaaaaaaaaaaaaaaaaaaaaaaaaaaaaaaaaaaaaaaaaaaaaaaaaaaaaaaaaaaaaaaaaaaaaaaaaaaaaaaaaaaaaaaaaaaaaaaaaaaaaccgtcttcaagctttctagaaattcactggccgtcgttttacaacgtcgtgactgggaaaaccctggcgttacccaacttaatcgccttgcagcacatccccctttcgccagctggcgtaatagcgaagaggcccgcaccgatcgcccttcccaacagttgcgcagcctgaatggcgaatggcgcctgatgcggtattttctccttacgcatctgtgcggtatttcacaccgcatatggtgcactctcagtacaatctgctctgatgccgcatagttaagccagccccgacacccgccaacacccgctgacgcgccctgacgggcttgtctgctcccggcatccgcttacagacaagctgtgaccgtctccgggagctgcatgtgtcagaggttttcaccgtcatcaccgaaacgcgcgagacgaaagggcctcgtgatacgcctatttttataggttaatgtcatgataataatggtttcttagacgtcaggtggcacttttcggggaaatgtgcgcggaacccctatttgtttatttttctaaatacattcaaatatgtatccgctcatgagacaataaccctgataaatgcttcaataatattgaaaaaggaagagtatgagtattcaacatttccgtgtcgcccttattcccttttttgcggcattttgccttcctgtttttgctcacccagaaacgctggtgaaagtaaaagatgctgaagatcagttgggtgcacgagtgggttacatcgaactggatctcaacagcggtaagatccttgagagttttcgccccgaagaacgttttccaatgatgagcacttttaaagttctgctatgtggcgcggtattatcccgtattgacgccgggcaagagcaactcggtcgccgcatacactattctcagaatgacttggttgagtactcaccagtcacagaaaagcatcttacggatggcatgacagtaagagaattatgcagtgctgccataaccatgagtgataacactgcggccaacttacttctgacaacgatcggaggaccgaaggagctaaccgcttttttgcacaacatgggggatcatgtaactcgccttgatcgttgggaaccggagctgaatgaagccataccaaacgacgagcgtgacaccacgatgcctgtagcaatggcaacaacgttgcgcaaactattaactggcgaactacttactctagcttcccggcaacaattaatagactggatggaggcggataaagttgcaggaccacttctgcgctcggcccttccggctggctggtttattgctgataaatctggagccggtgagcgtgggtctcgcggtatcattgcagcactggggccagatggtaagccctcccgtatcgtagttatctacacgacggggagtcaggcaactatggatgaacgaaatagacagatcgctgagataggtgcctcactgattaagcattggtaactgtcagaccaagtttac

SEQ ID NO: 198 - DNA, 9909 bp, synthetic construct
  misc_feature 1..9909: note = DNA of V4_D3a-D3l-dCas9-2xGCN4
  source 1..9909: mol_type = other DNA
tcatatatactttagattgatttaaaacttcatttttaatttaaaaggatctaggtgaagatcctttttgataatctcatgaccaaaatcccttaacgtgagttttcgttccactgagcgtcagaccccgtagaaaagatcaaaggatcttcttgagatcctttttttctgcgcgtaatctgctgcttgcaaacaaaaaaaccaccgctaccagcggtggtttgtttgccggatcaagagctaccaactctttttccgaaggtaactggcttcagcagagcgcagataccaaatactgttcttctagtgtagccgtagttaggccaccacttcaagaactctgtagcaccgcctacatacctcgctctgctaatcctgttaccagtggctgctgccagtggcgataagtcgtgtcttaccgggttggactcaagacgatagttaccggataaggcgcagcggtcgggctgaacggggggttcgtgcacacagcccagcttggagcgaacgacctacaccgaactgagatacctacagcgtgagctatgagaaagcgccacgcttcccgaagggagaaaggcggacaggtatccggtaagcggcagggtcggaacaggagagcgcacgagggagcttccagggggaaacgcctggtatctttatagtcctgtcgggtttcgccacctctgacttgagcgtcgatttttgtgatgctcgtcaggggggcggagcctatggaaaaacgccagcaacgcggcctttttacggttcctggccttttgctggccttttgctcacatgttctttcctgcgttatcccctgattctgtggataaccgtattaccgcctttgagtgagctgataccgctcgccgcagccgaacgaccgagcgcagcgagtcagtgagcgaggaagcggaagagcgcccaatacgcaaaccgcctctccccgcgcgttggccgattcattaatgcagctggcacgacaggtttcccgactggaaagcgggcagtgagcgcaacgcaattaatgtgagttagctcactcattaggcaccccaggctttacactttatgcttccggctcgtatgttgtgtggaattgtgagcggataacaatttcacacaggaaacagctatgaccatgattacgcctctagaaagctttaatacgactcactataaggactcactatttgttttcgcgcccagttgcaaaaagtgtcgacatttgcttctgacacaactgtgttcactagcaacctcaaacagacaccgccaccatgcctgctgctaagagagtgaaactggatggatccaaccatgaccaggaatttgaccccccaaaggtttacccacctgtgccagctgagaagaggaagcccatccgcgtgctgtctctctttgatgggattgctacagggctcctggtgctgaaggacctgggcatccaagtggaccgctacattgcctccgaggtgtgtgaggactccatcacggtgggcatggtgcggcaccagggaaagatcatgtacgtcggggacgtccgcagcgtcacacagaagcatatccaggagtggggcccattcgacctggtgattggaggcagtccctgcaatgacctctccattgtcaaccctgcccgcaagggactttatgagggtactggccgcctcttctttgagttctaccgcctcctgcatgatgcgcggcccaaggagggagatgatcgccccttcttctggctctttgagaatgtggtggccatgggcgttagtgacaagagggacatctcgcgatttcttgagtctaaccccgtgatgattgacgccaaagaagtgtctgctgcacacagggcccgttacttctggggtaaccttcctggcatgaacaggcctttggcatccactgtgaatgataagctggagctgcaagagtgtctggagcacggcagaatagccaagttcagcaaagtgaggaccattaccaccaggtcaaactctataaagcagggcaaagaccagcatttccccgtcttcatgaacgagaaggaggacatcctgtggtgcactgaaatggaaagggtgtttggcttccccgtccactacacagacgtctccaacatgagccgcttggcgaggcagagactgctgggccgatcgtggagcgtgccggtcatccgccacctcttcgctccgctgaaggaatattttgcttgtgtgtctagcggcaatagtaacgctaacagccgcgggccgagcttcagcagcggcctggtgccgttaagcttgcgcggcagccatatgggccctatggagatatacaagacagtgtctgcatggaagagacagccagtgcgggtactgagcctcttcagaaacatcgacaaggtactaaagagtttgggcttcttggaaagcggttctggttctgggggaggaacgctgaagtacgtggaagatgtcacaaatgtcgtgaggagagacgtggagaaatggggcccctttgacctggtgtacggctcgacgcagcccctaggcagctcttgtgatcgctgtcccggctggtacatgttccagttccaccggatcctgcagtatgcgctgcctcgccaggagagtcagcggcccttcttctggatattcatggacaatctgctgctgactgaggatgaccaagagacaactacccgcttccttcagacagaggctgtgaccctccaggatgtccgtggcagagactaccagaatgctatgcgggtgtggagcaacattccagggctgaagagcaagcatgcgcccctgaccccaaaggaagaagagtatctgcaagcccaagtcagaagcaggagcaagctggacgccccgaaagttgacctcctggtgaagaactgccttctcccgctgagagagtacttcaagtatttttctcaaaactcacttcctcttggagggccgagctctggcgcacccccaccaagtggagggtctcctgccgggtccccaacatctactgaagaaggcaccagcgaatccgcaacgcccgagtcaggccctggtacctccacagaaccatctgaaggtagtgcgcctggttccccagctggaagccctacttccaccgaagaaggcacgtcaaccgaaccaagtgaaggatctgcccctgggaccagcactgaaccatctgagccaaaaaagaagagaaaggtaatggacaagaagtacagcatcggcctggccatcggcaccaactctgtgggctgggccgtgatcaccgacgagtacaaggtgcccagcaagaaattcaaggtgctgggcaacaccgaccggcacagcatcaagaagaacctgatcggcgccctgctgttcgacagcggagaaacagccgaggccacccggctgaagagaaccgccagaagaagatacaccagacggaagaaccggatctgctatctgcaagagatcttcagcaacgagatggccaaggtggacgacagcttcttccacagactggaagagtccttcctggtggaagaggataagaagcacgagcggcaccccatcttcggcaacatcgtggacgaggtggcctaccacgagaagtaccccaccatctaccacctgagaaagaaactggtggacagcaccgacaaggccgacctgcggctgatctatctggccctggcccacatgatcaagttccggggccacttcctgatcgagggcgacctgaaccccgacaacagcgacgtggacaagctgttcatccagctggtgcagacctacaaccagctgttcgaggaaaaccccatcaacgccagcggcgtggacgccaaggccatcctgtctgccagactgagcaagagcagacggctggaaaatctgatcgcccagctgcccggcgagaagaagaatggcctgttcggcaacctgattgccctgagcctgggcctgacccccaacttcaagagcaacttcgacctggccgaggatgccaaactgcagctgagcaaggacacctacgacgacgacctggacaacctgctggcccagatcggcgaccagtacgccgacctgtttctggccgccaagaacctgtccgacgccatcctgctgagcgacatcctgagagtgaacaccgagatcaccaaggcccccctgagcgcctctatgatcaagagatacgacgagcaccaccaggacctgaccctgctgaaagctctcgtgcggcagcagctgcctgagaagtacaaagagattttcttcgaccagagcaagaacggctacgccggctacatcgatggcggagccagccaggaagagttctacaagttcatcaagcccatcctggaaaagatggacggcaccgaggaactgctcgtgaagctgaacagagaggacctgctgcggaagcagcggaccttcgacaacggcagcatcccccaccagatccacctgggagagctgcacgccattctgcggcggcaggaagatttttacccattcctgaaggacaaccgggaaaagatcgagaagatcctgaccttccgcatcccctactacgtgggccctctggccaggggaaacagcagattcgcctggatgaccagaaagagcgaggaaaccatcaccccctggaacttcgaggaagtggtggacaagggcgccagcgcccagagcttcatcgagcggatgaccaacttcgataagaacctgcccaacgagaaggtgctgcccaagcacagcctgctgtacgagtacttcaccgtgtacaacgagctgaccaaagtgaaatacgtgaccgagggaatgagaaagcccgccttcctgagcggcgagcagaaaaaagccatcgtggacctgctgttcaagaccaaccggaaagtgaccgtgaagcagctgaaagaggactacttcaagaaaatcgagtgcttcgactccgtggaaatctccggcgtggaagatcggttcaacgcctccctgggcacataccacgatctgctgaaaattatcaaggacaaggacttcctggacaatgaggaaaacgaggacattctggaagatatcgtgctgaccctgacactgtttgaggacagagagatgatcgaggaacggctgaaaacctatgcccacctgttcgacgacaaagtgatgaagcagctgaagcggcggagatacaccggctggggcaggctgagccggaagctgatcaacggcatccgggacaagcagtccggcaagacaatcctggatttcctgaagtccgacggcttcgccaacagaaacttcatgcagctgatccacgacgacagcctgacctttaaagaggacatccagaaagcccaggtgtccggccagggcgatagcctgcacgagcacattgccaatctggccggcagccccgccattaagaagggcatcctgcagacagtgaaggtggtggacgagctcgtgaaagtgatgggccggcacaagcccgagaacatcgtgatcgaaatggccagagagaaccagaccacccagaagggacagaagaacagccgcgagagaatgaagcggatcgaagagggcatcaaagagctgggcagccagatcctgaaagaacaccccgtggaaaacacccagctgcagaacgagaagctgtacctgtactacctgcagaatgggcgggatatgtacgtggaccaggaactggacatcaaccggctgtccgactacgatgtggacgctatcgtgcctcagagctttctgaaggacgactccatcgataacaaagtgctgactcggagcgacaagaaccggggcaagagcgacaacgtgccctccgaagaggtcgtgaagaagatgaagaactactggcgccagctgctgaatgccaagctgattacccagaggaagttcgacaatctgaccaaggccgagagaggcggcctgagcgaactggataaggccggcttcatcaagagacagctggtggaaacccggcagatcacaaagcacgtggcacagatcctggactcccggatgaacactaagtacgacgagaacgacaaactgatccgggaagtgaaagtgatcaccctgaagtccaagctggtgtccgatttccggaaggatttccagttttacaaagtgcgcgagatcaacaactaccaccacgcccacgacgcctacctgaacgccgtcgtgggaaccgccctgatcaaaaagtaccctaagctggaaagcgagttcgtgtacggcgactacaaggtgtacgacgtgcggaagatgatcgccaagagcgagcaggaaatcggcaaggctaccgccaagtacttcttctacagcaacatcatgaactttttcaagaccgagattaccctggccaacggcgagatccggaagcggcctctgatcgagacaaacggcgaaacaggcgagatcgtgtgggataagggccgggactttgccaccgtgcggaaagtgctgtctatgccccaagtgaatatcgtgaaaaagaccgaggtgcagacaggcggcttcagcaaagagtctatcctgcccaagaggaacagcgacaagctgatcgccagaaagaaggactgggaccctaagaagtacggcggcttcgacagccccaccgtggcctattctgtgctggtggtggccaaagtggaaaagggcaagtccaagaaactgaagagtgtgaaagagctgctggggatcaccatcatggaaagaagcagcttcgagaagaatcccatcgactttctggaagccaagggctacaaagaagtgaaaaaggacctgatcatcaagctgcctaagtactccctgttcgagctggaaaacggccggaagagaatgctggcctctgccggcgaactgcagaagggaaacgaactggccctgccctccaaatatgtgaacttcctgtacctggccagccactatgagaagctgaagggctcccccgaggataatgagcagaaacagctgtttgtggaacagcacaaacactacctggacgagatcatcgagcagatcagcgagttctccaagagagtgatcctggccgacgctaatctggacaaggtgctgagcgcctacaacaagcacagagacaagcctatcagagagcaggccgagaatatcatccacctgtttaccctgaccaatctgggagcccctgccgccttcaagtactttgacaccaccatcgaccggaagaggtacaccagcaccaaagaggtgctggacgccaccctgatccaccagagcatcaccggcctgtacgagacacggatcgacctgtctcagctgggaggcgacgcctatccctatgacgtgcccgattatgccagcctgggcagcggctcccccaagaaaaaacgcaaggtggaagatcctaagaaaaagcggaaagtggacggcattggtagtgggagcaacggcagcagcggagaggaactgctgagcaagaactaccacctggaaaacgaggtggccagactgaagaaaggctctggctctggcggaagcggttctggcggatcaggatctggaagtggcggctctggaagcggaggttctggatctggcgaagaactgctgtctaagaattatcacctcgagaatgaagtcgctcgtttgaagaaaggttcaggctccggccagcggggaagcaagcgcaccgccgatggttccgagttcgaaagccccaaaaaaaagcgcaaggtctgagatcccaagcacgcagcaatgcagctcaaaacgcttagcctagccacacccccacgggaaacagcagtgattaacctttagcaataaacgaaagtttaactaagctatactaaccccagggttggtcaatttcgtgccagccacaccctggtactgcatgcacgcaatgctagctgcccctttcccgtcctgggcaccccgagtctcccccgaccccgggtcccaggtatgctcccacctccacctgccccactcaccacctctgctagttccagacacctccgagacgaggaaaaaaaaaaaaaaaaaaaaaaaaaaaaaaaaaaaaaaaaaaaaaaaaaaaaaaaaaaaaaaaaaaaaaaaaaaaaaaaaaaaaaaaaaaaaaaaaaaaaaaaaaaaaaaaaaaaaaaaaaaaaaaaaaaaaaaaaaaaaaaaaaaaaaaaaaaaaaaaaaaaaaaaaaaaaaaaaaaaaaaaaaaaaaaaaaaaaaaaaaaaaaaaaaaaaaaaaaaaaaaaaaaaaaaaaaaaaaaaaaaaaaaaaaaaaaaaaaaaaaaaaaaaaaaaaaaaaaaaaaaaaaaaaaaaaaaaaaaaaaaaaaaaaaaaaaaaaaaaaaaaaaaaaaaaaaaaaaaaaaaaaaaaaaaaaaaaaaaaaaaaaaaaaaaaaaaaaaaaaaaaaaaaaaaaaaaccgtcttcaagctttctagaaattcactggccgtcgttttacaacgtcgtgactgggaaaaccctggcgttacccaacttaatcgccttgcagcacatccccctttcgccagctggcgtaatagcgaagaggcccgcaccgatcgcccttcccaacagttgcgcagcctgaatggcgaatggcgcctgatgcggtattttctccttacgcatctgtgcggtatttcacaccgcatatggtgcactctcagtacaatctgctctgatgccgcatagttaagccagccccgacacccgccaacacccgctgacgcgccctgacgggcttgtctgctcccggcatccgcttacagacaagctgtgaccgtctccgggagctgcatgtgtcagaggttttcaccgtcatcaccgaaacgcgcgagacgaaagggcctcgtgatacgcctatttttataggttaatgtcatgataataatggtttcttagacgtcaggtggcacttttcggggaaatgtgcgcggaacccctatttgtttatttttctaaatacattcaaatatgtatccgctcatgagacaataaccctgataaatgcttcaataatattgaaaaaggaagagtatgagtattcaacatttccgtgtcgcccttattcccttttttgcggcattttgccttcctgtttttgctcacccagaaacgctggtgaaagtaaaagatgctgaagatcagttgggtgcacgagtgggttacatcgaactggatctcaacagcggtaagatccttgagagttttcgccccgaagaacgttttccaatgatgagcacttttaaagttctgctatgtggcgcggtattatcccgtattgacgccgggcaagagcaactcggtcgccgcatacactattctcagaatgacttggttgagtactcaccagtcacagaaaagcatcttacggatggcatgacagtaagagaattatgcagtgctgccataaccatgagtgataacactgcggccaacttacttctgacaacgatcggaggaccgaaggagctaaccgcttttttgcacaacatgggggatcatgtaactcgccttgatcgttgggaaccggagctgaatgaagccataccaaacgacgagcgtgacaccacgatgcctgtagcaatggcaacaacgttgcgcaaactattaactggcgaactacttactctagcttcccggcaacaattaatagactggatggaggcggataaagttgcaggaccacttctgcgctcggcccttccggctggctggtttattgctgataaatctggagccggtgagcgtgggtctcgcggtatcattgcagcactggggccagatggtaagccctcccgtatcgtagttatctacacgacggggagtcaggcaactatggatgaacgaaatagacagatcgctgagataggtgcctcactgattaagcattggtaactgtcagaccaagtttac

SEQ ID NO: 199 - DNA, 10185 bp, synthetic construct
  misc_feature 1..10185: note = DNA of V5_D3a-D3l-dCas9-4xGCN4
  source 1..10185: mol_type = other DNA
tcatatatactttagattgatttaaaacttcatttttaatttaaaaggatctaggtgaagatcctttttgataatctcatgaccaaaatcccttaacgtgagttttcgttccactgagcgtcagaccccgtagaaaagatcaaaggatcttcttgagatcctttttttctgcgcgtaatctgctgcttgcaaacaaaaaaaccaccgctaccagcggtggtttgtttgccggatcaagagctaccaactctttttccgaaggtaactggcttcagcagagcgcagataccaaatactgttcttctagtgtagccgtagttaggccaccacttcaagaactctgtagcaccgcctacatacctcgctctgctaatcctgttaccagtggctgctgccagtggcgataagtcgtgtcttaccgggttggactcaagacgatagttaccggataaggcgcagcggtcgggctgaacggggggttcgtgcacacagcccagcttggagcgaacgacctacaccgaactgagatacctacagcgtgagctatgagaaagcgccacgcttcccgaagggagaaaggcggacaggtatccggtaagcggcagggtcggaacaggagagcgcacgagggagcttccagggggaaacgcctggtatctttatagtcctgtcgggtttcgccacctctgacttgagcgtcgatttttgtgatgctcgtcaggggggcggagcctatggaaaaacgccagcaacgcggcctttttacggttcctggccttttgctggccttttgctcacatgttctttcctgcgttatcccctgattctgtggataaccgtattaccgcctttgagtgagctgataccgctcgccgcagccgaacgaccgagcgcagcgagtcagtgagcgaggaagcggaagagcgcccaatacgcaaaccgcctctccccgcgcgttggccgattcattaatgcagctggcacgacaggtttcccgactggaaagcgggcagtgagcgcaacgcaattaatgtgagttagctcactcattaggcaccccaggctttacactttatgcttccggctcgtatgttgtgtggaattgtgagcggataacaatttcacacaggaaacagctatgaccatgattacgcctctagaaagctttaatacgactcactataaggactcactatttgttttcgcgcccagttgcaaaaagtgtcgacatttgcttctgacacaactgtgttcactagcaacctcaaacagacaccgccaccatgcctgctgctaagagagtgaaactggatggatccaaccatgaccaggaatttgaccccccaaaggtttacccacctgtgccagctgagaagaggaagcccatccgcgtgctgtctctctttgatgggattgctacagggctcctggtgctgaaggacctgggcatccaagtggaccgctacattgcctccgaggtgtgtgaggactccatcacggtgggcatggtgcggcaccagggaaagatcatgtacgtcggggacgtccgcagcgtcacacagaagcatatccaggagtggggcccattcgacctggtgattggaggcagtccctgcaatgacctctccattgtcaaccctgcccgcaagggactttatgagggtactggccgcctcttctttgagttctaccgcctcctgcatgatgcgcggcccaaggagggagatgatcgccccttcttctggctctttgagaatgtggtggccatgggcgttagtgacaagagggacatctcgcgatttcttgagtctaaccccgtgatgattgacgccaaagaagtgtctgctgcacacagggcccgttacttctggggtaaccttcctggcatgaacaggcctttggcatccactgtgaatgataagctggagctgcaagagtgtctggagcacggcagaatagccaagttcagcaaagtgaggaccattaccaccaggtcaaactctataaagcagggcaaagaccagcatttccccgtcttcatgaacgagaaggaggacatcctgtggtgcactgaaatggaaagggtgtttggcttccccgtccactacacagacgtctccaacatgagccgcttggcgaggcagagactgctgggccgatcgtggagcgtgccggtcatccgccacctcttcgctccgctgaaggaatattttgcttgtgtgtctagcggcaatagtaacgctaacagccgcgggccgagcttcagcagcggcctggtgccgttaagcttgcgcggcagccatatgggccctatggagatatacaagacagtgtctgcatggaagagacagccagtgcgggtactgagcctcttcagaaacatcgacaaggtactaaagagtttgggcttcttggaaagcggttctggttctgggggaggaacgctgaagtacgtggaagatgtcacaaatgtcgtgaggagagacgtggagaaatggggcccctttgacctggtgtacggctcgacgcagcccctaggcagctcttgtgatcgctgtcccggctggtacatgttccagttccaccggatcctgcagtatgcgctgcctcgccaggagagtcagcggcccttcttctggatattcatggacaatctgctgctgactgaggatgaccaagagacaactacccgcttccttcagacagaggctgtgaccctccaggatgtccgtggcagagactaccagaatgctatgcgggtgtggagcaacattccagggctgaagagcaagcatgcgcccctgaccccaaaggaagaagagtatctgcaagcccaagtcagaagcaggagcaagctggacgccccgaaagttgacctcctggtgaagaactgccttctcccgctgagagagtacttcaagtatttttctcaaaactcacttcctcttggagggccgagctctggcgcacccccaccaagtggagggtctcctgccgggtccccaacatctactgaagaaggcaccagcgaatccgcaacgcccgagtcaggccctggtacctccacagaaccatctgaaggtagtgcgcctggttccccagctggaagccctacttccaccgaagaaggcacgtcaaccgaaccaagtgaaggatctgcccctgggaccagcactgaaccatctgagccaaaaaagaagagaaaggtaatggacaagaagtacagcatcggcctggccatcggcaccaactctgtgggctgggccgtgatcaccgacgagtacaaggtgcccagcaagaaattcaaggtgctgggcaacaccgaccggcacagcatcaagaagaacctgatcggcgccctgctgttcgacagcggagaaacagccgaggccacccggctgaagagaaccgccagaagaagatacaccagacggaagaaccggatctgctatctgcaagagatcttcagcaacgagatggccaaggtggacgacagcttcttccacagactggaagagtccttcctggtggaagaggataagaagcacgagcggcaccccatcttcggcaacatcgtggacgaggtggcctaccacgagaagtaccccaccatctaccacctgagaaagaaactggtggacagcaccgacaaggccgacctgcggctgatctatctggccctggcccacatgatcaagttccggggccacttcctgatcgagggcgacctgaaccccgacaacagcgacgtggacaagctgttcatccagctggtgcagacctacaaccagctgttcgaggaaaaccccatcaacgccagcggcgtggacgccaaggccatcctgtctgccagactgagcaagagcagacggctggaaaatctgatcgcccagctgcccggcgagaagaagaatggcctgttcggcaacctgattgccctgagcctgggcctgacccccaacttcaagagcaacttcgacctggccgaggatgccaaactgcagctgagcaaggacacctacgacgacgacctggacaacctgctggcccagatcggcgaccagtacgccgacctgtttctggccgccaagaacctgtccgacgccatcctgctgagcgacatcctgagagtgaacaccgagatcaccaaggcccccctgagcgcctctatgatcaagagatacgacgagcaccaccaggacctgaccctgctgaaagctctcgtgcggcagcagctgcctgagaagtacaaagagattttcttcgaccagagcaagaacggctacgccggctacatcgatggcggagccagccaggaagagttctacaagttcatcaagcccatcctggaaaagatggacggcaccgaggaactgctcgtgaagctgaacagagaggacctgctgcggaagcagcggaccttcgacaacggcagcatcccccaccagatccacctgggagagctgcacgccattctgcggcggcaggaagatttttacccattcctgaaggacaaccgggaaaagatcgagaagatcctgaccttccgcatcccctactacgtgggccctctggccaggggaaacagcagattcgcctggatgaccagaaagagcgaggaaaccatcaccccctggaacttcgaggaagtggtggacaagggcgccagcgcccagagcttcatcgagcggatgaccaacttcgataagaacctgcccaacgagaaggtgctgcccaagcacagcctgctgtacgagtacttcaccgtgtacaacgagctgaccaaagtgaaatacgtgaccgagggaatgagaaagcccgccttcctgagcggcgagcagaaaaaagccatcgtggacctgctgttcaagaccaaccggaaagtgaccgtgaagcagctgaaagaggactacttcaagaaaatcgagtgcttcgactccgtggaaatctccggcgtggaagatcggttcaacgcctccctgggcacataccacgatctgctgaaaattatcaaggacaaggacttcctggacaatgaggaaaacgaggacattctggaagatatcgtgctgaccctgacactgtttgaggacagagagatgatcgaggaacggctgaaaacctatgcccacctgttcgacgacaaagtgatgaagcagctgaagcggcggagatacaccggctggggcaggctgagccggaagctgatcaacggcatccgggacaagcagtccggcaagacaatcctggatttcctgaagtccgacggcttcgccaacagaaacttcatgcagctgatccacgacgacagcctgacctttaaagaggacatccagaaagcccaggtgtccggccagggcgatagcctgcacgagcacattgccaatctggccggcagccccgccattaagaagggcatcctgcagacagtgaaggtggtggacgagctcgtgaaagtgatgggccggcacaagcccgagaacatcgtgatcgaaatggccagagagaaccagaccacccagaagggacagaagaacagccgcgagagaatgaagcggatcgaagagggcatcaaagagctgggcagccagatcctgaaagaacaccccgtggaaaacacccagctgcagaacgagaagctgtacctgtactacctgcagaatgggcgggatatgtacgtggaccaggaactggacatcaaccggctgtccgactacgatgtggacgctatcgtgcctcagagctttctgaaggacgactccatcgataacaaagtgctgactcggagcgacaagaaccggggcaagagcgacaacgtgccctccgaagaggtcgtgaagaagatgaagaactactggcgccagctgctgaatgccaagctgattacccagaggaagttcgacaatctgaccaaggccgagagaggcggcctgagcgaactggataaggccggcttcatcaagagacagctggtggaaacccggcagatcacaaagcacgtggcacagatcctggactcccggatgaacactaagtacgacgagaacgacaaactgatccgggaagtgaaagtgatcaccctgaagtccaagctggtgtccgatttccggaaggatttccagttttacaaagtgcgcgagatcaacaactaccaccacgcccacgacgcctacctgaacgccgtcgtgggaaccgccctgatcaaaaagtaccctaagctggaaagcgagttcgtgtacggcgactacaaggtgtacgacgtgcggaagatgatcgccaagagcgagcaggaaatcggcaaggctaccgccaagtacttcttctacagcaacatcatgaactttttcaagaccgagattaccctggccaacggcgagatccggaagcggcctctgatcgagacaaacggcgaaacaggcgagatcgtgtgggataagggccgggactttgccaccgtgcggaaagtgctgtctatgccccaagtgaatatcgtgaaaaagaccgaggtgcagacaggcggcttcagcaaagagtctatcctgcccaagaggaacagcgacaagctgatcgccagaaagaaggactgggaccctaagaagtacggcggcttcgacagccccaccgtggcctattctgtgctggtggtggccaaagtggaaaagggcaagtccaagaaactgaagagtgtgaaagagctgctggggatcaccatcatggaaagaagcagcttcgagaagaatcccatcgactttctggaagccaagggctacaaagaagtgaaaaaggacctgatcatcaagctgcctaagtactccctgttcgagctggaaaacggccggaagagaatgctggcctctgccggcgaactgcagaagggaaacgaactggccctgccctccaaatatgtgaacttcctgtacctggccagccactatgagaagctgaagggctcccccgaggataatgagcagaaacagctgtttgtggaacagcacaaacactacctggacgagatcatcgagcagatcagcgagttctccaagagagtgatcctggccgacgctaatctggacaaggtgctgagcgcctacaacaagcacagagacaagcctatcagagagcaggccgagaatatcatccacctgtttaccctgaccaatctgggagcccctgccgccttcaagtactttgacaccaccatcgaccggaagaggtacaccagcaccaaagaggtgctggacgccaccctgatccaccagagcatcaccggcctgtacgagacacggatcgacctgtctcagctgggaggcgacgcctatccctatgacgtgcccgattatgccagcctgggcagcggctcccccaagaaaaaacgcaaggtggaagatcctaagaaaaagcggaaagtggacggcattggtagtgggagcaacggcagcagcggagaggaactgctgagcaagaactaccacctggaaaacgaggtggccagactgaagaaaggctctggctctggcggaagcggttctggcggatcaggatctggaagtggcggctctggaagcggaggttctggatctggcgaagaactgctgtctaagaattatcacctcgagaacgaagtcgcccgcctcaagaaaggttctggcagcggaggctctggcagtggtggtagcggaagtggaagtggtggcagtggtagcggtggatctggaagcggcgaggaactcctgtcaaagaattaccatctcgaaaacgaggtcgcaaggctcaagaaaggctcaggatcaggcggctctggatccggcggttctggttccggctcaggtggaagtggatctggcggctcaggttccggcgaagaattgctttccaagaactaccatttggaaaatgaagtcgctcgtttgaagaaaggttcaggctccggccagcggggaagcaagcgcaccgccgatggttccgagttcgaaagccccaaaaaaaagcgcaaggtctgagatcccaagcacgcagcaatgcagctcaaaacgcttagcctagccacacccccacgggaaacagcagtgattaacctttagcaataaacgaaagtttaactaagctatactaaccccagggttggtcaatttcgtgccagccacaccctggtactgcatgcacgcaatgctagctgcccctttcccgtcctgggcaccccgagtctcccccgaccccgggtcccaggtatgctcccacctccacctgccccactcaccacctctgctagttccagacacctccgagacgaggaaaaaaaaaaaaaaaaaaaaaaaaaaaaaaaaaaaaaaaaaaaaaaaaaaaaaaaaaaaaaaaaaaaaaaaaaaaaaaaaaaaaaaaaaaaaaaaaaaaaaaaaaaaaaaaaaaaaaaaaaaaaaaaaaaaaaaaaaaaaaaaaaaaaaaaaaaaaaaaaaaaaaaaaaaaaaaaaaaaaaaaaaaaaaaaaaaaaaaaaaaaaaaaaaaaaaaaaaaaaaaaaaaaaaaaaaaaaaaaaaaaaaaaaaaaaaaaaaaaaaaaaaaaaaaaaaaaaaaaaaaaaaaaaaaaaaaaaaaaaaaaaaaaaaaaaaaaaaaaaaaaaaaaaaaaaaaaaaaaaaaaaaaaaaaaaaaaaaaaaaaaaaaaaaaaaaaaaaaaaaaaaaaaaaaaaaaccgtcttcaagctttctagaaattcactggccgtcgttttacaacgtcgtgactgggaaaaccctggcgttacccaacttaatcgccttgcagcacatccccctttcgccagctggcgtaatagcgaagaggcccgcaccgatcgcccttcccaacagttgcgcagcctgaatggcgaatggcgcctgatgcggtattttctccttacgcatctgtgcggtatttcacaccgcatatggtgcactctcagtacaatctgctctgatgccgcatagttaagccagccccgacacccgccaacacccgctgacgcgccctgacgggcttgtctgctcccggcatccgcttacagacaagctgtgaccgtctccgggagctgcatgtgtcagaggttttcaccgtcatcaccgaaacgcgcgagacgaaagggcctcgtgatacgcctatttttataggttaatgtcatgataataatggtttcttagacgtcaggtggcacttttcggggaaatgtgcgcggaacccctatttgtttatttttctaaatacattcaaatatgtatccgctcatgagacaataaccctgataaatgcttcaataatattgaaaaaggaagagtatgagtattcaacatttccgtgtcgcccttattcccttttttgcggcattttgccttcctgtttttgctcacccagaaacgctggtgaaagtaaaagatgctgaagatcagttgggtgcacgagtgggttacatcgaactggatctcaacagcggtaagatccttgagagttttcgccccgaagaacgttttccaatgatgagcacttttaaagttctgctatgtggcgcggtattatcccgtattgacgccgggcaagagcaactcggtcgccgcatacactattctcagaatgacttggttgagtactcaccagtcacagaaaagcatcttacggatggcatgacagtaagagaattatgcagtgctgccataaccatgagtgataacactgcggccaacttacttctgacaacgatcggaggaccgaaggagctaaccgcttttttgcacaacatgggggatcatgtaactcgccttgatcgttgggaaccggagctgaatgaagccataccaaacgacgagcgtgacaccacgatgcctgtagcaatggcaacaacgttgcgcaaactattaactggcgaactacttactctagcttcccggcaacaattaatagactggatggaggcggataaagttgcaggaccacttctgcgctcggcccttccggctggctggtttattgctgataaatctggagccggtgagcgtgggtctcgcggtatcattgcagcactggggccagatggtaagccctcccgtatcgtagttatctacacgacggggagtcaggcaactatggatgaacgaaatagacagatcgctgagataggtgcctcactgattaagcattggtaactgtcagaccaagtttac

SEQ ID NO: 200 - DNA, 11013 bp, synthetic construct
  misc_feature 1..11013: note = DNA of V6_D3a-D3l-dCas9-10xGCN4
  source 1..11013: mol_type = other DNA
tcatatatactttagattgatttaaaacttcatttttaatttaaaaggatctaggtgaagatcctttttgataatctcatgaccaaaatcccttaacgtgagttttcgttccactgagcgtcagaccccgtagaaaagatcaaaggatcttcttgagatcctttttttctgcgcgtaatctgctgcttgcaaacaaaaaaaccaccgctaccagcggtggtttgtttgccggatcaagagctaccaactctttttccgaaggtaactggcttcagcagagcgcagataccaaatactgttcttctagtgtagccgtagttaggccaccacttcaagaactctgtagcaccgcctacatacctcgctctgctaatcctgttaccagtggctgctgccagtggcgataagtcgtgtcttaccgggttggactcaagacgatagttaccggataaggcgcagcggtcgggctgaacggggggttcgtgcacacagcccagcttggagcgaacgacctacaccgaactgagatacctacagcgtgagctatgagaaagcgccacgcttcccgaagggagaaaggcggacaggtatccggtaagcggcagggtcggaacaggagagcgcacgagggagcttccagggggaaacgcctggtatctttatagtcctgtcgggtttcgccacctctgacttgagcgtcgatttttgtgatgctcgtcaggggggcggagcctatggaaaaacgccagcaacgcggcctttttacggttcctggccttttgctggccttttgctcacatgttctttcctgcgttatcccctgattctgtggataaccgtattaccgcctttgagtgagctgataccgctcgccgcagccgaacgaccgagcgcagcgagtcagtgagcgaggaagcggaagagcgcccaatacgcaaaccgcctctccccgcgcgttggccgattcattaatgcagctggcacgacaggtttcccgactggaaagcgggcagtgagcgcaacgcaattaatgtgagttagctcactcattaggcaccccaggctttacactttatgcttccggctcgtatgttgtgtggaattgtgagcggataacaatttcacacaggaaacagctatgaccatgattacgcctctagaaagctttaatacgactcactataaggactcactatttgttttcgcgcccagttgcaaaaagtgtcgacatttgcttctgacacaactgtgttcactagcaacctcaaacagacaccgccaccatgcctgctgctaagagagtgaaactggatggatccaaccatgaccaggaatttgaccccccaaaggtttacccacctgtgccagctgagaagaggaagcccatccgcgtgctgtctctctttgatgggattgctacagggctcctggtgctgaaggacctgggcatccaagtggaccgctacattgcctccgaggtgtgtgaggactccatcacggtgggcatggtgcggcaccagggaaagatcatgtacgtcggggacgtccgcagcgtcacacagaagcatatccaggagtggggcccattcgacctggtgattggaggcagtccctgcaatgacctctccattgtcaaccctgcccgcaagggactttatgagggtactggccgcctcttctttgagttctaccgcctcctgcatgatgcgcggcccaaggagggagatgatcgccccttcttctggctctttgagaatgtggtggccatgggcgttagtgacaagagggacatctcgcgatttcttgagtctaaccccgtgatgattgacgccaaagaagtgtctgctgcacacagggcccgttacttctggggtaaccttcctggcatgaacaggcctttggcatccactgtgaatgataagctggagctgcaagagtgtctggagcacggcagaatagccaagttcagcaaagtgaggaccattaccaccaggtcaaactctataaagcagggcaaagaccagcatttccccgtcttcatgaacgagaaggaggacatcctgtggtgcactgaaatggaaagggtgtttggcttccccgtccactacacagacgtctccaacatgagccgcttggcgaggcagagactgctgggccgatcgtggagcgtgccggtcatccgccacctcttcgctccgctgaaggaatattttgcttgtgtgtctagcggcaatagtaacgctaacagccgcgggccgagcttcagcagcggcctggtgccgttaagcttgcgcggcagccatatgggccctatggagatatacaagacagtgtctgcatggaagagacagccagtgcgggtactgagcctcttcagaaacatcgacaaggtactaaagagtttgggcttcttggaaagcggttctggttctgggggaggaacgctgaagtacgtggaagatgtcacaaatgtcgtgaggagagacgtggagaaatggggcccctttgacctggtgtacggctcgacgcagcccctaggcagctcttgtgatcgctgtcccggctggtacatgttccagttccaccggatcctgcagtatgcgctgcctcgccaggagagtcagcggcccttcttctggatattcatggacaatctgctgctgactgaggatgaccaagagacaactacccgcttccttcagacagaggctgtgaccctccaggatgtccgtggcagagactaccagaatgctatgcgggtgtggagcaacattccagggctgaagagcaagcatgcgcccctgaccccaaaggaagaagagtatctgcaagcccaagtcagaagcaggagcaagctggacgccccgaaagttgacctcctggtgaagaactgccttctcccgctgagagagtacttcaagtatttttctcaaaactcacttcctcttggagggccgagctctggcgcacccccaccaagtggagggtctcctgccgggtccccaacatctactgaagaaggcaccagcgaatccgcaacgcccgagtcaggccctggtacctccacagaaccatctgaaggtagtgcgcctggttccccagctggaagccctacttccaccgaagaaggcacgtcaaccgaaccaagtgaaggatctgcccctgggaccagcactgaaccatctgagccaaaaaagaagagaaaggtaatggacaagaagtacagcatcggcctggccatcggcaccaactctgtgggctgggccgtgatcaccgacgagtacaaggtgcccagcaagaaattcaaggtgctgggcaacaccgaccggcacagcatcaagaagaacctgatcggcgccctgctgttcgacagcggagaaacagccgaggccacccggctgaagagaaccgccagaagaagatacaccagacggaagaaccggatctgctatctgcaagagatcttcagcaacgagatggccaaggtggacgacagcttcttccacagactggaagagtccttcctggtggaagaggataagaagcacgagcggcaccccatcttcggcaacatcgtggacgaggtggcctaccacgagaagtaccccaccatctaccacctgagaaagaaactggtggacagcaccgacaaggccgacctgcggctgatctatctggccctggcccacatgatcaagttccggggccacttcctgatcgagggcgacctgaaccccgacaacagcgacgtggacaagctgttcatccagctggtgcagacctacaaccagctgttcgaggaaaaccccatcaacgccagcggcgtggacgccaaggccatcctgtctgccagactgagcaagagcagacggctggaaaatctgatcgcccagctgcccggcgagaagaagaatggcctgttcggcaacctgattgccctgagcctgggcctgacccccaacttcaagagcaacttcgacctggccgaggatgccaaactgcagctgagcaaggacacctacgacgacgacctggacaacctgctggcccagatcggcgaccagtacgccgacctgtttctggccgccaagaacctgtccgacgccatcctgctgagcgacatcctgagagtgaacaccgagatcaccaaggcccccctgagcgcctctatgatcaagagatacgacgagcaccaccaggacctgaccctgctgaaagctctcgtgcggcagcagctgcctgagaagtacaaagagattttcttcgaccagagcaagaacggctacgccggctacatcgatggcggagccagccaggaagagttctacaagttcatcaagcccatcctggaaaagatggacggcaccgaggaactgctcgtgaagctgaacagagaggacctgctgcggaagcagcggaccttcgacaacggcagcatcccccaccagatccacctgggagagctgcacgccattctgcggcggcaggaagatttttacccattcctgaaggacaaccgggaaaagatcgagaagatcctgaccttccgcatcccctactacgtgggccctctggccaggggaaacagcagattcgcctggatgaccagaaagagcgaggaaaccatcaccccctggaacttcgaggaagtggtggacaagggcgccagcgcccagagcttcatcgagcggatgaccaacttcgataagaacctgcccaacgagaaggtgctgcccaagcacagcctgctgtacgagtacttcaccgtgtacaacgagctgaccaaagtgaaatacgtgaccgagggaatgagaaagcccgccttcctgagcggcgagcagaaaaaagccatcgtggacctgctgttcaagaccaaccggaaagtgaccgtgaagcagctgaaagaggactacttcaagaaaatcgagtgcttcgactccgtggaaatctccggcgtggaagatcggttcaacgcctccctgggcacataccacgatctgctgaaaattatcaaggacaaggacttcctggacaatgaggaaaacgaggacattctggaagatatcgtgctgaccctgacactgtttgaggacagagagatgatcgaggaacggctgaaaacctatgcccacctgttcgacgacaaagtgatgaagcagctgaagcggcggagatacaccggctggggcaggctgagccggaagctgatcaacggcatccgggacaagcagtccggcaagacaatcctggatttcctgaagtccgacggcttcgccaacagaaacttcatgcagctgatccacgacgacagcctgacctttaaagaggacatccagaaagcccaggtgtccggccagggcgatagcctgcacgagcacattgccaatctggccggcagccccgccattaagaagggcatcctgcagacagtgaaggtggtggacgagctcgtgaaagtgatgggccggcacaagcccgagaacatcgtgatcgaaatggccagagagaaccagaccacccagaagggacagaagaacagccgcgagagaatgaagcggatcgaagagggcatcaaagagctgggcagccagatcctgaaagaacaccccgtggaaaacacccagctgcagaacgagaagctgtacctgtactacctgcagaatgggcgggatatgtacgtggaccaggaactggacatcaaccggctgtccgactacgatgtggacgctatcgtgcctcagagctttctgaaggacgactccatcgataacaaagtgctgactcggagcgacaagaaccggggcaagagcgacaacgtgccctccgaagaggtcgtgaagaagatgaagaactactggcgccagctgctgaatgccaagctgattacccagaggaagttcgacaatctgaccaaggccgagagaggcggcctgagcgaactggataaggccggcttcatcaagagacagctggtggaaacccggcagatcacaaagcacgtggcacagatcctggactcccggatgaacactaagtacgacgagaacgacaaactgatccgggaagtgaaagtgatcaccctgaagtccaagctggtgtccgatttccggaaggatttccagttttacaaagtgcgcgagatcaacaactaccaccacgcccacgacgcctacctgaacgccgtcgtgggaaccgccctgatcaaaaagtaccctaagctggaaagcgagttcgtgtacggcgactacaaggtgtacgacgtgcggaagatgatcgccaagagcgagcaggaaatcggcaaggctaccgccaagtacttcttctacagcaacatcatgaactttttcaagaccgagattaccctggccaacggcgagatccggaagcggcctctgatcgagacaaacggcgaaacaggcgagatcgtgtgggataagggccgggactttgccaccgtgcggaaagtgctgtctatgccccaagtgaatatcgtgaaaaagaccgaggtgcagacaggcggcttcagcaaagagtctatcctgcccaagaggaacagcgacaagctgatcgccagaaagaaggactgggaccctaagaagtacggcggcttcgacagccccaccgtggcctattctgtgctggtggtggccaaagtggaaaagggcaagtccaagaaactgaagagtgtgaaagagctgctggggatcaccatcatggaaagaagcagcttcgagaagaatcccatcgactttctggaagccaagggctacaaagaagtgaaaaaggacctgatcatcaagctgcctaagtactccctgttcgagctggaaaacggccggaagagaatgctggcctctgccggcgaactgcagaagggaaacgaactggccctgccctccaaatatgtgaacttcctgtacctggccagccactatgagaagctgaagggctcccccgaggataatgagcagaaacagctgtttgtggaacagcacaaacactacctggacgagatcatcgagcagatcagcgagttctccaagagagtgatcctggccgacgctaatctggacaaggtgctgagcgcctacaacaagcacagagacaagcctatcagagagcaggccgagaatatcatccacctgtttaccctgaccaatctgggagcccctgccgccttcaagtactttgacaccaccatcgaccggaagaggtacaccagcaccaaagaggtgctggacgccaccctgatccaccagagcatcaccggcctgtacgagacacggatcgacctgtctcagctgggaggcgacgcctatccctatgacgtgcccgattatgccagcctgggcagcggctcccccaagaaaaaacgcaaggtggaagatcctaagaaaaagcggaaagtggacggcattggtagtgggagcaacggcagcagcggagaggaactgctgagcaagaactaccacctggaaaacgaggtggccagactgaagaaaggctctggctctggcggaagcggttctggcggatcaggatctggaagtggcggctctggaagcggaggttctggatctggcgaagaactgctgtctaagaattatcacctcgagaacgaagtggctcggctcaagaaaggcagtggcagcggaggaagtggatccggcggtagtggtagtggaagcggcggatccggctcaggcggatctggttcaggggaagaactcctctccaaaaactaccatctcgagaatgaggtcgcccgcctgaaaaaaggatcaggttccggtggttctggcagcggtggttcaggctcaggcagcggcggtagcggtagcggtggaagcggaagcggagaagaacttctcagcaaaaattaccacttggagaatgaagttgcaagactcaaaaaaggttccggcagtggcggcagcggcagcggcggatctggtagtggatctggtggcagtggttcaggcggaagtggtagcggagaggaattgctctcaaagaactatcatttggagaacgaggttgcacgcttgaagaaaggcagcggatcaggcggatctggcagcggtggatctggttctggatccggcggctccggtagtggtggaagtggctctggggaagaattgcttagcaagaattatcatcttgaaaatgaggttgccaggcttaaaaaaggcagtggctccggcggatccggaagcggaggcagcggatctggatctggtggttcaggatctggcggttctggtagcggggaagaactgttgagtaaaaactatcaccttgagaacgaggtcgcaaggttgaaaaaaggatccggctctggcggctccggaagtggcggatctggctccggtagcggaggatcaggatccggcggaagcggatcaggcgaggaactgctttccaaaaattaccaccttgaaaacgaagtcgcccgcctcaagaaaggttctggcagcggaggctctggcagtggtggtagcggaagtggaagtggtggcagtggtagcggtggatctggaagcggcgaggaactcctgtcaaagaattaccatctcgaaaacgaggtcgcaaggctcaagaaaggctcaggatcaggcggctctggatccggcggttctggttccggctcaggtggaagtggatctggcggctcaggttccggcgaagaattgctttccaagaactaccatttggaaaatgaagtcgctcgtttgaagaaaggttcaggctccggccagcggggaagcaagcgcaccgccgatggttccgagttcgaaagccccaaaaaaaagcgcaaggtctgagatcccaagcacgcagcaatgcagctcaaaacgcttagcctagccacacccccacgggaaacagcagtgattaacctttagcaataaacgaaagtttaactaagctatactaaccccagggttggtcaatttcgtgccagccacaccctggtactgcatgcacgcaatgctagctgcccctttcccgtcctgggcaccccgagtctcccccgaccccgggtcccaggtatgctcccacctccacctgccccactcaccacctctgctagttccagacacctccgagacgaggaaaaaaaaaaaaaaaaaaaaaaaaaaaaaaaaaaaaaaaaaaaaaaaaaaaaaaaaaaaaaaaaaaaaaaaaaaaaaaaaaaaaaaaaaaaaaaaaaaaaaaaaaaaaaaaaaaaaaaaaaaaaaaaaaaaaaaaaaaaaaaaaaaaaaaaaaaaaaaaaaaaaaaaaaaaaaaaaaaaaaaaaaaaaaaaaaaaaaaaaaaaaaaaaaaaaaaaaaaaaaaaaaaaaaaaaaaaaaaaaaaaaaaaaaaaaaaaaaaaaaaaaaaaaaaaaaaaaaaaaaaaaaaaaaaaaaaaaaaaaaaaaaaaaaaaaaaaaaaaaaaaaaaaaaaaaaaaaaaaaaaaaaaaaaaaaaaaaaaaaaaaaaaaaaaaaaaaaaaaaaaaaaaaaaaaaaaccgtcttcaagctttctagaaattcactggccgtcgttttacaacgtcgtgactgggaaaaccctggcgttacccaacttaatcgccttgcagcacatccccctttcgccagctggcgtaatagcgaagaggcccgcaccgatcgcccttcccaacagttgcgcagcctgaatggcgaatggcgcctgatgcggtattttctccttacgcatctgtgcggtatttcacaccgcatatggtgcactctcagtacaatctgctctgatgccgcatagttaagccagccccgacacccgccaacacccgctgacgcgccctgacgggcttgtctgctcccggcatccgcttacagacaagctgtgaccgtctccgggagctgcatgtgtcagaggttttcaccgtcatcaccgaaacgcgcgagacgaaagggcctcgtgatacgcctatttttataggttaatgtcatgataataatggtttcttagacgtcaggtggcacttttcggggaaatgtgcgcggaacccctatttgtttatttttctaaatacattcaaatatgtatccgctcatgagacaataaccctgataaatgcttcaataatattgaaaaaggaagagtatgagtattcaacatttccgtgtcgcccttattcccttttttgcggcattttgccttcctgtttttgctcacccagaaacgctggtgaaagtaaaagatgctgaagatcagttgggtgcacgagtgggttacatcgaactggatctcaacagcggtaagatccttgagagttttcgccccgaagaacgttttccaatgatgagcacttttaaagttctgctatgtggcgcggtattatcccgtattgacgccgggcaagagcaactcggtcgccgcatacactattctcagaatgacttggttgagtactcaccagtcacagaaaagcatcttacggatggcatgacagtaagagaattatgcagtgctgccataaccatgagtgataacactgcggccaacttacttctgacaacgatcggaggaccgaaggagctaaccgcttttttgcacaacatgggggatcatgtaactcgccttgatcgttgggaaccggagctgaatgaagccataccaaacgacgagcgtgacaccacgatgcctgtagcaatggcaacaacgttgcgcaaactattaactggcgaactacttactctagcttcccggcaacaattaatagactggatggaggcggataaagttgcaggaccacttctgcgctcggcccttccggctggctggtttattgctgataaatctggagccggtgagcgtgggtctcgcggtatcattgcagcactggggccagatggtaagccctcccgtatcgtagttatctacacgacggggagtcaggcaactatggatgaacgaaatagacagatcgctgagataggtgcctcactgattaagcattggtaactgtcagaccaagtttac

SEQ ID NO: 201 - DNA, 6013 bp, synthetic construct
  misc_feature 1..6013: note = DNA of V7_D3a-D3l-scFv
  source 1..6013: mol_type = other DNA
gagatacctacagcgtgagctatgagaaagcgccacgcttcccgaagggagaaaggcggacaggtatccggtaagcggcagggtcggaacaggagagcgcacgagggagcttccagggggaaacgcctggtatctttatagtcctgtcgggtttcgccacctctgacttgagcgtcgatttttgtgatgctcgtcaggggggcggagcctatggaaaaacgccagcaacgcggcctttttacggttcctggccttttgctggccttttgctcacatgttctttcctgcgttatcccctgattctgtggataaccgtattaccgcctttgagtgagctgataccgctcgccgcagccgaacgaccgagcgcagcgagtcagtgagcgaggaagcggaagagcgcccaatacgcaaaccgcctctccccgcgcgttggccgattcattaatgcagctggcacgacaggtttcccgactggaaagcgggcagtgagcgcaacgcaattaatgtgagttagctcactcattaggcaccccaggctttacactttatgcttccggctcgtatgttgtgtggaattgtgagcggataacaatttcacacaggaaacagctatgaccatgattacgcctctagaaagctttaatacgactcactataaggactcactatttgttttcgcgcccagttgcaaaaagtgtcgacatttgcttctgacacaactgtgttcactagcaacctcaaacagacaccgccaccatgcctgctgctaagagagtgaaactggatggatccaaccatgaccaggaatttgaccccccaaaggtttacccacctgtgccagctgagaagaggaagcccatccgcgtgctgtctctctttgatgggattgctacagggctcctggtgctgaaggacctgggcatccaagtggaccgctacattgcctccgaggtgtgtgaggactccatcacggtgggcatggtgcggcaccagggaaagatcatgtacgtcggggacgtccgcagcgtcacacagaagcatatccaggagtggggcccattcgacctggtgattggaggcagtccctgcaatgacctctccattgtcaaccctgcccgcaagggactttatgagggtactggccgcctcttctttgagttctaccgcctcctgcatgatgcgcggcccaaggagggagatgatcgccccttcttctggctctttgagaatgtggtggccatgggcgttagtgacaagagggacatctcgcgatttcttgagtctaaccccgtgatgattgacgccaaagaagtgtctgctgcacacagggcccgttacttctggggtaaccttcctggcatgaacaggcctttggcatccactgtgaatgataagctggagctgcaagagtgtctggagcacggcagaatagccaagttcagcaaagtgaggaccattaccaccaggtcaaactctataaagcagggcaaagaccagcatttccccgtgttcatgaacgagaaggaggacatcctgtggtgcactgaaatggaaagggtgtttggcttccccgtccactacacagacgtctccaacatgagccgcttggcgaggcagagactgctgggccgatcgtggagcgtgccggtcatccgccacctcttcgctccgctgaaggaatattttgcttgtgtgtctagcggcaatagtaacgctaacagccgcgggccgagcttcagcagcggcctggtgccgttaagcttgcgcggcagccatatgggccctatggagatatacaagacagtgtctgcatggaagagacagccagtgcgggtactgagcctcttcagaaacatcgacaaggtactaaagagtttgggcttcttggaaagcggttctggttctgggggaggaacgctgaagtacgtggaagatgtcacaaatgtcgtgaggagagacgtggagaaatggggcccctttgacctggtgtacggctcgacgcagcccctaggcagctcttgtgatcgctgtcccggctggtacatgttccagttccaccggatcctgcagtatgcgctgcctcgccaggagagtcagcggcccttcttctggatattcatggacaatctgctgctgactgaggatgaccaagagacaactacccgcttccttcagacagaggctgtgaccctccaggatgtccgtggcagagactaccagaatgctatgcgggtgtggagcaacattccagggctgaagagcaagcatgcgcccctgaccccaaaggaagaagagtatctgcaagcccaagtcagaagcaggagcaagctggacgccccgaaagttgacctcctggtgaagaactgccttctcccgctgagagagtacttcaagtatttttctcaaaactcacttcctcttggagggccgagctctggcgcacccccaccaagtggagggtctcctgccgggtccccaacatctactgaagaaggcaccagcgaatccgcaacgcccgagtcaggccctggtacctccacagaaccatctgaaggtagtgcgcctggttccccagctggaagccctacttccaccgaagaaggcacgtcaaccgaaccaagtgaaggatctgcccctgggaccagcactgaaccatctgagggccccgacatcgtgatgacccagagccccagcagcctgagcgccagcgtgggcgaccgcgtgaccatcacctgccgcagcagcaccggcgccgtgaccaccagcaactacgccagctgggtgcaggagaagcccggcaagctgttcaagggcctgatcggcggcaccaacaaccgcgcccccggcgtgcccagccgcttcagcggcagcctgatcggcgacaaggccaccctgaccatcagcagcctgcagcccgaggacttcgccacctacttctgcgccctgtggtacagcaaccactgggtgttcggccagggcaccaaggtggagctgaagcgcggcggcggcggcagcggcggcggcggcagcggcggcggcggcagcagcggcggcggcagcgaggtgaagctgctggagagcggcggcggcctggtgcagcccggcggcagcctgaagctgagctgcgccgtgagcggcttcagcctgaccgactacggcgtgaactgggtgcgccaggcccccggccgcggcctggagtggatcggcgtgatctggggcgacggcatcaccgactacaacagcgccctgaaggaccgcttcatcatcagcaaggacaacggcaagaacaccgtgtacctgcagatgagcaaggtgcgcagcgacgacaccgccctgtactactgcgtgaccggcctgttcgactactggggccagggcaccctggtgaccgtgagcagctacccatacgatgttccagattacgctggtggaggcggaggttctgggggaggaggtagtggcggtggtggttcaggaggcggcggaagctagtgagatcccaagcacgcagcaatgcagctcaaaacgcttagcctagccacacccccacgggaaacagcagtgattaacctttagcaataaacgaaagtttaactaagctatactaaccccagggttggtcaatttcgtgccagccacaccctggtactgcatgcacgcaatgctagctgcccctttcccgtcctgggcaccccgagtctcccccgaccccgggtcccaggtatgctcccacctccacctgccccactcaccacctctgctagttccagacacctccgagacgaggaaaaaaaaaaaaaaaaaaaaaaaaaaaaaaaaaaaaaaaaaaaaaaaaaaaaaaaaaaaaaaaaaaaaaaaaaaaaaaaaaaaaaaaaaaaaaaaaaaaaaaaaaaaaaaaaaaaaaaaaaaaaaaaaaaaaaaaaaaaaaaaaaaaaaaaaaaaaaaaaaaaaaaaaaaaaaaaaaaaaaaaaaaaaaaaaaaaaaaaaccgtcttcaagctttctagaaattcactggccgtcgttttacaacgtcgtgactgggaaaaccctggcgttacccaacttaatcgccttgcagcacatccccctttcgccagctggcgtaatagcgaagaggcccgcaccgatcgcccttcccaacagttgcgcagcctgaatggcgaatggcgcctgatgcggtattttctccttacgcatctgtgcggtatttcacaccgcatatggtgcactctcagtacaatctgctctgatgccgcatagttaagccagccccgacacccgccaacacccgctgacgcgccctgacgggcttgtctgctcccggcatccgcttacagacaagctgtgaccgtctccgggagctgcatgtgtcagaggttttcaccgtcatcaccgaaacgcgcgagacgaaagggcctcgtgatacgcctatttttataggttaatgtcatgataataatggtttcttagacgtcaggtggcacttttcggggaaatgtgcgcggaacccctatttgtttatttttctaaatacattcaaatatgtatccgctcatgagacaataaccctgataaatgcttcaataatattgaaaaaggaagagtatgagtattcaacatttccgtgtcgcccttattcccttttttgcggcattttgccttcctgtttttgctcacccagaaacgctggtgaaagtaaaagatgctgaagatcagttgggtgcacgagtgggttacatcgaactggatctcaacagcggtaagatccttgagagttttcgccccgaagaacgttttccaatgatgagcacttttaaagttctgctatgtggcgcggtattatcccgtattgacgccgggcaagagcaactcggtcgccgcatacactattctcagaatgacttggttgagtactcaccagtcacagaaaagcatcttacggatggcatgacagtaagagaattatgcagtgctgccataaccatgagtgataacactgcggccaacttacttctgacaacgatcggaggaccgaaggagctaaccgcttttttgcacaacatgggggatcatgtaactcgccttgatcgttgggaaccggagctgaatgaagccataccaaacgacgagcgtgacaccacgatgcctgtagcaatggcaacaacgttgcgcaaactattaactggcgaactacttactctagcttcccggcaacaattaatagactggatggaggcggataaagttgcaggaccacttctgcgctcggcccttccggctggctggtttattgctgataaatctggagccggtgagcgtgggtctcgcggtatcattgcagcactggggccagatggtaagccctcccgtatcgtagttatctacacgacggggagtcaggcaactatggatgaacgaaatagacagatcgctgagataggtgcctcactgattaagcattggtaactgtcagaccaagtttactcatatatactttagattgatttaaaacttcatttttaatttaaaaggatctaggtgaagatcctttttgataatctcatgaccaaaatcccttaacgtgagttttcgttccactgagcgtcagaccccgtagaaaagatcaaaggatcttcttgagatcctttttttctgcgcgtaatctgctgcttgcaaacaaaaaaaccaccgctaccagcggtggtttgtttgccggatcaagagctaccaactctttttccgaaggtaactggcttcagcagagcgcagataccaaatactgttcttctagtgtagccgtagttaggccaccacttcaagaactctgtagcaccgcctacatacctcgctctgctaatcctgttaccagtggctgctgccagtggcgataagtcgtgtcttaccgggttggactcaagacgatagttaccggataaggcgcagcggtcgggctgaacggggggttcgtgcacacagcccagcttggagcgaacgacctacaccgaact

SEQ ID NO: 202 - DNA, 8382 bp, synthetic construct
  misc_feature 1..8382: note = DNA of V8_3xGCN4-dCas9-KRAB
  source 1..8382: mol_type = other DNA
atcgtgctgaccctgacactgtttgaggacagagagatgatcgaggaacggctgaaaacctatgcccacctgttcgacgacaaagtgatgaagcagctgaagcggcggagatacaccggctggggcaggctgagccggaagctgatcaacggcatccgggacaagcagtccggcaagacaatcctggatttcctgaagtccgacggcttcgccaacagaaacttcatgcagctgatccacgacgacagcctgacctttaaagaggacatccagaaagcccaggtgtccggccagggcgatagcctgcacgagcacattgccaatctggccggcagccccgccattaagaagggcatcctgcagacagtgaaggtggtggacgagctcgtgaaagtgatgggccggcacaagcccgagaacatcgtgatcgaaatggccagagagaaccagaccacccagaagggacagaagaacagccgcgagagaatgaagcggatcgaagagggcatcaaagagctgggcagccagatcctgaaagaacaccccgtggaaaacacccagctgcagaacgagaagctgtacctgtactacctgcagaatgggcgggatatgtacgtggaccaggaactggacatcaaccggctgtccgactacgatgtggacgctatcgtgcctcagagctttctgaaggacgactccatcgataacaaagtgctgactcggagcgacaagaaccggggcaagagcgacaacgtgccctccgaagaggtcgtgaagaagatgaagaactactggcgccagctgctgaatgccaagctgattacccagaggaagttcgacaatctgaccaaggccgagagaggcggcctgagcgaactggataaggccggcttcatcaagagacagctggtggaaacccggcagatcacaaagcacgtggcacagatcctggactcccggatgaacactaagtacgacgagaacgacaaactgatccgggaagtgaaagtgatcaccctgaagtccaagctggtgtccgatttccggaaggatttccagttttacaaagtgcgcgagatcaacaactaccaccacgcccacgacgcctacctgaacgccgtcgtgggaaccgccctgatcaaaaagtaccctaagctggaaagcgagttcgtgtacggcgactacaaggtgtacgacgtgcggaagatgatcgccaagagcgagcaggaaatcggcaaggctaccgccaagtacttcttctacagcaacatcatgaactttttcaagaccgagattaccctggccaacggcgagatccggaagcggcctctgatcgagacaaacggcgaaacaggcgagatcgtgtgggataagggccgggactttgccaccgtgcggaaagtgctgtctatgccccaagtgaatatcgtgaaaaagaccgaggtgcagacaggcggcttcagcaaagagtctatcctgcccaagaggaacagcgacaagctgatcgccagaaagaaggactgggaccctaagaagtacggcggcttcgacagccccaccgtggcctattctgtgctggtggtggccaaagtggaaaagggcaagtccaagaaactgaagagtgtgaaagagctgctggggatcaccatcatggaaagaagcagcttcgagaagaatcccatcgactttctggaagccaagggctacaaagaagtgaaaaaggacctgatcatcaagctgcctaagtactccctgttcgagctggaaaacggccggaagagaatgctggcctctgccggcgaactgcagaagggaaacgaactggccctgccctccaaatatgtgaacttcctgtacctggccagccactatgagaagctgaagggctcccccgaggataatgagcagaaacagctgtttgtggaacagcacaaacactacctggacgagatcatcgagcagatcagcgagttctccaagagagtgatcctggccgacgctaatctggacaaggtgctgagcgcctacaacaagcacagagacaagcctatcagagagcaggccgagaatatcatccacctgtttaccctgaccaatctgggagcccctgccgccttcaagtactttgacaccaccatcgaccggaagaggtacaccagcaccaaagaggtgctggacgccaccctgatccaccagagcatcaccggcctgtacgagacacggatcgacctgtctcagctgggaggcgacgcctatccctatgacgtgcccgattatgccagcctgggcagcggctcccccaagaaaaaacgcaaggtggaagatcctaagaaaaagcggaaagtggacggcagcggcagcgagacccccggtaccagcgagagcgccacccccgagagccggacactggtgaccttcaaggatgtatttgtggacttcaccagggaggagtggaagctgctggacactgctcagcagatcgtgtacagaaatgtgatgctggagaactataagaacctggtttccttgggttatcagcttactaagccagatgtgatcctccggttggagaagggagaagagccctgagatcccaagcacgcagcaatgcagctcaaaacgcttagcctagccacacccccacgggaaacagcagtgattaacctttagcaataaacgaaagtttaactaagctatactaaccccagggttggtcaatttcgtgccagccacaccctggtactgcatgcacgcaatgctagctgcccctttcccgtcctgggcaccccgagtctcccccgaccccgggtcccaggtatgctcccacctccacctgccccactcaccacctctgctagttccagacacctccgagacgaggaaaaaaaaaaaaaaaaaaaaaaaaaaaaaaaaaaaaaaaaaaaaaaaaaaaaaaaaaaaaaaaaaaaaaaaaaaaaaaaaaaaaaaaaaaaaaaaaaaaaaaaaaaaaaaaaaaaaaaaaaaaaaaaaaaaaaaaaaaaaaaaaaaaaaaaaaaaaaaaaaaaaaaaaaaaaaaaaaaaaaaaaaaaaaaaaaaaaaaaaaaaaaaaaaaaaaaaaaaaaaaaaaaaaaaaaaaaaaaaaaaaaaaaaaaaaaaaaaaaaaaaaaaaaaaaaaaaaaaaaaaaaaaaaaaaaaaaaaaaaaaaaaaaaaaaaaaaaaaaaaaaaaaaaaaaaaaaaaaaaaaaaaaaaaaaaaaaaaaaaaaaaaaaaaaaaaaaaaaaaaaaaaaaaaaaaaaccgtcttcaagctttctagaaattcactggccgtcgttttacaacgtcgtgactgggaaaaccctggcgttacccaacttaatcgccttgcagcacatccccctttcgccagctggcgtaatagcgaagaggcccgcaccgatcgcccttcccaacagttgcgcagcctgaatggcgaatggcgcctgatgcggtattttctccttacgcatctgtgcggtatttcacaccgcatatggtgcactctcagtacaatctgctctgatgccgcatagttaagccagccccgacacccgccaacacccgctgacgcgccctgacgggcttgtctgctcccggcatccgcttacagacaagctgtgaccgtctccgggagctgcatgtgtcagaggttttcaccgtcatcaccgaaacgcgcgagacgaaagggcctcgtgatacgcctatttttataggttaatgtcatgataataatggtttcttagacgtcaggtggcacttttcggggaaatgtgcgcggaacccctatttgtttatttttctaaatacattcaaatatgtatccgctcatgagacaataaccctgataaatgcttcaataatattgaaaaaggaagagtatgagtattcaacatttccgtgtcgcccttattcccttttttgcggcattttgccttcctgtttttgctcacccagaaacgctggtgaaagtaaaagatgctgaagatcagttgggtgcacgagtgggttacatcgaactggatctcaacagcggtaagatccttgagagttttcgccccgaagaacgttttccaatgatgagcacttttaaagttctgctatgtggcgcggtattatcccgtattgacgccgggcaagagcaactcggtcgccgcatacactattctcagaatgacttggttgagtactcaccagtcacagaaaagcatcttacggatggcatgacagtaagagaattatgcagtgctgccataaccatgagtgataacactgcggccaacttacttctgacaacgatcggaggaccgaaggagctaaccgcttttttgcacaacatgggggatcatgtaactcgccttgatcgttgggaaccggagctgaatgaagccataccaaacgacgagcgtgacaccacgatgcctgtagcaatggcaacaacgttgcgcaaactattaactggcgaactacttactctagcttcccggcaacaattaatagactggatggaggcggataaagttgcaggaccacttctgcgctcggcccttccggctggctggtttattgctgataaatctggagccggtgagcgtgggtctcgcggtatcattgcagcactggggccagatggtaagccctcccgtatcgtagttatctacacgacggggagtcaggcaactatggatgaacgaaatagacagatcgctgagataggtgcctcactgattaagcattggtaactgtcagaccaagtttactcatatatactttagattgatttaaaacttcatttttaatttaaaaggatctaggtgaagatcctttttgataatctcatgaccaaaatcccttaacgtgagttttcgttccactgagcgtcagaccccgtagaaaagatcaaaggatcttcttgagatcctttttttctgcgcgtaatctgctgcttgcaaacaaaaaaaccaccgctaccagcggtggtttgtttgccggatcaagagctaccaactctttttccgaaggtaactggcttcagcagagcgcagataccaaatactgttcttctagtgtagccgtagttaggccaccacttcaagaactctgtagcaccgcctacatacctcgctctgctaatcctgttaccagtggctgctgccagtggcgataagtcgtgtcttaccgggttggactcaagacgatagttaccggataaggcgcagcggtcgggctgaacggggggttcgtgcacacagcccagcttggagcgaacgacctacaccgaactgagatacctacagcgtgagctatgagaaagcgccacgcttcccgaagggagaaaggcggacaggtatccggtaagcggcagggtcggaacaggagagcgcacgagggagcttccagggggaaacgcctggtatctttatagtcctgtcgggtttcgccacctctgacttgagcgtcgatttttgtgatgctcgtcaggggggcggagcctatggaaaaacgccagcaacgcggcctttttacggttcctggccttttgctggccttttgctcacatgttctttcctgcgttatcccctgattctgtggataaccgtattaccgcctttgagtgagctgataccgctcgccgcagccgaacgaccgagcgcagcgagtcagtgagcgaggaagcggaagagcgcccaatacgcaaaccgcctctccccgcgcgttggccgattcattaatgcagctggcacgacaggtttcccgactggaaagcgggcagtgagcgcaacgcaattaatgtgagttagctcactcattaggcaccccaggctttacactttatgcttccggctcgtatgttgtgtggaattgtgagcggataacaatttcacacaggaaacagctatgaccatgattacgcctctagaaagctttaatacgactcactataaggactcactatttgttttcgcgcccagttgcaaaaagtgtcgacatttgcttctgacacaactgtgttcactagcaacctcaaacagacaccgccaccatgcctgctgctaagagagtgaaactggatggatccgaggaactgctgagcaagaactaccacctggaaaacgaggtggccagactgaagaaaggctctggctctggcggaagcggttctggcggatcaggatctggaagtggcggctctggaagcggaggttctggatctggcgaagaactgctgtctaagaattatcacctcgagaacgaagtggctcggctcaagaaaggcagtggcagcggaggaagtggatccggcggtagtggtagtggaagcggcggatccggctcaggcggatctggttcaggggaagaactcctctccaaaaactaccatctcgagaatgaggtcgcccgcctgaaaaaaggatcaggttccggtggttctggcagcggtggttcaggctcaggcagcggcggtagcggtagcggtggaagcggaagcggaccaaaaaagaagagaaaggtaatggacaagaagtacagcatcggcctggccatcggcaccaactctgtgggctgggccgtgatcaccgacgagtacaaggtgcccagcaagaaattcaaggtgctgggcaacaccgaccggcacagcatcaagaagaacctgatcggcgccctgctgttcgacagcggagaaacagccgaggccacccggctgaagagaaccgccagaagaagatacaccagacggaagaaccggatctgctatctgcaagagatcttcagcaacgagatggccaaggtggacgacagcttcttccacagactggaagagtccttcctggtggaagaggataagaagcacgagcggcaccccatcttcggcaacatcgtggacgaggtggcctaccacgagaagtaccccaccatctaccacctgagaaagaaactggtggacagcaccgacaaggccgacctgcggctgatctatctggccctggcccacatgatcaagttccggggccacttcctgatcgagggcgacctgaaccccgacaacagcgacgtggacaagctgttcatccagctggtgcagacctacaaccagctgttcgaggaaaaccccatcaacgccagcggcgtggacgccaaggccatcctgtctgccagactgagcaagagcagacggctggaaaatctgatcgcccagctgcccggcgagaagaagaatggcctgttcggcaacctgattgccctgagcctgggcctgacccccaacttcaagagcaacttcgacctggccgaggatgccaaactgcagctgagcaaggacacctacgacgacgacctggacaacctgctggcccagatcggcgaccagtacgccgacctgtttctggccgccaagaacctgtccgacgccatcctgctgagcgacatcctgagagtgaacaccgagatcaccaaggcccccctgagcgcctctatgatcaagagatacgacgagcaccaccaggacctgaccctgctgaaagctctcgtgcggcagcagctgcctgagaagtacaaagagattttcttcgaccagagcaagaacggctacgccggctacatcgatggcggagccagccaggaagagttctacaagttcatcaagcccatcctggaaaagatggacggcaccgaggaactgctcgtgaagctgaacagagaggacctgctgcggaagcagcggaccttcgacaacggcagcatcccccaccagatccacctgggagagctgcacgccattctgcggcggcaggaagatttttacccattcctgaaggacaaccgggaaaagatcgagaagatcctgaccttccgcatcccctactacgtgggccctctggccaggggaaacagcagattcgcctggatgaccagaaagagcgaggaaaccatcaccccctggaacttcgaggaagtggtggacaagggcgccagcgcccagagcttcatcgagcggatgaccaacttcgataagaacctgcccaacgagaaggtgctgcccaagcacagcctgctgtacgagtacttcaccgtgtacaacgagctgaccaaagtgaaatacgtgaccgagggaatgagaaagcccgccttcctgagcggcgagcagaaaaaagccatcgtggacctgctgttcaagaccaaccggaaagtgaccgtgaagcagctgaaagaggactacttcaagaaaatcgagtgcttcgactccgtggaaatctccggcgtggaagatcggttcaacgcctccctgggcacataccacgatctgctgaaaattatcaaggacaaggacttcctggacaatgaggaaaacgaggacattctggaagat

SEQ ID NO: 203 - DNA, 4165 bp, synthetic construct
  misc_feature 1..4165: note = DNA of V9_GFP1-10-KRAB
  source 1..4165: mol_type = other DNA
gagatacctacagcgtgagctatgagaaagcgccacgcttcccgaagggagaaaggcggacaggtatccggtaagcggcagggtcggaacaggagagcgcacgagggagcttccagggggaaacgcctggtatctttatagtcctgtcgggtttcgccacctctgacttgagcgtcgatttttgtgatgctcgtcaggggggcggagcctatggaaaaacgccagcaacgcggcctttttacggttcctggccttttgctggccttttgctcacatgttctttcctgcgttatcccctgattctgtggataaccgtattaccgcctttgagtgagctgataccgctcgccgcagccgaacgaccgagcgcagcgagtcagtgagcgaggaagcggaagagcgcccaatacgcaaaccgcctctccccgcgcgttggccgattcattaatgcagctggcacgacaggtttcccgactggaaagcgggcagtgagcgcaacgcaattaatgtgagttagctcactcattaggcaccccaggctttacactttatgcttccggctcgtatgttgtgtggaattgtgagcggataacaatttcacacaggaaacagctatgaccatgattacgcctctagaaagctttaatacgactcactataaggactcactatttgttttcgcgcccagttgcaaaaagtgtcgacatttgcttctgacacaactgtgttcactagcaacctcaaacagacaccgccaccatgcctgctgctaagagagtgaaactggatggatcctccaagggagaggagctgttcaccggagtggtgccaatcctggtggagctggacggcgatgtgaacggccacaagttttctgtgcgcggagagggagagggcgacgcaaccatcggcaagctgacactgaagttcatctgcaccacaggcaagctgcccgtgccttggccaaccctggtgaccacactgacatacggcgtgcagtgtttctctaggtatccagaccacatgaagagacacgatttctttaagagcgccatgccagagggatacgtgcaggagcggaccatctccttcaaggacgatggcaagtataagacccgcgccgtggtgaagtttgagggcgatacactggtgaacaggatcgagctgaagggcaccgacttcaaggaggatggcaatatcctgggccacaagctggagtacaactttaatagccacaacgtgtatatcacagccgacaagcagaagaacggcatcaaggccaacttcaccgtgaggcacaatgtggaggacggctccgtgcagctggccgatcactaccagcagaacacacctatcggcgacggacccgtgctgctgcctgataatcactatctgtccacccagacagtgctgtctaaggacccaaacgagaagttggatccaggtggaggtggaagcggtcggacactggtgaccttcaaggatgtatttgtggacttcaccagggaggagtggaagctgctggacactgctcagcagatcgtgtacagaaatgtgatgctggagaactataagaacctggtttccttgggttatcagcttactaagccagatgtgatcctccggttggagaagggagaagagccctgagatcccaagcacgcagcaatgcagctcaaaacgcttagcctagccacacccccacgggaaacagcagtgattaacctttagcaataaacgaaagtttaactaagctatactaaccccagggttggtcaatttcgtgccagccacaccctggtactgcatgcacgcaatgctagctgcccctttcccgtcctgggcaccccgagtctcccccgaccccgggtcccaggtatgctcccacctccacctgccccactcaccacctctgctagttccagacacctccgagacgaggaaaaaaaaaaaaaaaaaaaaaaaaaaaaaaaaaaaaaaaaaaaaaaaaaaaaaaaaaaaaaaaaaaaaaaaaaaaaaaaaaaaaaaaaaaaaaaaaaaaaaaaaaaaaaaaaaaaaaaaaaaaaaaaaaaaaaaaaaaaaaaaaaaaaaaaaaaaaaaaaaaaaaaaaaaaaaaaaaaaaaaaaaaaaaaaaaaaaaaaaccgtcttcaagctttctagaaattcactggccgtcgttttacaacgtcgtgactgggaaaaccctggcgttacccaacttaatcgccttgcagcacatccccctttcgccagctggcgtaatagcgaagaggcccgcaccgatcgcccttcccaacagttgcgcagcctgaatggcgaatggcgcctgatgcggtattttctccttacgcatctgtgcggtatttcacaccgcatatggtgcactctcagtacaatctgctctgatgccgcatagttaagccagccccgacacccgccaacacccgctgacgcgccctgacgggcttgtctgctcccggcatccgcttacagacaagctgtgaccgtctccgggagctgcatgtgtcagaggttttcaccgtcatcaccgaaacgcgcgagacgaaagggcctcgtgatacgcctatttttataggttaatgtcatgataataatggtttcttagacgtcaggtggcacttttcggggaaatgtgcgcggaacccctatttgtttatttttctaaatacattcaaatatgtatccgctcatgagacaataaccctgataaatgcttcaataatattgaaaaaggaagagtatgagtattcaacatttccgtgtcgcccttattcccttttttgcggcattttgccttcctgtttttgctcacccagaaacgctggtgaaagtaaaagatgctgaagatcagttgggtgcacgagtgggttacatcgaactggatctcaacagcggtaagatccttgagagttttcgccccgaagaacgttttccaatgatgagcacttttaaagttctgctatgtggcgcggtattatcccgtattgacgccgggcaagagcaactcggtcgccgcatacactattctcagaatgacttggttgagtactcaccagtcacagaaaagcatcttacggatggcatgacagtaagagaattatgcagtgctgccataaccatgagtgataacactgcggccaacttacttctgacaacgatcggaggaccgaaggagctaaccgcttttttgcacaacatgggggatcatgtaactcgccttgatcgttgggaaccggagctgaatgaagccataccaaacgacgagcgtgacaccacgatgcctgtagcaatggcaacaacgttgcgcaaactattaactggcgaactacttactctagcttcccggcaacaattaatagactggatggaggcggataaagttgcaggaccacttctgcgctcggcccttccggctggctggtttattgctgataaatctggagccggtgagcgtgggtctcgcggtatcattgcagcactggggccagatggtaagccctcccgtatcgtagttatctacacgacggggagtcaggcaactatggatgaacgaaatagacagatcgctgagataggtgcctcactgattaagcattggtaactgtcagaccaagtttactcatatatactttagattgatttaaaacttcatttttaatttaaaaggatctaggtgaagatcctttttgataatctcatgaccaaaatcccttaacgtgagttttcgttccactgagcgtcagaccccgtagaaaagatcaaaggatcttcttgagatcctttttttctgcgcgtaatctgctgcttgcaaacaaaaaaaccaccgctaccagcggtggtttgtttgccggatcaagagctaccaactctttttccgaaggtaactggcttcagcagagcgcagataccaaatactgttcttctagtgtagccgtagttaggccaccacttcaagaactctgtagcaccgcctacatacctcgctctgctaatcctgttaccagtggctgctgccagtggcgataagtcgtgtcttaccgggttggactcaagacgatagttaccggataaggcgcagcggtcgggctgaacggggggttcgtgcacacagcccagcttggagcgaacgacctacaccgaact

SEQ ID NO: 204 - DNA, 9837 bp, synthetic construct
  misc_feature 1..9837: note = DNA of V10_D3a-D3l-dCas9-1xGFP11
  source 1..9837: mol_type = other DNA
gtacctccacagaaccatctgaaggtagtgcgcctggttccccagctggaagccctacttccaccgaagaaggcacgtcaaccgaaccaagtgaaggatctgcccctgggaccagcactgaaccatctgagccaaaaaagaagagaaaggtaatggacaagaagtacagcatcggcctggccatcggcaccaactctgtgggctgggccgtgatcaccgacgagtacaaggtgcccagcaagaaattcaaggtgctgggcaacaccgaccggcacagcatcaagaagaacctgatcggcgccctgctgttcgacagcggagaaacagccgaggccacccggctgaagagaaccgccagaagaagatacaccagacggaagaaccggatctgctatctgcaagagatcttcagcaacgagatggccaaggtggacgacagcttcttccacagactggaagagtccttcctggtggaagaggataagaagcacgagcggcaccccatcttcggcaacatcgtggacgaggtggcctaccacgagaagtaccccaccatctaccacctgagaaagaaactggtggacagcaccgacaaggccgacctgcggctgatctatctggccctggcccacatgatcaagttccggggccacttcctgatcgagggcgacctgaaccccgacaacagcgacgtggacaagctgttcatccagctggtgcagacctacaaccagctgttcgaggaaaaccccatcaacgccagcggcgtggacgccaaggccatcctgtctgccagactgagcaagagcagacggctggaaaatctgatcgcccagctgcccggcgagaagaagaatggcctgttcggcaacctgattgccctgagcctgggcctgacccccaacttcaagagcaacttcgacctggccgaggatgccaaactgcagctgagcaaggacacctacgacgacgacctggacaacctgctggcccagatcggcgaccagtacgccgacctgtttctggccgccaagaacctgtccgacgccatcctgctgagcgacatcctgagagtgaacaccgagatcaccaaggcccccctgagcgcctctatgatcaagagatacgacgagcaccaccaggacctgaccctgctgaaagctctcgtgcggcagcagctgcctgagaagtacaaagagattttcttcgaccagagcaagaacggctacgccggctacatcgatggcggagccagccaggaagagttctacaagttcatcaagcccatcctggaaaagatggacggcaccgaggaactgctcgtgaagctgaacagagaggacctgctgcggaagcagcggaccttcgacaacggcagcatcccccaccagatccacctgggagagctgcacgccattctgcggcggcaggaagatttttacccattcctgaaggacaaccgggaaaagatcgagaagatcctgaccttccgcatcccctactacgtgggccctctggccaggggaaacagcagattcgcctggatgaccagaaagagcgaggaaaccatcaccccctggaacttcgaggaagtggtggacaagggcgccagcgcccagagcttcatcgagcggatgaccaacttcgataagaacctgcccaacgagaaggtgctgcccaagcacagcctgctgtacgagtacttcaccgtgtacaacgagctgaccaaagtgaaatacgtgaccgagggaatgagaaagcccgccttcctgagcggcgagcagaaaaaagccatcgtggacctgctgttcaagaccaaccggaaagtgaccgtgaagcagctgaaagaggactacttcaagaaaatcgagtgcttcgactccgtggaaatctccggcgtggaagatcggttcaacgcctccctgggcacataccacgatctgctgaaaattatcaaggacaaggacttcctggacaatgaggaaaacgaggacattctggaagatatcgtgctgaccctgacactgtttgaggacagagagatgatcgaggaacggctgaaaacctatgcccacctgttcgacgacaaagtgatgaagcagctgaagcggcggagatacaccggctggggcaggctgagccggaagctgatcaacggcatccgggacaagcagtccggcaagacaatcctggatttcctgaagtccgacggcttcgccaacagaaacttcatgcagctgatccacgacgacagcctgacctttaaagaggacatccagaaagcccaggtgtccggccagggcgatagcctgcacgagcacattgccaatctggccggcagccccgccattaagaagggcatcctgcagacagtgaaggtggtggacgagctcgtgaaagtgatgggccggcacaagcccgagaacatcgtgatcgaaatggccagagagaaccagaccacccagaagggacagaagaacagccgcgagagaatgaagcggatcgaagagggcatcaaagagctgggcagccagatcctgaaagaacaccccgtggaaaacacccagctgcagaacgagaagctgtacctgtactacctgcagaatgggcgggatatgtacgtggaccaggaactggacatcaaccggctgtccgactacgatgtggacgctatcgtgcctcagagctttctgaaggacgactccatcgataacaaagtgctgactcggagcgacaagaaccggggcaagagcgacaacgtgccctccgaagaggtcgtgaagaagatgaagaactactggcgccagctgctgaatgccaagctgattacccagaggaagttcgacaatctgaccaaggccgagagaggcggcctgagcgaactggataaggccggcttcatcaagagacagctggtggaaacccggcagatcacaaagcacgtggcacagatcctggactcccggatgaacactaagtacgacgagaacgacaaactgatccgggaagtgaaagtgatcaccctgaagtccaagctggtgtccgatttccggaaggatttccagttttacaaagtgcgcgagatcaacaactaccaccacgcccacgacgcctacctgaacgccgtcgtgggaaccgccctgatcaaaaagtaccctaagctggaaagcgagttcgtgtacggcgactacaaggtgtacgacgtgcggaagatgatcgccaagagcgagcaggaaatcggcaaggctaccgccaagtacttcttctacagcaacatcatgaactttttcaagaccgagattaccctggccaacggcgagatccggaagcggcctctgatcgagacaaacggcgaaacaggcgagatcgtgtgggataagggccgggactttgccaccgtgcggaaagtgctgtctatgccccaagtgaatatcgtgaaaaagaccgaggtgcagacaggcggcttcagcaaagagtctatcctgcccaagaggaacagcgacaagctgatcgccagaaagaaggactgggaccctaagaagtacggcggcttcgacagccccaccgtggcctattctgtgctggtggtggccaaagtggaaaagggcaagtccaagaaactgaagagtgtgaaagagctgctggggatcaccatcatggaaagaagcagcttcgagaagaatcccatcgactttctggaagccaagggctacaaagaagtgaaaaaggacctgatcatcaagctgcctaagtactccctgttcgagctggaaaacggccggaagagaatgctggcctctgccggcgaactgcagaagggaaacgaactggccctgccctccaaatatgtgaacttcctgtacctggccagccactatgagaagctgaagggctcccccgaggataatgagcagaaacagctgtttgtggaacagcacaaacactacctggacgagatcatcgagcagatcagcgagttctccaagagagtgatcctggccgacgctaatctggacaaggtgctgagcgcctacaacaagcacagagacaagcctatcagagagcaggccgagaatatcatccacctgtttaccctgaccaatctgggagcccctgccgccttcaagtactttgacaccaccatcgaccggaagaggtacaccagcaccaaagaggtgctggacgccaccctgatccaccagagcatcaccggcctgtacgagacacggatcgacctgtctcagctgggaggcgacgcctatccctatgacgtgcccgattatgccagcctgggcagcggctcccccaagaaaaaacgcaaggtggaagatcctaagaaaaagcggaaagtggacggcagcggcagcgagacccccggtaccagcgagagcgccacccccgagagcggtagtgggagcaacggcagcagcggatccatgcgtgaccacatggtccttcatgagtatgtaaatgctgctgggattacaggtggctctggaggtgcggccgcaaggtcaggctccggccagcggggaagcaagcgcaccgccgatggttccgagttcgaaagccccaaaaaaaagcgcaaggtctgagatcccaagcacgcagcaatgcagctcaaaacgcttagcctagccacacccccacgggaaacagcagtgattaacctttagcaataaacgaaagtttaactaagctatactaaccccagggttggtcaatttcgtgccagccacaccctggtactgcatgcacgcaatgctagctgcccctttcccgtcctgggcaccccgagtctcccccgaccccgggtcccaggtatgctcccacctccacctgccccactcaccacctctgctagttccagacacctccgagacgaggaaaaaaaaaaaaaaaaaaaaaaaaaaaaaaaaaaaaaaaaaaaaaaaaaaaaaaaaaaaaaaaaaaaaaaaaaaaaaaaaaaaaaaaaaaaaaaaaaaaaaaaaaaaaaaaaaaaaaaaaaaaaaaaaaaaaaaaaaaaaaaaaaaaaaaaaaaaaaaaaaaaaaaaaaaaaaaaaaaaaaaaaaaaaaaaaaaaaaaaaaaaaaaaaaaaaaaaaaaaaaaaaaaaaaaaaaaaaaaaaaaaaaaaaaaaaaaaaaaaaaaaaaaaaaaaaaaaaaaaaaaaaaaaaaaaaaaaaaaaaaaaaaaaaaaaaaaaaaaaaaaaaaaaaaaaaaaaaaaaaaaaaaaaaaaaaaaaaaaaaaaaaaaaaaaaaaaaaaaaaaaaaaaaaaaaaaaccgtcttcaagctttctagaaattcactggccgtcgttttacaacgtcgtgactgggaaaaccctggcgttacccaacttaatcgccttgcagcacatccccctttcgccagctggcgtaatagcgaagaggcccgcaccgatcgcccttcccaacagttgcgcagcctgaatggcgaatggcgcctgatgcggtattttctccttacgcatctgtgcggtatttcacaccgcatatggtgcactctcagtacaatctgctctgatgccgcatagttaagccagccccgacacccgccaacacccgctgacgcgccctgacgggcttgtctgctcccggcatccgcttacagacaagctgtgaccgtctccgggagctgcatgtgtcagaggttttcaccgtcatcaccgaaacgcgcgagacgaaagggcctcgtgatacgcctatttttataggttaatgtcatgataataatggtttcttagacgtcaggtggcacttttcggggaaatgtgcgcggaacccctatttgtttatttttctaaatacattcaaatatgtatccgctcatgagacaataaccctgataaatgcttcaataatattgaaaaaggaagagtatgagtattcaacatttccgtgtcgcccttattcccttttttgcggcattttgccttcctgtttttgctcacccagaaacgctggtgaaagtaaaagatgctgaagatcagttgggtgcacgagtgggttacatcgaactggatctcaacagcggtaagatccttgagagttttcgccccgaagaacgttttccaatgatgagcacttttaaagttctgctatgtggcgcggtattatcccgtattgacgccgggcaagagcaactcggtcgccgcatacactattctcagaatgacttggttgagtactcaccagtcacagaaaagcatcttacggatggcatgacagtaagagaattatgcagtgctgccataaccatgagtgataacactgcggccaacttacttctgacaacgatcggaggaccgaaggagctaaccgcttttttgcacaacatgggggatcatgtaactcgccttgatcgttgggaaccggagctgaatgaagccataccaaacgacgagcgtgacaccacgatgcctgtagcaatggcaacaacgttgcgcaaactattaactggcgaactacttactctagcttcccggcaacaattaatagactggatggaggcggataaagttgcaggaccacttctgcgctcggcccttccggctggctggtttattgctgataaatctggagccggtgagcgtgggtctcgcggtatcattgcagcactggggccagatggtaagccctcccgtatcgtagttatctacacgacggggagtcaggcaactatggatgaacgaaatagacagatcgctgagataggtgcctcactgattaagcattggtaactgtcagaccaagtttactcatatatactttagattgatttaaaacttcatttttaatttaaaaggatctaggtgaagatcctttttgataatctcatgaccaaaatcccttaacgtgagttttcgttccactgagcgtcagaccccgtagaaaagatcaaaggatcttcttgagatcctttttttctgcgcgtaatctgctgcttgcaaacaaaaaaaccaccgctaccagcggtggtttgtttgccggatcaagagctaccaactctttttccgaaggtaactggcttcagcagagcgcagataccaaatactgttcttctagtgtagccgtagttaggccaccacttcaagaactctgtagcaccgcctacatacctcgctctgctaatcctgttaccagtggctgctgccagtggcgataagtcgtgtcttaccgggttggactcaagacgatagttaccggataaggcgcagcggtcgggctgaacggggggttcgtgcacacagcccagcttggagcgaacgacctacaccgaactgagatacctacagcgtgagctatgagaaagcgccacgcttcccgaagggagaaaggcggacaggtatccggtaagcggcagggtcggaacaggagagcgcacgagggagcttccagggggaaacgcctggtatctttatagtcctgtcgggtttcgccacctctgacttgagcgtcgatttttgtgatgctcgtcaggggggcggagcctatggaaaaacgccagcaacgcggcctttttacggttcctggccttttgctggccttttgctcacatgttctttcctgcgttatcccctgattctgtggataaccgtattaccgcctttgagtgagctgataccgctcgccgcagccgaacgaccgagcgcagcgagtcagtgagcgaggaagcggaagagcgcccaatacgcaaaccgcctctccccgcgcgttggccgattcattaatgcagctggcacgacaggtttcccgactggaaagcgggcagtgagcgcaacgcaattaatgtgagttagctcactcattaggcaccccaggctttacactttatgcttccggctcgtatgttgtgtggaattgtgagcggataacaatttcacacaggaaacagctatgaccatgattacgcctctagaaagctttaatacgactcactataaggactcactatttgttttcgcgcccagttgcaaaaagtgtcgacatttgcttctgacacaactgtgttcactagcaacctcaaacagacaccgccaccatgcctgctgctaagagagtgaaactggatggatccaaccatgaccaggaatttgaccccccaaaggtttacccacctgtgccagctgagaagaggaagcccatccgcgtgctgtctctctttgatgggattgctacagggctcctggtgctgaaggacctgggcatccaagtggaccgctacattgcctccgaggtgtgtgaggactccatcacggtgggcatggtgcggcaccagggaaagatcatgtacgtcggggacgtccgcagcgtcacacagaagcatatccaggagtggggcccattcgacctggtgattggaggcagtccctgcaatgacctctccattgtcaaccctgcccgcaagggactttatgagggtactggccgcctcttctttgagttctaccgcctcctgcatgatgcgcggcccaaggagggagatgatcgccccttcttctggctctttgagaatgtggtggccatgggcgttagtgacaagagggacatctcgcgatttcttgagtctaaccccgtgatgattgacgccaaagaagtgtctgctgcacacagggcccgttacttctggggtaaccttcctggcatgaacaggcctttggcatccactgtgaatgataagctggagctgcaagagtgtctggagcacggcagaatagccaagttcagcaaagtgaggaccattaccaccaggtcaaactctataaagcagggcaaagaccagcatttccccgtgttcatgaacgagaaggaggacatcctgtggtgcactgaaatggaaagggtgtttggcttccccgtccactacacagacgtctccaacatgagccgcttggcgaggcagagactgctgggccgatcgtggagcgtgccggtcatccgccacctcttcgctccgctgaaggaatattttgcttgtgtgtctagcggcaatagtaacgctaacagccgcgggccgagcttcagcagcggcctggtgccgttaagcttgcgcggcagccatatgggccctatggagatatacaagacagtgtctgcatggaagagacagccagtgcgggtactgagcctcttcagaaacatcgacaaggtactaaagagtttgggcttcttggaaagcggttctggttctgggggaggaacgctgaagtacgtggaagatgtcacaaatgtcgtgaggagagacgtggagaaatggggcccctttgacctggtgtacggctcgacgcagcccctaggcagctcttgtgatcgctgtcccggctggtacatgttccagttccaccggatcctgcagtatgcgctgcctcgccaggagagtcagcggcccttcttctggatattcatggacaatctgctgctgactgaggatgaccaagagacaactacccgcttccttcagacagaggctgtgaccctccaggatgtccgtggcagagactaccagaatgctatgcgggtgtggagcaacattccagggctgaagagcaagcatgcgcccctgaccccaaaggaagaagagtatctgcaagcccaagtcagaagcaggagcaagctggacgccccgaaagttgacctcctggtgaagaactgccttctcccgctgagagagtacttcaagtatttttctcaaaactcacttcctcttggagggccgagctctggcgcacccccaccaagtggagggtctcctgccgggtccccaacatctactgaagaaggcaccagcgaatccgcaacgcccgagtcaggccctg

SEQ ID NO: 205 - DNA, 10200 bp, synthetic construct
  misc_feature 1..10200: note = DNA of V11_D3a-D3l-dCas9-8xGFP11
  source 1..10200: mol_type = other DNA
gtacctccacagaaccatctgaaggtagtgcgcctggttccccagctggaagccctacttccaccgaagaaggcacgtcaaccgaaccaagtgaaggatctgcccctgggaccagcactgaaccatctgagccaaaaaagaagagaaaggtaatggacaagaagtacagcatcggcctggccatcggcaccaactctgtgggctgggccgtgatcaccgacgagtacaaggtgcccagcaagaaattcaaggtgctgggcaacaccgaccggcacagcatcaagaagaacctgatcggcgccctgctgttcgacagcggagaaacagccgaggccacccggctgaagagaaccgccagaagaagatacaccagacggaagaaccggatctgctatctgcaagagatcttcagcaacgagatggccaaggtggacgacagcttcttccacagactggaagagtccttcctggtggaagaggataagaagcacgagcggcaccccatcttcggcaacatcgtggacgaggtggcctaccacgagaagtaccccaccatctaccacctgagaaagaaactggtggacagcaccgacaaggccgacctgcggctgatctatctggccctggcccacatgatcaagttccggggccacttcctgatcgagggcgacctgaaccccgacaacagcgacgtggacaagctgttcatccagctggtgcagacctacaaccagctgttcgaggaaaaccccatcaacgccagcggcgtggacgccaaggccatcctgtctgccagactgagcaagagcagacggctggaaaatctgatcgcccagctgcccggcgagaagaagaatggcctgttcggcaacctgattgccctgagcctgggcctgacccccaacttcaagagcaacttcgacctggccgaggatgccaaactgcagctgagcaaggacacctacgacgacgacctggacaacctgctggcccagatcggcgaccagtacgccgacctgtttctggccgccaagaacctgtccgacgccatcctgctgagcgacatcctgagagtgaacaccgagatcaccaaggcccccctgagcgcctctatgatcaagagatacgacgagcaccaccaggacctgaccctgctgaaagctctcgtgcggcagcagctgcctgagaagtacaaagagattttcttcgaccagagcaagaacggctacgccggctacatcgatggcggagccagccaggaagagttctacaagttcatcaagcccatcctggaaaagatggacggcaccgaggaactgctcgtgaagctgaacagagaggacctgctgcggaagcagcggaccttcgacaacggcagcatcccccaccagatccacctgggagagctgcacgccattctgcggcggcaggaagatttttacccattcctgaaggacaaccgggaaaagatcgagaagatcctgaccttccgcatcccctactacgtgggccctctggccaggggaaacagcagattcgcctggatgaccagaaagagcgaggaaaccatcaccccctggaacttcgaggaagtggtggacaagggcgccagcgcccagagcttcatcgagcggatgaccaacttcgataagaacctgcccaacgagaaggtgctgcccaagcacagcctgctgtacgagtacttcaccgtgtacaacgagctgaccaaagtgaaatacgtgaccgagggaatgagaaagcccgccttcctgagcggcgagcagaaaaaagccatcgtggacctgctgttcaagaccaaccggaaagtgaccgtgaagcagctgaaagaggactacttcaagaaaatcgagtgcttcgactccgtggaaatctccggcgtggaagatcggttcaacgcctccctgggcacataccacgatctgctgaaaattatcaaggacaaggacttcctggacaatgaggaaaacgaggacattctggaagatatcgtgctgaccctgacactgtttgaggacagagagatgatcgaggaacggctgaaaacctatgcccacctgttcgacgacaaagtgatgaagcagctgaagcggcggagatacaccggctggggcaggctgagccggaagctgatcaacggcatccgggacaagcagtccggcaagacaatcctggatttcctgaagtccgacggcttcgccaacagaaacttcatgcagctgatccacgacgacagcctgacctttaaagaggacatccagaaagcccaggtgtccggccagggcgatagcctgcacgagcacattgccaatctggccggcagccccgccattaagaagggcatcctgcagacagtgaaggtggtggacgagctcgtgaaagtgatgggccggcacaagcccgagaacatcgtgatcgaaatggccagagagaaccagaccacccagaagggacagaagaacagccgcgagagaatgaagcggatcgaagagggcatcaaagagctgggcagccagatcctgaaagaacaccccgtggaaaacacccagctgcagaacgagaagctgtacctgtactacctgcagaatgggcgggatatgtacgtggaccaggaactggacatcaaccggctgtccgactacgatgtggacgctatcgtgcctcagagctttctgaaggacgactccatcgataacaaagtgctgactcggagcgacaagaaccggggcaagagcgacaacgtgccctccgaagaggtcgtgaagaagatgaagaactactggcgccagctgctgaatgccaagctgattacccagaggaagttcgacaatctgaccaaggccgagagaggcggcctgagcgaactggataaggccggcttcatcaagagacagctggtggaaacccggcagatcacaaagcacgtggcacagatcctggactcccggatgaacactaagtacgacgagaacgacaaactgatccgggaagtgaaagtgatcaccctgaagtccaagctggtgtccgatttccggaaggatttccagttttacaaagtgcgcgagatcaacaactaccaccacgcccacgacgcctacctgaacgccgtcgtgggaaccgccctgatcaaaaagtaccctaagctggaaagcgagttcgtgtacggcgactacaaggtgtacgacgtgcggaagatgatcgccaagagcgagcaggaaatcggcaaggctaccgccaagtacttcttctacagcaacatcatgaactttttcaagaccgagattaccctggccaacggcgagatccggaagcggcctctgatcgagacaaacggcgaaacaggcgagatcgtgtgggataagggccgggactttgccaccgtgcggaaagtgctgtctatgccccaagtgaatatcgtgaaaaagaccgaggtgcagacaggcggcttcagcaaagagtctatcctgcccaagaggaacagcgacaagctgatcgccagaaagaaggactgggaccctaagaagtacggcggcttcgacagccccaccgtggcctattctgtgctggtggtggccaaagtggaaaagggcaagtccaagaaactgaagagtgtgaaagagctgctggggatcaccatcatggaaagaagcagcttcgagaagaatcccatcgactttctggaagccaagggctacaaagaagtgaaaaaggacctgatcatcaagctgcctaagtactccctgttcgagctggaaaacggccggaagagaatgctggcctctgccggcgaactgcagaagggaaacgaactggccctgccctccaaatatgtgaacttcctgtacctggccagccactatgagaagctgaagggctcccccgaggataatgagcagaaacagctgtttgtggaacagcacaaacactacctggacgagatcatcgagcagatcagcgagttctccaagagagtgatcctggccgacgctaatctggacaaggtgctgagcgcctacaacaagcacagagacaagcctatcagagagcaggccgagaatatcatccacctgtttaccctgaccaatctgggagcccctgccgccttcaagtactttgacaccaccatcgaccggaagaggtacaccagcaccaaagaggtgctggacgccaccctgatccaccagagcatcaccggcctgtacgagacacggatcgacctgtctcagctgggaggcgacgcctatccctatgacgtgcccgattatgccagcctgggcagcggctcccccaagaaaaaacgcaaggtggaagatcctaagaaaaagcggaaagtggacggcagcggcagcgagacccccggtaccagcgagagcgccacccccgagagcggtagtgggagcaacggcagcagcggatccatgcgtgaccacatggtccttcatgagtatgtaaatgctgctgggattacaggtggctctggaggtagagatcatatggttctccacgaatacgttaacgccgcaggcatcactggcggtagtggaggacgcgaccatatggtactacatgaatatgtcaatgcagccggaataaccggagggtccggaggccgggatcacatggtgctgcatgagtatgtgaacgcggcgggtataactggtgggtcgggcggacgagaccatatggtgcttcacgaatacgtaaacgcagctggcattactggcggatcaggtggcagggatcacatggtactccatgagtacgtgaacgctgctggaatcacaggcggtagcggcggtcgggaccatatggtcctgcacgaatatgtcaatgctgccggtatcaccgcggccgcaaggtcaggctccggccagcggggaagcaagcgcaccgccgatggttccgagttcgaaagccccaaaaaaaagcgcaaggtctgagatcccaagcacgcagcaatgcagctcaaaacgcttagcctagccacacccccacgggaaacagcagtgattaacctttagcaataaacgaaagtttaactaagctatactaaccccagggttggtcaatttcgtgccagccacaccctggtactgcatgcacgcaatgctagctgcccctttcccgtcctgggcaccccgagtctcccccgaccccgggtcccaggtatgctcccacctccacctgccccactcaccacctctgctagttccagacacctccgagacgaggaaaaaaaaaaaaaaaaaaaaaaaaaaaaaaaaaaaaaaaaaaaaaaaaaaaaaaaaaaaaaaaaaaaaaaaaaaaaaaaaaaaaaaaaaaaaaaaaaaaaaaaaaaaaaaaaaaaaaaaaaaaaaaaaaaaaaaaaaaaaaaaaaaaaaaaaaaaaaaaaaaaaaaaaaaaaaaaaaaaaaaaaaaaaaaaaaaaaaaaaaaaaaaaaaaaaaaaaaaaaaaaaaaaaaaaaaaaaaaaaaaaaaaaaaaaaaaaaaaaaaaaaaaaaaaaaaaaaaaaaaaaaaaaaaaaaaaaaaaaaaaaaaaaaaaaaaaaaaaaaaaaaaaaaaaaaaaaaaaaaaaaaaaaaaaaaaaaaaaaaaaaaaaaaaaaaaaaaaaaaaaaaaaaaaaaaaaccgtcttcaagctttctagaaattcactggccgtcgttttacaacgtcgtgactgggaaaaccctggcgttacccaacttaatcgccttgcagcacatccccctttcgccagctggcgtaatagcgaagaggcccgcaccgatcgcccttcccaacagttgcgcagcctgaatggcgaatggcgcctgatgcggtattttctccttacgcatctgtgcggtatttcacaccgcatatggtgcactctcagtacaatctgctctgatgccgcatagttaagccagccccgacacccgccaacacccgctgacgcgccctgacgggcttgtctgctcccggcatccgcttacagacaagctgtgaccgtctccgggagctgcatgtgtcagaggttttcaccgtcatcaccgaaacgcgcgagacgaaagggcctcgtgatacgcctatttttataggttaatgtcatgataataatggtttcttagacgtcaggtggcacttttcggggaaatgtgcgcggaacccctatttgtttatttttctaaatacattcaaatatgtatccgctcatgagacaataaccctgataaatgcttcaataatattgaaaaaggaagagtatgagtattcaacatttccgtgtcgcccttattcccttttttgcggcattttgccttcctgtttttgctcacccagaaacgctggtgaaagtaaaagatgctgaagatcagttgggtgcacgagtgggttacatcgaactggatctcaacagcggtaagatccttgagagttttcgccccgaagaacgttttccaatgatgagcacttttaaagttctgctatgtggcgcggtattatcccgtattgacgccgggcaagagcaactcggtcgccgcatacactattctcagaatgacttggttgagtactcaccagtcacagaaaagcatcttacggatggcatgacagtaagagaattatgcagtgctgccataaccatgagtgataacactgcggccaacttacttctgacaacgatcggaggaccgaaggagctaaccgcttttttgcacaacatgggggatcatgtaactcgccttgatcgttgggaaccggagctgaatgaagccataccaaacgacgagcgtgacaccacgatgcctgtagcaatggcaacaacgttgcgcaaactattaactggcgaactacttactctagcttcccggcaacaattaatagactggatggaggcggataaagttgcaggaccacttctgcgctcggcccttccggctggctggtttattgctgataaatctggagccggtgagcgtgggtctcgcggtatcattgcagcactggggccagatggtaagccctcccgtatcgtagttatctacacgacggggagtcaggcaactatggatgaacgaaatagacagatcgctgagataggtgcctcactgattaagcattggtaactgtcagaccaagtttactcatatatactttagattgatttaaaacttcatttttaatttaaaaggatctaggtgaagatcctttttgataatctcatgaccaaaatcccttaacgtgagttttcgttccactgagcgtcagaccccgtagaaaagatcaaaggatcttcttgagatcctttttttctgcgcgtaatctgctgcttgcaaacaaaaaaaccaccgctaccagcggtggtttgtttgccggatcaagagctaccaactctttttccgaaggtaactggcttcagcagagcgcagataccaaatactgttcttctagtgtagccgtagttaggccaccacttcaagaactctgtagcaccgcctacatacctcgctctgctaatcctgttaccagtggctgctgccagtggcgataagtcgtgtcttaccgggttggactcaagacgatagttaccggataaggcgcagcggtcgggctgaacggggggttcgtgcacacagcccagcttggagcgaacgacctacaccgaactgagatacctacagcgtgagctatgagaaagcgccacgcttcccgaagggagaaaggcggacaggtatccggtaagcggcagggtcggaacaggagagcgcacgagggagcttccagggggaaacgcctggtatctttatagtcctgtcgggtttcgccacctctgacttgagcgtcgatttttgtgatgctcgtcaggggggcggagcctatggaaaaacgccagcaacgcggcctttttacggttcctggccttttgctggccttttgctcacatgttctttcctgcgttatcccctgattctgtggataaccgtattaccgcctttgagtgagctgataccgctcgccgcagccgaacgaccgagcgcagcgagtcagtgagcgaggaagcggaagagcgcccaatacgcaaaccgcctctccccgcgcgttggccgattcattaatgcagctggcacgacaggtttcccgactggaaagcgggcagtgagcgcaacgcaattaatgtgagttagctcactcattaggcaccccaggctttacactttatgcttccggctcgtatgttgtgtggaattgtgagcggataacaatttcacacaggaaacagctatgaccatgattacgcctctagaaagctttaatacgactcactataaggactcactatttgttttcgcgcccagttgcaaaaagtgtcgacatttgcttctgacacaactgtgttcactagcaacctcaaacagacaccgccaccatgcctgctgctaagagagtgaaactggatggatccaaccatgaccaggaatttgaccccccaaaggtttacccacctgtgccagctgagaagaggaagcccatccgcgtgctgtctctctttgatgggattgctacagggctcctggtgctgaaggacctgggcatccaagtggaccgctacattgcctccgaggtgtgtgaggactccatcacggtgggcatggtgcggcaccagggaaagatcatgtacgtcggggacgtccgcagcgtcacacagaagcatatccaggagtggggcccattcgacctggtgattggaggcagtccctgcaatgacctctccattgtcaaccctgcccgcaagggactttatgagggtactggccgcctcttctttgagttctaccgcctcctgcatgatgcgcggcccaaggagggagatgatcgccccttcttctggctctttgagaatgtggtggccatgggcgttagtgacaagagggacatctcgcgatttcttgagtctaaccccgtgatgattgacgccaaagaagtgtctgctgcacacagggcccgttacttctggggtaaccttcctggcatgaacaggcctttggcatccactgtgaatgataagctggagctgcaagagtgtctggagcacggcagaatagccaagttcagcaaagtgaggaccattaccaccaggtcaaactctataaagcagggcaaagaccagcatttccccgtgttcatgaacgagaaggaggacatcctgtggtgcactgaaatggaaagggtgtttggcttccccgtccactacacagacgtctccaacatgagccgcttggcgaggcagagactgctgggccgatcgtggagcgtgccggtcatccgccacctcttcgctccgctgaaggaatattttgcttgtgtgtctagcggcaatagtaacgctaacagccgcgggccgagcttcagcagcggcctggtgccgttaagcttgcgcggcagccatatgggccctatggagatatacaagacagtgtctgcatggaagagacagccagtgcgggtactgagcctcttcagaaacatcgacaaggtactaaagagtttgggcttcttggaaagcggttctggttctgggggaggaacgctgaagtacgtggaagatgtcacaaatgtcgtgaggagagacgtggagaaatggggcccctttgacctggtgtacggctcgacgcagcccctaggcagctcttgtgatcgctgtcccggctggtacatgttccagttccaccggatcctgcagtatgcgctgcctcgccaggagagtcagcggcccttcttctggatattcatggacaatctgctgctgactgaggatgaccaagagacaactacccgcttccttcagacagaggctgtgaccctccaggatgtccgtggcagagactaccagaatgctatgcgggtgtggagcaacattccagggctgaagagcaagcatgcgcccctgaccccaaaggaagaagagtatctgcaagcccaagtcagaagcaggagcaagctggacgccccgaaagttgacctcctggtgaagaactgccttctcccgctgagagagtacttcaagtatttttctcaaaactcacttcctcttggagggccgagctctggcgcacccccaccaagtggagggtctcctgccgggtccccaacatctactgaagaaggcaccagcgaatccgcaacgcccgagtcaggccctg

SEQ ID NO: 206 - DNA, 11019 bp, synthetic construct
  misc_feature 1..11019: note = DNA of V12_scFv-KRAB-2a-D3a-D3l-dCas9-1xGCN4
  source 1..11019: mol_type = other DNA
tcatatatactttagattgatttaaaacttcatttttaatttaaaaggatctaggtgaagatcctttttgataatctcatgaccaaaatcccttaacgtgagttttcgttccactgagcgtcagaccccgtagaaaagatcaaaggatcttcttgagatcctttttttctgcgcgtaatctgctgcttgcaaacaaaaaaaccaccgctaccagcggtggtttgtttgccggatcaagagctaccaactctttttccgaaggtaactggcttcagcagagcgcagataccaaatactgttcttctagtgtagccgtagttaggccaccacttcaagaactctgtagcaccgcctacatacctcgctctgctaatcctgttaccagtggctgctgccagtggcgataagtcgtgtcttaccgggttggactcaagacgatagttaccggataaggcgcagcggtcgggctgaacggggggttcgtgcacacagcccagcttggagcgaacgacctacaccgaactgagatacctacagcgtgagctatgagaaagcgccacgcttcccgaagggagaaaggcggacaggtatccggtaagcggcagggtcggaacaggagagcgcacgagggagcttccagggggaaacgcctggtatctttatagtcctgtcgggtttcgccacctctgacttgagcgtcgatttttgtgatgctcgtcaggggggcggagcctatggaaaaacgccagcaacgcggcctttttacggttcctggccttttgctggccttttgctcacatgttctttcctgcgttatcccctgattctgtggataaccgtattaccgcctttgagtgagctgataccgctcgccgcagccgaacgaccgagcgcagcgagtcagtgagcgaggaagcggaagagcgcccaatacgcaaaccgcctctccccgcgcgttggccgattcattaatgcagctggcacgacaggtttcccgactggaaagcgggcagtgagcgcaacgcaattaatgtgagttagctcactcattaggcaccccaggctttacactttatgcttccggctcgtatgttgtgtggaattgtgagcggataacaatttcacacaggaaacagctatgaccatgattacgcctctagaaagctttaatacgactcactataaggactcactatttgttttcgcgcccagttgcaaaaagtgtcgacatttgcttctgacacaactgtgttcactagcaacctcaaacagacaccgccaccatgggccccgacatcgtgatgacccagagccccagcagcctgagcgccagcgtgggcgaccgcgtgaccatcacctgccgcagcagcaccggcgccgtgaccaccagcaactacgccagctgggtgcaggagaagcccggcaagctgttcaagggcctgatcggcggcaccaacaaccgcgcccccggcgtgcccagccgcttcagcggcagcctgatcggcgacaaggccaccctgaccatcagcagcctgcagcccgaggacttcgccacctacttctgcgccctgtggtacagcaaccactgggtgttcggccagggcaccaaggtggagctgaagcgcggcggcggcggcagcggcggcggcggcagcggcggcggcggcagcagcggcggcggcagcgaggtgaagctgctggagagcggcggcggcctggtgcagcccggcggcagcctgaagctgagctgcgccgtgagcggcttcagcctgaccgactacggcgtgaactgggtgcgccaggcccccggccgcggcctggagtggatcggcgtgatctggggcgacggcatcaccgactacaacagcgccctgaaggaccgcttcatcatcagcaaggacaacggcaagaacaccgtgtacctgcagatgagcaaggtgcgcagcgacgacaccgccctgtactactgcgtgaccggcctgttcgactactggggccagggcaccctggtgaccgtgagcagctacccatacgatgttccagattacgctggtggaggcggaggttctgggggaggaggtagtggcggtggtggttcaggaggcggcggaagcttggatccaggtggaggtggaagcggtcggacactggtgaccttcaaggatgtatttgtggacttcaccagggaggagtggaagctgctggacactgctcagcagatcgtgtacagaaatgtgatgctggagaactataagaacctggtttccttgggttatcagcttactaagccagatgtgatcctccggttggagaagggagaagagcccggaagcggaaagcgcaccgccgatggttccgagttcgaaagccccaaaaaaaagcgcaaggtcggaagcggagctactaacttcagcctgctgaagcaggctggagacgtggaggagaaccctggacctatgaaccatgaccaggaatttgaccccccaaaggtttacccacctgtgccagctgagaagaggaagcccatccgcgtgctgtctctctttgatgggattgctacagggctcctggtgctgaaggacctgggcatccaagtggaccgctacattgcctccgaggtgtgtgaggactccatcacggtgggcatggtgcggcaccagggaaagatcatgtacgtcggggacgtccgcagcgtcacacagaagcatatccaggagtggggcccattcgacctggtgattggaggcagtccctgcaatgacctctccattgtcaaccctgcccgcaagggactttatgagggtactggccgcctcttctttgagttctaccgcctcctgcatgatgcgcggcccaaggagggagatgatcgccccttcttctggctctttgagaatgtggtggccatgggcgttagtgacaagagggacatctcgcgatttcttgagtctaaccccgtgatgattgacgccaaagaagtgtctgctgcacacagggcccgttacttctggggtaaccttcctggcatgaacaggcctttggcatccactgtgaatgataagctggagctgcaagagtgtctggagcacggcagaatagccaagttcagcaaagtgaggaccattaccaccaggtcaaactctataaagcagggcaaagaccagcatttccccgtcttcatgaacgagaaggaggacatcctgtggtgcactgaaatggaaagggtgtttggcttccccgtccactacacagacgtctccaacatgagccgcttggcgaggcagagactgctgggccgatcgtggagcgtgccggtcatccgccacctcttcgctccgctgaaggaatattttgcttgtgtgtctagcggcaatagtaacgctaacagccgcgggccgagcttcagcagcggcctggtgccgttaagcttgcgcggcagccatatgggccctatggagatatacaagacagtgtctgcatggaagagacagccagtgcgggtactgagcctcttcagaaacatcgacaaggtactaaagagtttgggcttcttggaaagcggttctggttctgggggaggaacgctgaagtacgtggaagatgtcacaaatgtcgtgaggagagacgtggagaaatggggcccctttgacctggtgtacggctcgacgcagcccctaggcagctcttgtgatcgctgtcccggctggtacatgttccagttccaccggatcctgcagtatgcgctgcctcgccaggagagtcagcggcccttcttctggatattcatggacaatctgctgctgactgaggatgaccaagagacaactacccgcttccttcagacagaggctgtgaccctccaggatgtccgtggcagagactaccagaatgctatgcgggtgtggagcaacattccagggctgaagagcaagcatgcgcccctgaccccaaaggaagaagagtatctgcaagcccaagtcagaagcaggagcaagctggacgccccgaaagttgacctcctggtgaagaactgccttctcccgctgagagagtacttcaagtatttttctcaaaactcacttcctcttggagggccgagctctggcgcacccccaccaagtggagggtctcctgccgggtccccaacatctactgaagaaggcaccagcgaatccgcaacgcccgagtcaggccctggtacctccacagaaccatctgaaggtagtgcgcctggttccccagctggaagccctacttccaccgaagaaggcacgtcaaccgaaccaagtgaaggatctgcccctgggaccagcactgaaccatctgagccaaaaaagaagagaaaggtaatggacaagaagtacagcatcggcctggccatcggcaccaactctgtgggctgggccgtgatcaccgacgagtacaaggtgcccagcaagaaattcaaggtgctgggcaacaccgaccggcacagcatcaagaagaacctgatcggcgccctgctgttcgacagcggagaaacagccgaggccacccggctgaagagaaccgccagaagaagatacaccagacggaagaaccggatctgctatctgcaagagatcttcagcaacgagatggccaaggtggacgacagcttcttccacagactggaagagtccttcctggtggaagaggataagaagcacgagcggcaccccatcttcggcaacatcgtggacgaggtggcctaccacgagaagtaccccaccatctaccacctgagaaagaaactggtggacagcaccgacaaggccgacctgcggctgatctatctggccctggcccacatgatcaagttccggggccacttcctgatcgagggcgacctgaaccccgacaacagcgacgtggacaagctgttcatccagctggtgcagacctacaaccagctgttcgaggaaaaccccatcaacgccagcggcgtggacgccaaggccatcctgtctgccagactgagcaagagcagacggctggaaaatctgatcgcccagctgcccggcgagaagaagaatggcctgttcggcaacctgattgccctgagcctgggcctgacccccaacttcaagagcaacttcgacctggccgaggatgccaaactgcagctgagcaaggacacctacgacgacgacctggacaacctgctggcccagatcggcgaccagtacgccgacctgtttctggccgccaagaacctgtccgacgccatcctgctgagcgacatcctgagagtgaacaccgagatcaccaaggcccccctgagcgcctctatgatcaagagatacgacgagcaccaccaggacctgaccctgctgaaagctctcgtgcggcagcagctgcctgagaagtacaaagagattttcttcgaccagagcaagaacggctacgccggctacatcgatggcggagccagccaggaagagttctacaagttcatcaagcccatcctggaaaagatggacggcaccgaggaactgctcgtgaagctgaacagagaggacctgctgcggaagcagcggaccttcgacaacggcagcatcccccaccagatccacctgggagagctgcacgccattctgcggcggcaggaagatttttacccattcctgaaggacaaccgggaaaagatcgagaagatcctgaccttccgcatcccctactacgtgggccctctggccaggggaaacagcagattcgcctggatgaccagaaagagcgaggaaaccatcaccccctggaacttcgaggaagtggtggacaagggcgccagcgcccagagcttcatcgagcggatgaccaacttcgataagaacctgcccaacgagaaggtgctgcccaagcacagcctgctgtacgagtacttcaccgtgtacaacgagctgaccaaagtgaaatacgtgaccgagggaatgagaaagcccgccttcctgagcggcgagcagaaaaaagccatcgtggacctgctgttcaagaccaaccggaaagtgaccgtgaagcagctgaaagaggactacttcaagaaaatcgagtgcttcgactccgtggaaatctccggcgtggaagatcggttcaacgcctccctgggcacataccacgatctgctgaaaattatcaaggacaaggacttcctggacaatgaggaaaacgaggacattctggaagatatcgtgctgaccctgacactgtttgaggacagagagatgatcgaggaacggctgaaaacctatgcccacctgttcgacgacaaagtgatgaagcagctgaagcggcggagatacaccggctggggcaggctgagccggaagctgatcaacggcatccgggacaagcagtccggcaagacaatcctggatttcctgaagtccgacggcttcgccaacagaaacttcatgcagctgatccacgacgacagcctgacctttaaagaggacatccagaaagcccaggtgtccggccagggcgatagcctgcacgagcacattgccaatctggccggcagccccgccattaagaagggcatcctgcagacagtgaaggtggtggacgagctcgtgaaagtgatgggccggcacaagcccgagaacatcgtgatcgaaatggccagagagaaccagaccacccagaagggacagaagaacagccgcgagagaatgaagcggatcgaagagggcatcaaagagctgggcagccagatcctgaaagaacaccccgtggaaaacacccagctgcagaacgagaagctgtacctgtactacctgcagaatgggcgggatatgtacgtggaccaggaactggacatcaaccggctgtccgactacgatgtggacgctatcgtgcctcagagctttctgaaggacgactccatcgataacaaagtgctgactcggagcgacaagaaccggggcaagagcgacaacgtgccctccgaagaggtcgtgaagaagatgaagaactactggcgccagctgctgaatgccaagctgattacccagaggaagttcgacaatctgaccaaggccgagagaggcggcctgagcgaactggataaggccggcttcatcaagagacagctggtggaaacccggcagatcacaaagcacgtggcacagatcctggactcccggatgaacactaagtacgacgagaacgacaaactgatccgggaagtgaaagtgatcaccctgaagtccaagctggtgtccgatttccggaaggatttccagttttacaaagtgcgcgagatcaacaactaccaccacgcccacgacgcctacctgaacgccgtcgtgggaaccgccctgatcaaaaagtaccctaagctggaaagcgagttcgtgtacggcgactacaaggtgtacgacgtgcggaagatgatcgccaagagcgagcaggaaatcggcaaggctaccgccaagtacttcttctacagcaacatcatgaactttttcaagaccgagattaccctggccaacggcgagatccggaagcggcctctgatcgagacaaacggcgaaacaggcgagatcgtgtgggataagggccgggactttgccaccgtgcggaaagtgctgtctatgccccaagtgaatatcgtgaaaaagaccgaggtgcagacaggcggcttcagcaaagagtctatcctgcccaagaggaacagcgacaagctgatcgccagaaagaaggactgggaccctaagaagtacggcggcttcgacagccccaccgtggcctattctgtgctggtggtggccaaagtggaaaagggcaagtccaagaaactgaagagtgtgaaagagctgctggggatcaccatcatggaaagaagcagcttcgagaagaatcccatcgactttctggaagccaagggctacaaagaagtgaaaaaggacctgatcatcaagctgcctaagtactccctgttcgagctggaaaacggccggaagagaatgctggcctctgccggcgaactgcagaagggaaacgaactggccctgccctccaaatatgtgaacttcctgtacctggccagccactatgagaagctgaagggctcccccgaggataatgagcagaaacagctgtttgtggaacagcacaaacactacctggacgagatcatcgagcagatcagcgagttctccaagagagtgatcctggccgacgctaatctggacaaggtgctgagcgcctacaacaagcacagagacaagcctatcagagagcaggccgagaatatcatccacctgtttaccctgaccaatctgggagcccctgccgccttcaagtactttgacaccaccatcgaccggaagaggtacaccagcaccaaagaggtgctggacgccaccctgatccaccagagcatcaccggcctgtacgagacacggatcgacctgtctcagctgggaggcgacgcctatccctatgacgtgcccgattatgccagcctgggcagcggctcccccaagaaaaaacgcaaggtggaagatcctaagaaaaagcggaaagtggacggcattggtagtgggagcaacggcagcagcggagaggaactgctgagcaagaactaccacctggaaaacgaggtggccagactgaagaaaggctctggctctggcggaagcggttctggcggatcaggatctggaagtggcggctctggaagcggaggttctggatctggcgaagaactgctgtctaagaattatcacggttcaggctccggccagcggggaagcaagcgcaccgccgatggttccgagttcgaaagccccaaaaaaaagcgcaaggtctgagatcccaagcacgcagcaatgcagctcaaaacgcttagcctagccacacccccacgggaaacagcagtgattaacctttagcaataaacgaaagtttaactaagctatactaaccccagggttggtcaatttcgtgccagccacaccctggtactgcatgcacgcaatgctagctgcccctttcccgtcctgggcaccccgagtctcccccgaccccgggtcccaggtatgctcccacctccacctgccccactcaccacctctgctagttccagacacctccgagacgaggaaaaaaaaaaaaaaaaaaaaaaaaaaaaaaaaaaaaaaaaaaaaaaaaaaaaaaaaaaaaaaaaaaaaaaaaaaaaaaaaaaaaaaaaaaaaaaaaaaaaaaaaaaaaaaaaaaaaaaaaaaaaaaaaaaaaaaaaaaaaaaaaaaaaaaaaaaaaaaaaaaaaaaaaaaaaaaaaaaaaaaaaaaaaaaaaaaaaaaaaaaaaaaaaaaaaaaaaaaaaaaaaaaaaaaaaaaaaaaaaaaaaaaaaaaaaaaaaaaaaaaaaaaaaaaaaaaaaaaaaaaaaaaaaaaaaaaaaaaaaaaaaaaaaaaaaaaaaaaaaaaaaaaaaaaaaaaaaaaaaaaaaaaaaaaaaaaaaaaaaaaaaaaaaaaaaaaaaaaaaaaaaaaaaaaaaaaccgtcttcaagctttctagaaattcactggccgtcgttttacaacgtcgtgactgggaaaaccctggcgttacccaacttaatcgccttgcagcacatccccctttcgccagctggcgtaatagcgaagaggcccgcaccgatcgcccttcccaacagttgcgcagcctgaatggcgaatggcgcctgatgcggtattttctccttacgcatctgtgcggtatttcacaccgcatatggtgcactctcagtacaatctgctctgatgccgcatagttaagccagccccgacacccgccaacacccgctgacgcgccctgacgggcttgtctgctcccggcatccgcttacagacaagctgtgaccgtctccgggagctgcatgtgtcagaggttttcaccgtcatcaccgaaacgcgcgagacgaaagggcctcgtgatacgcctatttttataggttaatgtcatgataataatggtttcttagacgtcaggtggcacttttcggggaaatgtgcgcggaacccctatttgtttatttttctaaatacattcaaatatgtatccgctcatgagacaataaccctgataaatgcttcaataatattgaaaaaggaagagtatgagtattcaacatttccgtgtcgcccttattcccttttttgcggcattttgccttcctgtttttgctcacccagaaacgctggtgaaagtaaaagatgctgaagatcagttgggtgcacgagtgggttacatcgaactggatctcaacagcggtaagatccttgagagttttcgccccgaagaacgttttccaatgatgagcacttttaaagttctgctatgtggcgcggtattatcccgtattgacgccgggcaagagcaactcggtcgccgcatacactattctcagaatgacttggttgagtactcaccagtcacagaaaagcatcttacggatggcatgacagtaagagaattatgcagtgctgccataaccatgagtgataacactgcggccaacttacttctgacaacgatcggaggaccgaaggagctaaccgcttttttgcacaacatgggggatcatgtaactcgccttgatcgttgggaaccggagctgaatgaagccataccaaacgacgagcgtgacaccacgatgcctgtagcaatggcaacaacgttgcgcaaactattaactggcgaactacttactctagcttcccggcaacaattaatagactggatggaggcggataaagttgcaggaccacttctgcgctcggcccttccggctggctggtttattgctgataaatctggagccggtgagcgtgggtctcgcggtatcattgcagcactggggccagatggtaagccctcccgtatcgtagttatctacacgacggggagtcaggcaactatggatgaacgaaatagacagatcgctgagataggtgcctcactgattaagcattggtaactgtcagaccaagtttac

SEQ ID NO: 207 - DNA, 11049 bp, synthetic construct
  misc_feature 1..11049: note = DNA of V13_scFv-KRAB-2a-D3a-D3l-dCas9-2xGCN4
  source 1..11049: mol_type = other DNA
tcatatatactttagattgatttaaaacttcatttttaatttaaaaggatctaggtgaagatcctttttgataatctcatgaccaaaatcccttaacgtgagttttcgttccactgagcgtcagaccccgtagaaaagatcaaaggatcttcttgagatcctttttttctgcgcgtaatctgctgcttgcaaacaaaaaaaccaccgctaccagcggtggtttgtttgccggatcaagagctaccaactctttttccgaaggtaactggcttcagcagagcgcagataccaaatactgttcttctagtgtagccgtagttaggccaccacttcaagaactctgtagcaccgcctacatacctcgctctgctaatcctgttaccagtggctgctgccagtggcgataagtcgtgtcttaccgggttggactcaagacgatagttaccggataaggcgcagcggtcgggctgaacggggggttcgtgcacacagcccagcttggagcgaacgacctacaccgaactgagatacctacagcgtgagctatgagaaagcgccacgcttcccgaagggagaaaggcggacaggtatccggtaagcggcagggtcggaacaggagagcgcacgagggagcttccagggggaaacgcctggtatctttatagtcctgtcgggtttcgccacctctgacttgagcgtcgatttttgtgatgctcgtcaggggggcggagcctatggaaaaacgccagcaacgcggcctttttacggttcctggccttttgctggccttttgctcacatgttctttcctgcgttatcccctgattctgtggataaccgtattaccgcctttgagtgagctgataccgctcgccgcagccgaacgaccgagcgcagcgagtcagtgagcgaggaagcggaagagcgcccaatacgcaaaccgcctctccccgcgcgttggccgattcattaatgcagctggcacgacaggtttcccgactggaaagcgggcagtgagcgcaacgcaattaatgtgagttagctcactcattaggcaccccaggctttacactttatgcttccggctcgtatgttgtgtggaattgtgagcggataacaatttcacacaggaaacagctatgaccatgattacgcctctagaaagctttaatacgactcactataaggactcactatttgttttcgcgcccagttgcaaaaagtgtcgacatttgcttctgacacaactgtgttcactagcaacctcaaacagacaccgccaccatgggccccgacatcgtgatgacccagagccccagcagcctgagcgccagcgtgggcgaccgcgtgaccatcacctgccgcagcagcaccggcgccgtgaccaccagcaactacgccagctgggtgcaggagaagcccggcaagctgttcaagggcctgatcggcggcaccaacaaccgcgcccccggcgtgcccagccgcttcagcggcagcctgatcggcgacaaggccaccctgaccatcagcagcctgcagcccgaggacttcgccacctacttctgcgccctgtggtacagcaaccactgggtgttcggccagggcaccaaggtggagctgaagcgcggcggcggcggcagcggcggcggcggcagcggcggcggcggcagcagcggcggcggcagcgaggtgaagctgctggagagcggcggcggcctggtgcagcccggcggcagcctgaagctgagctgcgccgtgagcggcttcagcctgaccgactacggcgtgaactgggtgcgccaggcccccggccgcggcctggagtggatcggcgtgatctggggcgacggcatcaccgactacaacagcgccctgaaggaccgcttcatcatcagcaaggacaacggcaagaacaccgtgtacctgcagatgagcaaggtgcgcagcgacgacaccgccctgtactactgcgtgaccggcctgttcgactactggggccagggcaccctggtgaccgtgagcagctacccatacgatgttccagattacgctggtggaggcggaggttctgggggaggaggtagtggcggtggtggttcaggaggcggcggaagcttggatccaggtggaggtggaagcggtcggacactggtgaccttcaaggatgtatttgtggacttcaccagggaggagtggaagctgctggacactgctcagcagatcgtgtacagaaatgtgatgctggagaactataagaacctggtttccttgggttatcagcttactaagccagatgtgatcctccggttggagaagggagaagagcccggaagcggaaagcgcaccgccgatggttccgagttcgaaagccccaaaaaaaagcgcaaggtcggaagcggagctactaacttcagcctgctgaagcaggctggagacgtggaggagaaccctggacctatgaaccatgaccaggaatttgaccccccaaaggtttacccacctgtgccagctgagaagaggaagcccatccgcgtgctgtctctctttgatgggattgctacagggctcctggtgctgaaggacctgggcatccaagtggaccgctacattgcctccgaggtgtgtgaggactccatcacggtgggcatggtgcggcaccagggaaagatcatgtacgtcggggacgtccgcagcgtcacacagaagcatatccaggagtggggcccattcgacctggtgattggaggcagtccctgcaatgacctctccattgtcaaccctgcccgcaagggactttatgagggtactggccgcctcttctttgagttctaccgcctcctgcatgatgcgcggcccaaggagggagatgatcgccccttcttctggctctttgagaatgtggtggccatgggcgttagtgacaagagggacatctcgcgatttcttgagtctaaccccgtgatgattgacgccaaagaagtgtctgctgcacacagggcccgttacttctggggtaaccttcctggcatgaacaggcctttggcatccactgtgaatgataagctggagctgcaagagtgtctggagcacggcagaatagccaagttcagcaaagtgaggaccattaccaccaggtcaaactctataaagcagggcaaagaccagcatttccccgtcttcatgaacgagaaggaggacatcctgtggtgcactgaaatggaaagggtgtttggcttccccgtccactacacagacgtctccaacatgagccgcttggcgaggcagagactgctgggccgatcgtggagcgtgccggtcatccgccacctcttcgctccgctgaaggaatattttgcttgtgtgtctagcggcaatagtaacgctaacagccgcgggccgagcttcagcagcggcctggtgccgttaagcttgcgcggcagccatatgggccctatggagatatacaagacagtgtctgcatggaagagacagccagtgcgggtactgagcctcttcagaaacatcgacaaggtactaaagagtttgggcttcttggaaagcggttctggttctgggggaggaacgctgaagtacgtggaagatgtcacaaatgtcgtgaggagagacgtggagaaatggggcccctttgacctggtgtacggctcgacgcagcccctaggcagctcttgtgatcgctgtcccggctggtacatgttccagttccaccggatcctgcagtatgcgctgcctcgccaggagagtcagcggcccttcttctggatattcatggacaatctgctgctgactgaggatgaccaagagacaactacccgcttccttcagacagaggctgtgaccctccaggatgtccgtggcagagactaccagaatgctatgcgggtgtggagcaacattccagggctgaagagcaagcatgcgcccctgaccccaaaggaagaagagtatctgcaagcccaagtcagaagcaggagcaagctggacgccccgaaagttgacctcctggtgaagaactgccttctcccgctgagagagtacttcaagtatttttctcaaaactcacttcctcttggagggccgagctctggcgcacccccaccaagtggagggtctcctgccgggtccccaacatctactgaagaaggcaccagcgaatccgcaacgcccgagtcaggccctggtacctccacagaaccatctgaaggtagtgcgcctggttccccagctggaagccctacttccaccgaagaaggcacgtcaaccgaaccaagtgaaggatctgcccctgggaccagcactgaaccatctgagccaaaaaagaagagaaaggtaatggacaagaagtacagcatcggcctggccatcggcaccaactctgtgggctgggccgtgatcaccgacgagtacaaggtgcccagcaagaaattcaaggtgctgggcaacaccgaccggcacagcatcaagaagaacctgatcggcgccctgctgttcgacagcggagaaacagccgaggccacccggctgaagagaaccgccagaagaagatacaccagacggaagaaccggatctgctatctgcaagagatcttcagcaacgagatggccaaggtggacgacagcttcttccacagactggaagagtccttcctggtggaagaggataagaagcacgagcggcaccccatcttcggcaacatcgtggacgaggtggcctaccacgagaagtaccccaccatctaccacctgagaaagaaactggtggacagcaccgacaaggccgacctgcggctgatctatctggccctggcccacatgatcaagttccggggccacttcctgatcgagggcgacctgaaccccgacaacagcgacgtggacaagctgttcatccagctggtgcagacctacaaccagctgttcgaggaaaaccccatcaacgccagcggcgtggacgccaaggccatcctgtctgccagactgagcaagagcagacggctggaaaatctgatcgcccagctgcccggcgagaagaagaatggcctgttcggcaacctgattgccctgagcctgggcctgacccccaacttcaagagcaacttcgacctggccgaggatgccaaactgcagctgagcaaggacacctacgacgacgacctggacaacctgctggcccagatcggcgaccagtacgccgacctgtttctggccgccaagaacctgtccgacgccatcctgctgagcgacatcctgagagtgaacaccgagatcaccaaggcccccctgagcgcctctatgatcaagagatacgacgagcaccaccaggacctgaccctgctgaaagctctcgtgcggcagcagctgcctgagaagtacaaagagattttcttcgaccagagcaagaacggctacgccggctacatcgatggcggagccagccaggaagagttctacaagttcatcaagcccatcctggaaaagatggacggcaccgaggaactgctcgtgaagctgaacagagaggacctgctgcggaagcagcggaccttcgacaacggcagcatcccccaccagatccacctgggagagctgcacgccattctgcggcggcaggaagatttttacccattcctgaaggacaaccgggaaaagatcgagaagatcctgaccttccgcatcccctactacgtgggccctctggccaggggaaacagcagattcgcctggatgaccagaaagagcgaggaaaccatcaccccctggaacttcgaggaagtggtggacaagggcgccagcgcccagagcttcatcgagcggatgaccaacttcgataagaacctgcccaacgagaaggtgctgcccaagcacagcctgctgtacgagtacttcaccgtgtacaacgagctgaccaaagtgaaatacgtgaccgagggaatgagaaagcccgccttcctgagcggcgagcagaaaaaagccatcgtggacctgctgttcaagaccaaccggaaagtgaccgtgaagcagctgaaagaggactacttcaagaaaatcgagtgcttcgactccgtggaaatctccggcgtggaagatcggttcaacgcctccctgggcacataccacgatctgctgaaaattatcaaggacaaggacttcctggacaatgaggaaaacgaggacattctggaagatatcgtgctgaccctgacactgtttgaggacagagagatgatcgaggaacggctgaaaacctatgcccacctgttcgacgacaaagtgatgaagcagctgaagcggcggagatacaccggctggggcaggctgagccggaagctgatcaacggcatccgggacaagcagtccggcaagacaatcctggatttcctgaagtccgacggcttcgccaacagaaacttcatgcagctgatccacgacgacagcctgacctttaaagaggacatccagaaagcccaggtgtccggccagggcgatagcctgcacgagcacattgccaatctggccggcagccccgccattaagaagggcatcctgcagacagtgaaggtggtggacgagctcgtgaaagtgatgggccggcacaagcccgagaacatcgtgatcgaaatggccagagagaaccagaccacccagaagggacagaagaacagccgcgagagaatgaagcggatcgaagagggcatcaaagagctgggcagccagatcctgaaagaacaccccgtggaaaacacccagctgcagaacgagaagctgtacctgtactacctgcagaatgggcgggatatgtacgtggaccaggaactggacatcaaccggctgtccgactacgatgtggacgctatcgtgcctcagagctttctgaaggacgactccatcgataacaaagtgctgactcggagcgacaagaaccggggcaagagcgacaacgtgccctccgaagaggtcgtgaagaagatgaagaactactggcgccagctgctgaatgccaagctgattacccagaggaagttcgacaatctgaccaaggccgagagaggcggcctgagcgaactggataaggccggcttcatcaagagacagctggtggaaacccggcagatcacaaagcacgtggcacagatcctggactcccggatgaacactaagtacgacgagaacgacaaactgatccgggaagtgaaagtgatcaccctgaagtccaagctggtgtccgatttccggaaggatttccagttttacaaagtgcgcgagatcaacaactaccaccacgcccacgacgcctacctgaacgccgtcgtgggaaccgccctgatcaaaaagtaccctaagctggaaagcgagttcgtgtacggcgactacaaggtgtacgacgtgcggaagatgatcgccaagagcgagcaggaaatcggcaaggctaccgccaagtacttcttctacagcaacatcatgaactttttcaagaccgagattaccctggccaacggcgagatccggaagcggcctctgatcgagacaaacggcgaaacaggcgagatcgtgtgggataagggccgggactttgccaccgtgcggaaagtgctgtctatgccccaagtgaatatcgtgaaaaagaccgaggtgcagacaggcggcttcagcaaagagtctatcctgcccaagaggaacagcgacaagctgatcgccagaaagaaggactgggaccctaagaagtacggcggcttcgacagccccaccgtggcctattctgtgctggtggtggccaaagtggaaaagggcaagtccaagaaactgaagagtgtgaaagagctgctggggatcaccatcatggaaagaagcagcttcgagaagaatcccatcgactttctggaagccaagggctacaaagaagtgaaaaaggacctgatcatcaagctgcctaagtactccctgttcgagctggaaaacggccggaagagaatgctggcctctgccggcgaactgcagaagggaaacgaactggccctgccctccaaatatgtgaacttcctgtacctggccagccactatgagaagctgaagggctcccccgaggataatgagcagaaacagctgtttgtggaacagcacaaacactacctggacgagatcatcgagcagatcagcgagttctccaagagagtgatcctggccgacgctaatctggacaaggtgctgagcgcctacaacaagcacagagacaagcctatcagagagcaggccgagaatatcatccacctgtttaccctgaccaatctgggagcccctgccgccttcaagtactttgacaccaccatcgaccggaagaggtacaccagcaccaaagaggtgctggacgccaccctgatccaccagagcatcaccggcctgtacgagacacggatcgacctgtctcagctgggaggcgacgcctatccctatgacgtgcccgattatgccagcctgggcagcggctcccccaagaaaaaacgcaaggtggaagatcctaagaaaaagcggaaagtggacggcattggtagtgggagcaacggcagcagcggagaggaactgctgagcaagaactaccacctggaaaacgaggtggccagactgaagaaaggctctggctctggcggaagcggttctggcggatcaggatctggaagtggcggctctggaagcggaggttctggatctggcgaagaactgctgtctaagaattatcacctcgagaatgaagtcgctcgtttgaagaaaggttcaggctccggccagcggggaagcaagcgcaccgccgatggttccgagttcgaaagccccaaaaaaaagcgcaaggtctgagatcccaagcacgcagcaatgcagctcaaaacgcttagcctagccacacccccacgggaaacagcagtgattaacctttagcaataaacgaaagtttaactaagctatactaaccccagggttggtcaatttcgtgccagccacaccctggtactgcatgcacgcaatgctagctgcccctttcccgtcctgggcaccccgagtctcccccgaccccgggtcccaggtatgctcccacctccacctgccccactcaccacctctgctagttccagacacctccgagacgaggaaaaaaaaaaaaaaaaaaaaaaaaaaaaaaaaaaaaaaaaaaaaaaaaaaaaaaaaaaaaaaaaaaaaaaaaaaaaaaaaaaaaaaaaaaaaaaaaaaaaaaaaaaaaaaaaaaaaaaaaaaaaaaaaaaaaaaaaaaaaaaaaaaaaaaaaaaaaaaaaaaaaaaaaaaaaaaaaaaaaaaaaaaaaaaaaaaaaaaaaaaaaaaaaaaaaaaaaaaaaaaaaaaaaaaaaaaaaaaaaaaaaaaaaaaaaaaaaaaaaaaaaaaaaaaaaaaaaaaaaaaaaaaaaaaaaaaaaaaaaaaaaaaaaaaaaaaaaaaaaaaaaaaaaaaaaaaaaaaaaaaaaaaaaaaaaaaaaaaaaaaaaaaaaaaaaaaaaaaaaaaaaaaaaaaaaaaccgtcttcaagctttctagaaattcactggccgtcgttttacaacgtcgtgactgggaaaaccctggcgttacccaacttaatcgccttgcagcacatccccctttcgccagctggcgtaatagcgaagaggcccgcaccgatcgcccttcccaacagttgcgcagcctgaatggcgaatggcgcctgatgcggtattttctccttacgcatctgtgcggtatttcacaccgcatatggtgcactctcagtacaatctgctctgatgccgcatagttaagccagccccgacacccgccaacacccgctgacgcgccctgacgggcttgtctgctcccggcatccgcttacagacaagctgtgaccgtctccgggagctgcatgtgtcagaggttttcaccgtcatcaccgaaacgcgcgagacgaaagggcctcgtgatacgcctatttttataggttaatgtcatgataataatggtttcttagacgtcaggtggcacttttcggggaaatgtgcgcggaacccctatttgtttatttttctaaatacattcaaatatgtatccgctcatgagacaataaccctgataaatgcttcaataatattgaaaaaggaagagtatgagtattcaacatttccgtgtcgcccttattcccttttttgcggcattttgccttcctgtttttgctcacccagaaacgctggtgaaagtaaaagatgctgaagatcagttgggtgcacgagtgggttacatcgaactggatctcaacagcggtaagatccttgagagttttcgccccgaagaacgttttccaatgatgagcacttttaaagttctgctatgtggcgcggtattatcccgtattgacgccgggcaagagcaactcggtcgccgcatacactattctcagaatgacttggttgagtactcaccagtcacagaaaagcatcttacggatggcatgacagtaagagaattatgcagtgctgccataaccatgagtgataacactgcggccaacttacttctgacaacgatcggaggaccgaaggagctaaccgcttttttgcacaacatgggggatcatgtaactcgccttgatcgttgggaaccggagctgaatgaagccataccaaacgacgagcgtgacaccacgatgcctgtagcaatggcaacaacgttgcgcaaactattaactggcgaactacttactctagcttcccggcaacaattaatagactggatggaggcggataaagttgcaggaccacttctgcgctcggcccttccggctggctggtttattgctgataaatctggagccggtgagcgtgggtctcgcggtatcattgcagcactggggccagatggtaagccctcccgtatcgtagttatctacacgacggggagtcaggcaactatggatgaacgaaatagacagatcgctgagataggtgcctcactgattaagcattggtaactgtcagaccaagtttac

SEQ ID NO: 208 - DNA, 12153 bp, synthetic construct
  misc_feature 1..12153: note = DNA of V14-scFv-KRAB-2a-D3a-D3l-dCas9-10xGCN4
  source 1..12153: mol_type = other DNA
tcatatatactttagattgatttaaaacttcatttttaatttaaaaggatctaggtgaagatcctttttgataatctcatgaccaaaatcccttaacgtgagttttcgttccactgagcgtcagaccccgtagaaaagatcaaaggatcttcttgagatcctttttttctgcgcgtaatctgctgcttgcaaacaaaaaaaccaccgctaccagcggtggtttgtttgccggatcaagagctaccaactctttttccgaaggtaactggcttcagcagagcgcagataccaaatactgttcttctagtgtagccgtagttaggccaccacttcaagaactctgtagcaccgcctacatacctcgctctgctaatcctgttaccagtggctgctgccagtggcgataagtcgtgtcttaccgggttggactcaagacgatagttaccggataaggcgcagcggtcgggctgaacggggggttcgtgcacacagcccagcttggagcgaacgacctacaccgaactgagatacctacagcgtgagctatgagaaagcgccacgcttcccgaagggagaaaggcggacaggtatccggtaagcggcagggtcggaacaggagagcgcacgagggagcttccagggggaaacgcctggtatctttatagtcctgtcgggtttcgccacctctgacttgagcgtcgatttttgtgatgctcgtcaggggggcggagcctatggaaaaacgccagcaacgcggcctttttacggttcctggccttttgctggccttttgctcacatgttctttcctgcgttatcccctgattctgtggataaccgtattaccgcctttgagtgagctgataccgctcgccgcagccgaacgaccgagcgcagcgagtcagtgagcgaggaagcggaagagcgcccaatacgcaaaccgcctctccccgcgcgttggccgattcattaatgcagctggcacgacaggtttcccgactggaaagcgggcagtgagcgcaacgcaattaatgtgagttagctcactcattaggcaccccaggctttacactttatgcttccggctcgtatgttgtgtggaattgtgagcggataacaatttcacacaggaaacagctatgaccatgattacgcctctagaaagctttaatacgactcactataaggactcactatttgttttcgcgcccagttgcaaaaagtgtcgacatttgcttctgacacaactgtgttcactagcaacctcaaacagacaccgccaccatgggccccgacatcgtgatgacccagagccccagcagcctgagcgccagcgtgggcgaccgcgtgaccatcacctgccgcagcagcaccggcgccgtgaccaccagcaactacgccagctgggtgcaggagaagcccggcaagctgttcaagggcctgatcggcggcaccaacaaccgcgcccccggcgtgcccagccgcttcagcggcagcctgatcggcgacaaggccaccctgaccatcagcagcctgcagcccgaggacttcgccacctacttctgcgccctgtggtacagcaaccactgggtgttcggccagggcaccaaggtggagctgaagcgcggcggcggcggcagcggcggcggcggcagcggcggcggcggcagcagcggcggcggcagcgaggtgaagctgctggagagcggcggcggcctggtgcagcccggcggcagcctgaagctgagctgcgccgtgagcggcttcagcctgaccgactacggcgtgaactgggtgcgccaggcccccggccgcggcctggagtggatcggcgtgatctggggcgacggcatcaccgactacaacagcgccctgaaggaccgcttcatcatcagcaaggacaacggcaagaacaccgtgtacctgcagatgagcaaggtgcgcagcgacgacaccgccctgtactactgcgtgaccggcctgttcgactactggggccagggcaccctggtgaccgtgagcagctacccatacgatgttccagattacgctggtggaggcggaggttctgggggaggaggtagtggcggtggtggttcaggaggcggcggaagcttggatccaggtggaggtggaagcggtcggacactggtgaccttcaaggatgtatttgtggacttcaccagggaggagtggaagctgctggacactgctcagcagatcgtgtacagaaatgtgatgctggagaactataagaacctggtttccttgggttatcagcttactaagccagatgtgatcctccggttggagaagggagaagagcccggaagcggaaagcgcaccgccgatggttccgagttcgaaagccccaaaaaaaagcgcaaggtcggaagcggagctactaacttcagcctgctgaagcaggctggagacgtggaggagaaccctggacctatgaaccatgaccaggaatttgaccccccaaaggtttacccacctgtgccagctgagaagaggaagcccatccgcgtgctgtctctctttgatgggattgctacagggctcctggtgctgaaggacctgggcatccaagtggaccgctacattgcctccgaggtgtgtgaggactccatcacggtgggcatggtgcggcaccagggaaagatcatgtacgtcggggacgtccgcagcgtcacacagaagcatatccaggagtggggcccattcgacctggtgattggaggcagtccctgcaatgacctctccattgtcaaccctgcccgcaagggactttatgagggtactggccgcctcttctttgagttctaccgcctcctgcatgatgcgcggcccaaggagggagatgatcgccccttcttctggctctttgagaatgtggtggccatgggcgttagtgacaagagggacatctcgcgatttcttgagtctaaccccgtgatgattgacgccaaagaagtgtctgctgcacacagggcccgttacttctggggtaaccttcctggcatgaacaggcctttggcatccactgtgaatgataagctggagctgcaagagtgtctggagcacggcagaatagccaagttcagcaaagtgaggaccattaccaccaggtcaaactctataaagcagggcaaagaccagcatttccccgtcttcatgaacgagaaggaggacatcctgtggtgcactgaaatggaaagggtgtttggcttccccgtccactacacagacgtctccaacatgagccgcttggcgaggcagagactgctgggccgatcgtggagcgtgccggtcatccgccacctcttcgctccgctgaaggaatattttgcttgtgtgtctagcggcaatagtaacgctaacagccgcgggccgagcttcagcagcggcctggtgccgttaagcttgcgcggcagccatatgggccctatggagatatacaagacagtgtctgcatggaagagacagccagtgcgggtactgagcctcttcagaaacatcgacaaggtactaaagagtttgggcttcttggaaagcggttctggttctgggggaggaacgctgaagtacgtggaagatgtcacaaatgtcgtgaggagagacgtggagaaatggggcccctttgacctggtgtacggctcgacgcagcccctaggcagctcttgtgatcgctgtcccggctggtacatgttccagttccaccggatcctgcagtatgcgctgcctcgccaggagagtcagcggcccttcttctggatattcatggacaatctgctgctgactgaggatgaccaagagacaactacccgcttccttcagacagaggctgtgaccctccaggatgtccgtggcagagactaccagaatgctatgcgggtgtggagcaacattccagggctgaagagcaagcatgcgcccctgaccccaaaggaagaagagtatctgcaagcccaagtcagaagcaggagcaagctggacgccccgaaagttgacctcctggtgaagaactgccttctcccgctgagagagtacttcaagtatttttctcaaaactcacttcctcttggagggccgagctctggcgcacccccaccaagtggagggtctcctgccgggtccccaacatctactgaagaaggcaccagcgaatccgcaacgcccgagtcaggccctggtacctccacagaaccatctgaaggtagtgcgcctggttccccagctggaagccctacttccaccgaagaaggcacgtcaaccgaaccaagtgaaggatctgcccctgggaccagcactgaaccatctgagccaaaaaagaagagaaaggtaatggacaagaagtacagcatcggcctggccatcggcaccaactctgtgggctgggccgtgatcaccgacgagtacaaggtgcccagcaagaaattcaaggtgctgggcaacaccgaccggcacagcatcaagaagaacctgatcggcgccctgctgttcgacagcggagaaacagccgaggccacccggctgaagagaaccgccagaagaagatacaccagacggaagaaccggatctgctatctgcaagagatcttcagcaacgagatggccaaggtggacgacagcttcttccacagactggaagagtccttcctggtggaagaggataagaagcacgagcggcaccccatcttcggcaacatcgtggacgaggtggcctaccacgagaagtaccccaccatctaccacctgagaaagaaactggtggacagcaccgacaaggccgacctgcggctgatctatctggccctggcccacatgatcaagttccggggccacttcctgatcgagggcgacctgaaccccgacaacagcgacgtggacaagctgttcatccagctggtgcagacctacaaccagctgttcgaggaaaaccccatcaacgccagcggcgtggacgccaaggccatcctgtctgccagactgagcaagagcagacggctggaaaatctgatcgcccagctgcccggcgagaagaagaatggcctgttcggcaacctgattgccctgagcctgggcctgacccccaacttcaagagcaacttcgacctggccgaggatgccaaactgcagctgagcaaggacacctacgacgacgacctggacaacctgctggcccagatcggcgaccagtacgccgacctgtttctggccgccaagaacctgtccgacgccatcctgctgagcgacatcctgagagtgaacaccgagatcaccaaggcccccctgagcgcctctatgatcaagagatacgacgagcaccaccaggacctgaccctgctgaaagctctcgtgcggcagcagctgcctgagaagtacaaagagattttcttcgaccagagcaagaacggctacgccggctacatcgatggcggagccagccaggaagagttctacaagttcatcaagcccatcctggaaaagatggacggcaccgaggaactgctcgtgaagctgaacagagaggacctgctgcggaagcagcggaccttcgacaacggcagcatcccccaccagatccacctgggagagctgcacgccattctgcggcggcaggaagatttttacccattcctgaaggacaaccgggaaaagatcgagaagatcctgaccttccgcatcccctactacgtgggccctctggccaggggaaacagcagattcgcctggatgaccagaaagagcgaggaaaccatcaccccctggaacttcgaggaagtggtggacaagggcgccagcgcccagagcttcatcgagcggatgaccaacttcgataagaacctgcccaacgagaaggtgctgcccaagcacagcctgctgtacgagtacttcaccgtgtacaacgagctgaccaaagtgaaatacgtgaccgagggaatgagaaagcccgccttcctgagcggcgagcagaaaaaagccatcgtggacctgctgttcaagaccaaccggaaagtgaccgtgaagcagctgaaagaggactacttcaagaaaatcgagtgcttcgactccgtggaaatctccggcgtggaagatcggttcaacgcctccctgggcacataccacgatctgctgaaaattatcaaggacaaggacttcctggacaatgaggaaaacgaggacattctggaagatatcgtgctgaccctgacactgtttgaggacagagagatgatcgaggaacggctgaaaacctatgcccacctgttcgacgacaaagtgatgaagcagctgaagcggcggagatacaccggctggggcaggctgagccggaagctgatcaacggcatccgggacaagcagtccggcaagacaatcctggatttcctgaagtccgacggcttcgccaacagaaacttcatgcagctgatccacgacgacagcctgacctttaaagaggacatccagaaagcccaggtgtccggccagggcgatagcctgcacgagcacattgccaatctggccggcagccccgccattaagaagggcatcctgcagacagtgaaggtggtggacgagctcgtgaaagtgatgggccggcacaagcccgagaacatcgtgatcgaaatggccagagagaaccagaccacccagaagggacagaagaacagccgcgagagaatgaagcggatcgaagagggcatcaaagagctgggcagccagatcctgaaagaacaccccgtggaaaacacccagctgcagaacgagaagctgtacctgtactacctgcagaatgggcgggatatgtacgtggaccaggaactggacatcaaccggctgtccgactacgatgtggacgctatcgtgcctcagagctttctgaaggacgactccatcgataacaaagtgctgactcggagcgacaagaaccggggcaagagcgacaacgtgccctccgaagaggtcgtgaagaagatgaagaactactggcgccagctgctgaatgccaagctgattacccagaggaagttcgacaatctgaccaaggccgagagaggcggcctgagcgaactggataaggccggcttcatcaagagacagctggtggaaacccggcagatcacaaagcacgtggcacagatcctggactcccggatgaacactaagtacgacgagaacgacaaactgatccgggaagtgaaagtgatcaccctgaagtccaagctggtgtccgatttccggaaggatttccagttttacaaagtgcgcgagatcaacaactaccaccacgcccacgacgcctacctgaacgccgtcgtgggaaccgccctgatcaaaaagtaccctaagctggaaagcgagttcgtgtacggcgactacaaggtgtacgacgtgcggaagatgatcgccaagagcgagcaggaaatcggcaaggctaccgccaagtacttcttctacagcaacatcatgaactttttcaagaccgagattaccctggccaacggcgagatccggaagcggcctctgatcgagacaaacggcgaaacaggcgagatcgtgtgggataagggccgggactttgccaccgtgcggaaagtgctgtctatgccccaagtgaatatcgtgaaaaagaccgaggtgcagacaggcggcttcagcaaagagtctatcctgcccaagaggaacagcgacaagctgatcgccagaaagaaggactgggaccctaagaagtacggcggcttcgacagccccaccgtggcctattctgtgctggtggtggccaaagtggaaaagggcaagtccaagaaactgaagagtgtgaaagagctgctggggatcaccatcatggaaagaagcagcttcgagaagaatcccatcgactttctggaagccaagggctacaaagaagtgaaaaaggacctgatcatcaagctgcctaagtactccctgttcgagctggaaaacggccggaagagaatgctggcctctgccggcgaactgcagaagggaaacgaactggccctgccctccaaatatgtgaacttcctgtacctggccagccactatgagaagctgaagggctcccccgaggataatgagcagaaacagctgtttgtggaacagcacaaacactacctggacgagatcatcgagcagatcagcgagttctccaagagagtgatcctggccgacgctaatctggacaaggtgctgagcgcctacaacaagcacagagacaagcctatcagagagcaggccgagaatatcatccacctgtttaccctgaccaatctgggagcccctgccgccttcaagtactttgacaccaccatcgaccggaagaggtacaccagcaccaaagaggtgctggacgccaccctgatccaccagagcatcaccggcctgtacgagacacggatcgacctgtctcagctgggaggcgacgcctatccctatgacgtgcccgattatgccagcctgggcagcggctcccccaagaaaaaacgcaaggtggaagatcctaagaaaaagcggaaagtggacggcattggtagtgggagcaacggcagcagcggagaggaactgctgagcaagaactaccacctggaaaacgaggtggccagactgaagaaaggctctggctctggcggaagcggttctggcggatcaggatctggaagtggcggctctggaagcggaggttctggatctggcgaagaactgctgtctaagaattatcacctcgagaacgaagtggctcggctcaagaaaggcagtggcagcggaggaagtggatccggcggtagtggtagtggaagcggcggatccggctcaggcggatctggttcaggggaagaactcctctccaaaaactaccatctcgagaatgaggtcgcccgcctgaaaaaaggatcaggttccggtggttctggcagcggtggttcaggctcaggcagcggcggtagcggtagcggtggaagcggaagcggagaagaacttctcagcaaaaattaccacttggagaatgaagttgcaagactcaaaaaaggttccggcagtggcggcagcggcagcggcggatctggtagtggatctggtggcagtggttcaggcggaagtggtagcggagaggaattgctctcaaagaactatcatttggagaacgaggttgcacgcttgaagaaaggcagcggatcaggcggatctggcagcggtggatctggttctggatccggcggctccggtagtggtggaagtggctctggggaagaattgcttagcaagaattatcatcttgaaaatgaggttgccaggcttaaaaaaggcagtggctccggcggatccggaagcggaggcagcggatctggatctggtggttcaggatctggcggttctggtagcggggaagaactgttgagtaaaaactatcaccttgagaacgaggtcgcaaggttgaaaaaaggatccggctctggcggctccggaagtggcggatctggctccggtagcggaggatcaggatccggcggaagcggatcaggcgaggaactgctttccaaaaattaccaccttgaaaacgaagtcgcccgcctcaagaaaggttctggcagcggaggctctggcagtggtggtagcggaagtggaagtggtggcagtggtagcggtggatctggaagcggcgaggaactcctgtcaaagaattaccatctcgaaaacgaggtcgcaaggctcaagaaaggctcaggatcaggcggctctggatccggcggttctggttccggctcaggtggaagtggatctggcggctcaggttccggcgaagaattgctttccaagaactaccatttggaaaatgaagtcgctcgtttgaagaaaggttcaggctccggccagcggggaagcaagcgcaccgccgatggttccgagttcgaaagccccaaaaaaaagcgcaaggtctgagatcccaagcacgcagcaatgcagctcaaaacgcttagcctagccacacccccacgggaaacagcagtgattaacctttagcaataaacgaaagtttaactaagctatactaaccccagggttggtcaatttcgtgccagccacaccctggtactgcatgcacgcaatgctagctgcccctttcccgtcctgggcaccccgagtctcccccgaccccgggtcccaggtatgctcccacctccacctgccccactcaccacctctgctagttccagacacctccgagacgaggaaaaaaaaaaaaaaaaaaaaaaaaaaaaaaaaaaaaaaaaaaaaaaaaaaaaaaaaaaaaaaaaaaaaaaaaaaaaaaaaaaaaaaaaaaaaaaaaaaaaaaaaaaaaaaaaaaaaaaaaaaaaaaaaaaaaaaaaaaaaaaaaaaaaaaaaaaaaaaaaaaaaaaaaaaaaaaaaaaaaaaaaaaaaaaaaaaaaaaaaaaaaaaaaaaaaaaaaaaaaaaaaaaaaaaaaaaaaaaaaaaaaaaaaaaaaaaaaaaaaaaaaaaaaaaaaaaaaaaaaaaaaaaaaaaaaaaaaaaaaaaaaaaaaaaaaaaaaaaaaaaaaaaaaaaaaaaaaaaaaaaaaaaaaaaaaaaaaaaaaaaaaaaaaaaaaaaaaaaaaaaaaaaaaaaaaaaccgtcttcaagctttctagaaattcactggccgtcgttttacaacgtcgtgactgggaaaaccctggcgttacccaacttaatcgccttgcagcacatccccctttcgccagctggcgtaatagcgaagaggcccgcaccgatcgcccttcccaacagttgcgcagcctgaatggcgaatggcgcctgatgcggtattttctccttacgcatctgtgcggtatttcacaccgcatatggtgcactctcagtacaatctgctctgatgccgcatagttaagccagccccgacacccgccaacacccgctgacgcgccctgacgggcttgtctgctcccggcatccgcttacagacaagctgtgaccgtctccgggagctgcatgtgtcagaggttttcaccgtcatcaccgaaacgcgcgagacgaaagggcctcgtgatacgcctatttttataggttaatgtcatgataataatggtttcttagacgtcaggtggcacttttcggggaaatgtgcgcggaacccctatttgtttatttttctaaatacattcaaatatgtatccgctcatgagacaataaccctgataaatgcttcaataatattgaaaaaggaagagtatgagtattcaacatttccgtgtcgcccttattcccttttttgcggcattttgccttcctgtttttgctcacccagaaacgctggtgaaagtaaaagatgctgaagatcagttgggtgcacgagtgggttacatcgaactggatctcaacagcggtaagatccttgagagttttcgccccgaagaacgttttccaatgatgagcacttttaaagttctgctatgtggcgcggtattatcccgtattgacgccgggcaagagcaactcggtcgccgcatacactattctcagaatgacttggttgagtactcaccagtcacagaaaagcatcttacggatggcatgacagtaagagaattatgcagtgctgccataaccatgagtgataacactgcggccaacttacttctgacaacgatcggaggaccgaaggagctaaccgcttttttgcacaacatgggggatcatgtaactcgccttgatcgttgggaaccggagctgaatgaagccataccaaacgacgagcgtgacaccacgatgcctgtagcaatggcaacaacgttgcgcaaactattaactggcgaactacttactctagcttcccggcaacaattaatagactggatggaggcggataaagttgcaggaccacttctgcgctcggcccttccggctggctggtttattgctgataaatctggagccggtgagcgtgggtctcgcggtatcattgcagcactggggccagatggtaagccctcccgtatcgtagttatctacacgacggggagtcaggcaactatggatgaacgaaatagacagatcgctgagataggtgcctcactgattaagcattggtaactgtcagaccaagtttac

SEQ ID NO: 209 - DNA, 11100 bp, synthetic construct
  misc_feature 1..11100: note = DNA of V15_scFv-ZIM3-2a-D3a-hD3L-dCas9-1xGCN4
  source 1..11100: mol_type = other DNA
tcatatatactttagattgatttaaaacttcatttttaatttaaaaggatctaggtgaagatcctttttgataatctcatgaccaaaatcccttaacgtgagttttcgttccactgagcgtcagaccccgtagaaaagatcaaaggatcttcttgagatcctttttttctgcgcgtaatctgctgcttgcaaacaaaaaaaccaccgctaccagcggtggtttgtttgccggatcaagagctaccaactctttttccgaaggtaactggcttcagcagagcgcagataccaaatactgttcttctagtgtagccgtagttaggccaccacttcaagaactctgtagcaccgcctacatacctcgctctgctaatcctgttaccagtggctgctgccagtggcgataagtcgtgtcttaccgggttggactcaagacgatagttaccggataaggcgcagcggtcgggctgaacggggggttcgtgcacacagcccagcttggagcgaacgacctacaccgaactgagatacctacagcgtgagctatgagaaagcgccacgcttcccgaagggagaaaggcggacaggtatccggtaagcggcagggtcggaacaggagagcgcacgagggagcttccagggggaaacgcctggtatctttatagtcctgtcgggtttcgccacctctgacttgagcgtcgatttttgtgatgctcgtcaggggggcggagcctatggaaaaacgccagcaacgcggcctttttacggttcctggccttttgctggccttttgctcacatgttctttcctgcgttatcccctgattctgtggataaccgtattaccgcctttgagtgagctgataccgctcgccgcagccgaacgaccgagcgcagcgagtcagtgagcgaggaagcggaagagcgcccaatacgcaaaccgcctctccccgcgcgttggccgattcattaatgcagctggcacgacaggtttcccgactggaaagcgggcagtgagcgcaacgcaattaatgtgagttagctcactcattaggcaccccaggctttacactttatgcttccggctcgtatgttgtgtggaattgtgagcggataacaatttcacacaggaaacagctatgaccatgattacgcctctagaaagctttaatacgactcactataaggactcactatttgttttcgcgcccagttgcaaaaagtgtcgacatttgcttctgacacaactgtgttcactagcaacctcaaacagacaccgccaccatgcctgctgctaagagagtgaaactggatggatccggccccgacatcgtgatgacccagagccccagcagcctgagcgccagcgtgggcgaccgcgtgaccatcacctgccgcagcagcaccggcgccgtgaccaccagcaactacgccagctgggtgcaggagaagcccggcaagctgttcaagggcctgatcggcggcaccaacaaccgcgcccccggcgtgcccagccgcttcagcggcagcctgatcggcgacaaggccaccctgaccatcagcagcctgcagcccgaggacttcgccacctacttctgcgccctgtggtacagcaaccactgggtgttcggccagggcaccaaggtggagctgaagcgcggcggcggcggcagcggcggcggcggcagcggcggcggcggcagcagcggcggcggcagcgaggtgaagctgctggagagcggcggcggcctggtgcagcccggcggcagcctgaagctgagctgcgccgtgagcggcttcagcctgaccgactacggcgtgaactgggtgcgccaggcccccggccgcggcctggagtggatcggcgtgatctggggcgacggcatcaccgactacaacagcgccctgaaggaccgcttcatcatcagcaaggacaacggcaagaacaccgtgtacctgcagatgagcaaggtgcgcagcgacgacaccgccctgtactactgcgtgaccggcctgttcgactactggggccagggcaccctggtgaccgtgagcagctacccatacgatgttccagattacgctggtggaggcggaggttctgggggaggaggtagtggcggtggtggttcaggaggcggcggaagcttggatccaggtggaggtggaagcggtatgaacaattcccagggaagagtgaccttcgaggacgtgaccgtgaacttcacccaaggcgagtggcagagactgaaccccgagcagagaaacctgtaccgggacgtgatgctggaaaactacagcaacctggtgtccgtcggccagggcgagacaacaaagcctgacgtgatcctgcggctggaacagggcaaagagccttggctggaagaggaagaggtgctcggatctggcagagccgagaagaatggcgatatcggcggacagatctggaagccaaaggatgtgaaagagagtctcggaagcggagctactaacttcagcctgctgaagcaggctggagacgtggaggagaaccctggacctatgcctgctgctaagagagtgaaactggatggatccaaccatgaccaggaatttgaccccccaaaggtttacccacctgtgccagctgagaagaggaagcccatccgcgtgctgtctctctttgatgggattgctacagggctcctggtgctgaaggacctgggcatccaagtggaccgctacattgcctccgaggtgtgtgaggactccatcacggtgggcatggtgcggcaccagggaaagatcatgtacgtcggggacgtccgcagcgtcacacagaagcatatccaggagtggggcccattcgacctggtgattggaggcagtccctgcaatgacctctccattgtcaaccctgcccgcaagggactttatgagggtactggccgcctcttctttgagttctaccgcctcctgcatgatgcgcggcccaaggagggagatgatcgccccttcttctggctctttgagaatgtggtggccatgggcgttagtgacaagagggacatctcgcgatttcttgagtctaaccccgtgatgattgacgccaaagaagtgtctgctgcacacagggcccgttacttctggggtaaccttcctggcatgaacaggcctttggcatccactgtgaatgataagctggagctgcaagagtgtctggagcacggcagaatagccaagttcagcaaagtgaggaccattaccaccaggtcaaactctataaagcagggcaaagaccagcatttccccgtgttcatgaacgagaaggaggacatcctgtggtgcactgaaatggaaagggtgtttggcttccccgtccactacacagacgtctccaacatgagccgcttggcgaggcagagactgctgggccgatcgtggagcgtgccggtcatccgccacctcttcgctccgctgaaggaatattttgcttgtgtgtctagcggcaatagtaacgctaacagccgcgggccgagcttcagcagcggcctggtgccgttaagcttgcgcggcagccatatgttcgaaaccgtgcctgtgtggaggagacagccagtccgggtgctgtccctttttgaagacatcaagaaagagctgacgagtttgggctttttggaaagtggttctgacccgggacaactgaagcatgtggttgatgtcacagacacagtgaggaaggatgtggaggagtggggacccttcgatcttgtgtacggcgccacacctcccctgggccacacctgtgaccgtcctcccagctggtacctgttccagttccaccggctcctgcagtacgcacggcccaagccaggcagccccaggcccttcttctggatgttcgtggacaatctggtgctgaacaaggaagacctggacgtcgcatctcgcttcctggagatggagccagtcaccatcccagatgtccacggcggatccttgcagaatgctgtccgcgtgtggagcaacatcccagccataaggagcagcaggcactgggctctggtttcggaagaagaattgtccctgctggcccagaacaagcagagctcgaagctcgcggccaagtggcccaccaagctggtgaagaactgctttctccccctaagagaatatttcaagtatttttcaggagggccgagctctggcgcacccccaccaagtggagggtctcctgccgggtccccaacatctactgaagaaggcaccagcgaatccgcaacgcccgagtcaggccctggtacctccacagaaccatctgaaggtagtgcgcctggttccccagctggaagccctacttccaccgaagaaggcacgtcaaccgaaccaagtgaaggatctgcccctgggaccagcactgaaccatctgagccaaaaaagaagagaaaggtaatggacaagaagtacagcatcggcctggccatcggcaccaactctgtgggctgggccgtgatcaccgacgagtacaaggtgcccagcaagaaattcaaggtgctgggcaacaccgaccggcacagcatcaagaagaacctgatcggcgccctgctgttcgacagcggagaaacagccgaggccacccggctgaagagaaccgccagaagaagatacaccagacggaagaaccggatctgctatctgcaagagatcttcagcaacgagatggccaaggtggacgacagcttcttccacagactggaagagtccttcctggtggaagaggataagaagcacgagcggcaccccatcttcggcaacatcgtggacgaggtggcctaccacgagaagtaccccaccatctaccacctgagaaagaaactggtggacagcaccgacaaggccgacctgcggctgatctatctggccctggcccacatgatcaagttccggggccacttcctgatcgagggcgacctgaaccccgacaacagcgacgtggacaagctgttcatccagctggtgcagacctacaaccagctgttcgaggaaaaccccatcaacgccagcggcgtggacgccaaggccatcctgtctgccagactgagcaagagcagacggctggaaaatctgatcgcccagctgcccggcgagaagaagaatggcctgttcggcaacctgattgccctgagcctgggcctgacccccaacttcaagagcaacttcgacctggccgaggatgccaaactgcagctgagcaaggacacctacgacgacgacctggacaacctgctggcccagatcggcgaccagtacgccgacctgtttctggccgccaagaacctgtccgacgccatcctgctgagcgacatcctgagagtgaacaccgagatcaccaaggcccccctgagcgcctctatgatcaagagatacgacgagcaccaccaggacctgaccctgctgaaagctctcgtgcggcagcagctgcctgagaagtacaaagagattttcttcgaccagagcaagaacggctacgccggctacatcgatggcggagccagccaggaagagttctacaagttcatcaagcccatcctggaaaagatggacggcaccgaggaactgctcgtgaagctgaacagagaggacctgctgcggaagcagcggaccttcgacaacggcagcatcccccaccagatccacctgggagagctgcacgccattctgcggcggcaggaagatttttacccattcctgaaggacaaccgggaaaagatcgagaagatcctgaccttccgcatcccctactacgtgggccctctggccaggggaaacagcagattcgcctggatgaccagaaagagcgaggaaaccatcaccccctggaacttcgaggaagtggtggacaagggcgccagcgcccagagcttcatcgagcggatgaccaacttcgataagaacctgcccaacgagaaggtgctgcccaagcacagcctgctgtacgagtacttcaccgtgtacaacgagctgaccaaagtgaaatacgtgaccgagggaatgagaaagcccgccttcctgagcggcgagcagaaaaaagccatcgtggacctgctgttcaagaccaaccggaaagtgaccgtgaagcagctgaaagaggactacttcaagaaaatcgagtgcttcgactccgtggaaatctccggcgtggaagatcggttcaacgcctccctgggcacataccacgatctgctgaaaattatcaaggacaaggacttcctggacaatgaggaaaacgaggacattctggaagatatcgtgctgaccctgacactgtttgaggacagagagatgatcgaggaacggctgaaaacctatgcccacctgttcgacgacaaagtgatgaagcagctgaagcggcggagatacaccggctggggcaggctgagccggaagctgatcaacggcatccgggacaagcagtccggcaagacaatcctggatttcctgaagtccgacggcttcgccaacagaaacttcatgcagctgatccacgacgacagcctgacctttaaagaggacatccagaaagcccaggtgtccggccagggcgatagcctgcacgagcacattgccaatctggccggcagccccgccattaagaagggcatcctgcagacagtgaaggtggtggacgagctcgtgaaagtgatgggccggcacaagcccgagaacatcgtgatcgaaatggccagagagaaccagaccacccagaagggacagaagaacagccgcgagagaatgaagcggatcgaagagggcatcaaagagctgggcagccagatcctgaaagaacaccccgtggaaaacacccagctgcagaacgagaagctgtacctgtactacctgcagaatgggcgggatatgtacgtggaccaggaactggacatcaaccggctgtccgactacgatgtggacgctatcgtgcctcagagctttctgaaggacgactccatcgataacaaagtgctgactcggagcgacaagaaccggggcaagagcgacaacgtgccctccgaagaggtcgtgaagaagatgaagaactactggcgccagctgctgaatgccaagctgattacccagaggaagttcgacaatctgaccaaggccgagagaggcggcctgagcgaactggataaggccggcttcatcaagagacagctggtggaaacccggcagatcacaaagcacgtggcacagatcctggactcccggatgaacactaagtacgacgagaacgacaaactgatccgggaagtgaaagtgatcaccctgaagtccaagctggtgtccgatttccggaaggatttccagttttacaaagtgcgcgagatcaacaactaccaccacgcccacgacgcctacctgaacgccgtcgtgggaaccgccctgatcaaaaagtaccctaagctggaaagcgagttcgtgtacggcgactacaaggtgtacgacgtgcggaagatgatcgccaagagcgagcaggaaatcggcaaggctaccgccaagtacttcttctacagcaacatcatgaactttttcaagaccgagattaccctggccaacggcgagatccggaagcggcctctgatcgagacaaacggcgaaacaggcgagatcgtgtgggataagggccgggactttgccaccgtgcggaaagtgctgtctatgccccaagtgaatatcgtgaaaaagaccgaggtgcagacaggcggcttcagcaaagagtctatcctgcccaagaggaacagcgacaagctgatcgccagaaagaaggactgggaccctaagaagtacggcggcttcgacagccccaccgtggcctattctgtgctggtggtggccaaagtggaaaagggcaagtccaagaaactgaagagtgtgaaagagctgctggggatcaccatcatggaaagaagcagcttcgagaagaatcccatcgactttctggaagccaagggctacaaagaagtgaaaaaggacctgatcatcaagctgcctaagtactccctgttcgagctggaaaacggccggaagagaatgctggcctctgccggcgaactgcagaagggaaacgaactggccctgccctccaaatatgtgaacttcctgtacctggccagccactatgagaagctgaagggctcccccgaggataatgagcagaaacagctgtttgtggaacagcacaaacactacctggacgagatcatcgagcagatcagcgagttctccaagagagtgatcctggccgacgctaatctggacaaggtgctgagcgcctacaacaagcacagagacaagcctatcagagagcaggccgagaatatcatccacctgtttaccctgaccaatctgggagcccctgccgccttcaagtactttgacaccaccatcgaccggaagaggtacaccagcaccaaagaggtgctggacgccaccctgatccaccagagcatcaccggcctgtacgagacacggatcgacctgtctcagctgggaggcgacgcctatccctatgacgtgcccgattatgccagcctgggcagcggctcccccaagaaaaaacgcaaggtggaagatcctaagaaaaagcggaaagtggacggcattggtagtgggagcaacggcagcagcggagaggaactgctgagcaagaactaccacctggaaaacgaggtggccagactgaagaaaggctctggctctggcggaagcggttctggcggatcaggatctggaagtggcggctctggaagcggaggttctggatctggcgaagaactgctgtctaagaattatcacggttcaggctccggccagcggggaagcaagcgcaccgccgatggttccgagttcgaaagccccaaaaaaaagcgcaaggtctgagatcccaagcacgcagcaatgcagctcaaaacgcttagcctagccacacccccacgggaaacagcagtgattaacctttagcaataaacgaaagtttaactaagctatactaaccccagggttggtcaatttcgtgccagccacaccctggtactgcatgcacgcaatgctagctgcccctttcccgtcctgggcaccccgagtctcccccgaccccgggtcccaggtatgctcccacctccacctgccccactcaccacctctgctagttccagacacctccgagacgaggaaaaaaaaaaaaaaaaaaaaaaaaaaaaaaaaaaaaaaaaaaaaaaaaaaaaaaaaaaaaaaaaaaaaaaaaaaaaaaaaaaaaaaaaaaaaaaaaaaaaaaaaaaaaaaaaaaaaaaaaaaaaaaaaaaaaaaaaaaaaaaaaaaaaaaaaaaaaaaaaaaaaaaaaaaaaaaaaaaaaaaaaaaaaaaaaaaaaaaaaaaaaaaaaaaaaaaaaaaaaaaaaaaaaaaaaaaaaaaaaaaaaaaaaaaaaaaaaaaaaaaaaaaaaaaaaaaaaaaaaaaaaaaaaaaaaaaaaaaaaaaaaaaaaaaaaaaaaaaaaaaaaaaaaaaaaaaaaaaaaaaaaaaaaaaaaaaaaaaaaaaaaaaaaaaaaaaaaaaaaaaaaaaaaaaaaaaccgtcttcaagctttctagaaattcactggccgtcgttttacaacgtcgtgactgggaaaaccctggcgttacccaacttaatcgccttgcagcacatccccctttcgccagctggcgtaatagcgaagaggcccgcaccgatcgcccttcccaacagttgcgcagcctgaatggcgaatggcgcctgatgcggtattttctccttacgcatctgtgcggtatttcacaccgcatatggtgcactctcagtacaatctgctctgatgccgcatagttaagccagccccgacacccgccaacacccgctgacgcgccctgacgggcttgtctgctcccggcatccgcttacagacaagctgtgaccgtctccgggagctgcatgtgtcagaggttttcaccgtcatcaccgaaacgcgcgagacgaaagggcctcgtgatacgcctatttttataggttaatgtcatgataataatggtttcttagacgtcaggtggcacttttcggggaaatgtgcgcggaacccctatttgtttatttttctaaatacattcaaatatgtatccgctcatgagacaataaccctgataaatgcttcaataatattgaaaaaggaagagtatgagtattcaacatttccgtgtcgcccttattcccttttttgcggcattttgccttcctgtttttgctcacccagaaacgctggtgaaagtaaaagatgctgaagatcagttgggtgcacgagtgggttacatcgaactggatctcaacagcggtaagatccttgagagttttcgccccgaagaacgttttccaatgatgagcacttttaaagttctgctatgtggcgcggtattatcccgtattgacgccgggcaagagcaactcggtcgccgcatacactattctcagaatgacttggttgagtactcaccagtcacagaaaagcatcttacggatggcatgacagtaagagaattatgcagtgctgccataaccatgagtgataacactgcggccaacttacttctgacaacgatcggaggaccgaaggagctaaccgcttttttgcacaacatgggggatcatgtaactcgccttgatcgttgggaaccggagctgaatgaagccataccaaacgacgagcgtgacaccacgatgcctgtagcaatggcaacaacgttgcgcaaactattaactggcgaactacttactctagcttcccggcaacaattaatagactggatggaggcggataaagttgcaggaccacttctgcgctcggcccttccggctggctggtttattgctgataaatctggagccggtgagcgtgggtctcgcggtatcattgcagcactggggccagatggtaagccctcccgtatcgtagttatctacacgacggggagtcaggcaactatggatgaacgaaatagacagatcgctgagataggtgcctcactgattaagcattggtaactgtcagaccaagtttac

SEQ ID NO: 210 - DNA, 11130 bp, synthetic construct
  misc_feature 1..11130: note = DNA of V16_scFv-ZIM3-2a-D3a-hD3L-dCas9-2xGCN4
  source 1..11130: mol_type = other DNA
tcatatatactttagattgatttaaaacttcatttttaatttaaaaggatctaggtgaagatcctttttgataatctcatgaccaaaatcccttaacgtgagttttcgttccactgagcgtcagaccccgtagaaaagatcaaaggatcttcttgagatcctttttttctgcgcgtaatctgctgcttgcaaacaaaaaaaccaccgctaccagcggtggtttgtttgccggatcaagagctaccaactctttttccgaaggtaactggcttcagcagagcgcagataccaaatactgttcttctagtgtagccgtagttaggccaccacttcaagaactctgtagcaccgcctacatacctcgctctgctaatcctgttaccagtggctgctgccagtggcgataagtcgtgtcttaccgggttggactcaagacgatagttaccggataaggcgcagcggtcgggctgaacggggggttcgtgcacacagcccagcttggagcgaacgacctacaccgaactgagatacctacagcgtgagctatgagaaagcgccacgcttcccgaagggagaaaggcggacaggtatccggtaagcggcagggtcggaacaggagagcgcacgagggagcttccagggggaaacgcctggtatctttatagtcctgtcgggtttcgccacctctgacttgagcgtcgatttttgtgatgctcgtcaggggggcggagcctatggaaaaacgccagcaacgcggcctttttacggttcctggccttttgctggccttttgctcacatgttctttcctgcgttatcccctgattctgtggataaccgtattaccgcctttgagtgagctgataccgctcgccgcagccgaacgaccgagcgcagcgagtcagtgagcgaggaagcggaagagcgcccaatacgcaaaccgcctctccccgcgcgttggccgattcattaatgcagctggcacgacaggtttcccgactggaaagcgggcagtgagcgcaacgcaattaatgtgagttagctcactcattaggcaccccaggctttacactttatgcttccggctcgtatgttgtgtggaattgtgagcggataacaatttcacacaggaaacagctatgaccatgattacgcctctagaaagctttaatacgactcactataaggactcactatttgttttcgcgcccagttgcaaaaagtgtcgacatttgcttctgacacaactgtgttcactagcaacctcaaacagacaccgccaccatgcctgctgctaagagagtgaaactggatggatccggccccgacatcgtgatgacccagagccccagcagcctgagcgccagcgtgggcgaccgcgtgaccatcacctgccgcagcagcaccggcgccgtgaccaccagcaactacgccagctgggtgcaggagaagcccggcaagctgttcaagggcctgatcggcggcaccaacaaccgcgcccccggcgtgcccagccgcttcagcggcagcctgatcggcgacaaggccaccctgaccatcagcagcctgcagcccgaggacttcgccacctacttctgcgccctgtggtacagcaaccactgggtgttcggccagggcaccaaggtggagctgaagcgcggcggcggcggcagcggcggcggcggcagcggcggcggcggcagcagcggcggcggcagcgaggtgaagctgctggagagcggcggcggcctggtgcagcccggcggcagcctgaagctgagctgcgccgtgagcggcttcagcctgaccgactacggcgtgaactgggtgcgccaggcccccggccgcggcctggagtggatcggcgtgatctggggcgacggcatcaccgactacaacagcgccctgaaggaccgcttcatcatcagcaaggacaacggcaagaacaccgtgtacctgcagatgagcaaggtgcgcagcgacgacaccgccctgtactactgcgtgaccggcctgttcgactactggggccagggcaccctggtgaccgtgagcagctacccatacgatgttccagattacgctggtggaggcggaggttctgggggaggaggtagtggcggtggtggttcaggaggcggcggaagcttggatccaggtggaggtggaagcggtatgaacaattcccagggaagagtgaccttcgaggacgtgaccgtgaacttcacccaaggcgagtggcagagactgaaccccgagcagagaaacctgtaccgggacgtgatgctggaaaactacagcaacctggtgtccgtcggccagggcgagacaacaaagcctgacgtgatcctgcggctggaacagggcaaagagccttggctggaagaggaagaggtgctcggatctggcagagccgagaagaatggcgatatcggcggacagatctggaagccaaaggatgtgaaagagagtctcggaagcggagctactaacttcagcctgctgaagcaggctggagacgtggaggagaaccctggacctatgcctgctgctaagagagtgaaactggatggatccaaccatgaccaggaatttgaccccccaaaggtttacccacctgtgccagctgagaagaggaagcccatccgcgtgctgtctctctttgatgggattgctacagggctcctggtgctgaaggacctgggcatccaagtggaccgctacattgcctccgaggtgtgtgaggactccatcacggtgggcatggtgcggcaccagggaaagatcatgtacgtcggggacgtccgcagcgtcacacagaagcatatccaggagtggggcccattcgacctggtgattggaggcagtccctgcaatgacctctccattgtcaaccctgcccgcaagggactttatgagggtactggccgcctcttctttgagttctaccgcctcctgcatgatgcgcggcccaaggagggagatgatcgccccttcttctggctctttgagaatgtggtggccatgggcgttagtgacaagagggacatctcgcgatttcttgagtctaaccccgtgatgattgacgccaaagaagtgtctgctgcacacagggcccgttacttctggggtaaccttcctggcatgaacaggcctttggcatccactgtgaatgataagctggagctgcaagagtgtctggagcacggcagaatagccaagttcagcaaagtgaggaccattaccaccaggtcaaactctataaagcagggcaaagaccagcatttccccgtgttcatgaacgagaaggaggacatcctgtggtgcactgaaatggaaagggtgtttggcttccccgtccactacacagacgtctccaacatgagccgcttggcgaggcagagactgctgggccgatcgtggagcgtgccggtcatccgccacctcttcgctccgctgaaggaatattttgcttgtgtgtctagcggcaatagtaacgctaacagccgcgggccgagcttcagcagcggcctggtgccgttaagcttgcgcggcagccatatgttcgaaaccgtgcctgtgtggaggagacagccagtccgggtgctgtccctttttgaagacatcaagaaagagctgacgagtttgggctttttggaaagtggttctgacccgggacaactgaagcatgtggttgatgtcacagacacagtgaggaaggatgtggaggagtggggacccttcgatcttgtgtacggcgccacacctcccctgggccacacctgtgaccgtcctcccagctggtacctgttccagttccaccggctcctgcagtacgcacggcccaagccaggcagccccaggcccttcttctggatgttcgtggacaatctggtgctgaacaaggaagacctggacgtcgcatctcgcttcctggagatggagccagtcaccatcccagatgtccacggcggatccttgcagaatgctgtccgcgtgtggagcaacatcccagccataaggagcagcaggcactgggctctggtttcggaagaagaattgtccctgctggcccagaacaagcagagctcgaagctcgcggccaagtggcccaccaagctggtgaagaactgctttctccccctaagagaatatttcaagtatttttcaggagggccgagctctggcgcacccccaccaagtggagggtctcctgccgggtccccaacatctactgaagaaggcaccagcgaatccgcaacgcccgagtcaggccctggtacctccacagaaccatctgaaggtagtgcgcctggttccccagctggaagccctacttccaccgaagaaggcacgtcaaccgaaccaagtgaaggatctgcccctgggaccagcactgaaccatctgagccaaaaaagaagagaaaggtaatggacaagaagtacagcatcggcctggccatcggcaccaactctgtgggctgggccgtgatcaccgacgagtacaaggtgcccagcaagaaattcaaggtgctgggcaacaccgaccggcacagcatcaagaagaacctgatcggcgccctgctgttcgacagcggagaaacagccgaggccacccggctgaagagaaccgccagaagaagatacaccagacggaagaaccggatctgctatctgcaagagatcttcagcaacgagatggccaaggtggacgacagcttcttccacagactggaagagtccttcctggtggaagaggataagaagcacgagcggcaccccatcttcggcaacatcgtggacgaggtggcctaccacgagaagtaccccaccatctaccacctgagaaagaaactggtggacagcaccgacaaggccgacctgcggctgatctatctggccctggcccacatgatcaagttccggggccacttcctgatcgagggcgacctgaaccccgacaacagcgacgtggacaagctgttcatccagctggtgcagacctacaaccagctgttcgaggaaaaccccatcaacgccagcggcgtggacgccaaggccatcctgtctgccagactgagcaagagcagacggctggaaaatctgatcgcccagctgcccggcgagaagaagaatggcctgttcggcaacctgattgccctgagcctgggcctgacccccaacttcaagagcaacttcgacctggccgaggatgccaaactgcagctgagcaaggacacctacgacgacgacctggacaacctgctggcccagatcggcgaccagtacgccgacctgtttctggccgccaagaacctgtccgacgccatcctgctgagcgacatcctgagagtgaacaccgagatcaccaaggcccccctgagcgcctctatgatcaagagatacgacgagcaccaccaggacctgaccctgctgaaagctctcgtgcggcagcagctgcctgagaagtacaaagagattttcttcgaccagagcaagaacggctacgccggctacatcgatggcggagccagccaggaagagttctacaagttcatcaagcccatcctggaaaagatggacggcaccgaggaactgctcgtgaagctgaacagagaggacctgctgcggaagcagcggaccttcgacaacggcagcatcccccaccagatccacctgggagagctgcacgccattctgcggcggcaggaagatttttacccattcctgaaggacaaccgggaaaagatcgagaagatcctgaccttccgcatcccctactacgtgggccctctggccaggggaaacagcagattcgcctggatgaccagaaagagcgaggaaaccatcaccccctggaacttcgaggaagtggtggacaagggcgccagcgcccagagcttcatcgagcggatgaccaacttcgataagaacctgcccaacgagaaggtgctgcccaagcacagcctgctgtacgagtacttcaccgtgtacaacgagctgaccaaagtgaaatacgtgaccgagggaatgagaaagcccgccttcctgagcggcgagcagaaaaaagccatcgtggacctgctgttcaagaccaaccggaaagtgaccgtgaagcagctgaaagaggactacttcaagaaaatcgagtgcttcgactccgtggaaatctccggcgtggaagatcggttcaacgcctccctgggcacataccacgatctgctgaaaattatcaaggacaaggacttcctggacaatgaggaaaacgaggacattctggaagatatcgtgctgaccctgacactgtttgaggacagagagatgatcgaggaacggctgaaaacctatgcccacctgttcgacgacaaagtgatgaagcagctgaagcggcggagatacaccggctggggcaggctgagccggaagctgatcaacggcatccgggacaagcagtccggcaagacaatcctggatttcctgaagtccgacggcttcgccaacagaaacttcatgcagctgatccacgacgacagcctgacctttaaagaggacatccagaaagcccaggtgtccggccagggcgatagcctgcacgagcacattgccaatctggccggcagccccgccattaagaagggcatcctgcagacagtgaaggtggtggacgagctcgtgaaagtgatgggccggcacaagcccgagaacatcgtgatcgaaatggccagagagaaccagaccacccagaagggacagaagaacagccgcgagagaatgaagcggatcgaagagggcatcaaagagctgggcagccagatcctgaaagaacaccccgtggaaaacacccagctgcagaacgagaagctgtacctgtactacctgcagaatgggcgggatatgtacgtggaccaggaactggacatcaaccggctgtccgactacgatgtggacgctatcgtgcctcagagctttctgaaggacgactccatcgataacaaagtgctgactcggagcgacaagaaccggggcaagagcgacaacgtgccctccgaagaggtcgtgaagaagatgaagaactactggcgccagctgctgaatgccaagctgattacccagaggaagttcgacaatctgaccaaggccgagagaggcggcctgagcgaactggataaggccggcttcatcaagagacagctggtggaaacccggcagatcacaaagcacgtggcacagatcctggactcccggatgaacactaagtacgacgagaacgacaaactgatccgggaagtgaaagtgatcaccctgaagtccaagctggtgtccgatttccggaaggatttccagttttacaaagtgcgcgagatcaacaactaccaccacgcccacgacgcctacctgaacgccgtcgtgggaaccgccctgatcaaaaagtaccctaagctggaaagcgagttcgtgtacggcgactacaaggtgtacgacgtgcggaagatgatcgccaagagcgagcaggaaatcggcaaggctaccgccaagtacttcttctacagcaacatcatgaactttttcaagaccgagattaccctggccaacggcgagatccggaagcggcctctgatcgagacaaacggcgaaacaggcgagatcgtgtgggataagggccgggactttgccaccgtgcggaaagtgctgtctatgccccaagtgaatatcgtgaaaaagaccgaggtgcagacaggcggcttcagcaaagagtctatcctgcccaagaggaacagcgacaagctgatcgccagaaagaaggactgggaccctaagaagtacggcggcttcgacagccccaccgtggcctattctgtgctggtggtggccaaagtggaaaagggcaagtccaagaaactgaagagtgtgaaagagctgctggggatcaccatcatggaaagaagcagcttcgagaagaatcccatcgactttctggaagccaagggctacaaagaagtgaaaaaggacctgatcatcaagctgcctaagtactccctgttcgagctggaaaacggccggaagagaatgctggcctctgccggcgaactgcagaagggaaacgaactggccctgccctccaaatatgtgaacttcctgtacctggccagccactatgagaagctgaagggctcccccgaggataatgagcagaaacagctgtttgtggaacagcacaaacactacctggacgagatcatcgagcagatcagcgagttctccaagagagtgatcctggccgacgctaatctggacaaggtgctgagcgcctacaacaagcacagagacaagcctatcagagagcaggccgagaatatcatccacctgtttaccctgaccaatctgggagcccctgccgccttcaagtactttgacaccaccatcgaccggaagaggtacaccagcaccaaagaggtgctggacgccaccctgatccaccagagcatcaccggcctgtacgagacacggatcgacctgtctcagctgggaggcgacgcctatccctatgacgtgcccgattatgccagcctgggcagcggctcccccaagaaaaaacgcaaggtggaagatcctaagaaaaagcggaaagtggacggcattggtagtgggagcaacggcagcagcggagaggaactgctgagcaagaactaccacctggaaaacgaggtggccagactgaagaaaggctctggctctggcggaagcggttctggcggatcaggatctggaagtggcggctctggaagcggaggttctggatctggcgaagaactgctgtctaagaattatcacctcgagaatgaagtcgctcgtttgaagaaaggttcaggctccggccagcggggaagcaagcgcaccgccgatggttccgagttcgaaagccccaaaaaaaagcgcaaggtctgagatcccaagcacgcagcaatgcagctcaaaacgcttagcctagccacacccccacgggaaacagcagtgattaacctttagcaataaacgaaagtttaactaagctatactaaccccagggttggtcaatttcgtgccagccacaccctggtactgcatgcacgcaatgctagctgcccctttcccgtcctgggcaccccgagtctcccccgaccccgggtcccaggtatgctcccacctccacctgccccactcaccacctctgctagttccagacacctccgagacgaggaaaaaaaaaaaaaaaaaaaaaaaaaaaaaaaaaaaaaaaaaaaaaaaaaaaaaaaaaaaaaaaaaaaaaaaaaaaaaaaaaaaaaaaaaaaaaaaaaaaaaaaaaaaaaaaaaaaaaaaaaaaaaaaaaaaaaaaaaaaaaaaaaaaaaaaaaaaaaaaaaaaaaaaaaaaaaaaaaaaaaaaaaaaaaaaaaaaaaaaaaaaaaaaaaaaaaaaaaaaaaaaaaaaaaaaaaaaaaaaaaaaaaaaaaaaaaaaaaaaaaaaaaaaaaaaaaaaaaaaaaaaaaaaaaaaaaaaaaaaaaaaaaaaaaaaaaaaaaaaaaaaaaaaaaaaaaaaaaaaaaaaaaaaaaaaaaaaaaaaaaaaaaaaaaaaaaaaaaaaaaaaaaaaaaaaaaaccgtcttcaagctttctagaaattcactggccgtcgttttacaacgtcgtgactgggaaaaccctggcgttacccaacttaatcgccttgcagcacatccccctttcgccagctggcgtaatagcgaagaggcccgcaccgatcgcccttcccaacagttgcgcagcctgaatggcgaatggcgcctgatgcggtattttctccttacgcatctgtgcggtatttcacaccgcatatggtgcactctcagtacaatctgctctgatgccgcatagttaagccagccccgacacccgccaacacccgctgacgcgccctgacgggcttgtctgctcccggcatccgcttacagacaagctgtgaccgtctccgggagctgcatgtgtcagaggttttcaccgtcatcaccgaaacgcgcgagacgaaagggcctcgtgatacgcctatttttataggttaatgtcatgataataatggtttcttagacgtcaggtggcacttttcggggaaatgtgcgcggaacccctatttgtttatttttctaaatacattcaaatatgtatccgctcatgagacaataaccctgataaatgcttcaataatattgaaaaaggaagagtatgagtattcaacatttccgtgtcgcccttattcccttttttgcggcattttgccttcctgtttttgctcacccagaaacgctggtgaaagtaaaagatgctgaagatcagttgggtgcacgagtgggttacatcgaactggatctcaacagcggtaagatccttgagagttttcgccccgaagaacgttttccaatgatgagcacttttaaagttctgctatgtggcgcggtattatcccgtattgacgccgggcaagagcaactcggtcgccgcatacactattctcagaatgacttggttgagtactcaccagtcacagaaaagcatcttacggatggcatgacagtaagagaattatgcagtgctgccataaccatgagtgataacactgcggccaacttacttctgacaacgatcggaggaccgaaggagctaaccgcttttttgcacaacatgggggatcatgtaactcgccttgatcgttgggaaccggagctgaatgaagccataccaaacgacgagcgtgacaccacgatgcctgtagcaatggcaacaacgttgcgcaaactattaactggcgaactacttactctagcttcccggcaacaattaatagactggatggaggcggataaagttgcaggaccacttctgcgctcggcccttccggctggctggtttattgctgataaatctggagccggtgagcgtgggtctcgcggtatcattgcagcactggggccagatggtaagccctcccgtatcgtagttatctacacgacggggagtcaggcaactatggatgaacgaaatagacagatcgctgagataggtgcctcactgattaagcattggtaactgtcagaccaagtttac

SEQ ID NO: 211 - DNA, 12234 bp, synthetic construct
  misc_feature 1..12234: note = DNA of V17_scFv-ZIM3-2a-D3a-hD3L-dCas9-10xGCN4
  source 1..12234: mol_type = other DNA
tcatatatactttagattgatttaaaacttcatttttaatttaaaaggatctaggtgaagatcctttttgataatctcatgaccaaaatcccttaacgtgagttttcgttccactgagcgtcagaccccgtagaaaagatcaaaggatcttcttgagatcctttttttctgcgcgtaatctgctgcttgcaaacaaaaaaaccaccgctaccagcggtggtttgtttgccggatcaagagctaccaactctttttccgaaggtaactggcttcagcagagcgcagataccaaatactgttcttctagtgtagccgtagttaggccaccacttcaagaactctgtagcaccgcctacatacctcgctctgctaatcctgttaccagtggctgctgccagtggcgataagtcgtgtcttaccgggttggactcaagacgatagttaccggataaggcgcagcggtcgggctgaacggggggttcgtgcacacagcccagcttggagcgaacgacctacaccgaactgagatacctacagcgtgagctatgagaaagcgccacgcttcccgaagggagaaaggcggacaggtatccggtaagcggcagggtcggaacaggagagcgcacgagggagcttccagggggaaacgcctggtatctttatagtcctgtcgggtttcgccacctctgacttgagcgtcgatttttgtgatgctcgtcaggggggcggagcctatggaaaaacgccagcaacgcggcctttttacggttcctggccttttgctggccttttgctcacatgttctttcctgcgttatcccctgattctgtggataaccgtattaccgcctttgagtgagctgataccgctcgccgcagccgaacgaccgagcgcagcgagtcagtgagcgaggaagcggaagagcgcccaatacgcaaaccgcctctccccgcgcgttggccgattcattaatgcagctggcacgacaggtttcccgactggaaagcgggcagtgagcgcaacgcaattaatgtgagttagctcactcattaggcaccccaggctttacactttatgcttccggctcgtatgttgtgtggaattgtgagcggataacaatttcacacaggaaacagctatgaccatgattacgcctctagaaagctttaatacgactcactataaggactcactatttgttttcgcgcccagttgcaaaaagtgtcgacatttgcttctgacacaactgtgttcactagcaacctcaaacagacaccgccaccatgcctgctgctaagagagtgaaactggatggatccggccccgacatcgtgatgacccagagccccagcagcctgagcgccagcgtgggcgaccgcgtgaccatcacctgccgcagcagcaccggcgccgtgaccaccagcaactacgccagctgggtgcaggagaagcccggcaagctgttcaagggcctgatcggcggcaccaacaaccgcgcccccggcgtgcccagccgcttcagcggcagcctgatcggcgacaaggccaccctgaccatcagcagcctgcagcccgaggacttcgccacctacttctgcgccctgtggtacagcaaccactgggtgttcggccagggcaccaaggtggagctgaagcgcggcggcggcggcagcggcggcggcggcagcggcggcggcggcagcagcggcggcggcagcgaggtgaagctgctggagagcggcggcggcctggtgcagcccggcggcagcctgaagctgagctgcgccgtgagcggcttcagcctgaccgactacggcgtgaactgggtgcgccaggcccccggccgcggcctggagtggatcggcgtgatctggggcgacggcatcaccgactacaacagcgccctgaaggaccgcttcatcatcagcaaggacaacggcaagaacaccgtgtacctgcagatgagcaaggtgcgcagcgacgacaccgccctgtactactgcgtgaccggcctgttcgactactggggccagggcaccctggtgaccgtgagcagctacccatacgatgttccagattacgctggtggaggcggaggttctgggggaggaggtagtggcggtggtggttcaggaggcggcggaagcttggatccaggtggaggtggaagcggtatgaacaattcccagggaagagtgaccttcgaggacgtgaccgtgaacttcacccaaggcgagtggcagagactgaaccccgagcagagaaacctgtaccgggacgtgatgctggaaaactacagcaacctggtgtccgtcggccagggcgagacaacaaagcctgacgtgatcctgcggctggaacagggcaaagagccttggctggaagaggaagaggtgctcggatctggcagagccgagaagaatggcgatatcggcggacagatctggaagccaaaggatgtgaaagagagtctcggaagcggagctactaacttcagcctgctgaagcaggctggagacgtggaggagaaccctggacctatgcctgctgctaagagagtgaaactggatggatccaaccatgaccaggaatttgaccccccaaaggtttacccacctgtgccagctgagaagaggaagcccatccgcgtgctgtctctctttgatgggattgctacagggctcctggtgctgaaggacctgggcatccaagtggaccgctacattgcctccgaggtgtgtgaggactccatcacggtgggcatggtgcggcaccagggaaagatcatgtacgtcggggacgtccgcagcgtcacacagaagcatatccaggagtggggcccattcgacctggtgattggaggcagtccctgcaatgacctctccattgtcaaccctgcccgcaagggactttatgagggtactggccgcctcttctttgagttctaccgcctcctgcatgatgcgcggcccaaggagggagatgatcgccccttcttctggctctttgagaatgtggtggccatgggcgttagtgacaagagggacatctcgcgatttcttgagtctaaccccgtgatgattgacgccaaagaagtgtctgctgcacacagggcccgttacttctggggtaaccttcctggcatgaacaggcctttggcatccactgtgaatgataagctggagctgcaagagtgtctggagcacggcagaatagccaagttcagcaaagtgaggaccattaccaccaggtcaaactctataaagcagggcaaagaccagcatttccccgtgttcatgaacgagaaggaggacatcctgtggtgcactgaaatggaaagggtgtttggcttccccgtccactacacagacgtctccaacatgagccgcttggcgaggcagagactgctgggccgatcgtggagcgtgccggtcatccgccacctcttcgctccgctgaaggaatattttgcttgtgtgtctagcggcaatagtaacgctaacagccgcgggccgagcttcagcagcggcctggtgccgttaagcttgcgcggcagccatatgttcgaaaccgtgcctgtgtggaggagacagccagtccgggtgctgtccctttttgaagacatcaagaaagagctgacgagtttgggctttttggaaagtggttctgacccgggacaactgaagcatgtggttgatgtcacagacacagtgaggaaggatgtggaggagtggggacccttcgatcttgtgtacggcgccacacctcccctgggccacacctgtgaccgtcctcccagctggtacctgttccagttccaccggctcctgcagtacgcacggcccaagccaggcagccccaggcccttcttctggatgttcgtggacaatctggtgctgaacaaggaagacctggacgtcgcatctcgcttcctggagatggagccagtcaccatcccagatgtccacggcggatccttgcagaatgctgtccgcgtgtggagcaacatcccagccataaggagcagcaggcactgggctctggtttcggaagaagaattgtccctgctggcccagaacaagcagagctcgaagctcgcggccaagtggcccaccaagctggtgaagaactgctttctccccctaagagaatatttcaagtatttttcaggagggccgagctctggcgcacccccaccaagtggagggtctcctgccgggtccccaacatctactgaagaaggcaccagcgaatccgcaacgcccgagtcaggccctggtacctccacagaaccatctgaaggtagtgcgcctggttccccagctggaagccctacttccaccgaagaaggcacgtcaaccgaaccaagtgaaggatctgcccctgggaccagcactgaaccatctgagccaaaaaagaagagaaaggtaatggacaagaagtacagcatcggcctggccatcggcaccaactctgtgggctgggccgtgatcaccgacgagtacaaggtgcccagcaagaaattcaaggtgctgggcaacaccgaccggcacagcatcaagaagaacctgatcggcgccctgctgttcgacagcggagaaacagccgaggccacccggctgaagagaaccgccagaagaagatacaccagacggaagaaccggatctgctatctgcaagagatcttcagcaacgagatggccaaggtggacgacagcttcttccacagactggaagagtccttcctggtggaagaggataagaagcacgagcggcaccccatcttcggcaacatcgtggacgaggtggcctaccacgagaagtaccccaccatctaccacctgagaaagaaactggtggacagcaccgacaaggccgacctgcggctgatctatctggccctggcccacatgatcaagttccggggccacttcctgatcgagggcgacctgaaccccgacaacagcgacgtggacaagctgttcatccagctggtgcagacctacaaccagctgttcgaggaaaaccccatcaacgccagcggcgtggacgccaaggccatcctgtctgccagactgagcaagagcagacggctggaaaatctgatcgcccagctgcccggcgagaagaagaatggcctgttcggcaacctgattgccctgagcctgggcctgacccccaacttcaagagcaacttcgacctggccgaggatgccaaactgcagctgagcaaggacacctacgacgacgacctggacaacctgctggcccagatcggcgaccagtacgccgacctgtttctggccgccaagaacctgtccgacgccatcctgctgagcgacatcctgagagtgaacaccgagatcaccaaggcccccctgagcgcctctatgatcaagagatacgacgagcaccaccaggacctgaccctgctgaaagctctcgtgcggcagcagctgcctgagaagtacaaagagattttcttcgaccagagcaagaacggctacgccggctacatcgatggcggagccagccaggaagagttctacaagttcatcaagcccatcctggaaaagatggacggcaccgaggaactgctcgtgaagctgaacagagaggacctgctgcggaagcagcggaccttcgacaacggcagcatcccccaccagatccacctgggagagctgcacgccattctgcggcggcaggaagatttttacccattcctgaaggacaaccgggaaaagatcgagaagatcctgaccttccgcatcccctactacgtgggccctctggccaggggaaacagcagattcgcctggatgaccagaaagagcgaggaaaccatcaccccctggaacttcgaggaagtggtggacaagggcgccagcgcccagagcttcatcgagcggatgaccaacttcgataagaacctgcccaacgagaaggtgctgcccaagcacagcctgctgtacgagtacttcaccgtgtacaacgagctgaccaaagtgaaatacgtgaccgagggaatgagaaagcccgccttcctgagcggcgagcagaaaaaagccatcgtggacctgctgttcaagaccaaccggaaagtgaccgtgaagcagctgaaagaggactacttcaagaaaatcgagtgcttcgactccgtggaaatctccggcgtggaagatcggttcaacgcctccctgggcacataccacgatctgctgaaaattatcaaggacaaggacttcctggacaatgaggaaaacgaggacattctggaagatatcgtgctgaccctgacactgtttgaggacagagagatgatcgaggaacggctgaaaacctatgcccacctgttcgacgacaaagtgatgaagcagctgaagcggcggagatacaccggctggggcaggctgagccggaagctgatcaacggcatccgggacaagcagtccggcaagacaatcctggatttcctgaagtccgacggcttcgccaacagaaacttcatgcagctgatccacgacgacagcctgacctttaaagaggacatccagaaagcccaggtgtccggccagggcgatagcctgcacgagcacattgccaatctggccggcagccccgccattaagaagggcatcctgcagacagtgaaggtggtggacgagctcgtgaaagtgatgggccggcacaagcccgagaacatcgtgatcgaaatggccagagagaaccagaccacccagaagggacagaagaacagccgcgagagaatgaagcggatcgaagagggcatcaaagagctgggcagccagatcctgaaagaacaccccgtggaaaacacccagctgcagaacgagaagctgtacctgtactacctgcagaatgggcgggatatgtacgtggaccaggaactggacatcaaccggctgtccgactacgatgtggacgctatcgtgcctcagagctttctgaaggacgactccatcgataacaaagtgctgactcggagcgacaagaaccggggcaagagcgacaacgtgccctccgaagaggtcgtgaagaagatgaagaactactggcgccagctgctgaatgccaagctgattacccagaggaagttcgacaatctgaccaaggccgagagaggcggcctgagcgaactggataaggccggcttcatcaagagacagctggtggaaacccggcagatcacaaagcacgtggcacagatcctggactcccggatgaacactaagtacgacgagaacgacaaactgatccgggaagtgaaagtgatcaccctgaagtccaagctggtgtccgatttccggaaggatttccagttttacaaagtgcgcgagatcaacaactaccaccacgcccacgacgcctacctgaacgccgtcgtgggaaccgccctgatcaaaaagtaccctaagctggaaagcgagttcgtgtacggcgactacaaggtgtacgacgtgcggaagatgatcgccaagagcgagcaggaaatcggcaaggctaccgccaagtacttcttctacagcaacatcatgaactttttcaagaccgagattaccctggccaacggcgagatccggaagcggcctctgatcgagacaaacggcgaaacaggcgagatcgtgtgggataagggccgggactttgccaccgtgcggaaagtgctgtctatgccccaagtgaatatcgtgaaaaagaccgaggtgcagacaggcggcttcagcaaagagtctatcctgcccaagaggaacagcgacaagctgatcgccagaaagaaggactgggaccctaagaagtacggcggcttcgacagccccaccgtggcctattctgtgctggtggtggccaaagtggaaaagggcaagtccaagaaactgaagagtgtgaaagagctgctggggatcaccatcatggaaagaagcagcttcgagaagaatcccatcgactttctggaagccaagggctacaaagaagtgaaaaaggacctgatcatcaagctgcctaagtactccctgttcgagctggaaaacggccggaagagaatgctggcctctgccggcgaactgcagaagggaaacgaactggccctgccctccaaatatgtgaacttcctgtacctggccagccactatgagaagctgaagggctcccccgaggataatgagcagaaacagctgtttgtggaacagcacaaacactacctggacgagatcatcgagcagatcagcgagttctccaagagagtgatcctggccgacgctaatctggacaaggtgctgagcgcctacaacaagcacagagacaagcctatcagagagcaggccgagaatatcatccacctgtttaccctgaccaatctgggagcccctgccgccttcaagtactttgacaccaccatcgaccggaagaggtacaccagcaccaaagaggtgctggacgccaccctgatccaccagagcatcaccggcctgtacgagacacggatcgacctgtctcagctgggaggcgacgcctatccctatgacgtgcccgattatgccagcctgggcagcggctcccccaagaaaaaacgcaaggtggaagatcctaagaaaaagcggaaagtggacggcattggtagtgggagcaacggcagcagcggagaggaactgctgagcaagaactaccacctggaaaacgaggtggccagactgaagaaaggctctggctctggcggaagcggttctggcggatcaggatctggaagtggcggctctggaagcggaggttctggatctggcgaagaactgctgtctaagaattatcacctcgagaacgaagtggctcggctcaagaaaggcagtggcagcggaggaagtggatccggcggtagtggtagtggaagcggcggatccggctcaggcggatctggttcaggggaagaactcctctccaaaaactaccatctcgagaatgaggtcgcccgcctgaaaaaaggatcaggttccggtggttctggcagcggtggttcaggctcaggcagcggcggtagcggtagcggtggaagcggaagcggagaagaacttctcagcaaaaattaccacttggagaatgaagttgcaagactcaaaaaaggttccggcagtggcggcagcggcagcggcggatctggtagtggatctggtggcagtggttcaggcggaagtggtagcggagaggaattgctctcaaagaactatcatttggagaacgaggttgcacgcttgaagaaaggcagcggatcaggcggatctggcagcggtggatctggttctggatccggcggctccggtagtggtggaagtggctctggggaagaattgcttagcaagaattatcatcttgaaaatgaggttgccaggcttaaaaaaggcagtggctccggcggatccggaagcggaggcagcggatctggatctggtggttcaggatctggcggttctggtagcggggaagaactgttgagtaaaaactatcaccttgagaacgaggtcgcaaggttgaaaaaaggatccggctctggcggctccggaagtggcggatctggctccggtagcggaggatcaggatccggcggaagcggatcaggcgaggaactgctttccaaaaattaccaccttgaaaacgaagtcgcccgcctcaagaaaggttctggcagcggaggctctggcagtggtggtagcggaagtggaagtggtggcagtggtagcggtggatctggaagcggcgaggaactcctgtcaaagaattaccatctcgaaaacgaggtcgcaaggctcaagaaaggctcaggatcaggcggctctggatccggcggttctggttccggctcaggtggaagtggatctggcggctcaggttccggcgaagaattgctttccaagaactaccatttggaaaatgaagtcgctcgtttgaagaaaggttcaggctccggccagcggggaagcaagcgcaccgccgatggttccgagttcgaaagccccaaaaaaaagcgcaaggtctgagatcccaagcacgcagcaatgcagctcaaaacgcttagcctagccacacccccacgggaaacagcagtgattaacctttagcaataaacgaaagtttaactaagctatactaaccccagggttggtcaatttcgtgccagccacaccctggtactgcatgcacgcaatgctagctgcccctttcccgtcctgggcaccccgagtctcccccgaccccgggtcccaggtatgctcccacctccacctgccccactcaccacctctgctagttccagacacctccgagacgaggaaaaaaaaaaaaaaaaaaaaaaaaaaaaaaaaaaaaaaaaaaaaaaaaaaaaaaaaaaaaaaaaaaaaaaaaaaaaaaaaaaaaaaaaaaaaaaaaaaaaaaaaaaaaaaaaaaaaaaaaaaaaaaaaaaaaaaaaaaaaaaaaaaaaaaaaaaaaaaaaaaaaaaaaaaaaaaaaaaaaaaaaaaaaaaaaaaaaaaaaaaaaaaaaaaaaaaaaaaaaaaaaaaaaaaaaaaaaaaaaaaaaaaaaaaaaaaaaaaaaaaaaaaaaaaaaaaaaaaaaaaaaaaaaaaaaaaaaaaaaaaaaaaaaaaaaaaaaaaaaaaaaaaaaaaaaaaaaaaaaaaaaaaaaaaaaaaaaaaaaaaaaaaaaaaaaaaaaaaaaaaaaaaaaaaaaaaccgtcttcaagctttctagaaattcactggccgtcgttttacaacgtcgtgactgggaaaaccctggcgttacccaacttaatcgccttgcagcacatccccctttcgccagctggcgtaatagcgaagaggcccgcaccgatcgcccttcccaacagttgcgcagcctgaatggcgaatggcgcctgatgcggtattttctccttacgcatctgtgcggtatttcacaccgcatatggtgcactctcagtacaatctgctctgatgccgcatagttaagccagccccgacacccgccaacacccgctgacgcgccctgacgggcttgtctgctcccggcatccgcttacagacaagctgtgaccgtctccgggagctgcatgtgtcagaggttttcaccgtcatcaccgaaacgcgcgagacgaaagggcctcgtgatacgcctatttttataggttaatgtcatgataataatggtttcttagacgtcaggtggcacttttcggggaaatgtgcgcggaacccctatttgtttatttttctaaatacattcaaatatgtatccgctcatgagacaataaccctgataaatgcttcaataatattgaaaaaggaagagtatgagtattcaacatttccgtgtcgcccttattcccttttttgcggcattttgccttcctgtttttgctcacccagaaacgctggtgaaagtaaaagatgctgaagatcagttgggtgcacgagtgggttacatcgaactggatctcaacagcggtaagatccttgagagttttcgccccgaagaacgttttccaatgatgagcacttttaaagttctgctatgtggcgcggtattatcccgtattgacgccgggcaagagcaactcggtcgccgcatacactattctcagaatgacttggttgagtactcaccagtcacagaaaagcatcttacggatggcatgacagtaagagaattatgcagtgctgccataaccatgagtgataacactgcggccaacttacttctgacaacgatcggaggaccgaaggagctaaccgcttttttgcacaacatgggggatcatgtaactcgccttgatcgttgggaaccggagctgaatgaagccataccaaacgacgagcgtgacaccacgatgcctgtagcaatggcaacaacgttgcgcaaactattaactggcgaactacttactctagcttcccggcaacaattaatagactggatggaggcggataaagttgcaggaccacttctgcgctcggcccttccggctggctggtttattgctgataaatctggagccggtgagcgtgggtctcgcggtatcattgcagcactggggccagatggtaagccctcccgtatcgtagttatctacacgacggggagtcaggcaactatggatgaacgaaatagacagatcgctgagataggtgcctcactgattaagcattggtaactgtcagaccaagtttac

SEQ ID NO: 212 - DNA, 10680 bp, synthetic construct
  misc_feature 1..10680: note = DNA of V18_scFv-ZIM3-2a-D3a-hD3L-dCas12a-1xGCN4
  source 1..10680: mol_type = other DNA
tcatatatactttagattgatttaaaacttcatttttaatttaaaaggatctaggtgaagatcctttttgataatctcatgaccaaaatcccttaacgtgagttttcgttccactgagcgtcagaccccgtagaaaagatcaaaggatcttcttgagatcctttttttctgcgcgtaatctgctgcttgcaaacaaaaaaaccaccgctaccagcggtggtttgtttgccggatcaagagctaccaactctttttccgaaggtaactggcttcagcagagcgcagataccaaatactgttcttctagtgtagccgtagttaggccaccacttcaagaactctgtagcaccgcctacatacctcgctctgctaatcctgttaccagtggctgctgccagtggcgataagtcgtgtcttaccgggttggactcaagacgatagttaccggataaggcgcagcggtcgggctgaacggggggttcgtgcacacagcccagcttggagcgaacgacctacaccgaactgagatacctacagcgtgagctatgagaaagcgccacgcttcccgaagggagaaaggcggacaggtatccggtaagcggcagggtcggaacaggagagcgcacgagggagcttccagggggaaacgcctggtatctttatagtcctgtcgggtttcgccacctctgacttgagcgtcgatttttgtgatgctcgtcaggggggcggagcctatggaaaaacgccagcaacgcggcctttttacggttcctggccttttgctggccttttgctcacatgttctttcctgcgttatcccctgattctgtggataaccgtattaccgcctttgagtgagctgataccgctcgccgcagccgaacgaccgagcgcagcgagtcagtgagcgaggaagcggaagagcgcccaatacgcaaaccgcctctccccgcgcgttggccgattcattaatgcagctggcacgacaggtttcccgactggaaagcgggcagtgagcgcaacgcaattaatgtgagttagctcactcattaggcaccccaggctttacactttatgcttccggctcgtatgttgtgtggaattgtgagcggataacaatttcacacaggaaacagctatgaccatgattacgcctctagaaagctttaatacgactcactataaggactcactatttgttttcgcgcccagttgcaaaaagtgtcgacatttgcttctgacacaactgtgttcactagcaacctcaaacagacaccgccaccatgcctgctgctaagagagtgaaactggatggatccggccccgacatcgtgatgacccagagccccagcagcctgagcgccagcgtgggcgaccgcgtgaccatcacctgccgcagcagcaccggcgccgtgaccaccagcaactacgccagctgggtgcaggagaagcccggcaagctgttcaagggcctgatcggcggcaccaacaaccgcgcccccggcgtgcccagccgcttcagcggcagcctgatcggcgacaaggccaccctgaccatcagcagcctgcagcccgaggacttcgccacctacttctgcgccctgtggtacagcaaccactgggtgttcggccagggcaccaaggtggagctgaagcgcggcggcggcggcagcggcggcggcggcagcggcggcggcggcagcagcggcggcggcagcgaggtgaagctgctggagagcggcggcggcctggtgcagcccggcggcagcctgaagctgagctgcgccgtgagcggcttcagcctgaccgactacggcgtgaactgggtgcgccaggcccccggccgcggcctggagtggatcggcgtgatctggggcgacggcatcaccgactacaacagcgccctgaaggaccgcttcatcatcagcaaggacaacggcaagaacaccgtgtacctgcagatgagcaaggtgcgcagcgacgacaccgccctgtactactgcgtgaccggcctgttcgactactggggccagggcaccctggtgaccgtgagcagctacccatacgatgttccagattacgctggtggaggcggaggttctgggggaggaggtagtggcggtggtggttcaggaggcggcggaagcttggatccaggtggaggtggaagcggtatgaacaattcccagggaagagtgaccttcgaggacgtgaccgtgaacttcacccaaggcgagtggcagagactgaaccccgagcagagaaacctgtaccgggacgtgatgctggaaaactacagcaacctggtgtccgtcggccagggcgagacaacaaagcctgacgtgatcctgcggctggaacagggcaaagagccttggctggaagaggaagaggtgctcggatctggcagagccgagaagaatggcgatatcggcggacagatctggaagccaaaggatgtgaaagagagtctcggaagcggagctactaacttcagcctgctgaagcaggctggagacgtggaggagaaccctggacctatgcctgctgctaagagagtgaaactggatggatccaaccatgaccaggaatttgaccccccaaaggtttacccacctgtgccagctgagaagaggaagcccatccgcgtgctgtctctctttgatgggattgctacagggctcctggtgctgaaggacctgggcatccaagtggaccgctacattgcctccgaggtgtgtgaggactccatcacggtgggcatggtgcggcaccagggaaagatcatgtacgtcggggacgtccgcagcgtcacacagaagcatatccaggagtggggcccattcgacctggtgattggaggcagtccctgcaatgacctctccattgtcaaccctgcccgcaagggactttatgagggtactggccgcctcttctttgagttctaccgcctcctgcatgatgcgcggcccaaggagggagatgatcgccccttcttctggctctttgagaatgtggtggccatgggcgttagtgacaagagggacatctcgcgatttcttgagtctaaccccgtgatgattgacgccaaagaagtgtctgctgcacacagggcccgttacttctggggtaaccttcctggcatgaacaggcctttggcatccactgtgaatgataagctggagctgcaagagtgtctggagcacggcagaatagccaagttcagcaaagtgaggaccattaccaccaggtcaaactctataaagcagggcaaagaccagcatttccccgtgttcatgaacgagaaggaggacatcctgtggtgcactgaaatggaaagggtgtttggcttccccgtccactacacagacgtctccaacatgagccgcttggcgaggcagagactgctgggccgatcgtggagcgtgccggtcatccgccacctcttcgctccgctgaaggaatattttgcttgtgtgtctagcggcaatagtaacgctaacagccgcgggccgagcttcagcagcggcctggtgccgttaagcttgcgcggcagccatatgttcgaaaccgtgcctgtgtggaggagacagccagtccgggtgctgtccctttttgaagacatcaagaaagagctgacgagtttgggctttttggaaagtggttctgacccgggacaactgaagcatgtggttgatgtcacagacacagtgaggaaggatgtggaggagtggggacccttcgatcttgtgtacggcgccacacctcccctgggccacacctgtgaccgtcctcccagctggtacctgttccagttccaccggctcctgcagtacgcacggcccaagccaggcagccccaggcccttcttctggatgttcgtggacaatctggtgctgaacaaggaagacctggacgtcgcatctcgcttcctggagatggagccagtcaccatcccagatgtccacggcggatccttgcagaatgctgtccgcgtgtggagcaacatcccagccataaggagcagcaggcactgggctctggtttcggaagaagaattgtccctgctggcccagaacaagcagagctcgaagctcgcggccaagtggcccaccaagctggtgaagaactgctttctccccctaagagaatatttcaagtatttttcaggagggccgagctctggcgcacccccaccaagtggagggtctcctgccgggtccccaacatctactgaagaaggcaccagcgaatccgcaacgcccgagtcaggccctggtacctccacagaaccatctgaaggtagtgcgcctggttccccagctggaagccctacttccaccgaagaaggcacgtcaaccgaaccaagtgaaggatctgcccctgggaccagcactgaaccatctgagccaaaaaagaagagaaaggtaatgtcaaagctggagaaattcaccaactgttatagcctgtctaagaccctgcgcttcaaggcaatcccagtgggcaagacacaagagaacattgacaacaaacggctcctggtggaggatgagaagagggctgaagattacaagggcgttaagaagctgctggataggtactatctgtcattcatcaacgatgtcctccacagtatcaagctgaagaatctgaacaattacatttctctgttccggaagaagacacggaccgagaaggagaacaaagagctggagaatctggagatcaacctgaggaaagaaatagctaaggctttcaaagggaacgagggttacaagtccctgttcaagaaagacattatcgagactattctgcctgagttcctggacgataaagatgagatcgccctcgtcaattccttcaatgggtttaccacagcctttaccggcttcttcgacaatagagagaatatgttctctgaagaggccaaatccactagcatcgcctttcgctgcataaacgagaacctgactaggtacatcagcaatatggacatctttgagaaagtcgatgccatattcgacaaacatgaggtgcaggagattaaggagaagatcctgaactcagattacgatgtcgaagatttcttcgagggagagttcttcaacttcgtgctcacacaagagggcattgatgtgtacaatgcaatcattggagggttcgtgacagagagtggcgagaagataaagggcctgaacgagtatatcaacctctacaaccagaaaaccaagcagaaactgcctaagttcaagccactgtacaaacaagtgctctcagatagggaaagcctgagcttctacggtgaagggtatacatcagatgaagaagtgctcgaagtgttccgcaacaccctcaataagaacagtgaaatcttctcttcaatcaagaagctggagaaactgttcaagaatttcgatgagtactcctctgccggaatctttgtgaagaatggccctgcaatatccactattagcaaagacatctttggcgagtggaacgttatcagggataagtggaatgccgagtacgatgatattcatctcaagaagaaagccgtggttacagagaaatacgaggatgatagacgcaagagctttaagaagattggtagcttctctctcgaacagctgcaggagtacgccgacgctgacctgtcagtcgtggagaaactcaaggagatcataatccagaaggtggatgaaatctacaaagtgtatggaagctctgagaaactcttcgatgcagactttgttctggagaagagtctgaagaagaacgacgcagtggttgctatcatgaaggacctgctggattctgttaagtctttcgagaattacattaaggcattctttggtgaagggaaggagacaaatagggacgagagcttctatggcgactttgttctggcctacgacatcctcctcaaggttgaccacatctatgacgctatacggaattacgttacccagaagccctatagcaaagacaagttcaagctgtatttccagaatccacagtttatgggtgggtgggataaagacaaagaaacagattacagggccactatcctgcggtacggcagcaaatactatctggctatcatggataagaagtacgccaaatgcctccagaagatcgacaaggacgacgtgaacggtaactacgagaagatcaattacaagctcctgccaggacctaacaagatgctgcccaaggtgttcttctccaagaaatggatggcctactataacccaagcgaggacattcagaagatatacaagaatgggacattcaagaagggcgatatgttcaacctcaacgactgccacaagctgattgatttcttcaaggatagcatttctcgctatcccaagtggtctaatgcatacgatttcaacttcagcgagactgagaagtacaaagacatcgctggcttctaccgggaggtggaagagcaaggctataaggtgtcattcgaatccgcttctaagaaggaagtggataagctcgtggaagagggtaagctgtacatgttccagatatacaacaaagacttcagcgataagagccacggcactccaaacctccatactatgtatttcaagctgctgtttgacgagaacaaccacggacagattaggctgtcaggaggcgcagaactcttcatgcgcagagcttcactgaagaaggaggaactcgttgtccacccagccaatagccctatagccaataagaatccagacaatcctaagaaaaccactactctgtcttacgatgtgtataaggataagagattctctgaagatcagtacgaactgcacatacccattgccattaacaagtgccctaagaacatcttcaagattaacacagaggttagagtgctcctgaaacacgacgataacccttatgttataggcattgctcgcggagagagaaacctgctgtacatcgtcgtggtggacggcaaaggcaacatcgtggaacagtacagtctcaatgaaatcattaacaatttcaacggaatccgcattaagaccgactaccattctctcctcgacaagaaggagaaagaaaggttcgaagcaagacagaattggacaagtatagagaatatcaaagaactgaaggctgggtacatctctcaggttgtgcacaagatatgtgagctggtggagaagtacgacgctgttatcgccctcgcggacctgaatagcggcttcaagaactccagggtgaaggtggagaagcaggtgtatcagaagttcgagaagatgctgatcgacaagctcaactatatggtggacaagaaatccaatccttgcgctactggtggagccctgaagggctatcaaatcaccaataagttcgaatctttcaagtctatgagcacccagaatggcttcatcttctacatacccgcatggctgacatccaagattgatccctctaccggatttgttaatctgctcaagactaagtacacctctattgctgactcaaagaagttcatatcatcatttgaccgcatcatgtacgtgccagaagaggacctgttcgagtttgccctggattacaagaatttctctcggactgacgccgactacatcaagaagtggaagctctactcttatggtaatcggattcgcatattccgcaatcccaagaagaataacgtgttcgattgggaggaagtttgcctcaccagcgcttacaaggagctgttcaataagtatgggattaactaccagcagggcgacataagagccctgctgtgcgaacaatctgataaggcattctattcctctttcatggcactgatgtcactgatgctgcaaatgcgcaattccatcaccggaagaacagacgtggcctttctgatctctcctgtcaagaactcagatggcatcttctacgattcccgcaactatgaagcacaggagaatgctatcctgcctaagaatgccgatgcaaatggagcctataacatcgccagaaaggtcctctgggccataggacaattcaagaaagctgaagatgagaagctggacaaggtgaagatcgccatttcaaacaaagagtggctcgaatatgctcagacctcagtgaagcatgcctatccctatgacgtgcccgattatgccagcctgggcagcggctcccccaagaaaaaacgcaaggtggaagatcctaagaaaaagcggaaagtggacggcattggtagtgggagcaacggcagcagcggagaggaactgctgagcaagaactaccacctggaaaacgaggtggccagactgaagaaaggctctggctctggcggaagcggttctggcggatcaggatctggaagtggcggctctggaagcggaggttctggatctggcgaagaactgctgtctaagaattatcacggttcaggctccggccagcggggaagcaagcgcaccgccgatggttccgagttcgaaagccccaaaaaaaagcgcaaggtctgagatcccaagcacgcagcaatgcagctcaaaacgcttagcctagccacacccccacgggaaacagcagtgattaacctttagcaataaacgaaagtttaactaagctatactaaccccagggttggtcaatttcgtgccagccacaccctggtactgcatgcacgcaatgctagctgcccctttcccgtcctgggcaccccgagtctcccccgaccccgggtcccaggtatgctcccacctccacctgccccactcaccacctctgctagttccagacacctccgagacgaggaaaaaaaaaaaaaaaaaaaaaaaaaaaaaaaaaaaaaaaaaaaaaaaaaaaaaaaaaaaaaaaaaaaaaaaaaaaaaaaaaaaaaaaaaaaaaaaaaaaaaaaaaaaaaaaaaaaaaaaaaaaaaaaaaaaaaaaaaaaaaaaaaaaaaaaaaaaaaaaaaaaaaaaaaaaaaaaaaaaaaaaaaaaaaaaaaaaaaaaaaaaaaaaaaaaaaaaaaaaaaaaaaaaaaaaaaaaaaaaaaaaaaaaaaaaaaaaaaaaaaaaaaaaaaaaaaaaaaaaaaaaaaaaaaaaaaaaaaaaaaaaaaaaaaaaaaaaaaaaaaaaaaaaaaaaaaaaaaaaaaaaaaaaaaaaaaaaaaaaaaaaaaaaaaaaaaaaaaaaaaaaaaaaaaaaaaaccgtcttcaagctttctagaaattcactggccgtcgttttacaacgtcgtgactgggaaaaccctggcgttacccaacttaatcgccttgcagcacatccccctttcgccagctggcgtaatagcgaagaggcccgcaccgatcgcccttcccaacagttgcgcagcctgaatggcgaatggcgcctgatgcggtattttctccttacgcatctgtgcggtatttcacaccgcatatggtgcactctcagtacaatctgctctgatgccgcatagttaagccagccccgacacccgccaacacccgctgacgcgccctgacgggcttgtctgctcccggcatccgcttacagacaagctgtgaccgtctccgggagctgcatgtgtcagaggttttcaccgtcatcaccgaaacgcgcgagacgaaagggcctcgtgatacgcctatttttataggttaatgtcatgataataatggtttcttagacgtcaggtggcacttttcggggaaatgtgcgcggaacccctatttgtttatttttctaaatacattcaaatatgtatccgctcatgagacaataaccctgataaatgcttcaataatattgaaaaaggaagagtatgagtattcaacatttccgtgtcgcccttattcccttttttgcggcattttgccttcctgtttttgctcacccagaaacgctggtgaaagtaaaagatgctgaagatcagttgggtgcacgagtgggttacatcgaactggatctcaacagcggtaagatccttgagagttttcgccccgaagaacgttttccaatgatgagcacttttaaagttctgctatgtggcgcggtattatcccgtattgacgccgggcaagagcaactcggtcgccgcatacactattctcagaatgacttggttgagtactcaccagtcacagaaaagcatcttacggatggcatgacagtaagagaattatgcagtgctgccataaccatgagtgataacactgcggccaacttacttctgacaacgatcggaggaccgaaggagctaaccgcttttttgcacaacatgggggatcatgtaactcgccttgatcgttgggaaccggagctgaatgaagccataccaaacgacgagcgtgacaccacgatgcctgtagcaatggcaacaacgttgcgcaaactattaactggcgaactacttactctagcttcccggcaacaattaatagactggatggaggcggataaagttgcaggaccacttctgcgctcggcccttccggctggctggtttattgctgataaatctggagccggtgagcgtgggtctcgcggtatcattgcagcactggggccagatggtaagccctcccgtatcgtagttatctacacgacggggagtcaggcaactatggatgaacgaaatagacagatcgctgagataggtgcctcactgattaagcattggtaactgtcagaccaagtttac

SEQ ID NO: 213 - DNA, 9729 bp, synthetic construct
  misc_feature 1..9729: note = DNA of V19_scFv-ZIM3-2a-D3a-hD3L-dCas12i-1xGCN4
  source 1..9729: mol_type = other DNA
tcatatatactttagattgatttaaaacttcatttttaatttaaaaggatctaggtgaagatcctttttgataatctcatgaccaaaatcccttaacgtgagttttcgttccactgagcgtcagaccccgtagaaaagatcaaaggatcttcttgagatcctttttttctgcgcgtaatctgctgcttgcaaacaaaaaaaccaccgctaccagcggtggtttgtttgccggatcaagagctaccaactctttttccgaaggtaactggcttcagcagagcgcagataccaaatactgttcttctagtgtagccgtagttaggccaccacttcaagaactctgtagcaccgcctacatacctcgctctgctaatcctgttaccagtggctgctgccagtggcgataagtcgtgtcttaccgggttggactcaagacgatagttaccggataaggcgcagcggtcgggctgaacggggggttcgtgcacacagcccagcttggagcgaacgacctacaccgaactgagatacctacagcgtgagctatgagaaagcgccacgcttcccgaagggagaaaggcggacaggtatccggtaagcggcagggtcggaacaggagagcgcacgagggagcttccagggggaaacgcctggtatctttatagtcctgtcgggtttcgccacctctgacttgagcgtcgatttttgtgatgctcgtcaggggggcggagcctatggaaaaacgccagcaacgcggcctttttacggttcctggccttttgctggccttttgctcacatgttctttcctgcgttatcccctgattctgtggataaccgtattaccgcctttgagtgagctgataccgctcgccgcagccgaacgaccgagcgcagcgagtcagtgagcgaggaagcggaagagcgcccaatacgcaaaccgcctctccccgcgcgttggccgattcattaatgcagctggcacgacaggtttcccgactggaaagcgggcagtgagcgcaacgcaattaatgtgagttagctcactcattaggcaccccaggctttacactttatgcttccggctcgtatgttgtgtggaattgtgagcggataacaatttcacacaggaaacagctatgaccatgattacgcctctagaaagctttaatacgactcactataaggactcactatttgttttcgcgcccagttgcaaaaagtgtcgacatttgcttctgacacaactgtgttcactagcaacctcaaacagacaccgccaccatgcctgctgctaagagagtgaaactggatggatccggccccgacatcgtgatgacccagagccccagcagcctgagcgccagcgtgggcgaccgcgtgaccatcacctgccgcagcagcaccggcgccgtgaccaccagcaactacgccagctgggtgcaggagaagcccggcaagctgttcaagggcctgatcggcggcaccaacaaccgcgcccccggcgtgcccagccgcttcagcggcagcctgatcggcgacaaggccaccctgaccatcagcagcctgcagcccgaggacttcgccacctacttctgcgccctgtggtacagcaaccactgggtgttcggccagggcaccaaggtggagctgaagcgcggcggcggcggcagcggcggcggcggcagcggcggcggcggcagcagcggcggcggcagcgaggtgaagctgctggagagcggcggcggcctggtgcagcccggcggcagcctgaagctgagctgcgccgtgagcggcttcagcctgaccgactacggcgtgaactgggtgcgccaggcccccggccgcggcctggagtggatcggcgtgatctggggcgacggcatcaccgactacaacagcgccctgaaggaccgcttcatcatcagcaaggacaacggcaagaacaccgtgtacctgcagatgagcaaggtgcgcagcgacgacaccgccctgtactactgcgtgaccggcctgttcgactactggggccagggcaccctggtgaccgtgagcagctacccatacgatgttccagattacgctggtggaggcggaggttctgggggaggaggtagtggcggtggtggttcaggaggcggcggaagcttggatccaggtggaggtggaagcggtatgaacaattcccagggaagagtgaccttcgaggacgtgaccgtgaacttcacccaaggcgagtggcagagactgaaccccgagcagagaaacctgtaccgggacgtgatgctggaaaactacagcaacctggtgtccgtcggccagggcgagacaacaaagcctgacgtgatcctgcggctggaacagggcaaagagccttggctggaagaggaagaggtgctcggatctggcagagccgagaagaatggcgatatcggcggacagatctggaagccaaaggatgtgaaagagagtctcggaagcggagctactaacttcagcctgctgaagcaggctggagacgtggaggagaaccctggacctatgcctgctgctaagagagtgaaactggatggatccaaccatgaccaggaatttgaccccccaaaggtttacccacctgtgccagctgagaagaggaagcccatccgcgtgctgtctctctttgatgggattgctacagggctcctggtgctgaaggacctgggcatccaagtggaccgctacattgcctccgaggtgtgtgaggactccatcacggtgggcatggtgcggcaccagggaaagatcatgtacgtcggggacgtccgcagcgtcacacagaagcatatccaggagtggggcccattcgacctggtgattggaggcagtccctgcaatgacctctccattgtcaaccctgcccgcaagggactttatgagggtactggccgcctcttctttgagttctaccgcctcctgcatgatgcgcggcccaaggagggagatgatcgccccttcttctggctctttgagaatgtggtggccatgggcgttagtgacaagagggacatctcgcgatttcttgagtctaaccccgtgatgattgacgccaaagaagtgtctgctgcacacagggcccgttacttctggggtaaccttcctggcatgaacaggcctttggcatccactgtgaatgataagctggagctgcaagagtgtctggagcacggcagaatagccaagttcagcaaagtgaggaccattaccaccaggtcaaactctataaagcagggcaaagaccagcatttccccgtgttcatgaacgagaaggaggacatcctgtggtgcactgaaatggaaagggtgtttggcttccccgtccactacacagacgtctccaacatgagccgcttggcgaggcagagactgctgggccgatcgtggagcgtgccggtcatccgccacctcttcgctccgctgaaggaatattttgcttgtgtgtctagcggcaatagtaacgctaacagccgcgggccgagcttcagcagcggcctggtgccgttaagcttgcgcggcagccatatgttcgaaaccgtgcctgtgtggaggagacagccagtccgggtgctgtccctttttgaagacatcaagaaagagctgacgagtttgggctttttggaaagtggttctgacccgggacaactgaagcatgtggttgatgtcacagacacagtgaggaaggatgtggaggagtggggacccttcgatcttgtgtacggcgccacacctcccctgggccacacctgtgaccgtcctcccagctggtacctgttccagttccaccggctcctgcagtacgcacggcccaagccaggcagccccaggcccttcttctggatgttcgtggacaatctggtgctgaacaaggaagacctggacgtcgcatctcgcttcctggagatggagccagtcaccatcccagatgtccacggcggatccttgcagaatgctgtccgcgtgtggagcaacatcccagccataaggagcagcaggcactgggctctggtttcggaagaagaattgtccctgctggcccagaacaagcagagctcgaagctcgcggccaagtggcccaccaagctggtgaagaactgctttctccccctaagagaatatttcaagtatttttcaggagggccgagctctggcgcacccccaccaagtggagggtctcctgccgggtccccaacatctactgaagaaggcaccagcgaatccgcaacgcccgagtcaggccctggtacctccacagaaccatctgaaggtagtgcgcctggttccccagctggaagccctacttccaccgaagaaggcacgtcaaccgaaccaagtgaaggatctgcccctgggaccagcactgaaccatctgagccaaaaaagaagagaaaggtaatggaagagacacggacccctgagaagatcgcctgccagcaggatagaagcgccttcttcaagctgggcaagctgccccagaaaaccaccagcgccatctaccacctgatgcggtgtagcaagcggtacatcgacaacgtgtccgagacaatcagcaacaacatcgagaaggccgccatgaccagcgacaaccacatcttcagaagcgccctgaaagaagagtacaagaagatctaccgcgagaagttctaccccgacgtgaccggccagccttttccagataagggccccgacaacacccacatcgtggaacggaccgtggaaaacctgtgcggccagtacatctctgccctgaagggcgtgatgaaagtgcggaagcccaagtggcaggacgacatcttcgaggacgagagcgacaaagtgatcgccgagatgctgatggccagcggcaacgaggccgacattcaccccaagctggaaaagaagattgccagcgccaagaaaaaggacaagatggacgagtggcagaaggtgctggacagatacgactacatcaagagcaagaccgacatcgagtggacctacaccacactgctgtacgaccacattgcccgcgagtgcgccagatccatgttcgaggatggcaacaagcctaagttctgctacaccaacggcaacaagttcgccaaacaggtggtggacgagctgtggggctctgagagagtggaatacgagtacgagaagtacctgcactgcagaaccctggaagcctactggaacgaggaaaacaagtacttcttcctggaaaatcaaaagaagtccaagaaaacctacgaggcccggcagatcatcgaccacttcatcgagaacgaggacgccgtgaaggccgaaaccgaagagtatatggccaaggtggccaaagagttcggcgagaacggcggctgcaagttcagaaccgagaacatcctgtacctggtcaacagcgtgtccatcaacaagaagcaggacgaggaacggtgccccatcttcaaagtgaccgacattccccagtatgccgaggccggcatcgatagaatcggcgagtgcaaatacgtgatcaagctgaagctgttcaccgtgggcgagagatacggcaccacctatatgcctgaggccttcagcggcctgtacgacagaaggaccaaccagagatacgacctgatcgacagagcctgcaagggcagctacgtgtacctgcctatctacatcagcgacaaggacagccggaagtggagcgacagactgaagaacaccttcaccatgtccgccttcagcatcagcgagcgcaagaccaagaaagacggcagagtgctgtgcgtgaacctgccttacacacacatccagcacaagccccggaactacttcaaggtgtaccccacctacggcgtggacatcaacgtgaagcacagcctgttcagcaccaacgccaccaacctgaacggctacatcgacgtgaacggcgagctgatcgacttctacaacagcatcggcagacccgataagctcaagaacatcaacctggccgtgacactgggcgacaaaggcggcacagctggcaaccacaccaactttctgctggtgtccgacctcggcgactgggatgatcacggcaagaagcggaacgacagattcgtgaagagagaggacggcacctactacagcagacctgacctgctggccgccggcctgaacttcctgaagaagaagtatagcggcgaccggaagtcctacgattatatcaacaccacaatcgccttccggaacaaccagaccagactgagatgcatcgacaaagagtggaacgatcggaagcgggcctacgatgaggaacacggcaagcctgagaagggcgaaagaagcggcttctaccctaccgaggatgccgagcggctgacaatggaaagacaggccctgcggagagagattgccgagaacaccagacaagtgattgcctacatgctgtggctgttccaagagaacggcatcaagtctatcgccctggaacacctggattgcggcagctggaagaacttccgggaccagctgaagccaaagtggttctgcaacaactgcaagtactgggccgagaagtatggcatcccttacgaggccaccaagtactacagaagcaaccggaagtactttgacatcgaggacggggagctgattcccgagaatgtgaagctgaacgccctgggcgaagccgagaacgacaagagatacttccagacctctatcgccaaggccgtgggcatgagcagcatcaagcagatgttcagcatcgtgtcccagaactacgacatccaagtgaactacaccgagcaggcctacaccagccagaccgacagcagaaatggcaccgtggacaaggacttcagagtgtcccaagagtgctacatcggcagcgacggcaccaagatgaactgcgactttaacgccgccgtgaatatcgccgaccggatctccgatgacaccctgcgggaagagttcaacaaagaactgcccatgaaggaatttgtgaagtacggcgccacacagatcgtgtctcggaacagaagatggaacgccgaaaacgccgagagggtcacaatggccgccttccagaagagaaagaacgctgacggcggagcccataccgccgctgtgaagcctacatccaagaccgaggaaagcagcctgaagctggtggccgaagcctatccctatgacgtgcccgattatgccagcctgggcagcggctcccccaagaaaaaacgcaaggtggaagatcctaagaaaaagcggaaagtggacggcattggtagtgggagcaacggcagcagcggagaggaactgctgagcaagaactaccacctggaaaacgaggtggccagactgaagaaaggctctggctctggcggaagcggttctggcggatcaggatctggaagtggcggctctggaagcggaggttctggatctggcgaagaactgctgtctaagaattatcacggttcaggctccggccagcggggaagcaagcgcaccgccgatggttccgagttcgaaagccccaaaaaaaagcgcaaggtctgagatcccaagcacgcagcaatgcagctcaaaacgcttagcctagccacacccccacgggaaacagcagtgattaacctttagcaataaacgaaagtttaactaagctatactaaccccagggttggtcaatttcgtgccagccacaccctggtactgcatgcacgcaatgctagctgcccctttcccgtcctgggcaccccgagtctcccccgaccccgggtcccaggtatgctcccacctccacctgccccactcaccacctctgctagttccagacacctccgagacgaggaaaaaaaaaaaaaaaaaaaaaaaaaaaaaaaaaaaaaaaaaaaaaaaaaaaaaaaaaaaaaaaaaaaaaaaaaaaaaaaaaaaaaaaaaaaaaaaaaaaaaaaaaaaaaaaaaaaaaaaaaaaaaaaaaaaaaaaaaaaaaaaaaaaaaaaaaaaaaaaaaaaaaaaaaaaaaaaaaaaaaaaaaaaaaaaaaaaaaaaaaaaaaaaaaaaaaaaaaaaaaaaaaaaaaaaaaaaaaaaaaaaaaaaaaaaaaaaaaaaaaaaaaaaaaaaaaaaaaaaaaaaaaaaaaaaaaaaaaaaaaaaaaaaaaaaaaaaaaaaaaaaaaaaaaaaaaaaaaaaaaaaaaaaaaaaaaaaaaaaaaaaaaaaaaaaaaaaaaaaaaaaaaaaaaaaaaaccgtcttcaagctttctagaaattcactggccgtcgttttacaacgtcgtgactgggaaaaccctggcgttacccaacttaatcgccttgcagcacatccccctttcgccagctggcgtaatagcgaagaggcccgcaccgatcgcccttcccaacagttgcgcagcctgaatggcgaatggcgcctgatgcggtattttctccttacgcatctgtgcggtatttcacaccgcatatggtgcactctcagtacaatctgctctgatgccgcatagttaagccagccccgacacccgccaacacccgctgacgcgccctgacgggcttgtctgctcccggcatccgcttacagacaagctgtgaccgtctccgggagctgcatgtgtcagaggttttcaccgtcatcaccgaaacgcgcgagacgaaagggcctcgtgatacgcctatttttataggttaatgtcatgataataatggtttcttagacgtcaggtggcacttttcggggaaatgtgcgcggaacccctatttgtttatttttctaaatacattcaaatatgtatccgctcatgagacaataaccctgataaatgcttcaataatattgaaaaaggaagagtatgagtattcaacatttccgtgtcgcccttattcccttttttgcggcattttgccttcctgtttttgctcacccagaaacgctggtgaaagtaaaagatgctgaagatcagttgggtgcacgagtgggttacatcgaactggatctcaacagcggtaagatccttgagagttttcgccccgaagaacgttttccaatgatgagcacttttaaagttctgctatgtggcgcggtattatcccgtattgacgccgggcaagagcaactcggtcgccgcatacactattctcagaatgacttggttgagtactcaccagtcacagaaaagcatcttacggatggcatgacagtaagagaattatgcagtgctgccataaccatgagtgataacactgcggccaacttacttctgacaacgatcggaggaccgaaggagctaaccgcttttttgcacaacatgggggatcatgtaactcgccttgatcgttgggaaccggagctgaatgaagccataccaaacgacgagcgtgacaccacgatgcctgtagcaatggcaacaacgttgcgcaaactattaactggcgaactacttactctagcttcccggcaacaattaatagactggatggaggcggataaagttgcaggaccacttctgcgctcggcccttccggctggctggtttattgctgataaatctggagccggtgagcgtgggtctcgcggtatcattgcagcactggggccagatggtaagccctcccgtatcgtagttatctacacgacggggagtcaggcaactatggatgaacgaaatagacagatcgctgagataggtgcctcactgattaagcattggtaactgtcagaccaagtttac

SEQ ID NO: 214 - DNA, 11001 bp, synthetic construct
  misc_feature 1..11001: note = DNA of V20_KRAB-scFv-2a-D3a-D3l-dCas9-2xGCN4
  source 1..11001: mol_type = other DNA
tcatatatactttagattgatttaaaacttcatttttaatttaaaaggatctaggtgaagatcctttttgataatctcatgaccaaaatcccttaacgtgagttttcgttccactgagcgtcagaccccgtagaaaagatcaaaggatcttcttgagatcctttttttctgcgcgtaatctgctgcttgcaaacaaaaaaaccaccgctaccagcggtggtttgtttgccggatcaagagctaccaactctttttccgaaggtaactggcttcagcagagcgcagataccaaatactgttcttctagtgtagccgtagttaggccaccacttcaagaactctgtagcaccgcctacatacctcgctctgctaatcctgttaccagtggctgctgccagtggcgataagtcgtgtcttaccgggttggactcaagacgatagttaccggataaggcgcagcggtcgggctgaacggggggttcgtgcacacagcccagcttggagcgaacgacctacaccgaactgagatacctacagcgtgagctatgagaaagcgccacgcttcccgaagggagaaaggcggacaggtatccggtaagcggcagggtcggaacaggagagcgcacgagggagcttccagggggaaacgcctggtatctttatagtcctgtcgggtttcgccacctctgacttgagcgtcgatttttgtgatgctcgtcaggggggcggagcctatggaaaaacgccagcaacgcggcctttttacggttcctggccttttgctggccttttgctcacatgttctttcctgcgttatcccctgattctgtggataaccgtattaccgcctttgagtgagctgataccgctcgccgcagccgaacgaccgagcgcagcgagtcagtgagcgaggaagcggaagagcgcccaatacgcaaaccgcctctccccgcgcgttggccgattcattaatgcagctggcacgacaggtttcccgactggaaagcgggcagtgagcgcaacgcaattaatgtgagttagctcactcattaggcaccccaggctttacactttatgcttccggctcgtatgttgtgtggaattgtgagcggataacaatttcacacaggaaacagctatgaccatgattacgcctctagaaagctttaatacgactcactataaggactcactatttgttttcgcgcccagttgcaaaaagtgtcgacatttgcttctgacacaactgtgttcactagcaacctcaaacagacaccgccaccatgcctgctgctaagagagtgaaactggatggatcccggacactggtgaccttcaaggatgtatttgtggacttcaccagggaggagtggaagctgctggacactgctcagcagatcgtgtacagaaatgtgatgctggagaactataagaacctggtttccttgggttatcagcttactaagccagatgtgatcctccggttggagaagggagaagagcccggaagcggaatgggccccgacatcgtgatgacccagagccccagcagcctgagcgccagcgtgggcgaccgcgtgaccatcacctgccgcagcagcaccggcgccgtgaccaccagcaactacgccagctgggtgcaggagaagcccggcaagctgttcaagggcctgatcggcggcaccaacaaccgcgcccccggcgtgcccagccgcttcagcggcagcctgatcggcgacaaggccaccctgaccatcagcagcctgcagcccgaggacttcgccacctacttctgcgccctgtggtacagcaaccactgggtgttcggccagggcaccaaggtggagctgaagcgcggcggcggcggcagcggcggcggcggcagcggcggcggcggcagcagcggcggcggcagcgaggtgaagctgctggagagcggcggcggcctggtgcagcccggcggcagcctgaagctgagctgcgccgtgagcggcttcagcctgaccgactacggcgtgaactgggtgcgccaggcccccggccgcggcctggagtggatcggcgtgatctggggcgacggcatcaccgactacaacagcgccctgaaggaccgcttcatcatcagcaaggacaacggcaagaacaccgtgtacctgcagatgagcaaggtgcgcagcgacgacaccgccctgtactactgcgtgaccggcctgttcgactactggggccagggcaccctggtgaccgtgagcagctacccatacgatgttccagattacgctggtggaggcggaggttctgggggaggaggtagtggcggtggtggttcaggaggcggcggaagcggaagcggagctactaacttcagcctgctgaagcaggctggagacgtggaggagaaccctggacctatgcctgctgctaagagagtgaaactggatggatccaaccatgaccaggaatttgaccccccaaaggtttacccacctgtgccagctgagaagaggaagcccatccgcgtgctgtctctctttgatgggattgctacagggctcctggtgctgaaggacctgggcatccaagtggaccgctacattgcctccgaggtgtgtgaggactccatcacggtgggcatggtgcggcaccagggaaagatcatgtacgtcggggacgtccgcagcgtcacacagaagcatatccaggagtggggcccattcgacctggtgattggaggcagtccctgcaatgacctctccattgtcaaccctgcccgcaagggactttatgagggtactggccgcctcttctttgagttctaccgcctcctgcatgatgcgcggcccaaggagggagatgatcgccccttcttctggctctttgagaatgtggtggccatgggcgttagtgacaagagggacatctcgcgatttcttgagtctaaccccgtgatgattgacgccaaagaagtgtctgctgcacacagggcccgttacttctggggtaaccttcctggcatgaacaggcctttggcatccactgtgaatgataagctggagctgcaagagtgtctggagcacggcagaatagccaagttcagcaaagtgaggaccattaccaccaggtcaaactctataaagcagggcaaagaccagcatttccccgtgttcatgaacgagaaggaggacatcctgtggtgcactgaaatggaaagggtgtttggcttccccgtccactacacagacgtctccaacatgagccgcttggcgaggcagagactgctgggccgatcgtggagcgtgccggtcatccgccacctcttcgctccgctgaaggaatattttgcttgtgtgtctagcggcaatagtaacgctaacagccgcgggccgagcttcagcagcggcctggtgccgttaagcttgcgcggcagccatatgttcgaaaccgtgcctgtgtggaggagacagccagtccgggtgctgtccctttttgaagacatcaagaaagagctgacgagtttgggctttttggaaagtggttctgacccgggacaactgaagcatgtggttgatgtcacagacacagtgaggaaggatgtggaggagtggggacccttcgatcttgtgtacggcgccacacctcccctgggccacacctgtgaccgtcctcccagctggtacctgttccagttccaccggctcctgcagtacgcacggcccaagccaggcagccccaggcccttcttctggatgttcgtggacaatctggtgctgaacaaggaagacctggacgtcgcatctcgcttcctggagatggagccagtcaccatcccagatgtccacggcggatccttgcagaatgctgtccgcgtgtggagcaacatcccagccataaggagcagcaggcactgggctctggtttcggaagaagaattgtccctgctggcccagaacaagcagagctcgaagctcgcggccaagtggcccaccaagctggtgaagaactgctttctccccctaagagaatatttcaagtatttttcaggagggccgagctctggcgcacccccaccaagtggagggtctcctgccgggtccccaacatctactgaagaaggcaccagcgaatccgcaacgcccgagtcaggccctggtacctccacagaaccatctgaaggtagtgcgcctggttccccagctggaagccctacttccaccgaagaaggcacgtcaaccgaaccaagtgaaggatctgcccctgggaccagcactgaaccatctgagccaaaaaagaagagaaaggtaatggacaagaagtacagcatcggcctggccatcggcaccaactctgtgggctgggccgtgatcaccgacgagtacaaggtgcccagcaagaaattcaaggtgctgggcaacaccgaccggcacagcatcaagaagaacctgatcggcgccctgctgttcgacagcggagaaacagccgaggccacccggctgaagagaaccgccagaagaagatacaccagacggaagaaccggatctgctatctgcaagagatcttcagcaacgagatggccaaggtggacgacagcttcttccacagactggaagagtccttcctggtggaagaggataagaagcacgagcggcaccccatcttcggcaacatcgtggacgaggtggcctaccacgagaagtaccccaccatctaccacctgagaaagaaactggtggacagcaccgacaaggccgacctgcggctgatctatctggccctggcccacatgatcaagttccggggccacttcctgatcgagggcgacctgaaccccgacaacagcgacgtggacaagctgttcatccagctggtgcagacctacaaccagctgttcgaggaaaaccccatcaacgccagcggcgtggacgccaaggccatcctgtctgccagactgagcaagagcagacggctggaaaatctgatcgcccagctgcccggcgagaagaagaatggcctgttcggcaacctgattgccctgagcctgggcctgacccccaacttcaagagcaacttcgacctggccgaggatgccaaactgcagctgagcaaggacacctacgacgacgacctggacaacctgctggcccagatcggcgaccagtacgccgacctgtttctggccgccaagaacctgtccgacgccatcctgctgagcgacatcctgagagtgaacaccgagatcaccaaggcccccctgagcgcctctatgatcaagagatacgacgagcaccaccaggacctgaccctgctgaaagctctcgtgcggcagcagctgcctgagaagtacaaagagattttcttcgaccagagcaagaacggctacgccggctacatcgatggcggagccagccaggaagagttctacaagttcatcaagcccatcctggaaaagatggacggcaccgaggaactgctcgtgaagctgaacagagaggacctgctgcggaagcagcggaccttcgacaacggcagcatcccccaccagatccacctgggagagctgcacgccattctgcggcggcaggaagatttttacccattcctgaaggacaaccgggaaaagatcgagaagatcctgaccttccgcatcccctactacgtgggccctctggccaggggaaacagcagattcgcctggatgaccagaaagagcgaggaaaccatcaccccctggaacttcgaggaagtggtggacaagggcgccagcgcccagagcttcatcgagcggatgaccaacttcgataagaacctgcccaacgagaaggtgctgcccaagcacagcctgctgtacgagtacttcaccgtgtacaacgagctgaccaaagtgaaatacgtgaccgagggaatgagaaagcccgccttcctgagcggcgagcagaaaaaagccatcgtggacctgctgttcaagaccaaccggaaagtgaccgtgaagcagctgaaagaggactacttcaagaaaatcgagtgcttcgactccgtggaaatctccggcgtggaagatcggttcaacgcctccctgggcacataccacgatctgctgaaaattatcaaggacaaggacttcctggacaatgaggaaaacgaggacattctggaagatatcgtgctgaccctgacactgtttgaggacagagagatgatcgaggaacggctgaaaacctatgcccacctgttcgacgacaaagtgatgaagcagctgaagcggcggagatacaccggctggggcaggctgagccggaagctgatcaacggcatccgggacaagcagtccggcaagacaatcctggatttcctgaagtccgacggcttcgccaacagaaacttcatgcagctgatccacgacgacagcctgacctttaaagaggacatccagaaagcccaggtgtccggccagggcgatagcctgcacgagcacattgccaatctggccggcagccccgccattaagaagggcatcctgcagacagtgaaggtggtggacgagctcgtgaaagtgatgggccggcacaagcccgagaacatcgtgatcgaaatggccagagagaaccagaccacccagaagggacagaagaacagccgcgagagaatgaagcggatcgaagagggcatcaaagagctgggcagccagatcctgaaagaacaccccgtggaaaacacccagctgcagaacgagaagctgtacctgtactacctgcagaatgggcgggatatgtacgtggaccaggaactggacatcaaccggctgtccgactacgatgtggacgctatcgtgcctcagagctttctgaaggacgactccatcgataacaaagtgctgactcggagcgacaagaaccggggcaagagcgacaacgtgccctccgaagaggtcgtgaagaagatgaagaactactggcgccagctgctgaatgccaagctgattacccagaggaagttcgacaatctgaccaaggccgagagaggcggcctgagcgaactggataaggccggcttcatcaagagacagctggtggaaacccggcagatcacaaagcacgtggcacagatcctggactcccggatgaacactaagtacgacgagaacgacaaactgatccgggaagtgaaagtgatcaccctgaagtccaagctggtgtccgatttccggaaggatttccagttttacaaagtgcgcgagatcaacaactaccaccacgcccacgacgcctacctgaacgccgtcgtgggaaccgccctgatcaaaaagtaccctaagctggaaagcgagttcgtgtacggcgactacaaggtgtacgacgtgcggaagatgatcgccaagagcgagcaggaaatcggcaaggctaccgccaagtacttcttctacagcaacatcatgaactttttcaagaccgagattaccctggccaacggcgagatccggaagcggcctctgatcgagacaaacggcgaaacaggcgagatcgtgtgggataagggccgggactttgccaccgtgcggaaagtgctgtctatgccccaagtgaatatcgtgaaaaagaccgaggtgcagacaggcggcttcagcaaagagtctatcctgcccaagaggaacagcgacaagctgatcgccagaaagaaggactgggaccctaagaagtacggcggcttcgacagccccaccgtggcctattctgtgctggtggtggccaaagtggaaaagggcaagtccaagaaactgaagagtgtgaaagagctgctggggatcaccatcatggaaagaagcagcttcgagaagaatcccatcgactttctggaagccaagggctacaaagaagtgaaaaaggacctgatcatcaagctgcctaagtactccctgttcgagctggaaaacggccggaagagaatgctggcctctgccggcgaactgcagaagggaaacgaactggccctgccctccaaatatgtgaacttcctgtacctggccagccactatgagaagctgaagggctcccccgaggataatgagcagaaacagctgtttgtggaacagcacaaacactacctggacgagatcatcgagcagatcagcgagttctccaagagagtgatcctggccgacgctaatctggacaaggtgctgagcgcctacaacaagcacagagacaagcctatcagagagcaggccgagaatatcatccacctgtttaccctgaccaatctgggagcccctgccgccttcaagtactttgacaccaccatcgaccggaagaggtacaccagcaccaaagaggtgctggacgccaccctgatccaccagagcatcaccggcctgtacgagacacggatcgacctgtctcagctgggaggcgacgcctatccctatgacgtgcccgattatgccagcctgggcagcggctcccccaagaaaaaacgcaaggtggaagatcctaagaaaaagcggaaagtggacggcattggtagtgggagcaacggcagcagcggagaggaactgctgagcaagaactaccacctggaaaacgaggtggccagactgaagaaaggctctggctctggcggaagcggttctggcggatcaggatctggaagtggcggctctggaagcggaggttctggatctggcgaagaactgctgtctaagaattatcacctcgagaatgaagtcgctcgtttgaagaaaggttcaggctccggccagcggggaagcaagcgcaccgccgatggttccgagttcgaaagccccaaaaaaaagcgcaaggtctgagatcccaagcacgcagcaatgcagctcaaaacgcttagcctagccacacccccacgggaaacagcagtgattaacctttagcaataaacgaaagtttaactaagctatactaaccccagggttggtcaatttcgtgccagccacaccctggtactgcatgcacgcaatgctagctgcccctttcccgtcctgggcaccccgagtctcccccgaccccgggtcccaggtatgctcccacctccacctgccccactcaccacctctgctagttccagacacctccgagacgaggaaaaaaaaaaaaaaaaaaaaaaaaaaaaaaaaaaaaaaaaaaaaaaaaaaaaaaaaaaaaaaaaaaaaaaaaaaaaaaaaaaaaaaaaaaaaaaaaaaaaaaaaaaaaaaaaaaaaaaaaaaaaaaaaaaaaaaaaaaaaaaaaaaaaaaaaaaaaaaaaaaaaaaaaaaaaaaaaaaaaaaaaaaaaaaaaaaaaaaaaaaaaaaaaaaaaaaaaaaaaaaaaaaaaaaaaaaaaaaaaaaaaaaaaaaaaaaaaaaaaaaaaaaaaaaaaaaaaaaaaaaaaaaaaaaaaaaaaaaaaaaaaaaaaaaaaaaaaaaaaaaaaaaaaaaaaaaaaaaaaaaaaaaaaaaaaaaaaaaaaaaaaaaaaaaaaaaaaaaaaaaaaaaaaaaaaaaccgtcttcaagctttctagaaattcactggccgtcgttttacaacgtcgtgactgggaaaaccctggcgttacccaacttaatcgccttgcagcacatccccctttcgccagctggcgtaatagcgaagaggcccgcaccgatcgcccttcccaacagttgcgcagcctgaatggcgaatggcgcctgatgcggtattttctccttacgcatctgtgcggtatttcacaccgcatatggtgcactctcagtacaatctgctctgatgccgcatagttaagccagccccgacacccgccaacacccgctgacgcgccctgacgggcttgtctgctcccggcatccgcttacagacaagctgtgaccgtctccgggagctgcatgtgtcagaggttttcaccgtcatcaccgaaacgcgcgagacgaaagggcctcgtgatacgcctatttttataggttaatgtcatgataataatggtttcttagacgtcaggtggcacttttcggggaaatgtgcgcggaacccctatttgtttatttttctaaatacattcaaatatgtatccgctcatgagacaataaccctgataaatgcttcaataatattgaaaaaggaagagtatgagtattcaacatttccgtgtcgcccttattcccttttttgcggcattttgccttcctgtttttgctcacccagaaacgctggtgaaagtaaaagatgctgaagatcagttgggtgcacgagtgggttacatcgaactggatctcaacagcggtaagatccttgagagttttcgccccgaagaacgttttccaatgatgagcacttttaaagttctgctatgtggcgcggtattatcccgtattgacgccgggcaagagcaactcggtcgccgcatacactattctcagaatgacttggttgagtactcaccagtcacagaaaagcatcttacggatggcatgacagtaagagaattatgcagtgctgccataaccatgagtgataacactgcggccaacttacttctgacaacgatcggaggaccgaaggagctaaccgcttttttgcacaacatgggggatcatgtaactcgccttgatcgttgggaaccggagctgaatgaagccataccaaacgacgagcgtgacaccacgatgcctgtagcaatggcaacaacgttgcgcaaactattaactggcgaactacttactctagcttcccggcaacaattaatagactggatggaggcggataaagttgcaggaccacttctgcgctcggcccttccggctggctggtttattgctgataaatctggagccggtgagcgtgggtctcgcggtatcattgcagcactggggccagatggtaagccctcccgtatcgtagttatctacacgacggggagtcaggcaactatggatgaacgaaatagacagatcgctgagataggtgcctcactgattaagcattggtaactgtcagaccaagtttac

SEQ ID NO: 215 - DNA, 11718 bp, synthetic construct
  misc_feature 1..11718: note = DNA of V21_hSIRT1-scFv-2a-D3a-D3l-dCas9-2xGCN4
  source 1..11718: mol_type = other DNA
tcatatatactttagattgatttaaaacttcatttttaatttaaaaggatctaggtgaagatcctttttgataatctcatgaccaaaatcccttaacgtgagttttcgttccactgagcgtcagaccccgtagaaaagatcaaaggatcttcttgagatcctttttttctgcgcgtaatctgctgcttgcaaacaaaaaaaccaccgctaccagcggtggtttgtttgccggatcaagagctaccaactctttttccgaaggtaactggcttcagcagagcgcagataccaaatactgttcttctagtgtagccgtagttaggccaccacttcaagaactctgtagcaccgcctacatacctcgctctgctaatcctgttaccagtggctgctgccagtggcgataagtcgtgtcttaccgggttggactcaagacgatagttaccggataaggcgcagcggtcgggctgaacggggggttcgtgcacacagcccagcttggagcgaacgacctacaccgaactgagatacctacagcgtgagctatgagaaagcgccacgcttcccgaagggagaaaggcggacaggtatccggtaagcggcagggtcggaacaggagagcgcacgagggagcttccagggggaaacgcctggtatctttatagtcctgtcgggtttcgccacctctgacttgagcgtcgatttttgtgatgctcgtcaggggggcggagcctatggaaaaacgccagcaacgcggcctttttacggttcctggccttttgctggccttttgctcacatgttctttcctgcgttatcccctgattctgtggataaccgtattaccgcctttgagtgagctgataccgctcgccgcagccgaacgaccgagcgcagcgagtcagtgagcgaggaagcggaagagcgcccaatacgcaaaccgcctctccccgcgcgttggccgattcattaatgcagctggcacgacaggtttcccgactggaaagcgggcagtgagcgcaacgcaattaatgtgagttagctcactcattaggcaccccaggctttacactttatgcttccggctcgtatgttgtgtggaattgtgagcggataacaatttcacacaggaaacagctatgaccatgattacgcctctagaaagctttaatacgactcactataaggactcactatttgttttcgcgcccagttgcaaaaagtgtcgacatttgcttctgacacaactgtgttcactagcaacctcaaacagacaccgccaccatgcctgctgctaagagagtgaaactggatggatccacaattcttaaagatttattgccggaaacaatacctccacctgagttggatgatatgacactgtggcagattgttattaatatcctttcagaaccaccaaaaaggaaaaaaagaaaagatattaatacaattgaagatgctgtgaaattactgcaagagtgcaaaaaaattatagttctaactggagctggggtgtctgtttcatgtggaatacctgacttcaggtcaagggatggtatttatgctcgccttgctgtagacttcccagatcttccagatcctcaagcgatgtttgatattgaatatttcagaaaagatccaagaccattcttcaagtttgcaaaggaaatatatcctggacaattccagccatctctctgtcacaaattcatagccttgtcagataaggaaggaaaactacttcgcaactatacccagaacatagacacgctggaacaggttgcgggaatccaaaggataattcagtgtcatggttcctttgcaacagcatcttgcctgatttgtaaatacaaagttgactgtgaagctgtacgaggagatatttttaatcaggtagttcctcgatgtcctaggtgcccagctgatgaaccgcttgctatcatgaaaccagagattgtgttttttggtgaaaatttaccagaacagtttcatagagccatgaagtatgacaaagatgaagttgacctcctcattgttattgggtcttccctcaaagtaagaccagtagcactaattccaagttccataccccatgaagtgcctcagatattaattaatagagaacctttgcctcatctgcattttgatgtagagcttcttggagactgtgatgtcataattaatgaattgtgtcataggttaggtggtgaatatgccaaacttggaagcggaatgggccccgacatcgtgatgacccagagccccagcagcctgagcgccagcgtgggcgaccgcgtgaccatcacctgccgcagcagcaccggcgccgtgaccaccagcaactacgccagctgggtgcaggagaagcccggcaagctgttcaagggcctgatcggcggcaccaacaaccgcgcccccggcgtgcccagccgcttcagcggcagcctgatcggcgacaaggccaccctgaccatcagcagcctgcagcccgaggacttcgccacctacttctgcgccctgtggtacagcaaccactgggtgttcggccagggcaccaaggtggagctgaagcgcggcggcggcggcagcggcggcggcggcagcggcggcggcggcagcagcggcggcggcagcgaggtgaagctgctggagagcggcggcggcctggtgcagcccggcggcagcctgaagctgagctgcgccgtgagcggcttcagcctgaccgactacggcgtgaactgggtgcgccaggcccccggccgcggcctggagtggatcggcgtgatctggggcgacggcatcaccgactacaacagcgccctgaaggaccgcttcatcatcagcaaggacaacggcaagaacaccgtgtacctgcagatgagcaaggtgcgcagcgacgacaccgccctgtactactgcgtgaccggcctgttcgactactggggccagggcaccctggtgaccgtgagcagctacccatacgatgttccagattacgctggtggaggcggaggttctgggggaggaggtagtggcggtggtggttcaggaggcggcggaagcggaagcggagctactaacttcagcctgctgaagcaggctggagacgtggaggagaaccctggacctatgcctgctgctaagagagtgaaactggatggatccaaccatgaccaggaatttgaccccccaaaggtttacccacctgtgccagctgagaagaggaagcccatccgcgtgctgtctctctttgatgggattgctacagggctcctggtgctgaaggacctgggcatccaagtggaccgctacattgcctccgaggtgtgtgaggactccatcacggtgggcatggtgcggcaccagggaaagatcatgtacgtcggggacgtccgcagcgtcacacagaagcatatccaggagtggggcccattcgacctggtgattggaggcagtccctgcaatgacctctccattgtcaaccctgcccgcaagggactttatgagggtactggccgcctcttctttgagttctaccgcctcctgcatgatgcgcggcccaaggagggagatgatcgccccttcttctggctctttgagaatgtggtggccatgggcgttagtgacaagagggacatctcgcgatttcttgagtctaaccccgtgatgattgacgccaaagaagtgtctgctgcacacagggcccgttacttctggggtaaccttcctggcatgaacaggcctttggcatccactgtgaatgataagctggagctgcaagagtgtctggagcacggcagaatagccaagttcagcaaagtgaggaccattaccaccaggtcaaactctataaagcagggcaaagaccagcatttccccgtgttcatgaacgagaaggaggacatcctgtggtgcactgaaatggaaagggtgtttggcttccccgtccactacacagacgtctccaacatgagccgcttggcgaggcagagactgctgggccgatcgtggagcgtgccggtcatccgccacctcttcgctccgctgaaggaatattttgcttgtgtgtctagcggcaatagtaacgctaacagccgcgggccgagcttcagcagcggcctggtgccgttaagcttgcgcggcagccatatgttcgaaaccgtgcctgtgtggaggagacagccagtccgggtgctgtccctttttgaagacatcaagaaagagctgacgagtttgggctttttggaaagtggttctgacccgggacaactgaagcatgtggttgatgtcacagacacagtgaggaaggatgtggaggagtggggacccttcgatcttgtgtacggcgccacacctcccctgggccacacctgtgaccgtcctcccagctggtacctgttccagttccaccggctcctgcagtacgcacggcccaagccaggcagccccaggcccttcttctggatgttcgtggacaatctggtgctgaacaaggaagacctggacgtcgcatctcgcttcctggagatggagccagtcaccatcccagatgtccacggcggatccttgcagaatgctgtccgcgtgtggagcaacatcccagccataaggagcagcaggcactgggctctggtttcggaagaagaattgtccctgctggcccagaacaagcagagctcgaagctcgcggccaagtggcccaccaagctggtgaagaactgctttctccccctaagagaatatttcaagtatttttcaggagggccgagctctggcgcacccccaccaagtggagggtctcctgccgggtccccaacatctactgaagaaggcaccagcgaatccgcaacgcccgagtcaggccctggtacctccacagaaccatctgaaggtagtgcgcctggttccccagctggaagccctacttccaccgaagaaggcacgtcaaccgaaccaagtgaaggatctgcccctgggaccagcactgaaccatctgagccaaaaaagaagagaaaggtaatggacaagaagtacagcatcggcctggccatcggcaccaactctgtgggctgggccgtgatcaccgacgagtacaaggtgcccagcaagaaattcaaggtgctgggcaacaccgaccggcacagcatcaagaagaacctgatcggcgccctgctgttcgacagcggagaaacagccgaggccacccggctgaagagaaccgccagaagaagatacaccagacggaagaaccggatctgctatctgcaagagatcttcagcaacgagatggccaaggtggacgacagcttcttccacagactggaagagtccttcctggtggaagaggataagaagcacgagcggcaccccatcttcggcaacatcgtggacgaggtggcctaccacgagaagtaccccaccatctaccacctgagaaagaaactggtggacagcaccgacaaggccgacctgcggctgatctatctggccctggcccacatgatcaagttccggggccacttcctgatcgagggcgacctgaaccccgacaacagcgacgtggacaagctgttcatccagctggtgcagacctacaaccagctgttcgaggaaaaccccatcaacgccagcggcgtggacgccaaggccatcctgtctgccagactgagcaagagcagacggctggaaaatctgatcgcccagctgcccggcgagaagaagaatggcctgttcggcaacctgattgccctgagcctgggcctgacccccaacttcaagagcaacttcgacctggccgaggatgccaaactgcagctgagcaaggacacctacgacgacgacctggacaacctgctggcccagatcggcgaccagtacgccgacctgtttctggccgccaagaacctgtccgacgccatcctgctgagcgacatcctgagagtgaacaccgagatcaccaaggcccccctgagcgcctctatgatcaagagatacgacgagcaccaccaggacctgaccctgctgaaagctctcgtgcggcagcagctgcctgagaagtacaaagagattttcttcgaccagagcaagaacggctacgccggctacatcgatggcggagccagccaggaagagttctacaagttcatcaagcccatcctggaaaagatggacggcaccgaggaactgctcgtgaagctgaacagagaggacctgctgcggaagcagcggaccttcgacaacggcagcatcccccaccagatccacctgggagagctgcacgccattctgcggcggcaggaagatttttacccattcctgaaggacaaccgggaaaagatcgagaagatcctgaccttccgcatcccctactacgtgggccctctggccaggggaaacagcagattcgcctggatgaccagaaagagcgaggaaaccatcaccccctggaacttcgaggaagtggtggacaagggcgccagcgcccagagcttcatcgagcggatgaccaacttcgataagaacctgcccaacgagaaggtgctgcccaagcacagcctgctgtacgagtacttcaccgtgtacaacgagctgaccaaagtgaaatacgtgaccgagggaatgagaaagcccgccttcctgagcggcgagcagaaaaaagccatcgtggacctgctgttcaagaccaaccggaaagtgaccgtgaagcagctgaaagaggactacttcaagaaaatcgagtgcttcgactccgtggaaatctccggcgtggaagatcggttcaacgcctccctgggcacataccacgatctgctgaaaattatcaaggacaaggacttcctggacaatgaggaaaacgaggacattctggaagatatcgtgctgaccctgacactgtttgaggacagagagatgatcgaggaacggctgaaaacctatgcccacctgttcgacgacaaagtgatgaagcagctgaagcggcggagatacaccggctggggcaggctgagccggaagctgatcaacggcatccgggacaagcagtccggcaagacaatcctggatttcctgaagtccgacggcttcgccaacagaaacttcatgcagctgatccacgacgacagcctgacctttaaagaggacatccagaaagcccaggtgtccggccagggcgatagcctgcacgagcacattgccaatctggccggcagccccgccattaagaagggcatcctgcagacagtgaaggtggtggacgagctcgtgaaagtgatgggccggcacaagcccgagaacatcgtgatcgaaatggccagagagaaccagaccacccagaagggacagaagaacagccgcgagagaatgaagcggatcgaagagggcatcaaagagctgggcagccagatcctgaaagaacaccccgtggaaaacacccagctgcagaacgagaagctgtacctgtactacctgcagaatgggcgggatatgtacgtggaccaggaactggacatcaaccggctgtccgactacgatgtggacgctatcgtgcctcagagctttctgaaggacgactccatcgataacaaagtgctgactcggagcgacaagaaccggggcaagagcgacaacgtgccctccgaagaggtcgtgaagaagatgaagaactactggcgccagctgctgaatgccaagctgattacccagaggaagttcgacaatctgaccaaggccgagagaggcggcctgagcgaactggataaggccggcttcatcaagagacagctggtggaaacccggcagatcacaaagcacgtggcacagatcctggactcccggatgaacactaagtacgacgagaacgacaaactgatccgggaagtgaaagtgatcaccctgaagtccaagctggtgtccgatttccggaaggatttccagttttacaaagtgcgcgagatcaacaactaccaccacgcccacgacgcctacctgaacgccgtcgtgggaaccgccctgatcaaaaagtaccctaagctggaaagcgagttcgtgtacggcgactacaaggtgtacgacgtgcggaagatgatcgccaagagcgagcaggaaatcggcaaggctaccgccaagtacttcttctacagcaacatcatgaactttttcaagaccgagattaccctggccaacggcgagatccggaagcggcctctgatcgagacaaacggcgaaacaggcgagatcgtgtgggataagggccgggactttgccaccgtgcggaaagtgctgtctatgccccaagtgaatatcgtgaaaaagaccgaggtgcagacaggcggcttcagcaaagagtctatcctgcccaagaggaacagcgacaagctgatcgccagaaagaaggactgggaccctaagaagtacggcggcttcgacagccccaccgtggcctattctgtgctggtggtggccaaagtggaaaagggcaagtccaagaaactgaagagtgtgaaagagctgctggggatcaccatcatggaaagaagcagcttcgagaagaatcccatcgactttctggaagccaagggctacaaagaagtgaaaaaggacctgatcatcaagctgcctaagtactccctgttcgagctggaaaacggccggaagagaatgctggcctctgccggcgaactgcagaagggaaacgaactggccctgccctccaaatatgtgaacttcctgtacctggccagccactatgagaagctgaagggctcccccgaggataatgagcagaaacagctgtttgtggaacagcacaaacactacctggacgagatcatcgagcagatcagcgagttctccaagagagtgatcctggccgacgctaatctggacaaggtgctgagcgcctacaacaagcacagagacaagcctatcagagagcaggccgagaatatcatccacctgtttaccctgaccaatctgggagcccctgccgccttcaagtactttgacaccaccatcgaccggaagaggtacaccagcaccaaagaggtgctggacgccaccctgatccaccagagcatcaccggcctgtacgagacacggatcgacctgtctcagctgggaggcgacgcctatccctatgacgtgcccgattatgccagcctgggcagcggctcccccaagaaaaaacgcaaggtggaagatcctaagaaaaagcggaaagtggacggcattggtagtgggagcaacggcagcagcggagaggaactgctgagcaagaactaccacctggaaaacgaggtggccagactgaagaaaggctctggctctggcggaagcggttctggcggatcaggatctggaagtggcggctctggaagcggaggttctggatctggcgaagaactgctgtctaagaattatcacctcgagaatgaagtcgctcgtttgaagaaaggttcaggctccggccagcggggaagcaagcgcaccgccgatggttccgagttcgaaagccccaaaaaaaagcgcaaggtctgagatcccaagcacgcagcaatgcagctcaaaacgcttagcctagccacacccccacgggaaacagcagtgattaacctttagcaataaacgaaagtttaactaagctatactaaccccagggttggtcaatttcgtgccagccacaccctggtactgcatgcacgcaatgctagctgcccctttcccgtcctgggcaccccgagtctcccccgaccccgggtcccaggtatgctcccacctccacctgccccactcaccacctctgctagttccagacacctccgagacgaggaaaaaaaaaaaaaaaaaaaaaaaaaaaaaaaaaaaaaaaaaaaaaaaaaaaaaaaaaaaaaaaaaaaaaaaaaaaaaaaaaaaaaaaaaaaaaaaaaaaaaaaaaaaaaaaaaaaaaaaaaaaaaaaaaaaaaaaaaaaaaaaaaaaaaaaaaaaaaaaaaaaaaaaaaaaaaaaaaaaaaaaaaaaaaaaaaaaaaaaaaaaaaaaaaaaaaaaaaaaaaaaaaaaaaaaaaaaaaaaaaaaaaaaaaaaaaaaaaaaaaaaaaaaaaaaaaaaaaaaaaaaaaaaaaaaaaaaaaaaaaaaaaaaaaaaaaaaaaaaaaaaaaaaaaaaaaaaaaaaaaaaaaaaaaaaaaaaaaaaaaaaaaaaaaaaaaaaaaaaaaaaaaaaaaaaaaaccgtcttcaagctttctagaaattcactggccgtcgttttacaacgtcgtgactgggaaaaccctggcgttacccaacttaatcgccttgcagcacatccccctttcgccagctggcgtaatagcgaagaggcccgcaccgatcgcccttcccaacagttgcgcagcctgaatggcgaatggcgcctgatgcggtattttctccttacgcatctgtgcggtatttcacaccgcatatggtgcactctcagtacaatctgctctgatgccgcatagttaagccagccccgacacccgccaacacccgctgacgcgccctgacgggcttgtctgctcccggcatccgcttacagacaagctgtgaccgtctccgggagctgcatgtgtcagaggttttcaccgtcatcaccgaaacgcgcgagacgaaagggcctcgtgatacgcctatttttataggttaatgtcatgataataatggtttcttagacgtcaggtggcacttttcggggaaatgtgcgcggaacccctatttgtttatttttctaaatacattcaaatatgtatccgctcatgagacaataaccctgataaatgcttcaataatattgaaaaaggaagagtatgagtattcaacatttccgtgtcgcccttattcccttttttgcggcattttgccttcctgtttttgctcacccagaaacgctggtgaaagtaaaagatgctgaagatcagttgggtgcacgagtgggttacatcgaactggatctcaacagcggtaagatccttgagagttttcgccccgaagaacgttttccaatgatgagcacttttaaagttctgctatgtggcgcggtattatcccgtattgacgccgggcaagagcaactcggtcgccgcatacactattctcagaatgacttggttgagtactcaccagtcacagaaaagcatcttacggatggcatgacagtaagagaattatgcagtgctgccataaccatgagtgataacactgcggccaacttacttctgacaacgatcggaggaccgaaggagctaaccgcttttttgcacaacatgggggatcatgtaactcgccttgatcgttgggaaccggagctgaatgaagccataccaaacgacgagcgtgacaccacgatgcctgtagcaatggcaacaacgttgcgcaaactattaactggcgaactacttactctagcttcccggcaacaattaatagactggatggaggcggataaagttgcaggaccacttctgcgctcggcccttccggctggctggtttattgctgataaatctggagccggtgagcgtgggtctcgcggtatcattgcagcactggggccagatggtaagccctcccgtatcgtagttatctacacgacggggagtcaggcaactatggatgaacgaaatagacagatcgctgagataggtgcctcactgattaagcattggtaactgtcagaccaagtttac

SEQ ID NO: 216 - DNA, 10929 bp, synthetic construct
  misc_feature 1..10929: note = DNA of V22_D3a-D3l-scFv-2a-1xGCN4-dCas9-KRAB
  source 1..10929: mol_type = other DNA
atcgtgctgaccctgacactgtttgaggacagagagatgatcgaggaacggctgaaaacctatgcccacctgttcgacgacaaagtgatgaagcagctgaagcggcggagatacaccggctggggcaggctgagccggaagctgatcaacggcatccgggacaagcagtccggcaagacaatcctggatttcctgaagtccgacggcttcgccaacagaaacttcatgcagctgatccacgacgacagcctgacctttaaagaggacatccagaaagcccaggtgtccggccagggcgatagcctgcacgagcacattgccaatctggccggcagccccgccattaagaagggcatcctgcagacagtgaaggtggtggacgagctcgtgaaagtgatgggccggcacaagcccgagaacatcgtgatcgaaatggccagagagaaccagaccacccagaagggacagaagaacagccgcgagagaatgaagcggatcgaagagggcatcaaagagctgggcagccagatcctgaaagaacaccccgtggaaaacacccagctgcagaacgagaagctgtacctgtactacctgcagaatgggcgggatatgtacgtggaccaggaactggacatcaaccggctgtccgactacgatgtggacgctatcgtgcctcagagctttctgaaggacgactccatcgataacaaagtgctgactcggagcgacaagaaccggggcaagagcgacaacgtgccctccgaagaggtcgtgaagaagatgaagaactactggcgccagctgctgaatgccaagctgattacccagaggaagttcgacaatctgaccaaggccgagagaggcggcctgagcgaactggataaggccggcttcatcaagagacagctggtggaaacccggcagatcacaaagcacgtggcacagatcctggactcccggatgaacactaagtacgacgagaacgacaaactgatccgggaagtgaaagtgatcaccctgaagtccaagctggtgtccgatttccggaaggatttccagttttacaaagtgcgcgagatcaacaactaccaccacgcccacgacgcctacctgaacgccgtcgtgggaaccgccctgatcaaaaagtaccctaagctggaaagcgagttcgtgtacggcgactacaaggtgtacgacgtgcggaagatgatcgccaagagcgagcaggaaatcggcaaggctaccgccaagtacttcttctacagcaacatcatgaactttttcaagaccgagattaccctggccaacggcgagatccggaagcggcctctgatcgagacaaacggcgaaacaggcgagatcgtgtgggataagggccgggactttgccaccgtgcggaaagtgctgtctatgccccaagtgaatatcgtgaaaaagaccgaggtgcagacaggcggcttcagcaaagagtctatcctgcccaagaggaacagcgacaagctgatcgccagaaagaaggactgggaccctaagaagtacggcggcttcgacagccccaccgtggcctattctgtgctggtggtggccaaagtggaaaagggcaagtccaagaaactgaagagtgtgaaagagctgctggggatcaccatcatggaaagaagcagcttcgagaagaatcccatcgactttctggaagccaagggctacaaagaagtgaaaaaggacctgatcatcaagctgcctaagtactccctgttcgagctggaaaacggccggaagagaatgctggcctctgccggcgaactgcagaagggaaacgaactggccctgccctccaaatatgtgaacttcctgtacctggccagccactatgagaagctgaagggctcccccgaggataatgagcagaaacagctgtttgtggaacagcacaaacactacctggacgagatcatcgagcagatcagcgagttctccaagagagtgatcctggccgacgctaatctggacaaggtgctgagcgcctacaacaagcacagagacaagcctatcagagagcaggccgagaatatcatccacctgtttaccctgaccaatctgggagcccctgccgccttcaagtactttgacaccaccatcgaccggaagaggtacaccagcaccaaagaggtgctggacgccaccctgatccaccagagcatcaccggcctgtacgagacacggatcgacctgtctcagctgggaggcgacgcctatccctatgacgtgcccgattatgccagcctgggcagcggctcccccaagaaaaaacgcaaggtggaagatcctaagaaaaagcggaaagtggacggcagcggcagcgagacccccggtaccagcgagagcgccacccccgagagccggacactggtgaccttcaaggatgtatttgtggacttcaccagggaggagtggaagctgctggacactgctcagcagatcgtgtacagaaatgtgatgctggagaactataagaacctggtttccttgggttatcagcttactaagccagatgtgatcctccggttggagaagggagaagagccctgagatcccaagcacgcagcaatgcagctcaaaacgcttagcctagccacacccccacgggaaacagcagtgattaacctttagcaataaacgaaagtttaactaagctatactaaccccagggttggtcaatttcgtgccagccacaccctggtactgcatgcacgcaatgctagctgcccctttcccgtcctgggcaccccgagtctcccccgaccccgggtcccaggtatgctcccacctccacctgccccactcaccacctctgctagttccagacacctccgagacgaggaaaaaaaaaaaaaaaaaaaaaaaaaaaaaaaaaaaaaaaaaaaaaaaaaaaaaaaaaaaaaaaaaaaaaaaaaaaaaaaaaaaaaaaaaaaaaaaaaaaaaaaaaaaaaaaaaaaaaaaaaaaaaaaaaaaaaaaaaaaaaaaaaaaaaaaaaaaaaaaaaaaaaaaaaaaaaaaaaaaaaaaaaaaaaaaaaaaaaaaaaaaaaaaaaaaaaaaaaaaaaaaaaaaaaaaaaaaaaaaaaaaaaaaaaaaaaaaaaaaaaaaaaaaaaaaaaaaaaaaaaaaaaaaaaaaaaaaaaaaaaaaaaaaaaaaaaaaaaaaaaaaaaaaaaaaaaaaaaaaaaaaaaaaaaaaaaaaaaaaaaaaaaaaaaaaaaaaaaaaaaaaaaaaaaaaaaaccgtcttcaagctttctagaaattcactggccgtcgttttacaacgtcgtgactgggaaaaccctggcgttacccaacttaatcgccttgcagcacatccccctttcgccagctggcgtaatagcgaagaggcccgcaccgatcgcccttcccaacagttgcgcagcctgaatggcgaatggcgcctgatgcggtattttctccttacgcatctgtgcggtatttcacaccgcatatggtgcactctcagtacaatctgctctgatgccgcatagttaagccagccccgacacccgccaacacccgctgacgcgccctgacgggcttgtctgctcccggcatccgcttacagacaagctgtgaccgtctccgggagctgcatgtgtcagaggttttcaccgtcatcaccgaaacgcgcgagacgaaagggcctcgtgatacgcctatttttataggttaatgtcatgataataatggtttcttagacgtcaggtggcacttttcggggaaatgtgcgcggaacccctatttgtttatttttctaaatacattcaaatatgtatccgctcatgagacaataaccctgataaatgcttcaataatattgaaaaaggaagagtatgagtattcaacatttccgtgtcgcccttattcccttttttgcggcattttgccttcctgtttttgctcacccagaaacgctggtgaaagtaaaagatgctgaagatcagttgggtgcacgagtgggttacatcgaactggatctcaacagcggtaagatccttgagagttttcgccccgaagaacgttttccaatgatgagcacttttaaagttctgctatgtggcgcggtattatcccgtattgacgccgggcaagagcaactcggtcgccgcatacactattctcagaatgacttggttgagtactcaccagtcacagaaaagcatcttacggatggcatgacagtaagagaattatgcagtgctgccataaccatgagtgataacactgcggccaacttacttctgacaacgatcggaggaccgaaggagctaaccgcttttttgcacaacatgggggatcatgtaactcgccttgatcgttgggaaccggagctgaatgaagccataccaaacgacgagcgtgacaccacgatgcctgtagcaatggcaacaacgttgcgcaaactattaactggcgaactacttactctagcttcccggcaacaattaatagactggatggaggcggataaagttgcaggaccacttctgcgctcggcccttccggctggctggtttattgctgataaatctggagccggtgagcgtgggtctcgcggtatcattgcagcactggggccagatggtaagccctcccgtatcgtagttatctacacgacggggagtcaggcaactatggatgaacgaaatagacagatcgctgagataggtgcctcactgattaagcattggtaactgtcagaccaagtttactcatatatactttagattgatttaaaacttcatttttaatttaaaaggatctaggtgaagatcctttttgataatctcatgaccaaaatcccttaacgtgagttttcgttccactgagcgtcagaccccgtagaaaagatcaaaggatcttcttgagatcctttttttctgcgcgtaatctgctgcttgcaaacaaaaaaaccaccgctaccagcggtggtttgtttgccggatcaagagctaccaactctttttccgaaggtaactggcttcagcagagcgcagataccaaatactgttcttctagtgtagccgtagttaggccaccacttcaagaactctgtagcaccgcctacatacctcgctctgctaatcctgttaccagtggctgctgccagtggcgataagtcgtgtcttaccgggttggactcaagacgatagttaccggataaggcgcagcggtcgggctgaacggggggttcgtgcacacagcccagcttggagcgaacgacctacaccgaactgagatacctacagcgtgagctatgagaaagcgccacgcttcccgaagggagaaaggcggacaggtatccggtaagcggcagggtcggaacaggagagcgcacgagggagcttccagggggaaacgcctggtatctttatagtcctgtcgggtttcgccacctctgacttgagcgtcgatttttgtgatgctcgtcaggggggcggagcctatggaaaaacgccagcaacgcggcctttttacggttcctggccttttgctggccttttgctcacatgttctttcctgcgttatcccctgattctgtggataaccgtattaccgcctttgagtgagctgataccgctcgccgcagccgaacgaccgagcgcagcgagtcagtgagcgaggaagcggaagagcgcccaatacgcaaaccgcctctccccgcgcgttggccgattcattaatgcagctggcacgacaggtttcccgactggaaagcgggcagtgagcgcaacgcaattaatgtgagttagctcactcattaggcaccccaggctttacactttatgcttccggctcgtatgttgtgtggaattgtgagcggataacaatttcacacaggaaacagctatgaccatgattacgcctctagaaagctttaatacgactcactataaggactcactatttgttttcgcgcccagttgcaaaaagtgtcgacatttgcttctgacacaactgtgttcactagcaacctcaaacagacaccgccaccatgcctgctgctaagagagtgaaactggatggatccaaccatgaccaggaatttgaccccccaaaggtttacccacctgtgccagctgagaagaggaagcccatccgcgtgctgtctctctttgatgggattgctacagggctcctggtgctgaaggacctgggcatccaagtggaccgctacattgcctccgaggtgtgtgaggactccatcacggtgggcatggtgcggcaccagggaaagatcatgtacgtcggggacgtccgcagcgtcacacagaagcatatccaggagtggggcccattcgacctggtgattggaggcagtccctgcaatgacctctccattgtcaaccctgcccgcaagggactttatgagggtactggccgcctcttctttgagttctaccgcctcctgcatgatgcgcggcccaaggagggagatgatcgccccttcttctggctctttgagaatgtggtggccatgggcgttagtgacaagagggacatctcgcgatttcttgagtctaaccccgtgatgattgacgccaaagaagtgtctgctgcacacagggcccgttacttctggggtaaccttcctggcatgaacaggcctttggcatccactgtgaatgataagctggagctgcaagagtgtctggagcacggcagaatagccaagttcagcaaagtgaggaccattaccaccaggtcaaactctataaagcagggcaaagaccagcatttccccgtgttcatgaacgagaaggaggacatcctgtggtgcactgaaatggaaagggtgtttggcttccccgtccactacacagacgtctccaacatgagccgcttggcgaggcagagactgctgggccgatcgtggagcgtgccggtcatccgccacctcttcgctccgctgaaggaatattttgcttgtgtgtctagcggcaatagtaacgctaacagccgcgggccgagcttcagcagcggcctggtgccgttaagcttgcgcggcagccatatgggccctatggagatatacaagacagtgtctgcatggaagagacagccagtgcgggtactgagcctcttcagaaacatcgacaaggtactaaagagtttgggcttcttggaaagcggttctggttctgggggaggaacgctgaagtacgtggaagatgtcacaaatgtcgtgaggagagacgtggagaaatggggcccctttgacctggtgtacggctcgacgcagcccctaggcagctcttgtgatcgctgtcccggctggtacatgttccagttccaccggatcctgcagtatgcgctgcctcgccaggagagtcagcggcccttcttctggatattcatggacaatctgctgctgactgaggatgaccaagagacaactacccgcttccttcagacagaggctgtgaccctccaggatgtccgtggcagagactaccagaatgctatgcgggtgtggagcaacattccagggctgaagagcaagcatgcgcccctgaccccaaaggaagaagagtatctgcaagcccaagtcagaagcaggagcaagctggacgccccgaaagttgacctcctggtgaagaactgccttctcccgctgagagagtacttcaagtatttttctcaaaactcacttcctcttggagggccgagctctggcgcacccccaccaagtggagggtctcctgccgggtccccaacatctactgaagaaggcaccagcgaatccgcaacgcccgagtcaggccctggtacctccacagaaccatctgaaggtagtgcgcctggttccccagctggaagccctacttccaccgaagaaggcacgtcaaccgaaccaagtgaaggatctgcccctgggaccagcactgaaccatctgagggccccgacatcgtgatgacccagagccccagcagcctgagcgccagcgtgggcgaccgcgtgaccatcacctgccgcagcagcaccggcgccgtgaccaccagcaactacgccagctgggtgcaggagaagcccggcaagctgttcaagggcctgatcggcggcaccaacaaccgcgcccccggcgtgcccagccgcttcagcggcagcctgatcggcgacaaggccaccctgaccatcagcagcctgcagcccgaggacttcgccacctacttctgcgccctgtggtacagcaaccactgggtgttcggccagggcaccaaggtggagctgaagcgcggcggcggcggcagcggcggcggcggcagcggcggcggcggcagcagcggcggcggcagcgaggtgaagctgctggagagcggcggcggcctggtgcagcccggcggcagcctgaagctgagctgcgccgtgagcggcttcagcctgaccgactacggcgtgaactgggtgcgccaggcccccggccgcggcctggagtggatcggcgtgatctggggcgacggcatcaccgactacaacagcgccctgaaggaccgcttcatcatcagcaaggacaacggcaagaacaccgtgtacctgcagatgagcaaggtgcgcagcgacgacaccgccctgtactactgcgtgaccggcctgttcgactactggggccagggcaccctggtgaccgtgagcagctacccatacgatgttccagattacgctggtggaggcggaggttctgggggaggaggtagtggcggtggtggttcaggaggcggcggaagcggaagcggagctactaacttcagcctgctgaagcaggctggagacgtggaggagaaccctggacctatgcctgctgctaagagagtgaaactggatggatccggctcaggcggatctggttcaggggaagaactcctctccaaaaactaccatctcgagaatgaggtcgcccgcctgaaaaaaggatcaggttccggtggttctggcagcggtggttcaggctcaggcagcggcggtagcggtagcggtggaagcggaagcggaccaaaaaagaagagaaaggtaatggacaagaagtacagcatcggcctggccatcggcaccaactctgtgggctgggccgtgatcaccgacgagtacaaggtgcccagcaagaaattcaaggtgctgggcaacaccgaccggcacagcatcaagaagaacctgatcggcgccctgctgttcgacagcggagaaacagccgaggccacccggctgaagagaaccgccagaagaagatacaccagacggaagaaccggatctgctatctgcaagagatcttcagcaacgagatggccaaggtggacgacagcttcttccacagactggaagagtccttcctggtggaagaggataagaagcacgagcggcaccccatcttcggcaacatcgtggacgaggtggcctaccacgagaagtaccccaccatctaccacctgagaaagaaactggtggacagcaccgacaaggccgacctgcggctgatctatctggccctggcccacatgatcaagttccggggccacttcctgatcgagggcgacctgaaccccgacaacagcgacgtggacaagctgttcatccagctggtgcagacctacaaccagctgttcgaggaaaaccccatcaacgccagcggcgtggacgccaaggccatcctgtctgccagactgagcaagagcagacggctggaaaatctgatcgcccagctgcccggcgagaagaagaatggcctgttcggcaacctgattgccctgagcctgggcctgacccccaacttcaagagcaacttcgacctggccgaggatgccaaactgcagctgagcaaggacacctacgacgacgacctggacaacctgctggcccagatcggcgaccagtacgccgacctgtttctggccgccaagaacctgtccgacgccatcctgctgagcgacatcctgagagtgaacaccgagatcaccaaggcccccctgagcgcctctatgatcaagagatacgacgagcaccaccaggacctgaccctgctgaaagctctcgtgcggcagcagctgcctgagaagtacaaagagattttcttcgaccagagcaagaacggctacgccggctacatcgatggcggagccagccaggaagagttctacaagttcatcaagcccatcctggaaaagatggacggcaccgaggaactgctcgtgaagctgaacagagaggacctgctgcggaagcagcggaccttcgacaacggcagcatcccccaccagatccacctgggagagctgcacgccattctgcggcggcaggaagatttttacccattcctgaaggacaaccgggaaaagatcgagaagatcctgaccttccgcatcccctactacgtgggccctctggccaggggaaacagcagattcgcctggatgaccagaaagagcgaggaaaccatcaccccctggaacttcgaggaagtggtggacaagggcgccagcgcccagagcttcatcgagcggatgaccaacttcgataagaacctgcccaacgagaaggtgctgcccaagcacagcctgctgtacgagtacttcaccgtgtacaacgagctgaccaaagtgaaatacgtgaccgagggaatgagaaagcccgccttcctgagcggcgagcagaaaaaagccatcgtggacctgctgttcaagaccaaccggaaagtgaccgtgaagcagctgaaagaggactacttcaagaaaatcgagtgcttcgactccgtggaaatctccggcgtggaagatcggttcaacgcctccctgggcacataccacgatctgctgaaaattatcaaggacaaggacttcctggacaatgaggaaaacgaggacattctggaagat

SEQ ID NO: 217 - DNA, 11043 bp, synthetic construct
  misc_feature 1..11043: note = DNA of V23_D3a-D3l-scFv-2a-2xGCN4-dCas9-KRAB
  source 1..11043: mol_type = other DNA
atcgtgctgaccctgacactgtttgaggacagagagatgatcgaggaacggctgaaaacctatgcccacctgttcgacgacaaagtgatgaagcagctgaagcggcggagatacaccggctggggcaggctgagccggaagctgatcaacggcatccgggacaagcagtccggcaagacaatcctggatttcctgaagtccgacggcttcgccaacagaaacttcatgcagctgatccacgacgacagcctgacctttaaagaggacatccagaaagcccaggtgtccggccagggcgatagcctgcacgagcacattgccaatctggccggcagccccgccattaagaagggcatcctgcagacagtgaaggtggtggacgagctcgtgaaagtgatgggccggcacaagcccgagaacatcgtgatcgaaatggccagagagaaccagaccacccagaagggacagaagaacagccgcgagagaatgaagcggatcgaagagggcatcaaagagctgggcagccagatcctgaaagaacaccccgtggaaaacacccagctgcagaacgagaagctgtacctgtactacctgcagaatgggcgggatatgtacgtggaccaggaactggacatcaaccggctgtccgactacgatgtggacgctatcgtgcctcagagctttctgaaggacgactccatcgataacaaagtgctgactcggagcgacaagaaccggggcaagagcgacaacgtgccctccgaagaggtcgtgaagaagatgaagaactactggcgccagctgctgaatgccaagctgattacccagaggaagttcgacaatctgaccaaggccgagagaggcggcctgagcgaactggataaggccggcttcatcaagagacagctggtggaaacccggcagatcacaaagcacgtggcacagatcctggactcccggatgaacactaagtacgacgagaacgacaaactgatccgggaagtgaaagtgatcaccctgaagtccaagctggtgtccgatttccggaaggatttccagttttacaaagtgcgcgagatcaacaactaccaccacgcccacgacgcctacctgaacgccgtcgtgggaaccgccctgatcaaaaagtaccctaagctggaaagcgagttcgtgtacggcgactacaaggtgtacgacgtgcggaagatgatcgccaagagcgagcaggaaatcggcaaggctaccgccaagtacttcttctacagcaacatcatgaactttttcaagaccgagattaccctggccaacggcgagatccggaagcggcctctgatcgagacaaacggcgaaacaggcgagatcgtgtgggataagggccgggactttgccaccgtgcggaaagtgctgtctatgccccaagtgaatatcgtgaaaaagaccgaggtgcagacaggcggcttcagcaaagagtctatcctgcccaagaggaacagcgacaagctgatcgccagaaagaaggactgggaccctaagaagtacggcggcttcgacagccccaccgtggcctattctgtgctggtggtggccaaagtggaaaagggcaagtccaagaaactgaagagtgtgaaagagctgctggggatcaccatcatggaaagaagcagcttcgagaagaatcccatcgactttctggaagccaagggctacaaagaagtgaaaaaggacctgatcatcaagctgcctaagtactccctgttcgagctggaaaacggccggaagagaatgctggcctctgccggcgaactgcagaagggaaacgaactggccctgccctccaaatatgtgaacttcctgtacctggccagccactatgagaagctgaagggctcccccgaggataatgagcagaaacagctgtttgtggaacagcacaaacactacctggacgagatcatcgagcagatcagcgagttctccaagagagtgatcctggccgacgctaatctggacaaggtgctgagcgcctacaacaagcacagagacaagcctatcagagagcaggccgagaatatcatccacctgtttaccctgaccaatctgggagcccctgccgccttcaagtactttgacaccaccatcgaccggaagaggtacaccagcaccaaagaggtgctggacgccaccctgatccaccagagcatcaccggcctgtacgagacacggatcgacctgtctcagctgggaggcgacgcctatccctatgacgtgcccgattatgccagcctgggcagcggctcccccaagaaaaaacgcaaggtggaagatcctaagaaaaagcggaaagtggacggcagcggcagcgagacccccggtaccagcgagagcgccacccccgagagccggacactggtgaccttcaaggatgtatttgtggacttcaccagggaggagtggaagctgctggacactgctcagcagatcgtgtacagaaatgtgatgctggagaactataagaacctggtttccttgggttatcagcttactaagccagatgtgatcctccggttggagaagggagaagagccctgagatcccaagcacgcagcaatgcagctcaaaacgcttagcctagccacacccccacgggaaacagcagtgattaacctttagcaataaacgaaagtttaactaagctatactaaccccagggttggtcaatttcgtgccagccacaccctggtactgcatgcacgcaatgctagctgcccctttcccgtcctgggcaccccgagtctcccccgaccccgggtcccaggtatgctcccacctccacctgccccactcaccacctctgctagttccagacacctccgagacgaggaaaaaaaaaaaaaaaaaaaaaaaaaaaaaaaaaaaaaaaaaaaaaaaaaaaaaaaaaaaaaaaaaaaaaaaaaaaaaaaaaaaaaaaaaaaaaaaaaaaaaaaaaaaaaaaaaaaaaaaaaaaaaaaaaaaaaaaaaaaaaaaaaaaaaaaaaaaaaaaaaaaaaaaaaaaaaaaaaaaaaaaaaaaaaaaaaaaaaaaaaaaaaaaaaaaaaaaaaaaaaaaaaaaaaaaaaaaaaaaaaaaaaaaaaaaaaaaaaaaaaaaaaaaaaaaaaaaaaaaaaaaaaaaaaaaaaaaaaaaaaaaaaaaaaaaaaaaaaaaaaaaaaaaaaaaaaaaaaaaaaaaaaaaaaaaaaaaaaaaaaaaaaaaaaaaaaaaaaaaaaaaaaaaaaaaaaaccgtcttcaagctttctagaaattcactggccgtcgttttacaacgtcgtgactgggaaaaccctggcgttacccaacttaatcgccttgcagcacatccccctttcgccagctggcgtaatagcgaagaggcccgcaccgatcgcccttcccaacagttgcgcagcctgaatggcgaatggcgcctgatgcggtattttctccttacgcatctgtgcggtatttcacaccgcatatggtgcactctcagtacaatctgctctgatgccgcatagttaagccagccccgacacccgccaacacccgctgacgcgccctgacgggcttgtctgctcccggcatccgcttacagacaagctgtgaccgtctccgggagctgcatgtgtcagaggttttcaccgtcatcaccgaaacgcgcgagacgaaagggcctcgtgatacgcctatttttataggttaatgtcatgataataatggtttcttagacgtcaggtggcacttttcggggaaatgtgcgcggaacccctatttgtttatttttctaaatacattcaaatatgtatccgctcatgagacaataaccctgataaatgcttcaataatattgaaaaaggaagagtatgagtattcaacatttccgtgtcgcccttattcccttttttgcggcattttgccttcctgtttttgctcacccagaaacgctggtgaaagtaaaagatgctgaagatcagttgggtgcacgagtgggttacatcgaactggatctcaacagcggtaagatccttgagagttttcgccccgaagaacgttttccaatgatgagcacttttaaagttctgctatgtggcgcggtattatcccgtattgacgccgggcaagagcaactcggtcgccgcatacactattctcagaatgacttggttgagtactcaccagtcacagaaaagcatcttacggatggcatgacagtaagagaattatgcagtgctgccataaccatgagtgataacactgcggccaacttacttctgacaacgatcggaggaccgaaggagctaaccgcttttttgcacaacatgggggatcatgtaactcgccttgatcgttgggaaccggagctgaatgaagccataccaaacgacgagcgtgacaccacgatgcctgtagcaatggcaacaacgttgcgcaaactattaactggcgaactacttactctagcttcccggcaacaattaatagactggatggaggcggataaagttgcaggaccacttctgcgctcggcccttccggctggctggtttattgctgataaatctggagccggtgagcgtgggtctcgcggtatcattgcagcactggggccagatggtaagccctcccgtatcgtagttatctacacgacggggagtcaggcaactatggatgaacgaaatagacagatcgctgagataggtgcctcactgattaagcattggtaactgtcagaccaagtttactcatatatactttagattgatttaaaacttcatttttaatttaaaaggatctaggtgaagatcctttttgataatctcatgaccaaaatcccttaacgtgagttttcgttccactgagcgtcagaccccgtagaaaagatcaaaggatcttcttgagatcctttttttctgcgcgtaatctgctgcttgcaaacaaaaaaaccaccgctaccagcggtggtttgtttgccggatcaagagctaccaactctttttccgaaggtaactggcttcagcagagcgcagataccaaatactgttcttctagtgtagccgtagttaggccaccacttcaagaactctgtagcaccgcctacatacctcgctctgctaatcctgttaccagtggctgctgccagtggcgataagtcgtgtcttaccgggttggactcaagacgatagttaccggataaggcgcagcggtcgggctgaacggggggttcgtgcacacagcccagcttggagcgaacgacctacaccgaactgagatacctacagcgtgagctatgagaaagcgccacgcttcccgaagggagaaaggcggacaggtatccggtaagcggcagggtcggaacaggagagcgcacgagggagcttccagggggaaacgcctggtatctttatagtcctgtcgggtttcgccacctctgacttgagcgtcgatttttgtgatgctcgtcaggggggcggagcctatggaaaaacgccagcaacgcggcctttttacggttcctggccttttgctggccttttgctcacatgttctttcctgcgttatcccctgattctgtggataaccgtattaccgcctttgagtgagctgataccgctcgccgcagccgaacgaccgagcgcagcgagtcagtgagcgaggaagcggaagagcgcccaatacgcaaaccgcctctccccgcgcgttggccgattcattaatgcagctggcacgacaggtttcccgactggaaagcgggcagtgagcgcaacgcaattaatgtgagttagctcactcattaggcaccccaggctttacactttatgcttccggctcgtatgttgtgtggaattgtgagcggataacaatttcacacaggaaacagctatgaccatgattacgcctctagaaagctttaatacgactcactataaggactcactatttgttttcgcgcccagttgcaaaaagtgtcgacatttgcttctgacacaactgtgttcactagcaacctcaaacagacaccgccaccatgcctgctgctaagagagtgaaactggatggatccaaccatgaccaggaatttgaccccccaaaggtttacccacctgtgccagctgagaagaggaagcccatccgcgtgctgtctctctttgatgggattgctacagggctcctggtgctgaaggacctgggcatccaagtggaccgctacattgcctccgaggtgtgtgaggactccatcacggtgggcatggtgcggcaccagggaaagatcatgtacgtcggggacgtccgcagcgtcacacagaagcatatccaggagtggggcccattcgacctggtgattggaggcagtccctgcaatgacctctccattgtcaaccctgcccgcaagggactttatgagggtactggccgcctcttctttgagttctaccgcctcctgcatgatgcgcggcccaaggagggagatgatcgccccttcttctggctctttgagaatgtggtggccatgggcgttagtgacaagagggacatctcgcgatttcttgagtctaaccccgtgatgattgacgccaaagaagtgtctgctgcacacagggcccgttacttctggggtaaccttcctggcatgaacaggcctttggcatccactgtgaatgataagctggagctgcaagagtgtctggagcacggcagaatagccaagttcagcaaagtgaggaccattaccaccaggtcaaactctataaagcagggcaaagaccagcatttccccgtgttcatgaacgagaaggaggacatcctgtggtgcactgaaatggaaagggtgtttggcttccccgtccactacacagacgtctccaacatgagccgcttggcgaggcagagactgctgggccgatcgtggagcgtgccggtcatccgccacctcttcgctccgctgaaggaatattttgcttgtgtgtctagcggcaatagtaacgctaacagccgcgggccgagcttcagcagcggcctggtgccgttaagcttgcgcggcagccatatgggccctatggagatatacaagacagtgtctgcatggaagagacagccagtgcgggtactgagcctcttcagaaacatcgacaaggtactaaagagtttgggcttcttggaaagcggttctggttctgggggaggaacgctgaagtacgtggaagatgtcacaaatgtcgtgaggagagacgtggagaaatggggcccctttgacctggtgtacggctcgacgcagcccctaggcagctcttgtgatcgctgtcccggctggtacatgttccagttccaccggatcctgcagtatgcgctgcctcgccaggagagtcagcggcccttcttctggatattcatggacaatctgctgctgactgaggatgaccaagagacaactacccgcttccttcagacagaggctgtgaccctccaggatgtccgtggcagagactaccagaatgctatgcgggtgtggagcaacattccagggctgaagagcaagcatgcgcccctgaccccaaaggaagaagagtatctgcaagcccaagtcagaagcaggagcaagctggacgccccgaaagttgacctcctggtgaagaactgccttctcccgctgagagagtacttcaagtatttttctcaaaactcacttcctcttggagggccgagctctggcgcacccccaccaagtggagggtctcctgccgggtccccaacatctactgaagaaggcaccagcgaatccgcaacgcccgagtcaggccctggtacctccacagaaccatctgaaggtagtgcgcctggttccccagctggaagccctacttccaccgaagaaggcacgtcaaccgaaccaagtgaaggatctgcccctgggaccagcactgaaccatctgagggccccgacatcgtgatgacccagagccccagcagcctgagcgccagcgtgggcgaccgcgtgaccatcacctgccgcagcagcaccggcgccgtgaccaccagcaactacgccagctgggtgcaggagaagcccggcaagctgttcaagggcctgatcggcggcaccaacaaccgcgcccccggcgtgcccagccgcttcagcggcagcctgatcggcgacaaggccaccctgaccatcagcagcctgcagcccgaggacttcgccacctacttctgcgccctgtggtacagcaaccactgggtgttcggccagggcaccaaggtggagctgaagcgcggcggcggcggcagcggcggcggcggcagcggcggcggcggcagcagcggcggcggcagcgaggtgaagctgctggagagcggcggcggcctggtgcagcccggcggcagcctgaagctgagctgcgccgtgagcggcttcagcctgaccgactacggcgtgaactgggtgcgccaggcccccggccgcggcctggagtggatcggcgtgatctggggcgacggcatcaccgactacaacagcgccctgaaggaccgcttcatcatcagcaaggacaacggcaagaacaccgtgtacctgcagatgagcaaggtgcgcagcgacgacaccgccctgtactactgcgtgaccggcctgttcgactactggggccagggcaccctggtgaccgtgagcagctacccatacgatgttccagattacgctggtggaggcggaggttctgggggaggaggtagtggcggtggtggttcaggaggcggcggaagcggaagcggagctactaacttcagcctgctgaagcaggctggagacgtggaggagaaccctggacctatgcctgctgctaagagagtgaaactggatggatccgaggaactgctgagcaagaactaccacctggaaaacgaggtggccagactgaagaaaggctctggctctggcggaagcggttctggcggatcaggatctggaagtggcggctctggaagcggaggttctggatctggcgaagaactgctgtctaagaattatcacctcgagaatgaggtcgcccgcctgaaaaaaggatcaggttccggtggttctggcagcggtggttcaggctcaggcagcggcggtagcggtagcggtggaagcggaagcggaccaaaaaagaagagaaaggtaatggacaagaagtacagcatcggcctggccatcggcaccaactctgtgggctgggccgtgatcaccgacgagtacaaggtgcccagcaagaaattcaaggtgctgggcaacaccgaccggcacagcatcaagaagaacctgatcggcgccctgctgttcgacagcggagaaacagccgaggccacccggctgaagagaaccgccagaagaagatacaccagacggaagaaccggatctgctatctgcaagagatcttcagcaacgagatggccaaggtggacgacagcttcttccacagactggaagagtccttcctggtggaagaggataagaagcacgagcggcaccccatcttcggcaacatcgtggacgaggtggcctaccacgagaagtaccccaccatctaccacctgagaaagaaactggtggacagcaccgacaaggccgacctgcggctgatctatctggccctggcccacatgatcaagttccggggccacttcctgatcgagggcgacctgaaccccgacaacagcgacgtggacaagctgttcatccagctggtgcagacctacaaccagctgttcgaggaaaaccccatcaacgccagcggcgtggacgccaaggccatcctgtctgccagactgagcaagagcagacggctggaaaatctgatcgcccagctgcccggcgagaagaagaatggcctgttcggcaacctgattgccctgagcctgggcctgacccccaacttcaagagcaacttcgacctggccgaggatgccaaactgcagctgagcaaggacacctacgacgacgacctggacaacctgctggcccagatcggcgaccagtacgccgacctgtttctggccgccaagaacctgtccgacgccatcctgctgagcgacatcctgagagtgaacaccgagatcaccaaggcccccctgagcgcctctatgatcaagagatacgacgagcaccaccaggacctgaccctgctgaaagctctcgtgcggcagcagctgcctgagaagtacaaagagattttcttcgaccagagcaagaacggctacgccggctacatcgatggcggagccagccaggaagagttctacaagttcatcaagcccatcctggaaaagatggacggcaccgaggaactgctcgtgaagctgaacagagaggacctgctgcggaagcagcggaccttcgacaacggcagcatcccccaccagatccacctgggagagctgcacgccattctgcggcggcaggaagatttttacccattcctgaaggacaaccgggaaaagatcgagaagatcctgaccttccgcatcccctactacgtgggccctctggccaggggaaacagcagattcgcctggatgaccagaaagagcgaggaaaccatcaccccctggaacttcgaggaagtggtggacaagggcgccagcgcccagagcttcatcgagcggatgaccaacttcgataagaacctgcccaacgagaaggtgctgcccaagcacagcctgctgtacgagtacttcaccgtgtacaacgagctgaccaaagtgaaatacgtgaccgagggaatgagaaagcccgccttcctgagcggcgagcagaaaaaagccatcgtggacctgctgttcaagaccaaccggaaagtgaccgtgaagcagctgaaagaggactacttcaagaaaatcgagtgcttcgactccgtggaaatctccggcgtggaagatcggttcaacgcctccctgggcacataccacgatctgctgaaaattatcaaggacaaggacttcctggacaatgaggaaaacgaggacattctggaagat

SEQ ID NO: 218 - DNA, 11181 bp, synthetic construct
  misc_feature 1..11181: note = DNA of V24_D3a-D3l-scFv-2a-3xGCN4-dCas9-KRAB
  source 1..11181: mol_type = other DNA
atcgtgctgaccctgacactgtttgaggacagagagatgatcgaggaacggctgaaaacctatgcccacctgttcgacgacaaagtgatgaagcagctgaagcggcggagatacaccggctggggcaggctgagccggaagctgatcaacggcatccgggacaagcagtccggcaagacaatcctggatttcctgaagtccgacggcttcgccaacagaaacttcatgcagctgatccacgacgacagcctgacctttaaagaggacatccagaaagcccaggtgtccggccagggcgatagcctgcacgagcacattgccaatctggccggcagccccgccattaagaagggcatcctgcagacagtgaaggtggtggacgagctcgtgaaagtgatgggccggcacaagcccgagaacatcgtgatcgaaatggccagagagaaccagaccacccagaagggacagaagaacagccgcgagagaatgaagcggatcgaagagggcatcaaagagctgggcagccagatcctgaaagaacaccccgtggaaaacacccagctgcagaacgagaagctgtacctgtactacctgcagaatgggcgggatatgtacgtggaccaggaactggacatcaaccggctgtccgactacgatgtggacgctatcgtgcctcagagctttctgaaggacgactccatcgataacaaagtgctgactcggagcgacaagaaccggggcaagagcgacaacgtgccctccgaagaggtcgtgaagaagatgaagaactactggcgccagctgctgaatgccaagctgattacccagaggaagttcgacaatctgaccaaggccgagagaggcggcctgagcgaactggataaggccggcttcatcaagagacagctggtggaaacccggcagatcacaaagcacgtggcacagatcctggactcccggatgaacactaagtacgacgagaacgacaaactgatccgggaagtgaaagtgatcaccctgaagtccaagctggtgtccgatttccggaaggatttccagttttacaaagtgcgcgagatcaacaactaccaccacgcccacgacgcctacctgaacgccgtcgtgggaaccgccctgatcaaaaagtaccctaagctggaaagcgagttcgtgtacggcgactacaaggtgtacgacgtgcggaagatgatcgccaagagcgagcaggaaatcggcaaggctaccgccaagtacttcttctacagcaacatcatgaactttttcaagaccgagattaccctggccaacggcgagatccggaagcggcctctgatcgagacaaacggcgaaacaggcgagatcgtgtgggataagggccgggactttgccaccgtgcggaaagtgctgtctatgccccaagtgaatatcgtgaaaaagaccgaggtgcagacaggcggcttcagcaaagagtctatcctgcccaagaggaacagcgacaagctgatcgccagaaagaaggactgggaccctaagaagtacggcggcttcgacagccccaccgtggcctattctgtgctggtggtggccaaagtggaaaagggcaagtccaagaaactgaagagtgtgaaagagctgctggggatcaccatcatggaaagaagcagcttcgagaagaatcccatcgactttctggaagccaagggctacaaagaagtgaaaaaggacctgatcatcaagctgcctaagtactccctgttcgagctggaaaacggccggaagagaatgctggcctctgccggcgaactgcagaagggaaacgaactggccctgccctccaaatatgtgaacttcctgtacctggccagccactatgagaagctgaagggctcccccgaggataatgagcagaaacagctgtttgtggaacagcacaaacactacctggacgagatcatcgagcagatcagcgagttctccaagagagtgatcctggccgacgctaatctggacaaggtgctgagcgcctacaacaagcacagagacaagcctatcagagagcaggccgagaatatcatccacctgtttaccctgaccaatctgggagcccctgccgccttcaagtactttgacaccaccatcgaccggaagaggtacaccagcaccaaagaggtgctggacgccaccctgatccaccagagcatcaccggcctgtacgagacacggatcgacctgtctcagctgggaggcgacgcctatccctatgacgtgcccgattatgccagcctgggcagcggctcccccaagaaaaaacgcaaggtggaagatcctaagaaaaagcggaaagtggacggcagcggcagcgagacccccggtaccagcgagagcgccacccccgagagccggacactggtgaccttcaaggatgtatttgtggacttcaccagggaggagtggaagctgctggacactgctcagcagatcgtgtacagaaatgtgatgctggagaactataagaacctggtttccttgggttatcagcttactaagccagatgtgatcctccggttggagaagggagaagagccctgagatcccaagcacgcagcaatgcagctcaaaacgcttagcctagccacacccccacgggaaacagcagtgattaacctttagcaataaacgaaagtttaactaagctatactaaccccagggttggtcaatttcgtgccagccacaccctggtactgcatgcacgcaatgctagctgcccctttcccgtcctgggcaccccgagtctcccccgaccccgggtcccaggtatgctcccacctccacctgccccactcaccacctctgctagttccagacacctccgagacgaggaaaaaaaaaaaaaaaaaaaaaaaaaaaaaaaaaaaaaaaaaaaaaaaaaaaaaaaaaaaaaaaaaaaaaaaaaaaaaaaaaaaaaaaaaaaaaaaaaaaaaaaaaaaaaaaaaaaaaaaaaaaaaaaaaaaaaaaaaaaaaaaaaaaaaaaaaaaaaaaaaaaaaaaaaaaaaaaaaaaaaaaaaaaaaaaaaaaaaaaaaaaaaaaaaaaaaaaaaaaaaaaaaaaaaaaaaaaaaaaaaaaaaaaaaaaaaaaaaaaaaaaaaaaaaaaaaaaaaaaaaaaaaaaaaaaaaaaaaaaaaaaaaaaaaaaaaaaaaaaaaaaaaaaaaaaaaaaaaaaaaaaaaaaaaaaaaaaaaaaaaaaaaaaaaaaaaaaaaaaaaaaaaaaaaaaaaaccgtcttcaagctttctagaaattcactggccgtcgttttacaacgtcgtgactgggaaaaccctggcgttacccaacttaatcgccttgcagcacatccccctttcgccagctggcgtaatagcgaagaggcccgcaccgatcgcccttcccaacagttgcgcagcctgaatggcgaatggcgcctgatgcggtattttctccttacgcatctgtgcggtatttcacaccgcatatggtgcactctcagtacaatctgctctgatgccgcatagttaagccagccccgacacccgccaacacccgctgacgcgccctgacgggcttgtctgctcccggcatccgcttacagacaagctgtgaccgtctccgggagctgcatgtgtcagaggttttcaccgtcatcaccgaaacgcgcgagacgaaagggcctcgtgatacgcctatttttataggttaatgtcatgataataatggtttcttagacgtcaggtggcacttttcggggaaatgtgcgcggaacccctatttgtttatttttctaaatacattcaaatatgtatccgctcatgagacaataaccctgataaatgcttcaataatattgaaaaaggaagagtatgagtattcaacatttccgtgtcgcccttattcccttttttgcggcattttgccttcctgtttttgctcacccagaaacgctggtgaaagtaaaagatgctgaagatcagttgggtgcacgagtgggttacatcgaactggatctcaacagcggtaagatccttgagagttttcgccccgaagaacgttttccaatgatgagcacttttaaagttctgctatgtggcgcggtattatcccgtattgacgccgggcaagagcaactcggtcgccgcatacactattctcagaatgacttggttgagtactcaccagtcacagaaaagcatcttacggatggcatgacagtaagagaattatgcagtgctgccataaccatgagtgataacactgcggccaacttacttctgacaacgatcggaggaccgaaggagctaaccgcttttttgcacaacatgggggatcatgtaactcgccttgatcgttgggaaccggagctgaatgaagccataccaaacgacgagcgtgacaccacgatgcctgtagcaatggcaacaacgttgcgcaaactattaactggcgaactacttactctagcttcccggcaacaattaatagactggatggaggcggataaagttgcaggaccacttctgcgctcggcccttccggctggctggtttattgctgataaatctggagccggtgagcgtgggtctcgcggtatcattgcagcactggggccagatggtaagccctcccgtatcgtagttatctacacgacggggagtcaggcaactatggatgaacgaaatagacagatcgctgagataggtgcctcactgattaagcattggtaactgtcagaccaagtttactcatatatactttagattgatttaaaacttcatttttaatttaaaaggatctaggtgaagatcctttttgataatctcatgaccaaaatcccttaacgtgagttttcgttccactgagcgtcagaccccgtagaaaagatcaaaggatcttcttgagatcctttttttctgcgcgtaatctgctgcttgcaaacaaaaaaaccaccgctaccagcggtggtttgtttgccggatcaagagctaccaactctttttccgaaggtaactggcttcagcagagcgcagataccaaatactgttcttctagtgtagccgtagttaggccaccacttcaagaactctgtagcaccgcctacatacctcgctctgctaatcctgttaccagtggctgctgccagtggcgataagtcgtgtcttaccgggttggactcaagacgatagttaccggataaggcgcagcggtcgggctgaacggggggttcgtgcacacagcccagcttggagcgaacgacctacaccgaactgagatacctacagcgtgagctatgagaaagcgccacgcttcccgaagggagaaaggcggacaggtatccggtaagcggcagggtcggaacaggagagcgcacgagggagcttccagggggaaacgcctggtatctttatagtcctgtcgggtttcgccacctctgacttgagcgtcgatttttgtgatgctcgtcaggggggcggagcctatggaaaaacgccagcaacgcggcctttttacggttcctggccttttgctggccttttgctcacatgttctttcctgcgttatcccctgattctgtggataaccgtattaccgcctttgagtgagctgataccgctcgccgcagccgaacgaccgagcgcagcgagtcagtgagcgaggaagcggaagagcgcccaatacgcaaaccgcctctccccgcgcgttggccgattcattaatgcagctggcacgacaggtttcccgactggaaagcgggcagtgagcgcaacgcaattaatgtgagttagctcactcattaggcaccccaggctttacactttatgcttccggctcgtatgttgtgtggaattgtgagcggataacaatttcacacaggaaacagctatgaccatgattacgcctctagaaagctttaatacgactcactataaggactcactatttgttttcgcgcccagttgcaaaaagtgtcgacatttgcttctgacacaactgtgttcactagcaacctcaaacagacaccgccaccatgcctgctgctaagagagtgaaactggatggatccaaccatgaccaggaatttgaccccccaaaggtttacccacctgtgccagctgagaagaggaagcccatccgcgtgctgtctctctttgatgggattgctacagggctcctggtgctgaaggacctgggcatccaagtggaccgctacattgcctccgaggtgtgtgaggactccatcacggtgggcatggtgcggcaccagggaaagatcatgtacgtcggggacgtccgcagcgtcacacagaagcatatccaggagtggggcccattcgacctggtgattggaggcagtccctgcaatgacctctccattgtcaaccctgcccgcaagggactttatgagggtactggccgcctcttctttgagttctaccgcctcctgcatgatgcgcggcccaaggagggagatgatcgccccttcttctggctctttgagaatgtggtggccatgggcgttagtgacaagagggacatctcgcgatttcttgagtctaaccccgtgatgattgacgccaaagaagtgtctgctgcacacagggcccgttacttctggggtaaccttcctggcatgaacaggcctttggcatccactgtgaatgataagctggagctgcaagagtgtctggagcacggcagaatagccaagttcagcaaagtgaggaccattaccaccaggtcaaactctataaagcagggcaaagaccagcatttccccgtgttcatgaacgagaaggaggacatcctgtggtgcactgaaatggaaagggtgtttggcttccccgtccactacacagacgtctccaacatgagccgcttggcgaggcagagactgctgggccgatcgtggagcgtgccggtcatccgccacctcttcgctccgctgaaggaatattttgcttgtgtgtctagcggcaatagtaacgctaacagccgcgggccgagcttcagcagcggcctggtgccgttaagcttgcgcggcagccatatgggccctatggagatatacaagacagtgtctgcatggaagagacagccagtgcgggtactgagcctcttcagaaacatcgacaaggtactaaagagtttgggcttcttggaaagcggttctggttctgggggaggaacgctgaagtacgtggaagatgtcacaaatgtcgtgaggagagacgtggagaaatggggcccctttgacctggtgtacggctcgacgcagcccctaggcagctcttgtgatcgctgtcccggctggtacatgttccagttccaccggatcctgcagtatgcgctgcctcgccaggagagtcagcggcccttcttctggatattcatggacaatctgctgctgactgaggatgaccaagagacaactacccgcttccttcagacagaggctgtgaccctccaggatgtccgtggcagagactaccagaatgctatgcgggtgtggagcaacattccagggctgaagagcaagcatgcgcccctgaccccaaaggaagaagagtatctgcaagcccaagtcagaagcaggagcaagctggacgccccgaaagttgacctcctggtgaagaactgccttctcccgctgagagagtacttcaagtatttttctcaaaactcacttcctcttggagggccgagctctggcgcacccccaccaagtggagggtctcctgccgggtccccaacatctactgaagaaggcaccagcgaatccgcaacgcccgagtcaggccctggtacctccacagaaccatctgaaggtagtgcgcctggttccccagctggaagccctacttccaccgaagaaggcacgtcaaccgaaccaagtgaaggatctgcccctgggaccagcactgaaccatctgagggccccgacatcgtgatgacccagagccccagcagcctgagcgccagcgtgggcgaccgcgtgaccatcacctgccgcagcagcaccggcgccgtgaccaccagcaactacgccagctgggtgcaggagaagcccggcaagctgttcaagggcctgatcggcggcaccaacaaccgcgcccccggcgtgcccagccgcttcagcggcagcctgatcggcgacaaggccaccctgaccatcagcagcctgcagcccgaggacttcgccacctacttctgcgccctgtggtacagcaaccactgggtgttcggccagggcaccaaggtggagctgaagcgcggcggcggcggcagcggcggcggcggcagcggcggcggcggcagcagcggcggcggcagcgaggtgaagctgctggagagcggcggcggcctggtgcagcccggcggcagcctgaagctgagctgcgccgtgagcggcttcagcctgaccgactacggcgtgaactgggtgcgccaggcccccggccgcggcctggagtggatcggcgtgatctggggcgacggcatcaccgactacaacagcgccctgaaggaccgcttcatcatcagcaaggacaacggcaagaacaccgtgtacctgcagatgagcaaggtgcgcagcgacgacaccgccctgtactactgcgtgaccggcctgttcgactactggggccagggcaccctggtgaccgtgagcagctacccatacgatgttccagattacgctggtggaggcggaggttctgggggaggaggtagtggcggtggtggttcaggaggcggcggaagcggaagcggagctactaacttcagcctgctgaagcaggctggagacgtggaggagaaccctggacctatgcctgctgctaagagagtgaaactggatggatccgaggaactgctgagcaagaactaccacctggaaaacgaggtggccagactgaagaaaggctctggctctggcggaagcggttctggcggatcaggatctggaagtggcggctctggaagcggaggttctggatctggcgaagaactgctgtctaagaattatcacctcgagaacgaagtggctcggctcaagaaaggcagtggcagcggaggaagtggatccggcggtagtggtagtggaagcggcggatccggctcaggcggatctggttcaggggaagaactcctctccaaaaactaccatctcgagaatgaggtcgcccgcctgaaaaaaggatcaggttccggtggttctggcagcggtggttcaggctcaggcagcggcggtagcggtagcggtggaagcggaagcggaccaaaaaagaagagaaaggtaatggacaagaagtacagcatcggcctggccatcggcaccaactctgtgggctgggccgtgatcaccgacgagtacaaggtgcccagcaagaaattcaaggtgctgggcaacaccgaccggcacagcatcaagaagaacctgatcggcgccctgctgttcgacagcggagaaacagccgaggccacccggctgaagagaaccgccagaagaagatacaccagacggaagaaccggatctgctatctgcaagagatcttcagcaacgagatggccaaggtggacgacagcttcttccacagactggaagagtccttcctggtggaagaggataagaagcacgagcggcaccccatcttcggcaacatcgtggacgaggtggcctaccacgagaagtaccccaccatctaccacctgagaaagaaactggtggacagcaccgacaaggccgacctgcggctgatctatctggccctggcccacatgatcaagttccggggccacttcctgatcgagggcgacctgaaccccgacaacagcgacgtggacaagctgttcatccagctggtgcagacctacaaccagctgttcgaggaaaaccccatcaacgccagcggcgtggacgccaaggccatcctgtctgccagactgagcaagagcagacggctggaaaatctgatcgcccagctgcccggcgagaagaagaatggcctgttcggcaacctgattgccctgagcctgggcctgacccccaacttcaagagcaacttcgacctggccgaggatgccaaactgcagctgagcaaggacacctacgacgacgacctggacaacctgctggcccagatcggcgaccagtacgccgacctgtttctggccgccaagaacctgtccgacgccatcctgctgagcgacatcctgagagtgaacaccgagatcaccaaggcccccctgagcgcctctatgatcaagagatacgacgagcaccaccaggacctgaccctgctgaaagctctcgtgcggcagcagctgcctgagaagtacaaagagattttcttcgaccagagcaagaacggctacgccggctacatcgatggcggagccagccaggaagagttctacaagttcatcaagcccatcctggaaaagatggacggcaccgaggaactgctcgtgaagctgaacagagaggacctgctgcggaagcagcggaccttcgacaacggcagcatcccccaccagatccacctgggagagctgcacgccattctgcggcggcaggaagatttttacccattcctgaaggacaaccgggaaaagatcgagaagatcctgaccttccgcatcccctactacgtgggccctctggccaggggaaacagcagattcgcctggatgaccagaaagagcgaggaaaccatcaccccctggaacttcgaggaagtggtggacaagggcgccagcgcccagagcttcatcgagcggatgaccaacttcgataagaacctgcccaacgagaaggtgctgcccaagcacagcctgctgtacgagtacttcaccgtgtacaacgagctgaccaaagtgaaatacgtgaccgagggaatgagaaagcccgccttcctgagcggcgagcagaaaaaagccatcgtggacctgctgttcaagaccaaccggaaagtgaccgtgaagcagctgaaagaggactacttcaagaaaatcgagtgcttcgactccgtggaaatctccggcgtggaagatcggttcaacgcctccctgggcacataccacgatctgctgaaaattatcaaggacaaggacttcctggacaatgaggaaaacgaggacattctggaagat

SEQ ID NO: 219 - DNA, 11457 bp, synthetic construct
  misc_feature 1..11457: note = DNA of V25_D3a-D3l-scFv-2a-5xGCN4-dCas9-KRAB
  source 1..11457: mol_type = other DNA
atcgtgctgaccctgacactgtttgaggacagagagatgatcgaggaacggctgaaaacctatgcccacctgttcgacgacaaagtgatgaagcagctgaagcggcggagatacaccggctggggcaggctgagccggaagctgatcaacggcatccgggacaagcagtccggcaagacaatcctggatttcctgaagtccgacggcttcgccaacagaaacttcatgcagctgatccacgacgacagcctgacctttaaagaggacatccagaaagcccaggtgtccggccagggcgatagcctgcacgagcacattgccaatctggccggcagccccgccattaagaagggcatcctgcagacagtgaaggtggtggacgagctcgtgaaagtgatgggccggcacaagcccgagaacatcgtgatcgaaatggccagagagaaccagaccacccagaagggacagaagaacagccgcgagagaatgaagcggatcgaagagggcatcaaagagctgggcagccagatcctgaaagaacaccccgtggaaaacacccagctgcagaacgagaagctgtacctgtactacctgcagaatgggcgggatatgtacgtggaccaggaactggacatcaaccggctgtccgactacgatgtggacgctatcgtgcctcagagctttctgaaggacgactccatcgataacaaagtgctgactcggagcgacaagaaccggggcaagagcgacaacgtgccctccgaagaggtcgtgaagaagatgaagaactactggcgccagctgctgaatgccaagctgattacccagaggaagttcgacaatctgaccaaggccgagagaggcggcctgagcgaactggataaggccggcttcatcaagagacagctggtggaaacccggcagatcacaaagcacgtggcacagatcctggactcccggatgaacactaagtacgacgagaacgacaaactgatccgggaagtgaaagtgatcaccctgaagtccaagctggtgtccgatttccggaaggatttccagttttacaaagtgcgcgagatcaacaactaccaccacgcccacgacgcctacctgaacgccgtcgtgggaaccgccctgatcaaaaagtaccctaagctggaaagcgagttcgtgtacggcgactacaaggtgtacgacgtgcggaagatgatcgccaagagcgagcaggaaatcggcaaggctaccgccaagtacttcttctacagcaacatcatgaactttttcaagaccgagattaccctggccaacggcgagatccggaagcggcctctgatcgagacaaacggcgaaacaggcgagatcgtgtgggataagggccgggactttgccaccgtgcggaaagtgctgtctatgccccaagtgaatatcgtgaaaaagaccgaggtgcagacaggcggcttcagcaaagagtctatcctgcccaagaggaacagcgacaagctgatcgccagaaagaaggactgggaccctaagaagtacggcggcttcgacagccccaccgtggcctattctgtgctggtggtggccaaagtggaaaagggcaagtccaagaaactgaagagtgtgaaagagctgctggggatcaccatcatggaaagaagcagcttcgagaagaatcccatcgactttctggaagccaagggctacaaagaagtgaaaaaggacctgatcatcaagctgcctaagtactccctgttcgagctggaaaacggccggaagagaatgctggcctctgccggcgaactgcagaagggaaacgaactggccctgccctccaaatatgtgaacttcctgtacctggccagccactatgagaagctgaagggctcccccgaggataatgagcagaaacagctgtttgtggaacagcacaaacactacctggacgagatcatcgagcagatcagcgagttctccaagagagtgatcctggccgacgctaatctggacaaggtgctgagcgcctacaacaagcacagagacaagcctatcagagagcaggccgagaatatcatccacctgtttaccctgaccaatctgggagcccctgccgccttcaagtactttgacaccaccatcgaccggaagaggtacaccagcaccaaagaggtgctggacgccaccctgatccaccagagcatcaccggcctgtacgagacacggatcgacctgtctcagctgggaggcgacgcctatccctatgacgtgcccgattatgccagcctgggcagcggctcccccaagaaaaaacgcaaggtggaagatcctaagaaaaagcggaaagtggacggcagcggcagcgagacccccggtaccagcgagagcgccacccccgagagccggacactggtgaccttcaaggatgtatttgtggacttcaccagggaggagtggaagctgctggacactgctcagcagatcgtgtacagaaatgtgatgctggagaactataagaacctggtttccttgggttatcagcttactaagccagatgtgatcctccggttggagaagggagaagagccctgagatcccaagcacgcagcaatgcagctcaaaacgcttagcctagccacacccccacgggaaacagcagtgattaacctttagcaataaacgaaagtttaactaagctatactaaccccagggttggtcaatttcgtgccagccacaccctggtactgcatgcacgcaatgctagctgcccctttcccgtcctgggcaccccgagtctcccccgaccccgggtcccaggtatgctcccacctccacctgccccactcaccacctctgctagttccagacacctccgagacgaggaaaaaaaaaaaaaaaaaaaaaaaaaaaaaaaaaaaaaaaaaaaaaaaaaaaaaaaaaaaaaaaaaaaaaaaaaaaaaaaaaaaaaaaaaaaaaaaaaaaaaaaaaaaaaaaaaaaaaaaaaaaaaaaaaaaaaaaaaaaaaaaaaaaaaaaaaaaaaaaaaaaaaaaaaaaaaaaaaaaaaaaaaaaaaaaaaaaaaaaaaaaaaaaaaaaaaaaaaaaaaaaaaaaaaaaaaaaaaaaaaaaaaaaaaaaaaaaaaaaaaaaaaaaaaaaaaaaaaaaaaaaaaaaaaaaaaaaaaaaaaaaaaaaaaaaaaaaaaaaaaaaaaaaaaaaaaaaaaaaaaaaaaaaaaaaaaaaaaaaaaaaaaaaaaaaaaaaaaaaaaaaaaaaaaaaaaaccgtcttcaagctttctagaaattcactggccgtcgttttacaacgtcgtgactgggaaaaccctggcgttacccaacttaatcgccttgcagcacatccccctttcgccagctggcgtaatagcgaagaggcccgcaccgatcgcccttcccaacagttgcgcagcctgaatggcgaatggcgcctgatgcggtattttctccttacgcatctgtgcggtatttcacaccgcatatggtgcactctcagtacaatctgctctgatgccgcatagttaagccagccccgacacccgccaacacccgctgacgcgccctgacgggcttgtctgctcccggcatccgcttacagacaagctgtgaccgtctccgggagctgcatgtgtcagaggttttcaccgtcatcaccgaaacgcgcgagacgaaagggcctcgtgatacgcctatttttataggttaatgtcatgataataatggtttcttagacgtcaggtggcacttttcggggaaatgtgcgcggaacccctatttgtttatttttctaaatacattcaaatatgtatccgctcatgagacaataaccctgataaatgcttcaataatattgaaaaaggaagagtatgagtattcaacatttccgtgtcgcccttattcccttttttgcggcattttgccttcctgtttttgctcacccagaaacgctggtgaaagtaaaagatgctgaagatcagttgggtgcacgagtgggttacatcgaactggatctcaacagcggtaagatccttgagagttttcgccccgaagaacgttttccaatgatgagcacttttaaagttctgctatgtggcgcggtattatcccgtattgacgccgggcaagagcaactcggtcgccgcatacactattctcagaatgacttggttgagtactcaccagtcacagaaaagcatcttacggatggcatgacagtaagagaattatgcagtgctgccataaccatgagtgataacactgcggccaacttacttctgacaacgatcggaggaccgaaggagctaaccgcttttttgcacaacatgggggatcatgtaactcgccttgatcgttgggaaccggagctgaatgaagccataccaaacgacgagcgtgacaccacgatgcctgtagcaatggcaacaacgttgcgcaaactattaactggcgaactacttactctagcttcccggcaacaattaatagactggatggaggcggataaagttgcaggaccacttctgcgctcggcccttccggctggctggtttattgctgataaatctggagccggtgagcgtgggtctcgcggtatcattgcagcactggggccagatggtaagccctcccgtatcgtagttatctacacgacggggagtcaggcaactatggatgaacgaaatagacagatcgctgagataggtgcctcactgattaagcattggtaactgtcagaccaagtttactcatatatactttagattgatttaaaacttcatttttaatttaaaaggatctaggtgaagatcctttttgataatctcatgaccaaaatcccttaacgtgagttttcgttccactgagcgtcagaccccgtagaaaagatcaaaggatcttcttgagatcctttttttctgcgcgtaatctgctgcttgcaaacaaaaaaaccaccgctaccagcggtggtttgtttgccggatcaagagctaccaactctttttccgaaggtaactggcttcagcagagcgcagataccaaatactgttcttctagtgtagccgtagttaggccaccacttcaagaactctgtagcaccgcctacatacctcgctctgctaatcctgttaccagtggctgctgccagtggcgataagtcgtgtcttaccgggttggactcaagacgatagttaccggataaggcgcagcggtcgggctgaacggggggttcgtgcacacagcccagcttggagcgaacgacctacaccgaactgagatacctacagcgtgagctatgagaaagcgccacgcttcccgaagggagaaaggcggacaggtatccggtaagcggcagggtcggaacaggagagcgcacgagggagcttccagggggaaacgcctggtatctttatagtcctgtcgggtttcgccacctctgacttgagcgtcgatttttgtgatgctcgtcaggggggcggagcctatggaaaaacgccagcaacgcggcctttttacggttcctggccttttgctggccttttgctcacatgttctttcctgcgttatcccctgattctgtggataaccgtattaccgcctttgagtgagctgataccgctcgccgcagccgaacgaccgagcgcagcgagtcagtgagcgaggaagcggaagagcgcccaatacgcaaaccgcctctccccgcgcgttggccgattcattaatgcagctggcacgacaggtttcccgactggaaagcgggcagtgagcgcaacgcaattaatgtgagttagctcactcattaggcaccccaggctttacactttatgcttccggctcgtatgttgtgtggaattgtgagcggataacaatttcacacaggaaacagctatgaccatgattacgcctctagaaagctttaatacgactcactataaggactcactatttgttttcgcgcccagttgcaaaaagtgtcgacatttgcttctgacacaactgtgttcactagcaacctcaaacagacaccgccaccatgcctgctgctaagagagtgaaactggatggatccaaccatgaccaggaatttgaccccccaaaggtttacccacctgtgccagctgagaagaggaagcccatccgcgtgctgtctctctttgatgggattgctacagggctcctggtgctgaaggacctgggcatccaagtggaccgctacattgcctccgaggtgtgtgaggactccatcacggtgggcatggtgcggcaccagggaaagatcatgtacgtcggggacgtccgcagcgtcacacagaagcatatccaggagtggggcccattcgacctggtgattggaggcagtccctgcaatgacctctccattgtcaaccctgcccgcaagggactttatgagggtactggccgcctcttctttgagttctaccgcctcctgcatgatgcgcggcccaaggagggagatgatcgccccttcttctggctctttgagaatgtggtggccatgggcgttagtgacaagagggacatctcgcgatttcttgagtctaaccccgtgatgattgacgccaaagaagtgtctgctgcacacagggcccgttacttctggggtaaccttcctggcatgaacaggcctttggcatccactgtgaatgataagctggagctgcaagagtgtctggagcacggcagaatagccaagttcagcaaagtgaggaccattaccaccaggtcaaactctataaagcagggcaaagaccagcatttccccgtgttcatgaacgagaaggaggacatcctgtggtgcactgaaatggaaagggtgtttggcttccccgtccactacacagacgtctccaacatgagccgcttggcgaggcagagactgctgggccgatcgtggagcgtgccggtcatccgccacctcttcgctccgctgaaggaatattttgcttgtgtgtctagcggcaatagtaacgctaacagccgcgggccgagcttcagcagcggcctggtgccgttaagcttgcgcggcagccatatgggccctatggagatatacaagacagtgtctgcatggaagagacagccagtgcgggtactgagcctcttcagaaacatcgacaaggtactaaagagtttgggcttcttggaaagcggttctggttctgggggaggaacgctgaagtacgtggaagatgtcacaaatgtcgtgaggagagacgtggagaaatggggcccctttgacctggtgtacggctcgacgcagcccctaggcagctcttgtgatcgctgtcccggctggtacatgttccagttccaccggatcctgcagtatgcgctgcctcgccaggagagtcagcggcccttcttctggatattcatggacaatctgctgctgactgaggatgaccaagagacaactacccgcttccttcagacagaggctgtgaccctccaggatgtccgtggcagagactaccagaatgctatgcgggtgtggagcaacattccagggctgaagagcaagcatgcgcccctgaccccaaaggaagaagagtatctgcaagcccaagtcagaagcaggagcaagctggacgccccgaaagttgacctcctggtgaagaactgccttctcccgctgagagagtacttcaagtatttttctcaaaactcacttcctcttggagggccgagctctggcgcacccccaccaagtggagggtctcctgccgggtccccaacatctactgaagaaggcaccagcgaatccgcaacgcccgagtcaggccctggtacctccacagaaccatctgaaggtagtgcgcctggttccccagctggaagccctacttccaccgaagaaggcacgtcaaccgaaccaagtgaaggatctgcccctgggaccagcactgaaccatctgagggccccgacatcgtgatgacccagagccccagcagcctgagcgccagcgtgggcgaccgcgtgaccatcacctgccgcagcagcaccggcgccgtgaccaccagcaactacgccagctgggtgcaggagaagcccggcaagctgttcaagggcctgatcggcggcaccaacaaccgcgcccccggcgtgcccagccgcttcagcggcagcctgatcggcgacaaggccaccctgaccatcagcagcctgcagcccgaggacttcgccacctacttctgcgccctgtggtacagcaaccactgggtgttcggccagggcaccaaggtggagctgaagcgcggcggcggcggcagcggcggcggcggcagcggcggcggcggcagcagcggcggcggcagcgaggtgaagctgctggagagcggcggcggcctggtgcagcccggcggcagcctgaagctgagctgcgccgtgagcggcttcagcctgaccgactacggcgtgaactgggtgcgccaggcccccggccgcggcctggagtggatcggcgtgatctggggcgacggcatcaccgactacaacagcgccctgaaggaccgcttcatcatcagcaaggacaacggcaagaacaccgtgtacctgcagatgagcaaggtgcgcagcgacgacaccgccctgtactactgcgtgaccggcctgttcgactactggggccagggcaccctggtgaccgtgagcagctacccatacgatgttccagattacgctggtggaggcggaggttctgggggaggaggtagtggcggtggtggttcaggaggcggcggaagcggaagcggagctactaacttcagcctgctgaagcaggctggagacgtggaggagaaccctggacctatgcctgctgctaagagagtgaaactggatggatccgaggaactgctgagcaagaactaccacctggaaaacgaggtggccagactgaagaaaggctctggctctggcggaagcggttctggcggatcaggatctggaagtggcggctctggaagcggaggttctggatctggcgaagaactgctgtctaagaattatcacctcgagaacgaggttgcacgcttgaagaaaggcagcggatcaggcggatctggcagcggtggatctggttctggatccggcggctccggtagtggtggaagtggctctggggaagaattgcttagcaagaattatcatcttgaaaatgaggttgccaggcttaaaaaaggcagtggctccggcggatccggaagcggaggcagcggatctggatctggtggttcaggatctggcggttctggtagcggggaagaactgttgagtaaaaactatcaccttgagaacgaggtcgcaaggttgaaaaaaggatccggctctggcggctccggaagtggcggatctggctccggtagcggaggatcaggatccggcggaagcggatcaggcgaggaactgctttccaaaaattaccacctcgagaatgaggtcgcccgcctgaaaaaaggatcaggttccggtggttctggcagcggtggttcaggctcaggcagcggcggtagcggtagcggtggaagcggaagcggaccaaaaaagaagagaaaggtaatggacaagaagtacagcatcggcctggccatcggcaccaactctgtgggctgggccgtgatcaccgacgagtacaaggtgcccagcaagaaattcaaggtgctgggcaacaccgaccggcacagcatcaagaagaacctgatcggcgccctgctgttcgacagcggagaaacagccgaggccacccggctgaagagaaccgccagaagaagatacaccagacggaagaaccggatctgctatctgcaagagatcttcagcaacgagatggccaaggtggacgacagcttcttccacagactggaagagtccttcctggtggaagaggataagaagcacgagcggcaccccatcttcggcaacatcgtggacgaggtggcctaccacgagaagtaccccaccatctaccacctgagaaagaaactggtggacagcaccgacaaggccgacctgcggctgatctatctggccctggcccacatgatcaagttccggggccacttcctgatcgagggcgacctgaaccccgacaacagcgacgtggacaagctgttcatccagctggtgcagacctacaaccagctgttcgaggaaaaccccatcaacgccagcggcgtggacgccaaggccatcctgtctgccagactgagcaagagcagacggctggaaaatctgatcgcccagctgcccggcgagaagaagaatggcctgttcggcaacctgattgccctgagcctgggcctgacccccaacttcaagagcaacttcgacctggccgaggatgccaaactgcagctgagcaaggacacctacgacgacgacctggacaacctgctggcccagatcggcgaccagtacgccgacctgtttctggccgccaagaacctgtccgacgccatcctgctgagcgacatcctgagagtgaacaccgagatcaccaaggcccccctgagcgcctctatgatcaagagatacgacgagcaccaccaggacctgaccctgctgaaagctctcgtgcggcagcagctgcctgagaagtacaaagagattttcttcgaccagagcaagaacggctacgccggctacatcgatggcggagccagccaggaagagttctacaagttcatcaagcccatcctggaaaagatggacggcaccgaggaactgctcgtgaagctgaacagagaggacctgctgcggaagcagcggaccttcgacaacggcagcatcccccaccagatccacctgggagagctgcacgccattctgcggcggcaggaagatttttacccattcctgaaggacaaccgggaaaagatcgagaagatcctgaccttccgcatcccctactacgtgggccctctggccaggggaaacagcagattcgcctggatgaccagaaagagcgaggaaaccatcaccccctggaacttcgaggaagtggtggacaagggcgccagcgcccagagcttcatcgagcggatgaccaacttcgataagaacctgcccaacgagaaggtgctgcccaagcacagcctgctgtacgagtacttcaccgtgtacaacgagctgaccaaagtgaaatacgtgaccgagggaatgagaaagcccgccttcctgagcggcgagcagaaaaaagccatcgtggacctgctgttcaagaccaaccggaaagtgaccgtgaagcagctgaaagaggactacttcaagaaaatcgagtgcttcgactccgtggaaatctccggcgtggaagatcggttcaacgcctccctgggcacataccacgatctgctgaaaattatcaaggacaaggacttcctggacaatgaggaaaacgaggacattctggaagat

SEQ ID NO: 220 - DNA, 11108 bp, synthetic construct
  misc_feature 1..11108: note = DNA of V26_D3a-hD3L-scFv-2a-3xGCN4-dCas9-ZIM3
  source 1..11108: mol_type = other DNA
gagatacctacagcgtgagctatgagaaagcgccacgcttcccgaagggagaaaggcggacaggtatccggtaagcggcagggtcggaacaggagagcgcacgagggagcttccagggggaaacgcctggtatctttatagtcctgtcgggtttcgccacctctgacttgagcgtcgatttttgtgatgctcgtcaggggggcggagcctatggaaaaacgccagcaacgcggcctttttacggttcctggccttttgctggccttttgctcacatgttctttcctgcgttatcccctgattctgtggataaccgtattaccgcctttgagtgagctgataccgctcgccgcagccgaacgaccgagcgcagcgagtcagtgagcgaggaagcggaagagcgcccaatacgcaaaccgcctctccccgcgcgttggccgattcattaatgcagctggcacgacaggtttcccgactggaaagcgggcagtgagcgcaacgcaattaatgtgagttagctcactcattaggcaccccaggctttacactttatgcttccggctcgtatgttgtgtggaattgtgagcggataacaatttcacacaggaaacagctatgaccatgattacgcctctagaaagctttaatacgactcactataaggactcactatttgttttcgcgcccagttgcaaaaagtgtcgacatttgcttctgacacaactgtgttcactagcaacctcaaacagacaccgccaccatgcctgctgctaagagagtgaaactggatggatccaaccatgaccaggaatttgaccccccaaaggtttacccacctgtgccagctgagaagaggaagcccatccgcgtgctgtctctctttgatgggattgctacagggctcctggtgctgaaggacctgggcatccaagtggaccgctacattgcctccgaggtgtgtgaggactccatcacggtgggcatggtgcggcaccagggaaagatcatgtacgtcggggacgtccgcagcgtcacacagaagcatatccaggagtggggcccattcgacctggtgattggaggcagtccctgcaatgacctctccattgtcaaccctgcccgcaagggactttatgagggtactggccgcctcttctttgagttctaccgcctcctgcatgatgcgcggcccaaggagggagatgatcgccccttcttctggctctttgagaatgtggtggccatgggcgttagtgacaagagggacatctcgcgatttcttgagtctaaccccgtgatgattgacgccaaagaagtgtctgctgcacacagggcccgttacttctggggtaaccttcctggcatgaacaggcctttggcatccactgtgaatgataagctggagctgcaagagtgtctggagcacggcagaatagccaagttcagcaaagtgaggaccattaccaccaggtcaaactctataaagcagggcaaagaccagcatttccccgtgttcatgaacgagaaggaggacatcctgtggtgcactgaaatggaaagggtgtttggcttccccgtccactacacagacgtctccaacatgagccgcttggcgaggcagagactgctgggccgatcgtggagcgtgccggtcatccgccacctcttcgctccgctgaaggaatattttgcttgtgtgtctagcggcaatagtaacgctaacagccgcgggccgagcttcagcagcggcctggtgccgttaagcttgcgcggcagccatatgttcgaaaccgtgcctgtgtggaggagacagccagtccgggtgctgtccctttttgaagacatcaagaaagagctgacgagtttgggctttttggaaagtggttctgacccgggacaactgaagcatgtggttgatgtcacagacacagtgaggaaggatgtggaggagtggggacccttcgatcttgtgtacggcgccacacctcccctgggccacacctgtgaccgtcctcccagctggtacctgttccagttccaccggctcctgcagtacgcacggcccaagccaggcagccccaggcccttcttctggatgttcgtggacaatctggtgctgaacaaggaagacctggacgtcgcatctcgcttcctggagatggagccagtcaccatcccagatgtccacggcggatccttgcagaatgctgtccgcgtgtggagcaacatcccagccataaggagcagcaggcactgggctctggtttcggaagaagaattgtccctgctggcccagaacaagcagagctcgaagctcgcggccaagtggcccaccaagctggtgaagaactgctttctccccctaagagaatatttcaagtatttttcaggagggccgagctctggcgcacccccaccaagtggagggtctcctgccgggtccccaacatctactgaagaaggcaccagcgaatccgcaacgcccgagtcaggccctggtacctccacagaaccatctgaaggtagtgcgcctggttccccagctggaagccctacttccaccgaagaaggcacgtcaaccgaaccaagtgaaggatctgcccctgggaccagcactgaaccatctgagccaaaaaagaagagaaaggtaccatctgagggccccgacatcgtgatgacccagagccccagcagcctgagcgccagcgtgggcgaccgcgtgaccatcacctgccgcagcagcaccggcgccgtgaccaccagcaactacgccagctgggtgcaggagaagcccggcaagctgttcaagggcctgatcggcggcaccaacaaccgcgcccccggcgtgcccagccgcttcagcggcagcctgatcggcgacaaggccaccctgaccatcagcagcctgcagcccgaggacttcgccacctacttctgcgccctgtggtacagcaaccactgggtgttcggccagggcaccaaggtggagctgaagcgcggcggcggcggcagcggcggcggcggcagcggcggcggcggcagcagcggcggcggcagcgaggtgaagctgctggagagcggcggcggcctggtgcagcccggcggcagcctgaagctgagctgcgccgtgagcggcttcagcctgaccgactacggcgtgaactgggtgcgccaggcccccggccgcggcctggagtggatcggcgtgatctggggcgacggcatcaccgactacaacagcgccctgaaggaccgcttcatcatcagcaaggacaacggcaagaacaccgtgtacctgcagatgagcaaggtgcgcagcgacgacaccgccctgtactactgcgtgaccggcctgttcgactactggggccagggcaccctggtgaccgtgagcagctacccatacgatgttccagattacgctggtggaggcggaggttctgggggaggaggtagtggcggtggtggttcaggaggcggcggaagcggaagcggagctactaacttcagcctgctgaagcaggctggagacgtggaggagaaccctggacctatgcctgctgctaagagagtgaaactggatggatccgaggaactgctgagcaagaactaccacctggaaaacgaggtggccagactgaagaaaggctctggctctggcggaagcggttctggcggatcaggatctggaagtggcggctctggaagcggaggttctggatctggcgaagaactgctgtctaagaattatcacctcgagaacgaagtggctcggctcaagaaaggcagtggcagcggaggaagtggatccggcggtagtggtagtggaagcggcggatccggctcaggcggatctggttcaggggaagaactcctctccaaaaactaccatctcgagaatgaggtcgcccgcctgaaaaaaggatcaggttccggtggttctggcagcggtggttcaggctcaggcagcggcggtagcggtagcggtggaagcggaagcggaccaaaaaagaagagaaaggtaatggacaagaagtacagcatcggcctggccatcggcaccaactctgtgggctgggccgtgatcaccgacgagtacaaggtgcccagcaagaaattcaaggtgctgggcaacaccgaccggcacagcatcaagaagaacctgatcggcgccctgctgttcgacagcggagaaacagccgaggccacccggctgaagagaaccgccagaagaagatacaccagacggaagaaccggatctgctatctgcaagagatcttcagcaacgagatggccaaggtggacgacagcttcttccacagactggaagagtccttcctggtggaagaggataagaagcacgagcggcaccccatcttcggcaacatcgtggacgaggtggcctaccacgagaagtaccccaccatctaccacctgagaaagaaactggtggacagcaccgacaaggccgacctgcggctgatctatctggccctggcccacatgatcaagttccggggccacttcctgatcgagggcgacctgaaccccgacaacagcgacgtggacaagctgttcatccagctggtgcagacctacaaccagctgttcgaggaaaaccccatcaacgccagcggcgtggacgccaaggccatcctgtctgccagactgagcaagagcagacggctggaaaatctgatcgcccagctgcccggcgagaagaagaatggcctgttcggcaacctgattgccctgagcctgggcctgacccccaacttcaagagcaacttcgacctggccgaggatgccaaactgcagctgagcaaggacacctacgacgacgacctggacaacctgctggcccagatcggcgaccagtacgccgacctgtttctggccgccaagaacctgtccgacgccatcctgctgagcgacatcctgagagtgaacaccgagatcaccaaggcccccctgagcgcctctatgatcaagagatacgacgagcaccaccaggacctgaccctgctgaaagctctcgtgcggcagcagctgcctgagaagtacaaagagattttcttcgaccagagcaagaacggctacgccggctacatcgatggcggagccagccaggaagagttctacaagttcatcaagcccatcctggaaaagatggacggcaccgaggaactgctcgtgaagctgaacagagaggacctgctgcggaagcagcggaccttcgacaacggcagcatcccccaccagatccacctgggagagctgcacgccattctgcggcggcaggaagatttttacccattcctgaaggacaaccgggaaaagatcgagaagatcctgaccttccgcatcccctactacgtgggccctctggccaggggaaacagcagattcgcctggatgaccagaaagagcgaggaaaccatcaccccctggaacttcgaggaagtggtggacaagggcgccagcgcccagagcttcatcgagcggatgaccaacttcgataagaacctgcccaacgagaaggtgctgcccaagcacagcctgctgtacgagtacttcaccgtgtacaacgagctgaccaaagtgaaatacgtgaccgagggaatgagaaagcccgccttcctgagcggcgagcagaaaaaagccatcgtggacctgctgttcaagaccaaccggaaagtgaccgtgaagcagctgaaagaggactacttcaagaaaatcgagtgcttcgactccgtggaaatctccggcgtggaagatcggttcaacgcctccctgggcacataccacgatctgctgaaaattatcaaggacaaggacttcctggacaatgaggaaaacgaggacattctggaagatatcgtgctgaccctgacactgtttgaggacagagagatgatcgaggaacggctgaaaacctatgcccacctgttcgacgacaaagtgatgaagcagctgaagcggcggagatacaccggctggggcaggctgagccggaagctgatcaacggcatccgggacaagcagtccggcaagacaatcctggatttcctgaagtccgacggcttcgccaacagaaacttcatgcagctgatccacgacgacagcctgacctttaaagaggacatccagaaagcccaggtgtccggccagggcgatagcctgcacgagcacattgccaatctggccggcagccccgccattaagaagggcatcctgcagacagtgaaggtggtggacgagctcgtgaaagtgatgggccggcacaagcccgagaacatcgtgatcgaaatggccagagagaaccagaccacccagaagggacagaagaacagccgcgagagaatgaagcggatcgaagagggcatcaaagagctgggcagccagatcctgaaagaacaccccgtggaaaacacccagctgcagaacgagaagctgtacctgtactacctgcagaatgggcgggatatgtacgtggaccaggaactggacatcaaccggctgtccgactacgatgtggacgctatcgtgcctcagagctttctgaaggacgactccatcgataacaaagtgctgactcggagcgacaagaaccggggcaagagcgacaacgtgccctccgaagaggtcgtgaagaagatgaagaactactggcgccagctgctgaatgccaagctgattacccagaggaagttcgacaatctgaccaaggccgagagaggcggcctgagcgaactggataaggccggcttcatcaagagacagctggtggaaacccggcagatcacaaagcacgtggcacagatcctggactcccggatgaacactaagtacgacgagaacgacaaactgatccgggaagtgaaagtgatcaccctgaagtccaagctggtgtccgatttccggaaggatttccagttttacaaagtgcgcgagatcaacaactaccaccacgcccacgacgcctacctgaacgccgtcgtgggaaccgccctgatcaaaaagtaccctaagctggaaagcgagttcgtgtacggcgactacaaggtgtacgacgtgcggaagatgatcgccaagagcgagcaggaaatcggcaaggctaccgccaagtacttcttctacagcaacatcatgaactttttcaagaccgagattaccctggccaacggcgagatccggaagcggcctctgatcgagacaaacggcgaaacaggcgagatcgtgtgggataagggccgggactttgccaccgtgcggaaagtgctgtctatgccccaagtgaatatcgtgaaaaagaccgaggtgcagacaggcggcttcagcaaagagtctatcctgcccaagaggaacagcgacaagctgatcgccagaaagaaggactgggaccctaagaagtacggcggcttcgacagccccaccgtggcctattctgtgctggtggtggccaaagtggaaaagggcaagtccaagaaactgaagagtgtgaaagagctgctggggatcaccatcatggaaagaagcagcttcgagaagaatcccatcgactttctggaagccaagggctacaaagaagtgaaaaaggacctgatcatcaagctgcctaagtactccctgttcgagctggaaaacggccggaagagaatgctggcctctgccggcgaactgcagaagggaaacgaactggccctgccctccaaatatgtgaacttcctgtacctggccagccactatgagaagctgaagggctcccccgaggataatgagcagaaacagctgtttgtggaacagcacaaacactacctggacgagatcatcgagcagatcagcgagttctccaagagagtgatcctggccgacgctaatctggacaaggtgctgagcgcctacaacaagcacagagacaagcctatcagagagcaggccgagaatatcatccacctgtttaccctgaccaatctgggagcccctgccgccttcaagtactttgacaccaccatcgaccggaagaggtacaccagcaccaaagaggtgctggacgccaccctgatccaccagagcatcaccggcctgtacgagacacggatcgacctgtctcagctgggaggcgacgcctatccctatgacgtgcccgattatgccagcctgggcagcggctcccccaagaaaaaacgcaaggtggaagatcctaagaaaaagcggaaagtggacggcagcggcagcgagacccccggtaccagcgagagcgccacccccgagagcatgaacaattcccagggaagagtgaccttcgaggatgtcactgtgaacttcacccagggggagtggcagcggctgaatcccgaacagagaaacttgtacagggatgtgatgctggagaattacagcaaccttgtctctgtgggacaaggggaaaccaccaaacccgatgtgatcttgaggttggaacaaggaaaggagccatggttggaggaagaggaagtgctgggaagtggccgtgcagaaaaaaatggggacattggagggcagatttggaagccaaaggatgtgaaagagagtctcctcgagtgataatagggatcccaagcacgcagcaatgcagctcaaaacgcttagcctagccacacccccacgggaaacagcagtgattaacctttagcaataaacgaaagtttaactaagctatactaaccccagggttggtcaatttcgtgccagccacaccctggtactgcatgcacgcaatgctagctgcccctttcccgtcctgggcaccccgagtctcccccgaccccgggtcccaggtatgctcccacctccacctgccccactcaccacctctgctagttccagacacctccgagacgaggaaaaaaaaaaaaaaaaaaaaaaaaaaaaaaaaaaaaaaaaaaaaaaaaaaaaaaaaaaaaaaaaaaaaaaaaaaaaaaaaaaaaaaaaaaaaaaaaaaaaaaaaaaaaaaaaaaaaaaaaaaaaaaaaaaaaaaaaaaaaaaaaaaaaaaaaaaaaaaaaaaaaaaaaaaaaaaaaaaaaaaaaaaaaaaaaaaaaaaaaccgtcttcaagctttctagaaattcactggccgtcgttttacaacgtcgtgactgggaaaaccctggcgttacccaacttaatcgccttgcagcacatccccctttcgccagctggcgtaatagcgaagaggcccgcaccgatcgcccttcccaacagttgcgcagcctgaatggcgaatggcgcctgatgcggtattttctccttacgcatctgtgcggtatttcacaccgcatatggtgcactctcagtacaatctgctctgatgccgcatagttaagccagccccgacacccgccaacacccgctgacgcgccctgacgggcttgtctgctcccggcatccgcttacagacaagctgtgaccgtctccgggagctgcatgtgtcagaggttttcaccgtcatcaccgaaacgcgcgagacgaaagggcctcgtgatacgcctatttttataggttaatgtcatgataataatggtttcttagacgtcaggtggcacttttcggggaaatgtgcgcggaacccctatttgtttatttttctaaatacattcaaatatgtatccgctcatgagacaataaccctgataaatgcttcaataatattgaaaaaggaagagtatgagtattcaacatttccgtgtcgcccttattcccttttttgcggcattttgccttcctgtttttgctcacccagaaacgctggtgaaagtaaaagatgctgaagatcagttgggtgcacgagtgggttacatcgaactggatctcaacagcggtaagatccttgagagttttcgccccgaagaacgttttccaatgatgagcacttttaaagttctgctatgtggcgcggtattatcccgtattgacgccgggcaagagcaactcggtcgccgcatacactattctcagaatgacttggttgagtactcaccagtcacagaaaagcatcttacggatggcatgacagtaagagaattatgcagtgctgccataaccatgagtgataacactgcggccaacttacttctgacaacgatcggaggaccgaaggagctaaccgcttttttgcacaacatgggggatcatgtaactcgccttgatcgttgggaaccggagctgaatgaagccataccaaacgacgagcgtgacaccacgatgcctgtagcaatggcaacaacgttgcgcaaactattaactggcgaactacttactctagcttcccggcaacaattaatagactggatggaggcggataaagttgcaggaccacttctgcgctcggcccttccggctggctggtttattgctgataaatctggagccggtgagcgtgggtctcgcggtatcattgcagcactggggccagatggtaagccctcccgtatcgtagttatctacacgacggggagtcaggcaactatggatgaacgaaatagacagatcgctgagataggtgcctcactgattaagcattggtaactgtcagaccaagtttactcatatatactttagattgatttaaaacttcatttttaatttaaaaggatctaggtgaagatcctttttgataatctcatgaccaaaatcccttaacgtgagttttcgttccactgagcgtcagaccccgtagaaaagatcaaaggatcttcttgagatcctttttttctgcgcgtaatctgctgcttgcaaacaaaaaaaccaccgctaccagcggtggtttgtttgccggatcaagagctaccaactctttttccgaaggtaactggcttcagcagagcgcagataccaaatactgttcttctagtgtagccgtagttaggccaccacttcaagaactctgtagcaccgcctacatacctcgctctgctaatcctgttaccagtggctgctgccagtggcgataagtcgtgtcttaccgggttggactcaagacgatagttaccggataaggcgcagcggtcgggctgaacggggggttcgtgcacacagcccagcttggagcgaacgacctacaccgaact

SEQ ID NO: 221 - DNA, 11301 bp, synthetic construct
  misc_feature 1..11301: note = DNA of V27_3xGCN4-dCas9-ZIM3-2a-D3a-hD3L-scFv
  source 1..11301: mol_type = other DNA
tgagataggtgcctcactgattaagcattggtaactgtcagaccaagtttactcatatatactttagattgatttaaaacttcatttttaatttaaaaggatctaggtgaagatcctttttgataatctcatgaccaaaatcccttaacgtgagttttcgttccactgagcgtcagaccccgtagaaaagatcaaaggatcttcttgagatcctttttttctgcgcgtaatctgctgcttgcaaacaaaaaaaccaccgctaccagcggtggtttgtttgccggatcaagagctaccaactctttttccgaaggtaactggcttcagcagagcgcagataccaaatactgttcttctagtgtagccgtagttaggccaccacttcaagaactctgtagcaccgcctacatacctcgctctgctaatcctgttaccagtggctgctgccagtggcgataagtcgtgtcttaccgggttggactcaagacgatagttaccggataaggcgcagcggtcgggctgaacggggggttcgtgcacacagcccagcttggagcgaacgacctacaccgaactgagatacctacagcgtgagctatgagaaagcgccacgcttcccgaagggagaaaggcggacaggtatccggtaagcggcagggtcggaacaggagagcgcacgagggagcttccagggggaaacgcctggtatctttatagtcctgtcgggtttcgccacctctgacttgagcgtcgatttttgtgatgctcgtcaggggggcggagcctatggaaaaacgccagcaacgcggcctttttacggttcctggccttttgctggccttttgctcacatgttctttcctgcgttatcccctgattctgtggataaccgtattaccgcctttgagtgagctgataccgctcgccgcagccgaacgaccgagcgcagcgagtcagtgagcgaggaagcggaagagcgcccaatacgcaaaccgcctctccccgcgcgttggccgattcattaatgcagctggcacgacaggtttcccgactggaaagcgggcagtgagcgcaacgcaattaatgtgagttagctcactcattaggcaccccaggctttacactttatgcttccggctcgtatgttgtgtggaattgtgagcggataacaatttcacacaggaaacagctatgaccatgattacgcctctagaaagctttaatacgactcactataaggactcactatttgttttcgcgcccagttgcaaaaagtgtcgacatttgcttctgacacaactgtgttcactagcaacctcaaacagacaccgccaccatgcctgctgctaagagagtgaaactggatggatccgaggaactgctgagcaagaactaccacctggaaaacgaggtggccagactgaagaaaggctctggctctggcggaagcggttctggcggatcaggatctggaagtggcggctctggaagcggaggttctggatctggcgaagaactgctgtctaagaattatcacctcgagaacgaagtggctcggctcaagaaaggcagtggcagcggaggaagtggatccggcggtagtggtagtggaagcggcggatccggctcaggcggatctggttcaggggaagaactcctctccaaaaactaccatctcgagaatgaggtcgcccgcctgaaaaaaggatcaggttccggtggttctggcagcggtggttcaggctcaggcagcggcggtagcggtagcggtggaagcggaagcggaccaaaaaagaagagaaaggtaatggacaagaagtacagcatcggcctggccatcggcaccaactctgtgggctgggccgtgatcaccgacgagtacaaggtgcccagcaagaaattcaaggtgctgggcaacaccgaccggcacagcatcaagaagaacctgatcggcgccctgctgttcgacagcggagaaacagccgaggccacccggctgaagagaaccgccagaagaagatacaccagacggaagaaccggatctgctatctgcaagagatcttcagcaacgagatggccaaggtggacgacagcttcttccacagactggaagagtccttcctggtggaagaggataagaagcacgagcggcaccccatcttcggcaacatcgtggacgaggtggcctaccacgagaagtaccccaccatctaccacctgagaaagaaactggtggacagcaccgacaaggccgacctgcggctgatctatctggccctggcccacatgatcaagttccggggccacttcctgatcgagggcgacctgaaccccgacaacagcgacgtggacaagctgttcatccagctggtgcagacctacaaccagctgttcgaggaaaaccccatcaacgccagcggcgtggacgccaaggccatcctgtctgccagactgagcaagagcagacggctggaaaatctgatcgcccagctgcccggcgagaagaagaatggcctgttcggcaacctgattgccctgagcctgggcctgacccccaacttcaagagcaacttcgacctggccgaggatgccaaactgcagctgagcaaggacacctacgacgacgacctggacaacctgctggcccagatcggcgaccagtacgccgacctgtttctggccgccaagaacctgtccgacgccatcctgctgagcgacatcctgagagtgaacaccgagatcaccaaggcccccctgagcgcctctatgatcaagagatacgacgagcaccaccaggacctgaccctgctgaaagctctcgtgcggcagcagctgcctgagaagtacaaagagattttcttcgaccagagcaagaacggctacgccggctacatcgatggcggagccagccaggaagagttctacaagttcatcaagcccatcctggaaaagatggacggcaccgaggaactgctcgtgaagctgaacagagaggacctgctgcggaagcagcggaccttcgacaacggcagcatcccccaccagatccacctgggagagctgcacgccattctgcggcggcaggaagatttttacccattcctgaaggacaaccgggaaaagatcgagaagatcctgaccttccgcatcccctactacgtgggccctctggccaggggaaacagcagattcgcctggatgaccagaaagagcgaggaaaccatcaccccctggaacttcgaggaagtggtggacaagggcgccagcgcccagagcttcatcgagcggatgaccaacttcgataagaacctgcccaacgagaaggtgctgcccaagcacagcctgctgtacgagtacttcaccgtgtacaacgagctgaccaaagtgaaatacgtgaccgagggaatgagaaagcccgccttcctgagcggcgagcagaaaaaagccatcgtggacctgctgttcaagaccaaccggaaagtgaccgtgaagcagctgaaagaggactacttcaagaaaatcgagtgcttcgactccgtggaaatctccggcgtggaagatcggttcaacgcctccctgggcacataccacgatctgctgaaaattatcaaggacaaggacttcctggacaatgaggaaaacgaggacattctggaagatatcgtgctgaccctgacactgtttgaggacagagagatgatcgaggaacggctgaaaacctatgcccacctgttcgacgacaaagtgatgaagcagctgaagcggcggagatacaccggctggggcaggctgagccggaagctgatcaacggcatccgggacaagcagtccggcaagacaatcctggatttcctgaagtccgacggcttcgccaacagaaacttcatgcagctgatccacgacgacagcctgacctttaaagaggacatccagaaagcccaggtgtccggccagggcgatagcctgcacgagcacattgccaatctggccggcagccccgccattaagaagggcatcctgcagacagtgaaggtggtggacgagctcgtgaaagtgatgggccggcacaagcccgagaacatcgtgatcgaaatggccagagagaaccagaccacccagaagggacagaagaacagccgcgagagaatgaagcggatcgaagagggcatcaaagagctgggcagccagatcctgaaagaacaccccgtggaaaacacccagctgcagaacgagaagctgtacctgtactacctgcagaatgggcgggatatgtacgtggaccaggaactggacatcaaccggctgtccgactacgatgtggacgctatcgtgcctcagagctttctgaaggacgactccatcgataacaaagtgctgactcggagcgacaagaaccggggcaagagcgacaacgtgccctccgaagaggtcgtgaagaagatgaagaactactggcgccagctgctgaatgccaagctgattacccagaggaagttcgacaatctgaccaaggccgagagaggcggcctgagcgaactggataaggccggcttcatcaagagacagctggtggaaacccggcagatcacaaagcacgtggcacagatcctggactcccggatgaacactaagtacgacgagaacgacaaactgatccgggaagtgaaagtgatcaccctgaagtccaagctggtgtccgatttccggaaggatttccagttttacaaagtgcgcgagatcaacaactaccaccacgcccacgacgcctacctgaacgccgtcgtgggaaccgccctgatcaaaaagtaccctaagctggaaagcgagttcgtgtacggcgactacaaggtgtacgacgtgcggaagatgatcgccaagagcgagcaggaaatcggcaaggctaccgccaagtacttcttctacagcaacatcatgaactttttcaagaccgagattaccctggccaacggcgagatccggaagcggcctctgatcgagacaaacggcgaaacaggcgagatcgtgtgggataagggccgggactttgccaccgtgcggaaagtgctgtctatgccccaagtgaatatcgtgaaaaagaccgaggtgcagacaggcggcttcagcaaagagtctatcctgcccaagaggaacagcgacaagctgatcgccagaaagaaggactgggaccctaagaagtacggcggcttcgacagccccaccgtggcctattctgtgctggtggtggccaaagtggaaaagggcaagtccaagaaactgaagagtgtgaaagagctgctggggatcaccatcatggaaagaagcagcttcgagaagaatcccatcgactttctggaagccaagggctacaaagaagtgaaaaaggacctgatcatcaagctgcctaagtactccctgttcgagctggaaaacggccggaagagaatgctggcctctgccggcgaactgcagaagggaaacgaactggccctgccctccaaatatgtgaacttcctgtacctggccagccactatgagaagctgaagggctcccccgaggataatgagcagaaacagctgtttgtggaacagcacaaacactacctggacgagatcatcgagcagatcagcgagttctccaagagagtgatcctggccgacgctaatctggacaaggtgctgagcgcctacaacaagcacagagacaagcctatcagagagcaggccgagaatatcatccacctgtttaccctgaccaatctgggagcccctgccgccttcaagtactttgacaccaccatcgaccggaagaggtacaccagcaccaaagaggtgctggacgccaccctgatccaccagagcatcaccggcctgtacgagacacggatcgacctgtctcagctgggaggcgacgcctatccctatgacgtgcccgattatgccagcctgggcagcggctcccccaagaaaaaacgcaaggtggaagatcctaagaaaaagcggaaagtggacggcagcggcagcgagacccccggtaccagcgagagcgccacccccgagagcatgaacaattcccagggaagagtgaccttcgaggatgtcactgtgaacttcacccagggggagtggcagcggctgaatcccgaacagagaaacttgtacagggatgtgatgctggagaattacagcaaccttgtctctgtgggacaaggggaaaccaccaaacccgatgtgatcttgaggttggaacaaggaaaggagccatggttggaggaagaggaagtgctgggaagtggccgtgcagaaaaaaatggggacattggagggcagatttggaagccaaaggatgtgaaagagagtctcctcgagggaagcggagctactaacttcagcctgctgaagcaggctggagacgtggaggagaaccctggacctatgcctgctgctaagagagtgaaactggatggatccaaccatgaccaggaatttgaccccccaaaggtttacccacctgtgccagctgagaagaggaagcccatccgcgtgctgtctctctttgatgggattgctacagggctcctggtgctgaaggacctgggcatccaagtggaccgctacattgcctccgaggtgtgtgaggactccatcacggtgggcatggtgcggcaccagggaaagatcatgtacgtcggggacgtccgcagcgtcacacagaagcatatccaggagtggggcccattcgacctggtgattggaggcagtccctgcaatgacctctccattgtcaaccctgcccgcaagggactttatgagggtactggccgcctcttctttgagttctaccgcctcctgcatgatgcgcggcccaaggagggagatgatcgccccttcttctggctctttgagaatgtggtggccatgggcgttagtgacaagagggacatctcgcgatttcttgagtctaaccccgtgatgattgacgccaaagaagtgtctgctgcacacagggcccgttacttctggggtaaccttcctggcatgaacaggcctttggcatccactgtgaatgataagctggagctgcaagagtgtctggagcacggcagaatagccaagttcagcaaagtgaggaccattaccaccaggtcaaactctataaagcagggcaaagaccagcatttccccgtgttcatgaacgagaaggaggacatcctgtggtgcactgaaatggaaagggtgtttggcttccccgtccactacacagacgtctccaacatgagccgcttggcgaggcagagactgctgggccgatcgtggagcgtgccggtcatccgccacctcttcgctccgctgaaggaatattttgcttgtgtgtctagcggcaatagtaacgctaacagccgcgggccgagcttcagcagcggcctggtgccgttaagcttgcgcggcagccatatgttcgaaaccgtgcctgtgtggaggagacagccagtccgggtgctgtccctttttgaagacatcaagaaagagctgacgagtttgggctttttggaaagtggttctgacccgggacaactgaagcatgtggttgatgtcacagacacagtgaggaaggatgtggaggagtggggacccttcgatcttgtgtacggcgccacacctcccctgggccacacctgtgaccgtcctcccagctggtacctgttccagttccaccggctcctgcagtacgcacggcccaagccaggcagccccaggcccttcttctggatgttcgtggacaatctggtgctgaacaaggaagacctggacgtcgcatctcgcttcctggagatggagccagtcaccatcccagatgtccacggcggatccttgcagaatgctgtccgcgtgtggagcaacatcccagccataaggagcagcaggcactgggctctggtttcggaagaagaattgtccctgctggcccagaacaagcagagctcgaagctcgcggccaagtggcccaccaagctggtgaagaactgctttctccccctaagagaatatttcaagtatttttcaggagggccgagctctggcgcacccccaccaagtggagggtctcctgccgggtccccaacatctactgaagaaggcaccagcgaatccgcaacgcccgagtcaggccctggtacctccacagaaccatctgaaggtagtgcgcctggttccccagctggaagccctacttccaccgaagaaggcacgtcaaccgaaccaagtgaaggatctgcccctgggaccagcactgaaccatctgagccaaaaaagaagagaaaggtaccatctgagggccccgacatcgtgatgacccagagccccagcagcctgagcgccagcgtgggcgaccgcgtgaccatcacctgccgcagcagcaccggcgccgtgaccaccagcaactacgccagctgggtgcaggagaagcccggcaagctgttcaagggcctgatcggcggcaccaacaaccgcgcccccggcgtgcccagccgcttcagcggcagcctgatcggcgacaaggccaccctgaccatcagcagcctgcagcccgaggacttcgccacctacttctgcgccctgtggtacagcaaccactgggtgttcggccagggcaccaaggtggagctgaagcgcggcggcggcggcagcggcggcggcggcagcggcggcggcggcagcagcggcggcggcagcgaggtgaagctgctggagagcggcggcggcctggtgcagcccggcggcagcctgaagctgagctgcgccgtgagcggcttcagcctgaccgactacggcgtgaactgggtgcgccaggcccccggccgcggcctggagtggatcggcgtgatctggggcgacggcatcaccgactacaacagcgccctgaaggaccgcttcatcatcagcaaggacaacggcaagaacaccgtgtacctgcagatgagcaaggtgcgcagcgacgacaccgccctgtactactgcgtgaccggcctgttcgactactggggccagggcaccctggtgaccgtgagcagctacccatacgatgttccagattacgctggtggaggcggaggttctgggggaggaggtagtggcggtggtggttcaggaggcggcggaagctgataataggatcccaagcacgcagcaatgcagctcaaaacgcttagcctagccacacccccacgggaaacagcagtgattaacctttagcaataaacgaaagtttaactaagctatactaaccccagggttggtcaatttcgtgccagccacaccctggtactgcatgcacgcaatgctagctgcccctttcccgtcctgggcaccccgagtctcccccgaccccgggtcccaggtatgctcccacctccacctgccccactcaccacctctgctagttccagacacctccgagacgaggaaaaaaaaaaaaaaaaaaaaaaaaaaaaaaaaaaaaaaaaaaaaaaaaaaaaaaaaaaaaaaaaaaaaaaaaaaaaaaaaaaaaaaaaaaaaaaaaaaaaaaaaaaaaaaaaaaaaaaaaaaaaaaaaaaaaaaaaaaaaaaaaaaaaaaaaaaaaaaaaaaaaaaaaaaaaaaaaaaaaaaaaaaaaaaaaaaaaaaaaaaaaaaaaaaaaaaaaaaaaaaaaaaaaaaaaaaaaaaaaaaaaaaaaaaaaaaaaaaaaaaaaaaaaaaaaaaaaaaaaaaaaaaaaaaaaaaaaaaaaaaaaaaaaaaaaaaaaaaaaaaaaaaaaaaaaaaaaaaaaaaaaaaaaaaaaaaaaaaaaaaaaaaaaaaaaaaaaaaaaaaaaaaaaaaaaaaccgtcttcaagctttctagaaattcactggccgtcgttttacaacgtcgtgactgggaaaaccctggcgttacccaacttaatcgccttgcagcacatccccctttcgccagctggcgtaatagcgaagaggcccgcaccgatcgcccttcccaacagttgcgcagcctgaatggcgaatggcgcctgatgcggtattttctccttacgcatctgtgcggtatttcacaccgcatatggtgcactctcagtacaatctgctctgatgccgcatagttaagccagccccgacacccgccaacacccgctgacgcgccctgacgggcttgtctgctcccggcatccgcttacagacaagctgtgaccgtctccgggagctgcatgtgtcagaggttttcaccgtcatcaccgaaacgcgcgagacgaaagggcctcgtgatacgcctatttttataggttaatgtcatgataataatggtttcttagacgtcaggtggcacttttcggggaaatgtgcgcggaacccctatttgtttatttttctaaatacattcaaatatgtatccgctcatgagacaataaccctgataaatgcttcaataatattgaaaaaggaagagtatgagtattcaacatttccgtgtcgcccttattcccttttttgcggcattttgccttcctgtttttgctcacccagaaacgctggtgaaagtaaaagatgctgaagatcagttgggtgcacgagtgggttacatcgaactggatctcaacagcggtaagatccttgagagttttcgccccgaagaacgttttccaatgatgagcacttttaaagttctgctatgtggcgcggtattatcccgtattgacgccgggcaagagcaactcggtcgccgcatacactattctcagaatgacttggttgagtactcaccagtcacagaaaagcatcttacggatggcatgacagtaagagaattatgcagtgctgccataaccatgagtgataacactgcggccaacttacttctgacaacgatcggaggaccgaaggagctaaccgcttttttgcacaacatgggggatcatgtaactcgccttgatcgttgggaaccggagctgaatgaagccataccaaacgacgagcgtgacaccacgatgcctgtagcaatggcaacaacgttgcgcaaactattaactggcgaactacttactctagcttcccggcaacaattaatagactggatggaggcggataaagttgcaggaccacttctgcgctcggcccttccggctggctggtttattgctgataaatctggagccggtgagcgtgggtctcgcggtatcattgcagcactggggccagatggtaagccctcccgtatcgtagttatctacacgacggggagtcaggcaactatggatgaacgaaatagacagatcgc

SEQ ID NO: 222 - DNA, 10881 bp, synthetic construct
  misc_feature 1..10881: note = DNA of V28_3xGCN4-dCas12a-ZIM3-2a-D3a-hD3L-scFv
  source 1..10881: mol_type = other DNA
tgagataggtgcctcactgattaagcattggtaactgtcagaccaagtttactcatatatactttagattgatttaaaacttcatttttaatttaaaaggatctaggtgaagatcctttttgataatctcatgaccaaaatcccttaacgtgagttttcgttccactgagcgtcagaccccgtagaaaagatcaaaggatcttcttgagatcctttttttctgcgcgtaatctgctgcttgcaaacaaaaaaaccaccgctaccagcggtggtttgtttgccggatcaagagctaccaactctttttccgaaggtaactggcttcagcagagcgcagataccaaatactgttcttctagtgtagccgtagttaggccaccacttcaagaactctgtagcaccgcctacatacctcgctctgctaatcctgttaccagtggctgctgccagtggcgataagtcgtgtcttaccgggttggactcaagacgatagttaccggataaggcgcagcggtcgggctgaacggggggttcgtgcacacagcccagcttggagcgaacgacctacaccgaactgagatacctacagcgtgagctatgagaaagcgccacgcttcccgaagggagaaaggcggacaggtatccggtaagcggcagggtcggaacaggagagcgcacgagggagcttccagggggaaacgcctggtatctttatagtcctgtcgggtttcgccacctctgacttgagcgtcgatttttgtgatgctcgtcaggggggcggagcctatggaaaaacgccagcaacgcggcctttttacggttcctggccttttgctggccttttgctcacatgttctttcctgcgttatcccctgattctgtggataaccgtattaccgcctttgagtgagctgataccgctcgccgcagccgaacgaccgagcgcagcgagtcagtgagcgaggaagcggaagagcgcccaatacgcaaaccgcctctccccgcgcgttggccgattcattaatgcagctggcacgacaggtttcccgactggaaagcgggcagtgagcgcaacgcaattaatgtgagttagctcactcattaggcaccccaggctttacactttatgcttccggctcgtatgttgtgtggaattgtgagcggataacaatttcacacaggaaacagctatgaccatgattacgcctctagaaagctttaatacgactcactataaggactcactatttgttttcgcgcccagttgcaaaaagtgtcgacatttgcttctgacacaactgtgttcactagcaacctcaaacagacaccgccaccatgcctgctgctaagagagtgaaactggatggatccgaggaactgctgagcaagaactaccacctggaaaacgaggtggccagactgaagaaaggctctggctctggcggaagcggttctggcggatcaggatctggaagtggcggctctggaagcggaggttctggatctggcgaagaactgctgtctaagaattatcacctcgagaacgaagtggctcggctcaagaaaggcagtggcagcggaggaagtggatccggcggtagtggtagtggaagcggcggatccggctcaggcggatctggttcaggggaagaactcctctccaaaaactaccatctcgagaatgaggtcgcccgcctgaaaaaaggatcaggttccggtggttctggcagcggtggttcaggctcaggcagcggcggtagcggtagcggtggaagcggaagcggaccaaaaaagaagagaaaggtaatgtcaaagctggagaaattcaccaactgttatagcctgtctaagaccctgcgcttcaaggcaatcccagtgggcaagacacaagagaacattgacaacaaacggctcctggtggaggatgagaagagggctgaagattacaagggcgttaagaagctgctggataggtactatctgtcattcatcaacgatgtcctccacagtatcaagctgaagaatctgaacaattacatttctctgttccggaagaagacacggaccgagaaggagaacaaagagctggagaatctggagatcaacctgaggaaagaaatagctaaggctttcaaagggaacgagggttacaagtccctgttcaagaaagacattatcgagactattctgcctgagttcctggacgataaagatgagatcgccctcgtcaattccttcaatgggtttaccacagcctttaccggcttcttcgacaatagagagaatatgttctctgaagaggccaaatccactagcatcgcctttcgctgcataaacgagaacctgactaggtacatcagcaatatggacatctttgagaaagtcgatgccatattcgacaaacatgaggtgcaggagattaaggagaagatcctgaactcagattacgatgtcgaagatttcttcgagggagagttcttcaacttcgtgctcacacaagagggcattgatgtgtacaatgcaatcattggagggttcgtgacagagagtggcgagaagataaagggcctgaacgagtatatcaacctctacaaccagaaaaccaagcagaaactgcctaagttcaagccactgtacaaacaagtgctctcagatagggaaagcctgagcttctacggtgaagggtatacatcagatgaagaagtgctcgaagtgttccgcaacaccctcaataagaacagtgaaatcttctcttcaatcaagaagctggagaaactgttcaagaatttcgatgagtactcctctgccggaatctttgtgaagaatggccctgcaatatccactattagcaaagacatctttggcgagtggaacgttatcagggataagtggaatgccgagtacgatgatattcatctcaagaagaaagccgtggttacagagaaatacgaggatgatagacgcaagagctttaagaagattggtagcttctctctcgaacagctgcaggagtacgccgacgctgacctgtcagtcgtggagaaactcaaggagatcataatccagaaggtggatgaaatctacaaagtgtatggaagctctgagaaactcttcgatgcagactttgttctggagaagagtctgaagaagaacgacgcagtggttgctatcatgaaggacctgctggattctgttaagtctttcgagaattacattaaggcattctttggtgaagggaaggagacaaatagggacgagagcttctatggcgactttgttctggcctacgacatcctcctcaaggttgaccacatctatgacgctatacggaattacgttacccagaagccctatagcaaagacaagttcaagctgtatttccagaatccacagtttatgggtgggtgggataaagacaaagaaacagattacagggccactatcctgcggtacggcagcaaatactatctggctatcatggataagaagtacgccaaatgcctccagaagatcgacaaggacgacgtgaacggtaactacgagaagatcaattacaagctcctgccaggacctaacaagatgctgcccaaggtgttcttctccaagaaatggatggcctactataacccaagcgaggacattcagaagatatacaagaatgggacattcaagaagggcgatatgttcaacctcaacgactgccacaagctgattgatttcttcaaggatagcatttctcgctatcccaagtggtctaatgcatacgatttcaacttcagcgagactgagaagtacaaagacatcgctggcttctaccgggaggtggaagagcaaggctataaggtgtcattcgaatccgcttctaagaaggaagtggataagctcgtggaagagggtaagctgtacatgttccagatatacaacaaagacttcagcgataagagccacggcactccaaacctccatactatgtatttcaagctgctgtttgacgagaacaaccacggacagattaggctgtcaggaggcgcagaactcttcatgcgcagagcttcactgaagaaggaggaactcgttgtccacccagccaatagccctatagccaataagaatccagacaatcctaagaaaaccactactctgtcttacgatgtgtataaggataagagattctctgaagatcagtacgaactgcacatacccattgccattaacaagtgccctaagaacatcttcaagattaacacagaggttagagtgctcctgaaacacgacgataacccttatgttataggcattgctcgcggagagagaaacctgctgtacatcgtcgtggtggacggcaaaggcaacatcgtggaacagtacagtctcaatgaaatcattaacaatttcaacggaatccgcattaagaccgactaccattctctcctcgacaagaaggagaaagaaaggttcgaagcaagacagaattggacaagtatagagaatatcaaagaactgaaggctgggtacatctctcaggttgtgcacaagatatgtgagctggtggagaagtacgacgctgttatcgccctcgcggacctgaatagcggcttcaagaactccagggtgaaggtggagaagcaggtgtatcagaagttcgagaagatgctgatcgacaagctcaactatatggtggacaagaaatccaatccttgcgctactggtggagccctgaagggctatcaaatcaccaataagttcgaatctttcaagtctatgagcacccagaatggcttcatcttctacatacccgcatggctgacatccaagattgatccctctaccggatttgttaatctgctcaagactaagtacacctctattgctgactcaaagaagttcatatcatcatttgaccgcatcatgtacgtgccagaagaggacctgttcgagtttgccctggattacaagaatttctctcggactgacgccgactacatcaagaagtggaagctctactcttatggtaatcggattcgcatattccgcaatcccaagaagaataacgtgttcgattgggaggaagtttgcctcaccagcgcttacaaggagctgttcaataagtatgggattaactaccagcagggcgacataagagccctgctgtgcgaacaatctgataaggcattctattcctctttcatggcactgatgtcactgatgctgcaaatgcgcaattccatcaccggaagaacagacgtggcctttctgatctctcctgtcaagaactcagatggcatcttctacgattcccgcaactatgaagcacaggagaatgctatcctgcctaagaatgccgatgcaaatggagcctataacatcgccagaaaggtcctctgggccataggacaattcaagaaagctgaagatgagaagctggacaaggtgaagatcgccatttcaaacaaagagtggctcgaatatgctcagacctcagtgaagcatgcctatccctatgacgtgcccgattatgccagcctgggcagcggctcccccaagaaaaaacgcaaggtggaagatcctaagaaaaagcggaaagtggacggcagcggcagcgagacccccggtaccagcgagagcgccacccccgagagcatgaacaattcccagggaagagtgaccttcgaggatgtcactgtgaacttcacccagggggagtggcagcggctgaatcccgaacagagaaacttgtacagggatgtgatgctggagaattacagcaaccttgtctctgtgggacaaggggaaaccaccaaacccgatgtgatcttgaggttggaacaaggaaaggagccatggttggaggaagaggaagtgctgggaagtggccgtgcagaaaaaaatggggacattggagggcagatttggaagccaaaggatgtgaaagagagtctcctcgagggaagcggagctactaacttcagcctgctgaagcaggctggagacgtggaggagaaccctggacctatgcctgctgctaagagagtgaaactggatggatccaaccatgaccaggaatttgaccccccaaaggtttacccacctgtgccagctgagaagaggaagcccatccgcgtgctgtctctctttgatgggattgctacagggctcctggtgctgaaggacctgggcatccaagtggaccgctacattgcctccgaggtgtgtgaggactccatcacggtgggcatggtgcggcaccagggaaagatcatgtacgtcggggacgtccgcagcgtcacacagaagcatatccaggagtggggcccattcgacctggtgattggaggcagtccctgcaatgacctctccattgtcaaccctgcccgcaagggactttatgagggtactggccgcctcttctttgagttctaccgcctcctgcatgatgcgcggcccaaggagggagatgatcgccccttcttctggctctttgagaatgtggtggccatgggcgttagtgacaagagggacatctcgcgatttcttgagtctaaccccgtgatgattgacgccaaagaagtgtctgctgcacacagggcccgttacttctggggtaaccttcctggcatgaacaggcctttggcatccactgtgaatgataagctggagctgcaagagtgtctggagcacggcagaatagccaagttcagcaaagtgaggaccattaccaccaggtcaaactctataaagcagggcaaagaccagcatttccccgtgttcatgaacgagaaggaggacatcctgtggtgcactgaaatggaaagggtgtttggcttccccgtccactacacagacgtctccaacatgagccgcttggcgaggcagagactgctgggccgatcgtggagcgtgccggtcatccgccacctcttcgctccgctgaaggaatattttgcttgtgtgtctagcggcaatagtaacgctaacagccgcgggccgagcttcagcagcggcctggtgccgttaagcttgcgcggcagccatatgttcgaaaccgtgcctgtgtggaggagacagccagtccgggtgctgtccctttttgaagacatcaagaaagagctgacgagtttgggctttttggaaagtggttctgacccgggacaactgaagcatgtggttgatgtcacagacacagtgaggaaggatgtggaggagtggggacccttcgatcttgtgtacggcgccacacctcccctgggccacacctgtgaccgtcctcccagctggtacctgttccagttccaccggctcctgcagtacgcacggcccaagccaggcagccccaggcccttcttctggatgttcgtggacaatctggtgctgaacaaggaagacctggacgtcgcatctcgcttcctggagatggagccagtcaccatcccagatgtccacggcggatccttgcagaatgctgtccgcgtgtggagcaacatcccagccataaggagcagcaggcactgggctctggtttcggaagaagaattgtccctgctggcccagaacaagcagagctcgaagctcgcggccaagtggcccaccaagctggtgaagaactgctttctccccctaagagaatatttcaagtatttttcaggagggccgagctctggcgcacccccaccaagtggagggtctcctgccgggtccccaacatctactgaagaaggcaccagcgaatccgcaacgcccgagtcaggccctggtacctccacagaaccatctgaaggtagtgcgcctggttccccagctggaagccctacttccaccgaagaaggcacgtcaaccgaaccaagtgaaggatctgcccctgggaccagcactgaaccatctgagccaaaaaagaagagaaaggtaccatctgagggccccgacatcgtgatgacccagagccccagcagcctgagcgccagcgtgggcgaccgcgtgaccatcacctgccgcagcagcaccggcgccgtgaccaccagcaactacgccagctgggtgcaggagaagcccggcaagctgttcaagggcctgatcggcggcaccaacaaccgcgcccccggcgtgcccagccgcttcagcggcagcctgatcggcgacaaggccaccctgaccatcagcagcctgcagcccgaggacttcgccacctacttctgcgccctgtggtacagcaaccactgggtgttcggccagggcaccaaggtggagctgaagcgcggcggcggcggcagcggcggcggcggcagcggcggcggcggcagcagcggcggcggcagcgaggtgaagctgctggagagcggcggcggcctggtgcagcccggcggcagcctgaagctgagctgcgccgtgagcggcttcagcctgaccgactacggcgtgaactgggtgcgccaggcccccggccgcggcctggagtggatcggcgtgatctggggcgacggcatcaccgactacaacagcgccctgaaggaccgcttcatcatcagcaaggacaacggcaagaacaccgtgtacctgcagatgagcaaggtgcgcagcgacgacaccgccctgtactactgcgtgaccggcctgttcgactactggggccagggcaccctggtgaccgtgagcagctacccatacgatgttccagattacgctggtggaggcggaggttctgggggaggaggtagtggcggtggtggttcaggaggcggcggaagctgataataggatcccaagcacgcagcaatgcagctcaaaacgcttagcctagccacacccccacgggaaacagcagtgattaacctttagcaataaacgaaagtttaactaagctatactaaccccagggttggtcaatttcgtgccagccacaccctggtactgcatgcacgcaatgctagctgcccctttcccgtcctgggcaccccgagtctcccccgaccccgggtcccaggtatgctcccacctccacctgccccactcaccacctctgctagttccagacacctccgagacgaggaaaaaaaaaaaaaaaaaaaaaaaaaaaaaaaaaaaaaaaaaaaaaaaaaaaaaaaaaaaaaaaaaaaaaaaaaaaaaaaaaaaaaaaaaaaaaaaaaaaaaaaaaaaaaaaaaaaaaaaaaaaaaaaaaaaaaaaaaaaaaaaaaaaaaaaaaaaaaaaaaaaaaaaaaaaaaaaaaaaaaaaaaaaaaaaaaaaaaaaaaaaaaaaaaaaaaaaaaaaaaaaaaaaaaaaaaaaaaaaaaaaaaaaaaaaaaaaaaaaaaaaaaaaaaaaaaaaaaaaaaaaaaaaaaaaaaaaaaaaaaaaaaaaaaaaaaaaaaaaaaaaaaaaaaaaaaaaaaaaaaaaaaaaaaaaaaaaaaaaaaaaaaaaaaaaaaaaaaaaaaaaaaaaaaaaaaaccgtcttcaagctttctagaaattcactggccgtcgttttacaacgtcgtgactgggaaaaccctggcgttacccaacttaatcgccttgcagcacatccccctttcgccagctggcgtaatagcgaagaggcccgcaccgatcgcccttcccaacagttgcgcagcctgaatggcgaatggcgcctgatgcggtattttctccttacgcatctgtgcggtatttcacaccgcatatggtgcactctcagtacaatctgctctgatgccgcatagttaagccagccccgacacccgccaacacccgctgacgcgccctgacgggcttgtctgctcccggcatccgcttacagacaagctgtgaccgtctccgggagctgcatgtgtcagaggttttcaccgtcatcaccgaaacgcgcgagacgaaagggcctcgtgatacgcctatttttataggttaatgtcatgataataatggtttcttagacgtcaggtggcacttttcggggaaatgtgcgcggaacccctatttgtttatttttctaaatacattcaaatatgtatccgctcatgagacaataaccctgataaatgcttcaataatattgaaaaaggaagagtatgagtattcaacatttccgtgtcgcccttattcccttttttgcggcattttgccttcctgtttttgctcacccagaaacgctggtgaaagtaaaagatgctgaagatcagttgggtgcacgagtgggttacatcgaactggatctcaacagcggtaagatccttgagagttttcgccccgaagaacgttttccaatgatgagcacttttaaagttctgctatgtggcgcggtattatcccgtattgacgccgggcaagagcaactcggtcgccgcatacactattctcagaatgacttggttgagtactcaccagtcacagaaaagcatcttacggatggcatgacagtaagagaattatgcagtgctgccataaccatgagtgataacactgcggccaacttacttctgacaacgatcggaggaccgaaggagctaaccgcttttttgcacaacatgggggatcatgtaactcgccttgatcgttgggaaccggagctgaatgaagccataccaaacgacgagcgtgacaccacgatgcctgtagcaatggcaacaacgttgcgcaaactattaactggcgaactacttactctagcttcccggcaacaattaatagactggatggaggcggataaagttgcaggaccacttctgcgctcggcccttccggctggctggtttattgctgataaatctggagccggtgagcgtgggtctcgcggtatcattgcagcactggggccagatggtaagccctcccgtatcgtagttatctacacgacggggagtcaggcaactatggatgaacgaaatagacagatcgc

SEQ ID NO: 223 - DNA, 9930 bp, synthetic construct
  misc_feature 1..9930: note = DNA of V29_3xGCN4-dCas12i-ZIM3-2a-D3a-hD3L-scFv
  source 1..9930: mol_type = other DNA
tgagataggtgcctcactgattaagcattggtaactgtcagaccaagtttactcatatatactttagattgatttaaaacttcatttttaatttaaaaggatctaggtgaagatcctttttgataatctcatgaccaaaatcccttaacgtgagttttcgttccactgagcgtcagaccccgtagaaaagatcaaaggatcttcttgagatcctttttttctgcgcgtaatctgctgcttgcaaacaaaaaaaccaccgctaccagcggtggtttgtttgccggatcaagagctaccaactctttttccgaaggtaactggcttcagcagagcgcagataccaaatactgttcttctagtgtagccgtagttaggccaccacttcaagaactctgtagcaccgcctacatacctcgctctgctaatcctgttaccagtggctgctgccagtggcgataagtcgtgtcttaccgggttggactcaagacgatagttaccggataaggcgcagcggtcgggctgaacggggggttcgtgcacacagcccagcttggagcgaacgacctacaccgaactgagatacctacagcgtgagctatgagaaagcgccacgcttcccgaagggagaaaggcggacaggtatccggtaagcggcagggtcggaacaggagagcgcacgagggagcttccagggggaaacgcctggtatctttatagtcctgtcgggtttcgccacctctgacttgagcgtcgatttttgtgatgctcgtcaggggggcggagcctatggaaaaacgccagcaacgcggcctttttacggttcctggccttttgctggccttttgctcacatgttctttcctgcgttatcccctgattctgtggataaccgtattaccgcctttgagtgagctgataccgctcgccgcagccgaacgaccgagcgcagcgagtcagtgagcgaggaagcggaagagcgcccaatacgcaaaccgcctctccccgcgcgttggccgattcattaatgcagctggcacgacaggtttcccgactggaaagcgggcagtgagcgcaacgcaattaatgtgagttagctcactcattaggcaccccaggctttacactttatgcttccggctcgtatgttgtgtggaattgtgagcggataacaatttcacacaggaaacagctatgaccatgattacgcctctagaaagctttaatacgactcactataaggactcactatttgttttcgcgcccagttgcaaaaagtgtcgacatttgcttctgacacaactgtgttcactagcaacctcaaacagacaccgccaccatgcctgctgctaagagagtgaaactggatggatccgaggaactgctgagcaagaactaccacctggaaaacgaggtggccagactgaagaaaggctctggctctggcggaagcggttctggcggatcaggatctggaagtggcggctctggaagcggaggttctggatctggcgaagaactgctgtctaagaattatcacctcgagaacgaagtggctcggctcaagaaaggcagtggcagcggaggaagtggatccggcggtagtggtagtggaagcggcggatccggctcaggcggatctggttcaggggaagaactcctctccaaaaactaccatctcgagaatgaggtcgcccgcctgaaaaaaggatcaggttccggtggttctggcagcggtggttcaggctcaggcagcggcggtagcggtagcggtggaagcggaagcggaccaaaaaagaagagaaaggtaatggaagagacacggacccctgagaagatcgcctgccagcaggatagaagcgccttcttcaagctgggcaagctgccccagaaaaccaccagcgccatctaccacctgatgcggtgtagcaagcggtacatcgacaacgtgtccgagacaatcagcaacaacatcgagaaggccgccatgaccagcgacaaccacatcttcagaagcgccctgaaagaagagtacaagaagatctaccgcgagaagttctaccccgacgtgaccggccagccttttccagataagggccccgacaacacccacatcgtggaacggaccgtggaaaacctgtgcggccagtacatctctgccctgaagggcgtgatgaaagtgcggaagcccaagtggcaggacgacatcttcgaggacgagagcgacaaagtgatcgccgagatgctgatggccagcggcaacgaggccgacattcaccccaagctggaaaagaagattgccagcgccaagaaaaaggacaagatggacgagtggcagaaggtgctggacagatacgactacatcaagagcaagaccgacatcgagtggacctacaccacactgctgtacgaccacattgcccgcgagtgcgccagatccatgttcgaggatggcaacaagcctaagttctgctacaccaacggcaacaagttcgccaaacaggtggtggacgagctgtggggctctgagagagtggaatacgagtacgagaagtacctgcactgcagaaccctggaagcctactggaacgaggaaaacaagtacttcttcctggaaaatcaaaagaagtccaagaaaacctacgaggcccggcagatcatcgaccacttcatcgagaacgaggacgccgtgaaggccgaaaccgaagagtatatggccaaggtggccaaagagttcggcgagaacggcggctgcaagttcagaaccgagaacatcctgtacctggtcaacagcgtgtccatcaacaagaagcaggacgaggaacggtgccccatcttcaaagtgaccgacattccccagtatgccgaggccggcatcgatagaatcggcgagtgcaaatacgtgatcaagctgaagctgttcaccgtgggcgagagatacggcaccacctatatgcctgaggccttcagcggcctgtacgacagaaggaccaaccagagatacgacctgatcgacagagcctgcaagggcagctacgtgtacctgcctatctacatcagcgacaaggacagccggaagtggagcgacagactgaagaacaccttcaccatgtccgccttcagcatcagcgagcgcaagaccaagaaagacggcagagtgctgtgcgtgaacctgccttacacacacatccagcacaagccccggaactacttcaaggtgtaccccacctacggcgtggacatcaacgtgaagcacagcctgttcagcaccaacgccaccaacctgaacggctacatcgacgtgaacggcgagctgatcgacttctacaacagcatcggcagacccgataagctcaagaacatcaacctggccgtgacactgggcgacaaaggcggcacagctggcaaccacaccaactttctgctggtgtccgacctcggcgactgggatgatcacggcaagaagcggaacgacagattcgtgaagagagaggacggcacctactacagcagacctgacctgctggccgccggcctgaacttcctgaagaagaagtatagcggcgaccggaagtcctacgattatatcaacaccacaatcgccttccggaacaaccagaccagactgagatgcatcgacaaagagtggaacgatcggaagcgggcctacgatgaggaacacggcaagcctgagaagggcgaaagaagcggcttctaccctaccgaggatgccgagcggctgacaatggaaagacaggccctgcggagagagattgccgagaacaccagacaagtgattgcctacatgctgtggctgttccaagagaacggcatcaagtctatcgccctggaacacctggattgcggcagctggaagaacttccgggaccagctgaagccaaagtggttctgcaacaactgcaagtactgggccgagaagtatggcatcccttacgaggccaccaagtactacagaagcaaccggaagtactttgacatcgaggacggggagctgattcccgagaatgtgaagctgaacgccctgggcgaagccgagaacgacaagagatacttccagacctctatcgccaaggccgtgggcatgagcagcatcaagcagatgttcagcatcgtgtcccagaactacgacatccaagtgaactacaccgagcaggcctacaccagccagaccgacagcagaaatggcaccgtggacaaggacttcagagtgtcccaagagtgctacatcggcagcgacggcaccaagatgaactgcgactttaacgccgccgtgaatatcgccgaccggatctccgatgacaccctgcgggaagagttcaacaaagaactgcccatgaaggaatttgtgaagtacggcgccacacagatcgtgtctcggaacagaagatggaacgccgaaaacgccgagagggtcacaatggccgccttccagaagagaaagaacgctgacggcggagcccataccgccgctgtgaagcctacatccaagaccgaggaaagcagcctgaagctggtggccgaagcctatccctatgacgtgcccgattatgccagcctgggcagcggctcccccaagaaaaaacgcaaggtggaagatcctaagaaaaagcggaaagtggacggcagcggcagcgagacccccggtaccagcgagagcgccacccccgagagcatgaacaattcccagggaagagtgaccttcgaggatgtcactgtgaacttcacccagggggagtggcagcggctgaatcccgaacagagaaacttgtacagggatgtgatgctggagaattacagcaaccttgtctctgtgggacaaggggaaaccaccaaacccgatgtgatcttgaggttggaacaaggaaaggagccatggttggaggaagaggaagtgctgggaagtggccgtgcagaaaaaaatggggacattggagggcagatttggaagccaaaggatgtgaaagagagtctcctcgagggaagcggagctactaacttcagcctgctgaagcaggctggagacgtggaggagaaccctggacctatgcctgctgctaagagagtgaaactggatggatccaaccatgaccaggaatttgaccccccaaaggtttacccacctgtgccagctgagaagaggaagcccatccgcgtgctgtctctctttgatgggattgctacagggctcctggtgctgaaggacctgggcatccaagtggaccgctacattgcctccgaggtgtgtgaggactccatcacggtgggcatggtgcggcaccagggaaagatcatgtacgtcggggacgtccgcagcgtcacacagaagcatatccaggagtggggcccattcgacctggtgattggaggcagtccctgcaatgacctctccattgtcaaccctgcccgcaagggactttatgagggtactggccgcctcttctttgagttctaccgcctcctgcatgatgcgcggcccaaggagggagatgatcgccccttcttctggctctttgagaatgtggtggccatgggcgttagtgacaagagggacatctcgcgatttcttgagtctaaccccgtgatgattgacgccaaagaagtgtctgctgcacacagggcccgttacttctggggtaaccttcctggcatgaacaggcctttggcatccactgtgaatgataagctggagctgcaagagtgtctggagcacggcagaatagccaagttcagcaaagtgaggaccattaccaccaggtcaaactctataaagcagggcaaagaccagcatttccccgtgttcatgaacgagaaggaggacatcctgtggtgcactgaaatggaaagggtgtttggcttccccgtccactacacagacgtctccaacatgagccgcttggcgaggcagagactgctgggccgatcgtggagcgtgccggtcatccgccacctcttcgctccgctgaaggaatattttgcttgtgtgtctagcggcaatagtaacgctaacagccgcgggccgagcttcagcagcggcctggtgccgttaagcttgcgcggcagccatatgttcgaaaccgtgcctgtgtggaggagacagccagtccgggtgctgtccctttttgaagacatcaagaaagagctgacgagtttgggctttttggaaagtggttctgacccgggacaactgaagcatgtggttgatgtcacagacacagtgaggaaggatgtggaggagtggggacccttcgatcttgtgtacggcgccacacctcccctgggccacacctgtgaccgtcctcccagctggtacctgttccagttccaccggctcctgcagtacgcacggcccaagccaggcagccccaggcccttcttctggatgttcgtggacaatctggtgctgaacaaggaagacctggacgtcgcatctcgcttcctggagatggagccagtcaccatcccagatgtccacggcggatccttgcagaatgctgtccgcgtgtggagcaacatcccagccataaggagcagcaggcactgggctctggtttcggaagaagaattgtccctgctggcccagaacaagcagagctcgaagctcgcggccaagtggcccaccaagctggtgaagaactgctttctccccctaagagaatatttcaagtatttttcaggagggccgagctctggcgcacccccaccaagtggagggtctcctgccgggtccccaacatctactgaagaaggcaccagcgaatccgcaacgcccgagtcaggccctggtacctccacagaaccatctgaaggtagtgcgcctggttccccagctggaagccctacttccaccgaagaaggcacgtcaaccgaaccaagtgaaggatctgcccctgggaccagcactgaaccatctgagccaaaaaagaagagaaaggtaccatctgagggccccgacatcgtgatgacccagagccccagcagcctgagcgccagcgtgggcgaccgcgtgaccatcacctgccgcagcagcaccggcgccgtgaccaccagcaactacgccagctgggtgcaggagaagcccggcaagctgttcaagggcctgatcggcggcaccaacaaccgcgcccccggcgtgcccagccgcttcagcggcagcctgatcggcgacaaggccaccctgaccatcagcagcctgcagcccgaggacttcgccacctacttctgcgccctgtggtacagcaaccactgggtgttcggccagggcaccaaggtggagctgaagcgcggcggcggcggcagcggcggcggcggcagcggcggcggcggcagcagcggcggcggcagcgaggtgaagctgctggagagcggcggcggcctggtgcagcccggcggcagcctgaagctgagctgcgccgtgagcggcttcagcctgaccgactacggcgtgaactgggtgcgccaggcccccggccgcggcctggagtggatcggcgtgatctggggcgacggcatcaccgactacaacagcgccctgaaggaccgcttcatcatcagcaaggacaacggcaagaacaccgtgtacctgcagatgagcaaggtgcgcagcgacgacaccgccctgtactactgcgtgaccggcctgttcgactactggggccagggcaccctggtgaccgtgagcagctacccatacgatgttccagattacgctggtggaggcggaggttctgggggaggaggtagtggcggtggtggttcaggaggcggcggaagctgataataggatcccaagcacgcagcaatgcagctcaaaacgcttagcctagccacacccccacgggaaacagcagtgattaacctttagcaataaacgaaagtttaactaagctatactaaccccagggttggtcaatttcgtgccagccacaccctggtactgcatgcacgcaatgctagctgcccctttcccgtcctgggcaccccgagtctcccccgaccccgggtcccaggtatgctcccacctccacctgccccactcaccacctctgctagttccagacacctccgagacgaggaaaaaaaaaaaaaaaaaaaaaaaaaaaaaaaaaaaaaaaaaaaaaaaaaaaaaaaaaaaaaaaaaaaaaaaaaaaaaaaaaaaaaaaaaaaaaaaaaaaaaaaaaaaaaaaaaaaaaaaaaaaaaaaaaaaaaaaaaaaaaaaaaaaaaaaaaaaaaaaaaaaaaaaaaaaaaaaaaaaaaaaaaaaaaaaaaaaaaaaaaaaaaaaaaaaaaaaaaaaaaaaaaaaaaaaaaaaaaaaaaaaaaaaaaaaaaaaaaaaaaaaaaaaaaaaaaaaaaaaaaaaaaaaaaaaaaaaaaaaaaaaaaaaaaaaaaaaaaaaaaaaaaaaaaaaaaaaaaaaaaaaaaaaaaaaaaaaaaaaaaaaaaaaaaaaaaaaaaaaaaaaaaaaaaaaaaaccgtcttcaagctttctagaaattcactggccgtcgttttacaacgtcgtgactgggaaaaccctggcgttacccaacttaatcgccttgcagcacatccccctttcgccagctggcgtaatagcgaagaggcccgcaccgatcgcccttcccaacagttgcgcagcctgaatggcgaatggcgcctgatgcggtattttctccttacgcatctgtgcggtatttcacaccgcatatggtgcactctcagtacaatctgctctgatgccgcatagttaagccagccccgacacccgccaacacccgctgacgcgccctgacgggcttgtctgctcccggcatccgcttacagacaagctgtgaccgtctccgggagctgcatgtgtcagaggttttcaccgtcatcaccgaaacgcgcgagacgaaagggcctcgtgatacgcctatttttataggttaatgtcatgataataatggtttcttagacgtcaggtggcacttttcggggaaatgtgcgcggaacccctatttgtttatttttctaaatacattcaaatatgtatccgctcatgagacaataaccctgataaatgcttcaataatattgaaaaaggaagagtatgagtattcaacatttccgtgtcgcccttattcccttttttgcggcattttgccttcctgtttttgctcacccagaaacgctggtgaaagtaaaagatgctgaagatcagttgggtgcacgagtgggttacatcgaactggatctcaacagcggtaagatccttgagagttttcgccccgaagaacgttttccaatgatgagcacttttaaagttctgctatgtggcgcggtattatcccgtattgacgccgggcaagagcaactcggtcgccgcatacactattctcagaatgacttggttgagtactcaccagtcacagaaaagcatcttacggatggcatgacagtaagagaattatgcagtgctgccataaccatgagtgataacactgcggccaacttacttctgacaacgatcggaggaccgaaggagctaaccgcttttttgcacaacatgggggatcatgtaactcgccttgatcgttgggaaccggagctgaatgaagccataccaaacgacgagcgtgacaccacgatgcctgtagcaatggcaacaacgttgcgcaaactattaactggcgaactacttactctagcttcccggcaacaattaatagactggatggaggcggataaagttgcaggaccacttctgcgctcggcccttccggctggctggtttattgctgataaatctggagccggtgagcgtgggtctcgcggtatcattgcagcactggggccagatggtaagccctcccgtatcgtagttatctacacgacggggagtcaggcaactatggatgaacgaaatagacagatcgc

SEQ ID NO: 224 - DNA, 12201 bp, synthetic construct
  misc_feature 1..12201: note = DNA of V30_10xGCN4-dCas9-ZIM3-2a-D3a-hD3L-scFv
  source 1..12201: mol_type = other DNA
tgagataggtgcctcactgattaagcattggtaactgtcagaccaagtttactcatatatactttagattgatttaaaacttcatttttaatttaaaaggatctaggtgaagatcctttttgataatctcatgaccaaaatcccttaacgtgagttttcgttccactgagcgtcagaccccgtagaaaagatcaaaggatcttcttgagatcctttttttctgcgcgtaatctgctgcttgcaaacaaaaaaaccaccgctaccagcggtggtttgtttgccggatcaagagctaccaactctttttccgaaggtaactggcttcagcagagcgcagataccaaatactgttcttctagtgtagccgtagttaggccaccacttcaagaactctgtagcaccgcctacatacctcgctctgctaatcctgttaccagtggctgctgccagtggcgataagtcgtgtcttaccgggttggactcaagacgatagttaccggataaggcgcagcggtcgggctgaacggggggttcgtgcacacagcccagcttggagcgaacgacctacaccgaactgagatacctacagcgtgagctatgagaaagcgccacgcttcccgaagggagaaaggcggacaggtatccggtaagcggcagggtcggaacaggagagcgcacgagggagcttccagggggaaacgcctggtatctttatagtcctgtcgggtttcgccacctctgacttgagcgtcgatttttgtgatgctcgtcaggggggcggagcctatggaaaaacgccagcaacgcggcctttttacggttcctggccttttgctggccttttgctcacatgttctttcctgcgttatcccctgattctgtggataaccgtattaccgcctttgagtgagctgataccgctcgccgcagccgaacgaccgagcgcagcgagtcagtgagcgaggaagcggaagagcgcccaatacgcaaaccgcctctccccgcgcgttggccgattcattaatgcagctggcacgacaggtttcccgactggaaagcgggcagtgagcgcaacgcaattaatgtgagttagctcactcattaggcaccccaggctttacactttatgcttccggctcgtatgttgtgtggaattgtgagcggataacaatttcacacaggaaacagctatgaccatgattacgcctctagaaagctttaatacgactcactataaggactcactatttgttttcgcgcccagttgcaaaaagtgtcgacatttgcttctgacacaactgtgttcactagcaacctcaaacagacaccgccaccatgcctgctgctaagagagtgaaactggatggatccgaggaactgctgagcaagaactaccacctggaaaacgaggtggccagactgaagaaaggctctggctctggcggaagcggttctggcggatcaggatctggaagtggcggctctggaagcggaggttctggatctggcgaagaactgctgtctaagaattatcacctcgagaacgaagtggctcggctcaagaaaggcagtggcagcggaggaagtggatccggcggtagtggtagtggaagcggcggatccggctcaggcggatctggttcaggggaagaactcctctccaaaaactaccatctcgagaatgaggtcgcccgcctgaaaaaaggatcaggttccggtggttctggcagcggtggttcaggctcaggcagcggcggtagcggtagcggtggaagcggaagcggagaagaacttctcagcaaaaattaccacttggagaatgaagttgcaagactcaaaaaaggttccggcagtggcggcagcggcagcggcggatctggtagtggatctggtggcagtggttcaggcggaagtggtagcggagaggaattgctctcaaagaactatcatttggagaacgaggttgcacgcttgaagaaaggcagcggatcaggcggatctggcagcggtggatctggttctggatccggcggctccggtagtggtggaagtggctctggggaagaattgcttagcaagaattatcatcttgaaaatgaggttgccaggcttaaaaaaggcagtggctccggcggatccggaagcggaggcagcggatctggatctggtggttcaggatctggcggttctggtagcggggaagaactgttgagtaaaaactatcaccttgagaacgaggtcgcaaggttgaaaaaaggatccggctctggcggctccggaagtggcggatctggctccggtagcggaggatcaggatccggcggaagcggatcaggcgaggaactgctttccaaaaattaccaccttgaaaacgaagtcgcccgcctcaagaaaggttctggcagcggaggctctggcagtggtggtagcggaagtggaagtggtggcagtggtagcggtggatctggaagcggcgaggaactcctgtcaaagaattaccatctcgaaaacgaggtcgcaaggctcaagaaaggctcaggatcaggcggctctggatccggcggttctggttccggctcaggtggaagtggatctggcggctcaggttccggcgaagaattgctttccaagaactaccatttggaaaatgaagtcgctcgtttgaagaaaggttcaggctccggcccaaaaaagaagagaaaggtaatggacaagaagtacagcatcggcctggccatcggcaccaactctgtgggctgggccgtgatcaccgacgagtacaaggtgcccagcaagaaattcaaggtgctgggcaacaccgaccggcacagcatcaagaagaacctgatcggcgccctgctgttcgacagcggagaaacagccgaggccacccggctgaagagaaccgccagaagaagatacaccagacggaagaaccggatctgctatctgcaagagatcttcagcaacgagatggccaaggtggacgacagcttcttccacagactggaagagtccttcctggtggaagaggataagaagcacgagcggcaccccatcttcggcaacatcgtggacgaggtggcctaccacgagaagtaccccaccatctaccacctgagaaagaaactggtggacagcaccgacaaggccgacctgcggctgatctatctggccctggcccacatgatcaagttccggggccacttcctgatcgagggcgacctgaaccccgacaacagcgacgtggacaagctgttcatccagctggtgcagacctacaaccagctgttcgaggaaaaccccatcaacgccagcggcgtggacgccaaggccatcctgtctgccagactgagcaagagcagacggctggaaaatctgatcgcccagctgcccggcgagaagaagaatggcctgttcggcaacctgattgccctgagcctgggcctgacccccaacttcaagagcaacttcgacctggccgaggatgccaaactgcagctgagcaaggacacctacgacgacgacctggacaacctgctggcccagatcggcgaccagtacgccgacctgtttctggccgccaagaacctgtccgacgccatcctgctgagcgacatcctgagagtgaacaccgagatcaccaaggcccccctgagcgcctctatgatcaagagatacgacgagcaccaccaggacctgaccctgctgaaagctctcgtgcggcagcagctgcctgagaagtacaaagagattttcttcgaccagagcaagaacggctacgccggctacatcgatggcggagccagccaggaagagttctacaagttcatcaagcccatcctggaaaagatggacggcaccgaggaactgctcgtgaagctgaacagagaggacctgctgcggaagcagcggaccttcgacaacggcagcatcccccaccagatccacctgggagagctgcacgccattctgcggcggcaggaagatttttacccattcctgaaggacaaccgggaaaagatcgagaagatcctgaccttccgcatcccctactacgtgggccctctggccaggggaaacagcagattcgcctggatgaccagaaagagcgaggaaaccatcaccccctggaacttcgaggaagtggtggacaagggcgccagcgcccagagcttcatcgagcggatgaccaacttcgataagaacctgcccaacgagaaggtgctgcccaagcacagcctgctgtacgagtacttcaccgtgtacaacgagctgaccaaagtgaaatacgtgaccgagggaatgagaaagcccgccttcctgagcggcgagcagaaaaaagccatcgtggacctgctgttcaagaccaaccggaaagtgaccgtgaagcagctgaaagaggactacttcaagaaaatcgagtgcttcgactccgtggaaatctccggcgtggaagatcggttcaacgcctccctgggcacataccacgatctgctgaaaattatcaaggacaaggacttcctggacaatgaggaaaacgaggacattctggaagatatcgtgctgaccctgacactgtttgaggacagagagatgatcgaggaacggctgaaaacctatgcccacctgttcgacgacaaagtgatgaagcagctgaagcggcggagatacaccggctggggcaggctgagccggaagctgatcaacggcatccgggacaagcagtccggcaagacaatcctggatttcctgaagtccgacggcttcgccaacagaaacttcatgcagctgatccacgacgacagcctgacctttaaagaggacatccagaaagcccaggtgtccggccagggcgatagcctgcacgagcacattgccaatctggccggcagccccgccattaagaagggcatcctgcagacagtgaaggtggtggacgagctcgtgaaagtgatgggccggcacaagcccgagaacatcgtgatcgaaatggccagagagaaccagaccacccagaagggacagaagaacagccgcgagagaatgaagcggatcgaagagggcatcaaagagctgggcagccagatcctgaaagaacaccccgtggaaaacacccagctgcagaacgagaagctgtacctgtactacctgcagaatgggcgggatatgtacgtggaccaggaactggacatcaaccggctgtccgactacgatgtggacgctatcgtgcctcagagctttctgaaggacgactccatcgataacaaagtgctgactcggagcgacaagaaccggggcaagagcgacaacgtgccctccgaagaggtcgtgaagaagatgaagaactactggcgccagctgctgaatgccaagctgattacccagaggaagttcgacaatctgaccaaggccgagagaggcggcctgagcgaactggataaggccggcttcatcaagagacagctggtggaaacccggcagatcacaaagcacgtggcacagatcctggactcccggatgaacactaagtacgacgagaacgacaaactgatccgggaagtgaaagtgatcaccctgaagtccaagctggtgtccgatttccggaaggatttccagttttacaaagtgcgcgagatcaacaactaccaccacgcccacgacgcctacctgaacgccgtcgtgggaaccgccctgatcaaaaagtaccctaagctggaaagcgagttcgtgtacggcgactacaaggtgtacgacgtgcggaagatgatcgccaagagcgagcaggaaatcggcaaggctaccgccaagtacttcttctacagcaacatcatgaactttttcaagaccgagattaccctggccaacggcgagatccggaagcggcctctgatcgagacaaacggcgaaacaggcgagatcgtgtgggataagggccgggactttgccaccgtgcggaaagtgctgtctatgccccaagtgaatatcgtgaaaaagaccgaggtgcagacaggcggcttcagcaaagagtctatcctgcccaagaggaacagcgacaagctgatcgccagaaagaaggactgggaccctaagaagtacggcggcttcgacagccccaccgtggcctattctgtgctggtggtggccaaagtggaaaagggcaagtccaagaaactgaagagtgtgaaagagctgctggggatcaccatcatggaaagaagcagcttcgagaagaatcccatcgactttctggaagccaagggctacaaagaagtgaaaaaggacctgatcatcaagctgcctaagtactccctgttcgagctggaaaacggccggaagagaatgctggcctctgccggcgaactgcagaagggaaacgaactggccctgccctccaaatatgtgaacttcctgtacctggccagccactatgagaagctgaagggctcccccgaggataatgagcagaaacagctgtttgtggaacagcacaaacactacctggacgagatcatcgagcagatcagcgagttctccaagagagtgatcctggccgacgctaatctggacaaggtgctgagcgcctacaacaagcacagagacaagcctatcagagagcaggccgagaatatcatccacctgtttaccctgaccaatctgggagcccctgccgccttcaagtactttgacaccaccatcgaccggaagaggtacaccagcaccaaagaggtgctggacgccaccctgatccaccagagcatcaccggcctgtacgagacacggatcgacctgtctcagctgggaggcgacgcctatccctatgacgtgcccgattatgccagcctgggcagcggctcccccaagaaaaaacgcaaggtggaagatcctaagaaaaagcggaaagtggacggcagcggcagcgagacccccggtaccagcgagagcgccacccccgagagcatgaacaattcccagggaagagtgaccttcgaggatgtcactgtgaacttcacccagggggagtggcagcggctgaatcccgaacagagaaacttgtacagggatgtgatgctggagaattacagcaaccttgtctctgtgggacaaggggaaaccaccaaacccgatgtgatcttgaggttggaacaaggaaaggagccatggttggaggaagaggaagtgctgggaagtggccgtgcagaaaaaaatggggacattggagggcagatttggaagccaaaggatgtgaaagagagtctcctcgagggaagcggagctactaacttcagcctgctgaagcaggctggagacgtggaggagaaccctggacctatgcctgctgctaagagagtgaaactggatggatccaaccatgaccaggaatttgaccccccaaaggtttacccacctgtgccagctgagaagaggaagcccatccgcgtgctgtctctctttgatgggattgctacagggctcctggtgctgaaggacctgggcatccaagtggaccgctacattgcctccgaggtgtgtgaggactccatcacggtgggcatggtgcggcaccagggaaagatcatgtacgtcggggacgtccgcagcgtcacacagaagcatatccaggagtggggcccattcgacctggtgattggaggcagtccctgcaatgacctctccattgtcaaccctgcccgcaagggactttatgagggtactggccgcctcttctttgagttctaccgcctcctgcatgatgcgcggcccaaggagggagatgatcgccccttcttctggctctttgagaatgtggtggccatgggcgttagtgacaagagggacatctcgcgatttcttgagtctaaccccgtgatgattgacgccaaagaagtgtctgctgcacacagggcccgttacttctggggtaaccttcctggcatgaacaggcctttggcatccactgtgaatgataagctggagctgcaagagtgtctggagcacggcagaatagccaagttcagcaaagtgaggaccattaccaccaggtcaaactctataaagcagggcaaagaccagcatttccccgtgttcatgaacgagaaggaggacatcctgtggtgcactgaaatggaaagggtgtttggcttccccgtccactacacagacgtctccaacatgagccgcttggcgaggcagagactgctgggccgatcgtggagcgtgccggtcatccgccacctcttcgctccgctgaaggaatattttgcttgtgtgtctagcggcaatagtaacgctaacagccgcgggccgagcttcagcagcggcctggtgccgttaagcttgcgcggcagccatatgttcgaaaccgtgcctgtgtggaggagacagccagtccgggtgctgtccctttttgaagacatcaagaaagagctgacgagtttgggctttttggaaagtggttctgacccgggacaactgaagcatgtggttgatgtcacagacacagtgaggaaggatgtggaggagtggggacccttcgatcttgtgtacggcgccacacctcccctgggccacacctgtgaccgtcctcccagctggtacctgttccagttccaccggctcctgcagtacgcacggcccaagccaggcagccccaggcccttcttctggatgttcgtggacaatctggtgctgaacaaggaagacctggacgtcgcatctcgcttcctggagatggagccagtcaccatcccagatgtccacggcggatccttgcagaatgctgtccgcgtgtggagcaacatcccagccataaggagcagcaggcactgggctctggtttcggaagaagaattgtccctgctggcccagaacaagcagagctcgaagctcgcggccaagtggcccaccaagctggtgaagaactgctttctccccctaagagaatatttcaagtatttttcaggagggccgagctctggcgcacccccaccaagtggagggtctcctgccgggtccccaacatctactgaagaaggcaccagcgaatccgcaacgcccgagtcaggccctggtacctccacagaaccatctgaaggtagtgcgcctggttccccagctggaagccctacttccaccgaagaaggcacgtcaaccgaaccaagtgaaggatctgcccctgggaccagcactgaaccatctgagccaaaaaagaagagaaaggtaccatctgagggccccgacatcgtgatgacccagagccccagcagcctgagcgccagcgtgggcgaccgcgtgaccatcacctgccgcagcagcaccggcgccgtgaccaccagcaactacgccagctgggtgcaggagaagcccggcaagctgttcaagggcctgatcggcggcaccaacaaccgcgcccccggcgtgcccagccgcttcagcggcagcctgatcggcgacaaggccaccctgaccatcagcagcctgcagcccgaggacttcgccacctacttctgcgccctgtggtacagcaaccactgggtgttcggccagggcaccaaggtggagctgaagcgcggcggcggcggcagcggcggcggcggcagcggcggcggcggcagcagcggcggcggcagcgaggtgaagctgctggagagcggcggcggcctggtgcagcccggcggcagcctgaagctgagctgcgccgtgagcggcttcagcctgaccgactacggcgtgaactgggtgcgccaggcccccggccgcggcctggagtggatcggcgtgatctggggcgacggcatcaccgactacaacagcgccctgaaggaccgcttcatcatcagcaaggacaacggcaagaacaccgtgtacctgcagatgagcaaggtgcgcagcgacgacaccgccctgtactactgcgtgaccggcctgttcgactactggggccagggcaccctggtgaccgtgagcagctacccatacgatgttccagattacgctggtggaggcggaggttctgggggaggaggtagtggcggtggtggttcaggaggcggcggaagctgataataggatcccaagcacgcagcaatgcagctcaaaacgcttagcctagccacacccccacgggaaacagcagtgattaacctttagcaataaacgaaagtttaactaagctatactaaccccagggttggtcaatttcgtgccagccacaccctggtactgcatgcacgcaatgctagctgcccctttcccgtcctgggcaccccgagtctcccccgaccccgggtcccaggtatgctcccacctccacctgccccactcaccacctctgctagttccagacacctccgagacgaggaaaaaaaaaaaaaaaaaaaaaaaaaaaaaaaaaaaaaaaaaaaaaaaaaaaaaaaaaaaaaaaaaaaaaaaaaaaaaaaaaaaaaaaaaaaaaaaaaaaaaaaaaaaaaaaaaaaaaaaaaaaaaaaaaaaaaaaaaaaaaaaaaaaaaaaaaaaaaaaaaaaaaaaaaaaaaaaaaaaaaaaaaaaaaaaaaaaaaaaaaaaaaaaaaaaaaaaaaaaaaaaaaaaaaaaaaaaaaaaaaaaaaaaaaaaaaaaaaaaaaaaaaaaaaaaaaaaaaaaaaaaaaaaaaaaaaaaaaaaaaaaaaaaaaaaaaaaaaaaaaaaaaaaaaaaaaaaaaaaaaaaaaaaaaaaaaaaaaaaaaaaaaaaaaaaaaaaaaaaaaaaaaaaaaaaaaaccgtcttcaagctttctagaaattcactggccgtcgttttacaacgtcgtgactgggaaaaccctggcgttacccaacttaatcgccttgcagcacatccccctttcgccagctggcgtaatagcgaagaggcccgcaccgatcgcccttcccaacagttgcgcagcctgaatggcgaatggcgcctgatgcggtattttctccttacgcatctgtgcggtatttcacaccgcatatggtgcactctcagtacaatctgctctgatgccgcatagttaagccagccccgacacccgccaacacccgctgacgcgccctgacgggcttgtctgctcccggcatccgcttacagacaagctgtgaccgtctccgggagctgcatgtgtcagaggttttcaccgtcatcaccgaaacgcgcgagacgaaagggcctcgtgatacgcctatttttataggttaatgtcatgataataatggtttcttagacgtcaggtggcacttttcggggaaatgtgcgcggaacccctatttgtttatttttctaaatacattcaaatatgtatccgctcatgagacaataaccctgataaatgcttcaataatattgaaaaaggaagagtatgagtattcaacatttccgtgtcgcccttattcccttttttgcggcattttgccttcctgtttttgctcacccagaaacgctggtgaaagtaaaagatgctgaagatcagttgggtgcacgagtgggttacatcgaactggatctcaacagcggtaagatccttgagagttttcgccccgaagaacgttttccaatgatgagcacttttaaagttctgctatgtggcgcggtattatcccgtattgacgccgggcaagagcaactcggtcgccgcatacactattctcagaatgacttggttgagtactcaccagtcacagaaaagcatcttacggatggcatgacagtaagagaattatgcagtgctgccataaccatgagtgataacactgcggccaacttacttctgacaacgatcggaggaccgaaggagctaaccgcttttttgcacaacatgggggatcatgtaactcgccttgatcgttgggaaccggagctgaatgaagccataccaaacgacgagcgtgacaccacgatgcctgtagcaatggcaacaacgttgcgcaaactattaactggcgaactacttactctagcttcccggcaacaattaatagactggatggaggcggataaagttgcaggaccacttctgcgctcggcccttccggctggctggtttattgctgataaatctggagccggtgagcgtgggtctcgcggtatcattgcagcactggggccagatggtaagccctcccgtatcgtagttatctacacgacggggagtcaggcaactatggatgaacgaaatagacagatcgc

SEQ ID NO: 225 - DNA, 10929 bp, synthetic construct
  misc_feature 1..10929: note = DNA of V31_scFV-hD3L-D3a-2a-3xGCN4-dCas9-KRAB
  source 1..10929: mol_type = other DNA
atcgtgctgaccctgacactgtttgaggacagagagatgatcgaggaacggctgaaaacctatgcccacctgttcgacgacaaagtgatgaagcagctgaagcggcggagatacaccggctggggcaggctgagccggaagctgatcaacggcatccgggacaagcagtccggcaagacaatcctggatttcctgaagtccgacggcttcgccaacagaaacttcatgcagctgatccacgacgacagcctgacctttaaagaggacatccagaaagcccaggtgtccggccagggcgatagcctgcacgagcacattgccaatctggccggcagccccgccattaagaagggcatcctgcagacagtgaaggtggtggacgagctcgtgaaagtgatgggccggcacaagcccgagaacatcgtgatcgaaatggccagagagaaccagaccacccagaagggacagaagaacagccgcgagagaatgaagcggatcgaagagggcatcaaagagctgggcagccagatcctgaaagaacaccccgtggaaaacacccagctgcagaacgagaagctgtacctgtactacctgcagaatgggcgggatatgtacgtggaccaggaactggacatcaaccggctgtccgactacgatgtggacgctatcgtgcctcagagctttctgaaggacgactccatcgataacaaagtgctgactcggagcgacaagaaccggggcaagagcgacaacgtgccctccgaagaggtcgtgaagaagatgaagaactactggcgccagctgctgaatgccaagctgattacccagaggaagttcgacaatctgaccaaggccgagagaggcggcctgagcgaactggataaggccggcttcatcaagagacagctggtggaaacccggcagatcacaaagcacgtggcacagatcctggactcccggatgaacactaagtacgacgagaacgacaaactgatccgggaagtgaaagtgatcaccctgaagtccaagctggtgtccgatttccggaaggatttccagttttacaaagtgcgcgagatcaacaactaccaccacgcccacgacgcctacctgaacgccgtcgtgggaaccgccctgatcaaaaagtaccctaagctggaaagcgagttcgtgtacggcgactacaaggtgtacgacgtgcggaagatgatcgccaagagcgagcaggaaatcggcaaggctaccgccaagtacttcttctacagcaacatcatgaactttttcaagaccgagattaccctggccaacggcgagatccggaagcggcctctgatcgagacaaacggcgaaacaggcgagatcgtgtgggataagggccgggactttgccaccgtgcggaaagtgctgtctatgccccaagtgaatatcgtgaaaaagaccgaggtgcagacaggcggcttcagcaaagagtctatcctgcccaagaggaacagcgacaagctgatcgccagaaagaaggactgggaccctaagaagtacggcggcttcgacagccccaccgtggcctattctgtgctggtggtggccaaagtggaaaagggcaagtccaagaaactgaagagtgtgaaagagctgctggggatcaccatcatggaaagaagcagcttcgagaagaatcccatcgactttctggaagccaagggctacaaagaagtgaaaaaggacctgatcatcaagctgcctaagtactccctgttcgagctggaaaacggccggaagagaatgctggcctctgccggcgaactgcagaagggaaacgaactggccctgccctccaaatatgtgaacttcctgtacctggccagccactatgagaagctgaagggctcccccgaggataatgagcagaaacagctgtttgtggaacagcacaaacactacctggacgagatcatcgagcagatcagcgagttctccaagagagtgatcctggccgacgctaatctggacaaggtgctgagcgcctacaacaagcacagagacaagcctatcagagagcaggccgagaatatcatccacctgtttaccctgaccaatctgggagcccctgccgccttcaagtactttgacaccaccatcgaccggaagaggtacaccagcaccaaagaggtgctggacgccaccctgatccaccagagcatcaccggcctgtacgagacacggatcgacctgtctcagctgggaggcgacgcctatccctatgacgtgcccgattatgccagcctgggcagcggctcccccaagaaaaaacgcaaggtggaagatcctaagaaaaagcggaaagtggacggcagcggcagcgagacccccggtaccagcgagagcgccacccccgagagccggacactggtgaccttcaaggatgtatttgtggacttcaccagggaggagtggaagctgctggacactgctcagcagatcgtgtacagaaatgtgatgctggagaactataagaacctggtttccttgggttatcagcttactaagccagatgtgatcctccggttggagaagggagaagagccctgagatcccaagcacgcagcaatgcagctcaaaacgcttagcctagccacacccccacgggaaacagcagtgattaacctttagcaataaacgaaagtttaactaagctatactaaccccagggttggtcaatttcgtgccagccacaccctggtactgcatgcacgcaatgctagctgcccctttcccgtcctgggcaccccgagtctcccccgaccccgggtcccaggtatgctcccacctccacctgccccactcaccacctctgctagttccagacacctccgagacgaggaaaaaaaaaaaaaaaaaaaaaaaaaaaaaaaaaaaaaaaaaaaaaaaaaaaaaaaaaaaaaaaaaaaaaaaaaaaaaaaaaaaaaaaaaaaaaaaaaaaaaaaaaaaaaaaaaaaaaaaaaaaaaaaaaaaaaaaaaaaaaaaaaaaaaaaaaaaaaaaaaaaaaaaaaaaaaaaaaaaaaaaaaaaaaaaaaaaaaaaaaaaaaaaaaaaaaaaaaaaaaaaaaaaaaaaaaaaaaaaaaaaaaaaaaaaaaaaaaaaaaaaaaaaaaaaaaaaaaaaaaaaaaaaaaaaaaaaaaaaaaaaaaaaaaaaaaaaaaaaaaaaaaaaaaaaaaaaaaaaaaaaaaaaaaaaaaaaaaaaaaaaaaaaaaaaaaaaaaaaaaaaaaaaaaaaaaaccgtcttcaagctttctagaaattcactggccgtcgttttacaacgtcgtgactgggaaaaccctggcgttacccaacttaatcgccttgcagcacatccccctttcgccagctggcgtaatagcgaagaggcccgcaccgatcgcccttcccaacagttgcgcagcctgaatggcgaatggcgcctgatgcggtattttctccttacgcatctgtgcggtatttcacaccgcatatggtgcactctcagtacaatctgctctgatgccgcatagttaagccagccccgacacccgccaacacccgctgacgcgccctgacgggcttgtctgctcccggcatccgcttacagacaagctgtgaccgtctccgggagctgcatgtgtcagaggttttcaccgtcatcaccgaaacgcgcgagacgaaagggcctcgtgatacgcctatttttataggttaatgtcatgataataatggtttcttagacgtcaggtggcacttttcggggaaatgtgcgcggaacccctatttgtttatttttctaaatacattcaaatatgtatccgctcatgagacaataaccctgataaatgcttcaataatattgaaaaaggaagagtatgagtattcaacatttccgtgtcgcccttattcccttttttgcggcattttgccttcctgtttttgctcacccagaaacgctggtgaaagtaaaagatgctgaagatcagttgggtgcacgagtgggttacatcgaactggatctcaacagcggtaagatccttgagagttttcgccccgaagaacgttttccaatgatgagcacttttaaagttctgctatgtggcgcggtattatcccgtattgacgccgggcaagagcaactcggtcgccgcatacactattctcagaatgacttggttgagtactcaccagtcacagaaaagcatcttacggatggcatgacagtaagagaattatgcagtgctgccataaccatgagtgataacactgcggccaacttacttctgacaacgatcggaggaccgaaggagctaaccgcttttttgcacaacatgggggatcatgtaactcgccttgatcgttgggaaccggagctgaatgaagccataccaaacgacgagcgtgacaccacgatgcctgtagcaatggcaacaacgttgcgcaaactattaactggcgaactacttactctagcttcccggcaacaattaatagactggatggaggcggataaagttgcaggaccacttctgcgctcggcccttccggctggctggtttattgctgataaatctggagccggtgagcgtgggtctcgcggtatcattgcagcactggggccagatggtaagccctcccgtatcgtagttatctacacgacggggagtcaggcaactatggatgaacgaaatagacagatcgctgagataggtgcctcactgattaagcattggtaactgtcagaccaagtttactcatatatactttagattgatttaaaacttcatttttaatttaaaaggatctaggtgaagatcctttttgataatctcatgaccaaaatcccttaacgtgagttttcgttccactgagcgtcagaccccgtagaaaagatcaaaggatcttcttgagatcctttttttctgcgcgtaatctgctgcttgcaaacaaaaaaaccaccgctaccagcggtggtttgtttgccggatcaagagctaccaactctttttccgaaggtaactggcttcagcagagcgcagataccaaatactgttcttctagtgtagccgtagttaggccaccacttcaagaactctgtagcaccgcctacatacctcgctctgctaatcctgttaccagtggctgctgccagtggcgataagtcgtgtcttaccgggttggactcaagacgatagttaccggataaggcgcagcggtcgggctgaacggggggttcgtgcacacagcccagcttggagcgaacgacctacaccgaactgagatacctacagcgtgagctatgagaaagcgccacgcttcccgaagggagaaaggcggacaggtatccggtaagcggcagggtcggaacaggagagcgcacgagggagcttccagggggaaacgcctggtatctttatagtcctgtcgggtttcgccacctctgacttgagcgtcgatttttgtgatgctcgtcaggggggcggagcctatggaaaaacgccagcaacgcggcctttttacggttcctggccttttgctggccttttgctcacatgttctttcctgcgttatcccctgattctgtggataaccgtattaccgcctttgagtgagctgataccgctcgccgcagccgaacgaccgagcgcagcgagtcagtgagcgaggaagcggaagagcgcccaatacgcaaaccgcctctccccgcgcgttggccgattcattaatgcagctggcacgacaggtttcccgactggaaagcgggcagtgagcgcaacgcaattaatgtgagttagctcactcattaggcaccccaggctttacactttatgcttccggctcgtatgttgtgtggaattgtgagcggataacaatttcacacaggaaacagctatgaccatgattacgcctctagaaagctttaatacgactcactataaggactcactatttgttttcgcgcccagttgcaaaaagtgtcgacatttgcttctgacacaactgtgttcactagcaacctcaaacagacaccgccaccatgcctgctgctaagagagtgaaactggatggatccggccccgacatcgtgatgacccagagccccagcagcctgagcgccagcgtgggcgaccgcgtgaccatcacctgccgcagcagcaccggcgccgtgaccaccagcaactacgccagctgggtgcaggagaagcccggcaagctgttcaagggcctgatcggcggcaccaacaaccgcgcccccggcgtgcccagccgcttcagcggcagcctgatcggcgacaaggccaccctgaccatcagcagcctgcagcccgaggacttcgccacctacttctgcgccctgtggtacagcaaccactgggtgttcggccagggcaccaaggtggagctgaagcgcggcggcggcggcagcggcggcggcggcagcggcggcggcggcagcagcggcggcggcagcgaggtgaagctgctggagagcggcggcggcctggtgcagcccggcggcagcctgaagctgagctgcgccgtgagcggcttcagcctgaccgactacggcgtgaactgggtgcgccaggcccccggccgcggcctggagtggatcggcgtgatctggggcgacggcatcaccgactacaacagcgccctgaaggaccgcttcatcatcagcaaggacaacggcaagaacaccgtgtacctgcagatgagcaaggtgcgcagcgacgacaccgccctgtactactgcgtgaccggcctgttcgactactggggccagggcaccctggtgaccgtgagcagctacccatacgatgttccagattacgctggtggaggcggaggttctgggggaggaggtagtggcggtggtggttcaggaggcggcggaagcatgttcgaaaccgtgcctgtgtggaggagacagccagtccgggtgctgtccctttttgaagacatcaagaaagagctgacgagtttgggctttttggaaagtggttctgacccgggacaactgaagcatgtggttgatgtcacagacacagtgaggaaggatgtggaggagtggggacccttcgatcttgtgtacggcgccacacctcccctgggccacacctgtgaccgtcctcccagctggtacctgttccagttccaccggctcctgcagtacgcacggcccaagccaggcagccccaggcccttcttctggatgttcgtggacaatctggtgctgaacaaggaagacctggacgtcgcatctcgcttcctggagatggagccagtcaccatcccagatgtccacggcggatccttgcagaatgctgtccgcgtgtggagcaacatcccagccataaggagcagcaggcactgggctctggtttcggaagaagaattgtccctgctggcccagaacaagcagagctcgaagctcgcggccaagtggcccaccaagctggtgaagaactgctttctccccctaagagaatatttcaagtatttttcaacagaactcacttcctctttatctagcggcaatagtaacgctaacagccgcgggccgagcttcagcagcggcctggtgccgttaagcttgcgcggcagccatatgaaccatgaccaggaatttgaccccccaaaggtttacccacctgtgccagctgagaagaggaagcccatccgcgtgctgtctctctttgatgggattgctacagggctcctggtgctgaaggacctgggcatccaagtggaccgctacattgcctccgaggtgtgtgaggactccatcacggtgggcatggtgcggcaccagggaaagatcatgtacgtcggggacgtccgcagcgtcacacagaagcatatccaggagtggggcccattcgacctggtgattggaggcagtccctgcaatgacctctccattgtcaaccctgcccgcaagggactttatgagggtactggccgcctcttctttgagttctaccgcctcctgcatgatgcgcggcccaaggagggagatgatcgccccttcttctggctctttgagaatgtggtggccatgggcgttagtgacaagagggacatctcgcgatttcttgagtctaaccccgtgatgattgacgccaaagaagtgtctgctgcacacagggcccgttacttctggggtaaccttcctggcatgaacaggcctttggcatccactgtgaatgataagctggagctgcaagagtgtctggagcacggcagaatagccaagttcagcaaagtgaggaccattaccaccaggtcaaactctataaagcagggcaaagaccagcatttccccgtcttcatgaacgagaaggaggacatcctgtggtgcactgaaatggaaagggtgtttggcttccccgtccactacacagacgtctccaacatgagccgcttggcgaggcagagactgctgggccgatcgtggagcgtgccggtcatccgccacctcttcgctccgctgaaggaatattttgcttgtgtgggaagcggagctactaacttcagcctgctgaagcaggctggagacgtggaggagaaccctggacctatgcctgctgctaagagagtgaaactggatggatccgaggaactgctgagcaagaactaccacctggaaaacgaggtggccagactgaagaaaggctctggctctggcggaagcggttctggcggatcaggatctggaagtggcggctctggaagcggaggttctggatctggcgaagaactgctgtctaagaattatcacctcgagaacgaagtggctcggctcaagaaaggcagtggcagcggaggaagtggatccggcggtagtggtagtggaagcggcggatccggctcaggcggatctggttcaggggaagaactcctctccaaaaactaccatctcgagaatgaggtcgcccgcctgaaaaaaggatcaggttccggtggttctggcagcggtggttcaggctcaggcagcggcggtagcggtagcggtggaagcggaagcggaccaaaaaagaagagaaaggtaatggacaagaagtacagcatcggcctggccatcggcaccaactctgtgggctgggccgtgatcaccgacgagtacaaggtgcccagcaagaaattcaaggtgctgggcaacaccgaccggcacagcatcaagaagaacctgatcggcgccctgctgttcgacagcggagaaacagccgaggccacccggctgaagagaaccgccagaagaagatacaccagacggaagaaccggatctgctatctgcaagagatcttcagcaacgagatggccaaggtggacgacagcttcttccacagactggaagagtccttcctggtggaagaggataagaagcacgagcggcaccccatcttcggcaacatcgtggacgaggtggcctaccacgagaagtaccccaccatctaccacctgagaaagaaactggtggacagcaccgacaaggccgacctgcggctgatctatctggccctggcccacatgatcaagttccggggccacttcctgatcgagggcgacctgaaccccgacaacagcgacgtggacaagctgttcatccagctggtgcagacctacaaccagctgttcgaggaaaaccccatcaacgccagcggcgtggacgccaaggccatcctgtctgccagactgagcaagagcagacggctggaaaatctgatcgcccagctgcccggcgagaagaagaatggcctgttcggcaacctgattgccctgagcctgggcctgacccccaacttcaagagcaacttcgacctggccgaggatgccaaactgcagctgagcaaggacacctacgacgacgacctggacaacctgctggcccagatcggcgaccagtacgccgacctgtttctggccgccaagaacctgtccgacgccatcctgctgagcgacatcctgagagtgaacaccgagatcaccaaggcccccctgagcgcctctatgatcaagagatacgacgagcaccaccaggacctgaccctgctgaaagctctcgtgcggcagcagctgcctgagaagtacaaagagattttcttcgaccagagcaagaacggctacgccggctacatcgatggcggagccagccaggaagagttctacaagttcatcaagcccatcctggaaaagatggacggcaccgaggaactgctcgtgaagctgaacagagaggacctgctgcggaagcagcggaccttcgacaacggcagcatcccccaccagatccacctgggagagctgcacgccattctgcggcggcaggaagatttttacccattcctgaaggacaaccgggaaaagatcgagaagatcctgaccttccgcatcccctactacgtgggccctctggccaggggaaacagcagattcgcctggatgaccagaaagagcgaggaaaccatcaccccctggaacttcgaggaagtggtggacaagggcgccagcgcccagagcttcatcgagcggatgaccaacttcgataagaacctgcccaacgagaaggtgctgcccaagcacagcctgctgtacgagtacttcaccgtgtacaacgagctgaccaaagtgaaatacgtgaccgagggaatgagaaagcccgccttcctgagcggcgagcagaaaaaagccatcgtggacctgctgttcaagaccaaccggaaagtgaccgtgaagcagctgaaagaggactacttcaagaaaatcgagtgcttcgactccgtggaaatctccggcgtggaagatcggttcaacgcctccctgggcacataccacgatctgctgaaaattatcaaggacaaggacttcctggacaatgaggaaaacgaggacattctggaagat

SEQ ID NO: 226 - DNA, 10953 bp, synthetic construct
  misc_feature 1..10953: note = DNA of V32_1xGCN4-ZIM3-2a-D3a-hD3L-dCas9-scFv
  source 1..10953: mol_type = other DNA
atctaggtgaagatcctttttgataatctcatgaccaaaatcccttaacgtgagttttcgttccactgagcgtcagaccccgtagaaaagatcaaaggatcttcttgagatcctttttttctgcgcgtaatctgctgcttgcaaacaaaaaaaccaccgctaccagcggtggtttgtttgccggatcaagagctaccaactctttttccgaaggtaactggcttcagcagagcgcagataccaaatactgttcttctagtgtagccgtagttaggccaccacttcaagaactctgtagcaccgcctacatacctcgctctgctaatcctgttaccagtggctgctgccagtggcgataagtcgtgtcttaccgggttggactcaagacgatagttaccggataaggcgcagcggtcgggctgaacggggggttcgtgcacacagcccagcttggagcgaacgacctacaccgaactgagatacctacagcgtgagctatgagaaagcgccacgcttcccgaagggagaaaggcggacaggtatccggtaagcggcagggtcggaacaggagagcgcacgagggagcttccagggggaaacgcctggtatctttatagtcctgtcgggtttcgccacctctgacttgagcgtcgatttttgtgatgctcgtcaggggggcggagcctatggaaaaacgccagcaacgcggcctttttacggttcctggccttttgctggccttttgctcacatgttctttcctgcgttatcccctgattctgtggataaccgtattaccgcctttgagtgagctgataccgctcgccgcagccgaacgaccgagcgcagcgagtcagtgagcgaggaagcggaagagcgcccaatacgcaaaccgcctctccccgcgcgttggccgattcattaatgcagctggcacgacaggtttcccgactggaaagcgggcagtgagcgcaacgcaattaatgtgagttagctcactcattaggcaccccaggctttacactttatgcttccggctcgtatgttgtgtggaattgtgagcggataacaatttcacacaggaaacagctatgaccatgattacgcctctagaaagctttaatacgactcactataaggactcactatttgttttcgcgcccagttgcaaaaagtgtcgacatttgcttctgacacaactgtgttcactagcaacctcaaacagacaccgccaccatgcctgctgctaagagagtgaaactggatggatccgaggaactgctgagcaagaactaccacctggaaaacgaggtggccagactgaagaaaggctctggctctggcggaagcggttctggcggatcaggatctggaagtggcggctctggaagcggaggttctggatctggcatgaacaattcccagggaagagtgaccttcgaggacgtgaccgtgaacttcacccaaggcgagtggcagagactgaaccccgagcagagaaacctgtaccgggacgtgatgctggaaaactacagcaacctggtgtccgtcggccagggcgagacaacaaagcctgacgtgatcctgcggctggaacagggcaaagagccttggctggaagaggaagaggtgctcggatctggcagagccgagaagaatggcgatatcggcggacagatctggaagccaaaggatgtgaaagagagtctcggaagcggagctactaacttcagcctgctgaagcaggctggagacgtggaggagaaccctggacctatgcctgctgctaagagagtgaaactggatggatccaaccatgaccaggaatttgaccccccaaaggtttacccacctgtgccagctgagaagaggaagcccatccgcgtgctgtctctctttgatgggattgctacagggctcctggtgctgaaggacctgggcatccaagtggaccgctacattgcctccgaggtgtgtgaggactccatcacggtgggcatggtgcggcaccagggaaagatcatgtacgtcggggacgtccgcagcgtcacacagaagcatatccaggagtggggcccattcgacctggtgattggaggcagtccctgcaatgacctctccattgtcaaccctgcccgcaagggactttatgagggtactggccgcctcttctttgagttctaccgcctcctgcatgatgcgcggcccaaggagggagatgatcgccccttcttctggctctttgagaatgtggtggccatgggcgttagtgacaagagggacatctcgcgatttcttgagtctaaccccgtgatgattgacgccaaagaagtgtctgctgcacacagggcccgttacttctggggtaaccttcctggcatgaacaggcctttggcatccactgtgaatgataagctggagctgcaagagtgtctggagcacggcagaatagccaagttcagcaaagtgaggaccattaccaccaggtcaaactctataaagcagggcaaagaccagcatttccccgtgttcatgaacgagaaggaggacatcctgtggtgcactgaaatggaaagggtgtttggcttccccgtccactacacagacgtctccaacatgagccgcttggcgaggcagagactgctgggccgatcgtggagcgtgccggtcatccgccacctcttcgctccgctgaaggaatattttgcttgtgtgtctagcggcaatagtaacgctaacagccgcgggccgagcttcagcagcggcctggtgccgttaagcttgcgcggcagccatatgttcgaaaccgtgcctgtgtggaggagacagccagtccgggtgctgtccctttttgaagacatcaagaaagagctgacgagtttgggctttttggaaagtggttctgacccgggacaactgaagcatgtggttgatgtcacagacacagtgaggaaggatgtggaggagtggggacccttcgatcttgtgtacggcgccacacctcccctgggccacacctgtgaccgtcctcccagctggtacctgttccagttccaccggctcctgcagtacgcacggcccaagccaggcagccccaggcccttcttctggatgttcgtggacaatctggtgctgaacaaggaagacctggacgtcgcatctcgcttcctggagatggagccagtcaccatcccagatgtccacggcggatccttgcagaatgctgtccgcgtgtggagcaacatcccagccataaggagcagcaggcactgggctctggtttcggaagaagaattgtccctgctggcccagaacaagcagagctcgaagctcgcggccaagtggcccaccaagctggtgaagaactgctttctccccctaagagaatatttcaagtatttttcaggagggccgagctctggcgcacccccaccaagtggagggtctcctgccgggtccccaacatctactgaagaaggcaccagcgaatccgcaacgcccgagtcaggccctggtacctccacagaaccatctgaaggtagtgcgcctggttccccagctggaagccctacttccaccgaagaaggcacgtcaaccgaaccaagtgaaggatctgcccctgggaccagcactgaaccatctgagccaaaaaagaagagaaaggtaatggacaagaagtacagcatcggcctggccatcggcaccaactctgtgggctgggccgtgatcaccgacgagtacaaggtgcccagcaagaaattcaaggtgctgggcaacaccgaccggcacagcatcaagaagaacctgatcggcgccctgctgttcgacagcggagaaacagccgaggccacccggctgaagagaaccgccagaagaagatacaccagacggaagaaccggatctgctatctgcaagagatcttcagcaacgagatggccaaggtggacgacagcttcttccacagactggaagagtccttcctggtggaagaggataagaagcacgagcggcaccccatcttcggcaacatcgtggacgaggtggcctaccacgagaagtaccccaccatctaccacctgagaaagaaactggtggacagcaccgacaaggccgacctgcggctgatctatctggccctggcccacatgatcaagttccggggccacttcctgatcgagggcgacctgaaccccgacaacagcgacgtggacaagctgttcatccagctggtgcagacctacaaccagctgttcgaggaaaaccccatcaacgccagcggcgtggacgccaaggccatcctgtctgccagactgagcaagagcagacggctggaaaatctgatcgcccagctgcccggcgagaagaagaatggcctgttcggcaacctgattgccctgagcctgggcctgacccccaacttcaagagcaacttcgacctggccgaggatgccaaactgcagctgagcaaggacacctacgacgacgacctggacaacctgctggcccagatcggcgaccagtacgccgacctgtttctggccgccaagaacctgtccgacgccatcctgctgagcgacatcctgagagtgaacaccgagatcaccaaggcccccctgagcgcctctatgatcaagagatacgacgagcaccaccaggacctgaccctgctgaaagctctcgtgcggcagcagctgcctgagaagtacaaagagattttcttcgaccagagcaagaacggctacgccggctacatcgatggcggagccagccaggaagagttctacaagttcatcaagcccatcctggaaaagatggacggcaccgaggaactgctcgtgaagctgaacagagaggacctgctgcggaagcagcggaccttcgacaacggcagcatcccccaccagatccacctgggagagctgcacgccattctgcggcggcaggaagatttttacccattcctgaaggacaaccgggaaaagatcgagaagatcctgaccttccgcatcccctactacgtgggccctctggccaggggaaacagcagattcgcctggatgaccagaaagagcgaggaaaccatcaccccctggaacttcgaggaagtggtggacaagggcgccagcgcccagagcttcatcgagcggatgaccaacttcgataagaacctgcccaacgagaaggtgctgcccaagcacagcctgctgtacgagtacttcaccgtgtacaacgagctgaccaaagtgaaatacgtgaccgagggaatgagaaagcccgccttcctgagcggcgagcagaaaaaagccatcgtggacctgctgttcaagaccaaccggaaagtgaccgtgaagcagctgaaagaggactacttcaagaaaatcgagtgcttcgactccgtggaaatctccggcgtggaagatcggttcaacgcctccctgggcacataccacgatctgctgaaaattatcaaggacaaggacttcctggacaatgaggaaaacgaggacattctggaagatatcgtgctgaccctgacactgtttgaggacagagagatgatcgaggaacggctgaaaacctatgcccacctgttcgacgacaaagtgatgaagcagctgaagcggcggagatacaccggctggggcaggctgagccggaagctgatcaacggcatccgggacaagcagtccggcaagacaatcctggatttcctgaagtccgacggcttcgccaacagaaacttcatgcagctgatccacgacgacagcctgacctttaaagaggacatccagaaagcccaggtgtccggccagggcgatagcctgcacgagcacattgccaatctggccggcagccccgccattaagaagggcatcctgcagacagtgaaggtggtggacgagctcgtgaaagtgatgggccggcacaagcccgagaacatcgtgatcgaaatggccagagagaaccagaccacccagaagggacagaagaacagccgcgagagaatgaagcggatcgaagagggcatcaaagagctgggcagccagatcctgaaagaacaccccgtggaaaacacccagctgcagaacgagaagctgtacctgtactacctgcagaatgggcgggatatgtacgtggaccaggaactggacatcaaccggctgtccgactacgatgtggacgctatcgtgcctcagagctttctgaaggacgactccatcgataacaaagtgctgactcggagcgacaagaaccggggcaagagcgacaacgtgccctccgaagaggtcgtgaagaagatgaagaactactggcgccagctgctgaatgccaagctgattacccagaggaagttcgacaatctgaccaaggccgagagaggcggcctgagcgaactggataaggccggcttcatcaagagacagctggtggaaacccggcagatcacaaagcacgtggcacagatcctggactcccggatgaacactaagtacgacgagaacgacaaactgatccgggaagtgaaagtgatcaccctgaagtccaagctggtgtccgatttccggaaggatttccagttttacaaagtgcgcgagatcaacaactaccaccacgcccacgacgcctacctgaacgccgtcgtgggaaccgccctgatcaaaaagtaccctaagctggaaagcgagttcgtgtacggcgactacaaggtgtacgacgtgcggaagatgatcgccaagagcgagcaggaaatcggcaaggctaccgccaagtacttcttctacagcaacatcatgaactttttcaagaccgagattaccctggccaacggcgagatccggaagcggcctctgatcgagacaaacggcgaaacaggcgagatcgtgtgggataagggccgggactttgccaccgtgcggaaagtgctgtctatgccccaagtgaatatcgtgaaaaagaccgaggtgcagacaggcggcttcagcaaagagtctatcctgcccaagaggaacagcgacaagctgatcgccagaaagaaggactgggaccctaagaagtacggcggcttcgacagccccaccgtggcctattctgtgctggtggtggccaaagtggaaaagggcaagtccaagaaactgaagagtgtgaaagagctgctggggatcaccatcatggaaagaagcagcttcgagaagaatcccatcgactttctggaagccaagggctacaaagaagtgaaaaaggacctgatcatcaagctgcctaagtactccctgttcgagctggaaaacggccggaagagaatgctggcctctgccggcgaactgcagaagggaaacgaactggccctgccctccaaatatgtgaacttcctgtacctggccagccactatgagaagctgaagggctcccccgaggataatgagcagaaacagctgtttgtggaacagcacaaacactacctggacgagatcatcgagcagatcagcgagttctccaagagagtgatcctggccgacgctaatctggacaaggtgctgagcgcctacaacaagcacagagacaagcctatcagagagcaggccgagaatatcatccacctgtttaccctgaccaatctgggagcccctgccgccttcaagtactttgacaccaccatcgaccggaagaggtacaccagcaccaaagaggtgctggacgccaccctgatccaccagagcatcaccggcctgtacgagacacggatcgacctgtctcagctgggaggcgacgcctatccctatgacgtgcccgattatgccagcctgggcagcggctcccccaagaaaaaacgcaaggtggaagatcctaagaaaaagcggaaagtggacggcattggtagtgggagcggccccgacatcgtgatgacccagagccccagcagcctgagcgccagcgtgggcgaccgcgtgaccatcacctgccgcagcagcaccggcgccgtgaccaccagcaactacgccagctgggtgcaggagaagcccggcaagctgttcaagggcctgatcggcggcaccaacaaccgcgcccccggcgtgcccagccgcttcagcggcagcctgatcggcgacaaggccaccctgaccatcagcagcctgcagcccgaggacttcgccacctacttctgcgccctgtggtacagcaaccactgggtgttcggccagggcaccaaggtggagctgaagcgcggcggcggcggcagcggcggcggcggcagcggcggcggcggcagcagcggcggcggcagcgaggtgaagctgctggagagcggcggcggcctggtgcagcccggcggcagcctgaagctgagctgcgccgtgagcggcttcagcctgaccgactacggcgtgaactgggtgcgccaggcccccggccgcggcctggagtggatcggcgtgatctggggcgacggcatcaccgactacaacagcgccctgaaggaccgcttcatcatcagcaaggacaacggcaagaacaccgtgtacctgcagatgagcaaggtgcgcagcgacgacaccgccctgtactactgcgtgaccggcctgttcgactactggggccagggcaccctggtgaccgtgagcagctacccatacgatgttccagattacgctggtggaggcggaggttctgggggaggaggtagtggcggtggtggttcaggaggcggcggaagctagtgagatcccaagcacgcagcaatgcagctcaaaacgcttagcctagccacacccccacgggaaacagcagtgattaacctttagcaataaacgaaagtttaactaagctatactaaccccagggttggtcaatttcgtgccagccacaccctggtactgcatgcacgcaatgctagctgcccctttcccgtcctgggcaccccgagtctcccccgaccccgggtcccaggtatgctcccacctccacctgccccactcaccacctctgctagttccagacacctccgagacgaggaaaaaaaaaaaaaaaaaaaaaaaaaaaaaaaaaaaaaaaaaaaaaaaaaaaaaaaaaaaaaaaaaaaaaaaaaaaaaaaaaaaaaaaaaaaaaaaaaaaaaaaaaaaaaaaaaaaaaaaaaaaaaaaaaaaaaaaaaaaaaaaaaaaaaaaaaaaaaaaaaaaaaaaaaaaaaaaaaaaaaaaaaaaaaaaaaaaaaaaaaaaaaaaaaaaaaaaaaaaaaaaaaaaaaaaaaaaaaaaaaaaaaaaaaaaaaaaaaaaaaaaaaaaaaaaaaaaaaaaaaaaaaaaaaaaaaaaaaaaaaaaaaaaaaaaaaaaaaaaaaaaaaaaaaaaaaaaaaaaaaaaaaaaaaaaaaaaaaaaaaaaaaaaaaaaaaaaaaaaaaaaaaaaaaaaaaaccgtcttcaagctttctagaaattcactggccgtcgttttacaacgtcgtgactgggaaaaccctggcgttacccaacttaatcgccttgcagcacatccccctttcgccagctggcgtaatagcgaagaggcccgcaccgatcgcccttcccaacagttgcgcagcctgaatggcgaatggcgcctgatgcggtattttctccttacgcatctgtgcggtatttcacaccgcatatggtgcactctcagtacaatctgctctgatgccgcatagttaagccagccccgacacccgccaacacccgctgacgcgccctgacgggcttgtctgctcccggcatccgcttacagacaagctgtgaccgtctccgggagctgcatgtgtcagaggttttcaccgtcatcaccgaaacgcgcgagacgaaagggcctcgtgatacgcctatttttataggttaatgtcatgataataatggtttcttagacgtcaggtggcacttttcggggaaatgtgcgcggaacccctatttgtttatttttctaaatacattcaaatatgtatccgctcatgagacaataaccctgataaatgcttcaataatattgaaaaaggaagagtatgagtattcaacatttccgtgtcgcccttattcccttttttgcggcattttgccttcctgtttttgctcacccagaaacgctggtgaaagtaaaagatgctgaagatcagttgggtgcacgagtgggttacatcgaactggatctcaacagcggtaagatccttgagagttttcgccccgaagaacgttttccaatgatgagcacttttaaagttctgctatgtggcgcggtattatcccgtattgacgccgggcaagagcaactcggtcgccgcatacactattctcagaatgacttggttgagtactcaccagtcacagaaaagcatcttacggatggcatgacagtaagagaattatgcagtgctgccataaccatgagtgataacactgcggccaacttacttctgacaacgatcggaggaccgaaggagctaaccgcttttttgcacaacatgggggatcatgtaactcgccttgatcgttgggaaccggagctgaatgaagccataccaaacgacgagcgtgacaccacgatgcctgtagcaatggcaacaacgttgcgcaaactattaactggcgaactacttactctagcttcccggcaacaattaatagactggatggaggcggataaagttgcaggaccacttctgcgctcggcccttccggctggctggtttattgctgataaatctggagccggtgagcgtgggtctcgcggtatcattgcagcactggggccagatggtaagccctcccgtatcgtagttatctacacgacggggagtcaggcaactatggatgaacgaaatagacagatcgctgagataggtgcctcactgattaagcattggtaactgtcagaccaagtttactcatatatactttagattgatttaaaacttcatttttaatttaaaagg

SEQ ID NO: 227 - DNA, 10851 bp, synthetic construct
  misc_feature 1..10851: note = DNA of V33_KRAB-1xGCN4-2a-D3a-hD3l-dCas9-scFv
  source 1..10851: mol_type = other DNA
atctaggtgaagatcctttttgataatctcatgaccaaaatcccttaacgtgagttttcgttccactgagcgtcagaccccgtagaaaagatcaaaggatcttcttgagatcctttttttctgcgcgtaatctgctgcttgcaaacaaaaaaaccaccgctaccagcggtggtttgtttgccggatcaagagctaccaactctttttccgaaggtaactggcttcagcagagcgcagataccaaatactgttcttctagtgtagccgtagttaggccaccacttcaagaactctgtagcaccgcctacatacctcgctctgctaatcctgttaccagtggctgctgccagtggcgataagtcgtgtcttaccgggttggactcaagacgatagttaccggataaggcgcagcggtcgggctgaacggggggttcgtgcacacagcccagcttggagcgaacgacctacaccgaactgagatacctacagcgtgagctatgagaaagcgccacgcttcccgaagggagaaaggcggacaggtatccggtaagcggcagggtcggaacaggagagcgcacgagggagcttccagggggaaacgcctggtatctttatagtcctgtcgggtttcgccacctctgacttgagcgtcgatttttgtgatgctcgtcaggggggcggagcctatggaaaaacgccagcaacgcggcctttttacggttcctggccttttgctggccttttgctcacatgttctttcctgcgttatcccctgattctgtggataaccgtattaccgcctttgagtgagctgataccgctcgccgcagccgaacgaccgagcgcagcgagtcagtgagcgaggaagcggaagagcgcccaatacgcaaaccgcctctccccgcgcgttggccgattcattaatgcagctggcacgacaggtttcccgactggaaagcgggcagtgagcgcaacgcaattaatgtgagttagctcactcattaggcaccccaggctttacactttatgcttccggctcgtatgttgtgtggaattgtgagcggataacaatttcacacaggaaacagctatgaccatgattacgcctctagaaagctttaatacgactcactataaggactcactatttgttttcgcgcccagttgcaaaaagtgtcgacatttgcttctgacacaactgtgttcactagcaacctcaaacagacaccgccaccatgcctgctgctaagagagtgaaactggatggatcccggacactggtgaccttcaaggatgtatttgtggacttcaccagggaggagtggaagctgctggacactgctcagcagatcgtgtacagaaatgtgatgctggagaactataagaacctggtttccttgggttatcagcttactaagccagatgtgatcctccggttggagaagggagaagagcccggaagcggaatggaggaactgctgagcaagaactaccacctggaaaacgaggtggccagactgaagaaaggctctggctctggcggaagcggttctggcggatcaggatctggaagtggcggctctggaagcggaggttctggatctggcggaagcggagctactaacttcagcctgctgaagcaggctggagacgtggaggagaaccctggacctatgcctgctgctaagagagtgaaactggatggatccaaccatgaccaggaatttgaccccccaaaggtttacccacctgtgccagctgagaagaggaagcccatccgcgtgctgtctctctttgatgggattgctacagggctcctggtgctgaaggacctgggcatccaagtggaccgctacattgcctccgaggtgtgtgaggactccatcacggtgggcatggtgcggcaccagggaaagatcatgtacgtcggggacgtccgcagcgtcacacagaagcatatccaggagtggggcccattcgacctggtgattggaggcagtccctgcaatgacctctccattgtcaaccctgcccgcaagggactttatgagggtactggccgcctcttctttgagttctaccgcctcctgcatgatgcgcggcccaaggagggagatgatcgccccttcttctggctctttgagaatgtggtggccatgggcgttagtgacaagagggacatctcgcgatttcttgagtctaaccccgtgatgattgacgccaaagaagtgtctgctgcacacagggcccgttacttctggggtaaccttcctggcatgaacaggcctttggcatccactgtgaatgataagctggagctgcaagagtgtctggagcacggcagaatagccaagttcagcaaagtgaggaccattaccaccaggtcaaactctataaagcagggcaaagaccagcatttccccgtgttcatgaacgagaaggaggacatcctgtggtgcactgaaatggaaagggtgtttggcttccccgtccactacacagacgtctccaacatgagccgcttggcgaggcagagactgctgggccgatcgtggagcgtgccggtcatccgccacctcttcgctccgctgaaggaatattttgcttgtgtgtctagcggcaatagtaacgctaacagccgcgggccgagcttcagcagcggcctggtgccgttaagcttgcgcggcagccatatgttcgaaaccgtgcctgtgtggaggagacagccagtccgggtgctgtccctttttgaagacatcaagaaagagctgacgagtttgggctttttggaaagtggttctgacccgggacaactgaagcatgtggttgatgtcacagacacagtgaggaaggatgtggaggagtggggacccttcgatcttgtgtacggcgccacacctcccctgggccacacctgtgaccgtcctcccagctggtacctgttccagttccaccggctcctgcagtacgcacggcccaagccaggcagccccaggcccttcttctggatgttcgtggacaatctggtgctgaacaaggaagacctggacgtcgcatctcgcttcctggagatggagccagtcaccatcccagatgtccacggcggatccttgcagaatgctgtccgcgtgtggagcaacatcccagccataaggagcagcaggcactgggctctggtttcggaagaagaattgtccctgctggcccagaacaagcagagctcgaagctcgcggccaagtggcccaccaagctggtgaagaactgctttctccccctaagagaatatttcaagtatttttcaggagggccgagctctggcgcacccccaccaagtggagggtctcctgccgggtccccaacatctactgaagaaggcaccagcgaatccgcaacgcccgagtcaggccctggtacctccacagaaccatctgaaggtagtgcgcctggttccccagctggaagccctacttccaccgaagaaggcacgtcaaccgaaccaagtgaaggatctgcccctgggaccagcactgaaccatctgagccaaaaaagaagagaaaggtaatggacaagaagtacagcatcggcctggccatcggcaccaactctgtgggctgggccgtgatcaccgacgagtacaaggtgcccagcaagaaattcaaggtgctgggcaacaccgaccggcacagcatcaagaagaacctgatcggcgccctgctgttcgacagcggagaaacagccgaggccacccggctgaagagaaccgccagaagaagatacaccagacggaagaaccggatctgctatctgcaagagatcttcagcaacgagatggccaaggtggacgacagcttcttccacagactggaagagtccttcctggtggaagaggataagaagcacgagcggcaccccatcttcggcaacatcgtggacgaggtggcctaccacgagaagtaccccaccatctaccacctgagaaagaaactggtggacagcaccgacaaggccgacctgcggctgatctatctggccctggcccacatgatcaagttccggggccacttcctgatcgagggcgacctgaaccccgacaacagcgacgtggacaagctgttcatccagctggtgcagacctacaaccagctgttcgaggaaaaccccatcaacgccagcggcgtggacgccaaggccatcctgtctgccagactgagcaagagcagacggctggaaaatctgatcgcccagctgcccggcgagaagaagaatggcctgttcggcaacctgattgccctgagcctgggcctgacccccaacttcaagagcaacttcgacctggccgaggatgccaaactgcagctgagcaaggacacctacgacgacgacctggacaacctgctggcccagatcggcgaccagtacgccgacctgtttctggccgccaagaacctgtccgacgccatcctgctgagcgacatcctgagagtgaacaccgagatcaccaaggcccccctgagcgcctctatgatcaagagatacgacgagcaccaccaggacctgaccctgctgaaagctctcgtgcggcagcagctgcctgagaagtacaaagagattttcttcgaccagagcaagaacggctacgccggctacatcgatggcggagccagccaggaagagttctacaagttcatcaagcccatcctggaaaagatggacggcaccgaggaactgctcgtgaagctgaacagagaggacctgctgcggaagcagcggaccttcgacaacggcagcatcccccaccagatccacctgggagagctgcacgccattctgcggcggcaggaagatttttacccattcctgaaggacaaccgggaaaagatcgagaagatcctgaccttccgcatcccctactacgtgggccctctggccaggggaaacagcagattcgcctggatgaccagaaagagcgaggaaaccatcaccccctggaacttcgaggaagtggtggacaagggcgccagcgcccagagcttcatcgagcggatgaccaacttcgataagaacctgcccaacgagaaggtgctgcccaagcacagcctgctgtacgagtacttcaccgtgtacaacgagctgaccaaagtgaaatacgtgaccgagggaatgagaaagcccgccttcctgagcggcgagcagaaaaaagccatcgtggacctgctgttcaagaccaaccggaaagtgaccgtgaagcagctgaaagaggactacttcaagaaaatcgagtgcttcgactccgtggaaatctccggcgtggaagatcggttcaacgcctccctgggcacataccacgatctgctgaaaattatcaaggacaaggacttcctggacaatgaggaaaacgaggacattctggaagatatcgtgctgaccctgacactgtttgaggacagagagatgatcgaggaacggctgaaaacctatgcccacctgttcgacgacaaagtgatgaagcagctgaagcggcggagatacaccggctggggcaggctgagccggaagctgatcaacggcatccgggacaagcagtccggcaagacaatcctggatttcctgaagtccgacggcttcgccaacagaaacttcatgcagctgatccacgacgacagcctgacctttaaagaggacatccagaaagcccaggtgtccggccagggcgatagcctgcacgagcacattgccaatctggccggcagccccgccattaagaagggcatcctgcagacagtgaaggtggtggacgagctcgtgaaagtgatgggccggcacaagcccgagaacatcgtgatcgaaatggccagagagaaccagaccacccagaagggacagaagaacagccgcgagagaatgaagcggatcgaagagggcatcaaagagctgggcagccagatcctgaaagaacaccccgtggaaaacacccagctgcagaacgagaagctgtacctgtactacctgcagaatgggcgggatatgtacgtggaccaggaactggacatcaaccggctgtccgactacgatgtggacgctatcgtgcctcagagctttctgaaggacgactccatcgataacaaagtgctgactcggagcgacaagaaccggggcaagagcgacaacgtgccctccgaagaggtcgtgaagaagatgaagaactactggcgccagctgctgaatgccaagctgattacccagaggaagttcgacaatctgaccaaggccgagagaggcggcctgagcgaactggataaggccggcttcatcaagagacagctggtggaaacccggcagatcacaaagcacgtggcacagatcctggactcccggatgaacactaagtacgacgagaacgacaaactgatccgggaagtgaaagtgatcaccctgaagtccaagctggtgtccgatttccggaaggatttccagttttacaaagtgcgcgagatcaacaactaccaccacgcccacgacgcctacctgaacgccgtcgtgggaaccgccctgatcaaaaagtaccctaagctggaaagcgagttcgtgtacggcgactacaaggtgtacgacgtgcggaagatgatcgccaagagcgagcaggaaatcggcaaggctaccgccaagtacttcttctacagcaacatcatgaactttttcaagaccgagattaccctggccaacggcgagatccggaagcggcctctgatcgagacaaacggcgaaacaggcgagatcgtgtgggataagggccgggactttgccaccgtgcggaaagtgctgtctatgccccaagtgaatatcgtgaaaaagaccgaggtgcagacaggcggcttcagcaaagagtctatcctgcccaagaggaacagcgacaagctgatcgccagaaagaaggactgggaccctaagaagtacggcggcttcgacagccccaccgtggcctattctgtgctggtggtggccaaagtggaaaagggcaagtccaagaaactgaagagtgtgaaagagctgctggggatcaccatcatggaaagaagcagcttcgagaagaatcccatcgactttctggaagccaagggctacaaagaagtgaaaaaggacctgatcatcaagctgcctaagtactccctgttcgagctggaaaacggccggaagagaatgctggcctctgccggcgaactgcagaagggaaacgaactggccctgccctccaaatatgtgaacttcctgtacctggccagccactatgagaagctgaagggctcccccgaggataatgagcagaaacagctgtttgtggaacagcacaaacactacctggacgagatcatcgagcagatcagcgagttctccaagagagtgatcctggccgacgctaatctggacaaggtgctgagcgcctacaacaagcacagagacaagcctatcagagagcaggccgagaatatcatccacctgtttaccctgaccaatctgggagcccctgccgccttcaagtactttgacaccaccatcgaccggaagaggtacaccagcaccaaagaggtgctggacgccaccctgatccaccagagcatcaccggcctgtacgagacacggatcgacctgtctcagctgggaggcgacgcctatccctatgacgtgcccgattatgccagcctgggcagcggctcccccaagaaaaaacgcaaggtggaagatcctaagaaaaagcggaaagtggacggcattggtagtgggagcggccccgacatcgtgatgacccagagccccagcagcctgagcgccagcgtgggcgaccgcgtgaccatcacctgccgcagcagcaccggcgccgtgaccaccagcaactacgccagctgggtgcaggagaagcccggcaagctgttcaagggcctgatcggcggcaccaacaaccgcgcccccggcgtgcccagccgcttcagcggcagcctgatcggcgacaaggccaccctgaccatcagcagcctgcagcccgaggacttcgccacctacttctgcgccctgtggtacagcaaccactgggtgttcggccagggcaccaaggtggagctgaagcgcggcggcggcggcagcggcggcggcggcagcggcggcggcggcagcagcggcggcggcagcgaggtgaagctgctggagagcggcggcggcctggtgcagcccggcggcagcctgaagctgagctgcgccgtgagcggcttcagcctgaccgactacggcgtgaactgggtgcgccaggcccccggccgcggcctggagtggatcggcgtgatctggggcgacggcatcaccgactacaacagcgccctgaaggaccgcttcatcatcagcaaggacaacggcaagaacaccgtgtacctgcagatgagcaaggtgcgcagcgacgacaccgccctgtactactgcgtgaccggcctgttcgactactggggccagggcaccctggtgaccgtgagcagctacccatacgatgttccagattacgctggtggaggcggaggttctgggggaggaggtagtggcggtggtggttcaggaggcggcggaagctagtgagatcccaagcacgcagcaatgcagctcaaaacgcttagcctagccacacccccacgggaaacagcagtgattaacctttagcaataaacgaaagtttaactaagctatactaaccccagggttggtcaatttcgtgccagccacaccctggtactgcatgcacgcaatgctagctgcccctttcccgtcctgggcaccccgagtctcccccgaccccgggtcccaggtatgctcccacctccacctgccccactcaccacctctgctagttccagacacctccgagacgaggaaaaaaaaaaaaaaaaaaaaaaaaaaaaaaaaaaaaaaaaaaaaaaaaaaaaaaaaaaaaaaaaaaaaaaaaaaaaaaaaaaaaaaaaaaaaaaaaaaaaaaaaaaaaaaaaaaaaaaaaaaaaaaaaaaaaaaaaaaaaaaaaaaaaaaaaaaaaaaaaaaaaaaaaaaaaaaaaaaaaaaaaaaaaaaaaaaaaaaaaaaaaaaaaaaaaaaaaaaaaaaaaaaaaaaaaaaaaaaaaaaaaaaaaaaaaaaaaaaaaaaaaaaaaaaaaaaaaaaaaaaaaaaaaaaaaaaaaaaaaaaaaaaaaaaaaaaaaaaaaaaaaaaaaaaaaaaaaaaaaaaaaaaaaaaaaaaaaaaaaaaaaaaaaaaaaaaaaaaaaaaaaaaaaaaaaaaccgtcttcaagctttctagaaattcactggccgtcgttttacaacgtcgtgactgggaaaaccctggcgttacccaacttaatcgccttgcagcacatccccctttcgccagctggcgtaatagcgaagaggcccgcaccgatcgcccttcccaacagttgcgcagcctgaatggcgaatggcgcctgatgcggtattttctccttacgcatctgtgcggtatttcacaccgcatatggtgcactctcagtacaatctgctctgatgccgcatagttaagccagccccgacacccgccaacacccgctgacgcgccctgacgggcttgtctgctcccggcatccgcttacagacaagctgtgaccgtctccgggagctgcatgtgtcagaggttttcaccgtcatcaccgaaacgcgcgagacgaaagggcctcgtgatacgcctatttttataggttaatgtcatgataataatggtttcttagacgtcaggtggcacttttcggggaaatgtgcgcggaacccctatttgtttatttttctaaatacattcaaatatgtatccgctcatgagacaataaccctgataaatgcttcaataatattgaaaaaggaagagtatgagtattcaacatttccgtgtcgcccttattcccttttttgcggcattttgccttcctgtttttgctcacccagaaacgctggtgaaagtaaaagatgctgaagatcagttgggtgcacgagtgggttacatcgaactggatctcaacagcggtaagatccttgagagttttcgccccgaagaacgttttccaatgatgagcacttttaaagttctgctatgtggcgcggtattatcccgtattgacgccgggcaagagcaactcggtcgccgcatacactattctcagaatgacttggttgagtactcaccagtcacagaaaagcatcttacggatggcatgacagtaagagaattatgcagtgctgccataaccatgagtgataacactgcggccaacttacttctgacaacgatcggaggaccgaaggagctaaccgcttttttgcacaacatgggggatcatgtaactcgccttgatcgttgggaaccggagctgaatgaagccataccaaacgacgagcgtgacaccacgatgcctgtagcaatggcaacaacgttgcgcaaactattaactggcgaactacttactctagcttcccggcaacaattaatagactggatggaggcggataaagttgcaggaccacttctgcgctcggcccttccggctggctggtttattgctgataaatctggagccggtgagcgtgggtctcgcggtatcattgcagcactggggccagatggtaagccctcccgtatcgtagttatctacacgacggggagtcaggcaactatggatgaacgaaatagacagatcgctgagataggtgcctcactgattaagcattggtaactgtcagaccaagtttactcatatatactttagattgatttaaaacttcatttttaatttaaaagg

SEQ ID NO: 228 - DNA, 10869 bp, synthetic construct
  misc_feature 1..10869: note = DNA of V34_D3a-D3l-1xGCN4-2a-scFv-dCas9-KRAB
  source 1..10869: mol_type = other DNA
atcgtgctgaccctgacactgtttgaggacagagagatgatcgaggaacggctgaaaacctatgcccacctgttcgacgacaaagtgatgaagcagctgaagcggcggagatacaccggctggggcaggctgagccggaagctgatcaacggcatccgggacaagcagtccggcaagacaatcctggatttcctgaagtccgacggcttcgccaacagaaacttcatgcagctgatccacgacgacagcctgacctttaaagaggacatccagaaagcccaggtgtccggccagggcgatagcctgcacgagcacattgccaatctggccggcagccccgccattaagaagggcatcctgcagacagtgaaggtggtggacgagctcgtgaaagtgatgggccggcacaagcccgagaacatcgtgatcgaaatggccagagagaaccagaccacccagaagggacagaagaacagccgcgagagaatgaagcggatcgaagagggcatcaaagagctgggcagccagatcctgaaagaacaccccgtggaaaacacccagctgcagaacgagaagctgtacctgtactacctgcagaatgggcgggatatgtacgtggaccaggaactggacatcaaccggctgtccgactacgatgtggacgctatcgtgcctcagagctttctgaaggacgactccatcgataacaaagtgctgactcggagcgacaagaaccggggcaagagcgacaacgtgccctccgaagaggtcgtgaagaagatgaagaactactggcgccagctgctgaatgccaagctgattacccagaggaagttcgacaatctgaccaaggccgagagaggcggcctgagcgaactggataaggccggcttcatcaagagacagctggtggaaacccggcagatcacaaagcacgtggcacagatcctggactcccggatgaacactaagtacgacgagaacgacaaactgatccgggaagtgaaagtgatcaccctgaagtccaagctggtgtccgatttccggaaggatttccagttttacaaagtgcgcgagatcaacaactaccaccacgcccacgacgcctacctgaacgccgtcgtgggaaccgccctgatcaaaaagtaccctaagctggaaagcgagttcgtgtacggcgactacaaggtgtacgacgtgcggaagatgatcgccaagagcgagcaggaaatcggcaaggctaccgccaagtacttcttctacagcaacatcatgaactttttcaagaccgagattaccctggccaacggcgagatccggaagcggcctctgatcgagacaaacggcgaaacaggcgagatcgtgtgggataagggccgggactttgccaccgtgcggaaagtgctgtctatgccccaagtgaatatcgtgaaaaagaccgaggtgcagacaggcggcttcagcaaagagtctatcctgcccaagaggaacagcgacaagctgatcgccagaaagaaggactgggaccctaagaagtacggcggcttcgacagccccaccgtggcctattctgtgctggtggtggccaaagtggaaaagggcaagtccaagaaactgaagagtgtgaaagagctgctggggatcaccatcatggaaagaagcagcttcgagaagaatcccatcgactttctggaagccaagggctacaaagaagtgaaaaaggacctgatcatcaagctgcctaagtactccctgttcgagctggaaaacggccggaagagaatgctggcctctgccggcgaactgcagaagggaaacgaactggccctgccctccaaatatgtgaacttcctgtacctggccagccactatgagaagctgaagggctcccccgaggataatgagcagaaacagctgtttgtggaacagcacaaacactacctggacgagatcatcgagcagatcagcgagttctccaagagagtgatcctggccgacgctaatctggacaaggtgctgagcgcctacaacaagcacagagacaagcctatcagagagcaggccgagaatatcatccacctgtttaccctgaccaatctgggagcccctgccgccttcaagtactttgacaccaccatcgaccggaagaggtacaccagcaccaaagaggtgctggacgccaccctgatccaccagagcatcaccggcctgtacgagacacggatcgacctgtctcagctgggaggcgacgcctatccctatgacgtgcccgattatgccagcctgggcagcggctcccccaagaaaaaacgcaaggtggaagatcctaagaaaaagcggaaagtggacggcagcggcagcgagacccccggtaccagcgagagcgccacccccgagagccggacactggtgaccttcaaggatgtatttgtggacttcaccagggaggagtggaagctgctggacactgctcagcagatcgtgtacagaaatgtgatgctggagaactataagaacctggtttccttgggttatcagcttactaagccagatgtgatcctccggttggagaagggagaagagccctgagatcccaagcacgcagcaatgcagctcaaaacgcttagcctagccacacccccacgggaaacagcagtgattaacctttagcaataaacgaaagtttaactaagctatactaaccccagggttggtcaatttcgtgccagccacaccctggtactgcatgcacgcaatgctagctgcccctttcccgtcctgggcaccccgagtctcccccgaccccgggtcccaggtatgctcccacctccacctgccccactcaccacctctgctagttccagacacctccgagacgaggaaaaaaaaaaaaaaaaaaaaaaaaaaaaaaaaaaaaaaaaaaaaaaaaaaaaaaaaaaaaaaaaaaaaaaaaaaaaaaaaaaaaaaaaaaaaaaaaaaaaaaaaaaaaaaaaaaaaaaaaaaaaaaaaaaaaaaaaaaaaaaaaaaaaaaaaaaaaaaaaaaaaaaaaaaaaaaaaaaaaaaaaaaaaaaaaaaaaaaaaaaaaaaaaaaaaaaaaaaaaaaaaaaaaaaaaaaaaaaaaaaaaaaaaaaaaaaaaaaaaaaaaaaaaaaaaaaaaaaaaaaaaaaaaaaaaaaaaaaaaaaaaaaaaaaaaaaaaaaaaaaaaaaaaaaaaaaaaaaaaaaaaaaaaaaaaaaaaaaaaaaaaaaaaaaaaaaaaaaaaaaaaaaaaaaaaaaccgtcttcaagctttctagaaattcactggccgtcgttttacaacgtcgtgactgggaaaaccctggcgttacccaacttaatcgccttgcagcacatccccctttcgccagctggcgtaatagcgaagaggcccgcaccgatcgcccttcccaacagttgcgcagcctgaatggcgaatggcgcctgatgcggtattttctccttacgcatctgtgcggtatttcacaccgcatatggtgcactctcagtacaatctgctctgatgccgcatagttaagccagccccgacacccgccaacacccgctgacgcgccctgacgggcttgtctgctcccggcatccgcttacagacaagctgtgaccgtctccgggagctgcatgtgtcagaggttttcaccgtcatcaccgaaacgcgcgagacgaaagggcctcgtgatacgcctatttttataggttaatgtcatgataataatggtttcttagacgtcaggtggcacttttcggggaaatgtgcgcggaacccctatttgtttatttttctaaatacattcaaatatgtatccgctcatgagacaataaccctgataaatgcttcaataatattgaaaaaggaagagtatgagtattcaacatttccgtgtcgcccttattcccttttttgcggcattttgccttcctgtttttgctcacccagaaacgctggtgaaagtaaaagatgctgaagatcagttgggtgcacgagtgggttacatcgaactggatctcaacagcggtaagatccttgagagttttcgccccgaagaacgttttccaatgatgagcacttttaaagttctgctatgtggcgcggtattatcccgtattgacgccgggcaagagcaactcggtcgccgcatacactattctcagaatgacttggttgagtactcaccagtcacagaaaagcatcttacggatggcatgacagtaagagaattatgcagtgctgccataaccatgagtgataacactgcggccaacttacttctgacaacgatcggaggaccgaaggagctaaccgcttttttgcacaacatgggggatcatgtaactcgccttgatcgttgggaaccggagctgaatgaagccataccaaacgacgagcgtgacaccacgatgcctgtagcaatggcaacaacgttgcgcaaactattaactggcgaactacttactctagcttcccggcaacaattaatagactggatggaggcggataaagttgcaggaccacttctgcgctcggcccttccggctggctggtttattgctgataaatctggagccggtgagcgtgggtctcgcggtatcattgcagcactggggccagatggtaagccctcccgtatcgtagttatctacacgacggggagtcaggcaactatggatgaacgaaatagacagatcgctgagataggtgcctcactgattaagcattggtaactgtcagaccaagtttactcatatatactttagattgatttaaaacttcatttttaatttaaaaggatctaggtgaagatcctttttgataatctcatgaccaaaatcccttaacgtgagttttcgttccactgagcgtcagaccccgtagaaaagatcaaaggatcttcttgagatcctttttttctgcgcgtaatctgctgcttgcaaacaaaaaaaccaccgctaccagcggtggtttgtttgccggatcaagagctaccaactctttttccgaaggtaactggcttcagcagagcgcagataccaaatactgttcttctagtgtagccgtagttaggccaccacttcaagaactctgtagcaccgcctacatacctcgctctgctaatcctgttaccagtggctgctgccagtggcgataagtcgtgtcttaccgggttggactcaagacgatagttaccggataaggcgcagcggtcgggctgaacggggggttcgtgcacacagcccagcttggagcgaacgacctacaccgaactgagatacctacagcgtgagctatgagaaagcgccacgcttcccgaagggagaaaggcggacaggtatccggtaagcggcagggtcggaacaggagagcgcacgagggagcttccagggggaaacgcctggtatctttatagtcctgtcgggtttcgccacctctgacttgagcgtcgatttttgtgatgctcgtcaggggggcggagcctatggaaaaacgccagcaacgcggcctttttacggttcctggccttttgctggccttttgctcacatgttctttcctgcgttatcccctgattctgtggataaccgtattaccgcctttgagtgagctgataccgctcgccgcagccgaacgaccgagcgcagcgagtcagtgagcgaggaagcggaagagcgcccaatacgcaaaccgcctctccccgcgcgttggccgattcattaatgcagctggcacgacaggtttcccgactggaaagcgggcagtgagcgcaacgcaattaatgtgagttagctcactcattaggcaccccaggctttacactttatgcttccggctcgtatgttgtgtggaattgtgagcggataacaatttcacacaggaaacagctatgaccatgattacgcctctagaaagctttaatacgactcactataaggactcactatttgttttcgcgcccagttgcaaaaagtgtcgacatttgcttctgacacaactgtgttcactagcaacctcaaacagacaccgccaccatgcctgctgctaagagagtgaaactggatggatccaaccatgaccaggaatttgaccccccaaaggtttacccacctgtgccagctgagaagaggaagcccatccgcgtgctgtctctctttgatgggattgctacagggctcctggtgctgaaggacctgggcatccaagtggaccgctacattgcctccgaggtgtgtgaggactccatcacggtgggcatggtgcggcaccagggaaagatcatgtacgtcggggacgtccgcagcgtcacacagaagcatatccaggagtggggcccattcgacctggtgattggaggcagtccctgcaatgacctctccattgtcaaccctgcccgcaagggactttatgagggtactggccgcctcttctttgagttctaccgcctcctgcatgatgcgcggcccaaggagggagatgatcgccccttcttctggctctttgagaatgtggtggccatgggcgttagtgacaagagggacatctcgcgatttcttgagtctaaccccgtgatgattgacgccaaagaagtgtctgctgcacacagggcccgttacttctggggtaaccttcctggcatgaacaggcctttggcatccactgtgaatgataagctggagctgcaagagtgtctggagcacggcagaatagccaagttcagcaaagtgaggaccattaccaccaggtcaaactctataaagcagggcaaagaccagcatttccccgtgttcatgaacgagaaggaggacatcctgtggtgcactgaaatggaaagggtgtttggcttccccgtccactacacagacgtctccaacatgagccgcttggcgaggcagagactgctgggccgatcgtggagcgtgccggtcatccgccacctcttcgctccgctgaaggaatattttgcttgtgtgtctagcggcaatagtaacgctaacagccgcgggccgagcttcagcagcggcctggtgccgttaagcttgcgcggcagccatatgggccctatggagatatacaagacagtgtctgcatggaagagacagccagtgcgggtactgagcctcttcagaaacatcgacaaggtactaaagagtttgggcttcttggaaagcggttctggttctgggggaggaacgctgaagtacgtggaagatgtcacaaatgtcgtgaggagagacgtggagaaatggggcccctttgacctggtgtacggctcgacgcagcccctaggcagctcttgtgatcgctgtcccggctggtacatgttccagttccaccggatcctgcagtatgcgctgcctcgccaggagagtcagcggcccttcttctggatattcatggacaatctgctgctgactgaggatgaccaagagacaactacccgcttccttcagacagaggctgtgaccctccaggatgtccgtggcagagactaccagaatgctatgcgggtgtggagcaacattccagggctgaagagcaagcatgcgcccctgaccccaaaggaagaagagtatctgcaagcccaagtcagaagcaggagcaagctggacgccccgaaagttgacctcctggtgaagaactgccttctcccgctgagagagtacttcaagtatttttctcaaaactcacttcctcttggagggccgagctctggcgcacccccaccaagtggagggtctcctgccgggtccccaacatctactgaagaaggcaccagcgaatccgcaacgggcagtggcagcggaggaagtggatccggcggtagtggtagtggaagcggcggatccggctcaggcggatctggttcaggggaagaactcctctccaaaaactaccatctcgagaatgaggtcgcccgcctgaaaaaaggatcaggttccggtggttctggcagcggtggttcaggctcaggcagcggcggtagcggtagcggtggaagcggaagcggaccaaaaaagaagagaaaggtaggaagcggagctactaacttcagcctgctgaagcaggctggagacgtggaggagaaccctggacctatgcctgctgctaagagagtgaaactggatggatccggccccgacatcgtgatgacccagagccccagcagcctgagcgccagcgtgggcgaccgcgtgaccatcacctgccgcagcagcaccggcgccgtgaccaccagcaactacgccagctgggtgcaggagaagcccggcaagctgttcaagggcctgatcggcggcaccaacaaccgcgcccccggcgtgcccagccgcttcagcggcagcctgatcggcgacaaggccaccctgaccatcagcagcctgcagcccgaggacttcgccacctacttctgcgccctgtggtacagcaaccactgggtgttcggccagggcaccaaggtggagctgaagcgcggcggcggcggcagcggcggcggcggcagcggcggcggcggcagcagcggcggcggcagcgaggtgaagctgctggagagcggcggcggcctggtgcagcccggcggcagcctgaagctgagctgcgccgtgagcggcttcagcctgaccgactacggcgtgaactgggtgcgccaggcccccggccgcggcctggagtggatcggcgtgatctggggcgacggcatcaccgactacaacagcgccctgaaggaccgcttcatcatcagcaaggacaacggcaagaacaccgtgtacctgcagatgagcaaggtgcgcagcgacgacaccgccctgtactactgcgtgaccggcctgttcgactactggggccagggcaccctggtgaccgtgagcagctacccatacgatgttccagattacgctggtggaggcggaggttctgggggaggaggtagtggcggtggtggttcaggaggcggcggaagcggaagcggaccaaaaaagaagagaaaggtaatggacaagaagtacagcatcggcctggccatcggcaccaactctgtgggctgggccgtgatcaccgacgagtacaaggtgcccagcaagaaattcaaggtgctgggcaacaccgaccggcacagcatcaagaagaacctgatcggcgccctgctgttcgacagcggagaaacagccgaggccacccggctgaagagaaccgccagaagaagatacaccagacggaagaaccggatctgctatctgcaagagatcttcagcaacgagatggccaaggtggacgacagcttcttccacagactggaagagtccttcctggtggaagaggataagaagcacgagcggcaccccatcttcggcaacatcgtggacgaggtggcctaccacgagaagtaccccaccatctaccacctgagaaagaaactggtggacagcaccgacaaggccgacctgcggctgatctatctggccctggcccacatgatcaagttccggggccacttcctgatcgagggcgacctgaaccccgacaacagcgacgtggacaagctgttcatccagctggtgcagacctacaaccagctgttcgaggaaaaccccatcaacgccagcggcgtggacgccaaggccatcctgtctgccagactgagcaagagcagacggctggaaaatctgatcgcccagctgcccggcgagaagaagaatggcctgttcggcaacctgattgccctgagcctgggcctgacccccaacttcaagagcaacttcgacctggccgaggatgccaaactgcagctgagcaaggacacctacgacgacgacctggacaacctgctggcccagatcggcgaccagtacgccgacctgtttctggccgccaagaacctgtccgacgccatcctgctgagcgacatcctgagagtgaacaccgagatcaccaaggcccccctgagcgcctctatgatcaagagatacgacgagcaccaccaggacctgaccctgctgaaagctctcgtgcggcagcagctgcctgagaagtacaaagagattttcttcgaccagagcaagaacggctacgccggctacatcgatggcggagccagccaggaagagttctacaagttcatcaagcccatcctggaaaagatggacggcaccgaggaactgctcgtgaagctgaacagagaggacctgctgcggaagcagcggaccttcgacaacggcagcatcccccaccagatccacctgggagagctgcacgccattctgcggcggcaggaagatttttacccattcctgaaggacaaccgggaaaagatcgagaagatcctgaccttccgcatcccctactacgtgggccctctggccaggggaaacagcagattcgcctggatgaccagaaagagcgaggaaaccatcaccccctggaacttcgaggaagtggtggacaagggcgccagcgcccagagcttcatcgagcggatgaccaacttcgataagaacctgcccaacgagaaggtgctgcccaagcacagcctgctgtacgagtacttcaccgtgtacaacgagctgaccaaagtgaaatacgtgaccgagggaatgagaaagcccgccttcctgagcggcgagcagaaaaaagccatcgtggacctgctgttcaagaccaaccggaaagtgaccgtgaagcagctgaaagaggactacttcaagaaaatcgagtgcttcgactccgtggaaatctccggcgtggaagatcggttcaacgcctccctgggcacataccacgatctgctgaaaattatcaaggacaaggacttcctggacaatgaggaaaacgaggacattctggaagat

SEQ ID NO: 229 - DNA, 10840 bp, synthetic construct
  misc_feature 1..10840: note = DNA of V35_scFv-dCas9-KRAB-2a-1xGCN4-D3l-D3a
  source 1..10840: mol_type = other DNA
gagatacctacagcgtgagctatgagaaagcgccacgcttcccgaagggagaaaggcggacaggtatccggtaagcggcagggtcggaacaggagagcgcacgagggagcttccagggggaaacgcctggtatctttatagtcctgtcgggtttcgccacctctgacttgagcgtcgatttttgtgatgctcgtcaggggggcggagcctatggaaaaacgccagcaacgcggcctttttacggttcctggccttttgctggccttttgctcacatgttctttcctgcgttatcccctgattctgtggataaccgtattaccgcctttgagtgagctgataccgctcgccgcagccgaacgaccgagcgcagcgagtcagtgagcgaggaagcggaagagcgcccaatacgcaaaccgcctctccccgcgcgttggccgattcattaatgcagctggcacgacaggtttcccgactggaaagcgggcagtgagcgcaacgcaattaatgtgagttagctcactcattaggcaccccaggctttacactttatgcttccggctcgtatgttgtgtggaattgtgagcggataacaatttcacacaggaaacagctatgaccatgattacgcctctagaaagctttaatacgactcactataaggactcactatttgttttcgcgcccagttgcaaaaagtgtcgacatttgcttctgacacaactgtgttcactagcaacctcaaacagacaccgccaccatgcctgctgctaagagagtgaaactggatggatccggccccgacatcgtgatgacccagagccccagcagcctgagcgccagcgtgggcgaccgcgtgaccatcacctgccgcagcagcaccggcgccgtgaccaccagcaactacgccagctgggtgcaggagaagcccggcaagctgttcaagggcctgatcggcggcaccaacaaccgcgcccccggcgtgcccagccgcttcagcggcagcctgatcggcgacaaggccaccctgaccatcagcagcctgcagcccgaggacttcgccacctacttctgcgccctgtggtacagcaaccactgggtgttcggccagggcaccaaggtggagctgaagcgcggcggcggcggcagcggcggcggcggcagcggcggcggcggcagcagcggcggcggcagcgaggtgaagctgctggagagcggcggcggcctggtgcagcccggcggcagcctgaagctgagctgcgccgtgagcggcttcagcctgaccgactacggcgtgaactgggtgcgccaggcccccggccgcggcctggagtggatcggcgtgatctggggcgacggcatcaccgactacaacagcgccctgaaggaccgcttcatcatcagcaaggacaacggcaagaacaccgtgtacctgcagatgagcaaggtgcgcagcgacgacaccgccctgtactactgcgtgaccggcctgttcgactactggggccagggcaccctggtgaccgtgagcagctacccatacgatgttccagattacgctggtggaggcggaggttctgggggaggaggtagtggcggtggtggttcaggaggcggcggaagcggaagcggaccaaaaaagaagagaaaggtaatggacaagaagtacagcatcggcctggccatcggcaccaactctgtgggctgggccgtgatcaccgacgagtacaaggtgcccagcaagaaattcaaggtgctgggcaacaccgaccggcacagcatcaagaagaacctgatcggcgccctgctgttcgacagcggagaaacagccgaggccacccggctgaagagaaccgccagaagaagatacaccagacggaagaaccggatctgctatctgcaagagatcttcagcaacgagatggccaaggtggacgacagcttcttccacagactggaagagtccttcctggtggaagaggataagaagcacgagcggcaccccatcttcggcaacatcgtggacgaggtggcctaccacgagaagtaccccaccatctaccacctgagaaagaaactggtggacagcaccgacaaggccgacctgcggctgatctatctggccctggcccacatgatcaagttccggggccacttcctgatcgagggcgacctgaaccccgacaacagcgacgtggacaagctgttcatccagctggtgcagacctacaaccagctgttcgaggaaaaccccatcaacgccagcggcgtggacgccaaggccatcctgtctgccagactgagcaagagcagacggctggaaaatctgatcgcccagctgcccggcgagaagaagaatggcctgttcggcaacctgattgccctgagcctgggcctgacccccaacttcaagagcaacttcgacctggccgaggatgccaaactgcagctgagcaaggacacctacgacgacgacctggacaacctgctggcccagatcggcgaccagtacgccgacctgtttctggccgccaagaacctgtccgacgccatcctgctgagcgacatcctgagagtgaacaccgagatcaccaaggcccccctgagcgcctctatgatcaagagatacgacgagcaccaccaggacctgaccctgctgaaagctctcgtgcggcagcagctgcctgagaagtacaaagagattttcttcgaccagagcaagaacggctacgccggctacatcgatggcggagccagccaggaagagttctacaagttcatcaagcccatcctggaaaagatggacggcaccgaggaactgctcgtgaagctgaacagagaggacctgctgcggaagcagcggaccttcgacaacggcagcatcccccaccagatccacctgggagagctgcacgccattctgcggcggcaggaagatttttacccattcctgaaggacaaccgggaaaagatcgagaagatcctgaccttccgcatcccctactacgtgggccctctggccaggggaaacagcagattcgcctggatgaccagaaagagcgaggaaaccatcaccccctggaacttcgaggaagtggtggacaagggcgccagcgcccagagcttcatcgagcggatgaccaacttcgataagaacctgcccaacgagaaggtgctgcccaagcacagcctgctgtacgagtacttcaccgtgtacaacgagctgaccaaagtgaaatacgtgaccgagggaatgagaaagcccgccttcctgagcggcgagcagaaaaaagccatcgtggacctgctgttcaagaccaaccggaaagtgaccgtgaagcagctgaaagaggactacttcaagaaaatcgagtgcttcgactccgtggaaatctccggcgtggaagatcggttcaacgcctccctgggcacataccacgatctgctgaaaattatcaaggacaaggacttcctggacaatgaggaaaacgaggacattctggaagatatcgtgctgaccctgacactgtttgaggacagagagatgatcgaggaacggctgaaaacctatgcccacctgttcgacgacaaagtgatgaagcagctgaagcggcggagatacaccggctggggcaggctgagccggaagctgatcaacggcatccgggacaagcagtccggcaagacaatcctggatttcctgaagtccgacggcttcgccaacagaaacttcatgcagctgatccacgacgacagcctgacctttaaagaggacatccagaaagcccaggtgtccggccagggcgatagcctgcacgagcacattgccaatctggccggcagccccgccattaagaagggcatcctgcagacagtgaaggtggtggacgagctcgtgaaagtgatgggccggcacaagcccgagaacatcgtgatcgaaatggccagagagaaccagaccacccagaagggacagaagaacagccgcgagagaatgaagcggatcgaagagggcatcaaagagctgggcagccagatcctgaaagaacaccccgtggaaaacacccagctgcagaacgagaagctgtacctgtactacctgcagaatgggcgggatatgtacgtggaccaggaactggacatcaaccggctgtccgactacgatgtggacgctatcgtgcctcagagctttctgaaggacgactccatcgataacaaagtgctgactcggagcgacaagaaccggggcaagagcgacaacgtgccctccgaagaggtcgtgaagaagatgaagaactactggcgccagctgctgaatgccaagctgattacccagaggaagttcgacaatctgaccaaggccgagagaggcggcctgagcgaactggataaggccggcttcatcaagagacagctggtggaaacccggcagatcacaaagcacgtggcacagatcctggactcccggatgaacactaagtacgacgagaacgacaaactgatccgggaagtgaaagtgatcaccctgaagtccaagctggtgtccgatttccggaaggatttccagttttacaaagtgcgcgagatcaacaactaccaccacgcccacgacgcctacctgaacgccgtcgtgggaaccgccctgatcaaaaagtaccctaagctggaaagcgagttcgtgtacggcgactacaaggtgtacgacgtgcggaagatgatcgccaagagcgagcaggaaatcggcaaggctaccgccaagtacttcttctacagcaacatcatgaactttttcaagaccgagattaccctggccaacggcgagatccggaagcggcctctgatcgagacaaacggcgaaacaggcgagatcgtgtgggataagggccgggactttgccaccgtgcggaaagtgctgtctatgccccaagtgaatatcgtgaaaaagaccgaggtgcagacaggcggcttcagcaaagagtctatcctgcccaagaggaacagcgacaagctgatcgccagaaagaaggactgggaccctaagaagtacggcggcttcgacagccccaccgtggcctattctgtgctggtggtggccaaagtggaaaagggcaagtccaagaaactgaagagtgtgaaagagctgctggggatcaccatcatggaaagaagcagcttcgagaagaatcccatcgactttctggaagccaagggctacaaagaagtgaaaaaggacctgatcatcaagctgcctaagtactccctgttcgagctggaaaacggccggaagagaatgctggcctctgccggcgaactgcagaagggaaacgaactggccctgccctccaaatatgtgaacttcctgtacctggccagccactatgagaagctgaagggctcccccgaggataatgagcagaaacagctgtttgtggaacagcacaaacactacctggacgagatcatcgagcagatcagcgagttctccaagagagtgatcctggccgacgctaatctggacaaggtgctgagcgcctacaacaagcacagagacaagcctatcagagagcaggccgagaatatcatccacctgtttaccctgaccaatctgggagcccctgccgccttcaagtactttgacaccaccatcgaccggaagaggtacaccagcaccaaagaggtgctggacgccaccctgatccaccagagcatcaccggcctgtacgagacacggatcgacctgtctcagctgggaggcgacgcctatccctatgacgtgcccgattatgccagcctgggcagcggctcccccaagaaaaaacgcaaggtggaagatcctaagaaaaagcggaaagtggacggcagcggcagcgagacccccggtaccagcgagagcgccacccccgagagccggacactggtgaccttcaaggatgtatttgtggacttcaccagggaggagtggaagctgctggacactgctcagcagatcgtgtacagaaatgtgatgctggagaactataagaacctggtttccttgggttatcagcttactaagccagatgtgatcctccggttggagaagggagaagagcccggaagcggagctactaacttcagcctgctgaagcaggctggagacgtggaggagaaccctggacctatgcctgctgctaagagagtgaaactggatggatccggctcaggcggatctggttcaggggaagaactcctctccaaaaactaccatctcgagaatgaggtcgcccgcctgaaaaaaggatcaggttccggtggttctggcagcggtggttcaggctcaggcagcggcggtagcggtagcggtggaagcggaagcggaacccccggtaccagcgagggcggccctagcagcggcgcccctccccctagcggcggcagccctgccggatcccctacaagcaccgaagaaggcacaagcgagtccgctacccctgagtccggccctggcacctccacagagcctagcgagggatccgctcctggatcccctgccggaagccctacctccaccgaggagggcacaagcaccgagccttccgagggcagcgcccccggaacaagcaccgaacctagcgagagcgccacccccgagagcatgttcgaaaccgtgcctgtgtggaggagacagccagtccgggtgctgtccctttttgaagacatcaagaaagagctgacgagtttgggctttttggaaagtggttctgacccgggacaactgaagcatgtggttgatgtcacagacacagtgaggaaggatgtggaggagtggggacccttcgatcttgtgtacggcgccacacctcccctgggccacacctgtgaccgtcctcccagctggtacctgttccagttccaccggctcctgcagtacgcacggcccaagccaggcagccccaggcccttcttctggatgttcgtggacaatctggtgctgaacaaggaagacctggacgtcgcatctcgcttcctggagatggagccagtcaccatcccagatgtccacggcggatccttgcagaatgctgtccgcgtgtggagcaacatcccagccataaggagcagcaggcactgggctctggtttcggaagaagaattgtccctgctggcccagaacaagcagagctcgaagctcgcggccaagtggcccaccaagctggtgaagaactgctttctccccctaagagaatatttcaagtatttttcaacagaactcacttcctctttatctagcggcaatagtaacgctaacagccgcgggccgagcttcagcagcggcctggtgccgttaagcttgcgcggcagccatatgaaccatgaccaggaatttgaccccccaaaggtttacccacctgtgccagctgagaagaggaagcccatccgcgtgctgtctctctttgatgggattgctacagggctcctggtgctgaaggacctgggcatccaagtggaccgctacattgcctccgaggtgtgtgaggactccatcacggtgggcatggtgcggcaccagggaaagatcatgtacgtcggggacgtccgcagcgtcacacagaagcatatccaggagtggggcccattcgacctggtgattggaggcagtccctgcaatgacctctccattgtcaaccctgcccgcaagggactttatgagggtactggccgcctcttctttgagttctaccgcctcctgcatgatgcgcggcccaaggagggagatgatcgccccttcttctggctctttgagaatgtggtggccatgggcgttagtgacaagagggacatctcgcgatttcttgagtctaaccccgtgatgattgacgccaaagaagtgtctgctgcacacagggcccgttacttctggggtaaccttcctggcatgaacaggcctttggcatccactgtgaatgataagctggagctgcaagagtgtctggagcacggcagaatagccaagttcagcaaagtgaggaccattaccaccaggtcaaactctataaagcagggcaaagaccagcatttccccgtcttcatgaacgagaaggaggacatcctgtggtgcactgaaatggaaagggtgtttggcttccccgtccactacacagacgtctccaacatgagccgcttggcgaggcagagactgctgggccgatcgtggagcgtgccggtcatccgccacctcttcgctccgctgaaggaatattttgcttgtgtgctcgaggctactaacttcagcctgctgaagcaggctggagacgtggaggagaaccctggacctatgcattaatgagatcccaagcacgcagcaatgcagctcaaaacgcttagcctagccacacccccacgggaaacagcagtgattaacctttagcaataaacgaaagtttaactaagctatactaaccccagggttggtcaatttcgtgccagccacaccctggtactgcatgcacgcaatgctagctgcccctttcccgtcctgggcaccccgagtctcccccgaccccgggtcccaggtatgctcccacctccacctgccccactcaccacctctgctagttccagacacctccgagacgaggaaaaaaaaaaaaaaaaaaaaaaaaaaaaaaaaaaaaaaaaaaaaaaaaaaaaaaaaaaaaaaaaaaaaaaaaaaaaaaaaaaaaaaaaaaaaaaaaaaaaaaaaaaaaaaaaaaaaaaaaaaaaaaaaaaaaaaaaaaaaaaaaaaaaaaaaaaaaaaaaaaaaaaaaaaaaaaaaaaaaaaaaaaaaaaaaaaaaaaaaccgtcttcaagctttctagaaattcactggccgtcgttttacaacgtcgtgactgggaaaaccctggcgttacccaacttaatcgccttgcagcacatccccctttcgccagctggcgtaatagcgaagaggcccgcaccgatcgcccttcccaacagttgcgcagcctgaatggcgaatggcgcctgatgcggtattttctccttacgcatctgtgcggtatttcacaccgcatatggtgcactctcagtacaatctgctctgatgccgcatagttaagccagccccgacacccgccaacacccgctgacgcgccctgacgggcttgtctgctcccggcatccgcttacagacaagctgtgaccgtctccgggagctgcatgtgtcagaggttttcaccgtcatcaccgaaacgcgcgagacgaaagggcctcgtgatacgcctatttttataggttaatgtcatgataataatggtttcttagacgtcaggtggcacttttcggggaaatgtgcgcggaacccctatttgtttatttttctaaatacattcaaatatgtatccgctcatgagacaataaccctgataaatgcttcaataatattgaaaaaggaagagtatgagtattcaacatttccgtgtcgcccttattcccttttttgcggcattttgccttcctgtttttgctcacccagaaacgctggtgaaagtaaaagatgctgaagatcagttgggtgcacgagtgggttacatcgaactggatctcaacagcggtaagatccttgagagttttcgccccgaagaacgttttccaatgatgagcacttttaaagttctgctatgtggcgcggtattatcccgtattgacgccgggcaagagcaactcggtcgccgcatacactattctcagaatgacttggttgagtactcaccagtcacagaaaagcatcttacggatggcatgacagtaagagaattatgcagtgctgccataaccatgagtgataacactgcggccaacttacttctgacaacgatcggaggaccgaaggagctaaccgcttttttgcacaacatgggggatcatgtaactcgccttgatcgttgggaaccggagctgaatgaagccataccaaacgacgagcgtgacaccacgatgcctgtagcaatggcaacaacgttgcgcaaactattaactggcgaactacttactctagcttcccggcaacaattaatagactggatggaggcggataaagttgcaggaccacttctgcgctcggcccttccggctggctggtttattgctgataaatctggagccggtgagcgtgggtctcgcggtatcattgcagcactggggccagatggtaagccctcccgtatcgtagttatctacacgacggggagtcaggcaactatggatgaacgaaatagacagatcgctgagataggtgcctcactgattaagcattggtaactgtcagaccaagtttactcatatatactttagattgatttaaaacttcatttttaatttaaaaggatctaggtgaagatcctttttgataatctcatgaccaaaatcccttaacgtgagttttcgttccactgagcgtcagaccccgtagaaaagatcaaaggatcttcttgagatcctttttttctgcgcgtaatctgctgcttgcaaacaaaaaaaccaccgctaccagcggtggtttgtttgccggatcaagagctaccaactctttttccgaaggtaactggcttcagcagagcgcagataccaaatactgttcttctagtgtagccgtagttaggccaccacttcaagaactctgtagcaccgcctacatacctcgctctgctaatcctgttaccagtggctgctgccagtggcgataagtcgtgtcttaccgggttggactcaagacgatagttaccggataaggcgcagcggtcgggctgaacggggggttcgtgcacacagcccagcttggagcgaacgacctacaccgaact

SEQ ID NO: 230 - DNA, 11236 bp, synthetic construct
  misc_feature 1..11236: note = DNA of V36_scFv-dCas9-HP1a-2a-1xGCN4-D3l-D3a
  source 1..11236: mol_type = other DNA
gagatacctacagcgtgagctatgagaaagcgccacgcttcccgaagggagaaaggcggacaggtatccggtaagcggcagggtcggaacaggagagcgcacgagggagcttccagggggaaacgcctggtatctttatagtcctgtcgggtttcgccacctctgacttgagcgtcgatttttgtgatgctcgtcaggggggcggagcctatggaaaaacgccagcaacgcggcctttttacggttcctggccttttgctggccttttgctcacatgttctttcctgcgttatcccctgattctgtggataaccgtattaccgcctttgagtgagctgataccgctcgccgcagccgaacgaccgagcgcagcgagtcagtgagcgaggaagcggaagagcgcccaatacgcaaaccgcctctccccgcgcgttggccgattcattaatgcagctggcacgacaggtttcccgactggaaagcgggcagtgagcgcaacgcaattaatgtgagttagctcactcattaggcaccccaggctttacactttatgcttccggctcgtatgttgtgtggaattgtgagcggataacaatttcacacaggaaacagctatgaccatgattacgcctctagaaagctttaatacgactcactataaggactcactatttgttttcgcgcccagttgcaaaaagtgtcgacatttgcttctgacacaactgtgttcactagcaacctcaaacagacaccgccaccatgcctgctgctaagagagtgaaactggatggatccggccccgacatcgtgatgacccagagccccagcagcctgagcgccagcgtgggcgaccgcgtgaccatcacctgccgcagcagcaccggcgccgtgaccaccagcaactacgccagctgggtgcaggagaagcccggcaagctgttcaagggcctgatcggcggcaccaacaaccgcgcccccggcgtgcccagccgcttcagcggcagcctgatcggcgacaaggccaccctgaccatcagcagcctgcagcccgaggacttcgccacctacttctgcgccctgtggtacagcaaccactgggtgttcggccagggcaccaaggtggagctgaagcgcggcggcggcggcagcggcggcggcggcagcggcggcggcggcagcagcggcggcggcagcgaggtgaagctgctggagagcggcggcggcctggtgcagcccggcggcagcctgaagctgagctgcgccgtgagcggcttcagcctgaccgactacggcgtgaactgggtgcgccaggcccccggccgcggcctggagtggatcggcgtgatctggggcgacggcatcaccgactacaacagcgccctgaaggaccgcttcatcatcagcaaggacaacggcaagaacaccgtgtacctgcagatgagcaaggtgcgcagcgacgacaccgccctgtactactgcgtgaccggcctgttcgactactggggccagggcaccctggtgaccgtgagcagctacccatacgatgttccagattacgctggtggaggcggaggttctgggggaggaggtagtggcggtggtggttcaggaggcggcggaagcggaagcggaccaaaaaagaagagaaaggtaatggacaagaagtacagcatcggcctggccatcggcaccaactctgtgggctgggccgtgatcaccgacgagtacaaggtgcccagcaagaaattcaaggtgctgggcaacaccgaccggcacagcatcaagaagaacctgatcggcgccctgctgttcgacagcggagaaacagccgaggccacccggctgaagagaaccgccagaagaagatacaccagacggaagaaccggatctgctatctgcaagagatcttcagcaacgagatggccaaggtggacgacagcttcttccacagactggaagagtccttcctggtggaagaggataagaagcacgagcggcaccccatcttcggcaacatcgtggacgaggtggcctaccacgagaagtaccccaccatctaccacctgagaaagaaactggtggacagcaccgacaaggccgacctgcggctgatctatctggccctggcccacatgatcaagttccggggccacttcctgatcgagggcgacctgaaccccgacaacagcgacgtggacaagctgttcatccagctggtgcagacctacaaccagctgttcgaggaaaaccccatcaacgccagcggcgtggacgccaaggccatcctgtctgccagactgagcaagagcagacggctggaaaatctgatcgcccagctgcccggcgagaagaagaatggcctgttcggcaacctgattgccctgagcctgggcctgacccccaacttcaagagcaacttcgacctggccgaggatgccaaactgcagctgagcaaggacacctacgacgacgacctggacaacctgctggcccagatcggcgaccagtacgccgacctgtttctggccgccaagaacctgtccgacgccatcctgctgagcgacatcctgagagtgaacaccgagatcaccaaggcccccctgagcgcctctatgatcaagagatacgacgagcaccaccaggacctgaccctgctgaaagctctcgtgcggcagcagctgcctgagaagtacaaagagattttcttcgaccagagcaagaacggctacgccggctacatcgatggcggagccagccaggaagagttctacaagttcatcaagcccatcctggaaaagatggacggcaccgaggaactgctcgtgaagctgaacagagaggacctgctgcggaagcagcggaccttcgacaacggcagcatcccccaccagatccacctgggagagctgcacgccattctgcggcggcaggaagatttttacccattcctgaaggacaaccgggaaaagatcgagaagatcctgaccttccgcatcccctactacgtgggccctctggccaggggaaacagcagattcgcctggatgaccagaaagagcgaggaaaccatcaccccctggaacttcgaggaagtggtggacaagggcgccagcgcccagagcttcatcgagcggatgaccaacttcgataagaacctgcccaacgagaaggtgctgcccaagcacagcctgctgtacgagtacttcaccgtgtacaacgagctgaccaaagtgaaatacgtgaccgagggaatgagaaagcccgccttcctgagcggcgagcagaaaaaagccatcgtggacctgctgttcaagaccaaccggaaagtgaccgtgaagcagctgaaagaggactacttcaagaaaatcgagtgcttcgactccgtggaaatctccggcgtggaagatcggttcaacgcctccctgggcacataccacgatctgctgaaaattatcaaggacaaggacttcctggacaatgaggaaaacgaggacattctggaagatatcgtgctgaccctgacactgtttgaggacagagagatgatcgaggaacggctgaaaacctatgcccacctgttcgacgacaaagtgatgaagcagctgaagcggcggagatacaccggctggggcaggctgagccggaagctgatcaacggcatccgggacaagcagtccggcaagacaatcctggatttcctgaagtccgacggcttcgccaacagaaacttcatgcagctgatccacgacgacagcctgacctttaaagaggacatccagaaagcccaggtgtccggccagggcgatagcctgcacgagcacattgccaatctggccggcagccccgccattaagaagggcatcctgcagacagtgaaggtggtggacgagctcgtgaaagtgatgggccggcacaagcccgagaacatcgtgatcgaaatggccagagagaaccagaccacccagaagggacagaagaacagccgcgagagaatgaagcggatcgaagagggcatcaaagagctgggcagccagatcctgaaagaacaccccgtggaaaacacccagctgcagaacgagaagctgtacctgtactacctgcagaatgggcgggatatgtacgtggaccaggaactggacatcaaccggctgtccgactacgatgtggacgctatcgtgcctcagagctttctgaaggacgactccatcgataacaaagtgctgactcggagcgacaagaaccggggcaagagcgacaacgtgccctccgaagaggtcgtgaagaagatgaagaactactggcgccagctgctgaatgccaagctgattacccagaggaagttcgacaatctgaccaaggccgagagaggcggcctgagcgaactggataaggccggcttcatcaagagacagctggtggaaacccggcagatcacaaagcacgtggcacagatcctggactcccggatgaacactaagtacgacgagaacgacaaactgatccgggaagtgaaagtgatcaccctgaagtccaagctggtgtccgatttccggaaggatttccagttttacaaagtgcgcgagatcaacaactaccaccacgcccacgacgcctacctgaacgccgtcgtgggaaccgccctgatcaaaaagtaccctaagctggaaagcgagttcgtgtacggcgactacaaggtgtacgacgtgcggaagatgatcgccaagagcgagcaggaaatcggcaaggctaccgccaagtacttcttctacagcaacatcatgaactttttcaagaccgagattaccctggccaacggcgagatccggaagcggcctctgatcgagacaaacggcgaaacaggcgagatcgtgtgggataagggccgggactttgccaccgtgcggaaagtgctgtctatgccccaagtgaatatcgtgaaaaagaccgaggtgcagacaggcggcttcagcaaagagtctatcctgcccaagaggaacagcgacaagctgatcgccagaaagaaggactgggaccctaagaagtacggcggcttcgacagccccaccgtggcctattctgtgctggtggtggccaaagtggaaaagggcaagtccaagaaactgaagagtgtgaaagagctgctggggatcaccatcatggaaagaagcagcttcgagaagaatcccatcgactttctggaagccaagggctacaaagaagtgaaaaaggacctgatcatcaagctgcctaagtactccctgttcgagctggaaaacggccggaagagaatgctggcctctgccggcgaactgcagaagggaaacgaactggccctgccctccaaatatgtgaacttcctgtacctggccagccactatgagaagctgaagggctcccccgaggataatgagcagaaacagctgtttgtggaacagcacaaacactacctggacgagatcatcgagcagatcagcgagttctccaagagagtgatcctggccgacgctaatctggacaaggtgctgagcgcctacaacaagcacagagacaagcctatcagagagcaggccgagaatatcatccacctgtttaccctgaccaatctgggagcccctgccgccttcaagtactttgacaccaccatcgaccggaagaggtacaccagcaccaaagaggtgctggacgccaccctgatccaccagagcatcaccggcctgtacgagacacggatcgacctgtctcagctgggaggcgacgcctatccctatgacgtgcccgattatgccagcctgggcagcggctcccccaagaaaaaacgcaaggtggaagatcctaagaaaaagcggaaagtggacggcagcggcagcgagacccccggtaccagcgagagcgccacccccgagagccggacactcggaaagaaaaccaagcggacagctgacagttcttcttcagaggatgaggaggagtatgttgtggagaaggtgctagacaggcgcgtggttaagggacaagtggaatatctactgaagtggaaaggcttttctgaggagcacaatacttgggaacctgagaaaaacttggattgccctgagctaatttctgaatttatgaaaaagtataagaagatgaaggagggtgaaaataataaacccagggagaagtcagaaagtaacaagaggaaatccaatttctcaaacagtgccgatgacatcaaatctaaaaaaaagagagagcagagcaatgatatcgctcggggctttgagagaggactggaaccagaaaagatcattggggcaacagattcctgtggtgatttaatgttcctaatgaaatggaaagacacagatgaagctgacctggttcttgcaaaagaagctaatgtgaaatgtccacaaattgtgatagcattttatgaagagagactgacatggcatgcatatcctgaggatgcggaaaacaaagagaaagaaacagcaaagagcgagggcagcggcgctactaacttcagcctgctgaagcaggctggagacgtggaggagaaccctggacctatgcctgctgctaagagagtgaaactggatggatccggctcaggcggatctggttcaggggaagaactcctctccaaaaactaccatctcgagaatgaggtcgcccgcctgaaaaaaggatcaggttccggtggttctggcagcggtggttcaggctcaggcagcggcggtagcggtagcggtggaagcggaagcggaacccccggtaccagcgagggcggccctagcagcggcgcccctccccctagcggcggcagccctgccggatcccctacaagcaccgaagaaggcacaagcgagtccgctacccctgagtccggccctggcacctccacagagcctagcgagggatccgctcctggatcccctgccggaagccctacctccaccgaggagggcacaagcaccgagccttccgagggcagcgcccccggaacaagcaccgaacctagcgagagcgccacccccgagagcatgttcgaaaccgtgcctgtgtggaggagacagccagtccgggtgctgtccctttttgaagacatcaagaaagagctgacgagtttgggctttttggaaagtggttctgacccgggacaactgaagcatgtggttgatgtcacagacacagtgaggaaggatgtggaggagtggggacccttcgatcttgtgtacggcgccacacctcccctgggccacacctgtgaccgtcctcccagctggtacctgttccagttccaccggctcctgcagtacgcacggcccaagccaggcagccccaggcccttcttctggatgttcgtggacaatctggtgctgaacaaggaagacctggacgtcgcatctcgcttcctggagatggagccagtcaccatcccagatgtccacggcggatccttgcagaatgctgtccgcgtgtggagcaacatcccagccataaggagcagcaggcactgggctctggtttcggaagaagaattgtccctgctggcccagaacaagcagagctcgaagctcgcggccaagtggcccaccaagctggtgaagaactgctttctccccctaagagaatatttcaagtatttttcaacagaactcacttcctctttatctagcggcaatagtaacgctaacagccgcgggccgagcttcagcagcggcctggtgccgttaagcttgcgcggcagccatatgaaccatgaccaggaatttgaccccccaaaggtttacccacctgtgccagctgagaagaggaagcccatccgcgtgctgtctctctttgatgggattgctacagggctcctggtgctgaaggacctgggcatccaagtggaccgctacattgcctccgaggtgtgtgaggactccatcacggtgggcatggtgcggcaccagggaaagatcatgtacgtcggggacgtccgcagcgtcacacagaagcatatccaggagtggggcccattcgacctggtgattggaggcagtccctgcaatgacctctccattgtcaaccctgcccgcaagggactttatgagggtactggccgcctcttctttgagttctaccgcctcctgcatgatgcgcggcccaaggagggagatgatcgccccttcttctggctctttgagaatgtggtggccatgggcgttagtgacaagagggacatctcgcgatttcttgagtctaaccccgtgatgattgacgccaaagaagtgtctgctgcacacagggcccgttacttctggggtaaccttcctggcatgaacaggcctttggcatccactgtgaatgataagctggagctgcaagagtgtctggagcacggcagaatagccaagttcagcaaagtgaggaccattaccaccaggtcaaactctataaagcagggcaaagaccagcatttccccgtcttcatgaacgagaaggaggacatcctgtggtgcactgaaatggaaagggtgtttggcttccccgtccactacacagacgtctccaacatgagccgcttggcgaggcagagactgctgggccgatcgtggagcgtgccggtcatccgccacctcttcgctccgctgaaggaatattttgcttgtgtgctcgaggctactaacttcagcctgctgaagcaggctggagacgtggaggagaaccctggacctatgcattaatgagatcccaagcacgcagcaatgcagctcaaaacgcttagcctagccacacccccacgggaaacagcagtgattaacctttagcaataaacgaaagtttaactaagctatactaaccccagggttggtcaatttcgtgccagccacaccctggtactgcatgcacgcaatgctagctgcccctttcccgtcctgggcaccccgagtctcccccgaccccgggtcccaggtatgctcccacctccacctgccccactcaccacctctgctagttccagacacctccgagacgaggaaaaaaaaaaaaaaaaaaaaaaaaaaaaaaaaaaaaaaaaaaaaaaaaaaaaaaaaaaaaaaaaaaaaaaaaaaaaaaaaaaaaaaaaaaaaaaaaaaaaaaaaaaaaaaaaaaaaaaaaaaaaaaaaaaaaaaaaaaaaaaaaaaaaaaaaaaaaaaaaaaaaaaaaaaaaaaaaaaaaaaaaaaaaaaaaaaaaaaaaccgtcttcaagctttctagaaattcactggccgtcgttttacaacgtcgtgactgggaaaaccctggcgttacccaacttaatcgccttgcagcacatccccctttcgccagctggcgtaatagcgaagaggcccgcaccgatcgcccttcccaacagttgcgcagcctgaatggcgaatggcgcctgatgcggtattttctccttacgcatctgtgcggtatttcacaccgcatatggtgcactctcagtacaatctgctctgatgccgcatagttaagccagccccgacacccgccaacacccgctgacgcgccctgacgggcttgtctgctcccggcatccgcttacagacaagctgtgaccgtctccgggagctgcatgtgtcagaggttttcaccgtcatcaccgaaacgcgcgagacgaaagggcctcgtgatacgcctatttttataggttaatgtcatgataataatggtttcttagacgtcaggtggcacttttcggggaaatgtgcgcggaacccctatttgtttatttttctaaatacattcaaatatgtatccgctcatgagacaataaccctgataaatgcttcaataatattgaaaaaggaagagtatgagtattcaacatttccgtgtcgcccttattcccttttttgcggcattttgccttcctgtttttgctcacccagaaacgctggtgaaagtaaaagatgctgaagatcagttgggtgcacgagtgggttacatcgaactggatctcaacagcggtaagatccttgagagttttcgccccgaagaacgttttccaatgatgagcacttttaaagttctgctatgtggcgcggtattatcccgtattgacgccgggcaagagcaactcggtcgccgcatacactattctcagaatgacttggttgagtactcaccagtcacagaaaagcatcttacggatggcatgacagtaagagaattatgcagtgctgccataaccatgagtgataacactgcggccaacttacttctgacaacgatcggaggaccgaaggagctaaccgcttttttgcacaacatgggggatcatgtaactcgccttgatcgttgggaaccggagctgaatgaagccataccaaacgacgagcgtgacaccacgatgcctgtagcaatggcaacaacgttgcgcaaactattaactggcgaactacttactctagcttcccggcaacaattaatagactggatggaggcggataaagttgcaggaccacttctgcgctcggcccttccggctggctggtttattgctgataaatctggagccggtgagcgtgggtctcgcggtatcattgcagcactggggccagatggtaagccctcccgtatcgtagttatctacacgacggggagtcaggcaactatggatgaacgaaatagacagatcgctgagataggtgcctcactgattaagcattggtaactgtcagaccaagtttactcatatatactttagattgatttaaaacttcatttttaatttaaaaggatctaggtgaagatcctttttgataatctcatgaccaaaatcccttaacgtgagttttcgttccactgagcgtcagaccccgtagaaaagatcaaaggatcttcttgagatcctttttttctgcgcgtaatctgctgcttgcaaacaaaaaaaccaccgctaccagcggtggtttgtttgccggatcaagagctaccaactctttttccgaaggtaactggcttcagcagagcgcagataccaaatactgttcttctagtgtagccgtagttaggccaccacttcaagaactctgtagcaccgcctacatacctcgctctgctaatcctgttaccagtggctgctgccagtggcgataagtcgtgtcttaccgggttggactcaagacgatagttaccggataaggcgcagcggtcgggctgaacggggggttcgtgcacacagcccagcttggagcgaacgacctacaccgaact

SEQ ID NO: 231 - DNA, 11181 bp, synthetic construct
  misc_feature 1..11181: note = DNA of V37_GFP1-10-KRAB-2a-D3a-D3l-dCas9-7xGFP11
  source 1..11181: mol_type = other DNA
gtacctccacagaaccatctgaaggtagtgcgcctggttccccagctggaagccctacttccaccgaagaaggcacgtcaaccgaaccaagtgaaggatctgcccctgggaccagcactgaaccatctgagccaaaaaagaagagaaaggtaatggacaagaagtacagcatcggcctggccatcggcaccaactctgtgggctgggccgtgatcaccgacgagtacaaggtgcccagcaagaaattcaaggtgctgggcaacaccgaccggcacagcatcaagaagaacctgatcggcgccctgctgttcgacagcggagaaacagccgaggccacccggctgaagagaaccgccagaagaagatacaccagacggaagaaccggatctgctatctgcaagagatcttcagcaacgagatggccaaggtggacgacagcttcttccacagactggaagagtccttcctggtggaagaggataagaagcacgagcggcaccccatcttcggcaacatcgtggacgaggtggcctaccacgagaagtaccccaccatctaccacctgagaaagaaactggtggacagcaccgacaaggccgacctgcggctgatctatctggccctggcccacatgatcaagttccggggccacttcctgatcgagggcgacctgaaccccgacaacagcgacgtggacaagctgttcatccagctggtgcagacctacaaccagctgttcgaggaaaaccccatcaacgccagcggcgtggacgccaaggccatcctgtctgccagactgagcaagagcagacggctggaaaatctgatcgcccagctgcccggcgagaagaagaatggcctgttcggcaacctgattgccctgagcctgggcctgacccccaacttcaagagcaacttcgacctggccgaggatgccaaactgcagctgagcaaggacacctacgacgacgacctggacaacctgctggcccagatcggcgaccagtacgccgacctgtttctggccgccaagaacctgtccgacgccatcctgctgagcgacatcctgagagtgaacaccgagatcaccaaggcccccctgagcgcctctatgatcaagagatacgacgagcaccaccaggacctgaccctgctgaaagctctcgtgcggcagcagctgcctgagaagtacaaagagattttcttcgaccagagcaagaacggctacgccggctacatcgatggcggagccagccaggaagagttctacaagttcatcaagcccatcctggaaaagatggacggcaccgaggaactgctcgtgaagctgaacagagaggacctgctgcggaagcagcggaccttcgacaacggcagcatcccccaccagatccacctgggagagctgcacgccattctgcggcggcaggaagatttttacccattcctgaaggacaaccgggaaaagatcgagaagatcctgaccttccgcatcccctactacgtgggccctctggccaggggaaacagcagattcgcctggatgaccagaaagagcgaggaaaccatcaccccctggaacttcgaggaagtggtggacaagggcgccagcgcccagagcttcatcgagcggatgaccaacttcgataagaacctgcccaacgagaaggtgctgcccaagcacagcctgctgtacgagtacttcaccgtgtacaacgagctgaccaaagtgaaatacgtgaccgagggaatgagaaagcccgccttcctgagcggcgagcagaaaaaagccatcgtggacctgctgttcaagaccaaccggaaagtgaccgtgaagcagctgaaagaggactacttcaagaaaatcgagtgcttcgactccgtggaaatctccggcgtggaagatcggttcaacgcctccctgggcacataccacgatctgctgaaaattatcaaggacaaggacttcctggacaatgaggaaaacgaggacattctggaagatatcgtgctgaccctgacactgtttgaggacagagagatgatcgaggaacggctgaaaacctatgcccacctgttcgacgacaaagtgatgaagcagctgaagcggcggagatacaccggctggggcaggctgagccggaagctgatcaacggcatccgggacaagcagtccggcaagacaatcctggatttcctgaagtccgacggcttcgccaacagaaacttcatgcagctgatccacgacgacagcctgacctttaaagaggacatccagaaagcccaggtgtccggccagggcgatagcctgcacgagcacattgccaatctggccggcagccccgccattaagaagggcatcctgcagacagtgaaggtggtggacgagctcgtgaaagtgatgggccggcacaagcccgagaacatcgtgatcgaaatggccagagagaaccagaccacccagaagggacagaagaacagccgcgagagaatgaagcggatcgaagagggcatcaaagagctgggcagccagatcctgaaagaacaccccgtggaaaacacccagctgcagaacgagaagctgtacctgtactacctgcagaatgggcgggatatgtacgtggaccaggaactggacatcaaccggctgtccgactacgatgtggacgctatcgtgcctcagagctttctgaaggacgactccatcgataacaaagtgctgactcggagcgacaagaaccggggcaagagcgacaacgtgccctccgaagaggtcgtgaagaagatgaagaactactggcgccagctgctgaatgccaagctgattacccagaggaagttcgacaatctgaccaaggccgagagaggcggcctgagcgaactggataaggccggcttcatcaagagacagctggtggaaacccggcagatcacaaagcacgtggcacagatcctggactcccggatgaacactaagtacgacgagaacgacaaactgatccgggaagtgaaagtgatcaccctgaagtccaagctggtgtccgatttccggaaggatttccagttttacaaagtgcgcgagatcaacaactaccaccacgcccacgacgcctacctgaacgccgtcgtgggaaccgccctgatcaaaaagtaccctaagctggaaagcgagttcgtgtacggcgactacaaggtgtacgacgtgcggaagatgatcgccaagagcgagcaggaaatcggcaaggctaccgccaagtacttcttctacagcaacatcatgaactttttcaagaccgagattaccctggccaacggcgagatccggaagcggcctctgatcgagacaaacggcgaaacaggcgagatcgtgtgggataagggccgggactttgccaccgtgcggaaagtgctgtctatgccccaagtgaatatcgtgaaaaagaccgaggtgcagacaggcggcttcagcaaagagtctatcctgcccaagaggaacagcgacaagctgatcgccagaaagaaggactgggaccctaagaagtacggcggcttcgacagccccaccgtggcctattctgtgctggtggtggccaaagtggaaaagggcaagtccaagaaactgaagagtgtgaaagagctgctggggatcaccatcatggaaagaagcagcttcgagaagaatcccatcgactttctggaagccaagggctacaaagaagtgaaaaaggacctgatcatcaagctgcctaagtactccctgttcgagctggaaaacggccggaagagaatgctggcctctgccggcgaactgcagaagggaaacgaactggccctgccctccaaatatgtgaacttcctgtacctggccagccactatgagaagctgaagggctcccccgaggataatgagcagaaacagctgtttgtggaacagcacaaacactacctggacgagatcatcgagcagatcagcgagttctccaagagagtgatcctggccgacgctaatctggacaaggtgctgagcgcctacaacaagcacagagacaagcctatcagagagcaggccgagaatatcatccacctgtttaccctgaccaatctgggagcccctgccgccttcaagtactttgacaccaccatcgaccggaagaggtacaccagcaccaaagaggtgctggacgccaccctgatccaccagagcatcaccggcctgtacgagacacggatcgacctgtctcagctgggaggcgacgcctatccctatgacgtgcccgattatgccagcctgggcagcggctcccccaagaaaaaacgcaaggtggaagatcctaagaaaaagcggaaagtggacggcagcggcagcgagacccccggtaccagcgagagcgccacccccgagagcggtagtgggagcaacggcagcagcggatccatgcgtgaccacatggtccttcatgagtatgtaaatgctgctgggattacaggtggctctggaggtagagatcatatggttctccacgaatacgttaacgccgcaggcatcactggcggtagtggaggacgcgaccatatggtactacatgaatatgtcaatgcagccggaataaccggagggtccggaggccgggatcacatggtgctgcatgagtatgtgaacgcggcgggtataactggtgggtcgggcggacgagaccatatggtgcttcacgaatacgtaaacgcagctggcattactggcggatcaggtggcagggatcacatggtactccatgagtacgtgaacgctgctggaatcacaggcggtagcggcggtcgggaccatatggtcctgcacgaatatgtcaatgctgccggtatcaccgcggccgcaaggtcaggctccggccagcggggaagcaagcgcaccgccgatggttccgagttcgaaagccccaaaaaaaagcgcaaggtctgagatcccaagcacgcagcaatgcagctcaaaacgcttagcctagccacacccccacgggaaacagcagtgattaacctttagcaataaacgaaagtttaactaagctatactaaccccagggttggtcaatttcgtgccagccacaccctggtactgcatgcacgcaatgctagctgcccctttcccgtcctgggcaccccgagtctcccccgaccccgggtcccaggtatgctcccacctccacctgccccactcaccacctctgctagttccagacacctccgagacgaggaaaaaaaaaaaaaaaaaaaaaaaaaaaaaaaaaaaaaaaaaaaaaaaaaaaaaaaaaaaaaaaaaaaaaaaaaaaaaaaaaaaaaaaaaaaaaaaaaaaaaaaaaaaaaaaaaaaaaaaaaaaaaaaaaaaaaaaaaaaaaaaaaaaaaaaaaaaaaaaaaaaaaaaaaaaaaaaaaaaaaaaaaaaaaaaaaaaaaaaaaaaaaaaaaaaaaaaaaaaaaaaaaaaaaaaaaaaaaaaaaaaaaaaaaaaaaaaaaaaaaaaaaaaaaaaaaaaaaaaaaaaaaaaaaaaaaaaaaaaaaaaaaaaaaaaaaaaaaaaaaaaaaaaaaaaaaaaaaaaaaaaaaaaaaaaaaaaaaaaaaaaaaaaaaaaaaaaaaaaaaaaaaaaaaaaaaaccgtcttcaagctttctagaaattcactggccgtcgttttacaacgtcgtgactgggaaaaccctggcgttacccaacttaatcgccttgcagcacatccccctttcgccagctggcgtaatagcgaagaggcccgcaccgatcgcccttcccaacagttgcgcagcctgaatggcgaatggcgcctgatgcggtattttctccttacgcatctgtgcggtatttcacaccgcatatggtgcactctcagtacaatctgctctgatgccgcatagttaagccagccccgacacccgccaacacccgctgacgcgccctgacgggcttgtctgctcccggcatccgcttacagacaagctgtgaccgtctccgggagctgcatgtgtcagaggttttcaccgtcatcaccgaaacgcgcgagacgaaagggcctcgtgatacgcctatttttataggttaatgtcatgataataatggtttcttagacgtcaggtggcacttttcggggaaatgtgcgcggaacccctatttgtttatttttctaaatacattcaaatatgtatccgctcatgagacaataaccctgataaatgcttcaataatattgaaaaaggaagagtatgagtattcaacatttccgtgtcgcccttattcccttttttgcggcattttgccttcctgtttttgctcacccagaaacgctggtgaaagtaaaagatgctgaagatcagttgggtgcacgagtgggttacatcgaactggatctcaacagcggtaagatccttgagagttttcgccccgaagaacgttttccaatgatgagcacttttaaagttctgctatgtggcgcggtattatcccgtattgacgccgggcaagagcaactcggtcgccgcatacactattctcagaatgacttggttgagtactcaccagtcacagaaaagcatcttacggatggcatgacagtaagagaattatgcagtgctgccataaccatgagtgataacactgcggccaacttacttctgacaacgatcggaggaccgaaggagctaaccgcttttttgcacaacatgggggatcatgtaactcgccttgatcgttgggaaccggagctgaatgaagccataccaaacgacgagcgtgacaccacgatgcctgtagcaatggcaacaacgttgcgcaaactattaactggcgaactacttactctagcttcccggcaacaattaatagactggatggaggcggataaagttgcaggaccacttctgcgctcggcccttccggctggctggtttattgctgataaatctggagccggtgagcgtgggtctcgcggtatcattgcagcactggggccagatggtaagccctcccgtatcgtagttatctacacgacggggagtcaggcaactatggatgaacgaaatagacagatcgctgagataggtgcctcactgattaagcattggtaactgtcagaccaagtttactcatatatactttagattgatttaaaacttcatttttaatttaaaaggatctaggtgaagatcctttttgataatctcatgaccaaaatcccttaacgtgagttttcgttccactgagcgtcagaccccgtagaaaagatcaaaggatcttcttgagatcctttttttctgcgcgtaatctgctgcttgcaaacaaaaaaaccaccgctaccagcggtggtttgtttgccggatcaagagctaccaactctttttccgaaggtaactggcttcagcagagcgcagataccaaatactgttcttctagtgtagccgtagttaggccaccacttcaagaactctgtagcaccgcctacatacctcgctctgctaatcctgttaccagtggctgctgccagtggcgataagtcgtgtcttaccgggttggactcaagacgatagttaccggataaggcgcagcggtcgggctgaacggggggttcgtgcacacagcccagcttggagcgaacgacctacaccgaactgagatacctacagcgtgagctatgagaaagcgccacgcttcccgaagggagaaaggcggacaggtatccggtaagcggcagggtcggaacaggagagcgcacgagggagcttccagggggaaacgcctggtatctttatagtcctgtcgggtttcgccacctctgacttgagcgtcgatttttgtgatgctcgtcaggggggcggagcctatggaaaaacgccagcaacgcggcctttttacggttcctggccttttgctggccttttgctcacatgttctttcctgcgttatcccctgattctgtggataaccgtattaccgcctttgagtgagctgataccgctcgccgcagccgaacgaccgagcgcagcgagtcagtgagcgaggaagcggaagagcgcccaatacgcaaaccgcctctccccgcgcgttggccgattcattaatgcagctggcacgacaggtttcccgactggaaagcgggcagtgagcgcaacgcaattaatgtgagttagctcactcattaggcaccccaggctttacactttatgcttccggctcgtatgttgtgtggaattgtgagcggataacaatttcacacaggaaacagctatgaccatgattacgcctctagaaagctttaatacgactcactataaggactcactatttgttttcgcgcccagttgcaaaaagtgtcgacatttgcttctgacacaactgtgttcactagcaacctcaaacagacaccgccaccatgtccaagggagaggagctgttcaccggagtggtgccaatcctggtggagctggacggcgatgtgaacggccacaagttttctgtgcgcggagagggagagggcgacgcaaccatcggcaagctgacactgaagttcatctgcaccacaggcaagctgcccgtgccttggccaaccctggtgaccacactgacatacggcgtgcagtgtttctctaggtatccagaccacatgaagagacacgatttctttaagagcgccatgccagagggatacgtgcaggagcggaccatctccttcaaggacgatggcaagtataagacccgcgccgtggtgaagtttgagggcgatacactggtgaacaggatcgagctgaagggcaccgacttcaaggaggatggcaatatcctgggccacaagctggagtacaactttaatagccacaacgtgtatatcacagccgacaagcagaagaacggcatcaaggccaacttcaccgtgaggcacaatgtggaggacggctccgtgcagctggccgatcactaccagcagaacacacctatcggcgacggacccgtgctgctgcctgataatcactatctgtccacccagacagtgctgtctaaggacccaaacgagaagttggatccaggtggaggtggaagcggtcggacactggtgaccttcaaggatgtatttgtggacttcaccagggaggagtggaagctgctggacactgctcagcagatcgtgtacagaaatgtgatgctggagaactataagaacctggtttccttgggttatcagcttactaagccagatgtgatcctccggttggagaagggagaagagcccggaagcggaaagcgcaccgccgatggttccgagttcgaaagccccaaaaaaaagcgcaaggtcggaagcggagctactaacttcagcctgctgaagcaggctggagacgtggaggagaaccctggacctcctgctgctaagagagtgaaactggatggatccaaccatgaccaggaatttgaccccccaaaggtttacccacctgtgccagctgagaagaggaagcccatccgcgtgctgtctctctttgatgggattgctacagggctcctggtgctgaaggacctgggcatccaagtggaccgctacattgcctccgaggtgtgtgaggactccatcacggtgggcatggtgcggcaccagggaaagatcatgtacgtcggggacgtccgcagcgtcacacagaagcatatccaggagtggggcccattcgacctggtgattggaggcagtccctgcaatgacctctccattgtcaaccctgcccgcaagggactttatgagggtactggccgcctcttctttgagttctaccgcctcctgcatgatgcgcggcccaaggagggagatgatcgccccttcttctggctctttgagaatgtggtggccatgggcgttagtgacaagagggacatctcgcgatttcttgagtctaaccccgtgatgattgacgccaaagaagtgtctgctgcacacagggcccgttacttctggggtaaccttcctggcatgaacaggcctttggcatccactgtgaatgataagctggagctgcaagagtgtctggagcacggcagaatagccaagttcagcaaagtgaggaccattaccaccaggtcaaactctataaagcagggcaaagaccagcatttccccgtgttcatgaacgagaaggaggacatcctgtggtgcactgaaatggaaagggtgtttggcttccccgtccactacacagacgtctccaacatgagccgcttggcgaggcagagactgctgggccgatcgtggagcgtgccggtcatccgccacctcttcgctccgctgaaggaatattttgcttgtgtgtctagcggcaatagtaacgctaacagccgcgggccgagcttcagcagcggcctggtgccgttaagcttgcgcggcagccatatgggccctatggagatatacaagacagtgtctgcatggaagagacagccagtgcgggtactgagcctcttcagaaacatcgacaaggtactaaagagtttgggcttcttggaaagcggttctggttctgggggaggaacgctgaagtacgtggaagatgtcacaaatgtcgtgaggagagacgtggagaaatggggcccctttgacctggtgtacggctcgacgcagcccctaggcagctcttgtgatcgctgtcccggctggtacatgttccagttccaccggatcctgcagtatgcgctgcctcgccaggagagtcagcggcccttcttctggatattcatggacaatctgctgctgactgaggatgaccaagagacaactacccgcttccttcagacagaggctgtgaccctccaggatgtccgtggcagagactaccagaatgctatgcgggtgtggagcaacattccagggctgaagagcaagcatgcgcccctgaccccaaaggaagaagagtatctgcaagcccaagtcagaagcaggagcaagctggacgccccgaaagttgacctcctggtgaagaactgccttctcccgctgagagagtacttcaagtatttttctcaaaactcacttcctcttggagggccgagctctggcgcacccccaccaagtggagggtctcctgccgggtccccaacatctactgaagaaggcaccagcgaatccgcaacgcccgagtcaggccctg

SEQ ID NO: 232 - DNA, 10803 bp, synthetic construct
  misc_feature 1..10803: note = DNA of V38_GFP1-10-KRAB-2a-D3a-D3l-dCas9-1xGFP11
  source 1..10803: mol_type = other DNA
gcaaggtcaggctccggccagcggggaagcaagcgcaccgccgatggttccgagttcgaaagccccaaaaaaaagcgcaaggtctgagatcccaagcacgcagcaatgcagctcaaaacgcttagcctagccacacccccacgggaaacagcagtgattaacctttagcaataaacgaaagtttaactaagctatactaaccccagggttggtcaatttcgtgccagccacaccctggtactgcatgcacgcaatgctagctgcccctttcccgtcctgggcaccccgagtctcccccgaccccgggtcccaggtatgctcccacctccacctgccccactcaccacctctgctagttccagacacctccgagacgaggaaaaaaaaaaaaaaaaaaaaaaaaaaaaaaaaaaaaaaaaaaaaaaaaaaaaaaaaaaaaaaaaaaaaaaaaaaaaaaaaaaaaaaaaaaaaaaaaaaaaaaaaaaaaaaaaaaaaaaaaaaaaaaaaaaaaaaaaaaaaaaaaaaaaaaaaaaaaaaaaaaaaaaaaaaaaaaaaaaaaaaaaaaaaaaaaaaaaaaaaaaaaaaaaaaaaaaaaaaaaaaaaaaaaaaaaaaaaaaaaaaaaaaaaaaaaaaaaaaaaaaaaaaaaaaaaaaaaaaaaaaaaaaaaaaaaaaaaaaaaaaaaaaaaaaaaaaaaaaaaaaaaaaaaaaaaaaaaaaaaaaaaaaaaaaaaaaaaaaaaaaaaaaaaaaaaaaaaaaaaaaaaaaaaaaaaaaccgtcttcaagctttctagaaattcactggccgtcgttttacaacgtcgtgactgggaaaaccctggcgttacccaacttaatcgccttgcagcacatccccctttcgccagctggcgtaatagcgaagaggcccgcaccgatcgcccttcccaacagttgcgcagcctgaatggcgaatggcgcctgatgcggtattttctccttacgcatctgtgcggtatttcacaccgcatatggtgcactctcagtacaatctgctctgatgccgcatagttaagccagccccgacacccgccaacacccgctgacgcgccctgacgggcttgtctgctcccggcatccgcttacagacaagctgtgaccgtctccgggagctgcatgtgtcagaggttttcaccgtcatcaccgaaacgcgcgagacgaaagggcctcgtgatacgcctatttttataggttaatgtcatgataataatggtttcttagacgtcaggtggcacttttcggggaaatgtgcgcggaacccctatttgtttatttttctaaatacattcaaatatgtatccgctcatgagacaataaccctgataaatgcttcaataatattgaaaaaggaagagtatgagtattcaacatttccgtgtcgcccttattcccttttttgcggcattttgccttcctgtttttgctcacccagaaacgctggtgaaagtaaaagatgctgaagatcagttgggtgcacgagtgggttacatcgaactggatctcaacagcggtaagatccttgagagttttcgccccgaagaacgttttccaatgatgagcacttttaaagttctgctatgtggcgcggtattatcccgtattgacgccgggcaagagcaactcggtcgccgcatacactattctcagaatgacttggttgagtactcaccagtcacagaaaagcatcttacggatggcatgacagtaagagaattatgcagtgctgccataaccatgagtgataacactgcggccaacttacttctgacaacgatcggaggaccgaaggagctaaccgcttttttgcacaacatgggggatcatgtaactcgccttgatcgttgggaaccggagctgaatgaagccataccaaacgacgagcgtgacaccacgatgcctgtagcaatggcaacaacgttgcgcaaactattaactggcgaactacttactctagcttcccggcaacaattaatagactggatggaggcggataaagttgcaggaccacttctgcgctcggcccttccggctggctggtttattgctgataaatctggagccggtgagcgtgggtctcgcggtatcattgcagcactggggccagatggtaagccctcccgtatcgtagttatctacacgacggggagtcaggcaactatggatgaacgaaatagacagatcgctgagataggtgcctcactgattaagcattggtaactgtcagaccaagtttactcatatatactttagattgatttaaaacttcatttttaatttaaaaggatctaggtgaagatcctttttgataatctcatgaccaaaatcccttaacgtgagttttcgttccactgagcgtcagaccccgtagaaaagatcaaaggatcttcttgagatcctttttttctgcgcgtaatctgctgcttgcaaacaaaaaaaccaccgctaccagcggtggtttgtttgccggatcaagagctaccaactctttttccgaaggtaactggcttcagcagagcgcagataccaaatactgttcttctagtgtagccgtagttaggccaccacttcaagaactctgtagcaccgcctacatacctcgctctgctaatcctgttaccagtggctgctgccagtggcgataagtcgtgtcttaccgggttggactcaagacgatagttaccggataaggcgcagcggtcgggctgaacggggggttcgtgcacacagcccagcttggagcgaacgacctacaccgaactgagatacctacagcgtgagctatgagaaagcgccacgcttcccgaagggagaaaggcggacaggtatccggtaagcggcagggtcggaacaggagagcgcacgagggagcttccagggggaaacgcctggtatctttatagtcctgtcgggtttcgccacctctgacttgagcgtcgatttttgtgatgctcgtcaggggggcggagcctatggaaaaacgccagcaacgcggcctttttacggttcctggccttttgctggccttttgctcacatgttctttcctgcgttatcccctgattctgtggataaccgtattaccgcctttgagtgagctgataccgctcgccgcagccgaacgaccgagcgcagcgagtcagtgagcgaggaagcggaagagcgcccaatacgcaaaccgcctctccccgcgcgttggccgattcattaatgcagctggcacgacaggtttcccgactggaaagcgggcagtgagcgcaacgcaattaatgtgagttagctcactcattaggcaccccaggctttacactttatgcttccggctcgtatgttgtgtggaattgtgagcggataacaatttcacacaggaaacagctatgaccatgattacgcctctagaaagctttaatacgactcactataaggactcactatttgttttcgcgcccagttgcaaaaagtgtcgacatttgcttctgacacaactgtgttcactagcaacctcaaacagacaccgccaccatgtccaagggagaggagctgttcaccggagtggtgccaatcctggtggagctggacggcgatgtgaacggccacaagttttctgtgcgcggagagggagagggcgacgcaaccatcggcaagctgacactgaagttcatctgcaccacaggcaagctgcccgtgccttggccaaccctggtgaccacactgacatacggcgtgcagtgtttctctaggtatccagaccacatgaagagacacgatttctttaagagcgccatgccagagggatacgtgcaggagcggaccatctccttcaaggacgatggcaagtataagacccgcgccgtggtgaagtttgagggcgatacactggtgaacaggatcgagctgaagggcaccgacttcaaggaggatggcaatatcctgggccacaagctggagtacaactttaatagccacaacgtgtatatcacagccgacaagcagaagaacggcatcaaggccaacttcaccgtgaggcacaatgtggaggacggctccgtgcagctggccgatcactaccagcagaacacacctatcggcgacggacccgtgctgctgcctgataatcactatctgtccacccagacagtgctgtctaaggacccaaacgagaagttggatccaggtggaggtggaagcggtcggacactggtgaccttcaaggatgtatttgtggacttcaccagggaggagtggaagctgctggacactgctcagcagatcgtgtacagaaatgtgatgctggagaactataagaacctggtttccttgggttatcagcttactaagccagatgtgatcctccggttggagaagggagaagagcccggaagcggaaagcgcaccgccgatggttccgagttcgaaagccccaaaaaaaagcgcaaggtcggaagcggagctactaacttcagcctgctgaagcaggctggagacgtggaggagaaccctggacctcctgctgctaagagagtgaaactggatggatccaaccatgaccaggaatttgaccccccaaaggtttacccacctgtgccagctgagaagaggaagcccatccgcgtgctgtctctctttgatgggattgctacagggctcctggtgctgaaggacctgggcatccaagtggaccgctacattgcctccgaggtgtgtgaggactccatcacggtgggcatggtgcggcaccagggaaagatcatgtacgtcggggacgtccgcagcgtcacacagaagcatatccaggagtggggcccattcgacctggtgattggaggcagtccctgcaatgacctctccattgtcaaccctgcccgcaagggactttatgagggtactggccgcctcttctttgagttctaccgcctcctgcatgatgcgcggcccaaggagggagatgatcgccccttcttctggctctttgagaatgtggtggccatgggcgttagtgacaagagggacatctcgcgatttcttgagtctaaccccgtgatgattgacgccaaagaagtgtctgctgcacacagggcccgttacttctggggtaaccttcctggcatgaacaggcctttggcatccactgtgaatgataagctggagctgcaagagtgtctggagcacggcagaatagccaagttcagcaaagtgaggaccattaccaccaggtcaaactctataaagcagggcaaagaccagcatttccccgtgttcatgaacgagaaggaggacatcctgtggtgcactgaaatggaaagggtgtttggcttccccgtccactacacagacgtctccaacatgagccgcttggcgaggcagagactgctgggccgatcgtggagcgtgccggtcatccgccacctcttcgctccgctgaaggaatattttgcttgtgtgtctagcggcaatagtaacgctaacagccgcgggccgagcttcagcagcggcctggtgccgttaagcttgcgcggcagccatatgggccctatggagatatacaagacagtgtctgcatggaagagacagccagtgcgggtactgagcctcttcagaaacatcgacaaggtactaaagagtttgggcttcttggaaagcggttctggttctgggggaggaacgctgaagtacgtggaagatgtcacaaatgtcgtgaggagagacgtggagaaatggggcccctttgacctggtgtacggctcgacgcagcccctaggcagctcttgtgatcgctgtcccggctggtacatgttccagttccaccggatcctgcagtatgcgctgcctcgccaggagagtcagcggcccttcttctggatattcatggacaatctgctgctgactgaggatgaccaagagacaactacccgcttccttcagacagaggctgtgaccctccaggatgtccgtggcagagactaccagaatgctatgcgggtgtggagcaacattccagggctgaagagcaagcatgcgcccctgaccccaaaggaagaagagtatctgcaagcccaagtcagaagcaggagcaagctggacgccccgaaagttgacctcctggtgaagaactgccttctcccgctgagagagtacttcaagtatttttctcaaaactcacttcctcttggagggccgagctctggcgcacccccaccaagtggagggtctcctgccgggtccccaacatctactgaagaaggcaccagcgaatccgcaacgcccgagtcaggccctggtacctccacagaaccatctgaaggtagtgcgcctggttccccagctggaagccctacttccaccgaagaaggcacgtcaaccgaaccaagtgaaggatctgcccctgggaccagcactgaaccatctgagccaaaaaagaagagaaaggtaatggacaagaagtacagcatcggcctggccatcggcaccaactctgtgggctgggccgtgatcaccgacgagtacaaggtgcccagcaagaaattcaaggtgctgggcaacaccgaccggcacagcatcaagaagaacctgatcggcgccctgctgttcgacagcggagaaacagccgaggccacccggctgaagagaaccgccagaagaagatacaccagacggaagaaccggatctgctatctgcaagagatcttcagcaacgagatggccaaggtggacgacagcttcttccacagactggaagagtccttcctggtggaagaggataagaagcacgagcggcaccccatcttcggcaacatcgtggacgaggtggcctaccacgagaagtaccccaccatctaccacctgagaaagaaactggtggacagcaccgacaaggccgacctgcggctgatctatctggccctggcccacatgatcaagttccggggccacttcctgatcgagggcgacctgaaccccgacaacagcgacgtggacaagctgttcatccagctggtgcagacctacaaccagctgttcgaggaaaaccccatcaacgccagcggcgtggacgccaaggccatcctgtctgccagactgagcaagagcagacggctggaaaatctgatcgcccagctgcccggcgagaagaagaatggcctgttcggcaacctgattgccctgagcctgggcctgacccccaacttcaagagcaacttcgacctggccgaggatgccaaactgcagctgagcaaggacacctacgacgacgacctggacaacctgctggcccagatcggcgaccagtacgccgacctgtttctggccgccaagaacctgtccgacgccatcctgctgagcgacatcctgagagtgaacaccgagatcaccaaggcccccctgagcgcctctatgatcaagagatacgacgagcaccaccaggacctgaccctgctgaaagctctcgtgcggcagcagctgcctgagaagtacaaagagattttcttcgaccagagcaagaacggctacgccggctacatcgatggcggagccagccaggaagagttctacaagttcatcaagcccatcctggaaaagatggacggcaccgaggaactgctcgtgaagctgaacagagaggacctgctgcggaagcagcggaccttcgacaacggcagcatcccccaccagatccacctgggagagctgcacgccattctgcggcggcaggaagatttttacccattcctgaaggacaaccgggaaaagatcgagaagatcctgaccttccgcatcccctactacgtgggccctctggccaggggaaacagcagattcgcctggatgaccagaaagagcgaggaaaccatcaccccctggaacttcgaggaagtggtggacaagggcgccagcgcccagagcttcatcgagcggatgaccaacttcgataagaacctgcccaacgagaaggtgctgcccaagcacagcctgctgtacgagtacttcaccgtgtacaacgagctgaccaaagtgaaatacgtgaccgagggaatgagaaagcccgccttcctgagcggcgagcagaaaaaagccatcgtggacctgctgttcaagaccaaccggaaagtgaccgtgaagcagctgaaagaggactacttcaagaaaatcgagtgcttcgactccgtggaaatctccggcgtggaagatcggttcaacgcctccctgggcacataccacgatctgctgaaaattatcaaggacaaggacttcctggacaatgaggaaaacgaggacattctggaagatatcgtgctgaccctgacactgtttgaggacagagagatgatcgaggaacggctgaaaacctatgcccacctgttcgacgacaaagtgatgaagcagctgaagcggcggagatacaccggctggggcaggctgagccggaagctgatcaacggcatccgggacaagcagtccggcaagacaatcctggatttcctgaagtccgacggcttcgccaacagaaacttcatgcagctgatccacgacgacagcctgacctttaaagaggacatccagaaagcccaggtgtccggccagggcgatagcctgcacgagcacattgccaatctggccggcagccccgccattaagaagggcatcctgcagacagtgaaggtggtggacgagctcgtgaaagtgatgggccggcacaagcccgagaacatcgtgatcgaaatggccagagagaaccagaccacccagaagggacagaagaacagccgcgagagaatgaagcggatcgaagagggcatcaaagagctgggcagccagatcctgaaagaacaccccgtggaaaacacccagctgcagaacgagaagctgtacctgtactacctgcagaatgggcgggatatgtacgtggaccaggaactggacatcaaccggctgtccgactacgatgtggacgctatcgtgcctcagagctttctgaaggacgactccatcgataacaaagtgctgactcggagcgacaagaaccggggcaagagcgacaacgtgccctccgaagaggtcgtgaagaagatgaagaactactggcgccagctgctgaatgccaagctgattacccagaggaagttcgacaatctgaccaaggccgagagaggcggcctgagcgaactggataaggccggcttcatcaagagacagctggtggaaacccggcagatcacaaagcacgtggcacagatcctggactcccggatgaacactaagtacgacgagaacgacaaactgatccgggaagtgaaagtgatcaccctgaagtccaagctggtgtccgatttccggaaggatttccagttttacaaagtgcgcgagatcaacaactaccaccacgcccacgacgcctacctgaacgccgtcgtgggaaccgccctgatcaaaaagtaccctaagctggaaagcgagttcgtgtacggcgactacaaggtgtacgacgtgcggaagatgatcgccaagagcgagcaggaaatcggcaaggctaccgccaagtacttcttctacagcaacatcatgaactttttcaagaccgagattaccctggccaacggcgagatccggaagcggcctctgatcgagacaaacggcgaaacaggcgagatcgtgtgggataagggccgggactttgccaccgtgcggaaagtgctgtctatgccccaagtgaatatcgtgaaaaagaccgaggtgcagacaggcggcttcagcaaagagtctatcctgcccaagaggaacagcgacaagctgatcgccagaaagaaggactgggaccctaagaagtacggcggcttcgacagccccaccgtggcctattctgtgctggtggtggccaaagtggaaaagggcaagtccaagaaactgaagagtgtgaaagagctgctggggatcaccatcatggaaagaagcagcttcgagaagaatcccatcgactttctggaagccaagggctacaaagaagtgaaaaaggacctgatcatcaagctgcctaagtactccctgttcgagctggaaaacggccggaagagaatgctggcctctgccggcgaactgcagaagggaaacgaactggccctgccctccaaatatgtgaacttcctgtacctggccagccactatgagaagctgaagggctcccccgaggataatgagcagaaacagctgtttgtggaacagcacaaacactacctggacgagatcatcgagcagatcagcgagttctccaagagagtgatcctggccgacgctaatctggacaaggtgctgagcgcctacaacaagcacagagacaagcctatcagagagcaggccgagaatatcatccacctgtttaccctgaccaatctgggagcccctgccgccttcaagtactttgacaccaccatcgaccggaagaggtacaccagcaccaaagaggtgctggacgccaccctgatccaccagagcatcaccggcctgtacgagacacggatcgacctgtctcagctgggaggcgacgcctatccctatgacgtgcccgattatgccagcctgggcagcggctcccccaagaaaaaacgcaaggtggaagatcctaagaaaaagcggaaagtggacggcagcggcagcgagacccccggtaccagcgagagcgccacccccgagagcggtagtgggagcaacggcagcagcggatccatgcgtgaccacatggtccttcatgagtatgtaaatgctgctgggattacagcggcc

SEQ ID NO: 233 - DNA, 10821 bp, synthetic construct
  misc_feature 1..10821: note = DNA of V39_GFP1-10-ZIM3-2a-D3a-hD3L-dCas9-1xGFP11
  source 1..10821: mol_type = other DNA
gcaaggtcaggctccggccagcggggaagcaagcgcaccgccgatggttccgagttcgaaagccccaaaaaaaagcgcaaggtctgagatcccaagcacgcagcaatgcagctcaaaacgcttagcctagccacacccccacgggaaacagcagtgattaacctttagcaataaacgaaagtttaactaagctatactaaccccagggttggtcaatttcgtgccagccacaccctggtactgcatgcacgcaatgctagctgcccctttcccgtcctgggcaccccgagtctcccccgaccccgggtcccaggtatgctcccacctccacctgccccactcaccacctctgctagttccagacacctccgagacgaggaaaaaaaaaaaaaaaaaaaaaaaaaaaaaaaaaaaaaaaaaaaaaaaaaaaaaaaaaaaaaaaaaaaaaaaaaaaaaaaaaaaaaaaaaaaaaaaaaaaaaaaaaaaaaaaaaaaaaaaaaaaaaaaaaaaaaaaaaaaaaaaaaaaaaaaaaaaaaaaaaaaaaaaaaaaaaaaaaaaaaaaaaaaaaaaaaaaaaaaaaaaaaaaaaaaaaaaaaaaaaaaaaaaaaaaaaaaaaaaaaaaaaaaaaaaaaaaaaaaaaaaaaaaaaaaaaaaaaaaaaaaaaaaaaaaaaaaaaaaaaaaaaaaaaaaaaaaaaaaaaaaaaaaaaaaaaaaaaaaaaaaaaaaaaaaaaaaaaaaaaaaaaaaaaaaaaaaaaaaaaaaaaaaaaaaaaaccgtcttcaagctttctagaaattcactggccgtcgttttacaacgtcgtgactgggaaaaccctggcgttacccaacttaatcgccttgcagcacatccccctttcgccagctggcgtaatagcgaagaggcccgcaccgatcgcccttcccaacagttgcgcagcctgaatggcgaatggcgcctgatgcggtattttctccttacgcatctgtgcggtatttcacaccgcatatggtgcactctcagtacaatctgctctgatgccgcatagttaagccagccccgacacccgccaacacccgctgacgcgccctgacgggcttgtctgctcccggcatccgcttacagacaagctgtgaccgtctccgggagctgcatgtgtcagaggttttcaccgtcatcaccgaaacgcgcgagacgaaagggcctcgtgatacgcctatttttataggttaatgtcatgataataatggtttcttagacgtcaggtggcacttttcggggaaatgtgcgcggaacccctatttgtttatttttctaaatacattcaaatatgtatccgctcatgagacaataaccctgataaatgcttcaataatattgaaaaaggaagagtatgagtattcaacatttccgtgtcgcccttattcccttttttgcggcattttgccttcctgtttttgctcacccagaaacgctggtgaaagtaaaagatgctgaagatcagttgggtgcacgagtgggttacatcgaactggatctcaacagcggtaagatccttgagagttttcgccccgaagaacgttttccaatgatgagcacttttaaagttctgctatgtggcgcggtattatcccgtattgacgccgggcaagagcaactcggtcgccgcatacactattctcagaatgacttggttgagtactcaccagtcacagaaaagcatcttacggatggcatgacagtaagagaattatgcagtgctgccataaccatgagtgataacactgcggccaacttacttctgacaacgatcggaggaccgaaggagctaaccgcttttttgcacaacatgggggatcatgtaactcgccttgatcgttgggaaccggagctgaatgaagccataccaaacgacgagcgtgacaccacgatgcctgtagcaatggcaacaacgttgcgcaaactattaactggcgaactacttactctagcttcccggcaacaattaatagactggatggaggcggataaagttgcaggaccacttctgcgctcggcccttccggctggctggtttattgctgataaatctggagccggtgagcgtgggtctcgcggtatcattgcagcactggggccagatggtaagccctcccgtatcgtagttatctacacgacggggagtcaggcaactatggatgaacgaaatagacagatcgctgagataggtgcctcactgattaagcattggtaactgtcagaccaagtttactcatatatactttagattgatttaaaacttcatttttaatttaaaaggatctaggtgaagatcctttttgataatctcatgaccaaaatcccttaacgtgagttttcgttccactgagcgtcagaccccgtagaaaagatcaaaggatcttcttgagatcctttttttctgcgcgtaatctgctgcttgcaaacaaaaaaaccaccgctaccagcggtggtttgtttgccggatcaagagctaccaactctttttccgaaggtaactggcttcagcagagcgcagataccaaatactgttcttctagtgtagccgtagttaggccaccacttcaagaactctgtagcaccgcctacatacctcgctctgctaatcctgttaccagtggctgctgccagtggcgataagtcgtgtcttaccgggttggactcaagacgatagttaccggataaggcgcagcggtcgggctgaacggggggttcgtgcacacagcccagcttggagcgaacgacctacaccgaactgagatacctacagcgtgagctatgagaaagcgccacgcttcccgaagggagaaaggcggacaggtatccggtaagcggcagggtcggaacaggagagcgcacgagggagcttccagggggaaacgcctggtatctttatagtcctgtcgggtttcgccacctctgacttgagcgtcgatttttgtgatgctcgtcaggggggcggagcctatggaaaaacgccagcaacgcggcctttttacggttcctggccttttgctggccttttgctcacatgttctttcctgcgttatcccctgattctgtggataaccgtattaccgcctttgagtgagctgataccgctcgccgcagccgaacgaccgagcgcagcgagtcagtgagcgaggaagcggaagagcgcccaatacgcaaaccgcctctccccgcgcgttggccgattcattaatgcagctggcacgacaggtttcccgactggaaagcgggcagtgagcgcaacgcaattaatgtgagttagctcactcattaggcaccccaggctttacactttatgcttccggctcgtatgttgtgtggaattgtgagcggataacaatttcacacaggaaacagctatgaccatgattacgcctctagaaagctttaatacgactcactataaggactcactatttgttttcgcgcccagttgcaaaaagtgtcgacatttgcttctgacacaactgtgttcactagcaacctcaaacagacaccgccaccatgtccaagggagaggagctgttcaccggagtggtgccaatcctggtggagctggacggcgatgtgaacggccacaagttttctgtgcgcggagagggagagggcgacgcaaccatcggcaagctgacactgaagttcatctgcaccacaggcaagctgcccgtgccttggccaaccctggtgaccacactgacatacggcgtgcagtgtttctctaggtatccagaccacatgaagagacacgatttctttaagagcgccatgccagagggatacgtgcaggagcggaccatctccttcaaggacgatggcaagtataagacccgcgccgtggtgaagtttgagggcgatacactggtgaacaggatcgagctgaagggcaccgacttcaaggaggatggcaatatcctgggccacaagctggagtacaactttaatagccacaacgtgtatatcacagccgacaagcagaagaacggcatcaaggccaacttcaccgtgaggcacaatgtggaggacggctccgtgcagctggccgatcactaccagcagaacacacctatcggcgacggacccgtgctgctgcctgataatcactatctgtccacccagacagtgctgtctaaggacccaaacgagaagttggatccaggtggaggtggaagcggtatgaacaattcccagggaagagtgaccttcgaggacgtgaccgtgaacttcacccaaggcgagtggcagagactgaaccccgagcagagaaacctgtaccgggacgtgatgctggaaaactacagcaacctggtgtccgtcggccagggcgagacaacaaagcctgacgtgatcctgcggctggaacagggcaaagagccttggctggaagaggaagaggtgctcggatctggcagagccgagaagaatggcgatatcggcggacagatctggaagccaaaggatgtgaaagagagtctcggaagcggagctactaacttcagcctgctgaagcaggctggagacgtggaggagaaccctggacctatgcctgctgctaagagagtgaaactggatggatccaaccatgaccaggaatttgaccccccaaaggtttacccacctgtgccagctgagaagaggaagcccatccgcgtgctgtctctctttgatgggattgctacagggctcctggtgctgaaggacctgggcatccaagtggaccgctacattgcctccgaggtgtgtgaggactccatcacggtgggcatggtgcggcaccagggaaagatcatgtacgtcggggacgtccgcagcgtcacacagaagcatatccaggagtggggcccattcgacctggtgattggaggcagtccctgcaatgacctctccattgtcaaccctgcccgcaagggactttatgagggtactggccgcctcttctttgagttctaccgcctcctgcatgatgcgcggcccaaggagggagatgatcgccccttcttctggctctttgagaatgtggtggccatgggcgttagtgacaagagggacatctcgcgatttcttgagtctaaccccgtgatgattgacgccaaagaagtgtctgctgcacacagggcccgttacttctggggtaaccttcctggcatgaacaggcctttggcatccactgtgaatgataagctggagctgcaagagtgtctggagcacggcagaatagccaagttcagcaaagtgaggaccattaccaccaggtcaaactctataaagcagggcaaagaccagcatttccccgtgttcatgaacgagaaggaggacatcctgtggtgcactgaaatggaaagggtgtttggcttccccgtccactacacagacgtctccaacatgagccgcttggcgaggcagagactgctgggccgatcgtggagcgtgccggtcatccgccacctcttcgctccgctgaaggaatattttgcttgtgtgtctagcggcaatagtaacgctaacagccgcgggccgagcttcagcagcggcctggtgccgttaagcttgcgcggcagccatatgttcgaaaccgtgcctgtgtggaggagacagccagtccgggtgctgtccctttttgaagacatcaagaaagagctgacgagtttgggctttttggaaagtggttctgacccgggacaactgaagcatgtggttgatgtcacagacacagtgaggaaggatgtggaggagtggggacccttcgatcttgtgtacggcgccacacctcccctgggccacacctgtgaccgtcctcccagctggtacctgttccagttccaccggctcctgcagtacgcacggcccaagccaggcagccccaggcccttcttctggatgttcgtggacaatctggtgctgaacaaggaagacctggacgtcgcatctcgcttcctggagatggagccagtcaccatcccagatgtccacggcggatccttgcagaatgctgtccgcgtgtggagcaacatcccagccataaggagcagcaggcactgggctctggtttcggaagaagaattgtccctgctggcccagaacaagcagagctcgaagctcgcggccaagtggcccaccaagctggtgaagaactgctttctccccctaagagaatatttcaagtatttttcaggagggccgagctctggcgcacccccaccaagtggagggtctcctgccgggtccccaacatctactgaagaaggcaccagcgaatccgcaacgcccgagtcaggccctggtacctccacagaaccatctgaaggtagtgcgcctggttccccagctggaagccctacttccaccgaagaaggcacgtcaaccgaaccaagtgaaggatctgcccctgggaccagcactgaaccatctgagccaaaaaagaagagaaaggtaatggacaagaagtacagcatcggcctggccatcggcaccaactctgtgggctgggccgtgatcaccgacgagtacaaggtgcccagcaagaaattcaaggtgctgggcaacaccgaccggcacagcatcaagaagaacctgatcggcgccctgctgttcgacagcggagaaacagccgaggccacccggctgaagagaaccgccagaagaagatacaccagacggaagaaccggatctgctatctgcaagagatcttcagcaacgagatggccaaggtggacgacagcttcttccacagactggaagagtccttcctggtggaagaggataagaagcacgagcggcaccccatcttcggcaacatcgtggacgaggtggcctaccacgagaagtaccccaccatctaccacctgagaaagaaactggtggacagcaccgacaaggccgacctgcggctgatctatctggccctggcccacatgatcaagttccggggccacttcctgatcgagggcgacctgaaccccgacaacagcgacgtggacaagctgttcatccagctggtgcagacctacaaccagctgttcgaggaaaaccccatcaacgccagcggcgtggacgccaaggccatcctgtctgccagactgagcaagagcagacggctggaaaatctgatcgcccagctgcccggcgagaagaagaatggcctgttcggcaacctgattgccctgagcctgggcctgacccccaacttcaagagcaacttcgacctggccgaggatgccaaactgcagctgagcaaggacacctacgacgacgacctggacaacctgctggcccagatcggcgaccagtacgccgacctgtttctggccgccaagaacctgtccgacgccatcctgctgagcgacatcctgagagtgaacaccgagatcaccaaggcccccctgagcgcctctatgatcaagagatacgacgagcaccaccaggacctgaccctgctgaaagctctcgtgcggcagcagctgcctgagaagtacaaagagattttcttcgaccagagcaagaacggctacgccggctacatcgatggcggagccagccaggaagagttctacaagttcatcaagcccatcctggaaaagatggacggcaccgaggaactgctcgtgaagctgaacagagaggacctgctgcggaagcagcggaccttcgacaacggcagcatcccccaccagatccacctgggagagctgcacgccattctgcggcggcaggaagatttttacccattcctgaaggacaaccgggaaaagatcgagaagatcctgaccttccgcatcccctactacgtgggccctctggccaggggaaacagcagattcgcctggatgaccagaaagagcgaggaaaccatcaccccctggaacttcgaggaagtggtggacaagggcgccagcgcccagagcttcatcgagcggatgaccaacttcgataagaacctgcccaacgagaaggtgctgcccaagcacagcctgctgtacgagtacttcaccgtgtacaacgagctgaccaaagtgaaatacgtgaccgagggaatgagaaagcccgccttcctgagcggcgagcagaaaaaagccatcgtggacctgctgttcaagaccaaccggaaagtgaccgtgaagcagctgaaagaggactacttcaagaaaatcgagtgcttcgactccgtggaaatctccggcgtggaagatcggttcaacgcctccctgggcacataccacgatctgctgaaaattatcaaggacaaggacttcctggacaatgaggaaaacgaggacattctggaagatatcgtgctgaccctgacactgtttgaggacagagagatgatcgaggaacggctgaaaacctatgcccacctgttcgacgacaaagtgatgaagcagctgaagcggcggagatacaccggctggggcaggctgagccggaagctgatcaacggcatccgggacaagcagtccggcaagacaatcctggatttcctgaagtccgacggcttcgccaacagaaacttcatgcagctgatccacgacgacagcctgacctttaaagaggacatccagaaagcccaggtgtccggccagggcgatagcctgcacgagcacattgccaatctggccggcagccccgccattaagaagggcatcctgcagacagtgaaggtggtggacgagctcgtgaaagtgatgggccggcacaagcccgagaacatcgtgatcgaaatggccagagagaaccagaccacccagaagggacagaagaacagccgcgagagaatgaagcggatcgaagagggcatcaaagagctgggcagccagatcctgaaagaacaccccgtggaaaacacccagctgcagaacgagaagctgtacctgtactacctgcagaatgggcgggatatgtacgtggaccaggaactggacatcaaccggctgtccgactacgatgtggacgctatcgtgcctcagagctttctgaaggacgactccatcgataacaaagtgctgactcggagcgacaagaaccggggcaagagcgacaacgtgccctccgaagaggtcgtgaagaagatgaagaactactggcgccagctgctgaatgccaagctgattacccagaggaagttcgacaatctgaccaaggccgagagaggcggcctgagcgaactggataaggccggcttcatcaagagacagctggtggaaacccggcagatcacaaagcacgtggcacagatcctggactcccggatgaacactaagtacgacgagaacgacaaactgatccgggaagtgaaagtgatcaccctgaagtccaagctggtgtccgatttccggaaggatttccagttttacaaagtgcgcgagatcaacaactaccaccacgcccacgacgcctacctgaacgccgtcgtgggaaccgccctgatcaaaaagtaccctaagctggaaagcgagttcgtgtacggcgactacaaggtgtacgacgtgcggaagatgatcgccaagagcgagcaggaaatcggcaaggctaccgccaagtacttcttctacagcaacatcatgaactttttcaagaccgagattaccctggccaacggcgagatccggaagcggcctctgatcgagacaaacggcgaaacaggcgagatcgtgtgggataagggccgggactttgccaccgtgcggaaagtgctgtctatgccccaagtgaatatcgtgaaaaagaccgaggtgcagacaggcggcttcagcaaagagtctatcctgcccaagaggaacagcgacaagctgatcgccagaaagaaggactgggaccctaagaagtacggcggcttcgacagccccaccgtggcctattctgtgctggtggtggccaaagtggaaaagggcaagtccaagaaactgaagagtgtgaaagagctgctggggatcaccatcatggaaagaagcagcttcgagaagaatcccatcgactttctggaagccaagggctacaaagaagtgaaaaaggacctgatcatcaagctgcctaagtactccctgttcgagctggaaaacggccggaagagaatgctggcctctgccggcgaactgcagaagggaaacgaactggccctgccctccaaatatgtgaacttcctgtacctggccagccactatgagaagctgaagggctcccccgaggataatgagcagaaacagctgtttgtggaacagcacaaacactacctggacgagatcatcgagcagatcagcgagttctccaagagagtgatcctggccgacgctaatctggacaaggtgctgagcgcctacaacaagcacagagacaagcctatcagagagcaggccgagaatatcatccacctgtttaccctgaccaatctgggagcccctgccgccttcaagtactttgacaccaccatcgaccggaagaggtacaccagcaccaaagaggtgctggacgccaccctgatccaccagagcatcaccggcctgtacgagacacggatcgacctgtctcagctgggaggcgacgcctatccctatgacgtgcccgattatgccagcctgggcagcggctcccccaagaaaaaacgcaaggtggaagatcctaagaaaaagcggaaagtggacggcagcggcagcgagacccccggtaccagcgagagcgccacccccgagagcggtagtgggagcaacggcagcagcggatccatgcgtgaccacatggtccttcatgagtatgtaaatgctgctgggattacagcggcc

SEQ ID NO: 234 - DNA, 11967 bp, synthetic construct
  misc_feature 1..11967: note = DNA of V40_GFP1-10-HDAC1-2a-D3a-hD3L-dCas9-1xGFP11
  source 1..11967: mol_type = other DNA
gcaaggtcaggctccggccagcggggaagcaagcgcaccgccgatggttccgagttcgaaagccccaaaaaaaagcgcaaggtctgagatcccaagcacgcagcaatgcagctcaaaacgcttagcctagccacacccccacgggaaacagcagtgattaacctttagcaataaacgaaagtttaactaagctatactaaccccagggttggtcaatttcgtgccagccacaccctggtactgcatgcacgcaatgctagctgcccctttcccgtcctgggcaccccgagtctcccccgaccccgggtcccaggtatgctcccacctccacctgccccactcaccacctctgctagttccagacacctccgagacgaggaaaaaaaaaaaaaaaaaaaaaaaaaaaaaaaaaaaaaaaaaaaaaaaaaaaaaaaaaaaaaaaaaaaaaaaaaaaaaaaaaaaaaaaaaaaaaaaaaaaaaaaaaaaaaaaaaaaaaaaaaaaaaaaaaaaaaaaaaaaaaaaaaaaaaaaaaaaaaaaaaaaaaaaaaaaaaaaaaaaaaaaaaaaaaaaaaaaaaaaaaaaaaaaaaaaaaaaaaaaaaaaaaaaaaaaaaaaaaaaaaaaaaaaaaaaaaaaaaaaaaaaaaaaaaaaaaaaaaaaaaaaaaaaaaaaaaaaaaaaaaaaaaaaaaaaaaaaaaaaaaaaaaaaaaaaaaaaaaaaaaaaaaaaaaaaaaaaaaaaaaaaaaaaaaaaaaaaaaaaaaaaaaaaaaaaaaaccgtcttcaagctttctagaaattcactggccgtcgttttacaacgtcgtgactgggaaaaccctggcgttacccaacttaatcgccttgcagcacatccccctttcgccagctggcgtaatagcgaagaggcccgcaccgatcgcccttcccaacagttgcgcagcctgaatggcgaatggcgcctgatgcggtattttctccttacgcatctgtgcggtatttcacaccgcatatggtgcactctcagtacaatctgctctgatgccgcatagttaagccagccccgacacccgccaacacccgctgacgcgccctgacgggcttgtctgctcccggcatccgcttacagacaagctgtgaccgtctccgggagctgcatgtgtcagaggttttcaccgtcatcaccgaaacgcgcgagacgaaagggcctcgtgatacgcctatttttataggttaatgtcatgataataatggtttcttagacgtcaggtggcacttttcggggaaatgtgcgcggaacccctatttgtttatttttctaaatacattcaaatatgtatccgctcatgagacaataaccctgataaatgcttcaataatattgaaaaaggaagagtatgagtattcaacatttccgtgtcgcccttattcccttttttgcggcattttgccttcctgtttttgctcacccagaaacgctggtgaaagtaaaagatgctgaagatcagttgggtgcacgagtgggttacatcgaactggatctcaacagcggtaagatccttgagagttttcgccccgaagaacgttttccaatgatgagcacttttaaagttctgctatgtggcgcggtattatcccgtattgacgccgggcaagagcaactcggtcgccgcatacactattctcagaatgacttggttgagtactcaccagtcacagaaaagcatcttacggatggcatgacagtaagagaattatgcagtgctgccataaccatgagtgataacactgcggccaacttacttctgacaacgatcggaggaccgaaggagctaaccgcttttttgcacaacatgggggatcatgtaactcgccttgatcgttgggaaccggagctgaatgaagccataccaaacgacgagcgtgacaccacgatgcctgtagcaatggcaacaacgttgcgcaaactattaactggcgaactacttactctagcttcccggcaacaattaatagactggatggaggcggataaagttgcaggaccacttctgcgctcggcccttccggctggctggtttattgctgataaatctggagccggtgagcgtgggtctcgcggtatcattgcagcactggggccagatggtaagccctcccgtatcgtagttatctacacgacggggagtcaggcaactatggatgaacgaaatagacagatcgctgagataggtgcctcactgattaagcattggtaactgtcagaccaagtttactcatatatactttagattgatttaaaacttcatttttaatttaaaaggatctaggtgaagatcctttttgataatctcatgaccaaaatcccttaacgtgagttttcgttccactgagcgtcagaccccgtagaaaagatcaaaggatcttcttgagatcctttttttctgcgcgtaatctgctgcttgcaaacaaaaaaaccaccgctaccagcggtggtttgtttgccggatcaagagctaccaactctttttccgaaggtaactggcttcagcagagcgcagataccaaatactgttcttctagtgtagccgtagttaggccaccacttcaagaactctgtagcaccgcctacatacctcgctctgctaatcctgttaccagtggctgctgccagtggcgataagtcgtgtcttaccgggttggactcaagacgatagttaccggataaggcgcagcggtcgggctgaacggggggttcgtgcacacagcccagcttggagcgaacgacctacaccgaactgagatacctacagcgtgagctatgagaaagcgccacgcttcccgaagggagaaaggcggacaggtatccggtaagcggcagggtcggaacaggagagcgcacgagggagcttccagggggaaacgcctggtatctttatagtcctgtcgggtttcgccacctctgacttgagcgtcgatttttgtgatgctcgtcaggggggcggagcctatggaaaaacgccagcaacgcggcctttttacggttcctggccttttgctggccttttgctcacatgttctttcctgcgttatcccctgattctgtggataaccgtattaccgcctttgagtgagctgataccgctcgccgcagccgaacgaccgagcgcagcgagtcagtgagcgaggaagcggaagagcgcccaatacgcaaaccgcctctccccgcgcgttggccgattcattaatgcagctggcacgacaggtttcccgactggaaagcgggcagtgagcgcaacgcaattaatgtgagttagctcactcattaggcaccccaggctttacactttatgcttccggctcgtatgttgtgtggaattgtgagcggataacaatttcacacaggaaacagctatgaccatgattacgcctctagaaagctttaatacgactcactataaggactcactatttgttttcgcgcccagttgcaaaaagtgtcgacatttgcttctgacacaactgtgttcactagcaacctcaaacagacaccgccaccatgtccaagggagaggagctgttcaccggagtggtgccaatcctggtggagctggacggcgatgtgaacggccacaagttttctgtgcgcggagagggagagggcgacgcaaccatcggcaagctgacactgaagttcatctgcaccacaggcaagctgcccgtgccttggccaaccctggtgaccacactgacatacggcgtgcagtgtttctctaggtatccagaccacatgaagagacacgatttctttaagagcgccatgccagagggatacgtgcaggagcggaccatctccttcaaggacgatggcaagtataagacccgcgccgtggtgaagtttgagggcgatacactggtgaacaggatcgagctgaagggcaccgacttcaaggaggatggcaatatcctgggccacaagctggagtacaactttaatagccacaacgtgtatatcacagccgacaagcagaagaacggcatcaaggccaacttcaccgtgaggcacaatgtggaggacggctccgtgcagctggccgatcactaccagcagaacacacctatcggcgacggacccgtgctgctgcctgataatcactatctgtccacccagacagtgctgtctaaggacccaaacgagaagttggatccaggtggaggtggaagcggtatggcgcagacgcagggcacccggaggaaagtctgttactactacgacggggatgttggaaattactattatggacaaggccacccaatgaagcctcaccgaatccgcatgactcataatttgctgctcaactatggtctctaccgaaaaatggaaatctatcgccctcacaaagccaatgctgaggagatgaccaagtaccacagcgatgactacattaaattcttgcgctccatccgtccagataacatgtcggagtacagcaagcagatgcagagattcaacgttggtgaggactgtccagtattcgatggcctgtttgagttctgtcagttgtctactggtggttctgtggcaagtgctgtgaaacttaataagcagcagacggacatcgctgtgaattgggctgggggcctgcaccatgcaaagaagtccgaggcatctggcttctgttacgtcaatgatatcgtcttggccatcctggaactgctaaagtatcaccagagggtgctgtacattgacattgatattcaccatggtgacggcgtggaagaggccttctacaccacggaccgggtcatgactgtgtcctttcataagtatggagagtacttcccaggaactggggacctacgggatatcggggctggcaaaggcaagtattatgctgttaactacccgctccgagacgggattgatgacgagtcctatgaggccattttcaagccggtcatgtccaaagtaatggagatgttccagcctagtgcggtggtcttacagtgtggctcagactccctatctggggatcggttaggttgcttcaatctaactatcaaaggacacgccaagtgtgtggaatttgtcaagagctttaacctgcctatgctgatgctgggaggcggtggttacaccattcgtaacgttgcccggtgctggacatatgagacagctgtggccctggatacggagatccctaatgagcttccatacaatgactactttgaatactttggaccagatttcaagctccacatcagtccttccaatatgactaaccagaacacgaatgagtacctggagaagatcaaacagcgactgtttgagaaccttagaatgctgccgcacgcacctggggtccaaatgcaggcgattcctgaggacgccatccctgaggagagtggcgatgaggacgaagacgaccctgacaagcgcatctcgatctgctcctctgacaaacgaattgcctgtgaggaagagttctccgattctgaagaggagggagaggggggccgcaagaactcttccaacttcaaaaaagccaagagagtcaaaacagaggatgaaaaagagaaagacccagaggagaagaaagaagtcaccgaagaggagaaaaccaaggaggagaagccagaagccaaaggggtcaaggaggaggtcaagttggccggaagcggagctactaacttcagcctgctgaagcaggctggagacgtggaggagaaccctggacctatgcctgctgctaagagagtgaaactggatggatccaaccatgaccaggaatttgaccccccaaaggtttacccacctgtgccagctgagaagaggaagcccatccgcgtgctgtctctctttgatgggattgctacagggctcctggtgctgaaggacctgggcatccaagtggaccgctacattgcctccgaggtgtgtgaggactccatcacggtgggcatggtgcggcaccagggaaagatcatgtacgtcggggacgtccgcagcgtcacacagaagcatatccaggagtggggcccattcgacctggtgattggaggcagtccctgcaatgacctctccattgtcaaccctgcccgcaagggactttatgagggtactggccgcctcttctttgagttctaccgcctcctgcatgatgcgcggcccaaggagggagatgatcgccccttcttctggctctttgagaatgtggtggccatgggcgttagtgacaagagggacatctcgcgatttcttgagtctaaccccgtgatgattgacgccaaagaagtgtctgctgcacacagggcccgttacttctggggtaaccttcctggcatgaacaggcctttggcatccactgtgaatgataagctggagctgcaagagtgtctggagcacggcagaatagccaagttcagcaaagtgaggaccattaccaccaggtcaaactctataaagcagggcaaagaccagcatttccccgtgttcatgaacgagaaggaggacatcctgtggtgcactgaaatggaaagggtgtttggcttccccgtccactacacagacgtctccaacatgagccgcttggcgaggcagagactgctgggccgatcgtggagcgtgccggtcatccgccacctcttcgctccgctgaaggaatattttgcttgtgtgtctagcggcaatagtaacgctaacagccgcgggccgagcttcagcagcggcctggtgccgttaagcttgcgcggcagccatatgttcgaaaccgtgcctgtgtggaggagacagccagtccgggtgctgtccctttttgaagacatcaagaaagagctgacgagtttgggctttttggaaagtggttctgacccgggacaactgaagcatgtggttgatgtcacagacacagtgaggaaggatgtggaggagtggggacccttcgatcttgtgtacggcgccacacctcccctgggccacacctgtgaccgtcctcccagctggtacctgttccagttccaccggctcctgcagtacgcacggcccaagccaggcagccccaggcccttcttctggatgttcgtggacaatctggtgctgaacaaggaagacctggacgtcgcatctcgcttcctggagatggagccagtcaccatcccagatgtccacggcggatccttgcagaatgctgtccgcgtgtggagcaacatcccagccataaggagcagcaggcactgggctctggtttcggaagaagaattgtccctgctggcccagaacaagcagagctcgaagctcgcggccaagtggcccaccaagctggtgaagaactgctttctccccctaagagaatatttcaagtatttttcaggagggccgagctctggcgcacccccaccaagtggagggtctcctgccgggtccccaacatctactgaagaaggcaccagcgaatccgcaacgcccgagtcaggccctggtacctccacagaaccatctgaaggtagtgcgcctggttccccagctggaagccctacttccaccgaagaaggcacgtcaaccgaaccaagtgaaggatctgcccctgggaccagcactgaaccatctgagccaaaaaagaagagaaaggtaatggacaagaagtacagcatcggcctggccatcggcaccaactctgtgggctgggccgtgatcaccgacgagtacaaggtgcccagcaagaaattcaaggtgctgggcaacaccgaccggcacagcatcaagaagaacctgatcggcgccctgctgttcgacagcggagaaacagccgaggccacccggctgaagagaaccgccagaagaagatacaccagacggaagaaccggatctgctatctgcaagagatcttcagcaacgagatggccaaggtggacgacagcttcttccacagactggaagagtccttcctggtggaagaggataagaagcacgagcggcaccccatcttcggcaacatcgtggacgaggtggcctaccacgagaagtaccccaccatctaccacctgagaaagaaactggtggacagcaccgacaaggccgacctgcggctgatctatctggccctggcccacatgatcaagttccggggccacttcctgatcgagggcgacctgaaccccgacaacagcgacgtggacaagctgttcatccagctggtgcagacctacaaccagctgttcgaggaaaaccccatcaacgccagcggcgtggacgccaaggccatcctgtctgccagactgagcaagagcagacggctggaaaatctgatcgcccagctgcccggcgagaagaagaatggcctgttcggcaacctgattgccctgagcctgggcctgacccccaacttcaagagcaacttcgacctggccgaggatgccaaactgcagctgagcaaggacacctacgacgacgacctggacaacctgctggcccagatcggcgaccagtacgccgacctgtttctggccgccaagaacctgtccgacgccatcctgctgagcgacatcctgagagtgaacaccgagatcaccaaggcccccctgagcgcctctatgatcaagagatacgacgagcaccaccaggacctgaccctgctgaaagctctcgtgcggcagcagctgcctgagaagtacaaagagattttcttcgaccagagcaagaacggctacgccggctacatcgatggcggagccagccaggaagagttctacaagttcatcaagcccatcctggaaaagatggacggcaccgaggaactgctcgtgaagctgaacagagaggacctgctgcggaagcagcggaccttcgacaacggcagcatcccccaccagatccacctgggagagctgcacgccattctgcggcggcaggaagatttttacccattcctgaaggacaaccgggaaaagatcgagaagatcctgaccttccgcatcccctactacgtgggccctctggccaggggaaacagcagattcgcctggatgaccagaaagagcgaggaaaccatcaccccctggaacttcgaggaagtggtggacaagggcgccagcgcccagagcttcatcgagcggatgaccaacttcgataagaacctgcccaacgagaaggtgctgcccaagcacagcctgctgtacgagtacttcaccgtgtacaacgagctgaccaaagtgaaatacgtgaccgagggaatgagaaagcccgccttcctgagcggcgagcagaaaaaagccatcgtggacctgctgttcaagaccaaccggaaagtgaccgtgaagcagctgaaagaggactacttcaagaaaatcgagtgcttcgactccgtggaaatctccggcgtggaagatcggttcaacgcctccctgggcacataccacgatctgctgaaaattatcaaggacaaggacttcctggacaatgaggaaaacgaggacattctggaagatatcgtgctgaccctgacactgtttgaggacagagagatgatcgaggaacggctgaaaacctatgcccacctgttcgacgacaaagtgatgaagcagctgaagcggcggagatacaccggctggggcaggctgagccggaagctgatcaacggcatccgggacaagcagtccggcaagacaatcctggatttcctgaagtccgacggcttcgccaacagaaacttcatgcagctgatccacgacgacagcctgacctttaaagaggacatccagaaagcccaggtgtccggccagggcgatagcctgcacgagcacattgccaatctggccggcagccccgccattaagaagggcatcctgcagacagtgaaggtggtggacgagctcgtgaaagtgatgggccggcacaagcccgagaacatcgtgatcgaaatggccagagagaaccagaccacccagaagggacagaagaacagccgcgagagaatgaagcggatcgaagagggcatcaaagagctgggcagccagatcctgaaagaacaccccgtggaaaacacccagctgcagaacgagaagctgtacctgtactacctgcagaatgggcgggatatgtacgtggaccaggaactggacatcaaccggctgtccgactacgatgtggacgctatcgtgcctcagagctttctgaaggacgactccatcgataacaaagtgctgactcggagcgacaagaaccggggcaagagcgacaacgtgccctccgaagaggtcgtgaagaagatgaagaactactggcgccagctgctgaatgccaagctgattacccagaggaagttcgacaatctgaccaaggccgagagaggcggcctgagcgaactggataaggccggcttcatcaagagacagctggtggaaacccggcagatcacaaagcacgtggcacagatcctggactcccggatgaacactaagtacgacgagaacgacaaactgatccgggaagtgaaagtgatcaccctgaagtccaagctggtgtccgatttccggaaggatttccagttttacaaagtgcgcgagatcaacaactaccaccacgcccacgacgcctacctgaacgccgtcgtgggaaccgccctgatcaaaaagtaccctaagctggaaagcgagttcgtgtacggcgactacaaggtgtacgacgtgcggaagatgatcgccaagagcgagcaggaaatcggcaaggctaccgccaagtacttcttctacagcaacatcatgaactttttcaagaccgagattaccctggccaacggcgagatccggaagcggcctctgatcgagacaaacggcgaaacaggcgagatcgtgtgggataagggccgggactttgccaccgtgcggaaagtgctgtctatgccccaagtgaatatcgtgaaaaagaccgaggtgcagacaggcggcttcagcaaagagtctatcctgcccaagaggaacagcgacaagctgatcgccagaaagaaggactgggaccctaagaagtacggcggcttcgacagccccaccgtggcctattctgtgctggtggtggccaaagtggaaaagggcaagtccaagaaactgaagagtgtgaaagagctgctggggatcaccatcatggaaagaagcagcttcgagaagaatcccatcgactttctggaagccaagggctacaaagaagtgaaaaaggacctgatcatcaagctgcctaagtactccctgttcgagctggaaaacggccggaagagaatgctggcctctgccggcgaactgcagaagggaaacgaactggccctgccctccaaatatgtgaacttcctgtacctggccagccactatgagaagctgaagggctcccccgaggataatgagcagaaacagctgtttgtggaacagcacaaacactacctggacgagatcatcgagcagatcagcgagttctccaagagagtgatcctggccgacgctaatctggacaaggtgctgagcgcctacaacaagcacagagacaagcctatcagagagcaggccgagaatatcatccacctgtttaccctgaccaatctgggagcccctgccgccttcaagtactttgacaccaccatcgaccggaagaggtacaccagcaccaaagaggtgctggacgccaccctgatccaccagagcatcaccggcctgtacgagacacggatcgacctgtctcagctgggaggcgacgcctatccctatgacgtgcccgattatgccagcctgggcagcggctcccccaagaaaaaacgcaaggtggaagatcctaagaaaaagcggaaagtggacggcagcggcagcgagacccccggtaccagcgagagcgccacccccgagagcggtagtgggagcaacggcagcagcggatccatgcgtgaccacatggtccttcatgagtatgtaaatgctgctgggattacagcggcc

SEQ ID NO: 235 - DNA, 10401 bp, synthetic construct
  misc_feature 1..10401: note = DNA of V41_GFP1-10-ZIM3-2a-D3a-hD3L-dCas12a-1xGFP11
  source 1..10401: mol_type = other DNA
gcaaggtcaggctccggccagcggggaagcaagcgcaccgccgatggttccgagttcgaaagccccaaaaaaaagcgcaaggtctgagatcccaagcacgcagcaatgcagctcaaaacgcttagcctagccacacccccacgggaaacagcagtgattaacctttagcaataaacgaaagtttaactaagctatactaaccccagggttggtcaatttcgtgccagccacaccctggtactgcatgcacgcaatgctagctgcccctttcccgtcctgggcaccccgagtctcccccgaccccgggtcccaggtatgctcccacctccacctgccccactcaccacctctgctagttccagacacctccgagacgaggaaaaaaaaaaaaaaaaaaaaaaaaaaaaaaaaaaaaaaaaaaaaaaaaaaaaaaaaaaaaaaaaaaaaaaaaaaaaaaaaaaaaaaaaaaaaaaaaaaaaaaaaaaaaaaaaaaaaaaaaaaaaaaaaaaaaaaaaaaaaaaaaaaaaaaaaaaaaaaaaaaaaaaaaaaaaaaaaaaaaaaaaaaaaaaaaaaaaaaaaaaaaaaaaaaaaaaaaaaaaaaaaaaaaaaaaaaaaaaaaaaaaaaaaaaaaaaaaaaaaaaaaaaaaaaaaaaaaaaaaaaaaaaaaaaaaaaaaaaaaaaaaaaaaaaaaaaaaaaaaaaaaaaaaaaaaaaaaaaaaaaaaaaaaaaaaaaaaaaaaaaaaaaaaaaaaaaaaaaaaaaaaaaaaaaaaaaccgtcttcaagctttctagaaattcactggccgtcgttttacaacgtcgtgactgggaaaaccctggcgttacccaacttaatcgccttgcagcacatccccctttcgccagctggcgtaatagcgaagaggcccgcaccgatcgcccttcccaacagttgcgcagcctgaatggcgaatggcgcctgatgcggtattttctccttacgcatctgtgcggtatttcacaccgcatatggtgcactctcagtacaatctgctctgatgccgcatagttaagccagccccgacacccgccaacacccgctgacgcgccctgacgggcttgtctgctcccggcatccgcttacagacaagctgtgaccgtctccgggagctgcatgtgtcagaggttttcaccgtcatcaccgaaacgcgcgagacgaaagggcctcgtgatacgcctatttttataggttaatgtcatgataataatggtttcttagacgtcaggtggcacttttcggggaaatgtgcgcggaacccctatttgtttatttttctaaatacattcaaatatgtatccgctcatgagacaataaccctgataaatgcttcaataatattgaaaaaggaagagtatgagtattcaacatttccgtgtcgcccttattcccttttttgcggcattttgccttcctgtttttgctcacccagaaacgctggtgaaagtaaaagatgctgaagatcagttgggtgcacgagtgggttacatcgaactggatctcaacagcggtaagatccttgagagttttcgccccgaagaacgttttccaatgatgagcacttttaaagttctgctatgtggcgcggtattatcccgtattgacgccgggcaagagcaactcggtcgccgcatacactattctcagaatgacttggttgagtactcaccagtcacagaaaagcatcttacggatggcatgacagtaagagaattatgcagtgctgccataaccatgagtgataacactgcggccaacttacttctgacaacgatcggaggaccgaaggagctaaccgcttttttgcacaacatgggggatcatgtaactcgccttgatcgttgggaaccggagctgaatgaagccataccaaacgacgagcgtgacaccacgatgcctgtagcaatggcaacaacgttgcgcaaactattaactggcgaactacttactctagcttcccggcaacaattaatagactggatggaggcggataaagttgcaggaccacttctgcgctcggcccttccggctggctggtttattgctgataaatctggagccggtgagcgtgggtctcgcggtatcattgcagcactggggccagatggtaagccctcccgtatcgtagttatctacacgacggggagtcaggcaactatggatgaacgaaatagacagatcgctgagataggtgcctcactgattaagcattggtaactgtcagaccaagtttactcatatatactttagattgatttaaaacttcatttttaatttaaaaggatctaggtgaagatcctttttgataatctcatgaccaaaatcccttaacgtgagttttcgttccactgagcgtcagaccccgtagaaaagatcaaaggatcttcttgagatcctttttttctgcgcgtaatctgctgcttgcaaacaaaaaaaccaccgctaccagcggtggtttgtttgccggatcaagagctaccaactctttttccgaaggtaactggcttcagcagagcgcagataccaaatactgttcttctagtgtagccgtagttaggccaccacttcaagaactctgtagcaccgcctacatacctcgctctgctaatcctgttaccagtggctgctgccagtggcgataagtcgtgtcttaccgggttggactcaagacgatagttaccggataaggcgcagcggtcgggctgaacggggggttcgtgcacacagcccagcttggagcgaacgacctacaccgaactgagatacctacagcgtgagctatgagaaagcgccacgcttcccgaagggagaaaggcggacaggtatccggtaagcggcagggtcggaacaggagagcgcacgagggagcttccagggggaaacgcctggtatctttatagtcctgtcgggtttcgccacctctgacttgagcgtcgatttttgtgatgctcgtcaggggggcggagcctatggaaaaacgccagcaacgcggcctttttacggttcctggccttttgctggccttttgctcacatgttctttcctgcgttatcccctgattctgtggataaccgtattaccgcctttgagtgagctgataccgctcgccgcagccgaacgaccgagcgcagcgagtcagtgagcgaggaagcggaagagcgcccaatacgcaaaccgcctctccccgcgcgttggccgattcattaatgcagctggcacgacaggtttcccgactggaaagcgggcagtgagcgcaacgcaattaatgtgagttagctcactcattaggcaccccaggctttacactttatgcttccggctcgtatgttgtgtggaattgtgagcggataacaatttcacacaggaaacagctatgaccatgattacgcctctagaaagctttaatacgactcactataaggactcactatttgttttcgcgcccagttgcaaaaagtgtcgacatttgcttctgacacaactgtgttcactagcaacctcaaacagacaccgccaccatgtccaagggagaggagctgttcaccggagtggtgccaatcctggtggagctggacggcgatgtgaacggccacaagttttctgtgcgcggagagggagagggcgacgcaaccatcggcaagctgacactgaagttcatctgcaccacaggcaagctgcccgtgccttggccaaccctggtgaccacactgacatacggcgtgcagtgtttctctaggtatccagaccacatgaagagacacgatttctttaagagcgccatgccagagggatacgtgcaggagcggaccatctccttcaaggacgatggcaagtataagacccgcgccgtggtgaagtttgagggcgatacactggtgaacaggatcgagctgaagggcaccgacttcaaggaggatggcaatatcctgggccacaagctggagtacaactttaatagccacaacgtgtatatcacagccgacaagcagaagaacggcatcaaggccaacttcaccgtgaggcacaatgtggaggacggctccgtgcagctggccgatcactaccagcagaacacacctatcggcgacggacccgtgctgctgcctgataatcactatctgtccacccagacagtgctgtctaaggacccaaacgagaagttggatccaggtggaggtggaagcggtatgaacaattcccagggaagagtgaccttcgaggacgtgaccgtgaacttcacccaaggcgagtggcagagactgaaccccgagcagagaaacctgtaccgggacgtgatgctggaaaactacagcaacctggtgtccgtcggccagggcgagacaacaaagcctgacgtgatcctgcggctggaacagggcaaagagccttggctggaagaggaagaggtgctcggatctggcagagccgagaagaatggcgatatcggcggacagatctggaagccaaaggatgtgaaagagagtctcggaagcggagctactaacttcagcctgctgaagcaggctggagacgtggaggagaaccctggacctatgcctgctgctaagagagtgaaactggatggatccaaccatgaccaggaatttgaccccccaaaggtttacccacctgtgccagctgagaagaggaagcccatccgcgtgctgtctctctttgatgggattgctacagggctcctggtgctgaaggacctgggcatccaagtggaccgctacattgcctccgaggtgtgtgaggactccatcacggtgggcatggtgcggcaccagggaaagatcatgtacgtcggggacgtccgcagcgtcacacagaagcatatccaggagtggggcccattcgacctggtgattggaggcagtccctgcaatgacctctccattgtcaaccctgcccgcaagggactttatgagggtactggccgcctcttctttgagttctaccgcctcctgcatgatgcgcggcccaaggagggagatgatcgccccttcttctggctctttgagaatgtggtggccatgggcgttagtgacaagagggacatctcgcgatttcttgagtctaaccccgtgatgattgacgccaaagaagtgtctgctgcacacagggcccgttacttctggggtaaccttcctggcatgaacaggcctttggcatccactgtgaatgataagctggagctgcaagagtgtctggagcacggcagaatagccaagttcagcaaagtgaggaccattaccaccaggtcaaactctataaagcagggcaaagaccagcatttccccgtgttcatgaacgagaaggaggacatcctgtggtgcactgaaatggaaagggtgtttggcttccccgtccactacacagacgtctccaacatgagccgcttggcgaggcagagactgctgggccgatcgtggagcgtgccggtcatccgccacctcttcgctccgctgaaggaatattttgcttgtgtgtctagcggcaatagtaacgctaacagccgcgggccgagcttcagcagcggcctggtgccgttaagcttgcgcggcagccatatgttcgaaaccgtgcctgtgtggaggagacagccagtccgggtgctgtccctttttgaagacatcaagaaagagctgacgagtttgggctttttggaaagtggttctgacccgggacaactgaagcatgtggttgatgtcacagacacagtgaggaaggatgtggaggagtggggacccttcgatcttgtgtacggcgccacacctcccctgggccacacctgtgaccgtcctcccagctggtacctgttccagttccaccggctcctgcagtacgcacggcccaagccaggcagccccaggcccttcttctggatgttcgtggacaatctggtgctgaacaaggaagacctggacgtcgcatctcgcttcctggagatggagccagtcaccatcccagatgtccacggcggatccttgcagaatgctgtccgcgtgtggagcaacatcccagccataaggagcagcaggcactgggctctggtttcggaagaagaattgtccctgctggcccagaacaagcagagctcgaagctcgcggccaagtggcccaccaagctggtgaagaactgctttctccccctaagagaatatttcaagtatttttcaggagggccgagctctggcgcacccccaccaagtggagggtctcctgccgggtccccaacatctactgaagaaggcaccagcgaatccgcaacgcccgagtcaggccctggtacctccacagaaccatctgaaggtagtgcgcctggttccccagctggaagccctacttccaccgaagaaggcacgtcaaccgaaccaagtgaaggatctgcccctgggaccagcactgaaccatctgagccaaaaaagaagagaaaggtaatgtcaaagctggagaaattcaccaactgttatagcctgtctaagaccctgcgcttcaaggcaatcccagtgggcaagacacaagagaacattgacaacaaacggctcctggtggaggatgagaagagggctgaagattacaagggcgttaagaagctgctggataggtactatctgtcattcatcaacgatgtcctccacagtatcaagctgaagaatctgaacaattacatttctctgttccggaagaagacacggaccgagaaggagaacaaagagctggagaatctggagatcaacctgaggaaagaaatagctaaggctttcaaagggaacgagggttacaagtccctgttcaagaaagacattatcgagactattctgcctgagttcctggacgataaagatgagatcgccctcgtcaattccttcaatgggtttaccacagcctttaccggcttcttcgacaatagagagaatatgttctctgaagaggccaaatccactagcatcgcctttcgctgcataaacgagaacctgactaggtacatcagcaatatggacatctttgagaaagtcgatgccatattcgacaaacatgaggtgcaggagattaaggagaagatcctgaactcagattacgatgtcgaagatttcttcgagggagagttcttcaacttcgtgctcacacaagagggcattgatgtgtacaatgcaatcattggagggttcgtgacagagagtggcgagaagataaagggcctgaacgagtatatcaacctctacaaccagaaaaccaagcagaaactgcctaagttcaagccactgtacaaacaagtgctctcagatagggaaagcctgagcttctacggtgaagggtatacatcagatgaagaagtgctcgaagtgttccgcaacaccctcaataagaacagtgaaatcttctcttcaatcaagaagctggagaaactgttcaagaatttcgatgagtactcctctgccggaatctttgtgaagaatggccctgcaatatccactattagcaaagacatctttggcgagtggaacgttatcagggataagtggaatgccgagtacgatgatattcatctcaagaagaaagccgtggttacagagaaatacgaggatgatagacgcaagagctttaagaagattggtagcttctctctcgaacagctgcaggagtacgccgacgctgacctgtcagtcgtggagaaactcaaggagatcataatccagaaggtggatgaaatctacaaagtgtatggaagctctgagaaactcttcgatgcagactttgttctggagaagagtctgaagaagaacgacgcagtggttgctatcatgaaggacctgctggattctgttaagtctttcgagaattacattaaggcattctttggtgaagggaaggagacaaatagggacgagagcttctatggcgactttgttctggcctacgacatcctcctcaaggttgaccacatctatgacgctatacggaattacgttacccagaagccctatagcaaagacaagttcaagctgtatttccagaatccacagtttatgggtgggtgggataaagacaaagaaacagattacagggccactatcctgcggtacggcagcaaatactatctggctatcatggataagaagtacgccaaatgcctccagaagatcgacaaggacgacgtgaacggtaactacgagaagatcaattacaagctcctgccaggacctaacaagatgctgcccaaggtgttcttctccaagaaatggatggcctactataacccaagcgaggacattcagaagatatacaagaatgggacattcaagaagggcgatatgttcaacctcaacgactgccacaagctgattgatttcttcaaggatagcatttctcgctatcccaagtggtctaatgcatacgatttcaacttcagcgagactgagaagtacaaagacatcgctggcttctaccgggaggtggaagagcaaggctataaggtgtcattcgaatccgcttctaagaaggaagtggataagctcgtggaagagggtaagctgtacatgttccagatatacaacaaagacttcagcgataagagccacggcactccaaacctccatactatgtatttcaagctgctgtttgacgagaacaaccacggacagattaggctgtcaggaggcgcagaactcttcatgcgcagagcttcactgaagaaggaggaactcgttgtccacccagccaatagccctatagccaataagaatccagacaatcctaagaaaaccactactctgtcttacgatgtgtataaggataagagattctctgaagatcagtacgaactgcacatacccattgccattaacaagtgccctaagaacatcttcaagattaacacagaggttagagtgctcctgaaacacgacgataacccttatgttataggcattgctcgcggagagagaaacctgctgtacatcgtcgtggtggacggcaaaggcaacatcgtggaacagtacagtctcaatgaaatcattaacaatttcaacggaatccgcattaagaccgactaccattctctcctcgacaagaaggagaaagaaaggttcgaagcaagacagaattggacaagtatagagaatatcaaagaactgaaggctgggtacatctctcaggttgtgcacaagatatgtgagctggtggagaagtacgacgctgttatcgccctcgcggacctgaatagcggcttcaagaactccagggtgaaggtggagaagcaggtgtatcagaagttcgagaagatgctgatcgacaagctcaactatatggtggacaagaaatccaatccttgcgctactggtggagccctgaagggctatcaaatcaccaataagttcgaatctttcaagtctatgagcacccagaatggcttcatcttctacatacccgcatggctgacatccaagattgatccctctaccggatttgttaatctgctcaagactaagtacacctctattgctgactcaaagaagttcatatcatcatttgaccgcatcatgtacgtgccagaagaggacctgttcgagtttgccctggattacaagaatttctctcggactgacgccgactacatcaagaagtggaagctctactcttatggtaatcggattcgcatattccgcaatcccaagaagaataacgtgttcgattgggaggaagtttgcctcaccagcgcttacaaggagctgttcaataagtatgggattaactaccagcagggcgacataagagccctgctgtgcgaacaatctgataaggcattctattcctctttcatggcactgatgtcactgatgctgcaaatgcgcaattccatcaccggaagaacagacgtggcctttctgatctctcctgtcaagaactcagatggcatcttctacgattcccgcaactatgaagcacaggagaatgctatcctgcctaagaatgccgatgcaaatggagcctataacatcgccagaaaggtcctctgggccataggacaattcaagaaagctgaagatgagaagctggacaaggtgaagatcgccatttcaaacaaagagtggctcgaatatgctcagacctcagtgaagcatgcctatccctatgacgtgcccgattatgccagcctgggcagcggctcccccaagaaaaaacgcaaggtggaagatcctaagaaaaagcggaaagtggacggcagcggcagcgagacccccggtaccagcgagagcgccacccccgagagcggtagtgggagcaacggcagcagcggatccatgcgtgaccacatggtccttcatgagtatgtaaatgctgctgggattacagcggcc

SEQ ID NO: 236 - DNA, 9450 bp, synthetic construct
  misc_feature 1..9450: note = DNA of V42_GFP1-10-ZIM3-2a-D3a-hD3L-dCas12i-1xGFP11
  source 1..9450: mol_type = other DNA
gcaaggtcaggctccggccagcggggaagcaagcgcaccgccgatggttccgagttcgaaagccccaaaaaaaagcgcaaggtctgagatcccaagcacgcagcaatgcagctcaaaacgcttagcctagccacacccccacgggaaacagcagtgattaacctttagcaataaacgaaagtttaactaagctatactaaccccagggttggtcaatttcgtgccagccacaccctggtactgcatgcacgcaatgctagctgcccctttcccgtcctgggcaccccgagtctcccccgaccccgggtcccaggtatgctcccacctccacctgccccactcaccacctctgctagttccagacacctccgagacgaggaaaaaaaaaaaaaaaaaaaaaaaaaaaaaaaaaaaaaaaaaaaaaaaaaaaaaaaaaaaaaaaaaaaaaaaaaaaaaaaaaaaaaaaaaaaaaaaaaaaaaaaaaaaaaaaaaaaaaaaaaaaaaaaaaaaaaaaaaaaaaaaaaaaaaaaaaaaaaaaaaaaaaaaaaaaaaaaaaaaaaaaaaaaaaaaaaaaaaaaaaaaaaaaaaaaaaaaaaaaaaaaaaaaaaaaaaaaaaaaaaaaaaaaaaaaaaaaaaaaaaaaaaaaaaaaaaaaaaaaaaaaaaaaaaaaaaaaaaaaaaaaaaaaaaaaaaaaaaaaaaaaaaaaaaaaaaaaaaaaaaaaaaaaaaaaaaaaaaaaaaaaaaaaaaaaaaaaaaaaaaaaaaaaaaaaaaaccgtcttcaagctttctagaaattcactggccgtcgttttacaacgtcgtgactgggaaaaccctggcgttacccaacttaatcgccttgcagcacatccccctttcgccagctggcgtaatagcgaagaggcccgcaccgatcgcccttcccaacagttgcgcagcctgaatggcgaatggcgcctgatgcggtattttctccttacgcatctgtgcggtatttcacaccgcatatggtgcactctcagtacaatctgctctgatgccgcatagttaagccagccccgacacccgccaacacccgctgacgcgccctgacgggcttgtctgctcccggcatccgcttacagacaagctgtgaccgtctccgggagctgcatgtgtcagaggttttcaccgtcatcaccgaaacgcgcgagacgaaagggcctcgtgatacgcctatttttataggttaatgtcatgataataatggtttcttagacgtcaggtggcacttttcggggaaatgtgcgcggaacccctatttgtttatttttctaaatacattcaaatatgtatccgctcatgagacaataaccctgataaatgcttcaataatattgaaaaaggaagagtatgagtattcaacatttccgtgtcgcccttattcccttttttgcggcattttgccttcctgtttttgctcacccagaaacgctggtgaaagtaaaagatgctgaagatcagttgggtgcacgagtgggttacatcgaactggatctcaacagcggtaagatccttgagagttttcgccccgaagaacgttttccaatgatgagcacttttaaagttctgctatgtggcgcggtattatcccgtattgacgccgggcaagagcaactcggtcgccgcatacactattctcagaatgacttggttgagtactcaccagtcacagaaaagcatcttacggatggcatgacagtaagagaattatgcagtgctgccataaccatgagtgataacactgcggccaacttacttctgacaacgatcggaggaccgaaggagctaaccgcttttttgcacaacatgggggatcatgtaactcgccttgatcgttgggaaccggagctgaatgaagccataccaaacgacgagcgtgacaccacgatgcctgtagcaatggcaacaacgttgcgcaaactattaactggcgaactacttactctagcttcccggcaacaattaatagactggatggaggcggataaagttgcaggaccacttctgcgctcggcccttccggctggctggtttattgctgataaatctggagccggtgagcgtgggtctcgcggtatcattgcagcactggggccagatggtaagccctcccgtatcgtagttatctacacgacggggagtcaggcaactatggatgaacgaaatagacagatcgctgagataggtgcctcactgattaagcattggtaactgtcagaccaagtttactcatatatactttagattgatttaaaacttcatttttaatttaaaaggatctaggtgaagatcctttttgataatctcatgaccaaaatcccttaacgtgagttttcgttccactgagcgtcagaccccgtagaaaagatcaaaggatcttcttgagatcctttttttctgcgcgtaatctgctgcttgcaaacaaaaaaaccaccgctaccagcggtggtttgtttgccggatcaagagctaccaactctttttccgaaggtaactggcttcagcagagcgcagataccaaatactgttcttctagtgtagccgtagttaggccaccacttcaagaactctgtagcaccgcctacatacctcgctctgctaatcctgttaccagtggctgctgccagtggcgataagtcgtgtcttaccgggttggactcaagacgatagttaccggataaggcgcagcggtcgggctgaacggggggttcgtgcacacagcccagcttggagcgaacgacctacaccgaactgagatacctacagcgtgagctatgagaaagcgccacgcttcccgaagggagaaaggcggacaggtatccggtaagcggcagggtcggaacaggagagcgcacgagggagcttccagggggaaacgcctggtatctttatagtcctgtcgggtttcgccacctctgacttgagcgtcgatttttgtgatgctcgtcaggggggcggagcctatggaaaaacgccagcaacgcggcctttttacggttcctggccttttgctggccttttgctcacatgttctttcctgcgttatcccctgattctgtggataaccgtattaccgcctttgagtgagctgataccgctcgccgcagccgaacgaccgagcgcagcgagtcagtgagcgaggaagcggaagagcgcccaatacgcaaaccgcctctccccgcgcgttggccgattcattaatgcagctggcacgacaggtttcccgactggaaagcgggcagtgagcgcaacgcaattaatgtgagttagctcactcattaggcaccccaggctttacactttatgcttccggctcgtatgttgtgtggaattgtgagcggataacaatttcacacaggaaacagctatgaccatgattacgcctctagaaagctttaatacgactcactataaggactcactatttgttttcgcgcccagttgcaaaaagtgtcgacatttgcttctgacacaactgtgttcactagcaacctcaaacagacaccgccaccatgtccaagggagaggagctgttcaccggagtggtgccaatcctggtggagctggacggcgatgtgaacggccacaagttttctgtgcgcggagagggagagggcgacgcaaccatcggcaagctgacactgaagttcatctgcaccacaggcaagctgcccgtgccttggccaaccctggtgaccacactgacatacggcgtgcagtgtttctctaggtatccagaccacatgaagagacacgatttctttaagagcgccatgccagagggatacgtgcaggagcggaccatctccttcaaggacgatggcaagtataagacccgcgccgtggtgaagtttgagggcgatacactggtgaacaggatcgagctgaagggcaccgacttcaaggaggatggcaatatcctgggccacaagctggagtacaactttaatagccacaacgtgtatatcacagccgacaagcagaagaacggcatcaaggccaacttcaccgtgaggcacaatgtggaggacggctccgtgcagctggccgatcactaccagcagaacacacctatcggcgacggacccgtgctgctgcctgataatcactatctgtccacccagacagtgctgtctaaggacccaaacgagaagttggatccaggtggaggtggaagcggtatgaacaattcccagggaagagtgaccttcgaggacgtgaccgtgaacttcacccaaggcgagtggcagagactgaaccccgagcagagaaacctgtaccgggacgtgatgctggaaaactacagcaacctggtgtccgtcggccagggcgagacaacaaagcctgacgtgatcctgcggctggaacagggcaaagagccttggctggaagaggaagaggtgctcggatctggcagagccgagaagaatggcgatatcggcggacagatctggaagccaaaggatgtgaaagagagtctcggaagcggagctactaacttcagcctgctgaagcaggctggagacgtggaggagaaccctggacctatgcctgctgctaagagagtgaaactggatggatccaaccatgaccaggaatttgaccccccaaaggtttacccacctgtgccagctgagaagaggaagcccatccgcgtgctgtctctctttgatgggattgctacagggctcctggtgctgaaggacctgggcatccaagtggaccgctacattgcctccgaggtgtgtgaggactccatcacggtgggcatggtgcggcaccagggaaagatcatgtacgtcggggacgtccgcagcgtcacacagaagcatatccaggagtggggcccattcgacctggtgattggaggcagtccctgcaatgacctctccattgtcaaccctgcccgcaagggactttatgagggtactggccgcctcttctttgagttctaccgcctcctgcatgatgcgcggcccaaggagggagatgatcgccccttcttctggctctttgagaatgtggtggccatgggcgttagtgacaagagggacatctcgcgatttcttgagtctaaccccgtgatgattgacgccaaagaagtgtctgctgcacacagggcccgttacttctggggtaaccttcctggcatgaacaggcctttggcatccactgtgaatgataagctggagctgcaagagtgtctggagcacggcagaatagccaagttcagcaaagtgaggaccattaccaccaggtcaaactctataaagcagggcaaagaccagcatttccccgtgttcatgaacgagaaggaggacatcctgtggtgcactgaaatggaaagggtgtttggcttccccgtccactacacagacgtctccaacatgagccgcttggcgaggcagagactgctgggccgatcgtggagcgtgccggtcatccgccacctcttcgctccgctgaaggaatattttgcttgtgtgtctagcggcaatagtaacgctaacagccgcgggccgagcttcagcagcggcctggtgccgttaagcttgcgcggcagccatatgttcgaaaccgtgcctgtgtggaggagacagccagtccgggtgctgtccctttttgaagacatcaagaaagagctgacgagtttgggctttttggaaagtggttctgacccgggacaactgaagcatgtggttgatgtcacagacacagtgaggaaggatgtggaggagtggggacccttcgatcttgtgtacggcgccacacctcccctgggccacacctgtgaccgtcctcccagctggtacctgttccagttccaccggctcctgcagtacgcacggcccaagccaggcagccccaggcccttcttctggatgttcgtggacaatctggtgctgaacaaggaagacctggacgtcgcatctcgcttcctggagatggagccagtcaccatcccagatgtccacggcggatccttgcagaatgctgtccgcgtgtggagcaacatcccagccataaggagcagcaggcactgggctctggtttcggaagaagaattgtccctgctggcccagaacaagcagagctcgaagctcgcggccaagtggcccaccaagctggtgaagaactgctttctccccctaagagaatatttcaagtatttttcaggagggccgagctctggcgcacccccaccaagtggagggtctcctgccgggtccccaacatctactgaagaaggcaccagcgaatccgcaacgcccgagtcaggccctggtacctccacagaaccatctgaaggtagtgcgcctggttccccagctggaagccctacttccaccgaagaaggcacgtcaaccgaaccaagtgaaggatctgcccctgggaccagcactgaaccatctgagccaaaaaagaagagaaaggtaatggaagagacacggacccctgagaagatcgcctgccagcaggatagaagcgccttcttcaagctgggcaagctgccccagaaaaccaccagcgccatctaccacctgatgcggtgtagcaagcggtacatcgacaacgtgtccgagacaatcagcaacaacatcgagaaggccgccatgaccagcgacaaccacatcttcagaagcgccctgaaagaagagtacaagaagatctaccgcgagaagttctaccccgacgtgaccggccagccttttccagataagggccccgacaacacccacatcgtggaacggaccgtggaaaacctgtgcggccagtacatctctgccctgaagggcgtgatgaaagtgcggaagcccaagtggcaggacgacatcttcgaggacgagagcgacaaagtgatcgccgagatgctgatggccagcggcaacgaggccgacattcaccccaagctggaaaagaagattgccagcgccaagaaaaaggacaagatggacgagtggcagaaggtgctggacagatacgactacatcaagagcaagaccgacatcgagtggacctacaccacactgctgtacgaccacattgcccgcgagtgcgccagatccatgttcgaggatggcaacaagcctaagttctgctacaccaacggcaacaagttcgccaaacaggtggtggacgagctgtggggctctgagagagtggaatacgagtacgagaagtacctgcactgcagaaccctggaagcctactggaacgaggaaaacaagtacttcttcctggaaaatcaaaagaagtccaagaaaacctacgaggcccggcagatcatcgaccacttcatcgagaacgaggacgccgtgaaggccgaaaccgaagagtatatggccaaggtggccaaagagttcggcgagaacggcggctgcaagttcagaaccgagaacatcctgtacctggtcaacagcgtgtccatcaacaagaagcaggacgaggaacggtgccccatcttcaaagtgaccgacattccccagtatgccgaggccggcatcgatagaatcggcgagtgcaaatacgtgatcaagctgaagctgttcaccgtgggcgagagatacggcaccacctatatgcctgaggccttcagcggcctgtacgacagaaggaccaaccagagatacgacctgatcgacagagcctgcaagggcagctacgtgtacctgcctatctacatcagcgacaaggacagccggaagtggagcgacagactgaagaacaccttcaccatgtccgccttcagcatcagcgagcgcaagaccaagaaagacggcagagtgctgtgcgtgaacctgccttacacacacatccagcacaagccccggaactacttcaaggtgtaccccacctacggcgtggacatcaacgtgaagcacagcctgttcagcaccaacgccaccaacctgaacggctacatcgacgtgaacggcgagctgatcgacttctacaacagcatcggcagacccgataagctcaagaacatcaacctggccgtgacactgggcgacaaaggcggcacagctggcaaccacaccaactttctgctggtgtccgacctcggcgactgggatgatcacggcaagaagcggaacgacagattcgtgaagagagaggacggcacctactacagcagacctgacctgctggccgccggcctgaacttcctgaagaagaagtatagcggcgaccggaagtcctacgattatatcaacaccacaatcgccttccggaacaaccagaccagactgagatgcatcgacaaagagtggaacgatcggaagcgggcctacgatgaggaacacggcaagcctgagaagggcgaaagaagcggcttctaccctaccgaggatgccgagcggctgacaatggaaagacaggccctgcggagagagattgccgagaacaccagacaagtgattgcctacatgctgtggctgttccaagagaacggcatcaagtctatcgccctggaacacctggattgcggcagctggaagaacttccgggaccagctgaagccaaagtggttctgcaacaactgcaagtactgggccgagaagtatggcatcccttacgaggccaccaagtactacagaagcaaccggaagtactttgacatcgaggacggggagctgattcccgagaatgtgaagctgaacgccctgggcgaagccgagaacgacaagagatacttccagacctctatcgccaaggccgtgggcatgagcagcatcaagcagatgttcagcatcgtgtcccagaactacgacatccaagtgaactacaccgagcaggcctacaccagccagaccgacagcagaaatggcaccgtggacaaggacttcagagtgtcccaagagtgctacatcggcagcgacggcaccaagatgaactgcgactttaacgccgccgtgaatatcgccgaccggatctccgatgacaccctgcgggaagagttcaacaaagaactgcccatgaaggaatttgtgaagtacggcgccacacagatcgtgtctcggaacagaagatggaacgccgaaaacgccgagagggtcacaatggccgccttccagaagagaaagaacgctgacggcggagcccataccgccgctgtgaagcctacatccaagaccgaggaaagcagcctgaagctggtggccgaagcctatccctatgacgtgcccgattatgccagcctgggcagcggctcccccaagaaaaaacgcaaggtggaagatcctaagaaaaagcggaaagtggacggcagcggcagcgagacccccggtaccagcgagagcgccacccccgagagcggtagtgggagcaacggcagcagcggatccatgcgtgaccacatggtccttcatgagtatgtaaatgctgctgggattacagcggcc

SEQ ID NO: 237 - DNA, 10644 bp, synthetic construct
  misc_feature 1..10644: note = DNA of V43_D3a-D3l-GFP1-10-2a-1xGFP11-dCas9-KRAB
  source 1..10644: mol_type = other DNA
atcgtgctgaccctgacactgtttgaggacagagagatgatcgaggaacggctgaaaacctatgcccacctgttcgacgacaaagtgatgaagcagctgaagcggcggagatacaccggctggggcaggctgagccggaagctgatcaacggcatccgggacaagcagtccggcaagacaatcctggatttcctgaagtccgacggcttcgccaacagaaacttcatgcagctgatccacgacgacagcctgacctttaaagaggacatccagaaagcccaggtgtccggccagggcgatagcctgcacgagcacattgccaatctggccggcagccccgccattaagaagggcatcctgcagacagtgaaggtggtggacgagctcgtgaaagtgatgggccggcacaagcccgagaacatcgtgatcgaaatggccagagagaaccagaccacccagaagggacagaagaacagccgcgagagaatgaagcggatcgaagagggcatcaaagagctgggcagccagatcctgaaagaacaccccgtggaaaacacccagctgcagaacgagaagctgtacctgtactacctgcagaatgggcgggatatgtacgtggaccaggaactggacatcaaccggctgtccgactacgatgtggacgctatcgtgcctcagagctttctgaaggacgactccatcgataacaaagtgctgactcggagcgacaagaaccggggcaagagcgacaacgtgccctccgaagaggtcgtgaagaagatgaagaactactggcgccagctgctgaatgccaagctgattacccagaggaagttcgacaatctgaccaaggccgagagaggcggcctgagcgaactggataaggccggcttcatcaagagacagctggtggaaacccggcagatcacaaagcacgtggcacagatcctggactcccggatgaacactaagtacgacgagaacgacaaactgatccgggaagtgaaagtgatcaccctgaagtccaagctggtgtccgatttccggaaggatttccagttttacaaagtgcgcgagatcaacaactaccaccacgcccacgacgcctacctgaacgccgtcgtgggaaccgccctgatcaaaaagtaccctaagctggaaagcgagttcgtgtacggcgactacaaggtgtacgacgtgcggaagatgatcgccaagagcgagcaggaaatcggcaaggctaccgccaagtacttcttctacagcaacatcatgaactttttcaagaccgagattaccctggccaacggcgagatccggaagcggcctctgatcgagacaaacggcgaaacaggcgagatcgtgtgggataagggccgggactttgccaccgtgcggaaagtgctgtctatgccccaagtgaatatcgtgaaaaagaccgaggtgcagacaggcggcttcagcaaagagtctatcctgcccaagaggaacagcgacaagctgatcgccagaaagaaggactgggaccctaagaagtacggcggcttcgacagccccaccgtggcctattctgtgctggtggtggccaaagtggaaaagggcaagtccaagaaactgaagagtgtgaaagagctgctggggatcaccatcatggaaagaagcagcttcgagaagaatcccatcgactttctggaagccaagggctacaaagaagtgaaaaaggacctgatcatcaagctgcctaagtactccctgttcgagctggaaaacggccggaagagaatgctggcctctgccggcgaactgcagaagggaaacgaactggccctgccctccaaatatgtgaacttcctgtacctggccagccactatgagaagctgaagggctcccccgaggataatgagcagaaacagctgtttgtggaacagcacaaacactacctggacgagatcatcgagcagatcagcgagttctccaagagagtgatcctggccgacgctaatctggacaaggtgctgagcgcctacaacaagcacagagacaagcctatcagagagcaggccgagaatatcatccacctgtttaccctgaccaatctgggagcccctgccgccttcaagtactttgacaccaccatcgaccggaagaggtacaccagcaccaaagaggtgctggacgccaccctgatccaccagagcatcaccggcctgtacgagacacggatcgacctgtctcagctgggaggcgacgcctatccctatgacgtgcccgattatgccagcctgggcagcggctcccccaagaaaaaacgcaaggtggaagatcctaagaaaaagcggaaagtggacggcagcggcagcgagacccccggtaccagcgagagcgccacccccgagagccggacactggtgaccttcaaggatgtatttgtggacttcaccagggaggagtggaagctgctggacactgctcagcagatcgtgtacagaaatgtgatgctggagaactataagaacctggtttccttgggttatcagcttactaagccagatgtgatcctccggttggagaagggagaagagccctgagatcccaagcacgcagcaatgcagctcaaaacgcttagcctagccacacccccacgggaaacagcagtgattaacctttagcaataaacgaaagtttaactaagctatactaaccccagggttggtcaatttcgtgccagccacaccctggtactgcatgcacgcaatgctagctgcccctttcccgtcctgggcaccccgagtctcccccgaccccgggtcccaggtatgctcccacctccacctgccccactcaccacctctgctagttccagacacctccgagacgaggaaaaaaaaaaaaaaaaaaaaaaaaaaaaaaaaaaaaaaaaaaaaaaaaaaaaaaaaaaaaaaaaaaaaaaaaaaaaaaaaaaaaaaaaaaaaaaaaaaaaaaaaaaaaaaaaaaaaaaaaaaaaaaaaaaaaaaaaaaaaaaaaaaaaaaaaaaaaaaaaaaaaaaaaaaaaaaaaaaaaaaaaaaaaaaaaaaaaaaaaaaaaaaaaaaaaaaaaaaaaaaaaaaaaaaaaaaaaaaaaaaaaaaaaaaaaaaaaaaaaaaaaaaaaaaaaaaaaaaaaaaaaaaaaaaaaaaaaaaaaaaaaaaaaaaaaaaaaaaaaaaaaaaaaaaaaaaaaaaaaaaaaaaaaaaaaaaaaaaaaaaaaaaaaaaaaaaaaaaaaaaaaaaaaaaaaaaccgtcttcaagctttctagaaattcactggccgtcgttttacaacgtcgtgactgggaaaaccctggcgttacccaacttaatcgccttgcagcacatccccctttcgccagctggcgtaatagcgaagaggcccgcaccgatcgcccttcccaacagttgcgcagcctgaatggcgaatggcgcctgatgcggtattttctccttacgcatctgtgcggtatttcacaccgcatatggtgcactctcagtacaatctgctctgatgccgcatagttaagccagccccgacacccgccaacacccgctgacgcgccctgacgggcttgtctgctcccggcatccgcttacagacaagctgtgaccgtctccgggagctgcatgtgtcagaggttttcaccgtcatcaccgaaacgcgcgagacgaaagggcctcgtgatacgcctatttttataggttaatgtcatgataataatggtttcttagacgtcaggtggcacttttcggggaaatgtgcgcggaacccctatttgtttatttttctaaatacattcaaatatgtatccgctcatgagacaataaccctgataaatgcttcaataatattgaaaaaggaagagtatgagtattcaacatttccgtgtcgcccttattcccttttttgcggcattttgccttcctgtttttgctcacccagaaacgctggtgaaagtaaaagatgctgaagatcagttgggtgcacgagtgggttacatcgaactggatctcaacagcggtaagatccttgagagttttcgccccgaagaacgttttccaatgatgagcacttttaaagttctgctatgtggcgcggtattatcccgtattgacgccgggcaagagcaactcggtcgccgcatacactattctcagaatgacttggttgagtactcaccagtcacagaaaagcatcttacggatggcatgacagtaagagaattatgcagtgctgccataaccatgagtgataacactgcggccaacttacttctgacaacgatcggaggaccgaaggagctaaccgcttttttgcacaacatgggggatcatgtaactcgccttgatcgttgggaaccggagctgaatgaagccataccaaacgacgagcgtgacaccacgatgcctgtagcaatggcaacaacgttgcgcaaactattaactggcgaactacttactctagcttcccggcaacaattaatagactggatggaggcggataaagttgcaggaccacttctgcgctcggcccttccggctggctggtttattgctgataaatctggagccggtgagcgtgggtctcgcggtatcattgcagcactggggccagatggtaagccctcccgtatcgtagttatctacacgacggggagtcaggcaactatggatgaacgaaatagacagatcgctgagataggtgcctcactgattaagcattggtaactgtcagaccaagtttactcatatatactttagattgatttaaaacttcatttttaatttaaaaggatctaggtgaagatcctttttgataatctcatgaccaaaatcccttaacgtgagttttcgttccactgagcgtcagaccccgtagaaaagatcaaaggatcttcttgagatcctttttttctgcgcgtaatctgctgcttgcaaacaaaaaaaccaccgctaccagcggtggtttgtttgccggatcaagagctaccaactctttttccgaaggtaactggcttcagcagagcgcagataccaaatactgttcttctagtgtagccgtagttaggccaccacttcaagaactctgtagcaccgcctacatacctcgctctgctaatcctgttaccagtggctgctgccagtggcgataagtcgtgtcttaccgggttggactcaagacgatagttaccggataaggcgcagcggtcgggctgaacggggggttcgtgcacacagcccagcttggagcgaacgacctacaccgaactgagatacctacagcgtgagctatgagaaagcgccacgcttcccgaagggagaaaggcggacaggtatccggtaagcggcagggtcggaacaggagagcgcacgagggagcttccagggggaaacgcctggtatctttatagtcctgtcgggtttcgccacctctgacttgagcgtcgatttttgtgatgctcgtcaggggggcggagcctatggaaaaacgccagcaacgcggcctttttacggttcctggccttttgctggccttttgctcacatgttctttcctgcgttatcccctgattctgtggataaccgtattaccgcctttgagtgagctgataccgctcgccgcagccgaacgaccgagcgcagcgagtcagtgagcgaggaagcggaagagcgcccaatacgcaaaccgcctctccccgcgcgttggccgattcattaatgcagctggcacgacaggtttcccgactggaaagcgggcagtgagcgcaacgcaattaatgtgagttagctcactcattaggcaccccaggctttacactttatgcttccggctcgtatgttgtgtggaattgtgagcggataacaatttcacacaggaaacagctatgaccatgattacgcctctagaaagctttaatacgactcactataaggactcactatttgttttcgcgcccagttgcaaaaagtgtcgacatttgcttctgacacaactgtgttcactagcaacctcaaacagacaccgccaccatgcctgctgctaagagagtgaaactggatggatccaaccatgaccaggaatttgaccccccaaaggtttacccacctgtgccagctgagaagaggaagcccatccgcgtgctgtctctctttgatgggattgctacagggctcctggtgctgaaggacctgggcatccaagtggaccgctacattgcctccgaggtgtgtgaggactccatcacggtgggcatggtgcggcaccagggaaagatcatgtacgtcggggacgtccgcagcgtcacacagaagcatatccaggagtggggcccattcgacctggtgattggaggcagtccctgcaatgacctctccattgtcaaccctgcccgcaagggactttatgagggtactggccgcctcttctttgagttctaccgcctcctgcatgatgcgcggcccaaggagggagatgatcgccccttcttctggctctttgagaatgtggtggccatgggcgttagtgacaagagggacatctcgcgatttcttgagtctaaccccgtgatgattgacgccaaagaagtgtctgctgcacacagggcccgttacttctggggtaaccttcctggcatgaacaggcctttggcatccactgtgaatgataagctggagctgcaagagtgtctggagcacggcagaatagccaagttcagcaaagtgaggaccattaccaccaggtcaaactctataaagcagggcaaagaccagcatttccccgtgttcatgaacgagaaggaggacatcctgtggtgcactgaaatggaaagggtgtttggcttccccgtccactacacagacgtctccaacatgagccgcttggcgaggcagagactgctgggccgatcgtggagcgtgccggtcatccgccacctcttcgctccgctgaaggaatattttgcttgtgtgtctagcggcaatagtaacgctaacagccgcgggccgagcttcagcagcggcctggtgccgttaagcttgcgcggcagccatatgggccctatggagatatacaagacagtgtctgcatggaagagacagccagtgcgggtactgagcctcttcagaaacatcgacaaggtactaaagagtttgggcttcttggaaagcggttctggttctgggggaggaacgctgaagtacgtggaagatgtcacaaatgtcgtgaggagagacgtggagaaatggggcccctttgacctggtgtacggctcgacgcagcccctaggcagctcttgtgatcgctgtcccggctggtacatgttccagttccaccggatcctgcagtatgcgctgcctcgccaggagagtcagcggcccttcttctggatattcatggacaatctgctgctgactgaggatgaccaagagacaactacccgcttccttcagacagaggctgtgaccctccaggatgtccgtggcagagactaccagaatgctatgcgggtgtggagcaacattccagggctgaagagcaagcatgcgcccctgaccccaaaggaagaagagtatctgcaagcccaagtcagaagcaggagcaagctggacgccccgaaagttgacctcctggtgaagaactgccttctcccgctgagagagtacttcaagtatttttctcaaaactcacttcctcttggagggccgagctctggcgcacccccaccaagtggagggtctcctgccgggtccccaacatctactgaagaaggcaccagcgaatccgcaacgatgtccaagggagaggagctgttcaccggagtggtgccaatcctggtggagctggacggcgatgtgaacggccacaagttttctgtgcgcggagagggagagggcgacgcaaccatcggcaagctgacactgaagttcatctgcaccacaggcaagctgcccgtgccttggccaaccctggtgaccacactgacatacggcgtgcagtgtttctctaggtatccagaccacatgaagagacacgatttctttaagagcgccatgccagagggatacgtgcaggagcggaccatctccttcaaggacgatggcaagtataagacccgcgccgtggtgaagtttgagggcgatacactggtgaacaggatcgagctgaagggcaccgacttcaaggaggatggcaatatcctgggccacaagctggagtacaactttaatagccacaacgtgtatatcacagccgacaagcagaagaacggcatcaaggccaacttcaccgtgaggcacaatgtggaggacggctccgtgcagctggccgatcactaccagcagaacacacctatcggcgacggacccgtgctgctgcctgataatcactatctgtccacccagacagtgctgtctaaggacccaaacgagaagttggatccaggtggaggtggaagcggaagcggagctactaacttcagcctgctgaagcaggctggagacgtggaggagaaccctggacctatgcctgctgctaagagagtgaaactggatggatccggccccgacatcgtgatcggtagcggcggtcgggaccatatggtcctgcacgaatatgtcaatgctgccggtatcaccgcggccgcaaggtcaggctccggccagcggggaagcaagcgcaccgccgatggttccgagttcgaaagccccaaaaaaaagcgcaaggtcggcggaagcggaagcggaccaaaaaagaagagaaaggtaatggacaagaagtacagcatcggcctggccatcggcaccaactctgtgggctgggccgtgatcaccgacgagtacaaggtgcccagcaagaaattcaaggtgctgggcaacaccgaccggcacagcatcaagaagaacctgatcggcgccctgctgttcgacagcggagaaacagccgaggccacccggctgaagagaaccgccagaagaagatacaccagacggaagaaccggatctgctatctgcaagagatcttcagcaacgagatggccaaggtggacgacagcttcttccacagactggaagagtccttcctggtggaagaggataagaagcacgagcggcaccccatcttcggcaacatcgtggacgaggtggcctaccacgagaagtaccccaccatctaccacctgagaaagaaactggtggacagcaccgacaaggccgacctgcggctgatctatctggccctggcccacatgatcaagttccggggccacttcctgatcgagggcgacctgaaccccgacaacagcgacgtggacaagctgttcatccagctggtgcagacctacaaccagctgttcgaggaaaaccccatcaacgccagcggcgtggacgccaaggccatcctgtctgccagactgagcaagagcagacggctggaaaatctgatcgcccagctgcccggcgagaagaagaatggcctgttcggcaacctgattgccctgagcctgggcctgacccccaacttcaagagcaacttcgacctggccgaggatgccaaactgcagctgagcaaggacacctacgacgacgacctggacaacctgctggcccagatcggcgaccagtacgccgacctgtttctggccgccaagaacctgtccgacgccatcctgctgagcgacatcctgagagtgaacaccgagatcaccaaggcccccctgagcgcctctatgatcaagagatacgacgagcaccaccaggacctgaccctgctgaaagctctcgtgcggcagcagctgcctgagaagtacaaagagattttcttcgaccagagcaagaacggctacgccggctacatcgatggcggagccagccaggaagagttctacaagttcatcaagcccatcctggaaaagatggacggcaccgaggaactgctcgtgaagctgaacagagaggacctgctgcggaagcagcggaccttcgacaacggcagcatcccccaccagatccacctgggagagctgcacgccattctgcggcggcaggaagatttttacccattcctgaaggacaaccgggaaaagatcgagaagatcctgaccttccgcatcccctactacgtgggccctctggccaggggaaacagcagattcgcctggatgaccagaaagagcgaggaaaccatcaccccctggaacttcgaggaagtggtggacaagggcgccagcgcccagagcttcatcgagcggatgaccaacttcgataagaacctgcccaacgagaaggtgctgcccaagcacagcctgctgtacgagtacttcaccgtgtacaacgagctgaccaaagtgaaatacgtgaccgagggaatgagaaagcccgccttcctgagcggcgagcagaaaaaagccatcgtggacctgctgttcaagaccaaccggaaagtgaccgtgaagcagctgaaagaggactacttcaagaaaatcgagtgcttcgactccgtggaaatctccggcgtggaagatcggttcaacgcctccctgggcacataccacgatctgctgaaaattatcaaggacaaggacttcctggacaatgaggaaaacgaggacattctggaagat

SEQ ID NO: 238 - DNA, 11238 bp, synthetic construct
  misc_feature 1..11238: note = DNA of V44_7xGFP11-dCas9-ZIM3-2a-D3a-hD3L-GFP1-10
  source 1..11238: mol_type = other DNA
tgagataggtgcctcactgattaagcattggtaactgtcagaccaagtttactcatatatactttagattgatttaaaacttcatttttaatttaaaaggatctaggtgaagatcctttttgataatctcatgaccaaaatcccttaacgtgagttttcgttccactgagcgtcagaccccgtagaaaagatcaaaggatcttcttgagatcctttttttctgcgcgtaatctgctgcttgcaaacaaaaaaaccaccgctaccagcggtggtttgtttgccggatcaagagctaccaactctttttccgaaggtaactggcttcagcagagcgcagataccaaatactgttcttctagtgtagccgtagttaggccaccacttcaagaactctgtagcaccgcctacatacctcgctctgctaatcctgttaccagtggctgctgccagtggcgataagtcgtgtcttaccgggttggactcaagacgatagttaccggataaggcgcagcggtcgggctgaacggggggttcgtgcacacagcccagcttggagcgaacgacctacaccgaactgagatacctacagcgtgagctatgagaaagcgccacgcttcccgaagggagaaaggcggacaggtatccggtaagcggcagggtcggaacaggagagcgcacgagggagcttccagggggaaacgcctggtatctttatagtcctgtcgggtttcgccacctctgacttgagcgtcgatttttgtgatgctcgtcaggggggcggagcctatggaaaaacgccagcaacgcggcctttttacggttcctggccttttgctggccttttgctcacatgttctttcctgcgttatcccctgattctgtggataaccgtattaccgcctttgagtgagctgataccgctcgccgcagccgaacgaccgagcgcagcgagtcagtgagcgaggaagcggaagagcgcccaatacgcaaaccgcctctccccgcgcgttggccgattcattaatgcagctggcacgacaggtttcccgactggaaagcgggcagtgagcgcaacgcaattaatgtgagttagctcactcattaggcaccccaggctttacactttatgcttccggctcgtatgttgtgtggaattgtgagcggataacaatttcacacaggaaacagctatgaccatgattacgcctctagaaagctttaatacgactcactataaggactcactatttgttttcgcgcccagttgcaaaaagtgtcgacatttgcttctgacacaactgtgttcactagcaacctcaaacagacaccgccaccatgcctgctgctaagagagtgaaactggatggatccatgcgtgaccacatggtccttcatgagtatgtaaatgctgctgggattacaggtggctctggaggtagagatcatatggttctccacgaatacgttaacgccgcaggcatcactggcggtagtggaggacgcgaccatatggtactacatgaatatgtcaatgcagccggaataaccggagggtccggaggccgggatcacatggtgctgcatgagtatgtgaacgcggcgggtataactggtgggtcgggcggacgagaccatatggtgcttcacgaatacgtaaacgcagctggcattactggcggatcaggtggcagggatcacatggtactccatgagtacgtgaacgctgctggaatcacaggcggtagcggcggtcgggaccatatggtcctgcacgaatatgtcaatgctgccggtatcaccgcggccgcaaggtcaggctccggccagcggggaagcaagcgcaccgccgatggttccgagttcgaaagccccaaaaaaaagcgcaaggtcggcggaagcggaagcggaccaaaaaagaagagaaaggtaatggacaagaagtacagcatcggcctggccatcggcaccaactctgtgggctgggccgtgatcaccgacgagtacaaggtgcccagcaagaaattcaaggtgctgggcaacaccgaccggcacagcatcaagaagaacctgatcggcgccctgctgttcgacagcggagaaacagccgaggccacccggctgaagagaaccgccagaagaagatacaccagacggaagaaccggatctgctatctgcaagagatcttcagcaacgagatggccaaggtggacgacagcttcttccacagactggaagagtccttcctggtggaagaggataagaagcacgagcggcaccccatcttcggcaacatcgtggacgaggtggcctaccacgagaagtaccccaccatctaccacctgagaaagaaactggtggacagcaccgacaaggccgacctgcggctgatctatctggccctggcccacatgatcaagttccggggccacttcctgatcgagggcgacctgaaccccgacaacagcgacgtggacaagctgttcatccagctggtgcagacctacaaccagctgttcgaggaaaaccccatcaacgccagcggcgtggacgccaaggccatcctgtctgccagactgagcaagagcagacggctggaaaatctgatcgcccagctgcccggcgagaagaagaatggcctgttcggcaacctgattgccctgagcctgggcctgacccccaacttcaagagcaacttcgacctggccgaggatgccaaactgcagctgagcaaggacacctacgacgacgacctggacaacctgctggcccagatcggcgaccagtacgccgacctgtttctggccgccaagaacctgtccgacgccatcctgctgagcgacatcctgagagtgaacaccgagatcaccaaggcccccctgagcgcctctatgatcaagagatacgacgagcaccaccaggacctgaccctgctgaaagctctcgtgcggcagcagctgcctgagaagtacaaagagattttcttcgaccagagcaagaacggctacgccggctacatcgatggcggagccagccaggaagagttctacaagttcatcaagcccatcctggaaaagatggacggcaccgaggaactgctcgtgaagctgaacagagaggacctgctgcggaagcagcggaccttcgacaacggcagcatcccccaccagatccacctgggagagctgcacgccattctgcggcggcaggaagatttttacccattcctgaaggacaaccgggaaaagatcgagaagatcctgaccttccgcatcccctactacgtgggccctctggccaggggaaacagcagattcgcctggatgaccagaaagagcgaggaaaccatcaccccctggaacttcgaggaagtggtggacaagggcgccagcgcccagagcttcatcgagcggatgaccaacttcgataagaacctgcccaacgagaaggtgctgcccaagcacagcctgctgtacgagtacttcaccgtgtacaacgagctgaccaaagtgaaatacgtgaccgagggaatgagaaagcccgccttcctgagcggcgagcagaaaaaagccatcgtggacctgctgttcaagaccaaccggaaagtgaccgtgaagcagctgaaagaggactacttcaagaaaatcgagtgcttcgactccgtggaaatctccggcgtggaagatcggttcaacgcctccctgggcacataccacgatctgctgaaaattatcaaggacaaggacttcctggacaatgaggaaaacgaggacattctggaagatatcgtgctgaccctgacactgtttgaggacagagagatgatcgaggaacggctgaaaacctatgcccacctgttcgacgacaaagtgatgaagcagctgaagcggcggagatacaccggctggggcaggctgagccggaagctgatcaacggcatccgggacaagcagtccggcaagacaatcctggatttcctgaagtccgacggcttcgccaacagaaacttcatgcagctgatccacgacgacagcctgacctttaaagaggacatccagaaagcccaggtgtccggccagggcgatagcctgcacgagcacattgccaatctggccggcagccccgccattaagaagggcatcctgcagacagtgaaggtggtggacgagctcgtgaaagtgatgggccggcacaagcccgagaacatcgtgatcgaaatggccagagagaaccagaccacccagaagggacagaagaacagccgcgagagaatgaagcggatcgaagagggcatcaaagagctgggcagccagatcctgaaagaacaccccgtggaaaacacccagctgcagaacgagaagctgtacctgtactacctgcagaatgggcgggatatgtacgtggaccaggaactggacatcaaccggctgtccgactacgatgtggacgctatcgtgcctcagagctttctgaaggacgactccatcgataacaaagtgctgactcggagcgacaagaaccggggcaagagcgacaacgtgccctccgaagaggtcgtgaagaagatgaagaactactggcgccagctgctgaatgccaagctgattacccagaggaagttcgacaatctgaccaaggccgagagaggcggcctgagcgaactggataaggccggcttcatcaagagacagctggtggaaacccggcagatcacaaagcacgtggcacagatcctggactcccggatgaacactaagtacgacgagaacgacaaactgatccgggaagtgaaagtgatcaccctgaagtccaagctggtgtccgatttccggaaggatttccagttttacaaagtgcgcgagatcaacaactaccaccacgcccacgacgcctacctgaacgccgtcgtgggaaccgccctgatcaaaaagtaccctaagctggaaagcgagttcgtgtacggcgactacaaggtgtacgacgtgcggaagatgatcgccaagagcgagcaggaaatcggcaaggctaccgccaagtacttcttctacagcaacatcatgaactttttcaagaccgagattaccctggccaacggcgagatccggaagcggcctctgatcgagacaaacggcgaaacaggcgagatcgtgtgggataagggccgggactttgccaccgtgcggaaagtgctgtctatgccccaagtgaatatcgtgaaaaagaccgaggtgcagacaggcggcttcagcaaagagtctatcctgcccaagaggaacagcgacaagctgatcgccagaaagaaggactgggaccctaagaagtacggcggcttcgacagccccaccgtggcctattctgtgctggtggtggccaaagtggaaaagggcaagtccaagaaactgaagagtgtgaaagagctgctggggatcaccatcatggaaagaagcagcttcgagaagaatcccatcgactttctggaagccaagggctacaaagaagtgaaaaaggacctgatcatcaagctgcctaagtactccctgttcgagctggaaaacggccggaagagaatgctggcctctgccggcgaactgcagaagggaaacgaactggccctgccctccaaatatgtgaacttcctgtacctggccagccactatgagaagctgaagggctcccccgaggataatgagcagaaacagctgtttgtggaacagcacaaacactacctggacgagatcatcgagcagatcagcgagttctccaagagagtgatcctggccgacgctaatctggacaaggtgctgagcgcctacaacaagcacagagacaagcctatcagagagcaggccgagaatatcatccacctgtttaccctgaccaatctgggagcccctgccgccttcaagtactttgacaccaccatcgaccggaagaggtacaccagcaccaaagaggtgctggacgccaccctgatccaccagagcatcaccggcctgtacgagacacggatcgacctgtctcagctgggaggcgacgcctatccctatgacgtgcccgattatgccagcctgggcagcggctcccccaagaaaaaacgcaaggtggaagatcctaagaaaaagcggaaagtggacggcagcggcagcgagacccccggtaccagcgagagcgccacccccgagagcatgaacaattcccagggaagagtgaccttcgaggatgtcactgtgaacttcacccagggggagtggcagcggctgaatcccgaacagagaaacttgtacagggatgtgatgctggagaattacagcaaccttgtctctgtgggacaaggggaaaccaccaaacccgatgtgatcttgaggttggaacaaggaaaggagccatggttggaggaagaggaagtgctgggaagtggccgtgcagaaaaaaatggggacattggagggcagatttggaagccaaaggatgtgaaagagagtctcctcgagggaagcggagctactaacttcagcctgctgaagcaggctggagacgtggaggagaaccctggacctatgcctgctgctaagagagtgaaactggatggatccaaccatgaccaggaatttgaccccccaaaggtttacccacctgtgccagctgagaagaggaagcccatccgcgtgctgtctctctttgatgggattgctacagggctcctggtgctgaaggacctgggcatccaagtggaccgctacattgcctccgaggtgtgtgaggactccatcacggtgggcatggtgcggcaccagggaaagatcatgtacgtcggggacgtccgcagcgtcacacagaagcatatccaggagtggggcccattcgacctggtgattggaggcagtccctgcaatgacctctccattgtcaaccctgcccgcaagggactttatgagggtactggccgcctcttctttgagttctaccgcctcctgcatgatgcgcggcccaaggagggagatgatcgccccttcttctggctctttgagaatgtggtggccatgggcgttagtgacaagagggacatctcgcgatttcttgagtctaaccccgtgatgattgacgccaaagaagtgtctgctgcacacagggcccgttacttctggggtaaccttcctggcatgaacaggcctttggcatccactgtgaatgataagctggagctgcaagagtgtctggagcacggcagaatagccaagttcagcaaagtgaggaccattaccaccaggtcaaactctataaagcagggcaaagaccagcatttccccgtgttcatgaacgagaaggaggacatcctgtggtgcactgaaatggaaagggtgtttggcttccccgtccactacacagacgtctccaacatgagccgcttggcgaggcagagactgctgggccgatcgtggagcgtgccggtcatccgccacctcttcgctccgctgaaggaatattttgcttgtgtgtctagcggcaatagtaacgctaacagccgcgggccgagcttcagcagcggcctggtgccgttaagcttgcgcggcagccatatgttcgaaaccgtgcctgtgtggaggagacagccagtccgggtgctgtccctttttgaagacatcaagaaagagctgacgagtttgggctttttggaaagtggttctgacccgggacaactgaagcatgtggttgatgtcacagacacagtgaggaaggatgtggaggagtggggacccttcgatcttgtgtacggcgccacacctcccctgggccacacctgtgaccgtcctcccagctggtacctgttccagttccaccggctcctgcagtacgcacggcccaagccaggcagccccaggcccttcttctggatgttcgtggacaatctggtgctgaacaaggaagacctggacgtcgcatctcgcttcctggagatggagccagtcaccatcccagatgtccacggcggatccttgcagaatgctgtccgcgtgtggagcaacatcccagccataaggagcagcaggcactgggctctggtttcggaagaagaattgtccctgctggcccagaacaagcagagctcgaagctcgcggccaagtggcccaccaagctggtgaagaactgctttctccccctaagagaatatttcaagtatttttcaggagggccgagctctggcgcacccccaccaagtggagggtctcctgccgggtccccaacatctactgaagaaggcaccagcgaatccgcaacgcccgagtcaggccctggtacctccacagaaccatctgaaggtagtgcgcctggttccccagctggaagccctacttccaccgaagaaggcacgtcaaccgaaccaagtgaaggatctgcccctgggaccagcactgaaccatctgagccaaaaaagaagagaaaggtaccatctgagatgtccaagggagaggagctgttcaccggagtggtgccaatcctggtggagctggacggcgatgtgaacggccacaagttttctgtgcgcggagagggagagggcgacgcaaccatcggcaagctgacactgaagttcatctgcaccacaggcaagctgcccgtgccttggccaaccctggtgaccacactgacatacggcgtgcagtgtttctctaggtatccagaccacatgaagagacacgatttctttaagagcgccatgccagagggatacgtgcaggagcggaccatctccttcaaggacgatggcaagtataagacccgcgccgtggtgaagtttgagggcgatacactggtgaacaggatcgagctgaagggcaccgacttcaaggaggatggcaatatcctgggccacaagctggagtacaactttaatagccacaacgtgtatatcacagccgacaagcagaagaacggcatcaaggccaacttcaccgtgaggcacaatgtggaggacggctccgtgcagctggccgatcactaccagcagaacacacctatcggcgacggacccgtgctgctgcctgataatcactatctgtccacccagacagtgctgtctaaggacccaaacgagaagtgataataggatcccaagcacgcagcaatgcagctcaaaacgcttagcctagccacacccccacgggaaacagcagtgattaacctttagcaataaacgaaagtttaactaagctatactaaccccagggttggtcaatttcgtgccagccacaccctggtactgcatgcacgcaatgctagctgcccctttcccgtcctgggcaccccgagtctcccccgaccccgggtcccaggtatgctcccacctccacctgccccactcaccacctctgctagttccagacacctccgagacgaggaaaaaaaaaaaaaaaaaaaaaaaaaaaaaaaaaaaaaaaaaaaaaaaaaaaaaaaaaaaaaaaaaaaaaaaaaaaaaaaaaaaaaaaaaaaaaaaaaaaaaaaaaaaaaaaaaaaaaaaaaaaaaaaaaaaaaaaaaaaaaaaaaaaaaaaaaaaaaaaaaaaaaaaaaaaaaaaaaaaaaaaaaaaaaaaaaaaaaaaaaaaaaaaaaaaaaaaaaaaaaaaaaaaaaaaaaaaaaaaaaaaaaaaaaaaaaaaaaaaaaaaaaaaaaaaaaaaaaaaaaaaaaaaaaaaaaaaaaaaaaaaaaaaaaaaaaaaaaaaaaaaaaaaaaaaaaaaaaaaaaaaaaaaaaaaaaaaaaaaaaaaaaaaaaaaaaaaaaaaaaaaaaaaaaaaaaaccgtcttcaagctttctagaaattcactggccgtcgttttacaacgtcgtgactgggaaaaccctggcgttacccaacttaatcgccttgcagcacatccccctttcgccagctggcgtaatagcgaagaggcccgcaccgatcgcccttcccaacagttgcgcagcctgaatggcgaatggcgcctgatgcggtattttctccttacgcatctgtgcggtatttcacaccgcatatggtgcactctcagtacaatctgctctgatgccgcatagttaagccagccccgacacccgccaacacccgctgacgcgccctgacgggcttgtctgctcccggcatccgcttacagacaagctgtgaccgtctccgggagctgcatgtgtcagaggttttcaccgtcatcaccgaaacgcgcgagacgaaagggcctcgtgatacgcctatttttataggttaatgtcatgataataatggtttcttagacgtcaggtggcacttttcggggaaatgtgcgcggaacccctatttgtttatttttctaaatacattcaaatatgtatccgctcatgagacaataaccctgataaatgcttcaataatattgaaaaaggaagagtatgagtattcaacatttccgtgtcgcccttattcccttttttgcggcattttgccttcctgtttttgctcacccagaaacgctggtgaaagtaaaagatgctgaagatcagttgggtgcacgagtgggttacatcgaactggatctcaacagcggtaagatccttgagagttttcgccccgaagaacgttttccaatgatgagcacttttaaagttctgctatgtggcgcggtattatcccgtattgacgccgggcaagagcaactcggtcgccgcatacactattctcagaatgacttggttgagtactcaccagtcacagaaaagcatcttacggatggcatgacagtaagagaattatgcagtgctgccataaccatgagtgataacactgcggccaacttacttctgacaacgatcggaggaccgaaggagctaaccgcttttttgcacaacatgggggatcatgtaactcgccttgatcgttgggaaccggagctgaatgaagccataccaaacgacgagcgtgacaccacgatgcctgtagcaatggcaacaacgttgcgcaaactattaactggcgaactacttactctagcttcccggcaacaattaatagactggatggaggcggataaagttgcaggaccacttctgcgctcggcccttccggctggctggtttattgctgataaatctggagccggtgagcgtgggtctcgcggtatcattgcagcactggggccagatggtaagccctcccgtatcgtagttatctacacgacggggagtcaggcaactatggatgaacgaaatagacagatcgc

SEQ ID NO: 239 - DNA, 10635 bp, synthetic construct
  misc_feature 1..10635: note = DNA of V45_D3a-D3l-1xGFP11-2a-GFP1-10-dCas9-KRAB
  source 1..10635: mol_type = other DNA
atcgtgctgaccctgacactgtttgaggacagagagatgatcgaggaacggctgaaaacctatgcccacctgttcgacgacaaagtgatgaagcagctgaagcggcggagatacaccggctggggcaggctgagccggaagctgatcaacggcatccgggacaagcagtccggcaagacaatcctggatttcctgaagtccgacggcttcgccaacagaaacttcatgcagctgatccacgacgacagcctgacctttaaagaggacatccagaaagcccaggtgtccggccagggcgatagcctgcacgagcacattgccaatctggccggcagccccgccattaagaagggcatcctgcagacagtgaaggtggtggacgagctcgtgaaagtgatgggccggcacaagcccgagaacatcgtgatcgaaatggccagagagaaccagaccacccagaagggacagaagaacagccgcgagagaatgaagcggatcgaagagggcatcaaagagctgggcagccagatcctgaaagaacaccccgtggaaaacacccagctgcagaacgagaagctgtacctgtactacctgcagaatgggcgggatatgtacgtggaccaggaactggacatcaaccggctgtccgactacgatgtggacgctatcgtgcctcagagctttctgaaggacgactccatcgataacaaagtgctgactcggagcgacaagaaccggggcaagagcgacaacgtgccctccgaagaggtcgtgaagaagatgaagaactactggcgccagctgctgaatgccaagctgattacccagaggaagttcgacaatctgaccaaggccgagagaggcggcctgagcgaactggataaggccggcttcatcaagagacagctggtggaaacccggcagatcacaaagcacgtggcacagatcctggactcccggatgaacactaagtacgacgagaacgacaaactgatccgggaagtgaaagtgatcaccctgaagtccaagctggtgtccgatttccggaaggatttccagttttacaaagtgcgcgagatcaacaactaccaccacgcccacgacgcctacctgaacgccgtcgtgggaaccgccctgatcaaaaagtaccctaagctggaaagcgagttcgtgtacggcgactacaaggtgtacgacgtgcggaagatgatcgccaagagcgagcaggaaatcggcaaggctaccgccaagtacttcttctacagcaacatcatgaactttttcaagaccgagattaccctggccaacggcgagatccggaagcggcctctgatcgagacaaacggcgaaacaggcgagatcgtgtgggataagggccgggactttgccaccgtgcggaaagtgctgtctatgccccaagtgaatatcgtgaaaaagaccgaggtgcagacaggcggcttcagcaaagagtctatcctgcccaagaggaacagcgacaagctgatcgccagaaagaaggactgggaccctaagaagtacggcggcttcgacagccccaccgtggcctattctgtgctggtggtggccaaagtggaaaagggcaagtccaagaaactgaagagtgtgaaagagctgctggggatcaccatcatggaaagaagcagcttcgagaagaatcccatcgactttctggaagccaagggctacaaagaagtgaaaaaggacctgatcatcaagctgcctaagtactccctgttcgagctggaaaacggccggaagagaatgctggcctctgccggcgaactgcagaagggaaacgaactggccctgccctccaaatatgtgaacttcctgtacctggccagccactatgagaagctgaagggctcccccgaggataatgagcagaaacagctgtttgtggaacagcacaaacactacctggacgagatcatcgagcagatcagcgagttctccaagagagtgatcctggccgacgctaatctggacaaggtgctgagcgcctacaacaagcacagagacaagcctatcagagagcaggccgagaatatcatccacctgtttaccctgaccaatctgggagcccctgccgccttcaagtactttgacaccaccatcgaccggaagaggtacaccagcaccaaagaggtgctggacgccaccctgatccaccagagcatcaccggcctgtacgagacacggatcgacctgtctcagctgggaggcgacgcctatccctatgacgtgcccgattatgccagcctgggcagcggctcccccaagaaaaaacgcaaggtggaagatcctaagaaaaagcggaaagtggacggcagcggcagcgagacccccggtaccagcgagagcgccacccccgagagccggacactggtgaccttcaaggatgtatttgtggacttcaccagggaggagtggaagctgctggacactgctcagcagatcgtgtacagaaatgtgatgctggagaactataagaacctggtttccttgggttatcagcttactaagccagatgtgatcctccggttggagaagggagaagagccctgagatcccaagcacgcagcaatgcagctcaaaacgcttagcctagccacacccccacgggaaacagcagtgattaacctttagcaataaacgaaagtttaactaagctatactaaccccagggttggtcaatttcgtgccagccacaccctggtactgcatgcacgcaatgctagctgcccctttcccgtcctgggcaccccgagtctcccccgaccccgggtcccaggtatgctcccacctccacctgccccactcaccacctctgctagttccagacacctccgagacgaggaaaaaaaaaaaaaaaaaaaaaaaaaaaaaaaaaaaaaaaaaaaaaaaaaaaaaaaaaaaaaaaaaaaaaaaaaaaaaaaaaaaaaaaaaaaaaaaaaaaaaaaaaaaaaaaaaaaaaaaaaaaaaaaaaaaaaaaaaaaaaaaaaaaaaaaaaaaaaaaaaaaaaaaaaaaaaaaaaaaaaaaaaaaaaaaaaaaaaaaaaaaaaaaaaaaaaaaaaaaaaaaaaaaaaaaaaaaaaaaaaaaaaaaaaaaaaaaaaaaaaaaaaaaaaaaaaaaaaaaaaaaaaaaaaaaaaaaaaaaaaaaaaaaaaaaaaaaaaaaaaaaaaaaaaaaaaaaaaaaaaaaaaaaaaaaaaaaaaaaaaaaaaaaaaaaaaaaaaaaaaaaaaaaaaaaaaaccgtcttcaagctttctagaaattcactggccgtcgttttacaacgtcgtgactgggaaaaccctggcgttacccaacttaatcgccttgcagcacatccccctttcgccagctggcgtaatagcgaagaggcccgcaccgatcgcccttcccaacagttgcgcagcctgaatggcgaatggcgcctgatgcggtattttctccttacgcatctgtgcggtatttcacaccgcatatggtgcactctcagtacaatctgctctgatgccgcatagttaagccagccccgacacccgccaacacccgctgacgcgccctgacgggcttgtctgctcccggcatccgcttacagacaagctgtgaccgtctccgggagctgcatgtgtcagaggttttcaccgtcatcaccgaaacgcgcgagacgaaagggcctcgtgatacgcctatttttataggttaatgtcatgataataatggtttcttagacgtcaggtggcacttttcggggaaatgtgcgcggaacccctatttgtttatttttctaaatacattcaaatatgtatccgctcatgagacaataaccctgataaatgcttcaataatattgaaaaaggaagagtatgagtattcaacatttccgtgtcgcccttattcccttttttgcggcattttgccttcctgtttttgctcacccagaaacgctggtgaaagtaaaagatgctgaagatcagttgggtgcacgagtgggttacatcgaactggatctcaacagcggtaagatccttgagagttttcgccccgaagaacgttttccaatgatgagcacttttaaagttctgctatgtggcgcggtattatcccgtattgacgccgggcaagagcaactcggtcgccgcatacactattctcagaatgacttggttgagtactcaccagtcacagaaaagcatcttacggatggcatgacagtaagagaattatgcagtgctgccataaccatgagtgataacactgcggccaacttacttctgacaacgatcggaggaccgaaggagctaaccgcttttttgcacaacatgggggatcatgtaactcgccttgatcgttgggaaccggagctgaatgaagccataccaaacgacgagcgtgacaccacgatgcctgtagcaatggcaacaacgttgcgcaaactattaactggcgaactacttactctagcttcccggcaacaattaatagactggatggaggcggataaagttgcaggaccacttctgcgctcggcccttccggctggctggtttattgctgataaatctggagccggtgagcgtgggtctcgcggtatcattgcagcactggggccagatggtaagccctcccgtatcgtagttatctacacgacggggagtcaggcaactatggatgaacgaaatagacagatcgctgagataggtgcctcactgattaagcattggtaactgtcagaccaagtttactcatatatactttagattgatttaaaacttcatttttaatttaaaaggatctaggtgaagatcctttttgataatctcatgaccaaaatcccttaacgtgagttttcgttccactgagcgtcagaccccgtagaaaagatcaaaggatcttcttgagatcctttttttctgcgcgtaatctgctgcttgcaaacaaaaaaaccaccgctaccagcggtggtttgtttgccggatcaagagctaccaactctttttccgaaggtaactggcttcagcagagcgcagataccaaatactgttcttctagtgtagccgtagttaggccaccacttcaagaactctgtagcaccgcctacatacctcgctctgctaatcctgttaccagtggctgctgccagtggcgataagtcgtgtcttaccgggttggactcaagacgatagttaccggataaggcgcagcggtcgggctgaacggggggttcgtgcacacagcccagcttggagcgaacgacctacaccgaactgagatacctacagcgtgagctatgagaaagcgccacgcttcccgaagggagaaaggcggacaggtatccggtaagcggcagggtcggaacaggagagcgcacgagggagcttccagggggaaacgcctggtatctttatagtcctgtcgggtttcgccacctctgacttgagcgtcgatttttgtgatgctcgtcaggggggcggagcctatggaaaaacgccagcaacgcggcctttttacggttcctggccttttgctggccttttgctcacatgttctttcctgcgttatcccctgattctgtggataaccgtattaccgcctttgagtgagctgataccgctcgccgcagccgaacgaccgagcgcagcgagtcagtgagcgaggaagcggaagagcgcccaatacgcaaaccgcctctccccgcgcgttggccgattcattaatgcagctggcacgacaggtttcccgactggaaagcgggcagtgagcgcaacgcaattaatgtgagttagctcactcattaggcaccccaggctttacactttatgcttccggctcgtatgttgtgtggaattgtgagcggataacaatttcacacaggaaacagctatgaccatgattacgcctctagaaagctttaatacgactcactataaggactcactatttgttttcgcgcccagttgcaaaaagtgtcgacatttgcttctgacacaactgtgttcactagcaacctcaaacagacaccgccaccatgcctgctgctaagagagtgaaactggatggatccaaccatgaccaggaatttgaccccccaaaggtttacccacctgtgccagctgagaagaggaagcccatccgcgtgctgtctctctttgatgggattgctacagggctcctggtgctgaaggacctgggcatccaagtggaccgctacattgcctccgaggtgtgtgaggactccatcacggtgggcatggtgcggcaccagggaaagatcatgtacgtcggggacgtccgcagcgtcacacagaagcatatccaggagtggggcccattcgacctggtgattggaggcagtccctgcaatgacctctccattgtcaaccctgcccgcaagggactttatgagggtactggccgcctcttctttgagttctaccgcctcctgcatgatgcgcggcccaaggagggagatgatcgccccttcttctggctctttgagaatgtggtggccatgggcgttagtgacaagagggacatctcgcgatttcttgagtctaaccccgtgatgattgacgccaaagaagtgtctgctgcacacagggcccgttacttctggggtaaccttcctggcatgaacaggcctttggcatccactgtgaatgataagctggagctgcaagagtgtctggagcacggcagaatagccaagttcagcaaagtgaggaccattaccaccaggtcaaactctataaagcagggcaaagaccagcatttccccgtgttcatgaacgagaaggaggacatcctgtggtgcactgaaatggaaagggtgtttggcttccccgtccactacacagacgtctccaacatgagccgcttggcgaggcagagactgctgggccgatcgtggagcgtgccggtcatccgccacctcttcgctccgctgaaggaatattttgcttgtgtgtctagcggcaatagtaacgctaacagccgcgggccgagcttcagcagcggcctggtgccgttaagcttgcgcggcagccatatgggccctatggagatatacaagacagtgtctgcatggaagagacagccagtgcgggtactgagcctcttcagaaacatcgacaaggtactaaagagtttgggcttcttggaaagcggttctggttctgggggaggaacgctgaagtacgtggaagatgtcacaaatgtcgtgaggagagacgtggagaaatggggcccctttgacctggtgtacggctcgacgcagcccctaggcagctcttgtgatcgctgtcccggctggtacatgttccagttccaccggatcctgcagtatgcgctgcctcgccaggagagtcagcggcccttcttctggatattcatggacaatctgctgctgactgaggatgaccaagagacaactacccgcttccttcagacagaggctgtgaccctccaggatgtccgtggcagagactaccagaatgctatgcgggtgtggagcaacattccagggctgaagagcaagcatgcgcccctgaccccaaaggaagaagagtatctgcaagcccaagtcagaagcaggagcaagctggacgccccgaaagttgacctcctggtgaagaactgccttctcccgctgagagagtacttcaagtatttttctcaaaactcacttcctcttggagggccgagctctggcgcacccccaccaagtggagggtctcctgccgggtccccaacatctactgaagaaggcaccagcgaatccgcaacgggcggtagcggcggtcgggaccatatggtcctgcacgaatatgtcaatgctgccggtatcaccgcggccgcaaggtcaggctccggccagcggggaagcaagcgcaccgccgatggttccgagttcgaaagccccaaaaaaaagcgcaaggtcggaagcggagctactaacttcagcctgctgaagcaggctggagacgtggaggagaaccctggacctatgcctgctgctaagagagtgaaactggatggatccggccccgacatcgtgatgtccaagggagaggagctgttcaccggagtggtgccaatcctggtggagctggacggcgatgtgaacggccacaagttttctgtgcgcggagagggagagggcgacgcaaccatcggcaagctgacactgaagttcatctgcaccacaggcaagctgcccgtgccttggccaaccctggtgaccacactgacatacggcgtgcagtgtttctctaggtatccagaccacatgaagagacacgatttctttaagagcgccatgccagagggatacgtgcaggagcggaccatctccttcaaggacgatggcaagtataagacccgcgccgtggtgaagtttgagggcgatacactggtgaacaggatcgagctgaagggcaccgacttcaaggaggatggcaatatcctgggccacaagctggagtacaactttaatagccacaacgtgtatatcacagccgacaagcagaagaacggcatcaaggccaacttcaccgtgaggcacaatgtggaggacggctccgtgcagctggccgatcactaccagcagaacacacctatcggcgacggacccgtgctgctgcctgataatcactatctgtccacccagacagtgctgtctaaggacccaaacgagaagttggatccaggtggaggcggaagcggaagcggaccaaaaaagaagagaaaggtaatggacaagaagtacagcatcggcctggccatcggcaccaactctgtgggctgggccgtgatcaccgacgagtacaaggtgcccagcaagaaattcaaggtgctgggcaacaccgaccggcacagcatcaagaagaacctgatcggcgccctgctgttcgacagcggagaaacagccgaggccacccggctgaagagaaccgccagaagaagatacaccagacggaagaaccggatctgctatctgcaagagatcttcagcaacgagatggccaaggtggacgacagcttcttccacagactggaagagtccttcctggtggaagaggataagaagcacgagcggcaccccatcttcggcaacatcgtggacgaggtggcctaccacgagaagtaccccaccatctaccacctgagaaagaaactggtggacagcaccgacaaggccgacctgcggctgatctatctggccctggcccacatgatcaagttccggggccacttcctgatcgagggcgacctgaaccccgacaacagcgacgtggacaagctgttcatccagctggtgcagacctacaaccagctgttcgaggaaaaccccatcaacgccagcggcgtggacgccaaggccatcctgtctgccagactgagcaagagcagacggctggaaaatctgatcgcccagctgcccggcgagaagaagaatggcctgttcggcaacctgattgccctgagcctgggcctgacccccaacttcaagagcaacttcgacctggccgaggatgccaaactgcagctgagcaaggacacctacgacgacgacctggacaacctgctggcccagatcggcgaccagtacgccgacctgtttctggccgccaagaacctgtccgacgccatcctgctgagcgacatcctgagagtgaacaccgagatcaccaaggcccccctgagcgcctctatgatcaagagatacgacgagcaccaccaggacctgaccctgctgaaagctctcgtgcggcagcagctgcctgagaagtacaaagagattttcttcgaccagagcaagaacggctacgccggctacatcgatggcggagccagccaggaagagttctacaagttcatcaagcccatcctggaaaagatggacggcaccgaggaactgctcgtgaagctgaacagagaggacctgctgcggaagcagcggaccttcgacaacggcagcatcccccaccagatccacctgggagagctgcacgccattctgcggcggcaggaagatttttacccattcctgaaggacaaccgggaaaagatcgagaagatcctgaccttccgcatcccctactacgtgggccctctggccaggggaaacagcagattcgcctggatgaccagaaagagcgaggaaaccatcaccccctggaacttcgaggaagtggtggacaagggcgccagcgcccagagcttcatcgagcggatgaccaacttcgataagaacctgcccaacgagaaggtgctgcccaagcacagcctgctgtacgagtacttcaccgtgtacaacgagctgaccaaagtgaaatacgtgaccgagggaatgagaaagcccgccttcctgagcggcgagcagaaaaaagccatcgtggacctgctgttcaagaccaaccggaaagtgaccgtgaagcagctgaaagaggactacttcaagaaaatcgagtgcttcgactccgtggaaatctccggcgtggaagatcggttcaacgcctccctgggcacataccacgatctgctgaaaattatcaaggacaaggacttcctggacaatgaggaaaacgaggacattctggaagat

SEQ ID NO: 240 - DNA, 11442 bp, synthetic construct
  misc_feature 1..11442: note = DNA of V46_10xGFP11-dCas9-ZIM3-2a-D3a-hD3L-GFP1-10
  source 1..11442: mol_type = other DNA
tgagataggtgcctcactgattaagcattggtaactgtcagaccaagtttactcatatatactttagattgatttaaaacttcatttttaatttaaaaggatctaggtgaagatcctttttgataatctcatgaccaaaatcccttaacgtgagttttcgttccactgagcgtcagaccccgtagaaaagatcaaaggatcttcttgagatcctttttttctgcgcgtaatctgctgcttgcaaacaaaaaaaccaccgctaccagcggtggtttgtttgccggatcaagagctaccaactctttttccgaaggtaactggcttcagcagagcgcagataccaaatactgttcttctagtgtagccgtagttaggccaccacttcaagaactctgtagcaccgcctacatacctcgctctgctaatcctgttaccagtggctgctgccagtggcgataagtcgtgtcttaccgggttggactcaagacgatagttaccggataaggcgcagcggtcgggctgaacggggggttcgtgcacacagcccagcttggagcgaacgacctacaccgaactgagatacctacagcgtgagctatgagaaagcgccacgcttcccgaagggagaaaggcggacaggtatccggtaagcggcagggtcggaacaggagagcgcacgagggagcttccagggggaaacgcctggtatctttatagtcctgtcgggtttcgccacctctgacttgagcgtcgatttttgtgatgctcgtcaggggggcggagcctatggaaaaacgccagcaacgcggcctttttacggttcctggccttttgctggccttttgctcacatgttctttcctgcgttatcccctgattctgtggataaccgtattaccgcctttgagtgagctgataccgctcgccgcagccgaacgaccgagcgcagcgagtcagtgagcgaggaagcggaagagcgcccaatacgcaaaccgcctctccccgcgcgttggccgattcattaatgcagctggcacgacaggtttcccgactggaaagcgggcagtgagcgcaacgcaattaatgtgagttagctcactcattaggcaccccaggctttacactttatgcttccggctcgtatgttgtgtggaattgtgagcggataacaatttcacacaggaaacagctatgaccatgattacgcctctagaaagctttaatacgactcactataaggactcactatttgttttcgcgcccagttgcaaaaagtgtcgacatttgcttctgacacaactgtgttcactagcaacctcaaacagacaccgccaccatgcctgctgctaagagagtgaaactggatggatccatgcgtgaccacatggtccttcatgagtatgtaaatgctgctgggattacaggtggctctggaggtagagatcatatggttctccacgaatacgttaacgccgcaggcatcactggcggtagtggaggacgcgaccatatggtactacatgaatatgtcaatgcagccggaataaccggagggtccggaggccgggatcacatggtgctgcatgagtatgtgaacgcggcgggtataactggtgggtcgggcggacgagaccatatggtgcttcacgaatacgtaaacgcagctggcattactggcggatcaggtggcagggatcacatggtactccatgagtacgtgaacgctgctggaatcacaggcggtagcggcggtcgggaccatatggtcctgcacgaatatgtcaatgctgccggtatcaccgcggccgcaggtggctctggaggtagagatcatatggttctccacgaatacgttaacgccgcaggcatcactggcggtagtggaggacgcgaccatatggtactacatgaatatgtcaatgcagccggaataaccggagggtccggaggccgggatcacatggtgctgcatgagtatgtgaacgcggcgggtataactggtgggtcgggcggaaggtcaggctccggccagcggggaagcaagcgcaccgccgatggttccgagttcgaaagccccaaaaaaaagcgcaaggtcggcggaagcggaagcggaccaaaaaagaagagaaaggtaatggacaagaagtacagcatcggcctggccatcggcaccaactctgtgggctgggccgtgatcaccgacgagtacaaggtgcccagcaagaaattcaaggtgctgggcaacaccgaccggcacagcatcaagaagaacctgatcggcgccctgctgttcgacagcggagaaacagccgaggccacccggctgaagagaaccgccagaagaagatacaccagacggaagaaccggatctgctatctgcaagagatcttcagcaacgagatggccaaggtggacgacagcttcttccacagactggaagagtccttcctggtggaagaggataagaagcacgagcggcaccccatcttcggcaacatcgtggacgaggtggcctaccacgagaagtaccccaccatctaccacctgagaaagaaactggtggacagcaccgacaaggccgacctgcggctgatctatctggccctggcccacatgatcaagttccggggccacttcctgatcgagggcgacctgaaccccgacaacagcgacgtggacaagctgttcatccagctggtgcagacctacaaccagctgttcgaggaaaaccccatcaacgccagcggcgtggacgccaaggccatcctgtctgccagactgagcaagagcagacggctggaaaatctgatcgcccagctgcccggcgagaagaagaatggcctgttcggcaacctgattgccctgagcctgggcctgacccccaacttcaagagcaacttcgacctggccgaggatgccaaactgcagctgagcaaggacacctacgacgacgacctggacaacctgctggcccagatcggcgaccagtacgccgacctgtttctggccgccaagaacctgtccgacgccatcctgctgagcgacatcctgagagtgaacaccgagatcaccaaggcccccctgagcgcctctatgatcaagagatacgacgagcaccaccaggacctgaccctgctgaaagctctcgtgcggcagcagctgcctgagaagtacaaagagattttcttcgaccagagcaagaacggctacgccggctacatcgatggcggagccagccaggaagagttctacaagttcatcaagcccatcctggaaaagatggacggcaccgaggaactgctcgtgaagctgaacagagaggacctgctgcggaagcagcggaccttcgacaacggcagcatcccccaccagatccacctgggagagctgcacgccattctgcggcggcaggaagatttttacccattcctgaaggacaaccgggaaaagatcgagaagatcctgaccttccgcatcccctactacgtgggccctctggccaggggaaacagcagattcgcctggatgaccagaaagagcgaggaaaccatcaccccctggaacttcgaggaagtggtggacaagggcgccagcgcccagagcttcatcgagcggatgaccaacttcgataagaacctgcccaacgagaaggtgctgcccaagcacagcctgctgtacgagtacttcaccgtgtacaacgagctgaccaaagtgaaatacgtgaccgagggaatgagaaagcccgccttcctgagcggcgagcagaaaaaagccatcgtggacctgctgttcaagaccaaccggaaagtgaccgtgaagcagctgaaagaggactacttcaagaaaatcgagtgcttcgactccgtggaaatctccggcgtggaagatcggttcaacgcctccctgggcacataccacgatctgctgaaaattatcaaggacaaggacttcctggacaatgaggaaaacgaggacattctggaagatatcgtgctgaccctgacactgtttgaggacagagagatgatcgaggaacggctgaaaacctatgcccacctgttcgacgacaaagtgatgaagcagctgaagcggcggagatacaccggctggggcaggctgagccggaagctgatcaacggcatccgggacaagcagtccggcaagacaatcctggatttcctgaagtccgacggcttcgccaacagaaacttcatgcagctgatccacgacgacagcctgacctttaaagaggacatccagaaagcccaggtgtccggccagggcgatagcctgcacgagcacattgccaatctggccggcagccccgccattaagaagggcatcctgcagacagtgaaggtggtggacgagctcgtgaaagtgatgggccggcacaagcccgagaacatcgtgatcgaaatggccagagagaaccagaccacccagaagggacagaagaacagccgcgagagaatgaagcggatcgaagagggcatcaaagagctgggcagccagatcctgaaagaacaccccgtggaaaacacccagctgcagaacgagaagctgtacctgtactacctgcagaatgggcgggatatgtacgtggaccaggaactggacatcaaccggctgtccgactacgatgtggacgctatcgtgcctcagagctttctgaaggacgactccatcgataacaaagtgctgactcggagcgacaagaaccggggcaagagcgacaacgtgccctccgaagaggtcgtgaagaagatgaagaactactggcgccagctgctgaatgccaagctgattacccagaggaagttcgacaatctgaccaaggccgagagaggcggcctgagcgaactggataaggccggcttcatcaagagacagctggtggaaacccggcagatcacaaagcacgtggcacagatcctggactcccggatgaacactaagtacgacgagaacgacaaactgatccgggaagtgaaagtgatcaccctgaagtccaagctggtgtccgatttccggaaggatttccagttttacaaagtgcgcgagatcaacaactaccaccacgcccacgacgcctacctgaacgccgtcgtgggaaccgccctgatcaaaaagtaccctaagctggaaagcgagttcgtgtacggcgactacaaggtgtacgacgtgcggaagatgatcgccaagagcgagcaggaaatcggcaaggctaccgccaagtacttcttctacagcaacatcatgaactttttcaagaccgagattaccctggccaacggcgagatccggaagcggcctctgatcgagacaaacggcgaaacaggcgagatcgtgtgggataagggccgggactttgccaccgtgcggaaagtgctgtctatgccccaagtgaatatcgtgaaaaagaccgaggtgcagacaggcggcttcagcaaagagtctatcctgcccaagaggaacagcgacaagctgatcgccagaaagaaggactgggaccctaagaagtacggcggcttcgacagccccaccgtggcctattctgtgctggtggtggccaaagtggaaaagggcaagtccaagaaactgaagagtgtgaaagagctgctggggatcaccatcatggaaagaagcagcttcgagaagaatcccatcgactttctggaagccaagggctacaaagaagtgaaaaaggacctgatcatcaagctgcctaagtactccctgttcgagctggaaaacggccggaagagaatgctggcctctgccggcgaactgcagaagggaaacgaactggccctgccctccaaatatgtgaacttcctgtacctggccagccactatgagaagctgaagggctcccccgaggataatgagcagaaacagctgtttgtggaacagcacaaacactacctggacgagatcatcgagcagatcagcgagttctccaagagagtgatcctggccgacgctaatctggacaaggtgctgagcgcctacaacaagcacagagacaagcctatcagagagcaggccgagaatatcatccacctgtttaccctgaccaatctgggagcccctgccgccttcaagtactttgacaccaccatcgaccggaagaggtacaccagcaccaaagaggtgctggacgccaccctgatccaccagagcatcaccggcctgtacgagacacggatcgacctgtctcagctgggaggcgacgcctatccctatgacgtgcccgattatgccagcctgggcagcggctcccccaagaaaaaacgcaaggtggaagatcctaagaaaaagcggaaagtggacggcagcggcagcgagacccccggtaccagcgagagcgccacccccgagagcatgaacaattcccagggaagagtgaccttcgaggatgtcactgtgaacttcacccagggggagtggcagcggctgaatcccgaacagagaaacttgtacagggatgtgatgctggagaattacagcaaccttgtctctgtgggacaaggggaaaccaccaaacccgatgtgatcttgaggttggaacaaggaaaggagccatggttggaggaagaggaagtgctgggaagtggccgtgcagaaaaaaatggggacattggagggcagatttggaagccaaaggatgtgaaagagagtctcctcgagggaagcggagctactaacttcagcctgctgaagcaggctggagacgtggaggagaaccctggacctatgcctgctgctaagagagtgaaactggatggatccaaccatgaccaggaatttgaccccccaaaggtttacccacctgtgccagctgagaagaggaagcccatccgcgtgctgtctctctttgatgggattgctacagggctcctggtgctgaaggacctgggcatccaagtggaccgctacattgcctccgaggtgtgtgaggactccatcacggtgggcatggtgcggcaccagggaaagatcatgtacgtcggggacgtccgcagcgtcacacagaagcatatccaggagtggggcccattcgacctggtgattggaggcagtccctgcaatgacctctccattgtcaaccctgcccgcaagggactttatgagggtactggccgcctcttctttgagttctaccgcctcctgcatgatgcgcggcccaaggagggagatgatcgccccttcttctggctctttgagaatgtggtggccatgggcgttagtgacaagagggacatctcgcgatttcttgagtctaaccccgtgatgattgacgccaaagaagtgtctgctgcacacagggcccgttacttctggggtaaccttcctggcatgaacaggcctttggcatccactgtgaatgataagctggagctgcaagagtgtctggagcacggcagaatagccaagttcagcaaagtgaggaccattaccaccaggtcaaactctataaagcagggcaaagaccagcatttccccgtgttcatgaacgagaaggaggacatcctgtggtgcactgaaatggaaagggtgtttggcttccccgtccactacacagacgtctccaacatgagccgcttggcgaggcagagactgctgggccgatcgtggagcgtgccggtcatccgccacctcttcgctccgctgaaggaatattttgcttgtgtgtctagcggcaatagtaacgctaacagccgcgggccgagcttcagcagcggcctggtgccgttaagcttgcgcggcagccatatgttcgaaaccgtgcctgtgtggaggagacagccagtccgggtgctgtccctttttgaagacatcaagaaagagctgacgagtttgggctttttggaaagtggttctgacccgggacaactgaagcatgtggttgatgtcacagacacagtgaggaaggatgtggaggagtggggacccttcgatcttgtgtacggcgccacacctcccctgggccacacctgtgaccgtcctcccagctggtacctgttccagttccaccggctcctgcagtacgcacggcccaagccaggcagccccaggcccttcttctggatgttcgtggacaatctggtgctgaacaaggaagacctggacgtcgcatctcgcttcctggagatggagccagtcaccatcccagatgtccacggcggatccttgcagaatgctgtccgcgtgtggagcaacatcccagccataaggagcagcaggcactgggctctggtttcggaagaagaattgtccctgctggcccagaacaagcagagctcgaagctcgcggccaagtggcccaccaagctggtgaagaactgctttctccccctaagagaatatttcaagtatttttcaggagggccgagctctggcgcacccccaccaagtggagggtctcctgccgggtccccaacatctactgaagaaggcaccagcgaatccgcaacgcccgagtcaggccctggtacctccacagaaccatctgaaggtagtgcgcctggttccccagctggaagccctacttccaccgaagaaggcacgtcaaccgaaccaagtgaaggatctgcccctgggaccagcactgaaccatctgagccaaaaaagaagagaaaggtaccatctgagatgtccaagggagaggagctgttcaccggagtggtgccaatcctggtggagctggacggcgatgtgaacggccacaagttttctgtgcgcggagagggagagggcgacgcaaccatcggcaagctgacactgaagttcatctgcaccacaggcaagctgcccgtgccttggccaaccctggtgaccacactgacatacggcgtgcagtgtttctctaggtatccagaccacatgaagagacacgatttctttaagagcgccatgccagagggatacgtgcaggagcggaccatctccttcaaggacgatggcaagtataagacccgcgccgtggtgaagtttgagggcgatacactggtgaacaggatcgagctgaagggcaccgacttcaaggaggatggcaatatcctgggccacaagctggagtacaactttaatagccacaacgtgtatatcacagccgacaagcagaagaacggcatcaaggccaacttcaccgtgaggcacaatgtggaggacggctccgtgcagctggccgatcactaccagcagaacacacctatcggcgacggacccgtgctgctgcctgataatcactatctgtccacccagacagtgctgtctaaggacccaaacgagaagtgataataggatcccaagcacgcagcaatgcagctcaaaacgcttagcctagccacacccccacgggaaacagcagtgattaacctttagcaataaacgaaagtttaactaagctatactaaccccagggttggtcaatttcgtgccagccacaccctggtactgcatgcacgcaatgctagctgcccctttcccgtcctgggcaccccgagtctcccccgaccccgggtcccaggtatgctcccacctccacctgccccactcaccacctctgctagttccagacacctccgagacgaggaaaaaaaaaaaaaaaaaaaaaaaaaaaaaaaaaaaaaaaaaaaaaaaaaaaaaaaaaaaaaaaaaaaaaaaaaaaaaaaaaaaaaaaaaaaaaaaaaaaaaaaaaaaaaaaaaaaaaaaaaaaaaaaaaaaaaaaaaaaaaaaaaaaaaaaaaaaaaaaaaaaaaaaaaaaaaaaaaaaaaaaaaaaaaaaaaaaaaaaaaaaaaaaaaaaaaaaaaaaaaaaaaaaaaaaaaaaaaaaaaaaaaaaaaaaaaaaaaaaaaaaaaaaaaaaaaaaaaaaaaaaaaaaaaaaaaaaaaaaaaaaaaaaaaaaaaaaaaaaaaaaaaaaaaaaaaaaaaaaaaaaaaaaaaaaaaaaaaaaaaaaaaaaaaaaaaaaaaaaaaaaaaaaaaaaaaaccgtcttcaagctttctagaaattcactggccgtcgttttacaacgtcgtgactgggaaaaccctggcgttacccaacttaatcgccttgcagcacatccccctttcgccagctggcgtaatagcgaagaggcccgcaccgatcgcccttcccaacagttgcgcagcctgaatggcgaatggcgcctgatgcggtattttctccttacgcatctgtgcggtatttcacaccgcatatggtgcactctcagtacaatctgctctgatgccgcatagttaagccagccccgacacccgccaacacccgctgacgcgccctgacgggcttgtctgctcccggcatccgcttacagacaagctgtgaccgtctccgggagctgcatgtgtcagaggttttcaccgtcatcaccgaaacgcgcgagacgaaagggcctcgtgatacgcctatttttataggttaatgtcatgataataatggtttcttagacgtcaggtggcacttttcggggaaatgtgcgcggaacccctatttgtttatttttctaaatacattcaaatatgtatccgctcatgagacaataaccctgataaatgcttcaataatattgaaaaaggaagagtatgagtattcaacatttccgtgtcgcccttattcccttttttgcggcattttgccttcctgtttttgctcacccagaaacgctggtgaaagtaaaagatgctgaagatcagttgggtgcacgagtgggttacatcgaactggatctcaacagcggtaagatccttgagagttttcgccccgaagaacgttttccaatgatgagcacttttaaagttctgctatgtggcgcggtattatcccgtattgacgccgggcaagagcaactcggtcgccgcatacactattctcagaatgacttggttgagtactcaccagtcacagaaaagcatcttacggatggcatgacagtaagagaattatgcagtgctgccataaccatgagtgataacactgcggccaacttacttctgacaacgatcggaggaccgaaggagctaaccgcttttttgcacaacatgggggatcatgtaactcgccttgatcgttgggaaccggagctgaatgaagccataccaaacgacgagcgtgacaccacgatgcctgtagcaatggcaacaacgttgcgcaaactattaactggcgaactacttactctagcttcccggcaacaattaatagactggatggaggcggataaagttgcaggaccacttctgcgctcggcccttccggctggctggtttattgctgataaatctggagccggtgagcgtgggtctcgcggtatcattgcagcactggggccagatggtaagccctcccgtatcgtagttatctacacgacggggagtcaggcaactatggatgaacgaaatagacagatcgc

SEQ ID NO: 241 - DNA, 9980 bp, synthetic construct
  misc_feature 1..9980: note = DNA of V47_scFv-ZIM3-2a-D3a-hD3L-dCas9-1xGCN4
  source 1..9980: mol_type = other DNA
cgaaggtaactggcttcagcagagcgcagataccaaatactgttcttctagtgtagccgtagttaggccaccacttcaagaactctgtagcaccgcctacatacctcgctctgctaatcctgttaccagtggctgctgccagtggcgataagtcgtgtcttaccgggttggactcaagacgatagttaccggataaggcgcagcggtcgggctgaacggggggttcgtgcacacagcccagcttggagcgaacgacctacaccgaactgagatacctacagcgtgagctatgagaaagcgccacgcttcccgaagggagaaaggcggacaggtatccggtaagcggcagggtcggaacaggagagcgcacgagggagcttccagggggaaacgcctggtatctttatagtcctgtcgggtttcgccacctctgacttgagcgtcgatttttgtgatgctcgtcaggggggcggagcctatggaaaaacgccagcaacgcggcctttttacggttcctggccttttgctggccttttgctcacattctagataatacgactcactataaggactcactatttgttttcgcgcccagttgcaaaaagtgtcgacatttgcttctgacacaactgtgttcactagcaacctcaaacagacaccgccaccatggtgcctgccgccaagagagtgaagctggacggaagcggccctgacatcgtgatgacacagagcccttctagcctgagcgccagcgtgggagacagagtgaccatcacctgtagaagcagcacaggcgccgtgaccaccagcaattatgccagctgggtgcaagagaagcccggcaagctgttcaagggactgatcggcggcaccaacaatagagcacctggcgtgccaagcagattcagcggctctctgatcggagacaaggccacactgaccataagcagcctgcagcctgaggacttcgccacctacttttgcgccctgtggtacagcaaccactgggtgttcggccagggcaccaaggtggaactgaaaagaggcggcggaggatctggcggaggtggaagcggaggcggaggttctagtggtggtggcagcgaagtgaaactgctggaaagtggtggcggcctggttcagcctggcggatctctgaaactgagctgtgccgtgtccggcttcagcctgacagattacggcgtgaactgggtccgacaggcccctggaagaggactggaatggatcggagtgatctggggcgacggcatcaccgactacaatagcgccctgaaggaccggttcatcatcagcaaggacaacggcaagaacaccgtgtacctgcagatgagcaaagtgcggagcgacgacacagccctgtactactgtgtgaccggcctgttcgattactggggccagggaacactggtcaccgtgtctagctacccctacgacgtgccagattatgctggtggcggtggtggtagtggtggcggaggaagcggcggaggcggttctggtggcggcggttctcttgatcctggcggtggcggcagcggcatgaacaattctcagggcagagtgacattcgaggacgtgaccgtgaacttcacccaaggcgagtggcagagactgaaccccgagcagagaaacctgtaccgggacgtgatgctggaaaactactccaacctggtgtccgttggccagggcgaaaccaccaagcctgacgtgatcctgagactggaacagggcaaagagccctggctcgaagaggaagaggtgctcggatctggcagagccgagaagaatggcgatattggcggacagatctggaagcccaaggacgtgaaagagagccttggcagcggcgccaccaatttcagcctgctgaaacaggctggcgacgtggaagagaaccccggacctatgcctgccgccaagagagtgaagctggacggcagcaaccacgaccaagagttcgaccctcctaaggtgtaccctcctgtgccagccgagaagcggaagcctatcagagtgctgagcctgttcgacggaatcgccacaggactgctggtgctgaaggatctgggaatccaggtggaccggtatatcgccagcgaagtgtgcgaggacagcatcacagttggcatggttcgacaccagggcaagattatgtacgtgggcgacgtgcggagcgtgacccagaaacacattcaagagtggggccccttcgacctggttatcggcggcagcccttgcaacgatctgagcatcgtgaaccccgccagaaagggcctgtatgaaggcaccggcagactgttcttcgagttctacagactgctgcacgacgccagacctaaagagggcgacgacagaccattcttctggctgttcgagaacgtggtggctatgggcgtgtccgacaagcgggacatcagccggtttctggaaagcaaccccgtgatgatcgacgccaaagaggtgtccgctgctcaccgggccagatacttttggggcaatctgcccggcatgaacagacctctggccagcaccgtgaacgacaagctggaactgcaagagtgcctggaacacggccggatcgccaagtttagcaaagtgcggaccatcaccaccaggtccaacagcatcaagcagggcaaagaccagcacttccccgtgttcatgaatgagaaagaggacatcctgtggtgcaccgagatggaaagagtgttcggcttccctgtgcactacaccgacgtgtccaacatgagcagactggccagacagaggctgctgggcagatcttggagcgtgccagtgatcagacacctgttcgcccctctgaaagaatacttcgcctgcgtgtccagcggcaacagcaacgccaatagcagaggccctagcttcagctctggactggtgcctttgagcctgagaggcagccacatgttcgagacagtgcctgtgtggcggagacagcccgttagagtgctgtccctgtttgaggacatcaagaaagagctgaccagcctgggcttcctggaaagcggatctgatcctggccagctgaagcacgtggtggacgtgaccgataccgtgcggaaggatgtggaagaatggggcccttttgatctggtgtacggcgccacacctcctctgggccacacatgtgatagacctccaagctggtatctgttccagttccaccggctgctgcagtacgctagacccaagcctggaagccccaggcctttcttttggatgttcgtggacaacctggtcctgaacaaagaggacctggacgtcgccagccggttcctcgaaatggaacctgtgacaatccccgacgtgcacggcggatctctgcagaatgctgtcagagtgtggtctaacatccccgccatcagaagcagcagacactgggcccttgtgtccgaggaagaactgtctctgctggcccagaacaagcagagcagcaagctggccgccaagtggcctacaaagctggtcaagaactgcttcctgcctctgcgcgagtacttcaagtatttcagcggcggacctagctctggcgcccctccacctagcggaggatctccagcaggatctcctaccagcaccgaggaaggcacaagcgagtctgccacacctgagtctggccctggcacatctacagagcctagcgagggatctgcccctggatctcctgctggcagccctacatctaccgaagagggaaccagcacagagccttccgaaggttctgctcctggcacaagcaccgagccaagcgagcctaagaagaagagaaaagtcggcagcgacaagaagtacagcatcggcctggccatcggcaccaactctgtgggctgggccgtgatcaccgacgagtacaaggtgcccagcaagaaattcaaggtgctgggcaacaccgaccggcacagcatcaagaagaacctgatcggcgccctgctgttcgacagcggagaaacagccgaggccacccggctgaagagaaccgccagaagaagatacaccagacggaagaaccggatctgctatctgcaagagatcttcagcaacgagatggccaaggtggacgacagcttcttccacagactggaagagtccttcctggtggaagaggataagaagcacgagcggcaccccatcttcggcaacatcgtggacgaggtggcctaccacgagaagtaccccaccatctaccacctgagaaagaaactggtggacagcaccgacaaggccgacctgcggctgatctatctggccctggcccacatgatcaagttccggggccacttcctgatcgagggcgacctgaaccccgacaacagcgacgtggacaagctgttcatccagctggtgcagacctacaaccagctgttcgaggaaaaccccatcaacgccagcggcgtggacgccaaggccatcctgtctgccagactgagcaagagcagacggctggaaaatctgatcgcccagctgcccggcgagaagaagaatggcctgttcggcaacctgattgccctgagcctgggcctgacccccaacttcaagagcaacttcgacctggccgaggatgccaaactgcagctgagcaaggacacctacgacgacgacctggacaacctgctggcccagatcggcgaccagtacgccgacctgtttctggccgccaagaacctgtccgacgccatcctgctgagcgacatcctgagagtgaacaccgagatcaccaaggcccccctgagcgcctctatgatcaagagatacgacgagcaccaccaggacctgaccctgctgaaagctctcgtgcggcagcagctgcctgagaagtacaaagagattttcttcgaccagagcaagaacggctacgccggctacatcgatggcggagccagccaggaagagttctacaagttcatcaagcccatcctggaaaagatggacggcaccgaggaactgctcgtgaagctgaacagagaggacctgctgcggaagcagcggaccttcgacaacggcagcatcccccaccagatccacctgggagagctgcacgccattctgcggcggcaggaagatttttacccattcctgaaggacaaccgggaaaagatcgagaagatcctgaccttccgcatcccctactacgtgggccctctggccaggggaaacagcagattcgcctggatgaccagaaagagcgaggaaaccatcaccccctggaacttcgaggaagtggtggacaagggcgccagcgcccagagcttcatcgagcggatgaccaacttcgataagaacctgcccaacgagaaggtgctgcccaagcacagcctgctgtacgagtacttcaccgtgtacaacgagctgaccaaagtgaaatacgtgaccgagggaatgagaaagcccgccttcctgagcggcgagcagaaaaaagccatcgtggacctgctgttcaagaccaaccggaaagtgaccgtgaagcagctgaaagaggactacttcaagaaaatcgagtgcttcgactccgtggaaatctccggcgtggaagatcggttcaacgcctccctgggcacataccacgatctgctgaaaattatcaaggacaaggacttcctggacaatgaggaaaacgaggacattctggaagatatcgtgctgaccctgacactgtttgaggacagagagatgatcgaggaacggctgaaaacctatgcccacctgttcgacgacaaagtgatgaagcagctgaagcggcggagatacaccggctggggcaggctgagccggaagctgatcaacggcatccgggacaagcagtccggcaagacaatcctggatttcctgaagtccgacggcttcgccaacagaaacttcatgcagctgatccacgacgacagcctgacctttaaagaggacatccagaaagcccaggtgtccggccagggcgatagcctgcacgagcacattgccaatctggccggcagccccgccattaagaagggcatcctgcagacagtgaaggtggtggacgagctcgtgaaagtgatgggccggcacaagcccgagaacatcgtgatcgaaatggccagagagaaccagaccacccagaagggacagaagaacagccgcgagagaatgaagcggatcgaagagggcatcaaagagctgggcagccagatcctgaaagaacaccccgtggaaaacacccagctgcagaacgagaagctgtacctgtactacctgcagaatgggcgggatatgtacgtggaccaggaactggacatcaaccggctgtccgactacgatgtggacgctatcgtgcctcagagctttctgaaggacgactccatcgataacaaagtgctgactcggagcgacaagaaccggggcaagagcgacaacgtgccctccgaagaggtcgtgaagaagatgaagaactactggcgccagctgctgaatgccaagctgattacccagaggaagttcgacaatctgaccaaggccgagagaggcggcctgagcgaactggataaggccggcttcatcaagagacagctggtggaaacccggcagatcacaaagcacgtggcacagatcctggactcccggatgaacactaagtacgacgagaacgacaaactgatccgggaagtgaaagtgatcaccctgaagtccaagctggtgtccgatttccggaaggatttccagttttacaaagtgcgcgagatcaacaactaccaccacgcccacgacgcctacctgaacgccgtcgtgggaaccgccctgatcaaaaagtaccctaagctggaaagcgagttcgtgtacggcgactacaaggtgtacgacgtgcggaagatgatcgccaagagcgagcaggaaatcggcaaggctaccgccaagtacttcttctacagcaacatcatgaactttttcaagaccgagattaccctggccaacggcgagatccggaagcggcctctgatcgagacaaacggcgaaacaggcgagatcgtgtgggataagggccgggactttgccaccgtgcggaaagtgctgtctatgccccaagtgaatatcgtgaaaaagaccgaggtgcagacaggcggcttcagcaaagagtctatcctgcccaagaggaacagcgacaagctgatcgccagaaagaaggactgggaccctaagaagtacggcggcttcgacagccccaccgtggcctattctgtgctggtggtggccaaagtggaaaagggcaagtccaagaaactgaagagtgtgaaagagctgctggggatcaccatcatggaaagaagcagcttcgagaagaatcccatcgactttctggaagccaagggctacaaagaagtgaaaaaggacctgatcatcaagctgcctaagtactccctgttcgagctggaaaacggccggaagagaatgctggcctctgccggcgaactgcagaagggaaacgaactggccctgccctccaaatatgtgaacttcctgtacctggccagccactatgagaagctgaagggctcccccgaggataatgagcagaaacagctgtttgtggaacagcacaaacactacctggacgagatcatcgagcagatcagcgagttctccaagagagtgatcctggccgacgctaatctggacaaggtgctgagcgcctacaacaagcacagagacaagcctatcagagagcaggccgagaatatcatccacctgtttaccctgaccaatctgggagcccctgccgccttcaagtactttgacaccaccatcgaccggaagaggtacaccagcaccaaagaggtgctggacgccaccctgatccaccagagcatcaccggcctgtacgagacacggatcgacctgtctcagctgggaggcgacgcctatccctatgacgtgcccgattatgccagcctgggcagcggctcccccaagaaaaaacgcaaggtggaagatcctaagaaaaagcggaaagtggacggcatcggctccggctctaatggatctagcggagaggaactcctgtccaagaactaccaccttgagaacgaagtggcccgactcaagaaaggctctggtagcggaggctcaggttccggcggatcaggcagtggttctggcggttccggctcaggcggtagtggcagtggcgaagaacttctgagcaaaaactaccacggctctggctccggacagcggggctctaaaagaacagccgacggcagcgagtttgagagccctaaaaagaaaagaaaagtgtgataatagggatcccaagcacgcagcaatgcagctcaaaacgcttagcctagccacacccccacgggaaacagcagtgattaacctttagcaataaacgaaagtttaactaagctatactaaccccagggttggtcaatttcgtgccagccacaccctggtactgcatgcacgcaatgctagctgcccctttcccgtcctgggcaccccgagtctcccccgaccccgggtcccaggtatgctcccacctccacctgccccactcaccacctctgctagttccagacacctccgaagatggaaaaaaaaaaaaaaaaaaaaaaaaaaaaaaaaaaaaaaaaaaaaaaaaaaaaaaaaaaaaaaaaaaaaaaaaaaaaaaaaaaaaaaaaaaaaaaaaaaaaaaaaaaaaaaaaaaaaaaaaaaaagcttgagaccggatcattgtcactttcaccgtcatcaccgaaacgcgcgatgcagctctggcccgtgtctcaaaatctctgatgttacattgcacaagataaaaatatatcatcatgaacaataaaactgtctgcttacataaacagtaatacaaggggtgttatgagccatattcaacgggaaacgtcgaggccgcgattaaattccaacatggatgctgatttatatgggtataaatgggctcgcgataatgtcgggcaatcaggtgcgacaatctatcgcttgtatgggaagcccgatgcgccagagttgtttctgaaacatggcaaaggtagcgttgccaatgatgttacagatgagatggtcagactaaactggctgacggaatttatgcctcttccgaccatcaagcattttatccgtactcctgatgatgcatggttactcaccactgcgatccccggaaaaacagcattccaggtattagaagaatatcctgattcaggtgaaaatattgttgatgcgctggcagtgttcctgcgccggttgcattcgattcctgtttgtaattgtccttttaacagcgatcgcgtatttcgtctcgctcaggcgcaatcacgaatgaataacggtttggttgatgcgagtgattttgatgacgagcgtaatggctggcctgttgaacaagtctggaaagaaatgcataaacttttgccattctcaccggattcagtcgtcactcatggtgatttctcacttgataaccttatttttgacgaggggaaattaataggttgtattgatgttggacgagtcggaatcgcagaccgataccaggatcttgccatcctatggaactgcctcggtgagttttctccttcattacagaaacggctttttcaaaaatatggtattgataatcctgatatgaataaattgcagtttcatttgatgctcgatgagtttttctaatcagaattggttaattggttgtaacattattcagattgggcttgatttaaaacttcatttttaatttaaaaggatctaggtgaagatcctttttgataatctcatgaccaaaatcccttaacgtgagttttcgttccactgagcgtcagaccccgtagaaaagatcaaaggatcttcttgagatcctttttttctgcgcgtaatctgctgcttgcaaacaaaaaaaccaccgctaccagcggtggtttgtttgccggatcaagagctaccaactctttttc

SEQ ID NO: 242 - RNA, 5686 nt, synthetic construct
  misc_feature 1..5686: note = mRNA of V1_3xGCN4-dCas9-3xGCN4
  source 1..5686: mol_type = other RNA
aggactcactatttgttttcgcgcccagttgcaaaaagtgtcgacatttgcttctgacacaactgtgttcactagcaacctcaaacagacaccgccaccatgcctgctgctaagagagtgaaactggatggatccgaggaactgctgagcaagaactaccacctggaaaacgaggtggccagactgaagaaaggctctggctctggcggaagcggttctggcggatcaggatctggaagtggcggctctggaagcggaggttctggatctggcgaagaactgctgtctaagaattatcacctcgagaacgaagtggctcggctcaagaaaggcagtggcagcggaggaagtggatccggcggtagtggtagtggaagcggcggatccggctcaggcggatctggttcaggggaagaactcctctccaaaaactaccatctcgagaatgaggtcgcccgcctgaaaaaaggatcaggttccggtggttctggcagcggtggttcaggctcaggcagcggcggtagcggtagcggtggaagcggaagcggaccaaaaaagaagagaaaggtaatggacaagaagtacagcatcggcctggccatcggcaccaactctgtgggctgggccgtgatcaccgacgagtacaaggtgcccagcaagaaattcaaggtgctgggcaacaccgaccggcacagcatcaagaagaacctgatcggcgccctgctgttcgacagcggagaaacagccgaggccacccggctgaagagaaccgccagaagaagatacaccagacggaagaaccggatctgctatctgcaagagatcttcagcaacgagatggccaaggtggacgacagcttcttccacagactggaagagtccttcctggtggaagaggataagaagcacgagcggcaccccatcttcggcaacatcgtggacgaggtggcctaccacgagaagtaccccaccatctaccacctgagaaagaaactggtggacagcaccgacaaggccgacctgcggctgatctatctggccctggcccacatgatcaagttccggggccacttcctgatcgagggcgacctgaaccccgacaacagcgacgtggacaagctgttcatccagctggtgcagacctacaaccagctgttcgaggaaaaccccatcaacgccagcggcgtggacgccaaggccatcctgtctgccagactgagcaagagcagacggctggaaaatctgatcgcccagctgcccggcgagaagaagaatggcctgttcggcaacctgattgccctgagcctgggcctgacccccaacttcaagagcaacttcgacctggccgaggatgccaaactgcagctgagcaaggacacctacgacgacgacctggacaacctgctggcccagatcggcgaccagtacgccgacctgtttctggccgccaagaacctgtccgacgccatcctgctgagcgacatcctgagagtgaacaccgagatcaccaaggcccccctgagcgcctctatgatcaagagatacgacgagcaccaccaggacctgaccctgctgaaagctctcgtgcggcagcagctgcctgagaagtacaaagagattttcttcgaccagagcaagaacggctacgccggctacatcgatggcggagccagccaggaagagttctacaagttcatcaagcccatcctggaaaagatggacggcaccgaggaactgctcgtgaagctgaacagagaggacctgctgcggaagcagcggaccttcgacaacggcagcatcccccaccagatccacctgggagagctgcacgccattctgcggcggcaggaagatttttacccattcctgaaggacaaccgggaaaagatcgagaagatcctgaccttccgcatcccctactacgtgggccctctggccaggggaaacagcagattcgcctggatgaccagaaagagcgaggaaaccatcaccccctggaacttcgaggaagtggtggacaagggcgccagcgcccagagcttcatcgagcggatgaccaacttcgataagaacctgcccaacgagaaggtgctgcccaagcacagcctgctgtacgagtacttcaccgtgtacaacgagctgaccaaagtgaaatacgtgaccgagggaatgagaaagcccgccttcctgagcggcgagcagaaaaaagccatcgtggacctgctgttcaagaccaaccggaaagtgaccgtgaagcagctgaaagaggactacttcaagaaaatcgagtgcttcgactccgtggaaatctccggcgtggaagatcggttcaacgcctccctgggcacataccacgatctgctgaaaattatcaaggacaaggacttcctggacaatgaggaaaacgaggacattctggaagatatcgtgctgaccctgacactgtttgaggacagagagatgatcgaggaacggctgaaaacctatgcccacctgttcgacgacaaagtgatgaagcagctgaagcggcggagatacaccggctggggcaggctgagccggaagctgatcaacggcatccgggacaagcagtccggcaagacaatcctggatttcctgaagtccgacggcttcgccaacagaaacttcatgcagctgatccacgacgacagcctgacctttaaagaggacatccagaaagcccaggtgtccggccagggcgatagcctgcacgagcacattgccaatctggccggcagccccgccattaagaagggcatcctgcagacagtgaaggtggtggacgagctcgtgaaagtgatgggccggcacaagcccgagaacatcgtgatcgaaatggccagagagaaccagaccacccagaagggacagaagaacagccgcgagagaatgaagcggatcgaagagggcatcaaagagctgggcagccagatcctgaaagaacaccccgtggaaaacacccagctgcagaacgagaagctgtacctgtactacctgcagaatgggcgggatatgtacgtggaccaggaactggacatcaaccggctgtccgactacgatgtggacgctatcgtgcctcagagctttctgaaggacgactccatcgataacaaagtgctgactcggagcgacaagaaccggggcaagagcgacaacgtgccctccgaagaggtcgtgaagaagatgaagaactactggcgccagctgctgaatgccaagctgattacccagaggaagttcgacaatctgaccaaggccgagagaggcggcctgagcgaactggataaggccggcttcatcaagagacagctggtggaaacccggcagatcacaaagcacgtggcacagatcctggactcccggatgaacactaagtacgacgagaacgacaaactgatccgggaagtgaaagtgatcaccctgaagtccaagctggtgtccgatttccggaaggatttccagttttacaaagtgcgcgagatcaacaactaccaccacgcccacgacgcctacctgaacgccgtcgtgggaaccgccctgatcaaaaagtaccctaagctggaaagcgagttcgtgtacggcgactacaaggtgtacgacgtgcggaagatgatcgccaagagcgagcaggaaatcggcaaggctaccgccaagtacttcttctacagcaacatcatgaactttttcaagaccgagattaccctggccaacggcgagatccggaagcggcctctgatcgagacaaacggcgaaacaggcgagatcgtgtgggataagggccgggactttgccaccgtgcggaaagtgctgtctatgccccaagtgaatatcgtgaaaaagaccgaggtgcagacaggcggcttcagcaaagagtctatcctgcccaagaggaacagcgacaagctgatcgccagaaagaaggactgggaccctaagaagtacggcggcttcgacagccccaccgtggcctattctgtgctggtggtggccaaagtggaaaagggcaagtccaagaaactgaagagtgtgaaagagctgctggggatcaccatcatggaaagaagcagcttcgagaagaatcccatcgactttctggaagccaagggctacaaagaagtgaaaaaggacctgatcatcaagctgcctaagtactccctgttcgagctggaaaacggccggaagagaatgctggcctctgccggcgaactgcagaagggaaacgaactggccctgccctccaaatatgtgaacttcctgtacctggccagccactatgagaagctgaagggctcccccgaggataatgagcagaaacagctgtttgtggaacagcacaaacactacctggacgagatcatcgagcagatcagcgagttctccaagagagtgatcctggccgacgctaatctggacaaggtgctgagcgcctacaacaagcacagagacaagcctatcagagagcaggccgagaatatcatccacctgtttaccctgaccaatctgggagcccctgccgccttcaagtactttgacaccaccatcgaccggaagaggtacaccagcaccaaagaggtgctggacgccaccctgatccaccagagcatcaccggcctgtacgagacacggatcgacctgtctcagctgggaggcgacgcctatccctatgacgtgcccgattatgccagcctgggcagcggctcccccaagaaaaaacgcaaggtggaagatcctaagaaaaagcggaaagtggacggcagcggcagcgagacccccggtaccagtggcggatctggctccggtagcggaggatcaggatccggcggaagcggatcaggcgaggaactgctttccaaaaattaccaccttgaaaacgaagtcgcccgcctcaagaaaggttctggcagcggaggctctggcagtggtggtagcggaagtggaagtggtggcagtggtagcggtggatctggaagcggcgaggaactcctgtcaaagaattaccatctcgaaaacgaggtcgcaaggctcaagaaaggctcaggatcaggcggctctggatccggcggttctggttccggctcaggtggaagtggatctggcggctcaggttccggcgaagaattgctttccaagaactaccatttggaaaatgaagtcgctcgtttgaagaaaggttcaggctccggccagcggggaagcaagcgcaccgccgatggttccgagttcgaaagccccaaaaaaaagcgcaaggtctgagatcccaagcacgcagcaatgcagctcaaaacgcttagcctagccacacccccacgggaaacagcagtgattaacctttagcaataaacgaaagtttaactaagctatactaaccccagggttggtcaatttcgtgccagccacaccctggtactgcatgcacgcaatgctagctgcccctttcccgtcctgggcaccccgagtctcccccgaccccgggtcccaggtatgctcccacctccacctgccccactcaccacctctgctagttccagacacctccgagacgaggaaaaaaaaaaaaaaaaaaaaaaaaaaaaaaaaaaaaaaaaaaaaaaaaaaaaaaaaaaaaaaaaaaaaaaaaaaaaaaaaaaaaaaaaaaaaaaaaaaaaaaaaaaaaaaaaaaaaaaaa

SEQ ID NO: 243 - RNA, 1594 nt, synthetic construct
  misc_feature 1..1594: note = mRNA of V2_scFv-KRAB
  source 1..1594: mol_type = other RNA
aggactcactatttgttttcgcgcccagttgcaaaaagtgtcgacatttgcttctgacacaactgtgttcactagcaacctcaaacagacaccgccaccatgcctgctgctaagagagtgaaactggatggatccggccccgacatcgtgatgacccagagccccagcagcctgagcgccagcgtgggcgaccgcgtgaccatcacctgccgcagcagcaccggcgccgtgaccaccagcaactacgccagctgggtgcaggagaagcccggcaagctgttcaagggcctgatcggcggcaccaacaaccgcgcccccggcgtgcccagccgcttcagcggcagcctgatcggcgacaaggccaccctgaccatcagcagcctgcagcccgaggacttcgccacctacttctgcgccctgtggtacagcaaccactgggtgttcggccagggcaccaaggtggagctgaagcgcggcggcggcggcagcggcggcggcggcagcggcggcggcggcagcagcggcggcggcagcgaggtgaagctgctggagagcggcggcggcctggtgcagcccggcggcagcctgaagctgagctgcgccgtgagcggcttcagcctgaccgactacggcgtgaactgggtgcgccaggcccccggccgcggcctggagtggatcggcgtgatctggggcgacggcatcaccgactacaacagcgccctgaaggaccgcttcatcatcagcaaggacaacggcaagaacaccgtgtacctgcagatgagcaaggtgcgcagcgacgacaccgccctgtactactgcgtgaccggcctgttcgactactggggccagggcaccctggtgaccgtgagcagctacccatacgatgttccagattacgctggtggaggcggaggttctgggggaggaggtagtggcggtggtggttcaggaggcggcggaagcttggatccaggtggaggtggaagcggtcggacactggtgaccttcaaggatgtatttgtggacttcaccagggaggagtggaagctgctggacactgctcagcagatcgtgtacagaaatgtgatgctggagaactataagaacctggtttccttgggttatcagcttactaagccagatgtgatcctccggttggagaagggagaagagccctagtgagatcccaagcacgcagcaatgcagctcaaaacgcttagcctagccacacccccacgggaaacagcagtgattaacctttagcaataaacgaaagtttaactaagctatactaaccccagggttggtcaatttcgtgccagccacaccctggtactgcatgcacgcaatgctagctgcccctttcccgtcctgggcaccccgagtctcccccgaccccgggtcccaggtatgctcccacctccacctgccccactcaccacctctgctagttccagacacctccgagacgaggaaaaaaaaaaaaaaaaaaaaaaaaaaaaaaaaaaaaaaaaaaaaaaaaaaaaaaaaaaaaaaaaaaaaaaaaaaaaaaaaaaaaaaaaaaaaaaaaaaaaaaaaaaaaaaaaaaaaaaaa

SEQ ID NO: 244 - RNA, 6922 nt, synthetic construct
  misc_feature 1..6922: note = mRNA of V3_D3a-D3l-dCas9-1xGCN4
  source 1..6922: mol_type = other RNA
aggactcactatttgttttcgcgcccagttgcaaaaagtgtcgacatttgcttctgacacaactgtgttcactagcaacctcaaacagacaccgccaccatgcctgctgctaagagagtgaaactggatggatccaaccatgaccaggaatttgaccccccaaaggtttacccacctgtgccagctgagaagaggaagcccatccgcgtgctgtctctctttgatgggattgctacagggctcctggtgctgaaggacctgggcatccaagtggaccgctacattgcctccgaggtgtgtgaggactccatcacggtgggcatggtgcggcaccagggaaagatcatgtacgtcggggacgtccgcagcgtcacacagaagcatatccaggagtggggcccattcgacctggtgattggaggcagtccctgcaatgacctctccattgtcaaccctgcccgcaagggactttatgagggtactggccgcctcttctttgagttctaccgcctcctgcatgatgcgcggcccaaggagggagatgatcgccccttcttctggctctttgagaatgtggtggccatgggcgttagtgacaagagggacatctcgcgatttcttgagtctaaccccgtgatgattgacgccaaagaagtgtctgctgcacacagggcccgttacttctggggtaaccttcctggcatgaacaggcctttggcatccactgtgaatgataagctggagctgcaagagtgtctggagcacggcagaatagccaagttcagcaaagtgaggaccattaccaccaggtcaaactctataaagcagggcaaagaccagcatttccccgtcttcatgaacgagaaggaggacatcctgtggtgcactgaaatggaaagggtgtttggcttccccgtccactacacagacgtctccaacatgagccgcttggcgaggcagagactgctgggccgatcgtggagcgtgccggtcatccgccacctcttcgctccgctgaaggaatattttgcttgtgtgtctagcggcaatagtaacgctaacagccgcgggccgagcttcagcagcggcctggtgccgttaagcttgcgcggcagccatatgggccctatggagatatacaagacagtgtctgcatggaagagacagccagtgcgggtactgagcctcttcagaaacatcgacaaggtactaaagagtttgggcttcttggaaagcggttctggttctgggggaggaacgctgaagtacgtggaagatgtcacaaatgtcgtgaggagagacgtggagaaatggggcccctttgacctggtgtacggctcgacgcagcccctaggcagctcttgtgatcgctgtcccggctggtacatgttccagttccaccggatcctgcagtatgcgctgcctcgccaggagagtcagcggcccttcttctggatattcatggacaatctgctgctgactgaggatgaccaagagacaactacccgcttccttcagacagaggctgtgaccctccaggatgtccgtggcagagactaccagaatgctatgcgggtgtggagcaacattccagggctgaagagcaagcatgcgcccctgaccccaaaggaagaagagtatctgcaagcccaagtcagaagcaggagcaagctggacgccccgaaagttgacctcctggtgaagaactgccttctcccgctgagagagtacttcaagtatttttctcaaaactcacttcctcttggagggccgagctctggcgcacccccaccaagtggagggtctcctgccgggtccccaacatctactgaagaaggcaccagcgaatccgcaacgcccgagtcaggccctggtacctccacagaaccatctgaaggtagtgcgcctggttccccagctggaagccctacttccaccgaagaaggcacgtcaaccgaaccaagtgaaggatctgcccctgggaccagcactgaaccatctgagccaaaaaagaagagaaaggtaatggacaagaagtacagcatcggcctggccatcggcaccaactctgtgggctgggccgtgatcaccgacgagtacaaggtgcccagcaagaaattcaaggtgctgggcaacaccgaccggcacagcatcaagaagaacctgatcggcgccctgctgttcgacagcggagaaacagccgaggccacccggctgaagagaaccgccagaagaagatacaccagacggaagaaccggatctgctatctgcaagagatcttcagcaacgagatggccaaggtggacgacagcttcttccacagactggaagagtccttcctggtggaagaggataagaagcacgagcggcaccccatcttcggcaacatcgtggacgaggtggcctaccacgagaagtaccccaccatctaccacctgagaaagaaactggtggacagcaccgacaaggccgacctgcggctgatctatctggccctggcccacatgatcaagttccggggccacttcctgatcgagggcgacctgaaccccgacaacagcgacgtggacaagctgttcatccagctggtgcagacctacaaccagctgttcgaggaaaaccccatcaacgccagcggcgtggacgccaaggccatcctgtctgccagactgagcaagagcagacggctggaaaatctgatcgcccagctgcccggcgagaagaagaatggcctgttcggcaacctgattgccctgagcctgggcctgacccccaacttcaagagcaacttcgacctggccgaggatgccaaactgcagctgagcaaggacacctacgacgacgacctggacaacctgctggcccagatcggcgaccagtacgccgacctgtttctggccgccaagaacctgtccgacgccatcctgctgagcgacatcctgagagtgaacaccgagatcaccaaggcccccctgagcgcctctatgatcaagagatacgacgagcaccaccaggacctgaccctgctgaaagctctcgtgcggcagcagctgcctgagaagtacaaagagattttcttcgaccagagcaagaacggctacgccggctacatcgatggcggagccagccaggaagagttctacaagttcatcaagcccatcctggaaaagatggacggcaccgaggaactgctcgtgaagctgaacagagaggacctgctgcggaagcagcggaccttcgacaacggcagcatcccccaccagatccacctgggagagctgcacgccattctgcggcggcaggaagatttttacccattcctgaaggacaaccgggaaaagatcgagaagatcctgaccttccgcatcccctactacgtgggccctctggccaggggaaacagcagattcgcctggatgaccagaaagagcgaggaaaccatcaccccctggaacttcgaggaagtggtggacaagggcgccagcgcccagagcttcatcgagcggatgaccaacttcgataagaacctgcccaacgagaaggtgctgcccaagcacagcctgctgtacgagtacttcaccgtgtacaacgagctgaccaaagtgaaatacgtgaccgagggaatgagaaagcccgccttcctgagcggcgagcagaaaaaagccatcgtggacctgctgttcaagaccaaccggaaagtgaccgtgaagcagctgaaagaggactacttcaagaaaatcgagtgcttcgactccgtggaaatctccggcgtggaagatcggttcaacgcctccctgggcacataccacgatctgctgaaaattatcaaggacaaggacttcctggacaatgaggaaaacgaggacattctggaagatatcgtgctgaccctgacactgtttgaggacagagagatgatcgaggaacggctgaaaacctatgcccacctgttcgacgacaaagtgatgaagcagctgaagcggcggagatacaccggctggggcaggctgagccggaagctgatcaacggcatccgggacaagcagtccggcaagacaatcctggatttcctgaagtccgacggcttcgccaacagaaacttcatgcagctgatccacgacgacagcctgacctttaaagaggacatccagaaagcccaggtgtccggccagggcgatagcctgcacgagcacattgccaatctggccggcagccccgccattaagaagggcatcctgcagacagtgaaggtggtggacgagctcgtgaaagtgatgggccggcacaagcccgagaacatcgtgatcgaaatggccagagagaaccagaccacccagaagggacagaagaacagccgcgagagaatgaagcggatcgaagagggcatcaaagagctgggcagccagatcctgaaagaacaccccgtggaaaacacccagctgcagaacgagaagctgtacctgtactacctgcagaatgggcgggatatgtacgtggaccaggaactggacatcaaccggctgtccgactacgatgtggacgctatcgtgcctcagagctttctgaaggacgactccatcgataacaaagtgctgactcggagcgacaagaaccggggcaagagcgacaacgtgccctccgaagaggtcgtgaagaagatgaagaactactggcgccagctgctgaatgccaagctgattacccagaggaagttcgacaatctgaccaaggccgagagaggcggcctgagcgaactggataaggccggcttcatcaagagacagctggtggaaacccggcagatcacaaagcacgtggcacagatcctggactcccggatgaacactaagtacgacgagaacgacaaactgatccgggaagtgaaagtgatcaccctgaagtccaagctggtgtccgatttccggaaggatttccagttttacaaagtgcgcgagatcaacaactaccaccacgcccacgacgcctacctgaacgccgtcgtgggaaccgccctgatcaaaaagtaccctaagctggaaagcgagttcgtgtacggcgactacaaggtgtacgacgtgcggaagatgatcgccaagagcgagcaggaaatcggcaaggctaccgccaagtacttcttctacagcaacatcatgaactttttcaagaccgagattaccctggccaacggcgagatccggaagcggcctctgatcgagacaaacggcgaaacaggcgagatcgtgtgggataagggccgggactttgccaccgtgcggaaagtgctgtctatgccccaagtgaatatcgtgaaaaagaccgaggtgcagacaggcggcttcagcaaagagtctatcctgcccaagaggaacagcgacaagctgatcgccagaaagaaggactgggaccctaagaagtacggcggcttcgacagccccaccgtggcctattctgtgctggtggtggccaaagtggaaaagggcaagtccaagaaactgaagagtgtgaaagagctgctggggatcaccatcatggaaagaagcagcttcgagaagaatcccatcgactttctggaagccaagggctacaaagaagtgaaaaaggacctgatcatcaagctgcctaagtactccctgttcgagctggaaaacggccggaagagaatgctggcctctgccggcgaactgcagaagggaaacgaactggccctgccctccaaatatgtgaacttcctgtacctggccagccactatgagaagctgaagggctcccccgaggataatgagcagaaacagctgtttgtggaacagcacaaacactacctggacgagatcatcgagcagatcagcgagttctccaagagagtgatcctggccgacgctaatctggacaaggtgctgagcgcctacaacaagcacagagacaagcctatcagagagcaggccgagaatatcatccacctgtttaccctgaccaatctgggagcccctgccgccttcaagtactttgacaccaccatcgaccggaagaggtacaccagcaccaaagaggtgctggacgccaccctgatccaccagagcatcaccggcctgtacgagacacggatcgacctgtctcagctgggaggcgacgcctatccctatgacgtgcccgattatgccagcctgggcagcggctcccccaagaaaaaacgcaaggtggaagatcctaagaaaaagcggaaagtggacggcattggtagtgggagcaacggcagcagcggagaggaactgctgagcaagaactaccacctggaaaacgaggtggccagactgaagaaaggctctggctctggcggaagcggttctggcggatcaggatctggaagtggcggctctggaagcggaggttctggatctggcgaagaactgctgtctaagaattatcacggttcaggctccggccagcggggaagcaagcgcaccgccgatggttccgagttcgaaagccccaaaaaaaagcgcaaggtctgagatcccaagcacgcagcaatgcagctcaaaacgcttagcctagccacacccccacgggaaacagcagtgattaacctttagcaataaacgaaagtttaactaagctatactaaccccagggttggtcaatttcgtgccagccacaccctggtactgcatgcacgcaatgctagctgcccctttcccgtcctgggcaccccgagtctcccccgaccccgggtcccaggtatgctcccacctccacctgccccactcaccacctctgctagttccagacacctccgagacgaggaaaaaaaaaaaaaaaaaaaaaaaaaaaaaaaaaaaaaaaaaaaaaaaaaaaaaaaaaaaaaaaaaaaaaaaaaaaaaaaaaaaaaaaaaaaaaaaaaaaaaaaaaaaaaaaaaaaaaaaa

SEQ ID NO: 245 - RNA, 6952 nt, synthetic construct
  misc_feature 1..6952: note = mRNA of V4_D3a-D3l-dCas9-2xGCN4
  source 1..6952: mol_type = other RNA
aggactcactatttgttttcgcgcccagttgcaaaaagtgtcgacatttgcttctgacacaactgtgttcactagcaacctcaaacagacaccgccaccatgcctgctgctaagagagtgaaactggatggatccaaccatgaccaggaatttgaccccccaaaggtttacccacctgtgccagctgagaagaggaagcccatccgcgtgctgtctctctttgatgggattgctacagggctcctggtgctgaaggacctgggcatccaagtggaccgctacattgcctccgaggtgtgtgaggactccatcacggtgggcatggtgcggcaccagggaaagatcatgtacgtcggggacgtccgcagcgtcacacagaagcatatccaggagtggggcccattcgacctggtgattggaggcagtccctgcaatgacctctccattgtcaaccctgcccgcaagggactttatgagggtactggccgcctcttctttgagttctaccgcctcctgcatgatgcgcggcccaaggagggagatgatcgccccttcttctggctctttgagaatgtggtggccatgggcgttagtgacaagagggacatctcgcgatttcttgagtctaaccccgtgatgattgacgccaaagaagtgtctgctgcacacagggcccgttacttctggggtaaccttcctggcatgaacaggcctttggcatccactgtgaatgataagctggagctgcaagagtgtctggagcacggcagaatagccaagttcagcaaagtgaggaccattaccaccaggtcaaactctataaagcagggcaaagaccagcatttccccgtcttcatgaacgagaaggaggacatcctgtggtgcactgaaatggaaagggtgtttggcttccccgtccactacacagacgtctccaacatgagccgcttggcgaggcagagactgctgggccgatcgtggagcgtgccggtcatccgccacctcttcgctccgctgaaggaatattttgcttgtgtgtctagcggcaatagtaacgctaacagccgcgggccgagcttcagcagcggcctggtgccgttaagcttgcgcggcagccatatgggccctatggagatatacaagacagtgtctgcatggaagagacagccagtgcgggtactgagcctcttcagaaacatcgacaaggtactaaagagtttgggcttcttggaaagcggttctggttctgggggaggaacgctgaagtacgtggaagatgtcacaaatgtcgtgaggagagacgtggagaaatggggcccctttgacctggtgtacggctcgacgcagcccctaggcagctcttgtgatcgctgtcccggctggtacatgttccagttccaccggatcctgcagtatgcgctgcctcgccaggagagtcagcggcccttcttctggatattcatggacaatctgctgctgactgaggatgaccaagagacaactacccgcttccttcagacagaggctgtgaccctccaggatgtccgtggcagagactaccagaatgctatgcgggtgtggagcaacattccagggctgaagagcaagcatgcgcccctgaccccaaaggaagaagagtatctgcaagcccaagtcagaagcaggagcaagctggacgccccgaaagttgacctcctggtgaagaactgccttctcccgctgagagagtacttcaagtatttttctcaaaactcacttcctcttggagggccgagctctggcgcacccccaccaagtggagggtctcctgccgggtccccaacatctactgaagaaggcaccagcgaatccgcaacgcccgagtcaggccctggtacctccacagaaccatctgaaggtagtgcgcctggttccccagctggaagccctacttccaccgaagaaggcacgtcaaccgaaccaagtgaaggatctgcccctgggaccagcactgaaccatctgagccaaaaaagaagagaaaggtaatggacaagaagtacagcatcggcctggccatcggcaccaactctgtgggctgggccgtgatcaccgacgagtacaaggtgcccagcaagaaattcaaggtgctgggcaacaccgaccggcacagcatcaagaagaacctgatcggcgccctgctgttcgacagcggagaaacagccgaggccacccggctgaagagaaccgccagaagaagatacaccagacggaagaaccggatctgctatctgcaagagatcttcagcaacgagatggccaaggtggacgacagcttcttccacagactggaagagtccttcctggtggaagaggataagaagcacgagcggcaccccatcttcggcaacatcgtggacgaggtggcctaccacgagaagtaccccaccatctaccacctgagaaagaaactggtggacagcaccgacaaggccgacctgcggctgatctatctggccctggcccacatgatcaagttccggggccacttcctgatcgagggcgacctgaaccccgacaacagcgacgtggacaagctgttcatccagctggtgcagacctacaaccagctgttcgaggaaaaccccatcaacgccagcggcgtggacgccaaggccatcctgtctgccagactgagcaagagcagacggctggaaaatctgatcgcccagctgcccggcgagaagaagaatggcctgttcggcaacctgattgccctgagcctgggcctgacccccaacttcaagagcaacttcgacctggccgaggatgccaaactgcagctgagcaaggacacctacgacgacgacctggacaacctgctggcccagatcggcgaccagtacgccgacctgtttctggccgccaagaacctgtccgacgccatcctgctgagcgacatcctgagagtgaacaccgagatcaccaaggcccccctgagcgcctctatgatcaagagatacgacgagcaccaccaggacctgaccctgctgaaagctctcgtgcggcagcagctgcctgagaagtacaaagagattttcttcgaccagagcaagaacggctacgccggctacatcgatggcggagccagccaggaagagttctacaagttcatcaagcccatcctggaaaagatggacggcaccgaggaactgctcgtgaagctgaacagagaggacctgctgcggaagcagcggaccttcgacaacggcagcatcccccaccagatccacctgggagagctgcacgccattctgcggcggcaggaagatttttacccattcctgaaggacaaccgggaaaagatcgagaagatcctgaccttccgcatcccctactacgtgggccctctggccaggggaaacagcagattcgcctggatgaccagaaagagcgaggaaaccatcaccccctggaacttcgaggaagtggtggacaagggcgccagcgcccagagcttcatcgagcggatgaccaacttcgataagaacctgcccaacgagaaggtgctgcccaagcacagcctgctgtacgagtacttcaccgtgtacaacgagctgaccaaagtgaaatacgtgaccgagggaatgagaaagcccgccttcctgagcggcgagcagaaaaaagccatcgtggacctgctgttcaagaccaaccggaaagtgaccgtgaagcagctgaaagaggactacttcaagaaaatcgagtgcttcgactccgtggaaatctccggcgtggaagatcggttcaacgcctccctgggcacataccacgatctgctgaaaattatcaaggacaaggacttcctggacaatgaggaaaacgaggacattctggaagatatcgtgctgaccctgacactgtttgaggacagagagatgatcgaggaacggctgaaaacctatgcccacctgttcgacgacaaagtgatgaagcagctgaagcggcggagatacaccggctggggcaggctgagccggaagctgatcaacggcatccgggacaagcagtccggcaagacaatcctggatttcctgaagtccgacggcttcgccaacagaaacttcatgcagctgatccacgacgacagcctgacctttaaagaggacatccagaaagcccaggtgtccggccagggcgatagcctgcacgagcacattgccaatctggccggcagccccgccattaagaagggcatcctgcagacagtgaaggtggtggacgagctcgtgaaagtgatgggccggcacaagcccgagaacatcgtgatcgaaatggccagagagaaccagaccacccagaagggacagaagaacagccgcgagagaatgaagcggatcgaagagggcatcaaagagctgggcagccagatcctgaaagaacaccccgtggaaaacacccagctgcagaacgagaagctgtacctgtactacctgcagaatgggcgggatatgtacgtggaccaggaactggacatcaaccggctgtccgactacgatgtggacgctatcgtgcctcagagctttctgaaggacgactccatcgataacaaagtgctgactcggagcgacaagaaccggggcaagagcgacaacgtgccctccgaagaggtcgtgaagaagatgaagaactactggcgccagctgctgaatgccaagctgattacccagaggaagttcgacaatctgaccaaggccgagagaggcggcctgagcgaactggataaggccggcttcatcaagagacagctggtggaaacccggcagatcacaaagcacgtggcacagatcctggactcccggatgaacactaagtacgacgagaacgacaaactgatccgggaagtgaaagtgatcaccctgaagtccaagctggtgtccgatttccggaaggatttccagttttacaaagtgcgcgagatcaacaactaccaccacgcccacgacgcctacctgaacgccgtcgtgggaaccgccctgatcaaaaagtaccctaagctggaaagcgagttcgtgtacggcgactacaaggtgtacgacgtgcggaagatgatcgccaagagcgagcaggaaatcggcaaggctaccgccaagtacttcttctacagcaacatcatgaactttttcaagaccgagattaccctggccaacggcgagatccggaagcggcctctgatcgagacaaacggcgaaacaggcgagatcgtgtgggataagggccgggactttgccaccgtgcggaaagtgctgtctatgccccaagtgaatatcgtgaaaaagaccgaggtgcagacaggcggcttcagcaaagagtctatcctgcccaagaggaacagcgacaagctgatcgccagaaagaaggactgggaccctaagaagtacggcggcttcgacagccccaccgtggcctattctgtgctggtggtggccaaagtggaaaagggcaagtccaagaaactgaagagtgtgaaagagctgctggggatcaccatcatggaaagaagcagcttcgagaagaatcccatcgactttctggaagccaagggctacaaagaagtgaaaaaggacctgatcatcaagctgcctaagtactccctgttcgagctggaaaacggccggaagagaatgctggcctctgccggcgaactgcagaagggaaacgaactggccctgccctccaaatatgtgaacttcctgtacctggccagccactatgagaagctgaagggctcccccgaggataatgagcagaaacagctgtttgtggaacagcacaaacactacctggacgagatcatcgagcagatcagcgagttctccaagagagtgatcctggccgacgctaatctggacaaggtgctgagcgcctacaacaagcacagagacaagcctatcagagagcaggccgagaatatcatccacctgtttaccctgaccaatctgggagcccctgccgccttcaagtactttgacaccaccatcgaccggaagaggtacaccagcaccaaagaggtgctggacgccaccctgatccaccagagcatcaccggcctgtacgagacacggatcgacctgtctcagctgggaggcgacgcctatccctatgacgtgcccgattatgccagcctgggcagcggctcccccaagaaaaaacgcaaggtggaagatcctaagaaaaagcggaaagtggacggcattggtagtgggagcaacggcagcagcggagaggaactgctgagcaagaactaccacctggaaaacgaggtggccagactgaagaaaggctctggctctggcggaagcggttctggcggatcaggatctggaagtggcggctctggaagcggaggttctggatctggcgaagaactgctgtctaagaattatcacctcgagaatgaagtcgctcgtttgaagaaaggttcaggctccggccagcggggaagcaagcgcaccgccgatggttccgagttcgaaagccccaaaaaaaagcgcaaggtctgagatcccaagcacgcagcaatgcagctcaaaacgcttagcctagccacacccccacgggaaacagcagtgattaacctttagcaataaacgaaagtttaactaagctatactaaccccagggttggtcaatttcgtgccagccacaccctggtactgcatgcacgcaatgctagctgcccctttcccgtcctgggcaccccgagtctcccccgaccccgggtcccaggtatgctcccacctccacctgccccactcaccacctctgctagttccagacacctccgagacgaggaaaaaaaaaaaaaaaaaaaaaaaaaaaaaaaaaaaaaaaaaaaaaaaaaaaaaaaaaaaaaaaaaaaaaaaaaaaaaaaaaaaaaaaaaaaaaaaaaaaaaaaaaaaaaaaaaaaaaaaa

SEQ ID NO: 246 - RNA, 7228 nt, synthetic construct
  misc_feature 1..7228: note = mRNA of V5_D3a-D3l-dCas9-4xGCN4
  source 1..7228: mol_type = other RNA
aggactcactatttgttttcgcgcccagttgcaaaaagtgtcgacatttgcttctgacacaactgtgttcactagcaacctcaaacagacaccgccaccatgcctgctgctaagagagtgaaactggatggatccaaccatgaccaggaatttgaccccccaaaggtttacccacctgtgccagctgagaagaggaagcccatccgcgtgctgtctctctttgatgggattgctacagggctcctggtgctgaaggacctgggcatccaagtggaccgctacattgcctccgaggtgtgtgaggactccatcacggtgggcatggtgcggcaccagggaaagatcatgtacgtcggggacgtccgcagcgtcacacagaagcatatccaggagtggggcccattcgacctggtgattggaggcagtccctgcaatgacctctccattgtcaaccctgcccgcaagggactttatgagggtactggccgcctcttctttgagttctaccgcctcctgcatgatgcgcggcccaaggagggagatgatcgccccttcttctggctctttgagaatgtggtggccatgggcgttagtgacaagagggacatctcgcgatttcttgagtctaaccccgtgatgattgacgccaaagaagtgtctgctgcacacagggcccgttacttctggggtaaccttcctggcatgaacaggcctttggcatccactgtgaatgataagctggagctgcaagagtgtctggagcacggcagaatagccaagttcagcaaagtgaggaccattaccaccaggtcaaactctataaagcagggcaaagaccagcatttccccgtcttcatgaacgagaaggaggacatcctgtggtgcactgaaatggaaagggtgtttggcttccccgtccactacacagacgtctccaacatgagccgcttggcgaggcagagactgctgggccgatcgtggagcgtgccggtcatccgccacctcttcgctccgctgaaggaatattttgcttgtgtgtctagcggcaatagtaacgctaacagccgcgggccgagcttcagcagcggcctggtgccgttaagcttgcgcggcagccatatgggccctatggagatatacaagacagtgtctgcatggaagagacagccagtgcgggtactgagcctcttcagaaacatcgacaaggtactaaagagtttgggcttcttggaaagcggttctggttctgggggaggaacgctgaagtacgtggaagatgtcacaaatgtcgtgaggagagacgtggagaaatggggcccctttgacctggtgtacggctcgacgcagcccctaggcagctcttgtgatcgctgtcccggctggtacatgttccagttccaccggatcctgcagtatgcgctgcctcgccaggagagtcagcggcccttcttctggatattcatggacaatctgctgctgactgaggatgaccaagagacaactacccgcttccttcagacagaggctgtgaccctccaggatgtccgtggcagagactaccagaatgctatgcgggtgtggagcaacattccagggctgaagagcaagcatgcgcccctgaccccaaaggaagaagagtatctgcaagcccaagtcagaagcaggagcaagctggacgccccgaaagttgacctcctggtgaagaactgccttctcccgctgagagagtacttcaagtatttttctcaaaactcacttcctcttggagggccgagctctggcgcacccccaccaagtggagggtctcctgccgggtccccaacatctactgaagaaggcaccagcgaatccgcaacgcccgagtcaggccctggtacctccacagaaccatctgaaggtagtgcgcctggttccccagctggaagccctacttccaccgaagaaggcacgtcaaccgaaccaagtgaaggatctgcccctgggaccagcactgaaccatctgagccaaaaaagaagagaaaggtaatggacaagaagtacagcatcggcctggccatcggcaccaactctgtgggctgggccgtgatcaccgacgagtacaaggtgcccagcaagaaattcaaggtgctgggcaacaccgaccggcacagcatcaagaagaacctgatcggcgccctgctgttcgacagcggagaaacagccgaggccacccggctgaagagaaccgccagaagaagatacaccagacggaagaaccggatctgctatctgcaagagatcttcagcaacgagatggccaaggtggacgacagcttcttccacagactggaagagtccttcctggtggaagaggataagaagcacgagcggcaccccatcttcggcaacatcgtggacgaggtggcctaccacgagaagtaccccaccatctaccacctgagaaagaaactggtggacagcaccgacaaggccgacctgcggctgatctatctggccctggcccacatgatcaagttccggggccacttcctgatcgagggcgacctgaaccccgacaacagcgacgtggacaagctgttcatccagctggtgcagacctacaaccagctgttcgaggaaaaccccatcaacgccagcggcgtggacgccaaggccatcctgtctgccagactgagcaagagcagacggctggaaaatctgatcgcccagctgcccggcgagaagaagaatggcctgttcggcaacctgattgccctgagcctgggcctgacccccaacttcaagagcaacttcgacctggccgaggatgccaaactgcagctgagcaaggacacctacgacgacgacctggacaacctgctggcccagatcggcgaccagtacgccgacctgtttctggccgccaagaacctgtccgacgccatcctgctgagcgacatcctgagagtgaacaccgagatcaccaaggcccccctgagcgcctctatgatcaagagatacgacgagcaccaccaggacctgaccctgctgaaagctctcgtgcggcagcagctgcctgagaagtacaaagagattttcttcgaccagagcaagaacggctacgccggctacatcgatggcggagccagccaggaagagttctacaagttcatcaagcccatcctggaaaagatggacggcaccgaggaactgctcgtgaagctgaacagagaggacctgctgcggaagcagcggaccttcgacaacggcagcatcccccaccagatccacctgggagagctgcacgccattctgcggcggcaggaagatttttacccattcctgaaggacaaccgggaaaagatcgagaagatcctgaccttccgcatcccctactacgtgggccctctggccaggggaaacagcagattcgcctggatgaccagaaagagcgaggaaaccatcaccccctggaacttcgaggaagtggtggacaagggcgccagcgcccagagcttcatcgagcggatgaccaacttcgataagaacctgcccaacgagaaggtgctgcccaagcacagcctgctgtacgagtacttcaccgtgtacaacgagctgaccaaagtgaaatacgtgaccgagggaatgagaaagcccgccttcctgagcggcgagcagaaaaaagccatcgtggacctgctgttcaagaccaaccggaaagtgaccgtgaagcagctgaaagaggactacttcaagaaaatcgagtgcttcgactccgtggaaatctccggcgtggaagatcggttcaacgcctccctgggcacataccacgatctgctgaaaattatcaaggacaaggacttcctggacaatgaggaaaacgaggacattctggaagatatcgtgctgaccctgacactgtttgaggacagagagatgatcgaggaacggctgaaaacctatgcccacctgttcgacgacaaagtgatgaagcagctgaagcggcggagatacaccggctggggcaggctgagccggaagctgatcaacggcatccgggacaagcagtccggcaagacaatcctggatttcctgaagtccgacggcttcgccaacagaaacttcatgcagctgatccacgacgacagcctgacctttaaagaggacatccagaaagcccaggtgtccggccagggcgatagcctgcacgagcacattgccaatctggccggcagccccgccattaagaagggcatcctgcagacagtgaaggtggtggacgagctcgtgaaagtgatgggccggcacaagcccgagaacatcgtgatcgaaatggccagagagaaccagaccacccagaagggacagaagaacagccgcgagagaatgaagcggatcgaagagggcatcaaagagctgggcagccagatcctgaaagaacaccccgtggaaaacacccagctgcagaacgagaagctgtacctgtactacctgcagaatgggcgggatatgtacgtggaccaggaactggacatcaaccggctgtccgactacgatgtggacgctatcgtgcctcagagctttctgaaggacgactccatcgataacaaagtgctgactcggagcgacaagaaccggggcaagagcgacaacgtgccctccgaagaggtcgtgaagaagatgaagaactactggcgccagctgctgaatgccaagctgattacccagaggaagttcgacaatctgaccaaggccgagagaggcggcctgagcgaactggataaggccggcttcatcaagagacagctggtggaaacccggcagatcacaaagcacgtggcacagatcctggactcccggatgaacactaagtacgacgagaacgacaaactgatccgggaagtgaaagtgatcaccctgaagtccaagctggtgtccgatttccggaaggatttccagttttacaaagtgcgcgagatcaacaactaccaccacgcccacgacgcctacctgaacgccgtcgtgggaaccgccctgatcaaaaagtaccctaagctggaaagcgagttcgtgtacggcgactacaaggtgtacgacgtgcggaagatgatcgccaagagcgagcaggaaatcggcaaggctaccgccaagtacttcttctacagcaacatcatgaactttttcaagaccgagattaccctggccaacggcgagatccggaagcggcctctgatcgagacaaacggcgaaacaggcgagatcgtgtgggataagggccgggactttgccaccgtgcggaaagtgctgtctatgccccaagtgaatatcgtgaaaaagaccgaggtgcagacaggcggcttcagcaaagagtctatcctgcccaagaggaacagcgacaagctgatcgccagaaagaaggactgggaccctaagaagtacggcggcttcgacagccccaccgtggcctattctgtgctggtggtggccaaagtggaaaagggcaagtccaagaaactgaagagtgtgaaagagctgctggggatcaccatcatggaaagaagcagcttcgagaagaatcccatcgactttctggaagccaagggctacaaagaagtgaaaaaggacctgatcatcaagctgcctaagtactccctgttcgagctggaaaacggccggaagagaatgctggcctctgccggcgaactgcagaagggaaacgaactggccctgccctccaaatatgtgaacttcctgtacctggccagccactatgagaagctgaagggctcccccgaggataatgagcagaaacagctgtttgtggaacagcacaaacactacctggacgagatcatcgagcagatcagcgagttctccaagagagtgatcctggccgacgctaatctggacaaggtgctgagcgcctacaacaagcacagagacaagcctatcagagagcaggccgagaatatcatccacctgtttaccctgaccaatctgggagcccctgccgccttcaagtactttgacaccaccatcgaccggaagaggtacaccagcaccaaagaggtgctggacgccaccctgatccaccagagcatcaccggcctgtacgagacacggatcgacctgtctcagctgggaggcgacgcctatccctatgacgtgcccgattatgccagcctgggcagcggctcccccaagaaaaaacgcaaggtggaagatcctaagaaaaagcggaaagtggacggcattggtagtgggagcaacggcagcagcggagaggaactgctgagcaagaactaccacctggaaaacgaggtggccagactgaagaaaggctctggctctggcggaagcggttctggcggatcaggatctggaagtggcggctctggaagcggaggttctggatctggcgaagaactgctgtctaagaattatcacctcgagaacgaagtcgcccgcctcaagaaaggttctggcagcggaggctctggcagtggtggtagcggaagtggaagtggtggcagtggtagcggtggatctggaagcggcgaggaactcctgtcaaagaattaccatctcgaaaacgaggtcgcaaggctcaagaaaggctcaggatcaggcggctctggatccggcggttctggttccggctcaggtggaagtggatctggcggctcaggttccggcgaagaattgctttccaagaactaccatttggaaaatgaagtcgctcgtttgaagaaaggttcaggctccggccagcggggaagcaagcgcaccgccgatggttccgagttcgaaagccccaaaaaaaagcgcaaggtctgagatcccaagcacgcagcaatgcagctcaaaacgcttagcctagccacacccccacgggaaacagcagtgattaacctttagcaataaacgaaagtttaactaagctatactaaccccagggttggtcaatttcgtgccagccacaccctggtactgcatgcacgcaatgctagctgcccctttcccgtcctgggcaccccgagtctcccccgaccccgggtcccaggtatgctcccacctccacctgccccactcaccacctctgctagttccagacacctccgagacgaggaaaaaaaaaaaaaaaaaaaaaaaaaaaaaaaaaaaaaaaaaaaaaaaaaaaaaaaaaaaaaaaaaaaaaaaaaaaaaaaaaaaaaaaaaaaaaaaaaaaaaaaaaaaaaaaaaaaaaaaa

SEQ ID NO: 247 - RNA, 8056 nt, synthetic construct
  misc_feature 1..8056: note = mRNA of V6_D3a-D3l-dCas9-10xGCN4
  source 1..8056: mol_type = other RNA
aggactcactatttgttttcgcgcccagttgcaaaaagtgtcgacatttgcttctgacacaactgtgttcactagcaacctcaaacagacaccgccaccatgcctgctgctaagagagtgaaactggatggatccaaccatgaccaggaatttgaccccccaaaggtttacccacctgtgccagctgagaagaggaagcccatccgcgtgctgtctctctttgatgggattgctacagggctcctggtgctgaaggacctgggcatccaagtggaccgctacattgcctccgaggtgtgtgaggactccatcacggtgggcatggtgcggcaccagggaaagatcatgtacgtcggggacgtccgcagcgtcacacagaagcatatccaggagtggggcccattcgacctggtgattggaggcagtccctgcaatgacctctccattgtcaaccctgcccgcaagggactttatgagggtactggccgcctcttctttgagttctaccgcctcctgcatgatgcgcggcccaaggagggagatgatcgccccttcttctggctctttgagaatgtggtggccatgggcgttagtgacaagagggacatctcgcgatttcttgagtctaaccccgtgatgattgacgccaaagaagtgtctgctgcacacagggcccgttacttctggggtaaccttcctggcatgaacaggcctttggcatccactgtgaatgataagctggagctgcaagagtgtctggagcacggcagaatagccaagttcagcaaagtgaggaccattaccaccaggtcaaactctataaagcagggcaaagaccagcatttccccgtcttcatgaacgagaaggaggacatcctgtggtgcactgaaatggaaagggtgtttggcttccccgtccactacacagacgtctccaacatgagccgcttggcgaggcagagactgctgggccgatcgtggagcgtgccggtcatccgccacctcttcgctccgctgaaggaatattttgcttgtgtgtctagcggcaatagtaacgctaacagccgcgggccgagcttcagcagcggcctggtgccgttaagcttgcgcggcagccatatgggccctatggagatatacaagacagtgtctgcatggaagagacagccagtgcgggtactgagcctcttcagaaacatcgacaaggtactaaagagtttgggcttcttggaaagcggttctggttctgggggaggaacgctgaagtacgtggaagatgtcacaaatgtcgtgaggagagacgtggagaaatggggcccctttgacctggtgtacggctcgacgcagcccctaggcagctcttgtgatcgctgtcccggctggtacatgttccagttccaccggatcctgcagtatgcgctgcctcgccaggagagtcagcggcccttcttctggatattcatggacaatctgctgctgactgaggatgaccaagagacaactacccgcttccttcagacagaggctgtgaccctccaggatgtccgtggcagagactaccagaatgctatgcgggtgtggagcaacattccagggctgaagagcaagcatgcgcccctgaccccaaaggaagaagagtatctgcaagcccaagtcagaagcaggagcaagctggacgccccgaaagttgacctcctggtgaagaactgccttctcccgctgagagagtacttcaagtatttttctcaaaactcacttcctcttggagggccgagctctggcgcacccccaccaagtggagggtctcctgccgggtccccaacatctactgaagaaggcaccagcgaatccgcaacgcccgagtcaggccctggtacctccacagaaccatctgaaggtagtgcgcctggttccccagctggaagccctacttccaccgaagaaggcacgtcaaccgaaccaagtgaaggatctgcccctgggaccagcactgaaccatctgagccaaaaaagaagagaaaggtaatggacaagaagtacagcatcggcctggccatcggcaccaactctgtgggctgggccgtgatcaccgacgagtacaaggtgcccagcaagaaattcaaggtgctgggcaacaccgaccggcacagcatcaagaagaacctgatcggcgccctgctgttcgacagcggagaaacagccgaggccacccggctgaagagaaccgccagaagaagatacaccagacggaagaaccggatctgctatctgcaagagatcttcagcaacgagatggccaaggtggacgacagcttcttccacagactggaagagtccttcctggtggaagaggataagaagcacgagcggcaccccatcttcggcaacatcgtggacgaggtggcctaccacgagaagtaccccaccatctaccacctgagaaagaaactggtggacagcaccgacaaggccgacctgcggctgatctatctggccctggcccacatgatcaagttccggggccacttcctgatcgagggcgacctgaaccccgacaacagcgacgtggacaagctgttcatccagctggtgcagacctacaaccagctgttcgaggaaaaccccatcaacgccagcggcgtggacgccaaggccatcctgtctgccagactgagcaagagcagacggctggaaaatctgatcgcccagctgcccggcgagaagaagaatggcctgttcggcaacctgattgccctgagcctgggcctgacccccaacttcaagagcaacttcgacctggccgaggatgccaaactgcagctgagcaaggacacctacgacgacgacctggacaacctgctggcccagatcggcgaccagtacgccgacctgtttctggccgccaagaacctgtccgacgccatcctgctgagcgacatcctgagagtgaacaccgagatcaccaaggcccccctgagcgcctctatgatcaagagatacgacgagcaccaccaggacctgaccctgctgaaagctctcgtgcggcagcagctgcctgagaagtacaaagagattttcttcgaccagagcaagaacggctacgccggctacatcgatggcggagccagccaggaagagttctacaagttcatcaagcccatcctggaaaagatggacggcaccgaggaactgctcgtgaagctgaacagagaggacctgctgcggaagcagcggaccttcgacaacggcagcatcccccaccagatccacctgggagagctgcacgccattctgcggcggcaggaagatttttacccattcctgaaggacaaccgggaaaagatcgagaagatcctgaccttccgcatcccctactacgtgggccctctggccaggggaaacagcagattcgcctggatgaccagaaagagcgaggaaaccatcaccccctggaacttcgaggaagtggtggacaagggcgccagcgcccagagcttcatcgagcggatgaccaacttcgataagaacctgcccaacgagaaggtgctgcccaagcacagcctgctgtacgagtacttcaccgtgtacaacgagctgaccaaagtgaaatacgtgaccgagggaatgagaaagcccgccttcctgagcggcgagcagaaaaaagccatcgtggacctgctgttcaagaccaaccggaaagtgaccgtgaagcagctgaaagaggactacttcaagaaaatcgagtgcttcgactccgtggaaatctccggcgtggaagatcggttcaacgcctccctgggcacataccacgatctgctgaaaattatcaaggacaaggacttcctggacaatgaggaaaacgaggacattctggaagatatcgtgctgaccctgacactgtttgaggacagagagatgatcgaggaacggctgaaaacctatgcccacctgttcgacgacaaagtgatgaagcagctgaagcggcggagatacaccggctggggcaggctgagccggaagctgatcaacggcatccgggacaagcagtccggcaagacaatcctggatttcctgaagtccgacggcttcgccaacagaaacttcatgcagctgatccacgacgacagcctgacctttaaagaggacatccagaaagcccaggtgtccggccagggcgatagcctgcacgagcacattgccaatctggccggcagccccgccattaagaagggcatcctgcagacagtgaaggtggtggacgagctcgtgaaagtgatgggccggcacaagcccgagaacatcgtgatcgaaatggccagagagaaccagaccacccagaagggacagaagaacagccgcgagagaatgaagcggatcgaagagggcatcaaagagctgggcagccagatcctgaaagaacaccccgtggaaaacacccagctgcagaacgagaagctgtacctgtactacctgcagaatgggcgggatatgtacgtggaccaggaactggacatcaaccggctgtccgactacgatgtggacgctatcgtgcctcagagctttctgaaggacgactccatcgataacaaagtgctgactcggagcgacaagaaccggggcaagagcgacaacgtgccctccgaagaggtcgtgaagaagatgaagaactactggcgccagctgctgaatgccaagctgattacccagaggaagttcgacaatctgaccaaggccgagagaggcggcctgagcgaactggataaggccggcttcatcaagagacagctggtggaaacccggcagatcacaaagcacgtggcacagatcctggactcccggatgaacactaagtacgacgagaacgacaaactgatccgggaagtgaaagtgatcaccctgaagtccaagctggtgtccgatttccggaaggatttccagttttacaaagtgcgcgagatcaacaactaccaccacgcccacgacgcctacctgaacgccgtcgtgggaaccgccctgatcaaaaagtaccctaagctggaaagcgagttcgtgtacggcgactacaaggtgtacgacgtgcggaagatgatcgccaagagcgagcaggaaatcggcaaggctaccgccaagtacttcttctacagcaacatcatgaactttttcaagaccgagattaccctggccaacggcgagatccggaagcggcctctgatcgagacaaacggcgaaacaggcgagatcgtgtgggataagggccgggactttgccaccgtgcggaaagtgctgtctatgccccaagtgaatatcgtgaaaaagaccgaggtgcagacaggcggcttcagcaaagagtctatcctgcccaagaggaacagcgacaagctgatcgccagaaagaaggactgggaccctaagaagtacggcggcttcgacagccccaccgtggcctattctgtgctggtggtggccaaagtggaaaagggcaagtccaagaaactgaagagtgtgaaagagctgctggggatcaccatcatggaaagaagcagcttcgagaagaatcccatcgactttctggaagccaagggctacaaagaagtgaaaaaggacctgatcatcaagctgcctaagtactccctgttcgagctggaaaacggccggaagagaatgctggcctctgccggcgaactgcagaagggaaacgaactggccctgccctccaaatatgtgaacttcctgtacctggccagccactatgagaagctgaagggctcccccgaggataatgagcagaaacagctgtttgtggaacagcacaaacactacctggacgagatcatcgagcagatcagcgagttctccaagagagtgatcctggccgacgctaatctggacaaggtgctgagcgcctacaacaagcacagagacaagcctatcagagagcaggccgagaatatcatccacctgtttaccctgaccaatctgggagcccctgccgccttcaagtactttgacaccaccatcgaccggaagaggtacaccagcaccaaagaggtgctggacgccaccctgatccaccagagcatcaccggcctgtacgagacacggatcgacctgtctcagctgggaggcgacgcctatccctatgacgtgcccgattatgccagcctgggcagcggctcccccaagaaaaaacgcaaggtggaagatcctaagaaaaagcggaaagtggacggcattggtagtgggagcaacggcagcagcggagaggaactgctgagcaagaactaccacctggaaaacgaggtggccagactgaagaaaggctctggctctggcggaagcggttctggcggatcaggatctggaagtggcggctctggaagcggaggttctggatctggcgaagaactgctgtctaagaattatcacctcgagaacgaagtggctcggctcaagaaaggcagtggcagcggaggaagtggatccggcggtagtggtagtggaagcggcggatccggctcaggcggatctggttcaggggaagaactcctctccaaaaactaccatctcgagaatgaggtcgcccgcctgaaaaaaggatcaggttccggtggttctggcagcggtggttcaggctcaggcagcggcggtagcggtagcggtggaagcggaagcggagaagaacttctcagcaaaaattaccacttggagaatgaagttgcaagactcaaaaaaggttccggcagtggcggcagcggcagcggcggatctggtagtggatctggtggcagtggttcaggcggaagtggtagcggagaggaattgctctcaaagaactatcatttggagaacgaggttgcacgcttgaagaaaggcagcggatcaggcggatctggcagcggtggatctggttctggatccggcggctccggtagtggtggaagtggctctggggaagaattgcttagcaagaattatcatcttgaaaatgaggttgccaggcttaaaaaaggcagtggctccggcggatccggaagcggaggcagcggatctggatctggtggttcaggatctggcggttctggtagcggggaagaactgttgagtaaaaactatcaccttgagaacgaggtcgcaaggttgaaaaaaggatccggctctggcggctccggaagtggcggatctggctccggtagcggaggatcaggatccggcggaagcggatcaggcgaggaactgctttccaaaaattaccaccttgaaaacgaagtcgcccgcctcaagaaaggttctggcagcggaggctctggcagtggtggtagcggaagtggaagtggtggcagtggtagcggtggatctggaagcggcgaggaactcctgtcaaagaattaccatctcgaaaacgaggtcgcaaggctcaagaaaggctcaggatcaggcggctctggatccggcggttctggttccggctcaggtggaagtggatctggcggctcaggttccggcgaagaattgctttccaagaactaccatttggaaaatgaagtcgctcgtttgaagaaaggttcaggctccggccagcggggaagcaagcgcaccgccgatggttccgagttcgaaagccccaaaaaaaagcgcaaggtctgagatcccaagcacgcagcaatgcagctcaaaacgcttagcctagccacacccccacgggaaacagcagtgattaacctttagcaataaacgaaagtttaactaagctatactaaccccagggttggtcaatttcgtgccagccacaccctggtactgcatgcacgcaatgctagctgcccctttcccgtcctgggcaccccgagtctcccccgaccccgggtcccaggtatgctcccacctccacctgccccactcaccacctctgctagttccagacacctccgagacgaggaaaaaaaaaaaaaaaaaaaaaaaaaaaaaaaaaaaaaaaaaaaaaaaaaaaaaaaaaaaaaaaaaaaaaaaaaaaaaaaaaaaaaaaaaaaaaaaaaaaaaaaaaaaaaaaaaaaaaaaa

SEQ ID NO: 248 - RNA, 3250 nt, synthetic construct
  misc_feature 1..3250: note = mRNA of V7_D3a-D3l-scFv
  source 1..3250: mol_type = other RNA
aggactcactatttgttttcgcgcccagttgcaaaaagtgtcgacatttgcttctgacacaactgtgttcactagcaacctcaaacagacaccgccaccatgcctgctgctaagagagtgaaactggatggatccaaccatgaccaggaatttgaccccccaaaggtttacccacctgtgccagctgagaagaggaagcccatccgcgtgctgtctctctttgatgggattgctacagggctcctggtgctgaaggacctgggcatccaagtggaccgctacattgcctccgaggtgtgtgaggactccatcacggtgggcatggtgcggcaccagggaaagatcatgtacgtcggggacgtccgcagcgtcacacagaagcatatccaggagtggggcccattcgacctggtgattggaggcagtccctgcaatgacctctccattgtcaaccctgcccgcaagggactttatgagggtactggccgcctcttctttgagttctaccgcctcctgcatgatgcgcggcccaaggagggagatgatcgccccttcttctggctctttgagaatgtggtggccatgggcgttagtgacaagagggacatctcgcgatttcttgagtctaaccccgtgatgattgacgccaaagaagtgtctgctgcacacagggcccgttacttctggggtaaccttcctggcatgaacaggcctttggcatccactgtgaatgataagctggagctgcaagagtgtctggagcacggcagaatagccaagttcagcaaagtgaggaccattaccaccaggtcaaactctataaagcagggcaaagaccagcatttccccgtgttcatgaacgagaaggaggacatcctgtggtgcactgaaatggaaagggtgtttggcttccccgtccactacacagacgtctccaacatgagccgcttggcgaggcagagactgctgggccgatcgtggagcgtgccggtcatccgccacctcttcgctccgctgaaggaatattttgcttgtgtgtctagcggcaatagtaacgctaacagccgcgggccgagcttcagcagcggcctggtgccgttaagcttgcgcggcagccatatgggccctatggagatatacaagacagtgtctgcatggaagagacagccagtgcgggtactgagcctcttcagaaacatcgacaaggtactaaagagtttgggcttcttggaaagcggttctggttctgggggaggaacgctgaagtacgtggaagatgtcacaaatgtcgtgaggagagacgtggagaaatggggcccctttgacctggtgtacggctcgacgcagcccctaggcagctcttgtgatcgctgtcccggctggtacatgttccagttccaccggatcctgcagtatgcgctgcctcgccaggagagtcagcggcccttcttctggatattcatggacaatctgctgctgactgaggatgaccaagagacaactacccgcttccttcagacagaggctgtgaccctccaggatgtccgtggcagagactaccagaatgctatgcgggtgtggagcaacattccagggctgaagagcaagcatgcgcccctgaccccaaaggaagaagagtatctgcaagcccaagtcagaagcaggagcaagctggacgccccgaaagttgacctcctggtgaagaactgccttctcccgctgagagagtacttcaagtatttttctcaaaactcacttcctcttggagggccgagctctggcgcacccccaccaagtggagggtctcctgccgggtccccaacatctactgaagaaggcaccagcgaatccgcaacgcccgagtcaggccctggtacctccacagaaccatctgaaggtagtgcgcctggttccccagctggaagccctacttccaccgaagaaggcacgtcaaccgaaccaagtgaaggatctgcccctgggaccagcactgaaccatctgagggccccgacatcgtgatgacccagagccccagcagcctgagcgccagcgtgggcgaccgcgtgaccatcacctgccgcagcagcaccggcgccgtgaccaccagcaactacgccagctgggtgcaggagaagcccggcaagctgttcaagggcctgatcggcggcaccaacaaccgcgcccccggcgtgcccagccgcttcagcggcagcctgatcggcgacaaggccaccctgaccatcagcagcctgcagcccgaggacttcgccacctacttctgcgccctgtggtacagcaaccactgggtgttcggccagggcaccaaggtggagctgaagcgcggcggcggcggcagcggcggcggcggcagcggcggcggcggcagcagcggcggcggcagcgaggtgaagctgctggagagcggcggcggcctggtgcagcccggcggcagcctgaagctgagctgcgccgtgagcggcttcagcctgaccgactacggcgtgaactgggtgcgccaggcccccggccgcggcctggagtggatcggcgtgatctggggcgacggcatcaccgactacaacagcgccctgaaggaccgcttcatcatcagcaaggacaacggcaagaacaccgtgtacctgcagatgagcaaggtgcgcagcgacgacaccgccctgtactactgcgtgaccggcctgttcgactactggggccagggcaccctggtgaccgtgagcagctacccatacgatgttccagattacgctggtggaggcggaggttctgggggaggaggtagtggcggtggtggttcaggaggcggcggaagctagtgagatcccaagcacgcagcaatgcagctcaaaacgcttagcctagccacacccccacgggaaacagcagtgattaacctttagcaataaacgaaagtttaactaagctatactaaccccagggttggtcaatttcgtgccagccacaccctggtactgcatgcacgcaatgctagctgcccctttcccgtcctgggcaccccgagtctcccccgaccccgggtcccaggtatgctcccacctccacctgccccactcaccacctctgctagttccagacacctccgagacgaggaaaaaaaaaaaaaaaaaaaaaaaaaaaaaaaaaaaaaaaaaaaaaaaaaaaaaaaaaaaaaaaaaaaaaaaaaaaaaaaaaaaaaaaaaaaaaaaaaaaaaaaaaaaaaaaaaaaaaaaa

SEQ ID NO: 249 - RNA, 5425 nt, synthetic construct
  misc_feature 1..5425: note = mRNA of V8_3xGCN4-dCas9-KRAB
  source 1..5425: mol_type = other RNA
aggactcactatttgttttcgcgcccagttgcaaaaagtgtcgacatttgcttctgacacaactgtgttcactagcaacctcaaacagacaccgccaccatgcctgctgctaagagagtgaaactggatggatccgaggaactgctgagcaagaactaccacctggaaaacgaggtggccagactgaagaaaggctctggctctggcggaagcggttctggcggatcaggatctggaagtggcggctctggaagcggaggttctggatctggcgaagaactgctgtctaagaattatcacctcgagaacgaagtggctcggctcaagaaaggcagtggcagcggaggaagtggatccggcggtagtggtagtggaagcggcggatccggctcaggcggatctggttcaggggaagaactcctctccaaaaactaccatctcgagaatgaggtcgcccgcctgaaaaaaggatcaggttccggtggttctggcagcggtggttcaggctcaggcagcggcggtagcggtagcggtggaagcggaagcggaccaaaaaagaagagaaaggtaatggacaagaagtacagcatcggcctggccatcggcaccaactctgtgggctgggccgtgatcaccgacgagtacaaggtgcccagcaagaaattcaaggtgctgggcaacaccgaccggcacagcatcaagaagaacctgatcggcgccctgctgttcgacagcggagaaacagccgaggccacccggctgaagagaaccgccagaagaagatacaccagacggaagaaccggatctgctatctgcaagagatcttcagcaacgagatggccaaggtggacgacagcttcttccacagactggaagagtccttcctggtggaagaggataagaagcacgagcggcaccccatcttcggcaacatcgtggacgaggtggcctaccacgagaagtaccccaccatctaccacctgagaaagaaactggtggacagcaccgacaaggccgacctgcggctgatctatctggccctggcccacatgatcaagttccggggccacttcctgatcgagggcgacctgaaccccgacaacagcgacgtggacaagctgttcatccagctggtgcagacctacaaccagctgttcgaggaaaaccccatcaacgccagcggcgtggacgccaaggccatcctgtctgccagactgagcaagagcagacggctggaaaatctgatcgcccagctgcccggcgagaagaagaatggcctgttcggcaacctgattgccctgagcctgggcctgacccccaacttcaagagcaacttcgacctggccgaggatgccaaactgcagctgagcaaggacacctacgacgacgacctggacaacctgctggcccagatcggcgaccagtacgccgacctgtttctggccgccaagaacctgtccgacgccatcctgctgagcgacatcctgagagtgaacaccgagatcaccaaggcccccctgagcgcctctatgatcaagagatacgacgagcaccaccaggacctgaccctgctgaaagctctcgtgcggcagcagctgcctgagaagtacaaagagattttcttcgaccagagcaagaacggctacgccggctacatcgatggcggagccagccaggaagagttctacaagttcatcaagcccatcctggaaaagatggacggcaccgaggaactgctcgtgaagctgaacagagaggacctgctgcggaagcagcggaccttcgacaacggcagcatcccccaccagatccacctgggagagctgcacgccattctgcggcggcaggaagatttttacccattcctgaaggacaaccgggaaaagatcgagaagatcctgaccttccgcatcccctactacgtgggccctctggccaggggaaacagcagattcgcctggatgaccagaaagagcgaggaaaccatcaccccctggaacttcgaggaagtggtggacaagggcgccagcgcccagagcttcatcgagcggatgaccaacttcgataagaacctgcccaacgagaaggtgctgcccaagcacagcctgctgtacgagtacttcaccgtgtacaacgagctgaccaaagtgaaatacgtgaccgagggaatgagaaagcccgccttcctgagcggcgagcagaaaaaagccatcgtggacctgctgttcaagaccaaccggaaagtgaccgtgaagcagctgaaagaggactacttcaagaaaatcgagtgcttcgactccgtggaaatctccggcgtggaagatcggttcaacgcctccctgggcacataccacgatctgctgaaaattatcaaggacaaggacttcctggacaatgaggaaaacgaggacattctggaagatatcgtgctgaccctgacactgtttgaggacagagagatgatcgaggaacggctgaaaacctatgcccacctgttcgacgacaaagtgatgaagcagctgaagcggcggagatacaccggctggggcaggctgagccggaagctgatcaacggcatccgggacaagcagtccggcaagacaatcctggatttcctgaagtccgacggcttcgccaacagaaacttcatgcagctgatccacgacgacagcctgacctttaaagaggacatccagaaagcccaggtgtccggccagggcgatagcctgcacgagcacattgccaatctggccggcagccccgccattaagaagggcatcctgcagacagtgaaggtggtggacgagctcgtgaaagtgatgggccggcacaagcccgagaacatcgtgatcgaaatggccagagagaaccagaccacccagaagggacagaagaacagccgcgagagaatgaagcggatcgaagagggcatcaaagagctgggcagccagatcctgaaagaacaccccgtggaaaacacccagctgcagaacgagaagctgtacctgtactacctgcagaatgggcgggatatgtacgtggaccaggaactggacatcaaccggctgtccgactacgatgtggacgctatcgtgcctcagagctttctgaaggacgactccatcgataacaaagtgctgactcggagcgacaagaaccggggcaagagcgacaacgtgccctccgaagaggtcgtgaagaagatgaagaactactggcgccagctgctgaatgccaagctgattacccagaggaagttcgacaatctgaccaaggccgagagaggcggcctgagcgaactggataaggccggcttcatcaagagacagctggtggaaacccggcagatcacaaagcacgtggcacagatcctggactcccggatgaacactaagtacgacgagaacgacaaactgatccgggaagtgaaagtgatcaccctgaagtccaagctggtgtccgatttccggaaggatttccagttttacaaagtgcgcgagatcaacaactaccaccacgcccacgacgcctacctgaacgccgtcgtgggaaccgccctgatcaaaaagtaccctaagctggaaagcgagttcgtgtacggcgactacaaggtgtacgacgtgcggaagatgatcgccaagagcgagcaggaaatcggcaaggctaccgccaagtacttcttctacagcaacatcatgaactttttcaagaccgagattaccctggccaacggcgagatccggaagcggcctctgatcgagacaaacggcgaaacaggcgagatcgtgtgggataagggccgggactttgccaccgtgcggaaagtgctgtctatgccccaagtgaatatcgtgaaaaagaccgaggtgcagacaggcggcttcagcaaagagtctatcctgcccaagaggaacagcgacaagctgatcgccagaaagaaggactgggaccctaagaagtacggcggcttcgacagccccaccgtggcctattctgtgctggtggtggccaaagtggaaaagggcaagtccaagaaactgaagagtgtgaaagagctgctggggatcaccatcatggaaagaagcagcttcgagaagaatcccatcgactttctggaagccaagggctacaaagaagtgaaaaaggacctgatcatcaagctgcctaagtactccctgttcgagctggaaaacggccggaagagaatgctggcctctgccggcgaactgcagaagggaaacgaactggccctgccctccaaatatgtgaacttcctgtacctggccagccactatgagaagctgaagggctcccccgaggataatgagcagaaacagctgtttgtggaacagcacaaacactacctggacgagatcatcgagcagatcagcgagttctccaagagagtgatcctggccgacgctaatctggacaaggtgctgagcgcctacaacaagcacagagacaagcctatcagagagcaggccgagaatatcatccacctgtttaccctgaccaatctgggagcccctgccgccttcaagtactttgacaccaccatcgaccggaagaggtacaccagcaccaaagaggtgctggacgccaccctgatccaccagagcatcaccggcctgtacgagacacggatcgacctgtctcagctgggaggcgacgcctatccctatgacgtgcccgattatgccagcctgggcagcggctcccccaagaaaaaacgcaaggtggaagatcctaagaaaaagcggaaagtggacggcagcggcagcgagacccccggtaccagcgagagcgccacccccgagagccggacactggtgaccttcaaggatgtatttgtggacttcaccagggaggagtggaagctgctggacactgctcagcagatcgtgtacagaaatgtgatgctggagaactataagaacctggtttccttgggttatcagcttactaagccagatgtgatcctccggttggagaagggagaagagccctgagatcccaagcacgcagcaatgcagctcaaaacgcttagcctagccacacccccacgggaaacagcagtgattaacctttagcaataaacgaaagtttaactaagctatactaaccccagggttggtcaatttcgtgccagccacaccctggtactgcatgcacgcaatgctagctgcccctttcccgtcctgggcaccccgagtctcccccgaccccgggtcccaggtatgctcccacctccacctgccccactcaccacctctgctagttccagacacctccgagacgaggaaaaaaaaaaaaaaaaaaaaaaaaaaaaaaaaaaaaaaaaaaaaaaaaaaaaaaaaaaaaaaaaaaaaaaaaaaaaaaaaaaaaaaaaaaaaaaaaaaaaaaaaaaaaaaaaaaaaaaaa

SEQ ID NO: 250 - RNA, 1402 nt, synthetic construct
  misc_feature 1..1402: note = mRNA of V9_GFP1-10-KRAB
  source 1..1402: mol_type = other RNA
aggactcactatttgttttcgcgcccagttgcaaaaagtgtcgacatttgcttctgacacaactgtgttcactagcaacctcaaacagacaccgccaccatgcctgctgctaagagagtgaaactggatggatcctccaagggagaggagctgttcaccggagtggtgccaatcctggtggagctggacggcgatgtgaacggccacaagttttctgtgcgcggagagggagagggcgacgcaaccatcggcaagctgacactgaagttcatctgcaccacaggcaagctgcccgtgccttggccaaccctggtgaccacactgacatacggcgtgcagtgtttctctaggtatccagaccacatgaagagacacgatttctttaagagcgccatgccagagggatacgtgcaggagcggaccatctccttcaaggacgatggcaagtataagacccgcgccgtggtgaagtttgagggcgatacactggtgaacaggatcgagctgaagggcaccgacttcaaggaggatggcaatatcctgggccacaagctggagtacaactttaatagccacaacgtgtatatcacagccgacaagcagaagaacggcatcaaggccaacttcaccgtgaggcacaatgtggaggacggctccgtgcagctggccgatcactaccagcagaacacacctatcggcgacggacccgtgctgctgcctgataatcactatctgtccacccagacagtgctgtctaaggacccaaacgagaagttggatccaggtggaggtggaagcggtcggacactggtgaccttcaaggatgtatttgtggacttcaccagggaggagtggaagctgctggacactgctcagcagatcgtgtacagaaatgtgatgctggagaactataagaacctggtttccttgggttatcagcttactaagccagatgtgatcctccggttggagaagggagaagagccctgagatcccaagcacgcagcaatgcagctcaaaacgcttagcctagccacacccccacgggaaacagcagtgattaacctttagcaataaacgaaagtttaactaagctatactaaccccagggttggtcaatttcgtgccagccacaccctggtactgcatgcacgcaatgctagctgcccctttcccgtcctgggcaccccgagtctcccccgaccccgggtcccaggtatgctcccacctccacctgccccactcaccacctctgctagttccagacacctccgagacgaggaaaaaaaaaaaaaaaaaaaaaaaaaaaaaaaaaaaaaaaaaaaaaaaaaaaaaaaaaaaaaaaaaaaaaaaaaaaaaaaaaaaaaaaaaaaaaaaaaaaaaaaaaaaaaaaaaaaaaaaa

SEQ ID NO: 251 - RNA, 6880 nt, synthetic construct
  misc_feature 1..6880: note = mRNA of V10_D3a-D3l-dCas9-1xGFP11
  source 1..6880: mol_type = other RNA
aggactcactatttgttttcgcgcccagttgcaaaaagtgtcgacatttgcttctgacacaactgtgttcactagcaacctcaaacagacaccgccaccatgcctgctgctaagagagtgaaactggatggatccaaccatgaccaggaatttgaccccccaaaggtttacccacctgtgccagctgagaagaggaagcccatccgcgtgctgtctctctttgatgggattgctacagggctcctggtgctgaaggacctgggcatccaagtggaccgctacattgcctccgaggtgtgtgaggactccatcacggtgggcatggtgcggcaccagggaaagatcatgtacgtcggggacgtccgcagcgtcacacagaagcatatccaggagtggggcccattcgacctggtgattggaggcagtccctgcaatgacctctccattgtcaaccctgcccgcaagggactttatgagggtactggccgcctcttctttgagttctaccgcctcctgcatgatgcgcggcccaaggagggagatgatcgccccttcttctggctctttgagaatgtggtggccatgggcgttagtgacaagagggacatctcgcgatttcttgagtctaaccccgtgatgattgacgccaaagaagtgtctgctgcacacagggcccgttacttctggggtaaccttcctggcatgaacaggcctttggcatccactgtgaatgataagctggagctgcaagagtgtctggagcacggcagaatagccaagttcagcaaagtgaggaccattaccaccaggtcaaactctataaagcagggcaaagaccagcatttccccgtgttcatgaacgagaaggaggacatcctgtggtgcactgaaatggaaagggtgtttggcttccccgtccactacacagacgtctccaacatgagccgcttggcgaggcagagactgctgggccgatcgtggagcgtgccggtcatccgccacctcttcgctccgctgaaggaatattttgcttgtgtgtctagcggcaatagtaacgctaacagccgcgggccgagcttcagcagcggcctggtgccgttaagcttgcgcggcagccatatgggccctatggagatatacaagacagtgtctgcatggaagagacagccagtgcgggtactgagcctcttcagaaacatcgacaaggtactaaagagtttgggcttcttggaaagcggttctggttctgggggaggaacgctgaagtacgtggaagatgtcacaaatgtcgtgaggagagacgtggagaaatggggcccctttgacctggtgtacggctcgacgcagcccctaggcagctcttgtgatcgctgtcccggctggtacatgttccagttccaccggatcctgcagtatgcgctgcctcgccaggagagtcagcggcccttcttctggatattcatggacaatctgctgctgactgaggatgaccaagagacaactacccgcttccttcagacagaggctgtgaccctccaggatgtccgtggcagagactaccagaatgctatgcgggtgtggagcaacattccagggctgaagagcaagcatgcgcccctgaccccaaaggaagaagagtatctgcaagcccaagtcagaagcaggagcaagctggacgccccgaaagttgacctcctggtgaagaactgccttctcccgctgagagagtacttcaagtatttttctcaaaactcacttcctcttggagggccgagctctggcgcacccccaccaagtggagggtctcctgccgggtccccaacatctactgaagaaggcaccagcgaatccgcaacgcccgagtcaggccctggtacctccacagaaccatctgaaggtagtgcgcctggttccccagctggaagccctacttccaccgaagaaggcacgtcaaccgaaccaagtgaaggatctgcccctgggaccagcactgaaccatctgagccaaaaaagaagagaaaggtaatggacaagaagtacagcatcggcctggccatcggcaccaactctgtgggctgggccgtgatcaccgacgagtacaaggtgcccagcaagaaattcaaggtgctgggcaacaccgaccggcacagcatcaagaagaacctgatcggcgccctgctgttcgacagcggagaaacagccgaggccacccggctgaagagaaccgccagaagaagatacaccagacggaagaaccggatctgctatctgcaagagatcttcagcaacgagatggccaaggtggacgacagcttcttccacagactggaagagtccttcctggtggaagaggataagaagcacgagcggcaccccatcttcggcaacatcgtggacgaggtggcctaccacgagaagtaccccaccatctaccacctgagaaagaaactggtggacagcaccgacaaggccgacctgcggctgatctatctggccctggcccacatgatcaagttccggggccacttcctgatcgagggcgacctgaaccccgacaacagcgacgtggacaagctgttcatccagctggtgcagacctacaaccagctgttcgaggaaaaccccatcaacgccagcggcgtggacgccaaggccatcctgtctgccagactgagcaagagcagacggctggaaaatctgatcgcccagctgcccggcgagaagaagaatggcctgttcggcaacctgattgccctgagcctgggcctgacccccaacttcaagagcaacttcgacctggccgaggatgccaaactgcagctgagcaaggacacctacgacgacgacctggacaacctgctggcccagatcggcgaccagtacgccgacctgtttctggccgccaagaacctgtccgacgccatcctgctgagcgacatcctgagagtgaacaccgagatcaccaaggcccccctgagcgcctctatgatcaagagatacgacgagcaccaccaggacctgaccctgctgaaagctctcgtgcggcagcagctgcctgagaagtacaaagagattttcttcgaccagagcaagaacggctacgccggctacatcgatggcggagccagccaggaagagttctacaagttcatcaagcccatcctggaaaagatggacggcaccgaggaactgctcgtgaagctgaacagagaggacctgctgcggaagcagcggaccttcgacaacggcagcatcccccaccagatccacctgggagagctgcacgccattctgcggcggcaggaagatttttacccattcctgaaggacaaccgggaaaagatcgagaagatcctgaccttccgcatcccctactacgtgggccctctggccaggggaaacagcagattcgcctggatgaccagaaagagcgaggaaaccatcaccccctggaacttcgaggaagtggtggacaagggcgccagcgcccagagcttcatcgagcggatgaccaacttcgataagaacctgcccaacgagaaggtgctgcccaagcacagcctgctgtacgagtacttcaccgtgtacaacgagctgaccaaagtgaaatacgtgaccgagggaatgagaaagcccgccttcctgagcggcgagcagaaaaaagccatcgtggacctgctgttcaagaccaaccggaaagtgaccgtgaagcagctgaaagaggactacttcaagaaaatcgagtgcttcgactccgtggaaatctccggcgtggaagatcggttcaacgcctccctgggcacataccacgatctgctgaaaattatcaaggacaaggacttcctggacaatgaggaaaacgaggacattctggaagatatcgtgctgaccctgacactgtttgaggacagagagatgatcgaggaacggctgaaaacctatgcccacctgttcgacgacaaagtgatgaagcagctgaagcggcggagatacaccggctggggcaggctgagccggaagctgatcaacggcatccgggacaagcagtccggcaagacaatcctggatttcctgaagtccgacggcttcgccaacagaaacttcatgcagctgatccacgacgacagcctgacctttaaagaggacatccagaaagcccaggtgtccggccagggcgatagcctgcacgagcacattgccaatctggccggcagccccgccattaagaagggcatcctgcagacagtgaaggtggtggacgagctcgtgaaagtgatgggccggcacaagcccgagaacatcgtgatcgaaatggccagagagaaccagaccacccagaagggacagaagaacagccgcgagagaatgaagcggatcgaagagggcatcaaagagctgggcagccagatcctgaaagaacaccccgtggaaaacacccagctgcagaacgagaagctgtacctgtactacctgcagaatgggcgggatatgtacgtggaccaggaactggacatcaaccggctgtccgactacgatgtggacgctatcgtgcctcagagctttctgaaggacgactccatcgataacaaagtgctgactcggagcgacaagaaccggggcaagagcgacaacgtgccctccgaagaggtcgtgaagaagatgaagaactactggcgccagctgctgaatgccaagctgattacccagaggaagttcgacaatctgaccaaggccgagagaggcggcctgagcgaactggataaggccggcttcatcaagagacagctggtggaaacccggcagatcacaaagcacgtggcacagatcctggactcccggatgaacactaagtacgacgagaacgacaaactgatccgggaagtgaaagtgatcaccctgaagtccaagctggtgtccgatttccggaaggatttccagttttacaaagtgcgcgagatcaacaactaccaccacgcccacgacgcctacctgaacgccgtcgtgggaaccgccctgatcaaaaagtaccctaagctggaaagcgagttcgtgtacggcgactacaaggtgtacgacgtgcggaagatgatcgccaagagcgagcaggaaatcggcaaggctaccgccaagtacttcttctacagcaacatcatgaactttttcaagaccgagattaccctggccaacggcgagatccggaagcggcctctgatcgagacaaacggcgaaacaggcgagatcgtgtgggataagggccgggactttgccaccgtgcggaaagtgctgtctatgccccaagtgaatatcgtgaaaaagaccgaggtgcagacaggcggcttcagcaaagagtctatcctgcccaagaggaacagcgacaagctgatcgccagaaagaaggactgggaccctaagaagtacggcggcttcgacagccccaccgtggcctattctgtgctggtggtggccaaagtggaaaagggcaagtccaagaaactgaagagtgtgaaagagctgctggggatcaccatcatggaaagaagcagcttcgagaagaatcccatcgactttctggaagccaagggctacaaagaagtgaaaaaggacctgatcatcaagctgcctaagtactccctgttcgagctggaaaacggccggaagagaatgctggcctctgccggcgaactgcagaagggaaacgaactggccctgccctccaaatatgtgaacttcctgtacctggccagccactatgagaagctgaagggctcccccgaggataatgagcagaaacagctgtttgtggaacagcacaaacactacctggacgagatcatcgagcagatcagcgagttctccaagagagtgatcctggccgacgctaatctggacaaggtgctgagcgcctacaacaagcacagagacaagcctatcagagagcaggccgagaatatcatccacctgtttaccctgaccaatctgggagcccctgccgccttcaagtactttgacaccaccatcgaccggaagaggtacaccagcaccaaagaggtgctggacgccaccctgatccaccagagcatcaccggcctgtacgagacacggatcgacctgtctcagctgggaggcgacgcctatccctatgacgtgcccgattatgccagcctgggcagcggctcccccaagaaaaaacgcaaggtggaagatcctaagaaaaagcggaaagtggacggcagcggcagcgagacccccggtaccagcgagagcgccacccccgagagcggtagtgggagcaacggcagcagcggatccatgcgtgaccacatggtccttcatgagtatgtaaatgctgctgggattacaggtggctctggaggtgcggccgcaaggtcaggctccggccagcggggaagcaagcgcaccgccgatggttccgagttcgaaagccccaaaaaaaagcgcaaggtctgagatcccaagcacgcagcaatgcagctcaaaacgcttagcctagccacacccccacgggaaacagcagtgattaacctttagcaataaacgaaagtttaactaagctatactaaccccagggttggtcaatttcgtgccagccacaccctggtactgcatgcacgcaatgctagctgcccctttcccgtcctgggcaccccgagtctcccccgaccccgggtcccaggtatgctcccacctccacctgccccactcaccacctctgctagttccagacacctccgagacgaggaaaaaaaaaaaaaaaaaaaaaaaaaaaaaaaaaaaaaaaaaaaaaaaaaaaaaaaaaaaaaaaaaaaaaaaaaaaaaaaaaaaaaaaaaaaaaaaaaaaaaaaaaaaaaaaaaaaaaaaa

SEQ ID NO: 252 - RNA, 7243 nt, synthetic construct
  misc_feature 1..7243: note = mRNA of V11_D3a-D3l-dCas9-8xGFP11
  source 1..7243: mol_type = other RNA
aggactcactatttgttttcgcgcccagttgcaaaaagtgtcgacatttgcttctgacacaactgtgttcactagcaacctcaaacagacaccgccaccatgcctgctgctaagagagtgaaactggatggatccaaccatgaccaggaatttgaccccccaaaggtttacccacctgtgccagctgagaagaggaagcccatccgcgtgctgtctctctttgatgggattgctacagggctcctggtgctgaaggacctgggcatccaagtggaccgctacattgcctccgaggtgtgtgaggactccatcacggtgggcatggtgcggcaccagggaaagatcatgtacgtcggggacgtccgcagcgtcacacagaagcatatccaggagtggggcccattcgacctggtgattggaggcagtccctgcaatgacctctccattgtcaaccctgcccgcaagggactttatgagggtactggccgcctcttctttgagttctaccgcctcctgcatgatgcgcggcccaaggagggagatgatcgccccttcttctggctctttgagaatgtggtggccatgggcgttagtgacaagagggacatctcgcgatttcttgagtctaaccccgtgatgattgacgccaaagaagtgtctgctgcacacagggcccgttacttctggggtaaccttcctggcatgaacaggcctttggcatccactgtgaatgataagctggagctgcaagagtgtctggagcacggcagaatagccaagttcagcaaagtgaggaccattaccaccaggtcaaactctataaagcagggcaaagaccagcatttccccgtgttcatgaacgagaaggaggacatcctgtggtgcactgaaatggaaagggtgtttggcttccccgtccactacacagacgtctccaacatgagccgcttggcgaggcagagactgctgggccgatcgtggagcgtgccggtcatccgccacctcttcgctccgctgaaggaatattttgcttgtgtgtctagcggcaatagtaacgctaacagccgcgggccgagcttcagcagcggcctggtgccgttaagcttgcgcggcagccatatgggccctatggagatatacaagacagtgtctgcatggaagagacagccagtgcgggtactgagcctcttcagaaacatcgacaaggtactaaagagtttgggcttcttggaaagcggttctggttctgggggaggaacgctgaagtacgtggaagatgtcacaaatgtcgtgaggagagacgtggagaaatggggcccctttgacctggtgtacggctcgacgcagcccctaggcagctcttgtgatcgctgtcccggctggtacatgttccagttccaccggatcctgcagtatgcgctgcctcgccaggagagtcagcggcccttcttctggatattcatggacaatctgctgctgactgaggatgaccaagagacaactacccgcttccttcagacagaggctgtgaccctccaggatgtccgtggcagagactaccagaatgctatgcgggtgtggagcaacattccagggctgaagagcaagcatgcgcccctgaccccaaaggaagaagagtatctgcaagcccaagtcagaagcaggagcaagctggacgccccgaaagttgacctcctggtgaagaactgccttctcccgctgagagagtacttcaagtatttttctcaaaactcacttcctcttggagggccgagctctggcgcacccccaccaagtggagggtctcctgccgggtccccaacatctactgaagaaggcaccagcgaatccgcaacgcccgagtcaggccctggtacctccacagaaccatctgaaggtagtgcgcctggttccccagctggaagccctacttccaccgaagaaggcacgtcaaccgaaccaagtgaaggatctgcccctgggaccagcactgaaccatctgagccaaaaaagaagagaaaggtaatggacaagaagtacagcatcggcctggccatcggcaccaactctgtgggctgggccgtgatcaccgacgagtacaaggtgcccagcaagaaattcaaggtgctgggcaacaccgaccggcacagcatcaagaagaacctgatcggcgccctgctgttcgacagcggagaaacagccgaggccacccggctgaagagaaccgccagaagaagatacaccagacggaagaaccggatctgctatctgcaagagatcttcagcaacgagatggccaaggtggacgacagcttcttccacagactggaagagtccttcctggtggaagaggataagaagcacgagcggcaccccatcttcggcaacatcgtggacgaggtggcctaccacgagaagtaccccaccatctaccacctgagaaagaaactggtggacagcaccgacaaggccgacctgcggctgatctatctggccctggcccacatgatcaagttccggggccacttcctgatcgagggcgacctgaaccccgacaacagcgacgtggacaagctgttcatccagctggtgcagacctacaaccagctgttcgaggaaaaccccatcaacgccagcggcgtggacgccaaggccatcctgtctgccagactgagcaagagcagacggctggaaaatctgatcgcccagctgcccggcgagaagaagaatggcctgttcggcaacctgattgccctgagcctgggcctgacccccaacttcaagagcaacttcgacctggccgaggatgccaaactgcagctgagcaaggacacctacgacgacgacctggacaacctgctggcccagatcggcgaccagtacgccgacctgtttctggccgccaagaacctgtccgacgccatcctgctgagcgacatcctgagagtgaacaccgagatcaccaaggcccccctgagcgcctctatgatcaagagatacgacgagcaccaccaggacctgaccctgctgaaagctctcgtgcggcagcagctgcctgagaagtacaaagagattttcttcgaccagagcaagaacggctacgccggctacatcgatggcggagccagccaggaagagttctacaagttcatcaagcccatcctggaaaagatggacggcaccgaggaactgctcgtgaagctgaacagagaggacctgctgcggaagcagcggaccttcgacaacggcagcatcccccaccagatccacctgggagagctgcacgccattctgcggcggcaggaagatttttacccattcctgaaggacaaccgggaaaagatcgagaagatcctgaccttccgcatcccctactacgtgggccctctggccaggggaaacagcagattcgcctggatgaccagaaagagcgaggaaaccatcaccccctggaacttcgaggaagtggtggacaagggcgccagcgcccagagcttcatcgagcggatgaccaacttcgataagaacctgcccaacgagaaggtgctgcccaagcacagcctgctgtacgagtacttcaccgtgtacaacgagctgaccaaagtgaaatacgtgaccgagggaatgagaaagcccgccttcctgagcggcgagcagaaaaaagccatcgtggacctgctgttcaagaccaaccggaaagtgaccgtgaagcagctgaaagaggactacttcaagaaaatcgagtgcttcgactccgtggaaatctccggcgtggaagatcggttcaacgcctccctgggcacataccacgatctgctgaaaattatcaaggacaaggacttcctggacaatgaggaaaacgaggacattctggaagatatcgtgctgaccctgacactgtttgaggacagagagatgatcgaggaacggctgaaaacctatgcccacctgttcgacgacaaagtgatgaagcagctgaagcggcggagatacaccggctggggcaggctgagccggaagctgatcaacggcatccgggacaagcagtccggcaagacaatcctggatttcctgaagtccgacggcttcgccaacagaaacttcatgcagctgatccacgacgacagcctgacctttaaagaggacatccagaaagcccaggtgtccggccagggcgatagcctgcacgagcacattgccaatctggccggcagccccgccattaagaagggcatcctgcagacagtgaaggtggtggacgagctcgtgaaagtgatgggccggcacaagcccgagaacatcgtgatcgaaatggccagagagaaccagaccacccagaagggacagaagaacagccgcgagagaatgaagcggatcgaagagggcatcaaagagctgggcagccagatcctgaaagaacaccccgtggaaaacacccagctgcagaacgagaagctgtacctgtactacctgcagaatgggcgggatatgtacgtggaccaggaactggacatcaaccggctgtccgactacgatgtggacgctatcgtgcctcagagctttctgaaggacgactccatcgataacaaagtgctgactcggagcgacaagaaccggggcaagagcgacaacgtgccctccgaagaggtcgtgaagaagatgaagaactactggcgccagctgctgaatgccaagctgattacccagaggaagttcgacaatctgaccaaggccgagagaggcggcctgagcgaactggataaggccggcttcatcaagagacagctggtggaaacccggcagatcacaaagcacgtggcacagatcctggactcccggatgaacactaagtacgacgagaacgacaaactgatccgggaagtgaaagtgatcaccctgaagtccaagctggtgtccgatttccggaaggatttccagttttacaaagtgcgcgagatcaacaactaccaccacgcccacgacgcctacctgaacgccgtcgtgggaaccgccctgatcaaaaagtaccctaagctggaaagcgagttcgtgtacggcgactacaaggtgtacgacgtgcggaagatgatcgccaagagcgagcaggaaatcggcaaggctaccgccaagtacttcttctacagcaacatcatgaactttttcaagaccgagattaccctggccaacggcgagatccggaagcggcctctgatcgagacaaacggcgaaacaggcgagatcgtgtgggataagggccgggactttgccaccgtgcggaaagtgctgtctatgccccaagtgaatatcgtgaaaaagaccgaggtgcagacaggcggcttcagcaaagagtctatcctgcccaagaggaacagcgacaagctgatcgccagaaagaaggactgggaccctaagaagtacggcggcttcgacagccccaccgtggcctattctgtgctggtggtggccaaagtggaaaagggcaagtccaagaaactgaagagtgtgaaagagctgctggggatcaccatcatggaaagaagcagcttcgagaagaatcccatcgactttctggaagccaagggctacaaagaagtgaaaaaggacctgatcatcaagctgcctaagtactccctgttcgagctggaaaacggccggaagagaatgctggcctctgccggcgaactgcagaagggaaacgaactggccctgccctccaaatatgtgaacttcctgtacctggccagccactatgagaagctgaagggctcccccgaggataatgagcagaaacagctgtttgtggaacagcacaaacactacctggacgagatcatcgagcagatcagcgagttctccaagagagtgatcctggccgacgctaatctggacaaggtgctgagcgcctacaacaagcacagagacaagcctatcagagagcaggccgagaatatcatccacctgtttaccctgaccaatctgggagcccctgccgccttcaagtactttgacaccaccatcgaccggaagaggtacaccagcaccaaagaggtgctggacgccaccctgatccaccagagcatcaccggcctgtacgagacacggatcgacctgtctcagctgggaggcgacgcctatccctatgacgtgcccgattatgccagcctgggcagcggctcccccaagaaaaaacgcaaggtggaagatcctaagaaaaagcggaaagtggacggcagcggcagcgagacccccggtaccagcgagagcgccacccccgagagcggtagtgggagcaacggcagcagcggatccatgcgtgaccacatggtccttcatgagtatgtaaatgctgctgggattacaggtggctctggaggtagagatcatatggttctccacgaatacgttaacgccgcaggcatcactggcggtagtggaggacgcgaccatatggtactacatgaatatgtcaatgcagccggaataaccggagggtccggaggccgggatcacatggtgctgcatgagtatgtgaacgcggcgggtataactggtgggtcgggcggacgagaccatatggtgcttcacgaatacgtaaacgcagctggcattactggcggatcaggtggcagggatcacatggtactccatgagtacgtgaacgctgctggaatcacaggcggtagcggcggtcgggaccatatggtcctgcacgaatatgtcaatgctgccggtatcaccgcggccgcaaggtcaggctccggccagcggggaagcaagcgcaccgccgatggttccgagttcgaaagccccaaaaaaaagcgcaaggtctgagatcccaagcacgcagcaatgcagctcaaaacgcttagcctagccacacccccacgggaaacagcagtgattaacctttagcaataaacgaaagtttaactaagctatactaaccccagggttggtcaatttcgtgccagccacaccctggtactgcatgcacgcaatgctagctgcccctttcccgtcctgggcaccccgagtctcccccgaccccgggtcccaggtatgctcccacctccacctgccccactcaccacctctgctagttccagacacctccgagacgaggaaaaaaaaaaaaaaaaaaaaaaaaaaaaaaaaaaaaaaaaaaaaaaaaaaaaaaaaaaaaaaaaaaaaaaaaaaaaaaaaaaaaaaaaaaaaaaaaaaaaaaaaaaaaaaaaaaaaaaaa

SEQ ID NO: 253 - RNA, 8062 nt, synthetic construct
  misc_feature 1..8062: note = mRNA of V12_scFv-KRAB-2a-D3a-D3l-dCas9-1xGCN4
  source 1..8062: mol_type = other RNA
aggactcactatttgttttcgcgcccagttgcaaaaagtgtcgacatttgcttctgacacaactgtgttcactagcaacctcaaacagacaccgccaccatgggccccgacatcgtgatgacccagagccccagcagcctgagcgccagcgtgggcgaccgcgtgaccatcacctgccgcagcagcaccggcgccgtgaccaccagcaactacgccagctgggtgcaggagaagcccggcaagctgttcaagggcctgatcggcggcaccaacaaccgcgcccccggcgtgcccagccgcttcagcggcagcctgatcggcgacaaggccaccctgaccatcagcagcctgcagcccgaggacttcgccacctacttctgcgccctgtggtacagcaaccactgggtgttcggccagggcaccaaggtggagctgaagcgcggcggcggcggcagcggcggcggcggcagcggcggcggcggcagcagcggcggcggcagcgaggtgaagctgctggagagcggcggcggcctggtgcagcccggcggcagcctgaagctgagctgcgccgtgagcggcttcagcctgaccgactacggcgtgaactgggtgcgccaggcccccggccgcggcctggagtggatcggcgtgatctggggcgacggcatcaccgactacaacagcgccctgaaggaccgcttcatcatcagcaaggacaacggcaagaacaccgtgtacctgcagatgagcaaggtgcgcagcgacgacaccgccctgtactactgcgtgaccggcctgttcgactactggggccagggcaccctggtgaccgtgagcagctacccatacgatgttccagattacgctggtggaggcggaggttctgggggaggaggtagtggcggtggtggttcaggaggcggcggaagcttggatccaggtggaggtggaagcggtcggacactggtgaccttcaaggatgtatttgtggacttcaccagggaggagtggaagctgctggacactgctcagcagatcgtgtacagaaatgtgatgctggagaactataagaacctggtttccttgggttatcagcttactaagccagatgtgatcctccggttggagaagggagaagagcccggaagcggaaagcgcaccgccgatggttccgagttcgaaagccccaaaaaaaagcgcaaggtcggaagcggagctactaacttcagcctgctgaagcaggctggagacgtggaggagaaccctggacctatgaaccatgaccaggaatttgaccccccaaaggtttacccacctgtgccagctgagaagaggaagcccatccgcgtgctgtctctctttgatgggattgctacagggctcctggtgctgaaggacctgggcatccaagtggaccgctacattgcctccgaggtgtgtgaggactccatcacggtgggcatggtgcggcaccagggaaagatcatgtacgtcggggacgtccgcagcgtcacacagaagcatatccaggagtggggcccattcgacctggtgattggaggcagtccctgcaatgacctctccattgtcaaccctgcccgcaagggactttatgagggtactggccgcctcttctttgagttctaccgcctcctgcatgatgcgcggcccaaggagggagatgatcgccccttcttctggctctttgagaatgtggtggccatgggcgttagtgacaagagggacatctcgcgatttcttgagtctaaccccgtgatgattgacgccaaagaagtgtctgctgcacacagggcccgttacttctggggtaaccttcctggcatgaacaggcctttggcatccactgtgaatgataagctggagctgcaagagtgtctggagcacggcagaatagccaagttcagcaaagtgaggaccattaccaccaggtcaaactctataaagcagggcaaagaccagcatttccccgtcttcatgaacgagaaggaggacatcctgtggtgcactgaaatggaaagggtgtttggcttccccgtccactacacagacgtctccaacatgagccgcttggcgaggcagagactgctgggccgatcgtggagcgtgccggtcatccgccacctcttcgctccgctgaaggaatattttgcttgtgtgtctagcggcaatagtaacgctaacagccgcgggccgagcttcagcagcggcctggtgccgttaagcttgcgcggcagccatatgggccctatggagatatacaagacagtgtctgcatggaagagacagccagtgcgggtactgagcctcttcagaaacatcgacaaggtactaaagagtttgggcttcttggaaagcggttctggttctgggggaggaacgctgaagtacgtggaagatgtcacaaatgtcgtgaggagagacgtggagaaatggggcccctttgacctggtgtacggctcgacgcagcccctaggcagctcttgtgatcgctgtcccggctggtacatgttccagttccaccggatcctgcagtatgcgctgcctcgccaggagagtcagcggcccttcttctggatattcatggacaatctgctgctgactgaggatgaccaagagacaactacccgcttccttcagacagaggctgtgaccctccaggatgtccgtggcagagactaccagaatgctatgcgggtgtggagcaacattccagggctgaagagcaagcatgcgcccctgaccccaaaggaagaagagtatctgcaagcccaagtcagaagcaggagcaagctggacgccccgaaagttgacctcctggtgaagaactgccttctcccgctgagagagtacttcaagtatttttctcaaaactcacttcctcttggagggccgagctctggcgcacccccaccaagtggagggtctcctgccgggtccccaacatctactgaagaaggcaccagcgaatccgcaacgcccgagtcaggccctggtacctccacagaaccatctgaaggtagtgcgcctggttccccagctggaagccctacttccaccgaagaaggcacgtcaaccgaaccaagtgaaggatctgcccctgggaccagcactgaaccatctgagccaaaaaagaagagaaaggtaatggacaagaagtacagcatcggcctggccatcggcaccaactctgtgggctgggccgtgatcaccgacgagtacaaggtgcccagcaagaaattcaaggtgctgggcaacaccgaccggcacagcatcaagaagaacctgatcggcgccctgctgttcgacagcggagaaacagccgaggccacccggctgaagagaaccgccagaagaagatacaccagacggaagaaccggatctgctatctgcaagagatcttcagcaacgagatggccaaggtggacgacagcttcttccacagactggaagagtccttcctggtggaagaggataagaagcacgagcggcaccccatcttcggcaacatcgtggacgaggtggcctaccacgagaagtaccccaccatctaccacctgagaaagaaactggtggacagcaccgacaaggccgacctgcggctgatctatctggccctggcccacatgatcaagttccggggccacttcctgatcgagggcgacctgaaccccgacaacagcgacgtggacaagctgttcatccagctggtgcagacctacaaccagctgttcgaggaaaaccccatcaacgccagcggcgtggacgccaaggccatcctgtctgccagactgagcaagagcagacggctggaaaatctgatcgcccagctgcccggcgagaagaagaatggcctgttcggcaacctgattgccctgagcctgggcctgacccccaacttcaagagcaacttcgacctggccgaggatgccaaactgcagctgagcaaggacacctacgacgacgacctggacaacctgctggcccagatcggcgaccagtacgccgacctgtttctggccgccaagaacctgtccgacgccatcctgctgagcgacatcctgagagtgaacaccgagatcaccaaggcccccctgagcgcctctatgatcaagagatacgacgagcaccaccaggacctgaccctgctgaaagctctcgtgcggcagcagctgcctgagaagtacaaagagattttcttcgaccagagcaagaacggctacgccggctacatcgatggcggagccagccaggaagagttctacaagttcatcaagcccatcctggaaaagatggacggcaccgaggaactgctcgtgaagctgaacagagaggacctgctgcggaagcagcggaccttcgacaacggcagcatcccccaccagatccacctgggagagctgcacgccattctgcggcggcaggaagatttttacccattcctgaaggacaaccgggaaaagatcgagaagatcctgaccttccgcatcccctactacgtgggccctctggccaggggaaacagcagattcgcctggatgaccagaaagagcgaggaaaccatcaccccctggaacttcgaggaagtggtggacaagggcgccagcgcccagagcttcatcgagcggatgaccaacttcgataagaacctgcccaacgagaaggtgctgcccaagcacagcctgctgtacgagtacttcaccgtgtacaacgagctgaccaaagtgaaatacgtgaccgagggaatgagaaagcccgccttcctgagcggcgagcagaaaaaagccatcgtggacctgctgttcaagaccaaccggaaagtgaccgtgaagcagctgaaagaggactacttcaagaaaatcgagtgcttcgactccgtggaaatctccggcgtggaagatcggttcaacgcctccctgggcacataccacgatctgctgaaaattatcaaggacaaggacttcctggacaatgaggaaaacgaggacattctggaagatatcgtgctgaccctgacactgtttgaggacagagagatgatcgaggaacggctgaaaacctatgcccacctgttcgacgacaaagtgatgaagcagctgaagcggcggagatacaccggctggggcaggctgagccggaagctgatcaacggcatccgggacaagcagtccggcaagacaatcctggatttcctgaagtccgacggcttcgccaacagaaacttcatgcagctgatccacgacgacagcctgacctttaaagaggacatccagaaagcccaggtgtccggccagggcgatagcctgcacgagcacattgccaatctggccggcagccccgccattaagaagggcatcctgcagacagtgaaggtggtggacgagctcgtgaaagtgatgggccggcacaagcccgagaacatcgtgatcgaaatggccagagagaaccagaccacccagaagggacagaagaacagccgcgagagaatgaagcggatcgaagagggcatcaaagagctgggcagccagatcctgaaagaacaccccgtggaaaacacccagctgcagaacgagaagctgtacctgtactacctgcagaatgggcgggatatgtacgtggaccaggaactggacatcaaccggctgtccgactacgatgtggacgctatcgtgcctcagagctttctgaaggacgactccatcgataacaaagtgctgactcggagcgacaagaaccggggcaagagcgacaacgtgccctccgaagaggtcgtgaagaagatgaagaactactggcgccagctgctgaatgccaagctgattacccagaggaagttcgacaatctgaccaaggccgagagaggcggcctgagcgaactggataaggccggcttcatcaagagacagctggtggaaacccggcagatcacaaagcacgtggcacagatcctggactcccggatgaacactaagtacgacgagaacgacaaactgatccgggaagtgaaagtgatcaccctgaagtccaagctggtgtccgatttccggaaggatttccagttttacaaagtgcgcgagatcaacaactaccaccacgcccacgacgcctacctgaacgccgtcgtgggaaccgccctgatcaaaaagtaccctaagctggaaagcgagttcgtgtacggcgactacaaggtgtacgacgtgcggaagatgatcgccaagagcgagcaggaaatcggcaaggctaccgccaagtacttcttctacagcaacatcatgaactttttcaagaccgagattaccctggccaacggcgagatccggaagcggcctctgatcgagacaaacggcgaaacaggcgagatcgtgtgggataagggccgggactttgccaccgtgcggaaagtgctgtctatgccccaagtgaatatcgtgaaaaagaccgaggtgcagacaggcggcttcagcaaagagtctatcctgcccaagaggaacagcgacaagctgatcgccagaaagaaggactgggaccctaagaagtacggcggcttcgacagccccaccgtggcctattctgtgctggtggtggccaaagtggaaaagggcaagtccaagaaactgaagagtgtgaaagagctgctggggatcaccatcatggaaagaagcagcttcgagaagaatcccatcgactttctggaagccaagggctacaaagaagtgaaaaaggacctgatcatcaagctgcctaagtactccctgttcgagctggaaaacggccggaagagaatgctggcctctgccggcgaactgcagaagggaaacgaactggccctgccctccaaatatgtgaacttcctgtacctggccagccactatgagaagctgaagggctcccccgaggataatgagcagaaacagctgtttgtggaacagcacaaacactacctggacgagatcatcgagcagatcagcgagttctccaagagagtgatcctggccgacgctaatctggacaaggtgctgagcgcctacaacaagcacagagacaagcctatcagagagcaggccgagaatatcatccacctgtttaccctgaccaatctgggagcccctgccgccttcaagtactttgacaccaccatcgaccggaagaggtacaccagcaccaaagaggtgctggacgccaccctgatccaccagagcatcaccggcctgtacgagacacggatcgacctgtctcagctgggaggcgacgcctatccctatgacgtgcccgattatgccagcctgggcagcggctcccccaagaaaaaacgcaaggtggaagatcctaagaaaaagcggaaagtggacggcattggtagtgggagcaacggcagcagcggagaggaactgctgagcaagaactaccacctggaaaacgaggtggccagactgaagaaaggctctggctctggcggaagcggttctggcggatcaggatctggaagtggcggctctggaagcggaggttctggatctggcgaagaactgctgtctaagaattatcacggttcaggctccggccagcggggaagcaagcgcaccgccgatggttccgagttcgaaagccccaaaaaaaagcgcaaggtctgagatcccaagcacgcagcaatgcagctcaaaacgcttagcctagccacacccccacgggaaacagcagtgattaacctttagcaataaacgaaagtttaactaagctatactaaccccagggttggtcaatttcgtgccagccacaccctggtactgcatgcacgcaatgctagctgcccctttcccgtcctgggcaccccgagtctcccccgaccccgggtcccaggtatgctcccacctccacctgccccactcaccacctctgctagttccagacacctccgagacgaggaaaaaaaaaaaaaaaaaaaaaaaaaaaaaaaaaaaaaaaaaaaaaaaaaaaaaaaaaaaaaaaaaaaaaaaaaaaaaaaaaaaaaaaaaaaaaaaaaaaaaaaaaaaaaaaaaaaaaaaa

SEQ ID NO: 254 - RNA, 8092 nt, synthetic construct
  misc_feature 1..8092: note = mRNA of V13_scFv-KRAB-2a-D3a-D3l-dCas9-2xGCN4
  source 1..8092: mol_type = other RNA
aggactcactatttgttttcgcgcccagttgcaaaaagtgtcgacatttgcttctgacacaactgtgttcactagcaacctcaaacagacaccgccaccatgggccccgacatcgtgatgacccagagccccagcagcctgagcgccagcgtgggcgaccgcgtgaccatcacctgccgcagcagcaccggcgccgtgaccaccagcaactacgccagctgggtgcaggagaagcccggcaagctgttcaagggcctgatcggcggcaccaacaaccgcgcccccggcgtgcccagccgcttcagcggcagcctgatcggcgacaaggccaccctgaccatcagcagcctgcagcccgaggacttcgccacctacttctgcgccctgtggtacagcaaccactgggtgttcggccagggcaccaaggtggagctgaagcgcggcggcggcggcagcggcggcggcggcagcggcggcggcggcagcagcggcggcggcagcgaggtgaagctgctggagagcggcggcggcctggtgcagcccggcggcagcctgaagctgagctgcgccgtgagcggcttcagcctgaccgactacggcgtgaactgggtgcgccaggcccccggccgcggcctggagtggatcggcgtgatctggggcgacggcatcaccgactacaacagcgccctgaaggaccgcttcatcatcagcaaggacaacggcaagaacaccgtgtacctgcagatgagcaaggtgcgcagcgacgacaccgccctgtactactgcgtgaccggcctgttcgactactggggccagggcaccctggtgaccgtgagcagctacccatacgatgttccagattacgctggtggaggcggaggttctgggggaggaggtagtggcggtggtggttcaggaggcggcggaagcttggatccaggtggaggtggaagcggtcggacactggtgaccttcaaggatgtatttgtggacttcaccagggaggagtggaagctgctggacactgctcagcagatcgtgtacagaaatgtgatgctggagaactataagaacctggtttccttgggttatcagcttactaagccagatgtgatcctccggttggagaagggagaagagcccggaagcggaaagcgcaccgccgatggttccgagttcgaaagccccaaaaaaaagcgcaaggtcggaagcggagctactaacttcagcctgctgaagcaggctggagacgtggaggagaaccctggacctatgaaccatgaccaggaatttgaccccccaaaggtttacccacctgtgccagctgagaagaggaagcccatccgcgtgctgtctctctttgatgggattgctacagggctcctggtgctgaaggacctgggcatccaagtggaccgctacattgcctccgaggtgtgtgaggactccatcacggtgggcatggtgcggcaccagggaaagatcatgtacgtcggggacgtccgcagcgtcacacagaagcatatccaggagtggggcccattcgacctggtgattggaggcagtccctgcaatgacctctccattgtcaaccctgcccgcaagggactttatgagggtactggccgcctcttctttgagttctaccgcctcctgcatgatgcgcggcccaaggagggagatgatcgccccttcttctggctctttgagaatgtggtggccatgggcgttagtgacaagagggacatctcgcgatttcttgagtctaaccccgtgatgattgacgccaaagaagtgtctgctgcacacagggcccgttacttctggggtaaccttcctggcatgaacaggcctttggcatccactgtgaatgataagctggagctgcaagagtgtctggagcacggcagaatagccaagttcagcaaagtgaggaccattaccaccaggtcaaactctataaagcagggcaaagaccagcatttccccgtcttcatgaacgagaaggaggacatcctgtggtgcactgaaatggaaagggtgtttggcttccccgtccactacacagacgtctccaacatgagccgcttggcgaggcagagactgctgggccgatcgtggagcgtgccggtcatccgccacctcttcgctccgctgaaggaatattttgcttgtgtgtctagcggcaatagtaacgctaacagccgcgggccgagcttcagcagcggcctggtgccgttaagcttgcgcggcagccatatgggccctatggagatatacaagacagtgtctgcatggaagagacagccagtgcgggtactgagcctcttcagaaacatcgacaaggtactaaagagtttgggcttcttggaaagcggttctggttctgggggaggaacgctgaagtacgtggaagatgtcacaaatgtcgtgaggagagacgtggagaaatggggcccctttgacctggtgtacggctcgacgcagcccctaggcagctcttgtgatcgctgtcccggctggtacatgttccagttccaccggatcctgcagtatgcgctgcctcgccaggagagtcagcggcccttcttctggatattcatggacaatctgctgctgactgaggatgaccaagagacaactacccgcttccttcagacagaggctgtgaccctccaggatgtccgtggcagagactaccagaatgctatgcgggtgtggagcaacattccagggctgaagagcaagcatgcgcccctgaccccaaaggaagaagagtatctgcaagcccaagtcagaagcaggagcaagctggacgccccgaaagttgacctcctggtgaagaactgccttctcccgctgagagagtacttcaagtatttttctcaaaactcacttcctcttggagggccgagctctggcgcacccccaccaagtggagggtctcctgccgggtccccaacatctactgaagaaggcaccagcgaatccgcaacgcccgagtcaggccctggtacctccacagaaccatctgaaggtagtgcgcctggttccccagctggaagccctacttccaccgaagaaggcacgtcaaccgaaccaagtgaaggatctgcccctgggaccagcactgaaccatctgagccaaaaaagaagagaaaggtaatggacaagaagtacagcatcggcctggccatcggcaccaactctgtgggctgggccgtgatcaccgacgagtacaaggtgcccagcaagaaattcaaggtgctgggcaacaccgaccggcacagcatcaagaagaacctgatcggcgccctgctgttcgacagcggagaaacagccgaggccacccggctgaagagaaccgccagaagaagatacaccagacggaagaaccggatctgctatctgcaagagatcttcagcaacgagatggccaaggtggacgacagcttcttccacagactggaagagtccttcctggtggaagaggataagaagcacgagcggcaccccatcttcggcaacatcgtggacgaggtggcctaccacgagaagtaccccaccatctaccacctgagaaagaaactggtggacagcaccgacaaggccgacctgcggctgatctatctggccctggcccacatgatcaagttccggggccacttcctgatcgagggcgacctgaaccccgacaacagcgacgtggacaagctgttcatccagctggtgcagacctacaaccagctgttcgaggaaaaccccatcaacgccagcggcgtggacgccaaggccatcctgtctgccagactgagcaagagcagacggctggaaaatctgatcgcccagctgcccggcgagaagaagaatggcctgttcggcaacctgattgccctgagcctgggcctgacccccaacttcaagagcaacttcgacctggccgaggatgccaaactgcagctgagcaaggacacctacgacgacgacctggacaacctgctggcccagatcggcgaccagtacgccgacctgtttctggccgccaagaacctgtccgacgccatcctgctgagcgacatcctgagagtgaacaccgagatcaccaaggcccccctgagcgcctctatgatcaagagatacgacgagcaccaccaggacctgaccctgctgaaagctctcgtgcggcagcagctgcctgagaagtacaaagagattttcttcgaccagagcaagaacggctacgccggctacatcgatggcggagccagccaggaagagttctacaagttcatcaagcccatcctggaaaagatggacggcaccgaggaactgctcgtgaagctgaacagagaggacctgctgcggaagcagcggaccttcgacaacggcagcatcccccaccagatccacctgggagagctgcacgccattctgcggcggcaggaagatttttacccattcctgaaggacaaccgggaaaagatcgagaagatcctgaccttccgcatcccctactacgtgggccctctggccaggggaaacagcagattcgcctggatgaccagaaagagcgaggaaaccatcaccccctggaacttcgaggaagtggtggacaagggcgccagcgcccagagcttcatcgagcggatgaccaacttcgataagaacctgcccaacgagaaggtgctgcccaagcacagcctgctgtacgagtacttcaccgtgtacaacgagctgaccaaagtgaaatacgtgaccgagggaatgagaaagcccgccttcctgagcggcgagcagaaaaaagccatcgtggacctgctgttcaagaccaaccggaaagtgaccgtgaagcagctgaaagaggactacttcaagaaaatcgagtgcttcgactccgtggaaatctccggcgtggaagatcggttcaacgcctccctgggcacataccacgatctgctgaaaattatcaaggacaaggacttcctggacaatgaggaaaacgaggacattctggaagatatcgtgctgaccctgacactgtttgaggacagagagatgatcgaggaacggctgaaaacctatgcccacctgttcgacgacaaagtgatgaagcagctgaagcggcggagatacaccggctggggcaggctgagccggaagctgatcaacggcatccgggacaagcagtccggcaagacaatcctggatttcctgaagtccgacggcttcgccaacagaaacttcatgcagctgatccacgacgacagcctgacctttaaagaggacatccagaaagcccaggtgtccggccagggcgatagcctgcacgagcacattgccaatctggccggcagccccgccattaagaagggcatcctgcagacagtgaaggtggtggacgagctcgtgaaagtgatgggccggcacaagcccgagaacatcgtgatcgaaatggccagagagaaccagaccacccagaagggacagaagaacagccgcgagagaatgaagcggatcgaagagggcatcaaagagctgggcagccagatcctgaaagaacaccccgtggaaaacacccagctgcagaacgagaagctgtacctgtactacctgcagaatgggcgggatatgtacgtggaccaggaactggacatcaaccggctgtccgactacgatgtggacgctatcgtgcctcagagctttctgaaggacgactccatcgataacaaagtgctgactcggagcgacaagaaccggggcaagagcgacaacgtgccctccgaagaggtcgtgaagaagatgaagaactactggcgccagctgctgaatgccaagctgattacccagaggaagttcgacaatctgaccaaggccgagagaggcggcctgagcgaactggataaggccggcttcatcaagagacagctggtggaaacccggcagatcacaaagcacgtggcacagatcctggactcccggatgaacactaagtacgacgagaacgacaaactgatccgggaagtgaaagtgatcaccctgaagtccaagctggtgtccgatttccggaaggatttccagttttacaaagtgcgcgagatcaacaactaccaccacgcccacgacgcctacctgaacgccgtcgtgggaaccgccctgatcaaaaagtaccctaagctggaaagcgagttcgtgtacggcgactacaaggtgtacgacgtgcggaagatgatcgccaagagcgagcaggaaatcggcaaggctaccgccaagtacttcttctacagcaacatcatgaactttttcaagaccgagattaccctggccaacggcgagatccggaagcggcctctgatcgagacaaacggcgaaacaggcgagatcgtgtgggataagggccgggactttgccaccgtgcggaaagtgctgtctatgccccaagtgaatatcgtgaaaaagaccgaggtgcagacaggcggcttcagcaaagagtctatcctgcccaagaggaacagcgacaagctgatcgccagaaagaaggactgggaccctaagaagtacggcggcttcgacagccccaccgtggcctattctgtgctggtggtggccaaagtggaaaagggcaagtccaagaaactgaagagtgtgaaagagctgctggggatcaccatcatggaaagaagcagcttcgagaagaatcccatcgactttctggaagccaagggctacaaagaagtgaaaaaggacctgatcatcaagctgcctaagtactccctgttcgagctggaaaacggccggaagagaatgctggcctctgccggcgaactgcagaagggaaacgaactggccctgccctccaaatatgtgaacttcctgtacctggccagccactatgagaagctgaagggctcccccgaggataatgagcagaaacagctgtttgtggaacagcacaaacactacctggacgagatcatcgagcagatcagcgagttctccaagagagtgatcctggccgacgctaatctggacaaggtgctgagcgcctacaacaagcacagagacaagcctatcagagagcaggccgagaatatcatccacctgtttaccctgaccaatctgggagcccctgccgccttcaagtactttgacaccaccatcgaccggaagaggtacaccagcaccaaagaggtgctggacgccaccctgatccaccagagcatcaccggcctgtacgagacacggatcgacctgtctcagctgggaggcgacgcctatccctatgacgtgcccgattatgccagcctgggcagcggctcccccaagaaaaaacgcaaggtggaagatcctaagaaaaagcggaaagtggacggcattggtagtgggagcaacggcagcagcggagaggaactgctgagcaagaactaccacctggaaaacgaggtggccagactgaagaaaggctctggctctggcggaagcggttctggcggatcaggatctggaagtggcggctctggaagcggaggttctggatctggcgaagaactgctgtctaagaattatcacctcgagaatgaagtcgctcgtttgaagaaaggttcaggctccggccagcggggaagcaagcgcaccgccgatggttccgagttcgaaagccccaaaaaaaagcgcaaggtctgagatcccaagcacgcagcaatgcagctcaaaacgcttagcctagccacacccccacgggaaacagcagtgattaacctttagcaataaacgaaagtttaactaagctatactaaccccagggttggtcaatttcgtgccagccacaccctggtactgcatgcacgcaatgctagctgcccctttcccgtcctgggcaccccgagtctcccccgaccccgggtcccaggtatgctcccacctccacctgccccactcaccacctctgctagttccagacacctccgagacgaggaaaaaaaaaaaaaaaaaaaaaaaaaaaaaaaaaaaaaaaaaaaaaaaaaaaaaaaaaaaaaaaaaaaaaaaaaaaaaaaaaaaaaaaaaaaaaaaaaaaaaaaaaaaaaaaaaaaaaaaa

SEQ ID NO: 255 - RNA, 9196 nt, synthetic construct
  misc_feature 1..9196: note = mRNA of V14-scFv-KRAB-2a-D3a-D3l-dCas9-10xGCN4
  source 1..9196: mol_type = other RNA
aggactcactatttgttttcgcgcccagttgcaaaaagtgtcgacatttgcttctgacacaactgtgttcactagcaacctcaaacagacaccgccaccatgggccccgacatcgtgatgacccagagccccagcagcctgagcgccagcgtgggcgaccgcgtgaccatcacctgccgcagcagcaccggcgccgtgaccaccagcaactacgccagctgggtgcaggagaagcccggcaagctgttcaagggcctgatcggcggcaccaacaaccgcgcccccggcgtgcccagccgcttcagcggcagcctgatcggcgacaaggccaccctgaccatcagcagcctgcagcccgaggacttcgccacctacttctgcgccctgtggtacagcaaccactgggtgttcggccagggcaccaaggtggagctgaagcgcggcggcggcggcagcggcggcggcggcagcggcggcggcggcagcagcggcggcggcagcgaggtgaagctgctggagagcggcggcggcctggtgcagcccggcggcagcctgaagctgagctgcgccgtgagcggcttcagcctgaccgactacggcgtgaactgggtgcgccaggcccccggccgcggcctggagtggatcggcgtgatctggggcgacggcatcaccgactacaacagcgccctgaaggaccgcttcatcatcagcaaggacaacggcaagaacaccgtgtacctgcagatgagcaaggtgcgcagcgacgacaccgccctgtactactgcgtgaccggcctgttcgactactggggccagggcaccctggtgaccgtgagcagctacccatacgatgttccagattacgctggtggaggcggaggttctgggggaggaggtagtggcggtggtggttcaggaggcggcggaagcttggatccaggtggaggtggaagcggtcggacactggtgaccttcaaggatgtatttgtggacttcaccagggaggagtggaagctgctggacactgctcagcagatcgtgtacagaaatgtgatgctggagaactataagaacctggtttccttgggttatcagcttactaagccagatgtgatcctccggttggagaagggagaagagcccggaagcggaaagcgcaccgccgatggttccgagttcgaaagccccaaaaaaaagcgcaaggtcggaagcggagctactaacttcagcctgctgaagcaggctggagacgtggaggagaaccctggacctatgaaccatgaccaggaatttgaccccccaaaggtttacccacctgtgccagctgagaagaggaagcccatccgcgtgctgtctctctttgatgggattgctacagggctcctggtgctgaaggacctgggcatccaagtggaccgctacattgcctccgaggtgtgtgaggactccatcacggtgggcatggtgcggcaccagggaaagatcatgtacgtcggggacgtccgcagcgtcacacagaagcatatccaggagtggggcccattcgacctggtgattggaggcagtccctgcaatgacctctccattgtcaaccctgcccgcaagggactttatgagggtactggccgcctcttctttgagttctaccgcctcctgcatgatgcgcggcccaaggagggagatgatcgccccttcttctggctctttgagaatgtggtggccatgggcgttagtgacaagagggacatctcgcgatttcttgagtctaaccccgtgatgattgacgccaaagaagtgtctgctgcacacagggcccgttacttctggggtaaccttcctggcatgaacaggcctttggcatccactgtgaatgataagctggagctgcaagagtgtctggagcacggcagaatagccaagttcagcaaagtgaggaccattaccaccaggtcaaactctataaagcagggcaaagaccagcatttccccgtcttcatgaacgagaaggaggacatcctgtggtgcactgaaatggaaagggtgtttggcttccccgtccactacacagacgtctccaacatgagccgcttggcgaggcagagactgctgggccgatcgtggagcgtgccggtcatccgccacctcttcgctccgctgaaggaatattttgcttgtgtgtctagcggcaatagtaacgctaacagccgcgggccgagcttcagcagcggcctggtgccgttaagcttgcgcggcagccatatgggccctatggagatatacaagacagtgtctgcatggaagagacagccagtgcgggtactgagcctcttcagaaacatcgacaaggtactaaagagtttgggcttcttggaaagcggttctggttctgggggaggaacgctgaagtacgtggaagatgtcacaaatgtcgtgaggagagacgtggagaaatggggcccctttgacctggtgtacggctcgacgcagcccctaggcagctcttgtgatcgctgtcccggctggtacatgttccagttccaccggatcctgcagtatgcgctgcctcgccaggagagtcagcggcccttcttctggatattcatggacaatctgctgctgactgaggatgaccaagagacaactacccgcttccttcagacagaggctgtgaccctccaggatgtccgtggcagagactaccagaatgctatgcgggtgtggagcaacattccagggctgaagagcaagcatgcgcccctgaccccaaaggaagaagagtatctgcaagcccaagtcagaagcaggagcaagctggacgccccgaaagttgacctcctggtgaagaactgccttctcccgctgagagagtacttcaagtatttttctcaaaactcacttcctcttggagggccgagctctggcgcacccccaccaagtggagggtctcctgccgggtccccaacatctactgaagaaggcaccagcgaatccgcaacgcccgagtcaggccctggtacctccacagaaccatctgaaggtagtgcgcctggttccccagctggaagccctacttccaccgaagaaggcacgtcaaccgaaccaagtgaaggatctgcccctgggaccagcactgaaccatctgagccaaaaaagaagagaaaggtaatggacaagaagtacagcatcggcctggccatcggcaccaactctgtgggctgggccgtgatcaccgacgagtacaaggtgcccagcaagaaattcaaggtgctgggcaacaccgaccggcacagcatcaagaagaacctgatcggcgccctgctgttcgacagcggagaaacagccgaggccacccggctgaagagaaccgccagaagaagatacaccagacggaagaaccggatctgctatctgcaagagatcttcagcaacgagatggccaaggtggacgacagcttcttccacagactggaagagtccttcctggtggaagaggataagaagcacgagcggcaccccatcttcggcaacatcgtggacgaggtggcctaccacgagaagtaccccaccatctaccacctgagaaagaaactggtggacagcaccgacaaggccgacctgcggctgatctatctggccctggcccacatgatcaagttccggggccacttcctgatcgagggcgacctgaaccccgacaacagcgacgtggacaagctgttcatccagctggtgcagacctacaaccagctgttcgaggaaaaccccatcaacgccagcggcgtggacgccaaggccatcctgtctgccagactgagcaagagcagacggctggaaaatctgatcgcccagctgcccggcgagaagaagaatggcctgttcggcaacctgattgccctgagcctgggcctgacccccaacttcaagagcaacttcgacctggccgaggatgccaaactgcagctgagcaaggacacctacgacgacgacctggacaacctgctggcccagatcggcgaccagtacgccgacctgtttctggccgccaagaacctgtccgacgccatcctgctgagcgacatcctgagagtgaacaccgagatcaccaaggcccccctgagcgcctctatgatcaagagatacgacgagcaccaccaggacctgaccctgctgaaagctctcgtgcggcagcagctgcctgagaagtacaaagagattttcttcgaccagagcaagaacggctacgccggctacatcgatggcggagccagccaggaagagttctacaagttcatcaagcccatcctggaaaagatggacggcaccgaggaactgctcgtgaagctgaacagagaggacctgctgcggaagcagcggaccttcgacaacggcagcatcccccaccagatccacctgggagagctgcacgccattctgcggcggcaggaagatttttacccattcctgaaggacaaccgggaaaagatcgagaagatcctgaccttccgcatcccctactacgtgggccctctggccaggggaaacagcagattcgcctggatgaccagaaagagcgaggaaaccatcaccccctggaacttcgaggaagtggtggacaagggcgccagcgcccagagcttcatcgagcggatgaccaacttcgataagaacctgcccaacgagaaggtgctgcccaagcacagcctgctgtacgagtacttcaccgtgtacaacgagctgaccaaagtgaaatacgtgaccgagggaatgagaaagcccgccttcctgagcggcgagcagaaaaaagccatcgtggacctgctgttcaagaccaaccggaaagtgaccgtgaagcagctgaaagaggactacttcaagaaaatcgagtgcttcgactccgtggaaatctccggcgtggaagatcggttcaacgcctccctgggcacataccacgatctgctgaaaattatcaaggacaaggacttcctggacaatgaggaaaacgaggacattctggaagatatcgtgctgaccctgacactgtttgaggacagagagatgatcgaggaacggctgaaaacctatgcccacctgttcgacgacaaagtgatgaagcagctgaagcggcggagatacaccggctggggcaggctgagccggaagctgatcaacggcatccgggacaagcagtccggcaagacaatcctggatttcctgaagtccgacggcttcgccaacagaaacttcatgcagctgatccacgacgacagcctgacctttaaagaggacatccagaaagcccaggtgtccggccagggcgatagcctgcacgagcacattgccaatctggccggcagccccgccattaagaagggcatcctgcagacagtgaaggtggtggacgagctcgtgaaagtgatgggccggcacaagcccgagaacatcgtgatcgaaatggccagagagaaccagaccacccagaagggacagaagaacagccgcgagagaatgaagcggatcgaagagggcatcaaagagctgggcagccagatcctgaaagaacaccccgtggaaaacacccagctgcagaacgagaagctgtacctgtactacctgcagaatgggcgggatatgtacgtggaccaggaactggacatcaaccggctgtccgactacgatgtggacgctatcgtgcctcagagctttctgaaggacgactccatcgataacaaagtgctgactcggagcgacaagaaccggggcaagagcgacaacgtgccctccgaagaggtcgtgaagaagatgaagaactactggcgccagctgctgaatgccaagctgattacccagaggaagttcgacaatctgaccaaggccgagagaggcggcctgagcgaactggataaggccggcttcatcaagagacagctggtggaaacccggcagatcacaaagcacgtggcacagatcctggactcccggatgaacactaagtacgacgagaacgacaaactgatccgggaagtgaaagtgatcaccctgaagtccaagctggtgtccgatttccggaaggatttccagttttacaaagtgcgcgagatcaacaactaccaccacgcccacgacgcctacctgaacgccgtcgtgggaaccgccctgatcaaaaagtaccctaagctggaaagcgagttcgtgtacggcgactacaaggtgtacgacgtgcggaagatgatcgccaagagcgagcaggaaatcggcaaggctaccgccaagtacttcttctacagcaacatcatgaactttttcaagaccgagattaccctggccaacggcgagatccggaagcggcctctgatcgagacaaacggcgaaacaggcgagatcgtgtgggataagggccgggactttgccaccgtgcggaaagtgctgtctatgccccaagtgaatatcgtgaaaaagaccgaggtgcagacaggcggcttcagcaaagagtctatcctgcccaagaggaacagcgacaagctgatcgccagaaagaaggactgggaccctaagaagtacggcggcttcgacagccccaccgtggcctattctgtgctggtggtggccaaagtggaaaagggcaagtccaagaaactgaagagtgtgaaagagctgctggggatcaccatcatggaaagaagcagcttcgagaagaatcccatcgactttctggaagccaagggctacaaagaagtgaaaaaggacctgatcatcaagctgcctaagtactccctgttcgagctggaaaacggccggaagagaatgctggcctctgccggcgaactgcagaagggaaacgaactggccctgccctccaaatatgtgaacttcctgtacctggccagccactatgagaagctgaagggctcccccgaggataatgagcagaaacagctgtttgtggaacagcacaaacactacctggacgagatcatcgagcagatcagcgagttctccaagagagtgatcctggccgacgctaatctggacaaggtgctgagcgcctacaacaagcacagagacaagcctatcagagagcaggccgagaatatcatccacctgtttaccctgaccaatctgggagcccctgccgccttcaagtactttgacaccaccatcgaccggaagaggtacaccagcaccaaagaggtgctggacgccaccctgatccaccagagcatcaccggcctgtacgagacacggatcgacctgtctcagctgggaggcgacgcctatccctatgacgtgcccgattatgccagcctgggcagcggctcccccaagaaaaaacgcaaggtggaagatcctaagaaaaagcggaaagtggacggcattggtagtgggagcaacggcagcagcggagaggaactgctgagcaagaactaccacctggaaaacgaggtggccagactgaagaaaggctctggctctggcggaagcggttctggcggatcaggatctggaagtggcggctctggaagcggaggttctggatctggcgaagaactgctgtctaagaattatcacctcgagaacgaagtggctcggctcaagaaaggcagtggcagcggaggaagtggatccggcggtagtggtagtggaagcggcggatccggctcaggcggatctggttcaggggaagaactcctctccaaaaactaccatctcgagaatgaggtcgcccgcctgaaaaaaggatcaggttccggtggttctggcagcggtggttcaggctcaggcagcggcggtagcggtagcggtggaagcggaagcggagaagaacttctcagcaaaaattaccacttggagaatgaagttgcaagactcaaaaaaggttccggcagtggcggcagcggcagcggcggatctggtagtggatctggtggcagtggttcaggcggaagtggtagcggagaggaattgctctcaaagaactatcatttggagaacgaggttgcacgcttgaagaaaggcagcggatcaggcggatctggcagcggtggatctggttctggatccggcggctccggtagtggtggaagtggctctggggaagaattgcttagcaagaattatcatcttgaaaatgaggttgccaggcttaaaaaaggcagtggctccggcggatccggaagcggaggcagcggatctggatctggtggttcaggatctggcggttctggtagcggggaagaactgttgagtaaaaactatcaccttgagaacgaggtcgcaaggttgaaaaaaggatccggctctggcggctccggaagtggcggatctggctccggtagcggaggatcaggatccggcggaagcggatcaggcgaggaactgctttccaaaaattaccaccttgaaaacgaagtcgcccgcctcaagaaaggttctggcagcggaggctctggcagtggtggtagcggaagtggaagtggtggcagtggtagcggtggatctggaagcggcgaggaactcctgtcaaagaattaccatctcgaaaacgaggtcgcaaggctcaagaaaggctcaggatcaggcggctctggatccggcggttctggttccggctcaggtggaagtggatctggcggctcaggttccggcgaagaattgctttccaagaactaccatttggaaaatgaagtcgctcgtttgaagaaaggttcaggctccggccagcggggaagcaagcgcaccgccgatggttccgagttcgaaagccccaaaaaaaagcgcaaggtctgagatcccaagcacgcagcaatgcagctcaaaacgcttagcctagccacacccccacgggaaacagcagtgattaacctttagcaataaacgaaagtttaactaagctatactaaccccagggttggtcaatttcgtgccagccacaccctggtactgcatgcacgcaatgctagctgcccctttcccgtcctgggcaccccgagtctcccccgaccccgggtcccaggtatgctcccacctccacctgccccactcaccacctctgctagttccagacacctccgagacgaggaaaaaaaaaaaaaaaaaaaaaaaaaaaaaaaaaaaaaaaaaaaaaaaaaaaaaaaaaaaaaaaaaaaaaaaaaaaaaaaaaaaaaaaaaaaaaaaaaaaaaaaaaaaaaaaaaaaaaaaa

SEQ ID NO: 256 - RNA, 8143 nt, synthetic construct
  misc_feature 1..8143: note = mRNA of V15_scFv-ZIM3-2a-D3a-hD3L-dCas9-1xGCN4
  source 1..8143: mol_type = other RNA
aggactcactatttgttttcgcgcccagttgcaaaaagtgtcgacatttgcttctgacacaactgtgttcactagcaacctcaaacagacaccgccaccatgcctgctgctaagagagtgaaactggatggatccggccccgacatcgtgatgacccagagccccagcagcctgagcgccagcgtgggcgaccgcgtgaccatcacctgccgcagcagcaccggcgccgtgaccaccagcaactacgccagctgggtgcaggagaagcccggcaagctgttcaagggcctgatcggcggcaccaacaaccgcgcccccggcgtgcccagccgcttcagcggcagcctgatcggcgacaaggccaccctgaccatcagcagcctgcagcccgaggacttcgccacctacttctgcgccctgtggtacagcaaccactgggtgttcggccagggcaccaaggtggagctgaagcgcggcggcggcggcagcggcggcggcggcagcggcggcggcggcagcagcggcggcggcagcgaggtgaagctgctggagagcggcggcggcctggtgcagcccggcggcagcctgaagctgagctgcgccgtgagcggcttcagcctgaccgactacggcgtgaactgggtgcgccaggcccccggccgcggcctggagtggatcggcgtgatctggggcgacggcatcaccgactacaacagcgccctgaaggaccgcttcatcatcagcaaggacaacggcaagaacaccgtgtacctgcagatgagcaaggtgcgcagcgacgacaccgccctgtactactgcgtgaccggcctgttcgactactggggccagggcaccctggtgaccgtgagcagctacccatacgatgttccagattacgctggtggaggcggaggttctgggggaggaggtagtggcggtggtggttcaggaggcggcggaagcttggatccaggtggaggtggaagcggtatgaacaattcccagggaagagtgaccttcgaggacgtgaccgtgaacttcacccaaggcgagtggcagagactgaaccccgagcagagaaacctgtaccgggacgtgatgctggaaaactacagcaacctggtgtccgtcggccagggcgagacaacaaagcctgacgtgatcctgcggctggaacagggcaaagagccttggctggaagaggaagaggtgctcggatctggcagagccgagaagaatggcgatatcggcggacagatctggaagccaaaggatgtgaaagagagtctcggaagcggagctactaacttcagcctgctgaagcaggctggagacgtggaggagaaccctggacctatgcctgctgctaagagagtgaaactggatggatccaaccatgaccaggaatttgaccccccaaaggtttacccacctgtgccagctgagaagaggaagcccatccgcgtgctgtctctctttgatgggattgctacagggctcctggtgctgaaggacctgggcatccaagtggaccgctacattgcctccgaggtgtgtgaggactccatcacggtgggcatggtgcggcaccagggaaagatcatgtacgtcggggacgtccgcagcgtcacacagaagcatatccaggagtggggcccattcgacctggtgattggaggcagtccctgcaatgacctctccattgtcaaccctgcccgcaagggactttatgagggtactggccgcctcttctttgagttctaccgcctcctgcatgatgcgcggcccaaggagggagatgatcgccccttcttctggctctttgagaatgtggtggccatgggcgttagtgacaagagggacatctcgcgatttcttgagtctaaccccgtgatgattgacgccaaagaagtgtctgctgcacacagggcccgttacttctggggtaaccttcctggcatgaacaggcctttggcatccactgtgaatgataagctggagctgcaagagtgtctggagcacggcagaatagccaagttcagcaaagtgaggaccattaccaccaggtcaaactctataaagcagggcaaagaccagcatttccccgtgttcatgaacgagaaggaggacatcctgtggtgcactgaaatggaaagggtgtttggcttccccgtccactacacagacgtctccaacatgagccgcttggcgaggcagagactgctgggccgatcgtggagcgtgccggtcatccgccacctcttcgctccgctgaaggaatattttgcttgtgtgtctagcggcaatagtaacgctaacagccgcgggccgagcttcagcagcggcctggtgccgttaagcttgcgcggcagccatatgttcgaaaccgtgcctgtgtggaggagacagccagtccgggtgctgtccctttttgaagacatcaagaaagagctgacgagtttgggctttttggaaagtggttctgacccgggacaactgaagcatgtggttgatgtcacagacacagtgaggaaggatgtggaggagtggggacccttcgatcttgtgtacggcgccacacctcccctgggccacacctgtgaccgtcctcccagctggtacctgttccagttccaccggctcctgcagtacgcacggcccaagccaggcagccccaggcccttcttctggatgttcgtggacaatctggtgctgaacaaggaagacctggacgtcgcatctcgcttcctggagatggagccagtcaccatcccagatgtccacggcggatccttgcagaatgctgtccgcgtgtggagcaacatcccagccataaggagcagcaggcactgggctctggtttcggaagaagaattgtccctgctggcccagaacaagcagagctcgaagctcgcggccaagtggcccaccaagctggtgaagaactgctttctccccctaagagaatatttcaagtatttttcaggagggccgagctctggcgcacccccaccaagtggagggtctcctgccgggtccccaacatctactgaagaaggcaccagcgaatccgcaacgcccgagtcaggccctggtacctccacagaaccatctgaaggtagtgcgcctggttccccagctggaagccctacttccaccgaagaaggcacgtcaaccgaaccaagtgaaggatctgcccctgggaccagcactgaaccatctgagccaaaaaagaagagaaaggtaatggacaagaagtacagcatcggcctggccatcggcaccaactctgtgggctgggccgtgatcaccgacgagtacaaggtgcccagcaagaaattcaaggtgctgggcaacaccgaccggcacagcatcaagaagaacctgatcggcgccctgctgttcgacagcggagaaacagccgaggccacccggctgaagagaaccgccagaagaagatacaccagacggaagaaccggatctgctatctgcaagagatcttcagcaacgagatggccaaggtggacgacagcttcttccacagactggaagagtccttcctggtggaagaggataagaagcacgagcggcaccccatcttcggcaacatcgtggacgaggtggcctaccacgagaagtaccccaccatctaccacctgagaaagaaactggtggacagcaccgacaaggccgacctgcggctgatctatctggccctggcccacatgatcaagttccggggccacttcctgatcgagggcgacctgaaccccgacaacagcgacgtggacaagctgttcatccagctggtgcagacctacaaccagctgttcgaggaaaaccccatcaacgccagcggcgtggacgccaaggccatcctgtctgccagactgagcaagagcagacggctggaaaatctgatcgcccagctgcccggcgagaagaagaatggcctgttcggcaacctgattgccctgagcctgggcctgacccccaacttcaagagcaacttcgacctggccgaggatgccaaactgcagctgagcaaggacacctacgacgacgacctggacaacctgctggcccagatcggcgaccagtacgccgacctgtttctggccgccaagaacctgtccgacgccatcctgctgagcgacatcctgagagtgaacaccgagatcaccaaggcccccctgagcgcctctatgatcaagagatacgacgagcaccaccaggacctgaccctgctgaaagctctcgtgcggcagcagctgcctgagaagtacaaagagattttcttcgaccagagcaagaacggctacgccggctacatcgatggcggagccagccaggaagagttctacaagttcatcaagcccatcctggaaaagatggacggcaccgaggaactgctcgtgaagctgaacagagaggacctgctgcggaagcagcggaccttcgacaacggcagcatcccccaccagatccacctgggagagctgcacgccattctgcggcggcaggaagatttttacccattcctgaaggacaaccgggaaaagatcgagaagatcctgaccttccgcatcccctactacgtgggccctctggccaggggaaacagcagattcgcctggatgaccagaaagagcgaggaaaccatcaccccctggaacttcgaggaagtggtggacaagggcgccagcgcccagagcttcatcgagcggatgaccaacttcgataagaacctgcccaacgagaaggtgctgcccaagcacagcctgctgtacgagtacttcaccgtgtacaacgagctgaccaaagtgaaatacgtgaccgagggaatgagaaagcccgccttcctgagcggcgagcagaaaaaagccatcgtggacctgctgttcaagaccaaccggaaagtgaccgtgaagcagctgaaagaggactacttcaagaaaatcgagtgcttcgactccgtggaaatctccggcgtggaagatcggttcaacgcctccctgggcacataccacgatctgctgaaaattatcaaggacaaggacttcctggacaatgaggaaaacgaggacattctggaagatatcgtgctgaccctgacactgtttgaggacagagagatgatcgaggaacggctgaaaacctatgcccacctgttcgacgacaaagtgatgaagcagctgaagcggcggagatacaccggctggggcaggctgagccggaagctgatcaacggcatccgggacaagcagtccggcaagacaatcctggatttcctgaagtccgacggcttcgccaacagaaacttcatgcagctgatccacgacgacagcctgacctttaaagaggacatccagaaagcccaggtgtccggccagggcgatagcctgcacgagcacattgccaatctggccggcagccccgccattaagaagggcatcctgcagacagtgaaggtggtggacgagctcgtgaaagtgatgggccggcacaagcccgagaacatcgtgatcgaaatggccagagagaaccagaccacccagaagggacagaagaacagccgcgagagaatgaagcggatcgaagagggcatcaaagagctgggcagccagatcctgaaagaacaccccgtggaaaacacccagctgcagaacgagaagctgtacctgtactacctgcagaatgggcgggatatgtacgtggaccaggaactggacatcaaccggctgtccgactacgatgtggacgctatcgtgcctcagagctttctgaaggacgactccatcgataacaaagtgctgactcggagcgacaagaaccggggcaagagcgacaacgtgccctccgaagaggtcgtgaagaagatgaagaactactggcgccagctgctgaatgccaagctgattacccagaggaagttcgacaatctgaccaaggccgagagaggcggcctgagcgaactggataaggccggcttcatcaagagacagctggtggaaacccggcagatcacaaagcacgtggcacagatcctggactcccggatgaacactaagtacgacgagaacgacaaactgatccgggaagtgaaagtgatcaccctgaagtccaagctggtgtccgatttccggaaggatttccagttttacaaagtgcgcgagatcaacaactaccaccacgcccacgacgcctacctgaacgccgtcgtgggaaccgccctgatcaaaaagtaccctaagctggaaagcgagttcgtgtacggcgactacaaggtgtacgacgtgcggaagatgatcgccaagagcgagcaggaaatcggcaaggctaccgccaagtacttcttctacagcaacatcatgaactttttcaagaccgagattaccctggccaacggcgagatccggaagcggcctctgatcgagacaaacggcgaaacaggcgagatcgtgtgggataagggccgggactttgccaccgtgcggaaagtgctgtctatgccccaagtgaatatcgtgaaaaagaccgaggtgcagacaggcggcttcagcaaagagtctatcctgcccaagaggaacagcgacaagctgatcgccagaaagaaggactgggaccctaagaagtacggcggcttcgacagccccaccgtggcctattctgtgctggtggtggccaaagtggaaaagggcaagtccaagaaactgaagagtgtgaaagagctgctggggatcaccatcatggaaagaagcagcttcgagaagaatcccatcgactttctggaagccaagggctacaaagaagtgaaaaaggacctgatcatcaagctgcctaagtactccctgttcgagctggaaaacggccggaagagaatgctggcctctgccggcgaactgcagaagggaaacgaactggccctgccctccaaatatgtgaacttcctgtacctggccagccactatgagaagctgaagggctcccccgaggataatgagcagaaacagctgtttgtggaacagcacaaacactacctggacgagatcatcgagcagatcagcgagttctccaagagagtgatcctggccgacgctaatctggacaaggtgctgagcgcctacaacaagcacagagacaagcctatcagagagcaggccgagaatatcatccacctgtttaccctgaccaatctgggagcccctgccgccttcaagtactttgacaccaccatcgaccggaagaggtacaccagcaccaaagaggtgctggacgccaccctgatccaccagagcatcaccggcctgtacgagacacggatcgacctgtctcagctgggaggcgacgcctatccctatgacgtgcccgattatgccagcctgggcagcggctcccccaagaaaaaacgcaaggtggaagatcctaagaaaaagcggaaagtggacggcattggtagtgggagcaacggcagcagcggagaggaactgctgagcaagaactaccacctggaaaacgaggtggccagactgaagaaaggctctggctctggcggaagcggttctggcggatcaggatctggaagtggcggctctggaagcggaggttctggatctggcgaagaactgctgtctaagaattatcacggttcaggctccggccagcggggaagcaagcgcaccgccgatggttccgagttcgaaagccccaaaaaaaagcgcaaggtctgagatcccaagcacgcagcaatgcagctcaaaacgcttagcctagccacacccccacgggaaacagcagtgattaacctttagcaataaacgaaagtttaactaagctatactaaccccagggttggtcaatttcgtgccagccacaccctggtactgcatgcacgcaatgctagctgcccctttcccgtcctgggcaccccgagtctcccccgaccccgggtcccaggtatgctcccacctccacctgccccactcaccacctctgctagttccagacacctccgagacgaggaaaaaaaaaaaaaaaaaaaaaaaaaaaaaaaaaaaaaaaaaaaaaaaaaaaaaaaaaaaaaaaaaaaaaaaaaaaaaaaaaaaaaaaaaaaaaaaaaaaaaaaaaaaaaaaaaaaaaaaa

SEQ ID NO: 257 - RNA, 8173 nt, synthetic construct
  misc_feature 1..8173: note = mRNA of V16_scFv-ZIM3-2a-D3a-hD3L-dCas9-2xGCN4
  source 1..8173: mol_type = other RNA
aggactcactatttgttttcgcgcccagttgcaaaaagtgtcgacatttgcttctgacacaactgtgttcactagcaacctcaaacagacaccgccaccatgcctgctgctaagagagtgaaactggatggatccggccccgacatcgtgatgacccagagccccagcagcctgagcgccagcgtgggcgaccgcgtgaccatcacctgccgcagcagcaccggcgccgtgaccaccagcaactacgccagctgggtgcaggagaagcccggcaagctgttcaagggcctgatcggcggcaccaacaaccgcgcccccggcgtgcccagccgcttcagcggcagcctgatcggcgacaaggccaccctgaccatcagcagcctgcagcccgaggacttcgccacctacttctgcgccctgtggtacagcaaccactgggtgttcggccagggcaccaaggtggagctgaagcgcggcggcggcggcagcggcggcggcggcagcggcggcggcggcagcagcggcggcggcagcgaggtgaagctgctggagagcggcggcggcctggtgcagcccggcggcagcctgaagctgagctgcgccgtgagcggcttcagcctgaccgactacggcgtgaactgggtgcgccaggcccccggccgcggcctggagtggatcggcgtgatctggggcgacggcatcaccgactacaacagcgccctgaaggaccgcttcatcatcagcaaggacaacggcaagaacaccgtgtacctgcagatgagcaaggtgcgcagcgacgacaccgccctgtactactgcgtgaccggcctgttcgactactggggccagggcaccctggtgaccgtgagcagctacccatacgatgttccagattacgctggtggaggcggaggttctgggggaggaggtagtggcggtggtggttcaggaggcggcggaagcttggatccaggtggaggtggaagcggtatgaacaattcccagggaagagtgaccttcgaggacgtgaccgtgaacttcacccaaggcgagtggcagagactgaaccccgagcagagaaacctgtaccgggacgtgatgctggaaaactacagcaacctggtgtccgtcggccagggcgagacaacaaagcctgacgtgatcctgcggctggaacagggcaaagagccttggctggaagaggaagaggtgctcggatctggcagagccgagaagaatggcgatatcggcggacagatctggaagccaaaggatgtgaaagagagtctcggaagcggagctactaacttcagcctgctgaagcaggctggagacgtggaggagaaccctggacctatgcctgctgctaagagagtgaaactggatggatccaaccatgaccaggaatttgaccccccaaaggtttacccacctgtgccagctgagaagaggaagcccatccgcgtgctgtctctctttgatgggattgctacagggctcctggtgctgaaggacctgggcatccaagtggaccgctacattgcctccgaggtgtgtgaggactccatcacggtgggcatggtgcggcaccagggaaagatcatgtacgtcggggacgtccgcagcgtcacacagaagcatatccaggagtggggcccattcgacctggtgattggaggcagtccctgcaatgacctctccattgtcaaccctgcccgcaagggactttatgagggtactggccgcctcttctttgagttctaccgcctcctgcatgatgcgcggcccaaggagggagatgatcgccccttcttctggctctttgagaatgtggtggccatgggcgttagtgacaagagggacatctcgcgatttcttgagtctaaccccgtgatgattgacgccaaagaagtgtctgctgcacacagggcccgttacttctggggtaaccttcctggcatgaacaggcctttggcatccactgtgaatgataagctggagctgcaagagtgtctggagcacggcagaatagccaagttcagcaaagtgaggaccattaccaccaggtcaaactctataaagcagggcaaagaccagcatttccccgtgttcatgaacgagaaggaggacatcctgtggtgcactgaaatggaaagggtgtttggcttccccgtccactacacagacgtctccaacatgagccgcttggcgaggcagagactgctgggccgatcgtggagcgtgccggtcatccgccacctcttcgctccgctgaaggaatattttgcttgtgtgtctagcggcaatagtaacgctaacagccgcgggccgagcttcagcagcggcctggtgccgttaagcttgcgcggcagccatatgttcgaaaccgtgcctgtgtggaggagacagccagtccgggtgctgtccctttttgaagacatcaagaaagagctgacgagtttgggctttttggaaagtggttctgacccgggacaactgaagcatgtggttgatgtcacagacacagtgaggaaggatgtggaggagtggggacccttcgatcttgtgtacggcgccacacctcccctgggccacacctgtgaccgtcctcccagctggtacctgttccagttccaccggctcctgcagtacgcacggcccaagccaggcagccccaggcccttcttctggatgttcgtggacaatctggtgctgaacaaggaagacctggacgtcgcatctcgcttcctggagatggagccagtcaccatcccagatgtccacggcggatccttgcagaatgctgtccgcgtgtggagcaacatcccagccataaggagcagcaggcactgggctctggtttcggaagaagaattgtccctgctggcccagaacaagcagagctcgaagctcgcggccaagtggcccaccaagctggtgaagaactgctttctccccctaagagaatatttcaagtatttttcaggagggccgagctctggcgcacccccaccaagtggagggtctcctgccgggtccccaacatctactgaagaaggcaccagcgaatccgcaacgcccgagtcaggccctggtacctccacagaaccatctgaaggtagtgcgcctggttccccagctggaagccctacttccaccgaagaaggcacgtcaaccgaaccaagtgaaggatctgcccctgggaccagcactgaaccatctgagccaaaaaagaagagaaaggtaatggacaagaagtacagcatcggcctggccatcggcaccaactctgtgggctgggccgtgatcaccgacgagtacaaggtgcccagcaagaaattcaaggtgctgggcaacaccgaccggcacagcatcaagaagaacctgatcggcgccctgctgttcgacagcggagaaacagccgaggccacccggctgaagagaaccgccagaagaagatacaccagacggaagaaccggatctgctatctgcaagagatcttcagcaacgagatggccaaggtggacgacagcttcttccacagactggaagagtccttcctggtggaagaggataagaagcacgagcggcaccccatcttcggcaacatcgtggacgaggtggcctaccacgagaagtaccccaccatctaccacctgagaaagaaactggtggacagcaccgacaaggccgacctgcggctgatctatctggccctggcccacatgatcaagttccggggccacttcctgatcgagggcgacctgaaccccgacaacagcgacgtggacaagctgttcatccagctggtgcagacctacaaccagctgttcgaggaaaaccccatcaacgccagcggcgtggacgccaaggccatcctgtctgccagactgagcaagagcagacggctggaaaatctgatcgcccagctgcccggcgagaagaagaatggcctgttcggcaacctgattgccctgagcctgggcctgacccccaacttcaagagcaacttcgacctggccgaggatgccaaactgcagctgagcaaggacacctacgacgacgacctggacaacctgctggcccagatcggcgaccagtacgccgacctgtttctggccgccaagaacctgtccgacgccatcctgctgagcgacatcctgagagtgaacaccgagatcaccaaggcccccctgagcgcctctatgatcaagagatacgacgagcaccaccaggacctgaccctgctgaaagctctcgtgcggcagcagctgcctgagaagtacaaagagattttcttcgaccagagcaagaacggctacgccggctacatcgatggcggagccagccaggaagagttctacaagttcatcaagcccatcctggaaaagatggacggcaccgaggaactgctcgtgaagctgaacagagaggacctgctgcggaagcagcggaccttcgacaacggcagcatcccccaccagatccacctgggagagctgcacgccattctgcggcggcaggaagatttttacccattcctgaaggacaaccgggaaaagatcgagaagatcctgaccttccgcatcccctactacgtgggccctctggccaggggaaacagcagattcgcctggatgaccagaaagagcgaggaaaccatcaccccctggaacttcgaggaagtggtggacaagggcgccagcgcccagagcttcatcgagcggatgaccaacttcgataagaacctgcccaacgagaaggtgctgcccaagcacagcctgctgtacgagtacttcaccgtgtacaacgagctgaccaaagtgaaatacgtgaccgagggaatgagaaagcccgccttcctgagcggcgagcagaaaaaagccatcgtggacctgctgttcaagaccaaccggaaagtgaccgtgaagcagctgaaagaggactacttcaagaaaatcgagtgcttcgactccgtggaaatctccggcgtggaagatcggttcaacgcctccctgggcacataccacgatctgctgaaaattatcaaggacaaggacttcctggacaatgaggaaaacgaggacattctggaagatatcgtgctgaccctgacactgtttgaggacagagagatgatcgaggaacggctgaaaacctatgcccacctgttcgacgacaaagtgatgaagcagctgaagcggcggagatacaccggctggggcaggctgagccggaagctgatcaacggcatccgggacaagcagtccggcaagacaatcctggatttcctgaagtccgacggcttcgccaacagaaacttcatgcagctgatccacgacgacagcctgacctttaaagaggacatccagaaagcccaggtgtccggccagggcgatagcctgcacgagcacattgccaatctggccggcagccccgccattaagaagggcatcctgcagacagtgaaggtggtggacgagctcgtgaaagtgatgggccggcacaagcccgagaacatcgtgatcgaaatggccagagagaaccagaccacccagaagggacagaagaacagccgcgagagaatgaagcggatcgaagagggcatcaaagagctgggcagccagatcctgaaagaacaccccgtggaaaacacccagctgcagaacgagaagctgtacctgtactacctgcagaatgggcgggatatgtacgtggaccaggaactggacatcaaccggctgtccgactacgatgtggacgctatcgtgcctcagagctttctgaaggacgactccatcgataacaaagtgctgactcggagcgacaagaaccggggcaagagcgacaacgtgccctccgaagaggtcgtgaagaagatgaagaactactggcgccagctgctgaatgccaagctgattacccagaggaagttcgacaatctgaccaaggccgagagaggcggcctgagcgaactggataaggccggcttcatcaagagacagctggtggaaacccggcagatcacaaagcacgtggcacagatcctggactcccggatgaacactaagtacgacgagaacgacaaactgatccgggaagtgaaagtgatcaccctgaagtccaagctggtgtccgatttccggaaggatttccagttttacaaagtgcgcgagatcaacaactaccaccacgcccacgacgcctacctgaacgccgtcgtgggaaccgccctgatcaaaaagtaccctaagctggaaagcgagttcgtgtacggcgactacaaggtgtacgacgtgcggaagatgatcgccaagagcgagcaggaaatcggcaaggctaccgccaagtacttcttctacagcaacatcatgaactttttcaagaccgagattaccctggccaacggcgagatccggaagcggcctctgatcgagacaaacggcgaaacaggcgagatcgtgtgggataagggccgggactttgccaccgtgcggaaagtgctgtctatgccccaagtgaatatcgtgaaaaagaccgaggtgcagacaggcggcttcagcaaagagtctatcctgcccaagaggaacagcgacaagctgatcgccagaaagaaggactgggaccctaagaagtacggcggcttcgacagccccaccgtggcctattctgtgctggtggtggccaaagtggaaaagggcaagtccaagaaactgaagagtgtgaaagagctgctggggatcaccatcatggaaagaagcagcttcgagaagaatcccatcgactttctggaagccaagggctacaaagaagtgaaaaaggacctgatcatcaagctgcctaagtactccctgttcgagctggaaaacggccggaagagaatgctggcctctgccggcgaactgcagaagggaaacgaactggccctgccctccaaatatgtgaacttcctgtacctggccagccactatgagaagctgaagggctcccccgaggataatgagcagaaacagctgtttgtggaacagcacaaacactacctggacgagatcatcgagcagatcagcgagttctccaagagagtgatcctggccgacgctaatctggacaaggtgctgagcgcctacaacaagcacagagacaagcctatcagagagcaggccgagaatatcatccacctgtttaccctgaccaatctgggagcccctgccgccttcaagtactttgacaccaccatcgaccggaagaggtacaccagcaccaaagaggtgctggacgccaccctgatccaccagagcatcaccggcctgtacgagacacggatcgacctgtctcagctgggaggcgacgcctatccctatgacgtgcccgattatgccagcctgggcagcggctcccccaagaaaaaacgcaaggtggaagatcctaagaaaaagcggaaagtggacggcattggtagtgggagcaacggcagcagcggagaggaactgctgagcaagaactaccacctggaaaacgaggtggccagactgaagaaaggctctggctctggcggaagcggttctggcggatcaggatctggaagtggcggctctggaagcggaggttctggatctggcgaagaactgctgtctaagaattatcacctcgagaatgaagtcgctcgtttgaagaaaggttcaggctccggccagcggggaagcaagcgcaccgccgatggttccgagttcgaaagccccaaaaaaaagcgcaaggtctgagatcccaagcacgcagcaatgcagctcaaaacgcttagcctagccacacccccacgggaaacagcagtgattaacctttagcaataaacgaaagtttaactaagctatactaaccccagggttggtcaatttcgtgccagccacaccctggtactgcatgcacgcaatgctagctgcccctttcccgtcctgggcaccccgagtctcccccgaccccgggtcccaggtatgctcccacctccacctgccccactcaccacctctgctagttccagacacctccgagacgaggaaaaaaaaaaaaaaaaaaaaaaaaaaaaaaaaaaaaaaaaaaaaaaaaaaaaaaaaaaaaaaaaaaaaaaaaaaaaaaaaaaaaaaaaaaaaaaaaaaaaaaaaaaaaaaaaaaaaaaaa

SEQ ID NO: 258 - RNA, 9277 nt, synthetic construct
  misc_feature 1..9277: note = mRNA of V17_scFv-ZIM3-2a-D3a-hD3L-dCas9-10xGCN4
  source 1..9277: mol_type = other RNA
aggactcactatttgttttcgcgcccagttgcaaaaagtgtcgacatttgcttctgacacaactgtgttcactagcaacctcaaacagacaccgccaccatgcctgctgctaagagagtgaaactggatggatccggccccgacatcgtgatgacccagagccccagcagcctgagcgccagcgtgggcgaccgcgtgaccatcacctgccgcagcagcaccggcgccgtgaccaccagcaactacgccagctgggtgcaggagaagcccggcaagctgttcaagggcctgatcggcggcaccaacaaccgcgcccccggcgtgcccagccgcttcagcggcagcctgatcggcgacaaggccaccctgaccatcagcagcctgcagcccgaggacttcgccacctacttctgcgccctgtggtacagcaaccactgggtgttcggccagggcaccaaggtggagctgaagcgcggcggcggcggcagcggcggcggcggcagcggcggcggcggcagcagcggcggcggcagcgaggtgaagctgctggagagcggcggcggcctggtgcagcccggcggcagcctgaagctgagctgcgccgtgagcggcttcagcctgaccgactacggcgtgaactgggtgcgccaggcccccggccgcggcctggagtggatcggcgtgatctggggcgacggcatcaccgactacaacagcgccctgaaggaccgcttcatcatcagcaaggacaacggcaagaacaccgtgtacctgcagatgagcaaggtgcgcagcgacgacaccgccctgtactactgcgtgaccggcctgttcgactactggggccagggcaccctggtgaccgtgagcagctacccatacgatgttccagattacgctggtggaggcggaggttctgggggaggaggtagtggcggtggtggttcaggaggcggcggaagcttggatccaggtggaggtggaagcggtatgaacaattcccagggaagagtgaccttcgaggacgtgaccgtgaacttcacccaaggcgagtggcagagactgaaccccgagcagagaaacctgtaccgggacgtgatgctggaaaactacagcaacctggtgtccgtcggccagggcgagacaacaaagcctgacgtgatcctgcggctggaacagggcaaagagccttggctggaagaggaagaggtgctcggatctggcagagccgagaagaatggcgatatcggcggacagatctggaagccaaaggatgtgaaagagagtctcggaagcggagctactaacttcagcctgctgaagcaggctggagacgtggaggagaaccctggacctatgcctgctgctaagagagtgaaactggatggatccaaccatgaccaggaatttgaccccccaaaggtttacccacctgtgccagctgagaagaggaagcccatccgcgtgctgtctctctttgatgggattgctacagggctcctggtgctgaaggacctgggcatccaagtggaccgctacattgcctccgaggtgtgtgaggactccatcacggtgggcatggtgcggcaccagggaaagatcatgtacgtcggggacgtccgcagcgtcacacagaagcatatccaggagtggggcccattcgacctggtgattggaggcagtccctgcaatgacctctccattgtcaaccctgcccgcaagggactttatgagggtactggccgcctcttctttgagttctaccgcctcctgcatgatgcgcggcccaaggagggagatgatcgccccttcttctggctctttgagaatgtggtggccatgggcgttagtgacaagagggacatctcgcgatttcttgagtctaaccccgtgatgattgacgccaaagaagtgtctgctgcacacagggcccgttacttctggggtaaccttcctggcatgaacaggcctttggcatccactgtgaatgataagctggagctgcaagagtgtctggagcacggcagaatagccaagttcagcaaagtgaggaccattaccaccaggtcaaactctataaagcagggcaaagaccagcatttccccgtgttcatgaacgagaaggaggacatcctgtggtgcactgaaatggaaagggtgtttggcttccccgtccactacacagacgtctccaacatgagccgcttggcgaggcagagactgctgggccgatcgtggagcgtgccggtcatccgccacctcttcgctccgctgaaggaatattttgcttgtgtgtctagcggcaatagtaacgctaacagccgcgggccgagcttcagcagcggcctggtgccgttaagcttgcgcggcagccatatgttcgaaaccgtgcctgtgtggaggagacagccagtccgggtgctgtccctttttgaagacatcaagaaagagctgacgagtttgggctttttggaaagtggttctgacccgggacaactgaagcatgtggttgatgtcacagacacagtgaggaaggatgtggaggagtggggacccttcgatcttgtgtacggcgccacacctcccctgggccacacctgtgaccgtcctcccagctggtacctgttccagttccaccggctcctgcagtacgcacggcccaagccaggcagccccaggcccttcttctggatgttcgtggacaatctggtgctgaacaaggaagacctggacgtcgcatctcgcttcctggagatggagccagtcaccatcccagatgtccacggcggatccttgcagaatgctgtccgcgtgtggagcaacatcccagccataaggagcagcaggcactgggctctggtttcggaagaagaattgtccctgctggcccagaacaagcagagctcgaagctcgcggccaagtggcccaccaagctggtgaagaactgctttctccccctaagagaatatttcaagtatttttcaggagggccgagctctggcgcacccccaccaagtggagggtctcctgccgggtccccaacatctactgaagaaggcaccagcgaatccgcaacgcccgagtcaggccctggtacctccacagaaccatctgaaggtagtgcgcctggttccccagctggaagccctacttccaccgaagaaggcacgtcaaccgaaccaagtgaaggatctgcccctgggaccagcactgaaccatctgagccaaaaaagaagagaaaggtaatggacaagaagtacagcatcggcctggccatcggcaccaactctgtgggctgggccgtgatcaccgacgagtacaaggtgcccagcaagaaattcaaggtgctgggcaacaccgaccggcacagcatcaagaagaacctgatcggcgccctgctgttcgacagcggagaaacagccgaggccacccggctgaagagaaccgccagaagaagatacaccagacggaagaaccggatctgctatctgcaagagatcttcagcaacgagatggccaaggtggacgacagcttcttccacagactggaagagtccttcctggtggaagaggataagaagcacgagcggcaccccatcttcggcaacatcgtggacgaggtggcctaccacgagaagtaccccaccatctaccacctgagaaagaaactggtggacagcaccgacaaggccgacctgcggctgatctatctggccctggcccacatgatcaagttccggggccacttcctgatcgagggcgacctgaaccccgacaacagcgacgtggacaagctgttcatccagctggtgcagacctacaaccagctgttcgaggaaaaccccatcaacgccagcggcgtggacgccaaggccatcctgtctgccagactgagcaagagcagacggctggaaaatctgatcgcccagctgcccggcgagaagaagaatggcctgttcggcaacctgattgccctgagcctgggcctgacccccaacttcaagagcaacttcgacctggccgaggatgccaaactgcagctgagcaaggacacctacgacgacgacctggacaacctgctggcccagatcggcgaccagtacgccgacctgtttctggccgccaagaacctgtccgacgccatcctgctgagcgacatcctgagagtgaacaccgagatcaccaaggcccccctgagcgcctctatgatcaagagatacgacgagcaccaccaggacctgaccctgctgaaagctctcgtgcggcagcagctgcctgagaagtacaaagagattttcttcgaccagagcaagaacggctacgccggctacatcgatggcggagccagccaggaagagttctacaagttcatcaagcccatcctggaaaagatggacggcaccgaggaactgctcgtgaagctgaacagagaggacctgctgcggaagcagcggaccttcgacaacggcagcatcccccaccagatccacctgggagagctgcacgccattctgcggcggcaggaagatttttacccattcctgaaggacaaccgggaaaagatcgagaagatcctgaccttccgcatcccctactacgtgggccctctggccaggggaaacagcagattcgcctggatgaccagaaagagcgaggaaaccatcaccccctggaacttcgaggaagtggtggacaagggcgccagcgcccagagcttcatcgagcggatgaccaacttcgataagaacctgcccaacgagaaggtgctgcccaagcacagcctgctgtacgagtacttcaccgtgtacaacgagctgaccaaagtgaaatacgtgaccgagggaatgagaaagcccgccttcctgagcggcgagcagaaaaaagccatcgtggacctgctgttcaagaccaaccggaaagtgaccgtgaagcagctgaaagaggactacttcaagaaaatcgagtgcttcgactccgtggaaatctccggcgtggaagatcggttcaacgcctccctgggcacataccacgatctgctgaaaattatcaaggacaaggacttcctggacaatgaggaaaacgaggacattctggaagatatcgtgctgaccctgacactgtttgaggacagagagatgatcgaggaacggctgaaaacctatgcccacctgttcgacgacaaagtgatgaagcagctgaagcggcggagatacaccggctggggcaggctgagccggaagctgatcaacggcatccgggacaagcagtccggcaagacaatcctggatttcctgaagtccgacggcttcgccaacagaaacttcatgcagctgatccacgacgacagcctgacctttaaagaggacatccagaaagcccaggtgtccggccagggcgatagcctgcacgagcacattgccaatctggccggcagccccgccattaagaagggcatcctgcagacagtgaaggtggtggacgagctcgtgaaagtgatgggccggcacaagcccgagaacatcgtgatcgaaatggccagagagaaccagaccacccagaagggacagaagaacagccgcgagagaatgaagcggatcgaagagggcatcaaagagctgggcagccagatcctgaaagaacaccccgtggaaaacacccagctgcagaacgagaagctgtacctgtactacctgcagaatgggcgggatatgtacgtggaccaggaactggacatcaaccggctgtccgactacgatgtggacgctatcgtgcctcagagctttctgaaggacgactccatcgataacaaagtgctgactcggagcgacaagaaccggggcaagagcgacaacgtgccctccgaagaggtcgtgaagaagatgaagaactactggcgccagctgctgaatgccaagctgattacccagaggaagttcgacaatctgaccaaggccgagagaggcggcctgagcgaactggataaggccggcttcatcaagagacagctggtggaaacccggcagatcacaaagcacgtggcacagatcctggactcccggatgaacactaagtacgacgagaacgacaaactgatccgggaagtgaaagtgatcaccctgaagtccaagctggtgtccgatttccggaaggatttccagttttacaaagtgcgcgagatcaacaactaccaccacgcccacgacgcctacctgaacgccgtcgtgggaaccgccctgatcaaaaagtaccctaagctggaaagcgagttcgtgtacggcgactacaaggtgtacgacgtgcggaagatgatcgccaagagcgagcaggaaatcggcaaggctaccgccaagtacttcttctacagcaacatcatgaactttttcaagaccgagattaccctggccaacggcgagatccggaagcggcctctgatcgagacaaacggcgaaacaggcgagatcgtgtgggataagggccgggactttgccaccgtgcggaaagtgctgtctatgccccaagtgaatatcgtgaaaaagaccgaggtgcagacaggcggcttcagcaaagagtctatcctgcccaagaggaacagcgacaagctgatcgccagaaagaaggactgggaccctaagaagtacggcggcttcgacagccccaccgtggcctattctgtgctggtggtggccaaagtggaaaagggcaagtccaagaaactgaagagtgtgaaagagctgctggggatcaccatcatggaaagaagcagcttcgagaagaatcccatcgactttctggaagccaagggctacaaagaagtgaaaaaggacctgatcatcaagctgcctaagtactccctgttcgagctggaaaacggccggaagagaatgctggcctctgccggcgaactgcagaagggaaacgaactggccctgccctccaaatatgtgaacttcctgtacctggccagccactatgagaagctgaagggctcccccgaggataatgagcagaaacagctgtttgtggaacagcacaaacactacctggacgagatcatcgagcagatcagcgagttctccaagagagtgatcctggccgacgctaatctggacaaggtgctgagcgcctacaacaagcacagagacaagcctatcagagagcaggccgagaatatcatccacctgtttaccctgaccaatctgggagcccctgccgccttcaagtactttgacaccaccatcgaccggaagaggtacaccagcaccaaagaggtgctggacgccaccctgatccaccagagcatcaccggcctgtacgagacacggatcgacctgtctcagctgggaggcgacgcctatccctatgacgtgcccgattatgccagcctgggcagcggctcccccaagaaaaaacgcaaggtggaagatcctaagaaaaagcggaaagtggacggcattggtagtgggagcaacggcagcagcggagaggaactgctgagcaagaactaccacctggaaaacgaggtggccagactgaagaaaggctctggctctggcggaagcggttctggcggatcaggatctggaagtggcggctctggaagcggaggttctggatctggcgaagaactgctgtctaagaattatcacctcgagaacgaagtggctcggctcaagaaaggcagtggcagcggaggaagtggatccggcggtagtggtagtggaagcggcggatccggctcaggcggatctggttcaggggaagaactcctctccaaaaactaccatctcgagaatgaggtcgcccgcctgaaaaaaggatcaggttccggtggttctggcagcggtggttcaggctcaggcagcggcggtagcggtagcggtggaagcggaagcggagaagaacttctcagcaaaaattaccacttggagaatgaagttgcaagactcaaaaaaggttccggcagtggcggcagcggcagcggcggatctggtagtggatctggtggcagtggttcaggcggaagtggtagcggagaggaattgctctcaaagaactatcatttggagaacgaggttgcacgcttgaagaaaggcagcggatcaggcggatctggcagcggtggatctggttctggatccggcggctccggtagtggtggaagtggctctggggaagaattgcttagcaagaattatcatcttgaaaatgaggttgccaggcttaaaaaaggcagtggctccggcggatccggaagcggaggcagcggatctggatctggtggttcaggatctggcggttctggtagcggggaagaactgttgagtaaaaactatcaccttgagaacgaggtcgcaaggttgaaaaaaggatccggctctggcggctccggaagtggcggatctggctccggtagcggaggatcaggatccggcggaagcggatcaggcgaggaactgctttccaaaaattaccaccttgaaaacgaagtcgcccgcctcaagaaaggttctggcagcggaggctctggcagtggtggtagcggaagtggaagtggtggcagtggtagcggtggatctggaagcggcgaggaactcctgtcaaagaattaccatctcgaaaacgaggtcgcaaggctcaagaaaggctcaggatcaggcggctctggatccggcggttctggttccggctcaggtggaagtggatctggcggctcaggttccggcgaagaattgctttccaagaactaccatttggaaaatgaagtcgctcgtttgaagaaaggttcaggctccggccagcggggaagcaagcgcaccgccgatggttccgagttcgaaagccccaaaaaaaagcgcaaggtctgagatcccaagcacgcagcaatgcagctcaaaacgcttagcctagccacacccccacgggaaacagcagtgattaacctttagcaataaacgaaagtttaactaagctatactaaccccagggttggtcaatttcgtgccagccacaccctggtactgcatgcacgcaatgctagctgcccctttcccgtcctgggcaccccgagtctcccccgaccccgggtcccaggtatgctcccacctccacctgccccactcaccacctctgctagttccagacacctccgagacgaggaaaaaaaaaaaaaaaaaaaaaaaaaaaaaaaaaaaaaaaaaaaaaaaaaaaaaaaaaaaaaaaaaaaaaaaaaaaaaaaaaaaaaaaaaaaaaaaaaaaaaaaaaaaaaaaaaaaaaaaa

SEQ ID NO: 259 - RNA, 7723 nt, synthetic construct
  misc_feature 1..7723: note = mRNA of V18_scFv-ZIM3-2a-D3a-hD3L-dCas12a-1xGCN4
  source 1..7723: mol_type = other RNA
aggactcactatttgttttcgcgcccagttgcaaaaagtgtcgacatttgcttctgacacaactgtgttcactagcaacctcaaacagacaccgccaccatgcctgctgctaagagagtgaaactggatggatccggccccgacatcgtgatgacccagagccccagcagcctgagcgccagcgtgggcgaccgcgtgaccatcacctgccgcagcagcaccggcgccgtgaccaccagcaactacgccagctgggtgcaggagaagcccggcaagctgttcaagggcctgatcggcggcaccaacaaccgcgcccccggcgtgcccagccgcttcagcggcagcctgatcggcgacaaggccaccctgaccatcagcagcctgcagcccgaggacttcgccacctacttctgcgccctgtggtacagcaaccactgggtgttcggccagggcaccaaggtggagctgaagcgcggcggcggcggcagcggcggcggcggcagcggcggcggcggcagcagcggcggcggcagcgaggtgaagctgctggagagcggcggcggcctggtgcagcccggcggcagcctgaagctgagctgcgccgtgagcggcttcagcctgaccgactacggcgtgaactgggtgcgccaggcccccggccgcggcctggagtggatcggcgtgatctggggcgacggcatcaccgactacaacagcgccctgaaggaccgcttcatcatcagcaaggacaacggcaagaacaccgtgtacctgcagatgagcaaggtgcgcagcgacgacaccgccctgtactactgcgtgaccggcctgttcgactactggggccagggcaccctggtgaccgtgagcagctacccatacgatgttccagattacgctggtggaggcggaggttctgggggaggaggtagtggcggtggtggttcaggaggcggcggaagcttggatccaggtggaggtggaagcggtatgaacaattcccagggaagagtgaccttcgaggacgtgaccgtgaacttcacccaaggcgagtggcagagactgaaccccgagcagagaaacctgtaccgggacgtgatgctggaaaactacagcaacctggtgtccgtcggccagggcgagacaacaaagcctgacgtgatcctgcggctggaacagggcaaagagccttggctggaagaggaagaggtgctcggatctggcagagccgagaagaatggcgatatcggcggacagatctggaagccaaaggatgtgaaagagagtctcggaagcggagctactaacttcagcctgctgaagcaggctggagacgtggaggagaaccctggacctatgcctgctgctaagagagtgaaactggatggatccaaccatgaccaggaatttgaccccccaaaggtttacccacctgtgccagctgagaagaggaagcccatccgcgtgctgtctctctttgatgggattgctacagggctcctggtgctgaaggacctgggcatccaagtggaccgctacattgcctccgaggtgtgtgaggactccatcacggtgggcatggtgcggcaccagggaaagatcatgtacgtcggggacgtccgcagcgtcacacagaagcatatccaggagtggggcccattcgacctggtgattggaggcagtccctgcaatgacctctccattgtcaaccctgcccgcaagggactttatgagggtactggccgcctcttctttgagttctaccgcctcctgcatgatgcgcggcccaaggagggagatgatcgccccttcttctggctctttgagaatgtggtggccatgggcgttagtgacaagagggacatctcgcgatttcttgagtctaaccccgtgatgattgacgccaaagaagtgtctgctgcacacagggcccgttacttctggggtaaccttcctggcatgaacaggcctttggcatccactgtgaatgataagctggagctgcaagagtgtctggagcacggcagaatagccaagttcagcaaagtgaggaccattaccaccaggtcaaactctataaagcagggcaaagaccagcatttccccgtgttcatgaacgagaaggaggacatcctgtggtgcactgaaatggaaagggtgtttggcttccccgtccactacacagacgtctccaacatgagccgcttggcgaggcagagactgctgggccgatcgtggagcgtgccggtcatccgccacctcttcgctccgctgaaggaatattttgcttgtgtgtctagcggcaatagtaacgctaacagccgcgggccgagcttcagcagcggcctggtgccgttaagcttgcgcggcagccatatgttcgaaaccgtgcctgtgtggaggagacagccagtccgggtgctgtccctttttgaagacatcaagaaagagctgacgagtttgggctttttggaaagtggttctgacccgggacaactgaagcatgtggttgatgtcacagacacagtgaggaaggatgtggaggagtggggacccttcgatcttgtgtacggcgccacacctcccctgggccacacctgtgaccgtcctcccagctggtacctgttccagttccaccggctcctgcagtacgcacggcccaagccaggcagccccaggcccttcttctggatgttcgtggacaatctggtgctgaacaaggaagacctggacgtcgcatctcgcttcctggagatggagccagtcaccatcccagatgtccacggcggatccttgcagaatgctgtccgcgtgtggagcaacatcccagccataaggagcagcaggcactgggctctggtttcggaagaagaattgtccctgctggcccagaacaagcagagctcgaagctcgcggccaagtggcccaccaagctggtgaagaactgctttctccccctaagagaatatttcaagtatttttcaggagggccgagctctggcgcacccccaccaagtggagggtctcctgccgggtccccaacatctactgaagaaggcaccagcgaatccgcaacgcccgagtcaggccctggtacctccacagaaccatctgaaggtagtgcgcctggttccccagctggaagccctacttccaccgaagaaggcacgtcaaccgaaccaagtgaaggatctgcccctgggaccagcactgaaccatctgagccaaaaaagaagagaaaggtaatgtcaaagctggagaaattcaccaactgttatagcctgtctaagaccctgcgcttcaaggcaatcccagtgggcaagacacaagagaacattgacaacaaacggctcctggtggaggatgagaagagggctgaagattacaagggcgttaagaagctgctggataggtactatctgtcattcatcaacgatgtcctccacagtatcaagctgaagaatctgaacaattacatttctctgttccggaagaagacacggaccgagaaggagaacaaagagctggagaatctggagatcaacctgaggaaagaaatagctaaggctttcaaagggaacgagggttacaagtccctgttcaagaaagacattatcgagactattctgcctgagttcctggacgataaagatgagatcgccctcgtcaattccttcaatgggtttaccacagcctttaccggcttcttcgacaatagagagaatatgttctctgaagaggccaaatccactagcatcgcctttcgctgcataaacgagaacctgactaggtacatcagcaatatggacatctttgagaaagtcgatgccatattcgacaaacatgaggtgcaggagattaaggagaagatcctgaactcagattacgatgtcgaagatttcttcgagggagagttcttcaacttcgtgctcacacaagagggcattgatgtgtacaatgcaatcattggagggttcgtgacagagagtggcgagaagataaagggcctgaacgagtatatcaacctctacaaccagaaaaccaagcagaaactgcctaagttcaagccactgtacaaacaagtgctctcagatagggaaagcctgagcttctacggtgaagggtatacatcagatgaagaagtgctcgaagtgttccgcaacaccctcaataagaacagtgaaatcttctcttcaatcaagaagctggagaaactgttcaagaatttcgatgagtactcctctgccggaatctttgtgaagaatggccctgcaatatccactattagcaaagacatctttggcgagtggaacgttatcagggataagtggaatgccgagtacgatgatattcatctcaagaagaaagccgtggttacagagaaatacgaggatgatagacgcaagagctttaagaagattggtagcttctctctcgaacagctgcaggagtacgccgacgctgacctgtcagtcgtggagaaactcaaggagatcataatccagaaggtggatgaaatctacaaagtgtatggaagctctgagaaactcttcgatgcagactttgttctggagaagagtctgaagaagaacgacgcagtggttgctatcatgaaggacctgctggattctgttaagtctttcgagaattacattaaggcattctttggtgaagggaaggagacaaatagggacgagagcttctatggcgactttgttctggcctacgacatcctcctcaaggttgaccacatctatgacgctatacggaattacgttacccagaagccctatagcaaagacaagttcaagctgtatttccagaatccacagtttatgggtgggtgggataaagacaaagaaacagattacagggccactatcctgcggtacggcagcaaatactatctggctatcatggataagaagtacgccaaatgcctccagaagatcgacaaggacgacgtgaacggtaactacgagaagatcaattacaagctcctgccaggacctaacaagatgctgcccaaggtgttcttctccaagaaatggatggcctactataacccaagcgaggacattcagaagatatacaagaatgggacattcaagaagggcgatatgttcaacctcaacgactgccacaagctgattgatttcttcaaggatagcatttctcgctatcccaagtggtctaatgcatacgatttcaacttcagcgagactgagaagtacaaagacatcgctggcttctaccgggaggtggaagagcaaggctataaggtgtcattcgaatccgcttctaagaaggaagtggataagctcgtggaagagggtaagctgtacatgttccagatatacaacaaagacttcagcgataagagccacggcactccaaacctccatactatgtatttcaagctgctgtttgacgagaacaaccacggacagattaggctgtcaggaggcgcagaactcttcatgcgcagagcttcactgaagaaggaggaactcgttgtccacccagccaatagccctatagccaataagaatccagacaatcctaagaaaaccactactctgtcttacgatgtgtataaggataagagattctctgaagatcagtacgaactgcacatacccattgccattaacaagtgccctaagaacatcttcaagattaacacagaggttagagtgctcctgaaacacgacgataacccttatgttataggcattgctcgcggagagagaaacctgctgtacatcgtcgtggtggacggcaaaggcaacatcgtggaacagtacagtctcaatgaaatcattaacaatttcaacggaatccgcattaagaccgactaccattctctcctcgacaagaaggagaaagaaaggttcgaagcaagacagaattggacaagtatagagaatatcaaagaactgaaggctgggtacatctctcaggttgtgcacaagatatgtgagctggtggagaagtacgacgctgttatcgccctcgcggacctgaatagcggcttcaagaactccagggtgaaggtggagaagcaggtgtatcagaagttcgagaagatgctgatcgacaagctcaactatatggtggacaagaaatccaatccttgcgctactggtggagccctgaagggctatcaaatcaccaataagttcgaatctttcaagtctatgagcacccagaatggcttcatcttctacatacccgcatggctgacatccaagattgatccctctaccggatttgttaatctgctcaagactaagtacacctctattgctgactcaaagaagttcatatcatcatttgaccgcatcatgtacgtgccagaagaggacctgttcgagtttgccctggattacaagaatttctctcggactgacgccgactacatcaagaagtggaagctctactcttatggtaatcggattcgcatattccgcaatcccaagaagaataacgtgttcgattgggaggaagtttgcctcaccagcgcttacaaggagctgttcaataagtatgggattaactaccagcagggcgacataagagccctgctgtgcgaacaatctgataaggcattctattcctctttcatggcactgatgtcactgatgctgcaaatgcgcaattccatcaccggaagaacagacgtggcctttctgatctctcctgtcaagaactcagatggcatcttctacgattcccgcaactatgaagcacaggagaatgctatcctgcctaagaatgccgatgcaaatggagcctataacatcgccagaaaggtcctctgggccataggacaattcaagaaagctgaagatgagaagctggacaaggtgaagatcgccatttcaaacaaagagtggctcgaatatgctcagacctcagtgaagcatgcctatccctatgacgtgcccgattatgccagcctgggcagcggctcccccaagaaaaaacgcaaggtggaagatcctaagaaaaagcggaaagtggacggcattggtagtgggagcaacggcagcagcggagaggaactgctgagcaagaactaccacctggaaaacgaggtggccagactgaagaaaggctctggctctggcggaagcggttctggcggatcaggatctggaagtggcggctctggaagcggaggttctggatctggcgaagaactgctgtctaagaattatcacggttcaggctccggccagcggggaagcaagcgcaccgccgatggttccgagttcgaaagccccaaaaaaaagcgcaaggtctgagatcccaagcacgcagcaatgcagctcaaaacgcttagcctagccacacccccacgggaaacagcagtgattaacctttagcaataaacgaaagtttaactaagctatactaaccccagggttggtcaatttcgtgccagccacaccctggtactgcatgcacgcaatgctagctgcccctttcccgtcctgggcaccccgagtctcccccgaccccgggtcccaggtatgctcccacctccacctgccccactcaccacctctgctagttccagacacctccgagacgaggaaaaaaaaaaaaaaaaaaaaaaaaaaaaaaaaaaaaaaaaaaaaaaaaaaaaaaaaaaaaaaaaaaaaaaaaaaaaaaaaaaaaaaaaaaaaaaaaaaaaaaaaaaaaaaaaaaaaaaaa

SEQ ID NO: 260 - RNA, 7072 nt, synthetic construct
  misc_feature 1..7072: note = mRNA of V19_scFv-ZIM3-2a-D3a-hD3L-dCas12i-1xGCN4
  source 1..7072: mol_type = other RNA
aggactcactatttgttttcgcgcccagttgcaaaaagtgtcgacatttgcttctgacacaactgtgttcactagcaacctcaaacagacaccgccaccatgcctgctgctaagagagtgaaactggatggatccggccccgacatcgtgatgacccagagccccagcagcctgagcgccagcgtgggcgaccgcgtgaccatcacctgccgcagcagcaccggcgccgtgaccaccagcaactacgccagctgggtgcaggagaagcccggcaagctgttcaagggcctgatcggcggcaccaacaaccgcgcccccggcgtgcccagccgcttcagcggcagcctgatcggcgacaaggccaccctgaccatcagcagcctgcagcccgaggacttcgccacctacttctgcgccctgtggtacagcaaccactgggtgttcggccagggcaccaaggtggagctgaagcgcggcggcggcggcagcggcggcggcggcagcggcggcggcggcagcagcggcggcggcagcgaggtgaagctgctggagagcggcggcggcctggtgcagcccggcggcagcctgaagctgagctgcgccgtgagcggcttcagcctgaccgactacggcgtgaactgggtgcgccaggcccccggccgcggcctggagtggatcggcgtgatctggggcgacggcatcaccgactacaacagcgccctgaaggaccgcttcatcatcagcaaggacaacggcaagaacaccgtgtacctgcagatgagcaaggtgcgcagcgacgacaccgccctgtactactgcgtgaccggcctgttcgactactggggccagggcaccctggtgaccgtgagcagctacccatacgatgttccagattacgctggtggaggcggaggttctgggggaggaggtagtggcggtggtggttcaggaggcggcggaagcttggatccaggtggaggtggaagcggtatgaacaattcccagggaagagtgaccttcgaggacgtgaccgtgaacttcacccaaggcgagtggcagagactgaaccccgagcagagaaacctgtaccgggacgtgatgctggaaaactacagcaacctggtgtccgtcggccagggcgagacaacaaagcctgacgtgatcctgcggctggaacagggcaaagagccttggctggaagaggaagaggtgctcggatctggcagagccgagaagaatggcgatatcggcggacagatctggaagccaaaggatgtgaaagagagtctcggaagcggagctactaacttcagcctgctgaagcaggctggagacgtggaggagaaccctggacctatgcctgctgctaagagagtgaaactggatggatccaaccatgaccaggaatttgaccccccaaaggtttacccacctgtgccagctgagaagaggaagcccatccgcgtgctgtctctctttgatgggattgctacagggctcctggtgctgaaggacctgggcatccaagtggaccgctacattgcctccgaggtgtgtgaggactccatcacggtgggcatggtgcggcaccagggaaagatcatgtacgtcggggacgtccgcagcgtcacacagaagcatatccaggagtggggcccattcgacctggtgattggaggcagtccctgcaatgacctctccattgtcaaccctgcccgcaagggactttatgagggtactggccgcctcttctttgagttctaccgcctcctgcatgatgcgcggcccaaggagggagatgatcgccccttcttctggctctttgagaatgtggtggccatgggcgttagtgacaagagggacatctcgcgatttcttgagtctaaccccgtgatgattgacgccaaagaagtgtctgctgcacacagggcccgttacttctggggtaaccttcctggcatgaacaggcctttggcatccactgtgaatgataagctggagctgcaagagtgtctggagcacggcagaatagccaagttcagcaaagtgaggaccattaccaccaggtcaaactctataaagcagggcaaagaccagcatttccccgtgttcatgaacgagaaggaggacatcctgtggtgcactgaaatggaaagggtgtttggcttccccgtccactacacagacgtctccaacatgagccgcttggcgaggcagagactgctgggccgatcgtggagcgtgccggtcatccgccacctcttcgctccgctgaaggaatattttgcttgtgtgtctagcggcaatagtaacgctaacagccgcgggccgagcttcagcagcggcctggtgccgttaagcttgcgcggcagccatatgttcgaaaccgtgcctgtgtggaggagacagccagtccgggtgctgtccctttttgaagacatcaagaaagagctgacgagtttgggctttttggaaagtggttctgacccgggacaactgaagcatgtggttgatgtcacagacacagtgaggaaggatgtggaggagtggggacccttcgatcttgtgtacggcgccacacctcccctgggccacacctgtgaccgtcctcccagctggtacctgttccagttccaccggctcctgcagtacgcacggcccaagccaggcagccccaggcccttcttctggatgttcgtggacaatctggtgctgaacaaggaagacctggacgtcgcatctcgcttcctggagatggagccagtcaccatcccagatgtccacggcggatccttgcagaatgctgtccgcgtgtggagcaacatcccagccataaggagcagcaggcactgggctctggtttcggaagaagaattgtccctgctggcccagaacaagcagagctcgaagctcgcggccaagtggcccaccaagctggtgaagaactgctttctccccctaagagaatatttcaagtatttttcaggagggccgagctctggcgcacccccaccaagtggagggtctcctgccgggtccccaacatctactgaagaaggcaccagcgaatccgcaacgcccgagtcaggccctggtacctccacagaaccatctgaaggtagtgcgcctggttccccagctggaagccctacttccaccgaagaaggcacgtcaaccgaaccaagtgaaggatctgcccctgggaccagcactgaaccatctgagccaaaaaagaagagaaaggtaatgggcatcaccatgagcgacaccaccttcagaccctacaagagcaagctgaaccccaacgagcggaagatgcctatggtggtggacaccatgaattggtgcgacaacgcctgcagcgtgttcttcgatctgttcgtgggcctgtacggcggcgtgaagatcggcgacgtgaccaatttcctgaccgagaagcaggacaccaccaccgatgccgatctgctgtgcgccatcaactggttcagagccatgcctgtgtctaaccccgatgccgttgtgggacctgagcagctggttgtgcggttcagagactacagcggccacaatccatctccaatggccagcatgtacctgagcgcccctgtgaaccctagatacacctgggtcgactgccggttcctgtaccagcagatgtgtcagaccctgggcgccaacctggatgtggacatctctaccctggtgcagaccggcctgctgcctatccagaaggatacacagctgaacgcctacagcttctgcagcaacgtgttcggcgagggcgtgaaagaagatcccagcgccaaagtgaccagctacacagccgctgccaatgctctgagcggcgccaccaatcctatcatcacctacgaggactaccggcagatcctgtccagcgccatcaccaacagacccagcagaaagggcgccaaggatattctggccgccgatctggatagcaccaagacaggtgttctgcccggcaactacgtgtcccagagaatcgccatgtaccaggcctctgccgcctctaaagctagaggcgtggtgctgcccaaccggctgagagtgaaagcctacctgcagaacctcgtgggactgaactacatctgcaccacctgggccgctcctatgctgagagccgtgggcgacatcaagagcaagaacagcaacaactaccgcttcgtgggcgagagactggaacggcagcaagagatcgataacctgctggccgtgtccaacatcagaagcgcccaggccatcctgcagcagttcagggccaatgagagcaaccagttctacatcaagaagcggcacatcggcaagggcctgcctagcctgtacgacatgtgggatctgatggacgagaaagagggcatcgacaactacatccagagcctgaagggcgacaagaccgagaggctgccaatcagagagctgctgcagatcatctaccctcacagaaagagcgtgtccgccgagctgtttctgtctgccgccgaactgaccgacgtggaagatagacagaaccggtgcatggtgcaccctacagtgcggggctctctggtcatcaacttcggcaagagcagcaccatcttcggcgctatcacccctcctgacacactgatcaagttccggggcgaaatggtgcctgctggacagacaggcatgatctggttcacaatgcacctggtggacggcggcaaatgggtcaagcaccacattccttgccacagcagccggtacttcgaggaaatctacgcctggaagaaggacctgcctacactgccctttccacggcggagcctgtatggctatgccatcggcaacaagatcagcgacacccggaagatcgacctgcggagaaagaaggccagcaagcagtacctgcggaccctggaaaacatgacccacaacgtggaatttgaccccaccacacagttcatggtggaccaagagctgaacgtgaccatcaccgccagagtgaagaaaatccctcctgtgcgggatgtgcccgtgggcagcagaattatgggcctgaacaagaaccagaccatccgggactgctacagcatctgggagagagtggaagccaacaccagcggcagctttcagcatcccgtggtccaggatgtgtggctgagactggtggccgatggccacgtgacctctacagtgaatggccccaacggccagatcgaccagatgagctactctggccccgatgtggccaactgcggcaactggatgcaagagcggagcaacttcatcaccagcgtggacgacgccgaccagtctatcatgaagcactttctgtggaacaaccgcgtgaagctgtatgcctggaactgcgtgtacgccggcacactgatgaaggccatctctaagcagatgaccaccgccaaccggaacctgttcagaaacgagatcctgagcttcgttggcggcagattcggctgcagactgggatctctggcccaggtttcactggacctgctgcggaggatgaagtccgtgatcagctgctacttcagccggaacaacgccttcaccatcgaggaaagaagcgccttcgacaaagaactgatggaactgttcgagagcctggacaacaagatgaacaacaagcggaaagagaaagtcaaccggacactcagcagcatcttccaggtggccaagcagcacaatgttgtgcggctggtggtcaccaagaacctgcagacccctgatgccaatgtgcggagcgtgatgaatcagagatccgtggattggtgcgctcggaagattgaagagaagatcgtggacctgggcaacgtgatcggaatctatgtggatctggtggaagccctggatctgagccatctggaccccttcatctatatcgccaagggcgacgtgggcaaagagtgccagtttgacgaggtggaaagcagctccctgctgccaattcacaccagcatgtttcgcgactggcacggcctggttaacaagggcagaaccaccacacctatctaccacagcgccctgaggagcttcgccagccactacggcctgagattcgatgacctggccagaatcaaggccgctgagctggccaaaatgctgccagaccagaaggtgttcatcccacacagaggcggacggttcttcatgagcacataccccgtgaccagcaccagcagacccgtgtcttatgatggccggcagcggttcctgaacagcggcgatatggtggccccagtgaacaccatgctgcgcggattcagaagggccagatctgcctatccctatgacgtgcccgattatgccagcctgggcagcggctcccccaagaaaaaacgcaaggtggaagatcctaagaaaaagcggaaagtggacggcattggtagtgggagcaacggcagcagcggagaggaactgctgagcaagaactaccacctggaaaacgaggtggccagactgaagaaaggctctggctctggcggaagcggttctggcggatcaggatctggaagtggcggctctggaagcggaggttctggatctggcgaagaactgctgtctaagaattatcacggttcaggctccggccagcggggaagcaagcgcaccgccgatggttccgagttcgaaagccccaaaaaaaagcgcaaggtctgagatcccaagcacgcagcaatgcagctcaaaacgcttagcctagccacacccccacgggaaacagcagtgattaacctttagcaataaacgaaagtttaactaagctatactaaccccagggttggtcaatttcgtgccagccacaccctggtactgcatgcacgcaatgctagctgcccctttcccgtcctgggcaccccgagtctcccccgaccccgggtcccaggtatgctcccacctccacctgccccactcaccacctctgctagttccagacacctccgagacgaggaaaaaaaaaaaaaaaaaaaaaaaaaaaaaaaaaaaaaaaaaaaaaaaaaaaaaaaaaaaaaaaaaaaaaaaaaaaaaaaaaaaaaaaaaaaaaaaaaaaaaaaaaaaaaaaaaaaaaaaa

SEQ ID NO: 261 - RNA, 8044 nt, synthetic construct
  misc_feature 1..8044: note = mRNA of V20_KRAB-scFv-2a-D3a-D3l-dCas9-2xGCN4
  source 1..8044: mol_type = other RNA
aggactcactatttgttttcgcgcccagttgcaaaaagtgtcgacatttgcttctgacacaactgtgttcactagcaacctcaaacagacaccgccaccatgcctgctgctaagagagtgaaactggatggatcccggacactggtgaccttcaaggatgtatttgtggacttcaccagggaggagtggaagctgctggacactgctcagcagatcgtgtacagaaatgtgatgctggagaactataagaacctggtttccttgggttatcagcttactaagccagatgtgatcctccggttggagaagggagaagagcccggaagcggaatgggccccgacatcgtgatgacccagagccccagcagcctgagcgccagcgtgggcgaccgcgtgaccatcacctgccgcagcagcaccggcgccgtgaccaccagcaactacgccagctgggtgcaggagaagcccggcaagctgttcaagggcctgatcggcggcaccaacaaccgcgcccccggcgtgcccagccgcttcagcggcagcctgatcggcgacaaggccaccctgaccatcagcagcctgcagcccgaggacttcgccacctacttctgcgccctgtggtacagcaaccactgggtgttcggccagggcaccaaggtggagctgaagcgcggcggcggcggcagcggcggcggcggcagcggcggcggcggcagcagcggcggcggcagcgaggtgaagctgctggagagcggcggcggcctggtgcagcccggcggcagcctgaagctgagctgcgccgtgagcggcttcagcctgaccgactacggcgtgaactgggtgcgccaggcccccggccgcggcctggagtggatcggcgtgatctggggcgacggcatcaccgactacaacagcgccctgaaggaccgcttcatcatcagcaaggacaacggcaagaacaccgtgtacctgcagatgagcaaggtgcgcagcgacgacaccgccctgtactactgcgtgaccggcctgttcgactactggggccagggcaccctggtgaccgtgagcagctacccatacgatgttccagattacgctggtggaggcggaggttctgggggaggaggtagtggcggtggtggttcaggaggcggcggaagcggaagcggagctactaacttcagcctgctgaagcaggctggagacgtggaggagaaccctggacctatgcctgctgctaagagagtgaaactggatggatccaaccatgaccaggaatttgaccccccaaaggtttacccacctgtgccagctgagaagaggaagcccatccgcgtgctgtctctctttgatgggattgctacagggctcctggtgctgaaggacctgggcatccaagtggaccgctacattgcctccgaggtgtgtgaggactccatcacggtgggcatggtgcggcaccagggaaagatcatgtacgtcggggacgtccgcagcgtcacacagaagcatatccaggagtggggcccattcgacctggtgattggaggcagtccctgcaatgacctctccattgtcaaccctgcccgcaagggactttatgagggtactggccgcctcttctttgagttctaccgcctcctgcatgatgcgcggcccaaggagggagatgatcgccccttcttctggctctttgagaatgtggtggccatgggcgttagtgacaagagggacatctcgcgatttcttgagtctaaccccgtgatgattgacgccaaagaagtgtctgctgcacacagggcccgttacttctggggtaaccttcctggcatgaacaggcctttggcatccactgtgaatgataagctggagctgcaagagtgtctggagcacggcagaatagccaagttcagcaaagtgaggaccattaccaccaggtcaaactctataaagcagggcaaagaccagcatttccccgtgttcatgaacgagaaggaggacatcctgtggtgcactgaaatggaaagggtgtttggcttccccgtccactacacagacgtctccaacatgagccgcttggcgaggcagagactgctgggccgatcgtggagcgtgccggtcatccgccacctcttcgctccgctgaaggaatattttgcttgtgtgtctagcggcaatagtaacgctaacagccgcgggccgagcttcagcagcggcctggtgccgttaagcttgcgcggcagccatatgttcgaaaccgtgcctgtgtggaggagacagccagtccgggtgctgtccctttttgaagacatcaagaaagagctgacgagtttgggctttttggaaagtggttctgacccgggacaactgaagcatgtggttgatgtcacagacacagtgaggaaggatgtggaggagtggggacccttcgatcttgtgtacggcgccacacctcccctgggccacacctgtgaccgtcctcccagctggtacctgttccagttccaccggctcctgcagtacgcacggcccaagccaggcagccccaggcccttcttctggatgttcgtggacaatctggtgctgaacaaggaagacctggacgtcgcatctcgcttcctggagatggagccagtcaccatcccagatgtccacggcggatccttgcagaatgctgtccgcgtgtggagcaacatcccagccataaggagcagcaggcactgggctctggtttcggaagaagaattgtccctgctggcccagaacaagcagagctcgaagctcgcggccaagtggcccaccaagctggtgaagaactgctttctccccctaagagaatatttcaagtatttttcaggagggccgagctctggcgcacccccaccaagtggagggtctcctgccgggtccccaacatctactgaagaaggcaccagcgaatccgcaacgcccgagtcaggccctggtacctccacagaaccatctgaaggtagtgcgcctggttccccagctggaagccctacttccaccgaagaaggcacgtcaaccgaaccaagtgaaggatctgcccctgggaccagcactgaaccatctgagccaaaaaagaagagaaaggtaatggacaagaagtacagcatcggcctggccatcggcaccaactctgtgggctgggccgtgatcaccgacgagtacaaggtgcccagcaagaaattcaaggtgctgggcaacaccgaccggcacagcatcaagaagaacctgatcggcgccctgctgttcgacagcggagaaacagccgaggccacccggctgaagagaaccgccagaagaagatacaccagacggaagaaccggatctgctatctgcaagagatcttcagcaacgagatggccaaggtggacgacagcttcttccacagactggaagagtccttcctggtggaagaggataagaagcacgagcggcaccccatcttcggcaacatcgtggacgaggtggcctaccacgagaagtaccccaccatctaccacctgagaaagaaactggtggacagcaccgacaaggccgacctgcggctgatctatctggccctggcccacatgatcaagttccggggccacttcctgatcgagggcgacctgaaccccgacaacagcgacgtggacaagctgttcatccagctggtgcagacctacaaccagctgttcgaggaaaaccccatcaacgccagcggcgtggacgccaaggccatcctgtctgccagactgagcaagagcagacggctggaaaatctgatcgcccagctgcccggcgagaagaagaatggcctgttcggcaacctgattgccctgagcctgggcctgacccccaacttcaagagcaacttcgacctggccgaggatgccaaactgcagctgagcaaggacacctacgacgacgacctggacaacctgctggcccagatcggcgaccagtacgccgacctgtttctggccgccaagaacctgtccgacgccatcctgctgagcgacatcctgagagtgaacaccgagatcaccaaggcccccctgagcgcctctatgatcaagagatacgacgagcaccaccaggacctgaccctgctgaaagctctcgtgcggcagcagctgcctgagaagtacaaagagattttcttcgaccagagcaagaacggctacgccggctacatcgatggcggagccagccaggaagagttctacaagttcatcaagcccatcctggaaaagatggacggcaccgaggaactgctcgtgaagctgaacagagaggacctgctgcggaagcagcggaccttcgacaacggcagcatcccccaccagatccacctgggagagctgcacgccattctgcggcggcaggaagatttttacccattcctgaaggacaaccgggaaaagatcgagaagatcctgaccttccgcatcccctactacgtgggccctctggccaggggaaacagcagattcgcctggatgaccagaaagagcgaggaaaccatcaccccctggaacttcgaggaagtggtggacaagggcgccagcgcccagagcttcatcgagcggatgaccaacttcgataagaacctgcccaacgagaaggtgctgcccaagcacagcctgctgtacgagtacttcaccgtgtacaacgagctgaccaaagtgaaatacgtgaccgagggaatgagaaagcccgccttcctgagcggcgagcagaaaaaagccatcgtggacctgctgttcaagaccaaccggaaagtgaccgtgaagcagctgaaagaggactacttcaagaaaatcgagtgcttcgactccgtggaaatctccggcgtggaagatcggttcaacgcctccctgggcacataccacgatctgctgaaaattatcaaggacaaggacttcctggacaatgaggaaaacgaggacattctggaagatatcgtgctgaccctgacactgtttgaggacagagagatgatcgaggaacggctgaaaacctatgcccacctgttcgacgacaaagtgatgaagcagctgaagcggcggagatacaccggctggggcaggctgagccggaagctgatcaacggcatccgggacaagcagtccggcaagacaatcctggatttcctgaagtccgacggcttcgccaacagaaacttcatgcagctgatccacgacgacagcctgacctttaaagaggacatccagaaagcccaggtgtccggccagggcgatagcctgcacgagcacattgccaatctggccggcagccccgccattaagaagggcatcctgcagacagtgaaggtggtggacgagctcgtgaaagtgatgggccggcacaagcccgagaacatcgtgatcgaaatggccagagagaaccagaccacccagaagggacagaagaacagccgcgagagaatgaagcggatcgaagagggcatcaaagagctgggcagccagatcctgaaagaacaccccgtggaaaacacccagctgcagaacgagaagctgtacctgtactacctgcagaatgggcgggatatgtacgtggaccaggaactggacatcaaccggctgtccgactacgatgtggacgctatcgtgcctcagagctttctgaaggacgactccatcgataacaaagtgctgactcggagcgacaagaaccggggcaagagcgacaacgtgccctccgaagaggtcgtgaagaagatgaagaactactggcgccagctgctgaatgccaagctgattacccagaggaagttcgacaatctgaccaaggccgagagaggcggcctgagcgaactggataaggccggcttcatcaagagacagctggtggaaacccggcagatcacaaagcacgtggcacagatcctggactcccggatgaacactaagtacgacgagaacgacaaactgatccgggaagtgaaagtgatcaccctgaagtccaagctggtgtccgatttccggaaggatttccagttttacaaagtgcgcgagatcaacaactaccaccacgcccacgacgcctacctgaacgccgtcgtgggaaccgccctgatcaaaaagtaccctaagctggaaagcgagttcgtgtacggcgactacaaggtgtacgacgtgcggaagatgatcgccaagagcgagcaggaaatcggcaaggctaccgccaagtacttcttctacagcaacatcatgaactttttcaagaccgagattaccctggccaacggcgagatccggaagcggcctctgatcgagacaaacggcgaaacaggcgagatcgtgtgggataagggccgggactttgccaccgtgcggaaagtgctgtctatgccccaagtgaatatcgtgaaaaagaccgaggtgcagacaggcggcttcagcaaagagtctatcctgcccaagaggaacagcgacaagctgatcgccagaaagaaggactgggaccctaagaagtacggcggcttcgacagccccaccgtggcctattctgtgctggtggtggccaaagtggaaaagggcaagtccaagaaactgaagagtgtgaaagagctgctggggatcaccatcatggaaagaagcagcttcgagaagaatcccatcgactttctggaagccaagggctacaaagaagtgaaaaaggacctgatcatcaagctgcctaagtactccctgttcgagctggaaaacggccggaagagaatgctggcctctgccggcgaactgcagaagggaaacgaactggccctgccctccaaatatgtgaacttcctgtacctggccagccactatgagaagctgaagggctcccccgaggataatgagcagaaacagctgtttgtggaacagcacaaacactacctggacgagatcatcgagcagatcagcgagttctccaagagagtgatcctggccgacgctaatctggacaaggtgctgagcgcctacaacaagcacagagacaagcctatcagagagcaggccgagaatatcatccacctgtttaccctgaccaatctgggagcccctgccgccttcaagtactttgacaccaccatcgaccggaagaggtacaccagcaccaaagaggtgctggacgccaccctgatccaccagagcatcaccggcctgtacgagacacggatcgacctgtctcagctgggaggcgacgcctatccctatgacgtgcccgattatgccagcctgggcagcggctcccccaagaaaaaacgcaaggtggaagatcctaagaaaaagcggaaagtggacggcattggtagtgggagcaacggcagcagcggagaggaactgctgagcaagaactaccacctggaaaacgaggtggccagactgaagaaaggctctggctctggcggaagcggttctggcggatcaggatctggaagtggcggctctggaagcggaggttctggatctggcgaagaactgctgtctaagaattatcacctcgagaatgaagtcgctcgtttgaagaaaggttcaggctccggccagcggggaagcaagcgcaccgccgatggttccgagttcgaaagccccaaaaaaaagcgcaaggtctgagatcccaagcacgcagcaatgcagctcaaaacgcttagcctagccacacccccacgggaaacagcagtgattaacctttagcaataaacgaaagtttaactaagctatactaaccccagggttggtcaatttcgtgccagccacaccctggtactgcatgcacgcaatgctagctgcccctttcccgtcctgggcaccccgagtctcccccgaccccgggtcccaggtatgctcccacctccacctgccccactcaccacctctgctagttccagacacctccgagacgaggaaaaaaaaaaaaaaaaaaaaaaaaaaaaaaaaaaaaaaaaaaaaaaaaaaaaaaaaaaaaaaaaaaaaaaaaaaaaaaaaaaaaaaaaaaaaaaaaaaaaaaaaaaaaaaaaaaaaaaaa

SEQ ID NO: 262 - RNA, 8761 nt, synthetic construct
  misc_feature 1..8761: note = mRNA of V21_hSIRT1-scFv-2a-D3a-D3l-dCas9-2xGCN4
  source 1..8761: mol_type = other RNA
aggactcactatttgttttcgcgcccagttgcaaaaagtgtcgacatttgcttctgacacaactgtgttcactagcaacctcaaacagacaccgccaccatgcctgctgctaagagagtgaaactggatggatccacaattcttaaagatttattgccggaaacaatacctccacctgagttggatgatatgacactgtggcagattgttattaatatcctttcagaaccaccaaaaaggaaaaaaagaaaagatattaatacaattgaagatgctgtgaaattactgcaagagtgcaaaaaaattatagttctaactggagctggggtgtctgtttcatgtggaatacctgacttcaggtcaagggatggtatttatgctcgccttgctgtagacttcccagatcttccagatcctcaagcgatgtttgatattgaatatttcagaaaagatccaagaccattcttcaagtttgcaaaggaaatatatcctggacaattccagccatctctctgtcacaaattcatagccttgtcagataaggaaggaaaactacttcgcaactatacccagaacatagacacgctggaacaggttgcgggaatccaaaggataattcagtgtcatggttcctttgcaacagcatcttgcctgatttgtaaatacaaagttgactgtgaagctgtacgaggagatatttttaatcaggtagttcctcgatgtcctaggtgcccagctgatgaaccgcttgctatcatgaaaccagagattgtgttttttggtgaaaatttaccagaacagtttcatagagccatgaagtatgacaaagatgaagttgacctcctcattgttattgggtcttccctcaaagtaagaccagtagcactaattccaagttccataccccatgaagtgcctcagatattaattaatagagaacctttgcctcatctgcattttgatgtagagcttcttggagactgtgatgtcataattaatgaattgtgtcataggttaggtggtgaatatgccaaacttggaagcggaatgggccccgacatcgtgatgacccagagccccagcagcctgagcgccagcgtgggcgaccgcgtgaccatcacctgccgcagcagcaccggcgccgtgaccaccagcaactacgccagctgggtgcaggagaagcccggcaagctgttcaagggcctgatcggcggcaccaacaaccgcgcccccggcgtgcccagccgcttcagcggcagcctgatcggcgacaaggccaccctgaccatcagcagcctgcagcccgaggacttcgccacctacttctgcgccctgtggtacagcaaccactgggtgttcggccagggcaccaaggtggagctgaagcgcggcggcggcggcagcggcggcggcggcagcggcggcggcggcagcagcggcggcggcagcgaggtgaagctgctggagagcggcggcggcctggtgcagcccggcggcagcctgaagctgagctgcgccgtgagcggcttcagcctgaccgactacggcgtgaactgggtgcgccaggcccccggccgcggcctggagtggatcggcgtgatctggggcgacggcatcaccgactacaacagcgccctgaaggaccgcttcatcatcagcaaggacaacggcaagaacaccgtgtacctgcagatgagcaaggtgcgcagcgacgacaccgccctgtactactgcgtgaccggcctgttcgactactggggccagggcaccctggtgaccgtgagcagctacccatacgatgttccagattacgctggtggaggcggaggttctgggggaggaggtagtggcggtggtggttcaggaggcggcggaagcggaagcggagctactaacttcagcctgctgaagcaggctggagacgtggaggagaaccctggacctatgcctgctgctaagagagtgaaactggatggatccaaccatgaccaggaatttgaccccccaaaggtttacccacctgtgccagctgagaagaggaagcccatccgcgtgctgtctctctttgatgggattgctacagggctcctggtgctgaaggacctgggcatccaagtggaccgctacattgcctccgaggtgtgtgaggactccatcacggtgggcatggtgcggcaccagggaaagatcatgtacgtcggggacgtccgcagcgtcacacagaagcatatccaggagtggggcccattcgacctggtgattggaggcagtccctgcaatgacctctccattgtcaaccctgcccgcaagggactttatgagggtactggccgcctcttctttgagttctaccgcctcctgcatgatgcgcggcccaaggagggagatgatcgccccttcttctggctctttgagaatgtggtggccatgggcgttagtgacaagagggacatctcgcgatttcttgagtctaaccccgtgatgattgacgccaaagaagtgtctgctgcacacagggcccgttacttctggggtaaccttcctggcatgaacaggcctttggcatccactgtgaatgataagctggagctgcaagagtgtctggagcacggcagaatagccaagttcagcaaagtgaggaccattaccaccaggtcaaactctataaagcagggcaaagaccagcatttccccgtgttcatgaacgagaaggaggacatcctgtggtgcactgaaatggaaagggtgtttggcttccccgtccactacacagacgtctccaacatgagccgcttggcgaggcagagactgctgggccgatcgtggagcgtgccggtcatccgccacctcttcgctccgctgaaggaatattttgcttgtgtgtctagcggcaatagtaacgctaacagccgcgggccgagcttcagcagcggcctggtgccgttaagcttgcgcggcagccatatgttcgaaaccgtgcctgtgtggaggagacagccagtccgggtgctgtccctttttgaagacatcaagaaagagctgacgagtttgggctttttggaaagtggttctgacccgggacaactgaagcatgtggttgatgtcacagacacagtgaggaaggatgtggaggagtggggacccttcgatcttgtgtacggcgccacacctcccctgggccacacctgtgaccgtcctcccagctggtacctgttccagttccaccggctcctgcagtacgcacggcccaagccaggcagccccaggcccttcttctggatgttcgtggacaatctggtgctgaacaaggaagacctggacgtcgcatctcgcttcctggagatggagccagtcaccatcccagatgtccacggcggatccttgcagaatgctgtccgcgtgtggagcaacatcccagccataaggagcagcaggcactgggctctggtttcggaagaagaattgtccctgctggcccagaacaagcagagctcgaagctcgcggccaagtggcccaccaagctggtgaagaactgctttctccccctaagagaatatttcaagtatttttcaggagggccgagctctggcgcacccccaccaagtggagggtctcctgccgggtccccaacatctactgaagaaggcaccagcgaatccgcaacgcccgagtcaggccctggtacctccacagaaccatctgaaggtagtgcgcctggttccccagctggaagccctacttccaccgaagaaggcacgtcaaccgaaccaagtgaaggatctgcccctgggaccagcactgaaccatctgagccaaaaaagaagagaaaggtaatggacaagaagtacagcatcggcctggccatcggcaccaactctgtgggctgggccgtgatcaccgacgagtacaaggtgcccagcaagaaattcaaggtgctgggcaacaccgaccggcacagcatcaagaagaacctgatcggcgccctgctgttcgacagcggagaaacagccgaggccacccggctgaagagaaccgccagaagaagatacaccagacggaagaaccggatctgctatctgcaagagatcttcagcaacgagatggccaaggtggacgacagcttcttccacagactggaagagtccttcctggtggaagaggataagaagcacgagcggcaccccatcttcggcaacatcgtggacgaggtggcctaccacgagaagtaccccaccatctaccacctgagaaagaaactggtggacagcaccgacaaggccgacctgcggctgatctatctggccctggcccacatgatcaagttccggggccacttcctgatcgagggcgacctgaaccccgacaacagcgacgtggacaagctgttcatccagctggtgcagacctacaaccagctgttcgaggaaaaccccatcaacgccagcggcgtggacgccaaggccatcctgtctgccagactgagcaagagcagacggctggaaaatctgatcgcccagctgcccggcgagaagaagaatggcctgttcggcaacctgattgccctgagcctgggcctgacccccaacttcaagagcaacttcgacctggccgaggatgccaaactgcagctgagcaaggacacctacgacgacgacctggacaacctgctggcccagatcggcgaccagtacgccgacctgtttctggccgccaagaacctgtccgacgccatcctgctgagcgacatcctgagagtgaacaccgagatcaccaaggcccccctgagcgcctctatgatcaagagatacgacgagcaccaccaggacctgaccctgctgaaagctctcgtgcggcagcagctgcctgagaagtacaaagagattttcttcgaccagagcaagaacggctacgccggctacatcgatggcggagccagccaggaagagttctacaagttcatcaagcccatcctggaaaagatggacggcaccgaggaactgctcgtgaagctgaacagagaggacctgctgcggaagcagcggaccttcgacaacggcagcatcccccaccagatccacctgggagagctgcacgccattctgcggcggcaggaagatttttacccattcctgaaggacaaccgggaaaagatcgagaagatcctgaccttccgcatcccctactacgtgggccctctggccaggggaaacagcagattcgcctggatgaccagaaagagcgaggaaaccatcaccccctggaacttcgaggaagtggtggacaagggcgccagcgcccagagcttcatcgagcggatgaccaacttcgataagaacctgcccaacgagaaggtgctgcccaagcacagcctgctgtacgagtacttcaccgtgtacaacgagctgaccaaagtgaaatacgtgaccgagggaatgagaaagcccgccttcctgagcggcgagcagaaaaaagccatcgtggacctgctgttcaagaccaaccggaaagtgaccgtgaagcagctgaaagaggactacttcaagaaaatcgagtgcttcgactccgtggaaatctccggcgtggaagatcggttcaacgcctccctgggcacataccacgatctgctgaaaattatcaaggacaaggacttcctggacaatgaggaaaacgaggacattctggaagatatcgtgctgaccctgacactgtttgaggacagagagatgatcgaggaacggctgaaaacctatgcccacctgttcgacgacaaagtgatgaagcagctgaagcggcggagatacaccggctggggcaggctgagccggaagctgatcaacggcatccgggacaagcagtccggcaagacaatcctggatttcctgaagtccgacggcttcgccaacagaaacttcatgcagctgatccacgacgacagcctgacctttaaagaggacatccagaaagcccaggtgtccggccagggcgatagcctgcacgagcacattgccaatctggccggcagccccgccattaagaagggcatcctgcagacagtgaaggtggtggacgagctcgtgaaagtgatgggccggcacaagcccgagaacatcgtgatcgaaatggccagagagaaccagaccacccagaagggacagaagaacagccgcgagagaatgaagcggatcgaagagggcatcaaagagctgggcagccagatcctgaaagaacaccccgtggaaaacacccagctgcagaacgagaagctgtacctgtactacctgcagaatgggcgggatatgtacgtggaccaggaactggacatcaaccggctgtccgactacgatgtggacgctatcgtgcctcagagctttctgaaggacgactccatcgataacaaagtgctgactcggagcgacaagaaccggggcaagagcgacaacgtgccctccgaagaggtcgtgaagaagatgaagaactactggcgccagctgctgaatgccaagctgattacccagaggaagttcgacaatctgaccaaggccgagagaggcggcctgagcgaactggataaggccggcttcatcaagagacagctggtggaaacccggcagatcacaaagcacgtggcacagatcctggactcccggatgaacactaagtacgacgagaacgacaaactgatccgggaagtgaaagtgatcaccctgaagtccaagctggtgtccgatttccggaaggatttccagttttacaaagtgcgcgagatcaacaactaccaccacgcccacgacgcctacctgaacgccgtcgtgggaaccgccctgatcaaaaagtaccctaagctggaaagcgagttcgtgtacggcgactacaaggtgtacgacgtgcggaagatgatcgccaagagcgagcaggaaatcggcaaggctaccgccaagtacttcttctacagcaacatcatgaactttttcaagaccgagattaccctggccaacggcgagatccggaagcggcctctgatcgagacaaacggcgaaacaggcgagatcgtgtgggataagggccgggactttgccaccgtgcggaaagtgctgtctatgccccaagtgaatatcgtgaaaaagaccgaggtgcagacaggcggcttcagcaaagagtctatcctgcccaagaggaacagcgacaagctgatcgccagaaagaaggactgggaccctaagaagtacggcggcttcgacagccccaccgtggcctattctgtgctggtggtggccaaagtggaaaagggcaagtccaagaaactgaagagtgtgaaagagctgctggggatcaccatcatggaaagaagcagcttcgagaagaatcccatcgactttctggaagccaagggctacaaagaagtgaaaaaggacctgatcatcaagctgcctaagtactccctgttcgagctggaaaacggccggaagagaatgctggcctctgccggcgaactgcagaagggaaacgaactggccctgccctccaaatatgtgaacttcctgtacctggccagccactatgagaagctgaagggctcccccgaggataatgagcagaaacagctgtttgtggaacagcacaaacactacctggacgagatcatcgagcagatcagcgagttctccaagagagtgatcctggccgacgctaatctggacaaggtgctgagcgcctacaacaagcacagagacaagcctatcagagagcaggccgagaatatcatccacctgtttaccctgaccaatctgggagcccctgccgccttcaagtactttgacaccaccatcgaccggaagaggtacaccagcaccaaagaggtgctggacgccaccctgatccaccagagcatcaccggcctgtacgagacacggatcgacctgtctcagctgggaggcgacgcctatccctatgacgtgcccgattatgccagcctgggcagcggctcccccaagaaaaaacgcaaggtggaagatcctaagaaaaagcggaaagtggacggcattggtagtgggagcaacggcagcagcggagaggaactgctgagcaagaactaccacctggaaaacgaggtggccagactgaagaaaggctctggctctggcggaagcggttctggcggatcaggatctggaagtggcggctctggaagcggaggttctggatctggcgaagaactgctgtctaagaattatcacctcgagaatgaagtcgctcgtttgaagaaaggttcaggctccggccagcggggaagcaagcgcaccgccgatggttccgagttcgaaagccccaaaaaaaagcgcaaggtctgagatcccaagcacgcagcaatgcagctcaaaacgcttagcctagccacacccccacgggaaacagcagtgattaacctttagcaataaacgaaagtttaactaagctatactaaccccagggttggtcaatttcgtgccagccacaccctggtactgcatgcacgcaatgctagctgcccctttcccgtcctgggcaccccgagtctcccccgaccccgggtcccaggtatgctcccacctccacctgccccactcaccacctctgctagttccagacacctccgagacgaggaaaaaaaaaaaaaaaaaaaaaaaaaaaaaaaaaaaaaaaaaaaaaaaaaaaaaaaaaaaaaaaaaaaaaaaaaaaaaaaaaaaaaaaaaaaaaaaaaaaaaaaaaaaaaaaaaaaaaaaa

SEQ ID NO: 263 - RNA, 7972 nt, synthetic construct
  misc_feature 1..7972: note = mRNA of V22_D3a-D3l-scFv-2a-1xGCN4-dCas9-KRAB
  source 1..7972: mol_type = other RNA
aggactcactatttgttttcgcgcccagttgcaaaaagtgtcgacatttgcttctgacacaactgtgttcactagcaacctcaaacagacaccgccaccatgcctgctgctaagagagtgaaactggatggatccaaccatgaccaggaatttgaccccccaaaggtttacccacctgtgccagctgagaagaggaagcccatccgcgtgctgtctctctttgatgggattgctacagggctcctggtgctgaaggacctgggcatccaagtggaccgctacattgcctccgaggtgtgtgaggactccatcacggtgggcatggtgcggcaccagggaaagatcatgtacgtcggggacgtccgcagcgtcacacagaagcatatccaggagtggggcccattcgacctggtgattggaggcagtccctgcaatgacctctccattgtcaaccctgcccgcaagggactttatgagggtactggccgcctcttctttgagttctaccgcctcctgcatgatgcgcggcccaaggagggagatgatcgccccttcttctggctctttgagaatgtggtggccatgggcgttagtgacaagagggacatctcgcgatttcttgagtctaaccccgtgatgattgacgccaaagaagtgtctgctgcacacagggcccgttacttctggggtaaccttcctggcatgaacaggcctttggcatccactgtgaatgataagctggagctgcaagagtgtctggagcacggcagaatagccaagttcagcaaagtgaggaccattaccaccaggtcaaactctataaagcagggcaaagaccagcatttccccgtgttcatgaacgagaaggaggacatcctgtggtgcactgaaatggaaagggtgtttggcttccccgtccactacacagacgtctccaacatgagccgcttggcgaggcagagactgctgggccgatcgtggagcgtgccggtcatccgccacctcttcgctccgctgaaggaatattttgcttgtgtgtctagcggcaatagtaacgctaacagccgcgggccgagcttcagcagcggcctggtgccgttaagcttgcgcggcagccatatgggccctatggagatatacaagacagtgtctgcatggaagagacagccagtgcgggtactgagcctcttcagaaacatcgacaaggtactaaagagtttgggcttcttggaaagcggttctggttctgggggaggaacgctgaagtacgtggaagatgtcacaaatgtcgtgaggagagacgtggagaaatggggcccctttgacctggtgtacggctcgacgcagcccctaggcagctcttgtgatcgctgtcccggctggtacatgttccagttccaccggatcctgcagtatgcgctgcctcgccaggagagtcagcggcccttcttctggatattcatggacaatctgctgctgactgaggatgaccaagagacaactacccgcttccttcagacagaggctgtgaccctccaggatgtccgtggcagagactaccagaatgctatgcgggtgtggagcaacattccagggctgaagagcaagcatgcgcccctgaccccaaaggaagaagagtatctgcaagcccaagtcagaagcaggagcaagctggacgccccgaaagttgacctcctggtgaagaactgccttctcccgctgagagagtacttcaagtatttttctcaaaactcacttcctcttggagggccgagctctggcgcacccccaccaagtggagggtctcctgccgggtccccaacatctactgaagaaggcaccagcgaatccgcaacgcccgagtcaggccctggtacctccacagaaccatctgaaggtagtgcgcctggttccccagctggaagccctacttccaccgaagaaggcacgtcaaccgaaccaagtgaaggatctgcccctgggaccagcactgaaccatctgagggccccgacatcgtgatgacccagagccccagcagcctgagcgccagcgtgggcgaccgcgtgaccatcacctgccgcagcagcaccggcgccgtgaccaccagcaactacgccagctgggtgcaggagaagcccggcaagctgttcaagggcctgatcggcggcaccaacaaccgcgcccccggcgtgcccagccgcttcagcggcagcctgatcggcgacaaggccaccctgaccatcagcagcctgcagcccgaggacttcgccacctacttctgcgccctgtggtacagcaaccactgggtgttcggccagggcaccaaggtggagctgaagcgcggcggcggcggcagcggcggcggcggcagcggcggcggcggcagcagcggcggcggcagcgaggtgaagctgctggagagcggcggcggcctggtgcagcccggcggcagcctgaagctgagctgcgccgtgagcggcttcagcctgaccgactacggcgtgaactgggtgcgccaggcccccggccgcggcctggagtggatcggcgtgatctggggcgacggcatcaccgactacaacagcgccctgaaggaccgcttcatcatcagcaaggacaacggcaagaacaccgtgtacctgcagatgagcaaggtgcgcagcgacgacaccgccctgtactactgcgtgaccggcctgttcgactactggggccagggcaccctggtgaccgtgagcagctacccatacgatgttccagattacgctggtggaggcggaggttctgggggaggaggtagtggcggtggtggttcaggaggcggcggaagcggaagcggagctactaacttcagcctgctgaagcaggctggagacgtggaggagaaccctggacctatgcctgctgctaagagagtgaaactggatggatccggctcaggcggatctggttcaggggaagaactcctctccaaaaactaccatctcgagaatgaggtcgcccgcctgaaaaaaggatcaggttccggtggttctggcagcggtggttcaggctcaggcagcggcggtagcggtagcggtggaagcggaagcggaccaaaaaagaagagaaaggtaatggacaagaagtacagcatcggcctggccatcggcaccaactctgtgggctgggccgtgatcaccgacgagtacaaggtgcccagcaagaaattcaaggtgctgggcaacaccgaccggcacagcatcaagaagaacctgatcggcgccctgctgttcgacagcggagaaacagccgaggccacccggctgaagagaaccgccagaagaagatacaccagacggaagaaccggatctgctatctgcaagagatcttcagcaacgagatggccaaggtggacgacagcttcttccacagactggaagagtccttcctggtggaagaggataagaagcacgagcggcaccccatcttcggcaacatcgtggacgaggtggcctaccacgagaagtaccccaccatctaccacctgagaaagaaactggtggacagcaccgacaaggccgacctgcggctgatctatctggccctggcccacatgatcaagttccggggccacttcctgatcgagggcgacctgaaccccgacaacagcgacgtggacaagctgttcatccagctggtgcagacctacaaccagctgttcgaggaaaaccccatcaacgccagcggcgtggacgccaaggccatcctgtctgccagactgagcaagagcagacggctggaaaatctgatcgcccagctgcccggcgagaagaagaatggcctgttcggcaacctgattgccctgagcctgggcctgacccccaacttcaagagcaacttcgacctggccgaggatgccaaactgcagctgagcaaggacacctacgacgacgacctggacaacctgctggcccagatcggcgaccagtacgccgacctgtttctggccgccaagaacctgtccgacgccatcctgctgagcgacatcctgagagtgaacaccgagatcaccaaggcccccctgagcgcctctatgatcaagagatacgacgagcaccaccaggacctgaccctgctgaaagctctcgtgcggcagcagctgcctgagaagtacaaagagattttcttcgaccagagcaagaacggctacgccggctacatcgatggcggagccagccaggaagagttctacaagttcatcaagcccatcctggaaaagatggacggcaccgaggaactgctcgtgaagctgaacagagaggacctgctgcggaagcagcggaccttcgacaacggcagcatcccccaccagatccacctgggagagctgcacgccattctgcggcggcaggaagatttttacccattcctgaaggacaaccgggaaaagatcgagaagatcctgaccttccgcatcccctactacgtgggccctctggccaggggaaacagcagattcgcctggatgaccagaaagagcgaggaaaccatcaccccctggaacttcgaggaagtggtggacaagggcgccagcgcccagagcttcatcgagcggatgaccaacttcgataagaacctgcccaacgagaaggtgctgcccaagcacagcctgctgtacgagtacttcaccgtgtacaacgagctgaccaaagtgaaatacgtgaccgagggaatgagaaagcccgccttcctgagcggcgagcagaaaaaagccatcgtggacctgctgttcaagaccaaccggaaagtgaccgtgaagcagctgaaagaggactacttcaagaaaatcgagtgcttcgactccgtggaaatctccggcgtggaagatcggttcaacgcctccctgggcacataccacgatctgctgaaaattatcaaggacaaggacttcctggacaatgaggaaaacgaggacattctggaagatatcgtgctgaccctgacactgtttgaggacagagagatgatcgaggaacggctgaaaacctatgcccacctgttcgacgacaaagtgatgaagcagctgaagcggcggagatacaccggctggggcaggctgagccggaagctgatcaacggcatccgggacaagcagtccggcaagacaatcctggatttcctgaagtccgacggcttcgccaacagaaacttcatgcagctgatccacgacgacagcctgacctttaaagaggacatccagaaagcccaggtgtccggccagggcgatagcctgcacgagcacattgccaatctggccggcagccccgccattaagaagggcatcctgcagacagtgaaggtggtggacgagctcgtgaaagtgatgggccggcacaagcccgagaacatcgtgatcgaaatggccagagagaaccagaccacccagaagggacagaagaacagccgcgagagaatgaagcggatcgaagagggcatcaaagagctgggcagccagatcctgaaagaacaccccgtggaaaacacccagctgcagaacgagaagctgtacctgtactacctgcagaatgggcgggatatgtacgtggaccaggaactggacatcaaccggctgtccgactacgatgtggacgctatcgtgcctcagagctttctgaaggacgactccatcgataacaaagtgctgactcggagcgacaagaaccggggcaagagcgacaacgtgccctccgaagaggtcgtgaagaagatgaagaactactggcgccagctgctgaatgccaagctgattacccagaggaagttcgacaatctgaccaaggccgagagaggcggcctgagcgaactggataaggccggcttcatcaagagacagctggtggaaacccggcagatcacaaagcacgtggcacagatcctggactcccggatgaacactaagtacgacgagaacgacaaactgatccgggaagtgaaagtgatcaccctgaagtccaagctggtgtccgatttccggaaggatttccagttttacaaagtgcgcgagatcaacaactaccaccacgcccacgacgcctacctgaacgccgtcgtgggaaccgccctgatcaaaaagtaccctaagctggaaagcgagttcgtgtacggcgactacaaggtgtacgacgtgcggaagatgatcgccaagagcgagcaggaaatcggcaaggctaccgccaagtacttcttctacagcaacatcatgaactttttcaagaccgagattaccctggccaacggcgagatccggaagcggcctctgatcgagacaaacggcgaaacaggcgagatcgtgtgggataagggccgggactttgccaccgtgcggaaagtgctgtctatgccccaagtgaatatcgtgaaaaagaccgaggtgcagacaggcggcttcagcaaagagtctatcctgcccaagaggaacagcgacaagctgatcgccagaaagaaggactgggaccctaagaagtacggcggcttcgacagccccaccgtggcctattctgtgctggtggtggccaaagtggaaaagggcaagtccaagaaactgaagagtgtgaaagagctgctggggatcaccatcatggaaagaagcagcttcgagaagaatcccatcgactttctggaagccaagggctacaaagaagtgaaaaaggacctgatcatcaagctgcctaagtactccctgttcgagctggaaaacggccggaagagaatgctggcctctgccggcgaactgcagaagggaaacgaactggccctgccctccaaatatgtgaacttcctgtacctggccagccactatgagaagctgaagggctcccccgaggataatgagcagaaacagctgtttgtggaacagcacaaacactacctggacgagatcatcgagcagatcagcgagttctccaagagagtgatcctggccgacgctaatctggacaaggtgctgagcgcctacaacaagcacagagacaagcctatcagagagcaggccgagaatatcatccacctgtttaccctgaccaatctgggagcccctgccgccttcaagtactttgacaccaccatcgaccggaagaggtacaccagcaccaaagaggtgctggacgccaccctgatccaccagagcatcaccggcctgtacgagacacggatcgacctgtctcagctgggaggcgacgcctatccctatgacgtgcccgattatgccagcctgggcagcggctcccccaagaaaaaacgcaaggtggaagatcctaagaaaaagcggaaagtggacggcagcggcagcgagacccccggtaccagcgagagcgccacccccgagagccggacactggtgaccttcaaggatgtatttgtggacttcaccagggaggagtggaagctgctggacactgctcagcagatcgtgtacagaaatgtgatgctggagaactataagaacctggtttccttgggttatcagcttactaagccagatgtgatcctccggttggagaagggagaagagccctgagatcccaagcacgcagcaatgcagctcaaaacgcttagcctagccacacccccacgggaaacagcagtgattaacctttagcaataaacgaaagtttaactaagctatactaaccccagggttggtcaatttcgtgccagccacaccctggtactgcatgcacgcaatgctagctgcccctttcccgtcctgggcaccccgagtctcccccgaccccgggtcccaggtatgctcccacctccacctgccccactcaccacctctgctagttccagacacctccgagacgaggaaaaaaaaaaaaaaaaaaaaaaaaaaaaaaaaaaaaaaaaaaaaaaaaaaaaaaaaaaaaaaaaaaaaaaaaaaaaaaaaaaaaaaaaaaaaaaaaaaaaaaaaaaaaaaaaaaaaaaaa

SEQ ID NO: 264 - RNA, 8086 nt, synthetic construct
  misc_feature 1..8086: note = mRNA of V23_D3a-D3l-scFv-2a-2xGCN4-dCas9-KRAB
  source 1..8086: mol_type = other RNA
aggactcactatttgttttcgcgcccagttgcaaaaagtgtcgacatttgcttctgacacaactgtgttcactagcaacctcaaacagacaccgccaccatgcctgctgctaagagagtgaaactggatggatccaaccatgaccaggaatttgaccccccaaaggtttacccacctgtgccagctgagaagaggaagcccatccgcgtgctgtctctctttgatgggattgctacagggctcctggtgctgaaggacctgggcatccaagtggaccgctacattgcctccgaggtgtgtgaggactccatcacggtgggcatggtgcggcaccagggaaagatcatgtacgtcggggacgtccgcagcgtcacacagaagcatatccaggagtggggcccattcgacctggtgattggaggcagtccctgcaatgacctctccattgtcaaccctgcccgcaagggactttatgagggtactggccgcctcttctttgagttctaccgcctcctgcatgatgcgcggcccaaggagggagatgatcgccccttcttctggctctttgagaatgtggtggccatgggcgttagtgacaagagggacatctcgcgatttcttgagtctaaccccgtgatgattgacgccaaagaagtgtctgctgcacacagggcccgttacttctggggtaaccttcctggcatgaacaggcctttggcatccactgtgaatgataagctggagctgcaagagtgtctggagcacggcagaatagccaagttcagcaaagtgaggaccattaccaccaggtcaaactctataaagcagggcaaagaccagcatttccccgtgttcatgaacgagaaggaggacatcctgtggtgcactgaaatggaaagggtgtttggcttccccgtccactacacagacgtctccaacatgagccgcttggcgaggcagagactgctgggccgatcgtggagcgtgccggtcatccgccacctcttcgctccgctgaaggaatattttgcttgtgtgtctagcggcaatagtaacgctaacagccgcgggccgagcttcagcagcggcctggtgccgttaagcttgcgcggcagccatatgggccctatggagatatacaagacagtgtctgcatggaagagacagccagtgcgggtactgagcctcttcagaaacatcgacaaggtactaaagagtttgggcttcttggaaagcggttctggttctgggggaggaacgctgaagtacgtggaagatgtcacaaatgtcgtgaggagagacgtggagaaatggggcccctttgacctggtgtacggctcgacgcagcccctaggcagctcttgtgatcgctgtcccggctggtacatgttccagttccaccggatcctgcagtatgcgctgcctcgccaggagagtcagcggcccttcttctggatattcatggacaatctgctgctgactgaggatgaccaagagacaactacccgcttccttcagacagaggctgtgaccctccaggatgtccgtggcagagactaccagaatgctatgcgggtgtggagcaacattccagggctgaagagcaagcatgcgcccctgaccccaaaggaagaagagtatctgcaagcccaagtcagaagcaggagcaagctggacgccccgaaagttgacctcctggtgaagaactgccttctcccgctgagagagtacttcaagtatttttctcaaaactcacttcctcttggagggccgagctctggcgcacccccaccaagtggagggtctcctgccgggtccccaacatctactgaagaaggcaccagcgaatccgcaacgcccgagtcaggccctggtacctccacagaaccatctgaaggtagtgcgcctggttccccagctggaagccctacttccaccgaagaaggcacgtcaaccgaaccaagtgaaggatctgcccctgggaccagcactgaaccatctgagggccccgacatcgtgatgacccagagccccagcagcctgagcgccagcgtgggcgaccgcgtgaccatcacctgccgcagcagcaccggcgccgtgaccaccagcaactacgccagctgggtgcaggagaagcccggcaagctgttcaagggcctgatcggcggcaccaacaaccgcgcccccggcgtgcccagccgcttcagcggcagcctgatcggcgacaaggccaccctgaccatcagcagcctgcagcccgaggacttcgccacctacttctgcgccctgtggtacagcaaccactgggtgttcggccagggcaccaaggtggagctgaagcgcggcggcggcggcagcggcggcggcggcagcggcggcggcggcagcagcggcggcggcagcgaggtgaagctgctggagagcggcggcggcctggtgcagcccggcggcagcctgaagctgagctgcgccgtgagcggcttcagcctgaccgactacggcgtgaactgggtgcgccaggcccccggccgcggcctggagtggatcggcgtgatctggggcgacggcatcaccgactacaacagcgccctgaaggaccgcttcatcatcagcaaggacaacggcaagaacaccgtgtacctgcagatgagcaaggtgcgcagcgacgacaccgccctgtactactgcgtgaccggcctgttcgactactggggccagggcaccctggtgaccgtgagcagctacccatacgatgttccagattacgctggtggaggcggaggttctgggggaggaggtagtggcggtggtggttcaggaggcggcggaagcggaagcggagctactaacttcagcctgctgaagcaggctggagacgtggaggagaaccctggacctatgcctgctgctaagagagtgaaactggatggatccgaggaactgctgagcaagaactaccacctggaaaacgaggtggccagactgaagaaaggctctggctctggcggaagcggttctggcggatcaggatctggaagtggcggctctggaagcggaggttctggatctggcgaagaactgctgtctaagaattatcacctcgagaatgaggtcgcccgcctgaaaaaaggatcaggttccggtggttctggcagcggtggttcaggctcaggcagcggcggtagcggtagcggtggaagcggaagcggaccaaaaaagaagagaaaggtaatggacaagaagtacagcatcggcctggccatcggcaccaactctgtgggctgggccgtgatcaccgacgagtacaaggtgcccagcaagaaattcaaggtgctgggcaacaccgaccggcacagcatcaagaagaacctgatcggcgccctgctgttcgacagcggagaaacagccgaggccacccggctgaagagaaccgccagaagaagatacaccagacggaagaaccggatctgctatctgcaagagatcttcagcaacgagatggccaaggtggacgacagcttcttccacagactggaagagtccttcctggtggaagaggataagaagcacgagcggcaccccatcttcggcaacatcgtggacgaggtggcctaccacgagaagtaccccaccatctaccacctgagaaagaaactggtggacagcaccgacaaggccgacctgcggctgatctatctggccctggcccacatgatcaagttccggggccacttcctgatcgagggcgacctgaaccccgacaacagcgacgtggacaagctgttcatccagctggtgcagacctacaaccagctgttcgaggaaaaccccatcaacgccagcggcgtggacgccaaggccatcctgtctgccagactgagcaagagcagacggctggaaaatctgatcgcccagctgcccggcgagaagaagaatggcctgttcggcaacctgattgccctgagcctgggcctgacccccaacttcaagagcaacttcgacctggccgaggatgccaaactgcagctgagcaaggacacctacgacgacgacctggacaacctgctggcccagatcggcgaccagtacgccgacctgtttctggccgccaagaacctgtccgacgccatcctgctgagcgacatcctgagagtgaacaccgagatcaccaaggcccccctgagcgcctctatgatcaagagatacgacgagcaccaccaggacctgaccctgctgaaagctctcgtgcggcagcagctgcctgagaagtacaaagagattttcttcgaccagagcaagaacggctacgccggctacatcgatggcggagccagccaggaagagttctacaagttcatcaagcccatcctggaaaagatggacggcaccgaggaactgctcgtgaagctgaacagagaggacctgctgcggaagcagcggaccttcgacaacggcagcatcccccaccagatccacctgggagagctgcacgccattctgcggcggcaggaagatttttacccattcctgaaggacaaccgggaaaagatcgagaagatcctgaccttccgcatcccctactacgtgggccctctggccaggggaaacagcagattcgcctggatgaccagaaagagcgaggaaaccatcaccccctggaacttcgaggaagtggtggacaagggcgccagcgcccagagcttcatcgagcggatgaccaacttcgataagaacctgcccaacgagaaggtgctgcccaagcacagcctgctgtacgagtacttcaccgtgtacaacgagctgaccaaagtgaaatacgtgaccgagggaatgagaaagcccgccttcctgagcggcgagcagaaaaaagccatcgtggacctgctgttcaagaccaaccggaaagtgaccgtgaagcagctgaaagaggactacttcaagaaaatcgagtgcttcgactccgtggaaatctccggcgtggaagatcggttcaacgcctccctgggcacataccacgatctgctgaaaattatcaaggacaaggacttcctggacaatgaggaaaacgaggacattctggaagatatcgtgctgaccctgacactgtttgaggacagagagatgatcgaggaacggctgaaaacctatgcccacctgttcgacgacaaagtgatgaagcagctgaagcggcggagatacaccggctggggcaggctgagccggaagctgatcaacggcatccgggacaagcagtccggcaagacaatcctggatttcctgaagtccgacggcttcgccaacagaaacttcatgcagctgatccacgacgacagcctgacctttaaagaggacatccagaaagcccaggtgtccggccagggcgatagcctgcacgagcacattgccaatctggccggcagccccgccattaagaagggcatcctgcagacagtgaaggtggtggacgagctcgtgaaagtgatgggccggcacaagcccgagaacatcgtgatcgaaatggccagagagaaccagaccacccagaagggacagaagaacagccgcgagagaatgaagcggatcgaagagggcatcaaagagctgggcagccagatcctgaaagaacaccccgtggaaaacacccagctgcagaacgagaagctgtacctgtactacctgcagaatgggcgggatatgtacgtggaccaggaactggacatcaaccggctgtccgactacgatgtggacgctatcgtgcctcagagctttctgaaggacgactccatcgataacaaagtgctgactcggagcgacaagaaccggggcaagagcgacaacgtgccctccgaagaggtcgtgaagaagatgaagaactactggcgccagctgctgaatgccaagctgattacccagaggaagttcgacaatctgaccaaggccgagagaggcggcctgagcgaactggataaggccggcttcatcaagagacagctggtggaaacccggcagatcacaaagcacgtggcacagatcctggactcccggatgaacactaagtacgacgagaacgacaaactgatccgggaagtgaaagtgatcaccctgaagtccaagctggtgtccgatttccggaaggatttccagttttacaaagtgcgcgagatcaacaactaccaccacgcccacgacgcctacctgaacgccgtcgtgggaaccgccctgatcaaaaagtaccctaagctggaaagcgagttcgtgtacggcgactacaaggtgtacgacgtgcggaagatgatcgccaagagcgagcaggaaatcggcaaggctaccgccaagtacttcttctacagcaacatcatgaactttttcaagaccgagattaccctggccaacggcgagatccggaagcggcctctgatcgagacaaacggcgaaacaggcgagatcgtgtgggataagggccgggactttgccaccgtgcggaaagtgctgtctatgccccaagtgaatatcgtgaaaaagaccgaggtgcagacaggcggcttcagcaaagagtctatcctgcccaagaggaacagcgacaagctgatcgccagaaagaaggactgggaccctaagaagtacggcggcttcgacagccccaccgtggcctattctgtgctggtggtggccaaagtggaaaagggcaagtccaagaaactgaagagtgtgaaagagctgctggggatcaccatcatggaaagaagcagcttcgagaagaatcccatcgactttctggaagccaagggctacaaagaagtgaaaaaggacctgatcatcaagctgcctaagtactccctgttcgagctggaaaacggccggaagagaatgctggcctctgccggcgaactgcagaagggaaacgaactggccctgccctccaaatatgtgaacttcctgtacctggccagccactatgagaagctgaagggctcccccgaggataatgagcagaaacagctgtttgtggaacagcacaaacactacctggacgagatcatcgagcagatcagcgagttctccaagagagtgatcctggccgacgctaatctggacaaggtgctgagcgcctacaacaagcacagagacaagcctatcagagagcaggccgagaatatcatccacctgtttaccctgaccaatctgggagcccctgccgccttcaagtactttgacaccaccatcgaccggaagaggtacaccagcaccaaagaggtgctggacgccaccctgatccaccagagcatcaccggcctgtacgagacacggatcgacctgtctcagctgggaggcgacgcctatccctatgacgtgcccgattatgccagcctgggcagcggctcccccaagaaaaaacgcaaggtggaagatcctaagaaaaagcggaaagtggacggcagcggcagcgagacccccggtaccagcgagagcgccacccccgagagccggacactggtgaccttcaaggatgtatttgtggacttcaccagggaggagtggaagctgctggacactgctcagcagatcgtgtacagaaatgtgatgctggagaactataagaacctggtttccttgggttatcagcttactaagccagatgtgatcctccggttggagaagggagaagagccctgagatcccaagcacgcagcaatgcagctcaaaacgcttagcctagccacacccccacgggaaacagcagtgattaacctttagcaataaacgaaagtttaactaagctatactaaccccagggttggtcaatttcgtgccagccacaccctggtactgcatgcacgcaatgctagctgcccctttcccgtcctgggcaccccgagtctcccccgaccccgggtcccaggtatgctcccacctccacctgccccactcaccacctctgctagttccagacacctccgagacgaggaaaaaaaaaaaaaaaaaaaaaaaaaaaaaaaaaaaaaaaaaaaaaaaaaaaaaaaaaaaaaaaaaaaaaaaaaaaaaaaaaaaaaaaaaaaaaaaaaaaaaaaaaaaaaaaaaaaaaaaa

SEQ ID NO: 265 - RNA, 8224 nt, synthetic construct
  misc_feature 1..8224: note = mRNA of V24_D3a-D3l-scFv-2a-3xGCN4-dCas9-KRAB
  source 1..8224: mol_type = other RNA
aggactcactatttgttttcgcgcccagttgcaaaaagtgtcgacatttgcttctgacacaactgtgttcactagcaacctcaaacagacaccgccaccatgcctgctgctaagagagtgaaactggatggatccaaccatgaccaggaatttgaccccccaaaggtttacccacctgtgccagctgagaagaggaagcccatccgcgtgctgtctctctttgatgggattgctacagggctcctggtgctgaaggacctgggcatccaagtggaccgctacattgcctccgaggtgtgtgaggactccatcacggtgggcatggtgcggcaccagggaaagatcatgtacgtcggggacgtccgcagcgtcacacagaagcatatccaggagtggggcccattcgacctggtgattggaggcagtccctgcaatgacctctccattgtcaaccctgcccgcaagggactttatgagggtactggccgcctcttctttgagttctaccgcctcctgcatgatgcgcggcccaaggagggagatgatcgccccttcttctggctctttgagaatgtggtggccatgggcgttagtgacaagagggacatctcgcgatttcttgagtctaaccccgtgatgattgacgccaaagaagtgtctgctgcacacagggcccgttacttctggggtaaccttcctggcatgaacaggcctttggcatccactgtgaatgataagctggagctgcaagagtgtctggagcacggcagaatagccaagttcagcaaagtgaggaccattaccaccaggtcaaactctataaagcagggcaaagaccagcatttccccgtgttcatgaacgagaaggaggacatcctgtggtgcactgaaatggaaagggtgtttggcttccccgtccactacacagacgtctccaacatgagccgcttggcgaggcagagactgctgggccgatcgtggagcgtgccggtcatccgccacctcttcgctccgctgaaggaatattttgcttgtgtgtctagcggcaatagtaacgctaacagccgcgggccgagcttcagcagcggcctggtgccgttaagcttgcgcggcagccatatgggccctatggagatatacaagacagtgtctgcatggaagagacagccagtgcgggtactgagcctcttcagaaacatcgacaaggtactaaagagtttgggcttcttggaaagcggttctggttctgggggaggaacgctgaagtacgtggaagatgtcacaaatgtcgtgaggagagacgtggagaaatggggcccctttgacctggtgtacggctcgacgcagcccctaggcagctcttgtgatcgctgtcccggctggtacatgttccagttccaccggatcctgcagtatgcgctgcctcgccaggagagtcagcggcccttcttctggatattcatggacaatctgctgctgactgaggatgaccaagagacaactacccgcttccttcagacagaggctgtgaccctccaggatgtccgtggcagagactaccagaatgctatgcgggtgtggagcaacattccagggctgaagagcaagcatgcgcccctgaccccaaaggaagaagagtatctgcaagcccaagtcagaagcaggagcaagctggacgccccgaaagttgacctcctggtgaagaactgccttctcccgctgagagagtacttcaagtatttttctcaaaactcacttcctcttggagggccgagctctggcgcacccccaccaagtggagggtctcctgccgggtccccaacatctactgaagaaggcaccagcgaatccgcaacgcccgagtcaggccctggtacctccacagaaccatctgaaggtagtgcgcctggttccccagctggaagccctacttccaccgaagaaggcacgtcaaccgaaccaagtgaaggatctgcccctgggaccagcactgaaccatctgagggccccgacatcgtgatgacccagagccccagcagcctgagcgccagcgtgggcgaccgcgtgaccatcacctgccgcagcagcaccggcgccgtgaccaccagcaactacgccagctgggtgcaggagaagcccggcaagctgttcaagggcctgatcggcggcaccaacaaccgcgcccccggcgtgcccagccgcttcagcggcagcctgatcggcgacaaggccaccctgaccatcagcagcctgcagcccgaggacttcgccacctacttctgcgccctgtggtacagcaaccactgggtgttcggccagggcaccaaggtggagctgaagcgcggcggcggcggcagcggcggcggcggcagcggcggcggcggcagcagcggcggcggcagcgaggtgaagctgctggagagcggcggcggcctggtgcagcccggcggcagcctgaagctgagctgcgccgtgagcggcttcagcctgaccgactacggcgtgaactgggtgcgccaggcccccggccgcggcctggagtggatcggcgtgatctggggcgacggcatcaccgactacaacagcgccctgaaggaccgcttcatcatcagcaaggacaacggcaagaacaccgtgtacctgcagatgagcaaggtgcgcagcgacgacaccgccctgtactactgcgtgaccggcctgttcgactactggggccagggcaccctggtgaccgtgagcagctacccatacgatgttccagattacgctggtggaggcggaggttctgggggaggaggtagtggcggtggtggttcaggaggcggcggaagcggaagcggagctactaacttcagcctgctgaagcaggctggagacgtggaggagaaccctggacctatgcctgctgctaagagagtgaaactggatggatccgaggaactgctgagcaagaactaccacctggaaaacgaggtggccagactgaagaaaggctctggctctggcggaagcggttctggcggatcaggatctggaagtggcggctctggaagcggaggttctggatctggcgaagaactgctgtctaagaattatcacctcgagaacgaagtggctcggctcaagaaaggcagtggcagcggaggaagtggatccggcggtagtggtagtggaagcggcggatccggctcaggcggatctggttcaggggaagaactcctctccaaaaactaccatctcgagaatgaggtcgcccgcctgaaaaaaggatcaggttccggtggttctggcagcggtggttcaggctcaggcagcggcggtagcggtagcggtggaagcggaagcggaccaaaaaagaagagaaaggtaatggacaagaagtacagcatcggcctggccatcggcaccaactctgtgggctgggccgtgatcaccgacgagtacaaggtgcccagcaagaaattcaaggtgctgggcaacaccgaccggcacagcatcaagaagaacctgatcggcgccctgctgttcgacagcggagaaacagccgaggccacccggctgaagagaaccgccagaagaagatacaccagacggaagaaccggatctgctatctgcaagagatcttcagcaacgagatggccaaggtggacgacagcttcttccacagactggaagagtccttcctggtggaagaggataagaagcacgagcggcaccccatcttcggcaacatcgtggacgaggtggcctaccacgagaagtaccccaccatctaccacctgagaaagaaactggtggacagcaccgacaaggccgacctgcggctgatctatctggccctggcccacatgatcaagttccggggccacttcctgatcgagggcgacctgaaccccgacaacagcgacgtggacaagctgttcatccagctggtgcagacctacaaccagctgttcgaggaaaaccccatcaacgccagcggcgtggacgccaaggccatcctgtctgccagactgagcaagagcagacggctggaaaatctgatcgcccagctgcccggcgagaagaagaatggcctgttcggcaacctgattgccctgagcctgggcctgacccccaacttcaagagcaacttcgacctggccgaggatgccaaactgcagctgagcaaggacacctacgacgacgacctggacaacctgctggcccagatcggcgaccagtacgccgacctgtttctggccgccaagaacctgtccgacgccatcctgctgagcgacatcctgagagtgaacaccgagatcaccaaggcccccctgagcgcctctatgatcaagagatacgacgagcaccaccaggacctgaccctgctgaaagctctcgtgcggcagcagctgcctgagaagtacaaagagattttcttcgaccagagcaagaacggctacgccggctacatcgatggcggagccagccaggaagagttctacaagttcatcaagcccatcctggaaaagatggacggcaccgaggaactgctcgtgaagctgaacagagaggacctgctgcggaagcagcggaccttcgacaacggcagcatcccccaccagatccacctgggagagctgcacgccattctgcggcggcaggaagatttttacccattcctgaaggacaaccgggaaaagatcgagaagatcctgaccttccgcatcccctactacgtgggccctctggccaggggaaacagcagattcgcctggatgaccagaaagagcgaggaaaccatcaccccctggaacttcgaggaagtggtggacaagggcgccagcgcccagagcttcatcgagcggatgaccaacttcgataagaacctgcccaacgagaaggtgctgcccaagcacagcctgctgtacgagtacttcaccgtgtacaacgagctgaccaaagtgaaatacgtgaccgagggaatgagaaagcccgccttcctgagcggcgagcagaaaaaagccatcgtggacctgctgttcaagaccaaccggaaagtgaccgtgaagcagctgaaagaggactacttcaagaaaatcgagtgcttcgactccgtggaaatctccggcgtggaagatcggttcaacgcctccctgggcacataccacgatctgctgaaaattatcaaggacaaggacttcctggacaatgaggaaaacgaggacattctggaagatatcgtgctgaccctgacactgtttgaggacagagagatgatcgaggaacggctgaaaacctatgcccacctgttcgacgacaaagtgatgaagcagctgaagcggcggagatacaccggctggggcaggctgagccggaagctgatcaacggcatccgggacaagcagtccggcaagacaatcctggatttcctgaagtccgacggcttcgccaacagaaacttcatgcagctgatccacgacgacagcctgacctttaaagaggacatccagaaagcccaggtgtccggccagggcgatagcctgcacgagcacattgccaatctggccggcagccccgccattaagaagggcatcctgcagacagtgaaggtggtggacgagctcgtgaaagtgatgggccggcacaagcccgagaacatcgtgatcgaaatggccagagagaaccagaccacccagaagggacagaagaacagccgcgagagaatgaagcggatcgaagagggcatcaaagagctgggcagccagatcctgaaagaacaccccgtggaaaacacccagctgcagaacgagaagctgtacctgtactacctgcagaatgggcgggatatgtacgtggaccaggaactggacatcaaccggctgtccgactacgatgtggacgctatcgtgcctcagagctttctgaaggacgactccatcgataacaaagtgctgactcggagcgacaagaaccggggcaagagcgacaacgtgccctccgaagaggtcgtgaagaagatgaagaactactggcgccagctgctgaatgccaagctgattacccagaggaagttcgacaatctgaccaaggccgagagaggcggcctgagcgaactggataaggccggcttcatcaagagacagctggtggaaacccggcagatcacaaagcacgtggcacagatcctggactcccggatgaacactaagtacgacgagaacgacaaactgatccgggaagtgaaagtgatcaccctgaagtccaagctggtgtccgatttccggaaggatttccagttttacaaagtgcgcgagatcaacaactaccaccacgcccacgacgcctacctgaacgccgtcgtgggaaccgccctgatcaaaaagtaccctaagctggaaagcgagttcgtgtacggcgactacaaggtgtacgacgtgcggaagatgatcgccaagagcgagcaggaaatcggcaaggctaccgccaagtacttcttctacagcaacatcatgaactttttcaagaccgagattaccctggccaacggcgagatccggaagcggcctctgatcgagacaaacggcgaaacaggcgagatcgtgtgggataagggccgggactttgccaccgtgcggaaagtgctgtctatgccccaagtgaatatcgtgaaaaagaccgaggtgcagacaggcggcttcagcaaagagtctatcctgcccaagaggaacagcgacaagctgatcgccagaaagaaggactgggaccctaagaagtacggcggcttcgacagccccaccgtggcctattctgtgctggtggtggccaaagtggaaaagggcaagtccaagaaactgaagagtgtgaaagagctgctggggatcaccatcatggaaagaagcagcttcgagaagaatcccatcgactttctggaagccaagggctacaaagaagtgaaaaaggacctgatcatcaagctgcctaagtactccctgttcgagctggaaaacggccggaagagaatgctggcctctgccggcgaactgcagaagggaaacgaactggccctgccctccaaatatgtgaacttcctgtacctggccagccactatgagaagctgaagggctcccccgaggataatgagcagaaacagctgtttgtggaacagcacaaacactacctggacgagatcatcgagcagatcagcgagttctccaagagagtgatcctggccgacgctaatctggacaaggtgctgagcgcctacaacaagcacagagacaagcctatcagagagcaggccgagaatatcatccacctgtttaccctgaccaatctgggagcccctgccgccttcaagtactttgacaccaccatcgaccggaagaggtacaccagcaccaaagaggtgctggacgccaccctgatccaccagagcatcaccggcctgtacgagacacggatcgacctgtctcagctgggaggcgacgcctatccctatgacgtgcccgattatgccagcctgggcagcggctcccccaagaaaaaacgcaaggtggaagatcctaagaaaaagcggaaagtggacggcagcggcagcgagacccccggtaccagcgagagcgccacccccgagagccggacactggtgaccttcaaggatgtatttgtggacttcaccagggaggagtggaagctgctggacactgctcagcagatcgtgtacagaaatgtgatgctggagaactataagaacctggtttccttgggttatcagcttactaagccagatgtgatcctccggttggagaagggagaagagccctgagatcccaagcacgcagcaatgcagctcaaaacgcttagcctagccacacccccacgggaaacagcagtgattaacctttagcaataaacgaaagtttaactaagctatactaaccccagggttggtcaatttcgtgccagccacaccctggtactgcatgcacgcaatgctagctgcccctttcccgtcctgggcaccccgagtctcccccgaccccgggtcccaggtatgctcccacctccacctgccccactcaccacctctgctagttccagacacctccgagacgaggaaaaaaaaaaaaaaaaaaaaaaaaaaaaaaaaaaaaaaaaaaaaaaaaaaaaaaaaaaaaaaaaaaaaaaaaaaaaaaaaaaaaaaaaaaaaaaaaaaaaaaaaaaaaaaaaaaaaaaaa

SEQ ID NO: 266 - RNA, 8500 nt, synthetic construct
  misc_feature 1..8500: note = mRNA of V25_D3a-D3l-scFv-2a-5xGCN4-dCas9-KRAB
  source 1..8500: mol_type = other RNA
aggactcactatttgttttcgcgcccagttgcaaaaagtgtcgacatttgcttctgacacaactgtgttcactagcaacctcaaacagacaccgccaccatgcctgctgctaagagagtgaaactggatggatccaaccatgaccaggaatttgaccccccaaaggtttacccacctgtgccagctgagaagaggaagcccatccgcgtgctgtctctctttgatgggattgctacagggctcctggtgctgaaggacctgggcatccaagtggaccgctacattgcctccgaggtgtgtgaggactccatcacggtgggcatggtgcggcaccagggaaagatcatgtacgtcggggacgtccgcagcgtcacacagaagcatatccaggagtggggcccattcgacctggtgattggaggcagtccctgcaatgacctctccattgtcaaccctgcccgcaagggactttatgagggtactggccgcctcttctttgagttctaccgcctcctgcatgatgcgcggcccaaggagggagatgatcgccccttcttctggctctttgagaatgtggtggccatgggcgttagtgacaagagggacatctcgcgatttcttgagtctaaccccgtgatgattgacgccaaagaagtgtctgctgcacacagggcccgttacttctggggtaaccttcctggcatgaacaggcctttggcatccactgtgaatgataagctggagctgcaagagtgtctggagcacggcagaatagccaagttcagcaaagtgaggaccattaccaccaggtcaaactctataaagcagggcaaagaccagcatttccccgtgttcatgaacgagaaggaggacatcctgtggtgcactgaaatggaaagggtgtttggcttccccgtccactacacagacgtctccaacatgagccgcttggcgaggcagagactgctgggccgatcgtggagcgtgccggtcatccgccacctcttcgctccgctgaaggaatattttgcttgtgtgtctagcggcaatagtaacgctaacagccgcgggccgagcttcagcagcggcctggtgccgttaagcttgcgcggcagccatatgggccctatggagatatacaagacagtgtctgcatggaagagacagccagtgcgggtactgagcctcttcagaaacatcgacaaggtactaaagagtttgggcttcttggaaagcggttctggttctgggggaggaacgctgaagtacgtggaagatgtcacaaatgtcgtgaggagagacgtggagaaatggggcccctttgacctggtgtacggctcgacgcagcccctaggcagctcttgtgatcgctgtcccggctggtacatgttccagttccaccggatcctgcagtatgcgctgcctcgccaggagagtcagcggcccttcttctggatattcatggacaatctgctgctgactgaggatgaccaagagacaactacccgcttccttcagacagaggctgtgaccctccaggatgtccgtggcagagactaccagaatgctatgcgggtgtggagcaacattccagggctgaagagcaagcatgcgcccctgaccccaaaggaagaagagtatctgcaagcccaagtcagaagcaggagcaagctggacgccccgaaagttgacctcctggtgaagaactgccttctcccgctgagagagtacttcaagtatttttctcaaaactcacttcctcttggagggccgagctctggcgcacccccaccaagtggagggtctcctgccgggtccccaacatctactgaagaaggcaccagcgaatccgcaacgcccgagtcaggccctggtacctccacagaaccatctgaaggtagtgcgcctggttccccagctggaagccctacttccaccgaagaaggcacgtcaaccgaaccaagtgaaggatctgcccctgggaccagcactgaaccatctgagggccccgacatcgtgatgacccagagccccagcagcctgagcgccagcgtgggcgaccgcgtgaccatcacctgccgcagcagcaccggcgccgtgaccaccagcaactacgccagctgggtgcaggagaagcccggcaagctgttcaagggcctgatcggcggcaccaacaaccgcgcccccggcgtgcccagccgcttcagcggcagcctgatcggcgacaaggccaccctgaccatcagcagcctgcagcccgaggacttcgccacctacttctgcgccctgtggtacagcaaccactgggtgttcggccagggcaccaaggtggagctgaagcgcggcggcggcggcagcggcggcggcggcagcggcggcggcggcagcagcggcggcggcagcgaggtgaagctgctggagagcggcggcggcctggtgcagcccggcggcagcctgaagctgagctgcgccgtgagcggcttcagcctgaccgactacggcgtgaactgggtgcgccaggcccccggccgcggcctggagtggatcggcgtgatctggggcgacggcatcaccgactacaacagcgccctgaaggaccgcttcatcatcagcaaggacaacggcaagaacaccgtgtacctgcagatgagcaaggtgcgcagcgacgacaccgccctgtactactgcgtgaccggcctgttcgactactggggccagggcaccctggtgaccgtgagcagctacccatacgatgttccagattacgctggtggaggcggaggttctgggggaggaggtagtggcggtggtggttcaggaggcggcggaagcggaagcggagctactaacttcagcctgctgaagcaggctggagacgtggaggagaaccctggacctatgcctgctgctaagagagtgaaactggatggatccgaggaactgctgagcaagaactaccacctggaaaacgaggtggccagactgaagaaaggctctggctctggcggaagcggttctggcggatcaggatctggaagtggcggctctggaagcggaggttctggatctggcgaagaactgctgtctaagaattatcacctcgagaacgaggttgcacgcttgaagaaaggcagcggatcaggcggatctggcagcggtggatctggttctggatccggcggctccggtagtggtggaagtggctctggggaagaattgcttagcaagaattatcatcttgaaaatgaggttgccaggcttaaaaaaggcagtggctccggcggatccggaagcggaggcagcggatctggatctggtggttcaggatctggcggttctggtagcggggaagaactgttgagtaaaaactatcaccttgagaacgaggtcgcaaggttgaaaaaaggatccggctctggcggctccggaagtggcggatctggctccggtagcggaggatcaggatccggcggaagcggatcaggcgaggaactgctttccaaaaattaccacctcgagaatgaggtcgcccgcctgaaaaaaggatcaggttccggtggttctggcagcggtggttcaggctcaggcagcggcggtagcggtagcggtggaagcggaagcggaccaaaaaagaagagaaaggtaatggacaagaagtacagcatcggcctggccatcggcaccaactctgtgggctgggccgtgatcaccgacgagtacaaggtgcccagcaagaaattcaaggtgctgggcaacaccgaccggcacagcatcaagaagaacctgatcggcgccctgctgttcgacagcggagaaacagccgaggccacccggctgaagagaaccgccagaagaagatacaccagacggaagaaccggatctgctatctgcaagagatcttcagcaacgagatggccaaggtggacgacagcttcttccacagactggaagagtccttcctggtggaagaggataagaagcacgagcggcaccccatcttcggcaacatcgtggacgaggtggcctaccacgagaagtaccccaccatctaccacctgagaaagaaactggtggacagcaccgacaaggccgacctgcggctgatctatctggccctggcccacatgatcaagttccggggccacttcctgatcgagggcgacctgaaccccgacaacagcgacgtggacaagctgttcatccagctggtgcagacctacaaccagctgttcgaggaaaaccccatcaacgccagcggcgtggacgccaaggccatcctgtctgccagactgagcaagagcagacggctggaaaatctgatcgcccagctgcccggcgagaagaagaatggcctgttcggcaacctgattgccctgagcctgggcctgacccccaacttcaagagcaacttcgacctggccgaggatgccaaactgcagctgagcaaggacacctacgacgacgacctggacaacctgctggcccagatcggcgaccagtacgccgacctgtttctggccgccaagaacctgtccgacgccatcctgctgagcgacatcctgagagtgaacaccgagatcaccaaggcccccctgagcgcctctatgatcaagagatacgacgagcaccaccaggacctgaccctgctgaaagctctcgtgcggcagcagctgcctgagaagtacaaagagattttcttcgaccagagcaagaacggctacgccggctacatcgatggcggagccagccaggaagagttctacaagttcatcaagcccatcctggaaaagatggacggcaccgaggaactgctcgtgaagctgaacagagaggacctgctgcggaagcagcggaccttcgacaacggcagcatcccccaccagatccacctgggagagctgcacgccattctgcggcggcaggaagatttttacccattcctgaaggacaaccgggaaaagatcgagaagatcctgaccttccgcatcccctactacgtgggccctctggccaggggaaacagcagattcgcctggatgaccagaaagagcgaggaaaccatcaccccctggaacttcgaggaagtggtggacaagggcgccagcgcccagagcttcatcgagcggatgaccaacttcgataagaacctgcccaacgagaaggtgctgcccaagcacagcctgctgtacgagtacttcaccgtgtacaacgagctgaccaaagtgaaatacgtgaccgagggaatgagaaagcccgccttcctgagcggcgagcagaaaaaagccatcgtggacctgctgttcaagaccaaccggaaagtgaccgtgaagcagctgaaagaggactacttcaagaaaatcgagtgcttcgactccgtggaaatctccggcgtggaagatcggttcaacgcctccctgggcacataccacgatctgctgaaaattatcaaggacaaggacttcctggacaatgaggaaaacgaggacattctggaagatatcgtgctgaccctgacactgtttgaggacagagagatgatcgaggaacggctgaaaacctatgcccacctgttcgacgacaaagtgatgaagcagctgaagcggcggagatacaccggctggggcaggctgagccggaagctgatcaacggcatccgggacaagcagtccggcaagacaatcctggatttcctgaagtccgacggcttcgccaacagaaacttcatgcagctgatccacgacgacagcctgacctttaaagaggacatccagaaagcccaggtgtccggccagggcgatagcctgcacgagcacattgccaatctggccggcagccccgccattaagaagggcatcctgcagacagtgaaggtggtggacgagctcgtgaaagtgatgggccggcacaagcccgagaacatcgtgatcgaaatggccagagagaaccagaccacccagaagggacagaagaacagccgcgagagaatgaagcggatcgaagagggcatcaaagagctgggcagccagatcctgaaagaacaccccgtggaaaacacccagctgcagaacgagaagctgtacctgtactacctgcagaatgggcgggatatgtacgtggaccaggaactggacatcaaccggctgtccgactacgatgtggacgctatcgtgcctcagagctttctgaaggacgactccatcgataacaaagtgctgactcggagcgacaagaaccggggcaagagcgacaacgtgccctccgaagaggtcgtgaagaagatgaagaactactggcgccagctgctgaatgccaagctgattacccagaggaagttcgacaatctgaccaaggccgagagaggcggcctgagcgaactggataaggccggcttcatcaagagacagctggtggaaacccggcagatcacaaagcacgtggcacagatcctggactcccggatgaacactaagtacgacgagaacgacaaactgatccgggaagtgaaagtgatcaccctgaagtccaagctggtgtccgatttccggaaggatttccagttttacaaagtgcgcgagatcaacaactaccaccacgcccacgacgcctacctgaacgccgtcgtgggaaccgccctgatcaaaaagtaccctaagctggaaagcgagttcgtgtacggcgactacaaggtgtacgacgtgcggaagatgatcgccaagagcgagcaggaaatcggcaaggctaccgccaagtacttcttctacagcaacatcatgaactttttcaagaccgagattaccctggccaacggcgagatccggaagcggcctctgatcgagacaaacggcgaaacaggcgagatcgtgtgggataagggccgggactttgccaccgtgcggaaagtgctgtctatgccccaagtgaatatcgtgaaaaagaccgaggtgcagacaggcggcttcagcaaagagtctatcctgcccaagaggaacagcgacaagctgatcgccagaaagaaggactgggaccctaagaagtacggcggcttcgacagccccaccgtggcctattctgtgctggtggtggccaaagtggaaaagggcaagtccaagaaactgaagagtgtgaaagagctgctggggatcaccatcatggaaagaagcagcttcgagaagaatcccatcgactttctggaagccaagggctacaaagaagtgaaaaaggacctgatcatcaagctgcctaagtactccctgttcgagctggaaaacggccggaagagaatgctggcctctgccggcgaactgcagaagggaaacgaactggccctgccctccaaatatgtgaacttcctgtacctggccagccactatgagaagctgaagggctcccccgaggataatgagcagaaacagctgtttgtggaacagcacaaacactacctggacgagatcatcgagcagatcagcgagttctccaagagagtgatcctggccgacgctaatctggacaaggtgctgagcgcctacaacaagcacagagacaagcctatcagagagcaggccgagaatatcatccacctgtttaccctgaccaatctgggagcccctgccgccttcaagtactttgacaccaccatcgaccggaagaggtacaccagcaccaaagaggtgctggacgccaccctgatccaccagagcatcaccggcctgtacgagacacggatcgacctgtctcagctgggaggcgacgcctatccctatgacgtgcccgattatgccagcctgggcagcggctcccccaagaaaaaacgcaaggtggaagatcctaagaaaaagcggaaagtggacggcagcggcagcgagacccccggtaccagcgagagcgccacccccgagagccggacactggtgaccttcaaggatgtatttgtggacttcaccagggaggagtggaagctgctggacactgctcagcagatcgtgtacagaaatgtgatgctggagaactataagaacctggtttccttgggttatcagcttactaagccagatgtgatcctccggttggagaagggagaagagccctgagatcccaagcacgcagcaatgcagctcaaaacgcttagcctagccacacccccacgggaaacagcagtgattaacctttagcaataaacgaaagtttaactaagctatactaaccccagggttggtcaatttcgtgccagccacaccctggtactgcatgcacgcaatgctagctgcccctttcccgtcctgggcaccccgagtctcccccgaccccgggtcccaggtatgctcccacctccacctgccccactcaccacctctgctagttccagacacctccgagacgaggaaaaaaaaaaaaaaaaaaaaaaaaaaaaaaaaaaaaaaaaaaaaaaaaaaaaaaaaaaaaaaaaaaaaaaaaaaaaaaaaaaaaaaaaaaaaaaaaaaaaaaaaaaaaaaaaaaaaaaaa

SEQ ID NO: 267 - RNA, 8345 nt, synthetic construct
  misc_feature 1..8345: note = mRNA of V26_D3a-hD3L-scFv-2a-3xGCN4-dCas9-ZIM3
  source 1..8345: mol_type = other RNA
aggactcactatttgttttcgcgcccagttgcaaaaagtgtcgacatttgcttctgacacaactgtgttcactagcaacctcaaacagacaccgccaccatgcctgctgctaagagagtgaaactggatggatccaaccatgaccaggaatttgaccccccaaaggtttacccacctgtgccagctgagaagaggaagcccatccgcgtgctgtctctctttgatgggattgctacagggctcctggtgctgaaggacctgggcatccaagtggaccgctacattgcctccgaggtgtgtgaggactccatcacggtgggcatggtgcggcaccagggaaagatcatgtacgtcggggacgtccgcagcgtcacacagaagcatatccaggagtggggcccattcgacctggtgattggaggcagtccctgcaatgacctctccattgtcaaccctgcccgcaagggactttatgagggtactggccgcctcttctttgagttctaccgcctcctgcatgatgcgcggcccaaggagggagatgatcgccccttcttctggctctttgagaatgtggtggccatgggcgttagtgacaagagggacatctcgcgatttcttgagtctaaccccgtgatgattgacgccaaagaagtgtctgctgcacacagggcccgttacttctggggtaaccttcctggcatgaacaggcctttggcatccactgtgaatgataagctggagctgcaagagtgtctggagcacggcagaatagccaagttcagcaaagtgaggaccattaccaccaggtcaaactctataaagcagggcaaagaccagcatttccccgtgttcatgaacgagaaggaggacatcctgtggtgcactgaaatggaaagggtgtttggcttccccgtccactacacagacgtctccaacatgagccgcttggcgaggcagagactgctgggccgatcgtggagcgtgccggtcatccgccacctcttcgctccgctgaaggaatattttgcttgtgtgtctagcggcaatagtaacgctaacagccgcgggccgagcttcagcagcggcctggtgccgttaagcttgcgcggcagccatatgttcgaaaccgtgcctgtgtggaggagacagccagtccgggtgctgtccctttttgaagacatcaagaaagagctgacgagtttgggctttttggaaagtggttctgacccgggacaactgaagcatgtggttgatgtcacagacacagtgaggaaggatgtggaggagtggggacccttcgatcttgtgtacggcgccacacctcccctgggccacacctgtgaccgtcctcccagctggtacctgttccagttccaccggctcctgcagtacgcacggcccaagccaggcagccccaggcccttcttctggatgttcgtggacaatctggtgctgaacaaggaagacctggacgtcgcatctcgcttcctggagatggagccagtcaccatcccagatgtccacggcggatccttgcagaatgctgtccgcgtgtggagcaacatcccagccataaggagcagcaggcactgggctctggtttcggaagaagaattgtccctgctggcccagaacaagcagagctcgaagctcgcggccaagtggcccaccaagctggtgaagaactgctttctccccctaagagaatatttcaagtatttttcaggagggccgagctctggcgcacccccaccaagtggagggtctcctgccgggtccccaacatctactgaagaaggcaccagcgaatccgcaacgcccgagtcaggccctggtacctccacagaaccatctgaaggtagtgcgcctggttccccagctggaagccctacttccaccgaagaaggcacgtcaaccgaaccaagtgaaggatctgcccctgggaccagcactgaaccatctgagccaaaaaagaagagaaaggtaccatctgagggccccgacatcgtgatgacccagagccccagcagcctgagcgccagcgtgggcgaccgcgtgaccatcacctgccgcagcagcaccggcgccgtgaccaccagcaactacgccagctgggtgcaggagaagcccggcaagctgttcaagggcctgatcggcggcaccaacaaccgcgcccccggcgtgcccagccgcttcagcggcagcctgatcggcgacaaggccaccctgaccatcagcagcctgcagcccgaggacttcgccacctacttctgcgccctgtggtacagcaaccactgggtgttcggccagggcaccaaggtggagctgaagcgcggcggcggcggcagcggcggcggcggcagcggcggcggcggcagcagcggcggcggcagcgaggtgaagctgctggagagcggcggcggcctggtgcagcccggcggcagcctgaagctgagctgcgccgtgagcggcttcagcctgaccgactacggcgtgaactgggtgcgccaggcccccggccgcggcctggagtggatcggcgtgatctggggcgacggcatcaccgactacaacagcgccctgaaggaccgcttcatcatcagcaaggacaacggcaagaacaccgtgtacctgcagatgagcaaggtgcgcagcgacgacaccgccctgtactactgcgtgaccggcctgttcgactactggggccagggcaccctggtgaccgtgagcagctacccatacgatgttccagattacgctggtggaggcggaggttctgggggaggaggtagtggcggtggtggttcaggaggcggcggaagcggaagcggagctactaacttcagcctgctgaagcaggctggagacgtggaggagaaccctggacctatgcctgctgctaagagagtgaaactggatggatccgaggaactgctgagcaagaactaccacctggaaaacgaggtggccagactgaagaaaggctctggctctggcggaagcggttctggcggatcaggatctggaagtggcggctctggaagcggaggttctggatctggcgaagaactgctgtctaagaattatcacctcgagaacgaagtggctcggctcaagaaaggcagtggcagcggaggaagtggatccggcggtagtggtagtggaagcggcggatccggctcaggcggatctggttcaggggaagaactcctctccaaaaactaccatctcgagaatgaggtcgcccgcctgaaaaaaggatcaggttccggtggttctggcagcggtggttcaggctcaggcagcggcggtagcggtagcggtggaagcggaagcggaccaaaaaagaagagaaaggtaatggacaagaagtacagcatcggcctggccatcggcaccaactctgtgggctgggccgtgatcaccgacgagtacaaggtgcccagcaagaaattcaaggtgctgggcaacaccgaccggcacagcatcaagaagaacctgatcggcgccctgctgttcgacagcggagaaacagccgaggccacccggctgaagagaaccgccagaagaagatacaccagacggaagaaccggatctgctatctgcaagagatcttcagcaacgagatggccaaggtggacgacagcttcttccacagactggaagagtccttcctggtggaagaggataagaagcacgagcggcaccccatcttcggcaacatcgtggacgaggtggcctaccacgagaagtaccccaccatctaccacctgagaaagaaactggtggacagcaccgacaaggccgacctgcggctgatctatctggccctggcccacatgatcaagttccggggccacttcctgatcgagggcgacctgaaccccgacaacagcgacgtggacaagctgttcatccagctggtgcagacctacaaccagctgttcgaggaaaaccccatcaacgccagcggcgtggacgccaaggccatcctgtctgccagactgagcaagagcagacggctggaaaatctgatcgcccagctgcccggcgagaagaagaatggcctgttcggcaacctgattgccctgagcctgggcctgacccccaacttcaagagcaacttcgacctggccgaggatgccaaactgcagctgagcaaggacacctacgacgacgacctggacaacctgctggcccagatcggcgaccagtacgccgacctgtttctggccgccaagaacctgtccgacgccatcctgctgagcgacatcctgagagtgaacaccgagatcaccaaggcccccctgagcgcctctatgatcaagagatacgacgagcaccaccaggacctgaccctgctgaaagctctcgtgcggcagcagctgcctgagaagtacaaagagattttcttcgaccagagcaagaacggctacgccggctacatcgatggcggagccagccaggaagagttctacaagttcatcaagcccatcctggaaaagatggacggcaccgaggaactgctcgtgaagctgaacagagaggacctgctgcggaagcagcggaccttcgacaacggcagcatcccccaccagatccacctgggagagctgcacgccattctgcggcggcaggaagatttttacccattcctgaaggacaaccgggaaaagatcgagaagatcctgaccttccgcatcccctactacgtgggccctctggccaggggaaacagcagattcgcctggatgaccagaaagagcgaggaaaccatcaccccctggaacttcgaggaagtggtggacaagggcgccagcgcccagagcttcatcgagcggatgaccaacttcgataagaacctgcccaacgagaaggtgctgcccaagcacagcctgctgtacgagtacttcaccgtgtacaacgagctgaccaaagtgaaatacgtgaccgagggaatgagaaagcccgccttcctgagcggcgagcagaaaaaagccatcgtggacctgctgttcaagaccaaccggaaagtgaccgtgaagcagctgaaagaggactacttcaagaaaatcgagtgcttcgactccgtggaaatctccggcgtggaagatcggttcaacgcctccctgggcacataccacgatctgctgaaaattatcaaggacaaggacttcctggacaatgaggaaaacgaggacattctggaagatatcgtgctgaccctgacactgtttgaggacagagagatgatcgaggaacggctgaaaacctatgcccacctgttcgacgacaaagtgatgaagcagctgaagcggcggagatacaccggctggggcaggctgagccggaagctgatcaacggcatccgggacaagcagtccggcaagacaatcctggatttcctgaagtccgacggcttcgccaacagaaacttcatgcagctgatccacgacgacagcctgacctttaaagaggacatccagaaagcccaggtgtccggccagggcgatagcctgcacgagcacattgccaatctggccggcagccccgccattaagaagggcatcctgcagacagtgaaggtggtggacgagctcgtgaaagtgatgggccggcacaagcccgagaacatcgtgatcgaaatggccagagagaaccagaccacccagaagggacagaagaacagccgcgagagaatgaagcggatcgaagagggcatcaaagagctgggcagccagatcctgaaagaacaccccgtggaaaacacccagctgcagaacgagaagctgtacctgtactacctgcagaatgggcgggatatgtacgtggaccaggaactggacatcaaccggctgtccgactacgatgtggacgctatcgtgcctcagagctttctgaaggacgactccatcgataacaaagtgctgactcggagcgacaagaaccggggcaagagcgacaacgtgccctccgaagaggtcgtgaagaagatgaagaactactggcgccagctgctgaatgccaagctgattacccagaggaagttcgacaatctgaccaaggccgagagaggcggcctgagcgaactggataaggccggcttcatcaagagacagctggtggaaacccggcagatcacaaagcacgtggcacagatcctggactcccggatgaacactaagtacgacgagaacgacaaactgatccgggaagtgaaagtgatcaccctgaagtccaagctggtgtccgatttccggaaggatttccagttttacaaagtgcgcgagatcaacaactaccaccacgcccacgacgcctacctgaacgccgtcgtgggaaccgccctgatcaaaaagtaccctaagctggaaagcgagttcgtgtacggcgactacaaggtgtacgacgtgcggaagatgatcgccaagagcgagcaggaaatcggcaaggctaccgccaagtacttcttctacagcaacatcatgaactttttcaagaccgagattaccctggccaacggcgagatccggaagcggcctctgatcgagacaaacggcgaaacaggcgagatcgtgtgggataagggccgggactttgccaccgtgcggaaagtgctgtctatgccccaagtgaatatcgtgaaaaagaccgaggtgcagacaggcggcttcagcaaagagtctatcctgcccaagaggaacagcgacaagctgatcgccagaaagaaggactgggaccctaagaagtacggcggcttcgacagccccaccgtggcctattctgtgctggtggtggccaaagtggaaaagggcaagtccaagaaactgaagagtgtgaaagagctgctggggatcaccatcatggaaagaagcagcttcgagaagaatcccatcgactttctggaagccaagggctacaaagaagtgaaaaaggacctgatcatcaagctgcctaagtactccctgttcgagctggaaaacggccggaagagaatgctggcctctgccggcgaactgcagaagggaaacgaactggccctgccctccaaatatgtgaacttcctgtacctggccagccactatgagaagctgaagggctcccccgaggataatgagcagaaacagctgtttgtggaacagcacaaacactacctggacgagatcatcgagcagatcagcgagttctccaagagagtgatcctggccgacgctaatctggacaaggtgctgagcgcctacaacaagcacagagacaagcctatcagagagcaggccgagaatatcatccacctgtttaccctgaccaatctgggagcccctgccgccttcaagtactttgacaccaccatcgaccggaagaggtacaccagcaccaaagaggtgctggacgccaccctgatccaccagagcatcaccggcctgtacgagacacggatcgacctgtctcagctgggaggcgacgcctatccctatgacgtgcccgattatgccagcctgggcagcggctcccccaagaaaaaacgcaaggtggaagatcctaagaaaaagcggaaagtggacggcagcggcagcgagacccccggtaccagcgagagcgccacccccgagagcatgaacaattcccagggaagagtgaccttcgaggatgtcactgtgaacttcacccagggggagtggcagcggctgaatcccgaacagagaaacttgtacagggatgtgatgctggagaattacagcaaccttgtctctgtgggacaaggggaaaccaccaaacccgatgtgatcttgaggttggaacaaggaaaggagccatggttggaggaagaggaagtgctgggaagtggccgtgcagaaaaaaatggggacattggagggcagatttggaagccaaaggatgtgaaagagagtctcctcgagtgataatagggatcccaagcacgcagcaatgcagctcaaaacgcttagcctagccacacccccacgggaaacagcagtgattaacctttagcaataaacgaaagtttaactaagctatactaaccccagggttggtcaatttcgtgccagccacaccctggtactgcatgcacgcaatgctagctgcccctttcccgtcctgggcaccccgagtctcccccgaccccgggtcccaggtatgctcccacctccacctgccccactcaccacctctgctagttccagacacctccgagacgaggaaaaaaaaaaaaaaaaaaaaaaaaaaaaaaaaaaaaaaaaaaaaaaaaaaaaaaaaaaaaaaaaaaaaaaaaaaaaaaaaaaaaaaaaaaaaaaaaaaaaaaaaaaaaaaaaaaaaaaaa

SEQ ID NO: 268 - RNA, 8344 nt, synthetic construct
  misc_feature 1..8344: note = mRNA of V27_3xGCN4-dCas9-ZIM3-2a-D3a-hD3L-scFv
  source 1..8344: mol_type = other RNA
aggactcactatttgttttcgcgcccagttgcaaaaagtgtcgacatttgcttctgacacaactgtgttcactagcaacctcaaacagacaccgccaccatgcctgctgctaagagagtgaaactggatggatccgaggaactgctgagcaagaactaccacctggaaaacgaggtggccagactgaagaaaggctctggctctggcggaagcggttctggcggatcaggatctggaagtggcggctctggaagcggaggttctggatctggcgaagaactgctgtctaagaattatcacctcgagaacgaagtggctcggctcaagaaaggcagtggcagcggaggaagtggatccggcggtagtggtagtggaagcggcggatccggctcaggcggatctggttcaggggaagaactcctctccaaaaactaccatctcgagaatgaggtcgcccgcctgaaaaaaggatcaggttccggtggttctggcagcggtggttcaggctcaggcagcggcggtagcggtagcggtggaagcggaagcggaccaaaaaagaagagaaaggtaatggacaagaagtacagcatcggcctggccatcggcaccaactctgtgggctgggccgtgatcaccgacgagtacaaggtgcccagcaagaaattcaaggtgctgggcaacaccgaccggcacagcatcaagaagaacctgatcggcgccctgctgttcgacagcggagaaacagccgaggccacccggctgaagagaaccgccagaagaagatacaccagacggaagaaccggatctgctatctgcaagagatcttcagcaacgagatggccaaggtggacgacagcttcttccacagactggaagagtccttcctggtggaagaggataagaagcacgagcggcaccccatcttcggcaacatcgtggacgaggtggcctaccacgagaagtaccccaccatctaccacctgagaaagaaactggtggacagcaccgacaaggccgacctgcggctgatctatctggccctggcccacatgatcaagttccggggccacttcctgatcgagggcgacctgaaccccgacaacagcgacgtggacaagctgttcatccagctggtgcagacctacaaccagctgttcgaggaaaaccccatcaacgccagcggcgtggacgccaaggccatcctgtctgccagactgagcaagagcagacggctggaaaatctgatcgcccagctgcccggcgagaagaagaatggcctgttcggcaacctgattgccctgagcctgggcctgacccccaacttcaagagcaacttcgacctggccgaggatgccaaactgcagctgagcaaggacacctacgacgacgacctggacaacctgctggcccagatcggcgaccagtacgccgacctgtttctggccgccaagaacctgtccgacgccatcctgctgagcgacatcctgagagtgaacaccgagatcaccaaggcccccctgagcgcctctatgatcaagagatacgacgagcaccaccaggacctgaccctgctgaaagctctcgtgcggcagcagctgcctgagaagtacaaagagattttcttcgaccagagcaagaacggctacgccggctacatcgatggcggagccagccaggaagagttctacaagttcatcaagcccatcctggaaaagatggacggcaccgaggaactgctcgtgaagctgaacagagaggacctgctgcggaagcagcggaccttcgacaacggcagcatcccccaccagatccacctgggagagctgcacgccattctgcggcggcaggaagatttttacccattcctgaaggacaaccgggaaaagatcgagaagatcctgaccttccgcatcccctactacgtgggccctctggccaggggaaacagcagattcgcctggatgaccagaaagagcgaggaaaccatcaccccctggaacttcgaggaagtggtggacaagggcgccagcgcccagagcttcatcgagcggatgaccaacttcgataagaacctgcccaacgagaaggtgctgcccaagcacagcctgctgtacgagtacttcaccgtgtacaacgagctgaccaaagtgaaatacgtgaccgagggaatgagaaagcccgccttcctgagcggcgagcagaaaaaagccatcgtggacctgctgttcaagaccaaccggaaagtgaccgtgaagcagctgaaagaggactacttcaagaaaatcgagtgcttcgactccgtggaaatctccggcgtggaagatcggttcaacgcctccctgggcacataccacgatctgctgaaaattatcaaggacaaggacttcctggacaatgaggaaaacgaggacattctggaagatatcgtgctgaccctgacactgtttgaggacagagagatgatcgaggaacggctgaaaacctatgcccacctgttcgacgacaaagtgatgaagcagctgaagcggcggagatacaccggctggggcaggctgagccggaagctgatcaacggcatccgggacaagcagtccggcaagacaatcctggatttcctgaagtccgacggcttcgccaacagaaacttcatgcagctgatccacgacgacagcctgacctttaaagaggacatccagaaagcccaggtgtccggccagggcgatagcctgcacgagcacattgccaatctggccggcagccccgccattaagaagggcatcctgcagacagtgaaggtggtggacgagctcgtgaaagtgatgggccggcacaagcccgagaacatcgtgatcgaaatggccagagagaaccagaccacccagaagggacagaagaacagccgcgagagaatgaagcggatcgaagagggcatcaaagagctgggcagccagatcctgaaagaacaccccgtggaaaacacccagctgcagaacgagaagctgtacctgtactacctgcagaatgggcgggatatgtacgtggaccaggaactggacatcaaccggctgtccgactacgatgtggacgctatcgtgcctcagagctttctgaaggacgactccatcgataacaaagtgctgactcggagcgacaagaaccggggcaagagcgacaacgtgccctccgaagaggtcgtgaagaagatgaagaactactggcgccagctgctgaatgccaagctgattacccagaggaagttcgacaatctgaccaaggccgagagaggcggcctgagcgaactggataaggccggcttcatcaagagacagctggtggaaacccggcagatcacaaagcacgtggcacagatcctggactcccggatgaacactaagtacgacgagaacgacaaactgatccgggaagtgaaagtgatcaccctgaagtccaagctggtgtccgatttccggaaggatttccagttttacaaagtgcgcgagatcaacaactaccaccacgcccacgacgcctacctgaacgccgtcgtgggaaccgccctgatcaaaaagtaccctaagctggaaagcgagttcgtgtacggcgactacaaggtgtacgacgtgcggaagatgatcgccaagagcgagcaggaaatcggcaaggctaccgccaagtacttcttctacagcaacatcatgaactttttcaagaccgagattaccctggccaacggcgagatccggaagcggcctctgatcgagacaaacggcgaaacaggcgagatcgtgtgggataagggccgggactttgccaccgtgcggaaagtgctgtctatgccccaagtgaatatcgtgaaaaagaccgaggtgcagacaggcggcttcagcaaagagtctatcctgcccaagaggaacagcgacaagctgatcgccagaaagaaggactgggaccctaagaagtacggcggcttcgacagccccaccgtggcctattctgtgctggtggtggccaaagtggaaaagggcaagtccaagaaactgaagagtgtgaaagagctgctggggatcaccatcatggaaagaagcagcttcgagaagaatcccatcgactttctggaagccaagggctacaaagaagtgaaaaaggacctgatcatcaagctgcctaagtactccctgttcgagctggaaaacggccggaagagaatgctggcctctgccggcgaactgcagaagggaaacgaactggccctgccctccaaatatgtgaacttcctgtacctggccagccactatgagaagctgaagggctcccccgaggataatgagcagaaacagctgtttgtggaacagcacaaacactacctggacgagatcatcgagcagatcagcgagttctccaagagagtgatcctggccgacgctaatctggacaaggtgctgagcgcctacaacaagcacagagacaagcctatcagagagcaggccgagaatatcatccacctgtttaccctgaccaatctgggagcccctgccgccttcaagtactttgacaccaccatcgaccggaagaggtacaccagcaccaaagaggtgctggacgccaccctgatccaccagagcatcaccggcctgtacgagacacggatcgacctgtctcagctgggaggcgacgcctatccctatgacgtgcccgattatgccagcctgggcagcggctcccccaagaaaaaacgcaaggtggaagatcctaagaaaaagcggaaagtggacggcagcggcagcgagacccccggtaccagcgagagcgccacccccgagagcatgaacaattcccagggaagagtgaccttcgaggatgtcactgtgaacttcacccagggggagtggcagcggctgaatcccgaacagagaaacttgtacagggatgtgatgctggagaattacagcaaccttgtctctgtgggacaaggggaaaccaccaaacccgatgtgatcttgaggttggaacaaggaaaggagccatggttggaggaagaggaagtgctgggaagtggccgtgcagaaaaaaatggggacattggagggcagatttggaagccaaaggatgtgaaagagagtctcctcgagggaagcggagctactaacttcagcctgctgaagcaggctggagacgtggaggagaaccctggacctatgcctgctgctaagagagtgaaactggatggatccaaccatgaccaggaatttgaccccccaaaggtttacccacctgtgccagctgagaagaggaagcccatccgcgtgctgtctctctttgatgggattgctacagggctcctggtgctgaaggacctgggcatccaagtggaccgctacattgcctccgaggtgtgtgaggactccatcacggtgggcatggtgcggcaccagggaaagatcatgtacgtcggggacgtccgcagcgtcacacagaagcatatccaggagtggggcccattcgacctggtgattggaggcagtccctgcaatgacctctccattgtcaaccctgcccgcaagggactttatgagggtactggccgcctcttctttgagttctaccgcctcctgcatgatgcgcggcccaaggagggagatgatcgccccttcttctggctctttgagaatgtggtggccatgggcgttagtgacaagagggacatctcgcgatttcttgagtctaaccccgtgatgattgacgccaaagaagtgtctgctgcacacagggcccgttacttctggggtaaccttcctggcatgaacaggcctttggcatccactgtgaatgataagctggagctgcaagagtgtctggagcacggcagaatagccaagttcagcaaagtgaggaccattaccaccaggtcaaactctataaagcagggcaaagaccagcatttccccgtgttcatgaacgagaaggaggacatcctgtggtgcactgaaatggaaagggtgtttggcttccccgtccactacacagacgtctccaacatgagccgcttggcgaggcagagactgctgggccgatcgtggagcgtgccggtcatccgccacctcttcgctccgctgaaggaatattttgcttgtgtgtctagcggcaatagtaacgctaacagccgcgggccgagcttcagcagcggcctggtgccgttaagcttgcgcggcagccatatgttcgaaaccgtgcctgtgtggaggagacagccagtccgggtgctgtccctttttgaagacatcaagaaagagctgacgagtttgggctttttggaaagtggttctgacccgggacaactgaagcatgtggttgatgtcacagacacagtgaggaaggatgtggaggagtggggacccttcgatcttgtgtacggcgccacacctcccctgggccacacctgtgaccgtcctcccagctggtacctgttccagttccaccggctcctgcagtacgcacggcccaagccaggcagccccaggcccttcttctggatgttcgtggacaatctggtgctgaacaaggaagacctggacgtcgcatctcgcttcctggagatggagccagtcaccatcccagatgtccacggcggatccttgcagaatgctgtccgcgtgtggagcaacatcccagccataaggagcagcaggcactgggctctggtttcggaagaagaattgtccctgctggcccagaacaagcagagctcgaagctcgcggccaagtggcccaccaagctggtgaagaactgctttctccccctaagagaatatttcaagtatttttcaggagggccgagctctggcgcacccccaccaagtggagggtctcctgccgggtccccaacatctactgaagaaggcaccagcgaatccgcaacgcccgagtcaggccctggtacctccacagaaccatctgaaggtagtgcgcctggttccccagctggaagccctacttccaccgaagaaggcacgtcaaccgaaccaagtgaaggatctgcccctgggaccagcactgaaccatctgagccaaaaaagaagagaaaggtaccatctgagggccccgacatcgtgatgacccagagccccagcagcctgagcgccagcgtgggcgaccgcgtgaccatcacctgccgcagcagcaccggcgccgtgaccaccagcaactacgccagctgggtgcaggagaagcccggcaagctgttcaagggcctgatcggcggcaccaacaaccgcgcccccggcgtgcccagccgcttcagcggcagcctgatcggcgacaaggccaccctgaccatcagcagcctgcagcccgaggacttcgccacctacttctgcgccctgtggtacagcaaccactgggtgttcggccagggcaccaaggtggagctgaagcgcggcggcggcggcagcggcggcggcggcagcggcggcggcggcagcagcggcggcggcagcgaggtgaagctgctggagagcggcggcggcctggtgcagcccggcggcagcctgaagctgagctgcgccgtgagcggcttcagcctgaccgactacggcgtgaactgggtgcgccaggcccccggccgcggcctggagtggatcggcgtgatctggggcgacggcatcaccgactacaacagcgccctgaaggaccgcttcatcatcagcaaggacaacggcaagaacaccgtgtacctgcagatgagcaaggtgcgcagcgacgacaccgccctgtactactgcgtgaccggcctgttcgactactggggccagggcaccctggtgaccgtgagcagctacccatacgatgttccagattacgctggtggaggcggaggttctgggggaggaggtagtggcggtggtggttcaggaggcggcggaagctgataataggatcccaagcacgcagcaatgcagctcaaaacgcttagcctagccacacccccacgggaaacagcagtgattaacctttagcaataaacgaaagtttaactaagctatactaaccccagggttggtcaatttcgtgccagccacaccctggtactgcatgcacgcaatgctagctgcccctttcccgtcctgggcaccccgagtctcccccgaccccgggtcccaggtatgctcccacctccacctgccccactcaccacctctgctagttccagacacctccgagacgaggaaaaaaaaaaaaaaaaaaaaaaaaaaaaaaaaaaaaaaaaaaaaaaaaaaaaaaaaaaaaaaaaaaaaaaaaaaaaaaaaaaaaaaaaaaaaaaaaaaaaaaaaaaaaaaaaaaaaaaaa

SEQ ID NO: 269 - RNA, 7924 nt, synthetic construct
  misc_feature 1..7924: note = mRNA of V28_3xGCN4-dCas12a-ZIM3-2a-D3a-hD3L-scFv
  source 1..7924: mol_type = other RNA
aggactcactatttgttttcgcgcccagttgcaaaaagtgtcgacatttgcttctgacacaactgtgttcactagcaacctcaaacagacaccgccaccatgcctgctgctaagagagtgaaactggatggatccgaggaactgctgagcaagaactaccacctggaaaacgaggtggccagactgaagaaaggctctggctctggcggaagcggttctggcggatcaggatctggaagtggcggctctggaagcggaggttctggatctggcgaagaactgctgtctaagaattatcacctcgagaacgaagtggctcggctcaagaaaggcagtggcagcggaggaagtggatccggcggtagtggtagtggaagcggcggatccggctcaggcggatctggttcaggggaagaactcctctccaaaaactaccatctcgagaatgaggtcgcccgcctgaaaaaaggatcaggttccggtggttctggcagcggtggttcaggctcaggcagcggcggtagcggtagcggtggaagcggaagcggaccaaaaaagaagagaaaggtaatgtcaaagctggagaaattcaccaactgttatagcctgtctaagaccctgcgcttcaaggcaatcccagtgggcaagacacaagagaacattgacaacaaacggctcctggtggaggatgagaagagggctgaagattacaagggcgttaagaagctgctggataggtactatctgtcattcatcaacgatgtcctccacagtatcaagctgaagaatctgaacaattacatttctctgttccggaagaagacacggaccgagaaggagaacaaagagctggagaatctggagatcaacctgaggaaagaaatagctaaggctttcaaagggaacgagggttacaagtccctgttcaagaaagacattatcgagactattctgcctgagttcctggacgataaagatgagatcgccctcgtcaattccttcaatgggtttaccacagcctttaccggcttcttcgacaatagagagaatatgttctctgaagaggccaaatccactagcatcgcctttcgctgcataaacgagaacctgactaggtacatcagcaatatggacatctttgagaaagtcgatgccatattcgacaaacatgaggtgcaggagattaaggagaagatcctgaactcagattacgatgtcgaagatttcttcgagggagagttcttcaacttcgtgctcacacaagagggcattgatgtgtacaatgcaatcattggagggttcgtgacagagagtggcgagaagataaagggcctgaacgagtatatcaacctctacaaccagaaaaccaagcagaaactgcctaagttcaagccactgtacaaacaagtgctctcagatagggaaagcctgagcttctacggtgaagggtatacatcagatgaagaagtgctcgaagtgttccgcaacaccctcaataagaacagtgaaatcttctcttcaatcaagaagctggagaaactgttcaagaatttcgatgagtactcctctgccggaatctttgtgaagaatggccctgcaatatccactattagcaaagacatctttggcgagtggaacgttatcagggataagtggaatgccgagtacgatgatattcatctcaagaagaaagccgtggttacagagaaatacgaggatgatagacgcaagagctttaagaagattggtagcttctctctcgaacagctgcaggagtacgccgacgctgacctgtcagtcgtggagaaactcaaggagatcataatccagaaggtggatgaaatctacaaagtgtatggaagctctgagaaactcttcgatgcagactttgttctggagaagagtctgaagaagaacgacgcagtggttgctatcatgaaggacctgctggattctgttaagtctttcgagaattacattaaggcattctttggtgaagggaaggagacaaatagggacgagagcttctatggcgactttgttctggcctacgacatcctcctcaaggttgaccacatctatgacgctatacggaattacgttacccagaagccctatagcaaagacaagttcaagctgtatttccagaatccacagtttatgggtgggtgggataaagacaaagaaacagattacagggccactatcctgcggtacggcagcaaatactatctggctatcatggataagaagtacgccaaatgcctccagaagatcgacaaggacgacgtgaacggtaactacgagaagatcaattacaagctcctgccaggacctaacaagatgctgcccaaggtgttcttctccaagaaatggatggcctactataacccaagcgaggacattcagaagatatacaagaatgggacattcaagaagggcgatatgttcaacctcaacgactgccacaagctgattgatttcttcaaggatagcatttctcgctatcccaagtggtctaatgcatacgatttcaacttcagcgagactgagaagtacaaagacatcgctggcttctaccgggaggtggaagagcaaggctataaggtgtcattcgaatccgcttctaagaaggaagtggataagctcgtggaagagggtaagctgtacatgttccagatatacaacaaagacttcagcgataagagccacggcactccaaacctccatactatgtatttcaagctgctgtttgacgagaacaaccacggacagattaggctgtcaggaggcgcagaactcttcatgcgcagagcttcactgaagaaggaggaactcgttgtccacccagccaatagccctatagccaataagaatccagacaatcctaagaaaaccactactctgtcttacgatgtgtataaggataagagattctctgaagatcagtacgaactgcacatacccattgccattaacaagtgccctaagaacatcttcaagattaacacagaggttagagtgctcctgaaacacgacgataacccttatgttataggcattgctcgcggagagagaaacctgctgtacatcgtcgtggtggacggcaaaggcaacatcgtggaacagtacagtctcaatgaaatcattaacaatttcaacggaatccgcattaagaccgactaccattctctcctcgacaagaaggagaaagaaaggttcgaagcaagacagaattggacaagtatagagaatatcaaagaactgaaggctgggtacatctctcaggttgtgcacaagatatgtgagctggtggagaagtacgacgctgttatcgccctcgcggacctgaatagcggcttcaagaactccagggtgaaggtggagaagcaggtgtatcagaagttcgagaagatgctgatcgacaagctcaactatatggtggacaagaaatccaatccttgcgctactggtggagccctgaagggctatcaaatcaccaataagttcgaatctttcaagtctatgagcacccagaatggcttcatcttctacatacccgcatggctgacatccaagattgatccctctaccggatttgttaatctgctcaagactaagtacacctctattgctgactcaaagaagttcatatcatcatttgaccgcatcatgtacgtgccagaagaggacctgttcgagtttgccctggattacaagaatttctctcggactgacgccgactacatcaagaagtggaagctctactcttatggtaatcggattcgcatattccgcaatcccaagaagaataacgtgttcgattgggaggaagtttgcctcaccagcgcttacaaggagctgttcaataagtatgggattaactaccagcagggcgacataagagccctgctgtgcgaacaatctgataaggcattctattcctctttcatggcactgatgtcactgatgctgcaaatgcgcaattccatcaccggaagaacagacgtggcctttctgatctctcctgtcaagaactcagatggcatcttctacgattcccgcaactatgaagcacaggagaatgctatcctgcctaagaatgccgatgcaaatggagcctataacatcgccagaaaggtcctctgggccataggacaattcaagaaagctgaagatgagaagctggacaaggtgaagatcgccatttcaaacaaagagtggctcgaatatgctcagacctcagtgaagcatgcctatccctatgacgtgcccgattatgccagcctgggcagcggctcccccaagaaaaaacgcaaggtggaagatcctaagaaaaagcggaaagtggacggcagcggcagcgagacccccggtaccagcgagagcgccacccccgagagcatgaacaattcccagggaagagtgaccttcgaggatgtcactgtgaacttcacccagggggagtggcagcggctgaatcccgaacagagaaacttgtacagggatgtgatgctggagaattacagcaaccttgtctctgtgggacaaggggaaaccaccaaacccgatgtgatcttgaggttggaacaaggaaaggagccatggttggaggaagaggaagtgctgggaagtggccgtgcagaaaaaaatggggacattggagggcagatttggaagccaaaggatgtgaaagagagtctcctcgagggaagcggagctactaacttcagcctgctgaagcaggctggagacgtggaggagaaccctggacctatgcctgctgctaagagagtgaaactggatggatccaaccatgaccaggaatttgaccccccaaaggtttacccacctgtgccagctgagaagaggaagcccatccgcgtgctgtctctctttgatgggattgctacagggctcctggtgctgaaggacctgggcatccaagtggaccgctacattgcctccgaggtgtgtgaggactccatcacggtgggcatggtgcggcaccagggaaagatcatgtacgtcggggacgtccgcagcgtcacacagaagcatatccaggagtggggcccattcgacctggtgattggaggcagtccctgcaatgacctctccattgtcaaccctgcccgcaagggactttatgagggtactggccgcctcttctttgagttctaccgcctcctgcatgatgcgcggcccaaggagggagatgatcgccccttcttctggctctttgagaatgtggtggccatgggcgttagtgacaagagggacatctcgcgatttcttgagtctaaccccgtgatgattgacgccaaagaagtgtctgctgcacacagggcccgttacttctggggtaaccttcctggcatgaacaggcctttggcatccactgtgaatgataagctggagctgcaagagtgtctggagcacggcagaatagccaagttcagcaaagtgaggaccattaccaccaggtcaaactctataaagcagggcaaagaccagcatttccccgtgttcatgaacgagaaggaggacatcctgtggtgcactgaaatggaaagggtgtttggcttccccgtccactacacagacgtctccaacatgagccgcttggcgaggcagagactgctgggccgatcgtggagcgtgccggtcatccgccacctcttcgctccgctgaaggaatattttgcttgtgtgtctagcggcaatagtaacgctaacagccgcgggccgagcttcagcagcggcctggtgccgttaagcttgcgcggcagccatatgttcgaaaccgtgcctgtgtggaggagacagccagtccgggtgctgtccctttttgaagacatcaagaaagagctgacgagtttgggctttttggaaagtggttctgacccgggacaactgaagcatgtggttgatgtcacagacacagtgaggaaggatgtggaggagtggggacccttcgatcttgtgtacggcgccacacctcccctgggccacacctgtgaccgtcctcccagctggtacctgttccagttccaccggctcctgcagtacgcacggcccaagccaggcagccccaggcccttcttctggatgttcgtggacaatctggtgctgaacaaggaagacctggacgtcgcatctcgcttcctggagatggagccagtcaccatcccagatgtccacggcggatccttgcagaatgctgtccgcgtgtggagcaacatcccagccataaggagcagcaggcactgggctctggtttcggaagaagaattgtccctgctggcccagaacaagcagagctcgaagctcgcggccaagtggcccaccaagctggtgaagaactgctttctccccctaagagaatatttcaagtatttttcaggagggccgagctctggcgcacccccaccaagtggagggtctcctgccgggtccccaacatctactgaagaaggcaccagcgaatccgcaacgcccgagtcaggccctggtacctccacagaaccatctgaaggtagtgcgcctggttccccagctggaagccctacttccaccgaagaaggcacgtcaaccgaaccaagtgaaggatctgcccctgggaccagcactgaaccatctgagccaaaaaagaagagaaaggtaccatctgagggccccgacatcgtgatgacccagagccccagcagcctgagcgccagcgtgggcgaccgcgtgaccatcacctgccgcagcagcaccggcgccgtgaccaccagcaactacgccagctgggtgcaggagaagcccggcaagctgttcaagggcctgatcggcggcaccaacaaccgcgcccccggcgtgcccagccgcttcagcggcagcctgatcggcgacaaggccaccctgaccatcagcagcctgcagcccgaggacttcgccacctacttctgcgccctgtggtacagcaaccactgggtgttcggccagggcaccaaggtggagctgaagcgcggcggcggcggcagcggcggcggcggcagcggcggcggcggcagcagcggcggcggcagcgaggtgaagctgctggagagcggcggcggcctggtgcagcccggcggcagcctgaagctgagctgcgccgtgagcggcttcagcctgaccgactacggcgtgaactgggtgcgccaggcccccggccgcggcctggagtggatcggcgtgatctggggcgacggcatcaccgactacaacagcgccctgaaggaccgcttcatcatcagcaaggacaacggcaagaacaccgtgtacctgcagatgagcaaggtgcgcagcgacgacaccgccctgtactactgcgtgaccggcctgttcgactactggggccagggcaccctggtgaccgtgagcagctacccatacgatgttccagattacgctggtggaggcggaggttctgggggaggaggtagtggcggtggtggttcaggaggcggcggaagctgataataggatcccaagcacgcagcaatgcagctcaaaacgcttagcctagccacacccccacgggaaacagcagtgattaacctttagcaataaacgaaagtttaactaagctatactaaccccagggttggtcaatttcgtgccagccacaccctggtactgcatgcacgcaatgctagctgcccctttcccgtcctgggcaccccgagtctcccccgaccccgggtcccaggtatgctcccacctccacctgccccactcaccacctctgctagttccagacacctccgagacgaggaaaaaaaaaaaaaaaaaaaaaaaaaaaaaaaaaaaaaaaaaaaaaaaaaaaaaaaaaaaaaaaaaaaaaaaaaaaaaaaaaaaaaaaaaaaaaaaaaaaaaaaaaaaaaaaaaaaaaaaa

SEQ ID NO: 270 - RNA, 7273 nt, synthetic construct
  misc_feature 1..7273: note = mRNA of V29_3xGCN4-dCas12i-ZIM3-2a-D3a-hD3L-scFv
  source 1..7273: mol_type = other RNA
aggactcactatttgttttcgcgcccagttgcaaaaagtgtcgacatttgcttctgacacaactgtgttcactagcaacctcaaacagacaccgccaccatgcctgctgctaagagagtgaaactggatggatccgaggaactgctgagcaagaactaccacctggaaaacgaggtggccagactgaagaaaggctctggctctggcggaagcggttctggcggatcaggatctggaagtggcggctctggaagcggaggttctggatctggcgaagaactgctgtctaagaattatcacctcgagaacgaagtggctcggctcaagaaaggcagtggcagcggaggaagtggatccggcggtagtggtagtggaagcggcggatccggctcaggcggatctggttcaggggaagaactcctctccaaaaactaccatctcgagaatgaggtcgcccgcctgaaaaaaggatcaggttccggtggttctggcagcggtggttcaggctcaggcagcggcggtagcggtagcggtggaagcggaagcggaccaaaaaagaagagaaaggtaatgggcatcaccatgagcgacaccaccttcagaccctacaagagcaagctgaaccccaacgagcggaagatgcctatggtggtggacaccatgaattggtgcgacaacgcctgcagcgtgttcttcgatctgttcgtgggcctgtacggcggcgtgaagatcggcgacgtgaccaatttcctgaccgagaagcaggacaccaccaccgatgccgatctgctgtgcgccatcaactggttcagagccatgcctgtgtctaaccccgatgccgttgtgggacctgagcagctggttgtgcggttcagagactacagcggccacaatccatctccaatggccagcatgtacctgagcgcccctgtgaaccctagatacacctgggtcgactgccggttcctgtaccagcagatgtgtcagaccctgggcgccaacctggatgtggacatctctaccctggtgcagaccggcctgctgcctatccagaaggatacacagctgaacgcctacagcttctgcagcaacgtgttcggcgagggcgtgaaagaagatcccagcgccaaagtgaccagctacacagccgctgccaatgctctgagcggcgccaccaatcctatcatcacctacgaggactaccggcagatcctgtccagcgccatcaccaacagacccagcagaaagggcgccaaggatattctggccgccgatctggatagcaccaagacaggtgttctgcccggcaactacgtgtcccagagaatcgccatgtaccaggcctctgccgcctctaaagctagaggcgtggtgctgcccaaccggctgagagtgaaagcctacctgcagaacctcgtgggactgaactacatctgcaccacctgggccgctcctatgctgagagccgtgggcgacatcaagagcaagaacagcaacaactaccgcttcgtgggcgagagactggaacggcagcaagagatcgataacctgctggccgtgtccaacatcagaagcgcccaggccatcctgcagcagttcagggccaatgagagcaaccagttctacatcaagaagcggcacatcggcaagggcctgcctagcctgtacgacatgtgggatctgatggacgagaaagagggcatcgacaactacatccagagcctgaagggcgacaagaccgagaggctgccaatcagagagctgctgcagatcatctaccctcacagaaagagcgtgtccgccgagctgtttctgtctgccgccgaactgaccgacgtggaagatagacagaaccggtgcatggtgcaccctacagtgcggggctctctggtcatcaacttcggcaagagcagcaccatcttcggcgctatcacccctcctgacacactgatcaagttccggggcgaaatggtgcctgctggacagacaggcatgatctggttcacaatgcacctggtggacggcggcaaatgggtcaagcaccacattccttgccacagcagccggtacttcgaggaaatctacgcctggaagaaggacctgcctacactgccctttccacggcggagcctgtatggctatgccatcggcaacaagatcagcgacacccggaagatcgacctgcggagaaagaaggccagcaagcagtacctgcggaccctggaaaacatgacccacaacgtggaatttgaccccaccacacagttcatggtggaccaagagctgaacgtgaccatcaccgccagagtgaagaaaatccctcctgtgcgggatgtgcccgtgggcagcagaattatgggcctgaacaagaaccagaccatccgggactgctacagcatctgggagagagtggaagccaacaccagcggcagctttcagcatcccgtggtccaggatgtgtggctgagactggtggccgatggccacgtgacctctacagtgaatggccccaacggccagatcgaccagatgagctactctggccccgatgtggccaactgcggcaactggatgcaagagcggagcaacttcatcaccagcgtggacgacgccgaccagtctatcatgaagcactttctgtggaacaaccgcgtgaagctgtatgcctggaactgcgtgtacgccggcacactgatgaaggccatctctaagcagatgaccaccgccaaccggaacctgttcagaaacgagatcctgagcttcgttggcggcagattcggctgcagactgggatctctggcccaggtttcactggacctgctgcggaggatgaagtccgtgatcagctgctacttcagccggaacaacgccttcaccatcgaggaaagaagcgccttcgacaaagaactgatggaactgttcgagagcctggacaacaagatgaacaacaagcggaaagagaaagtcaaccggacactcagcagcatcttccaggtggccaagcagcacaatgttgtgcggctggtggtcaccaagaacctgcagacccctgatgccaatgtgcggagcgtgatgaatcagagatccgtggattggtgcgctcggaagattgaagagaagatcgtggacctgggcaacgtgatcggaatctatgtggatctggtggaagccctggatctgagccatctggaccccttcatctatatcgccaagggcgacgtgggcaaagagtgccagtttgacgaggtggaaagcagctccctgctgccaattcacaccagcatgtttcgcgactggcacggcctggttaacaagggcagaaccaccacacctatctaccacagcgccctgaggagcttcgccagccactacggcctgagattcgatgacctggccagaatcaaggccgctgagctggccaaaatgctgccagaccagaaggtgttcatcccacacagaggcggacggttcttcatgagcacataccccgtgaccagcaccagcagacccgtgtcttatgatggccggcagcggttcctgaacagcggcgatatggtggccccagtgaacaccatgctgcgcggattcagaagggccagatctgcctatccctatgacgtgcccgattatgccagcctgggcagcggctcccccaagaaaaaacgcaaggtggaagatcctaagaaaaagcggaaagtggacggcagcggcagcgagacccccggtaccagcgagagcgccacccccgagagcatgaacaattcccagggaagagtgaccttcgaggatgtcactgtgaacttcacccagggggagtggcagcggctgaatcccgaacagagaaacttgtacagggatgtgatgctggagaattacagcaaccttgtctctgtgggacaaggggaaaccaccaaacccgatgtgatcttgaggttggaacaaggaaaggagccatggttggaggaagaggaagtgctgggaagtggccgtgcagaaaaaaatggggacattggagggcagatttggaagccaaaggatgtgaaagagagtctcctcgagggaagcggagctactaacttcagcctgctgaagcaggctggagacgtggaggagaaccctggacctatgcctgctgctaagagagtgaaactggatggatccaaccatgaccaggaatttgaccccccaaaggtttacccacctgtgccagctgagaagaggaagcccatccgcgtgctgtctctctttgatgggattgctacagggctcctggtgctgaaggacctgggcatccaagtggaccgctacattgcctccgaggtgtgtgaggactccatcacggtgggcatggtgcggcaccagggaaagatcatgtacgtcggggacgtccgcagcgtcacacagaagcatatccaggagtggggcccattcgacctggtgattggaggcagtccctgcaatgacctctccattgtcaaccctgcccgcaagggactttatgagggtactggccgcctcttctttgagttctaccgcctcctgcatgatgcgcggcccaaggagggagatgatcgccccttcttctggctctttgagaatgtggtggccatgggcgttagtgacaagagggacatctcgcgatttcttgagtctaaccccgtgatgattgacgccaaagaagtgtctgctgcacacagggcccgttacttctggggtaaccttcctggcatgaacaggcctttggcatccactgtgaatgataagctggagctgcaagagtgtctggagcacggcagaatagccaagttcagcaaagtgaggaccattaccaccaggtcaaactctataaagcagggcaaagaccagcatttccccgtgttcatgaacgagaaggaggacatcctgtggtgcactgaaatggaaagggtgtttggcttccccgtccactacacagacgtctccaacatgagccgcttggcgaggcagagactgctgggccgatcgtggagcgtgccggtcatccgccacctcttcgctccgctgaaggaatattttgcttgtgtgtctagcggcaatagtaacgctaacagccgcgggccgagcttcagcagcggcctggtgccgttaagcttgcgcggcagccatatgttcgaaaccgtgcctgtgtggaggagacagccagtccgggtgctgtccctttttgaagacatcaagaaagagctgacgagtttgggctttttggaaagtggttctgacccgggacaactgaagcatgtggttgatgtcacagacacagtgaggaaggatgtggaggagtggggacccttcgatcttgtgtacggcgccacacctcccctgggccacacctgtgaccgtcctcccagctggtacctgttccagttccaccggctcctgcagtacgcacggcccaagccaggcagccccaggcccttcttctggatgttcgtggacaatctggtgctgaacaaggaagacctggacgtcgcatctcgcttcctggagatggagccagtcaccatcccagatgtccacggcggatccttgcagaatgctgtccgcgtgtggagcaacatcccagccataaggagcagcaggcactgggctctggtttcggaagaagaattgtccctgctggcccagaacaagcagagctcgaagctcgcggccaagtggcccaccaagctggtgaagaactgctttctccccctaagagaatatttcaagtatttttcaggagggccgagctctggcgcacccccaccaagtggagggtctcctgccgggtccccaacatctactgaagaaggcaccagcgaatccgcaacgcccgagtcaggccctggtacctccacagaaccatctgaaggtagtgcgcctggttccccagctggaagccctacttccaccgaagaaggcacgtcaaccgaaccaagtgaaggatctgcccctgggaccagcactgaaccatctgagccaaaaaagaagagaaaggtaccatctgagggccccgacatcgtgatgacccagagccccagcagcctgagcgccagcgtgggcgaccgcgtgaccatcacctgccgcagcagcaccggcgccgtgaccaccagcaactacgccagctgggtgcaggagaagcccggcaagctgttcaagggcctgatcggcggcaccaacaaccgcgcccccggcgtgcccagccgcttcagcggcagcctgatcggcgacaaggccaccctgaccatcagcagcctgcagcccgaggacttcgccacctacttctgcgccctgtggtacagcaaccactgggtgttcggccagggcaccaaggtggagctgaagcgcggcggcggcggcagcggcggcggcggcagcggcggcggcggcagcagcggcggcggcagcgaggtgaagctgctggagagcggcggcggcctggtgcagcccggcggcagcctgaagctgagctgcgccgtgagcggcttcagcctgaccgactacggcgtgaactgggtgcgccaggcccccggccgcggcctggagtggatcggcgtgatctggggcgacggcatcaccgactacaacagcgccctgaaggaccgcttcatcatcagcaaggacaacggcaagaacaccgtgtacctgcagatgagcaaggtgcgcagcgacgacaccgccctgtactactgcgtgaccggcctgttcgactactggggccagggcaccctggtgaccgtgagcagctacccatacgatgttccagattacgctggtggaggcggaggttctgggggaggaggtagtggcggtggtggttcaggaggcggcggaagctgataataggatcccaagcacgcagcaatgcagctcaaaacgcttagcctagccacacccccacgggaaacagcagtgattaacctttagcaataaacgaaagtttaactaagctatactaaccccagggttggtcaatttcgtgccagccacaccctggtactgcatgcacgcaatgctagctgcccctttcccgtcctgggcaccccgagtctcccccgaccccgggtcccaggtatgctcccacctccacctgccccactcaccacctctgctagttccagacacctccgagacgaggaaaaaaaaaaaaaaaaaaaaaaaaaaaaaaaaaaaaaaaaaaaaaaaaaaaaaaaaaaaaaaaaaaaaaaaaaaaaaaaaaaaaaaaaaaaaaaaaaaaaaaaaaaaaaaaaaaaaaaaa

SEQ ID NO: 271 - RNA, 9244 nt, synthetic construct
  misc_feature 1..9244: note = mRNA of V30_10xGCN4-dCas9-ZIM3-2a-D3a-hD3L-scFv
  source 1..9244: mol_type = other RNA
aggactcactatttgttttcgcgcccagttgcaaaaagtgtcgacatttgcttctgacacaactgtgttcactagcaacctcaaacagacaccgccaccatgcctgctgctaagagagtgaaactggatggatccgaggaactgctgagcaagaactaccacctggaaaacgaggtggccagactgaagaaaggctctggctctggcggaagcggttctggcggatcaggatctggaagtggcggctctggaagcggaggttctggatctggcgaagaactgctgtctaagaattatcacctcgagaacgaagtggctcggctcaagaaaggcagtggcagcggaggaagtggatccggcggtagtggtagtggaagcggcggatccggctcaggcggatctggttcaggggaagaactcctctccaaaaactaccatctcgagaatgaggtcgcccgcctgaaaaaaggatcaggttccggtggttctggcagcggtggttcaggctcaggcagcggcggtagcggtagcggtggaagcggaagcggagaagaacttctcagcaaaaattaccacttggagaatgaagttgcaagactcaaaaaaggttccggcagtggcggcagcggcagcggcggatctggtagtggatctggtggcagtggttcaggcggaagtggtagcggagaggaattgctctcaaagaactatcatttggagaacgaggttgcacgcttgaagaaaggcagcggatcaggcggatctggcagcggtggatctggttctggatccggcggctccggtagtggtggaagtggctctggggaagaattgcttagcaagaattatcatcttgaaaatgaggttgccaggcttaaaaaaggcagtggctccggcggatccggaagcggaggcagcggatctggatctggtggttcaggatctggcggttctggtagcggggaagaactgttgagtaaaaactatcaccttgagaacgaggtcgcaaggttgaaaaaaggatccggctctggcggctccggaagtggcggatctggctccggtagcggaggatcaggatccggcggaagcggatcaggcgaggaactgctttccaaaaattaccaccttgaaaacgaagtcgcccgcctcaagaaaggttctggcagcggaggctctggcagtggtggtagcggaagtggaagtggtggcagtggtagcggtggatctggaagcggcgaggaactcctgtcaaagaattaccatctcgaaaacgaggtcgcaaggctcaagaaaggctcaggatcaggcggctctggatccggcggttctggttccggctcaggtggaagtggatctggcggctcaggttccggcgaagaattgctttccaagaactaccatttggaaaatgaagtcgctcgtttgaagaaaggttcaggctccggcccaaaaaagaagagaaaggtaatggacaagaagtacagcatcggcctggccatcggcaccaactctgtgggctgggccgtgatcaccgacgagtacaaggtgcccagcaagaaattcaaggtgctgggcaacaccgaccggcacagcatcaagaagaacctgatcggcgccctgctgttcgacagcggagaaacagccgaggccacccggctgaagagaaccgccagaagaagatacaccagacggaagaaccggatctgctatctgcaagagatcttcagcaacgagatggccaaggtggacgacagcttcttccacagactggaagagtccttcctggtggaagaggataagaagcacgagcggcaccccatcttcggcaacatcgtggacgaggtggcctaccacgagaagtaccccaccatctaccacctgagaaagaaactggtggacagcaccgacaaggccgacctgcggctgatctatctggccctggcccacatgatcaagttccggggccacttcctgatcgagggcgacctgaaccccgacaacagcgacgtggacaagctgttcatccagctggtgcagacctacaaccagctgttcgaggaaaaccccatcaacgccagcggcgtggacgccaaggccatcctgtctgccagactgagcaagagcagacggctggaaaatctgatcgcccagctgcccggcgagaagaagaatggcctgttcggcaacctgattgccctgagcctgggcctgacccccaacttcaagagcaacttcgacctggccgaggatgccaaactgcagctgagcaaggacacctacgacgacgacctggacaacctgctggcccagatcggcgaccagtacgccgacctgtttctggccgccaagaacctgtccgacgccatcctgctgagcgacatcctgagagtgaacaccgagatcaccaaggcccccctgagcgcctctatgatcaagagatacgacgagcaccaccaggacctgaccctgctgaaagctctcgtgcggcagcagctgcctgagaagtacaaagagattttcttcgaccagagcaagaacggctacgccggctacatcgatggcggagccagccaggaagagttctacaagttcatcaagcccatcctggaaaagatggacggcaccgaggaactgctcgtgaagctgaacagagaggacctgctgcggaagcagcggaccttcgacaacggcagcatcccccaccagatccacctgggagagctgcacgccattctgcggcggcaggaagatttttacccattcctgaaggacaaccgggaaaagatcgagaagatcctgaccttccgcatcccctactacgtgggccctctggccaggggaaacagcagattcgcctggatgaccagaaagagcgaggaaaccatcaccccctggaacttcgaggaagtggtggacaagggcgccagcgcccagagcttcatcgagcggatgaccaacttcgataagaacctgcccaacgagaaggtgctgcccaagcacagcctgctgtacgagtacttcaccgtgtacaacgagctgaccaaagtgaaatacgtgaccgagggaatgagaaagcccgccttcctgagcggcgagcagaaaaaagccatcgtggacctgctgttcaagaccaaccggaaagtgaccgtgaagcagctgaaagaggactacttcaagaaaatcgagtgcttcgactccgtggaaatctccggcgtggaagatcggttcaacgcctccctgggcacataccacgatctgctgaaaattatcaaggacaaggacttcctggacaatgaggaaaacgaggacattctggaagatatcgtgctgaccctgacactgtttgaggacagagagatgatcgaggaacggctgaaaacctatgcccacctgttcgacgacaaagtgatgaagcagctgaagcggcggagatacaccggctggggcaggctgagccggaagctgatcaacggcatccgggacaagcagtccggcaagacaatcctggatttcctgaagtccgacggcttcgccaacagaaacttcatgcagctgatccacgacgacagcctgacctttaaagaggacatccagaaagcccaggtgtccggccagggcgatagcctgcacgagcacattgccaatctggccggcagccccgccattaagaagggcatcctgcagacagtgaaggtggtggacgagctcgtgaaagtgatgggccggcacaagcccgagaacatcgtgatcgaaatggccagagagaaccagaccacccagaagggacagaagaacagccgcgagagaatgaagcggatcgaagagggcatcaaagagctgggcagccagatcctgaaagaacaccccgtggaaaacacccagctgcagaacgagaagctgtacctgtactacctgcagaatgggcgggatatgtacgtggaccaggaactggacatcaaccggctgtccgactacgatgtggacgctatcgtgcctcagagctttctgaaggacgactccatcgataacaaagtgctgactcggagcgacaagaaccggggcaagagcgacaacgtgccctccgaagaggtcgtgaagaagatgaagaactactggcgccagctgctgaatgccaagctgattacccagaggaagttcgacaatctgaccaaggccgagagaggcggcctgagcgaactggataaggccggcttcatcaagagacagctggtggaaacccggcagatcacaaagcacgtggcacagatcctggactcccggatgaacactaagtacgacgagaacgacaaactgatccgggaagtgaaagtgatcaccctgaagtccaagctggtgtccgatttccggaaggatttccagttttacaaagtgcgcgagatcaacaactaccaccacgcccacgacgcctacctgaacgccgtcgtgggaaccgccctgatcaaaaagtaccctaagctggaaagcgagttcgtgtacggcgactacaaggtgtacgacgtgcggaagatgatcgccaagagcgagcaggaaatcggcaaggctaccgccaagtacttcttctacagcaacatcatgaactttttcaagaccgagattaccctggccaacggcgagatccggaagcggcctctgatcgagacaaacggcgaaacaggcgagatcgtgtgggataagggccgggactttgccaccgtgcggaaagtgctgtctatgccccaagtgaatatcgtgaaaaagaccgaggtgcagacaggcggcttcagcaaagagtctatcctgcccaagaggaacagcgacaagctgatcgccagaaagaaggactgggaccctaagaagtacggcggcttcgacagccccaccgtggcctattctgtgctggtggtggccaaagtggaaaagggcaagtccaagaaactgaagagtgtgaaagagctgctggggatcaccatcatggaaagaagcagcttcgagaagaatcccatcgactttctggaagccaagggctacaaagaagtgaaaaaggacctgatcatcaagctgcctaagtactccctgttcgagctggaaaacggccggaagagaatgctggcctctgccggcgaactgcagaagggaaacgaactggccctgccctccaaatatgtgaacttcctgtacctggccagccactatgagaagctgaagggctcccccgaggataatgagcagaaacagctgtttgtggaacagcacaaacactacctggacgagatcatcgagcagatcagcgagttctccaagagagtgatcctggccgacgctaatctggacaaggtgctgagcgcctacaacaagcacagagacaagcctatcagagagcaggccgagaatatcatccacctgtttaccctgaccaatctgggagcccctgccgccttcaagtactttgacaccaccatcgaccggaagaggtacaccagcaccaaagaggtgctggacgccaccctgatccaccagagcatcaccggcctgtacgagacacggatcgacctgtctcagctgggaggcgacgcctatccctatgacgtgcccgattatgccagcctgggcagcggctcccccaagaaaaaacgcaaggtggaagatcctaagaaaaagcggaaagtggacggcagcggcagcgagacccccggtaccagcgagagcgccacccccgagagcatgaacaattcccagggaagagtgaccttcgaggatgtcactgtgaacttcacccagggggagtggcagcggctgaatcccgaacagagaaacttgtacagggatgtgatgctggagaattacagcaaccttgtctctgtgggacaaggggaaaccaccaaacccgatgtgatcttgaggttggaacaaggaaaggagccatggttggaggaagaggaagtgctgggaagtggccgtgcagaaaaaaatggggacattggagggcagatttggaagccaaaggatgtgaaagagagtctcctcgagggaagcggagctactaacttcagcctgctgaagcaggctggagacgtggaggagaaccctggacctatgcctgctgctaagagagtgaaactggatggatccaaccatgaccaggaatttgaccccccaaaggtttacccacctgtgccagctgagaagaggaagcccatccgcgtgctgtctctctttgatgggattgctacagggctcctggtgctgaaggacctgggcatccaagtggaccgctacattgcctccgaggtgtgtgaggactccatcacggtgggcatggtgcggcaccagggaaagatcatgtacgtcggggacgtccgcagcgtcacacagaagcatatccaggagtggggcccattcgacctggtgattggaggcagtccctgcaatgacctctccattgtcaaccctgcccgcaagggactttatgagggtactggccgcctcttctttgagttctaccgcctcctgcatgatgcgcggcccaaggagggagatgatcgccccttcttctggctctttgagaatgtggtggccatgggcgttagtgacaagagggacatctcgcgatttcttgagtctaaccccgtgatgattgacgccaaagaagtgtctgctgcacacagggcccgttacttctggggtaaccttcctggcatgaacaggcctttggcatccactgtgaatgataagctggagctgcaagagtgtctggagcacggcagaatagccaagttcagcaaagtgaggaccattaccaccaggtcaaactctataaagcagggcaaagaccagcatttccccgtgttcatgaacgagaaggaggacatcctgtggtgcactgaaatggaaagggtgtttggcttccccgtccactacacagacgtctccaacatgagccgcttggcgaggcagagactgctgggccgatcgtggagcgtgccggtcatccgccacctcttcgctccgctgaaggaatattttgcttgtgtgtctagcggcaatagtaacgctaacagccgcgggccgagcttcagcagcggcctggtgccgttaagcttgcgcggcagccatatgttcgaaaccgtgcctgtgtggaggagacagccagtccgggtgctgtccctttttgaagacatcaagaaagagctgacgagtttgggctttttggaaagtggttctgacccgggacaactgaagcatgtggttgatgtcacagacacagtgaggaaggatgtggaggagtggggacccttcgatcttgtgtacggcgccacacctcccctgggccacacctgtgaccgtcctcccagctggtacctgttccagttccaccggctcctgcagtacgcacggcccaagccaggcagccccaggcccttcttctggatgttcgtggacaatctggtgctgaacaaggaagacctggacgtcgcatctcgcttcctggagatggagccagtcaccatcccagatgtccacggcggatccttgcagaatgctgtccgcgtgtggagcaacatcccagccataaggagcagcaggcactgggctctggtttcggaagaagaattgtccctgctggcccagaacaagcagagctcgaagctcgcggccaagtggcccaccaagctggtgaagaactgctttctccccctaagagaatatttcaagtatttttcaggagggccgagctctggcgcacccccaccaagtggagggtctcctgccgggtccccaacatctactgaagaaggcaccagcgaatccgcaacgcccgagtcaggccctggtacctccacagaaccatctgaaggtagtgcgcctggttccccagctggaagccctacttccaccgaagaaggcacgtcaaccgaaccaagtgaaggatctgcccctgggaccagcactgaaccatctgagccaaaaaagaagagaaaggtaccatctgagggccccgacatcgtgatgacccagagccccagcagcctgagcgccagcgtgggcgaccgcgtgaccatcacctgccgcagcagcaccggcgccgtgaccaccagcaactacgccagctgggtgcaggagaagcccggcaagctgttcaagggcctgatcggcggcaccaacaaccgcgcccccggcgtgcccagccgcttcagcggcagcctgatcggcgacaaggccaccctgaccatcagcagcctgcagcccgaggacttcgccacctacttctgcgccctgtggtacagcaaccactgggtgttcggccagggcaccaaggtggagctgaagcgcggcggcggcggcagcggcggcggcggcagcggcggcggcggcagcagcggcggcggcagcgaggtgaagctgctggagagcggcggcggcctggtgcagcccggcggcagcctgaagctgagctgcgccgtgagcggcttcagcctgaccgactacggcgtgaactgggtgcgccaggcccccggccgcggcctggagtggatcggcgtgatctggggcgacggcatcaccgactacaacagcgccctgaaggaccgcttcatcatcagcaaggacaacggcaagaacaccgtgtacctgcagatgagcaaggtgcgcagcgacgacaccgccctgtactactgcgtgaccggcctgttcgactactggggccagggcaccctggtgaccgtgagcagctacccatacgatgttccagattacgctggtggaggcggaggttctgggggaggaggtagtggcggtggtggttcaggaggcggcggaagctgataataggatcccaagcacgcagcaatgcagctcaaaacgcttagcctagccacacccccacgggaaacagcagtgattaacctttagcaataaacgaaagtttaactaagctatactaaccccagggttggtcaatttcgtgccagccacaccctggtactgcatgcacgcaatgctagctgcccctttcccgtcctgggcaccccgagtctcccccgaccccgggtcccaggtatgctcccacctccacctgccccactcaccacctctgctagttccagacacctccgagacgaggaaaaaaaaaaaaaaaaaaaaaaaaaaaaaaaaaaaaaaaaaaaaaaaaaaaaaaaaaaaaaaaaaaaaaaaaaaaaaaaaaaaaaaaaaaaaaaaaaaaaaaaaaaaaaaaaaaaaaaaa

SEQ ID NO: 272 - RNA, 7972 nt, synthetic construct
  misc_feature 1..7972: note = mRNA of V31_scFV-hD3L-D3a-2a-3xGCN4-dCas9-KRAB
  source 1..7972: mol_type = other RNA
aggactcactatttgttttcgcgcccagttgcaaaaagtgtcgacatttgcttctgacacaactgtgttcactagcaacctcaaacagacaccgccaccatgcctgctgctaagagagtgaaactggatggatccggccccgacatcgtgatgacccagagccccagcagcctgagcgccagcgtgggcgaccgcgtgaccatcacctgccgcagcagcaccggcgccgtgaccaccagcaactacgccagctgggtgcaggagaagcccggcaagctgttcaagggcctgatcggcggcaccaacaaccgcgcccccggcgtgcccagccgcttcagcggcagcctgatcggcgacaaggccaccctgaccatcagcagcctgcagcccgaggacttcgccacctacttctgcgccctgtggtacagcaaccactgggtgttcggccagggcaccaaggtggagctgaagcgcggcggcggcggcagcggcggcggcggcagcggcggcggcggcagcagcggcggcggcagcgaggtgaagctgctggagagcggcggcggcctggtgcagcccggcggcagcctgaagctgagctgcgccgtgagcggcttcagcctgaccgactacggcgtgaactgggtgcgccaggcccccggccgcggcctggagtggatcggcgtgatctggggcgacggcatcaccgactacaacagcgccctgaaggaccgcttcatcatcagcaaggacaacggcaagaacaccgtgtacctgcagatgagcaaggtgcgcagcgacgacaccgccctgtactactgcgtgaccggcctgttcgactactggggccagggcaccctggtgaccgtgagcagctacccatacgatgttccagattacgctggtggaggcggaggttctgggggaggaggtagtggcggtggtggttcaggaggcggcggaagcatgttcgaaaccgtgcctgtgtggaggagacagccagtccgggtgctgtccctttttgaagacatcaagaaagagctgacgagtttgggctttttggaaagtggttctgacccgggacaactgaagcatgtggttgatgtcacagacacagtgaggaaggatgtggaggagtggggacccttcgatcttgtgtacggcgccacacctcccctgggccacacctgtgaccgtcctcccagctggtacctgttccagttccaccggctcctgcagtacgcacggcccaagccaggcagccccaggcccttcttctggatgttcgtggacaatctggtgctgaacaaggaagacctggacgtcgcatctcgcttcctggagatggagccagtcaccatcccagatgtccacggcggatccttgcagaatgctgtccgcgtgtggagcaacatcccagccataaggagcagcaggcactgggctctggtttcggaagaagaattgtccctgctggcccagaacaagcagagctcgaagctcgcggccaagtggcccaccaagctggtgaagaactgctttctccccctaagagaatatttcaagtatttttcaacagaactcacttcctctttatctagcggcaatagtaacgctaacagccgcgggccgagcttcagcagcggcctggtgccgttaagcttgcgcggcagccatatgaaccatgaccaggaatttgaccccccaaaggtttacccacctgtgccagctgagaagaggaagcccatccgcgtgctgtctctctttgatgggattgctacagggctcctggtgctgaaggacctgggcatccaagtggaccgctacattgcctccgaggtgtgtgaggactccatcacggtgggcatggtgcggcaccagggaaagatcatgtacgtcggggacgtccgcagcgtcacacagaagcatatccaggagtggggcccattcgacctggtgattggaggcagtccctgcaatgacctctccattgtcaaccctgcccgcaagggactttatgagggtactggccgcctcttctttgagttctaccgcctcctgcatgatgcgcggcccaaggagggagatgatcgccccttcttctggctctttgagaatgtggtggccatgggcgttagtgacaagagggacatctcgcgatttcttgagtctaaccccgtgatgattgacgccaaagaagtgtctgctgcacacagggcccgttacttctggggtaaccttcctggcatgaacaggcctttggcatccactgtgaatgataagctggagctgcaagagtgtctggagcacggcagaatagccaagttcagcaaagtgaggaccattaccaccaggtcaaactctataaagcagggcaaagaccagcatttccccgtcttcatgaacgagaaggaggacatcctgtggtgcactgaaatggaaagggtgtttggcttccccgtccactacacagacgtctccaacatgagccgcttggcgaggcagagactgctgggccgatcgtggagcgtgccggtcatccgccacctcttcgctccgctgaaggaatattttgcttgtgtgggaagcggagctactaacttcagcctgctgaagcaggctggagacgtggaggagaaccctggacctatgcctgctgctaagagagtgaaactggatggatccgaggaactgctgagcaagaactaccacctggaaaacgaggtggccagactgaagaaaggctctggctctggcggaagcggttctggcggatcaggatctggaagtggcggctctggaagcggaggttctggatctggcgaagaactgctgtctaagaattatcacctcgagaacgaagtggctcggctcaagaaaggcagtggcagcggaggaagtggatccggcggtagtggtagtggaagcggcggatccggctcaggcggatctggttcaggggaagaactcctctccaaaaactaccatctcgagaatgaggtcgcccgcctgaaaaaaggatcaggttccggtggttctggcagcggtggttcaggctcaggcagcggcggtagcggtagcggtggaagcggaagcggaccaaaaaagaagagaaaggtaatggacaagaagtacagcatcggcctggccatcggcaccaactctgtgggctgggccgtgatcaccgacgagtacaaggtgcccagcaagaaattcaaggtgctgggcaacaccgaccggcacagcatcaagaagaacctgatcggcgccctgctgttcgacagcggagaaacagccgaggccacccggctgaagagaaccgccagaagaagatacaccagacggaagaaccggatctgctatctgcaagagatcttcagcaacgagatggccaaggtggacgacagcttcttccacagactggaagagtccttcctggtggaagaggataagaagcacgagcggcaccccatcttcggcaacatcgtggacgaggtggcctaccacgagaagtaccccaccatctaccacctgagaaagaaactggtggacagcaccgacaaggccgacctgcggctgatctatctggccctggcccacatgatcaagttccggggccacttcctgatcgagggcgacctgaaccccgacaacagcgacgtggacaagctgttcatccagctggtgcagacctacaaccagctgttcgaggaaaaccccatcaacgccagcggcgtggacgccaaggccatcctgtctgccagactgagcaagagcagacggctggaaaatctgatcgcccagctgcccggcgagaagaagaatggcctgttcggcaacctgattgccctgagcctgggcctgacccccaacttcaagagcaacttcgacctggccgaggatgccaaactgcagctgagcaaggacacctacgacgacgacctggacaacctgctggcccagatcggcgaccagtacgccgacctgtttctggccgccaagaacctgtccgacgccatcctgctgagcgacatcctgagagtgaacaccgagatcaccaaggcccccctgagcgcctctatgatcaagagatacgacgagcaccaccaggacctgaccctgctgaaagctctcgtgcggcagcagctgcctgagaagtacaaagagattttcttcgaccagagcaagaacggctacgccggctacatcgatggcggagccagccaggaagagttctacaagttcatcaagcccatcctggaaaagatggacggcaccgaggaactgctcgtgaagctgaacagagaggacctgctgcggaagcagcggaccttcgacaacggcagcatcccccaccagatccacctgggagagctgcacgccattctgcggcggcaggaagatttttacccattcctgaaggacaaccgggaaaagatcgagaagatcctgaccttccgcatcccctactacgtgggccctctggccaggggaaacagcagattcgcctggatgaccagaaagagcgaggaaaccatcaccccctggaacttcgaggaagtggtggacaagggcgccagcgcccagagcttcatcgagcggatgaccaacttcgataagaacctgcccaacgagaaggtgctgcccaagcacagcctgctgtacgagtacttcaccgtgtacaacgagctgaccaaagtgaaatacgtgaccgagggaatgagaaagcccgccttcctgagcggcgagcagaaaaaagccatcgtggacctgctgttcaagaccaaccggaaagtgaccgtgaagcagctgaaagaggactacttcaagaaaatcgagtgcttcgactccgtggaaatctccggcgtggaagatcggttcaacgcctccctgggcacataccacgatctgctgaaaattatcaaggacaaggacttcctggacaatgaggaaaacgaggacattctggaagatatcgtgctgaccctgacactgtttgaggacagagagatgatcgaggaacggctgaaaacctatgcccacctgttcgacgacaaagtgatgaagcagctgaagcggcggagatacaccggctggggcaggctgagccggaagctgatcaacggcatccgggacaagcagtccggcaagacaatcctggatttcctgaagtccgacggcttcgccaacagaaacttcatgcagctgatccacgacgacagcctgacctttaaagaggacatccagaaagcccaggtgtccggccagggcgatagcctgcacgagcacattgccaatctggccggcagccccgccattaagaagggcatcctgcagacagtgaaggtggtggacgagctcgtgaaagtgatgggccggcacaagcccgagaacatcgtgatcgaaatggccagagagaaccagaccacccagaagggacagaagaacagccgcgagagaatgaagcggatcgaagagggcatcaaagagctgggcagccagatcctgaaagaacaccccgtggaaaacacccagctgcagaacgagaagctgtacctgtactacctgcagaatgggcgggatatgtacgtggaccaggaactggacatcaaccggctgtccgactacgatgtggacgctatcgtgcctcagagctttctgaaggacgactccatcgataacaaagtgctgactcggagcgacaagaaccggggcaagagcgacaacgtgccctccgaagaggtcgtgaagaagatgaagaactactggcgccagctgctgaatgccaagctgattacccagaggaagttcgacaatctgaccaaggccgagagaggcggcctgagcgaactggataaggccggcttcatcaagagacagctggtggaaacccggcagatcacaaagcacgtggcacagatcctggactcccggatgaacactaagtacgacgagaacgacaaactgatccgggaagtgaaagtgatcaccctgaagtccaagctggtgtccgatttccggaaggatttccagttttacaaagtgcgcgagatcaacaactaccaccacgcccacgacgcctacctgaacgccgtcgtgggaaccgccctgatcaaaaagtaccctaagctggaaagcgagttcgtgtacggcgactacaaggtgtacgacgtgcggaagatgatcgccaagagcgagcaggaaatcggcaaggctaccgccaagtacttcttctacagcaacatcatgaactttttcaagaccgagattaccctggccaacggcgagatccggaagcggcctctgatcgagacaaacggcgaaacaggcgagatcgtgtgggataagggccgggactttgccaccgtgcggaaagtgctgtctatgccccaagtgaatatcgtgaaaaagaccgaggtgcagacaggcggcttcagcaaagagtctatcctgcccaagaggaacagcgacaagctgatcgccagaaagaaggactgggaccctaagaagtacggcggcttcgacagccccaccgtggcctattctgtgctggtggtggccaaagtggaaaagggcaagtccaagaaactgaagagtgtgaaagagctgctggggatcaccatcatggaaagaagcagcttcgagaagaatcccatcgactttctggaagccaagggctacaaagaagtgaaaaaggacctgatcatcaagctgcctaagtactccctgttcgagctggaaaacggccggaagagaatgctggcctctgccggcgaactgcagaagggaaacgaactggccctgccctccaaatatgtgaacttcctgtacctggccagccactatgagaagctgaagggctcccccgaggataatgagcagaaacagctgtttgtggaacagcacaaacactacctggacgagatcatcgagcagatcagcgagttctccaagagagtgatcctggccgacgctaatctggacaaggtgctgagcgcctacaacaagcacagagacaagcctatcagagagcaggccgagaatatcatccacctgtttaccctgaccaatctgggagcccctgccgccttcaagtactttgacaccaccatcgaccggaagaggtacaccagcaccaaagaggtgctggacgccaccctgatccaccagagcatcaccggcctgtacgagacacggatcgacctgtctcagctgggaggcgacgcctatccctatgacgtgcccgattatgccagcctgggcagcggctcccccaagaaaaaacgcaaggtggaagatcctaagaaaaagcggaaagtggacggcagcggcagcgagacccccggtaccagcgagagcgccacccccgagagccggacactggtgaccttcaaggatgtatttgtggacttcaccagggaggagtggaagctgctggacactgctcagcagatcgtgtacagaaatgtgatgctggagaactataagaacctggtttccttgggttatcagcttactaagccagatgtgatcctccggttggagaagggagaagagccctgagatcccaagcacgcagcaatgcagctcaaaacgcttagcctagccacacccccacgggaaacagcagtgattaacctttagcaataaacgaaagtttaactaagctatactaaccccagggttggtcaatttcgtgccagccacaccctggtactgcatgcacgcaatgctagctgcccctttcccgtcctgggcaccccgagtctcccccgaccccgggtcccaggtatgctcccacctccacctgccccactcaccacctctgctagttccagacacctccgagacgaggaaaaaaaaaaaaaaaaaaaaaaaaaaaaaaaaaaaaaaaaaaaaaaaaaaaaaaaaaaaaaaaaaaaaaaaaaaaaaaaaaaaaaaaaaaaaaaaaaaaaaaaaaaaaaaaaaaaaaaaa

SEQ ID NO: 273 - RNA, 7996 nt, synthetic construct
  misc_feature 1..7996: note = mRNA of V32_1xGCN4-ZIM3-2a-D3a-hD3L-dCas9-scFv
  source 1..7996: mol_type = other RNA
aggactcactatttgttttcgcgcccagttgcaaaaagtgtcgacatttgcttctgacacaactgtgttcactagcaacctcaaacagacaccgccaccatgcctgctgctaagagagtgaaactggatggatccgaggaactgctgagcaagaactaccacctggaaaacgaggtggccagactgaagaaaggctctggctctggcggaagcggttctggcggatcaggatctggaagtggcggctctggaagcggaggttctggatctggcatgaacaattcccagggaagagtgaccttcgaggacgtgaccgtgaacttcacccaaggcgagtggcagagactgaaccccgagcagagaaacctgtaccgggacgtgatgctggaaaactacagcaacctggtgtccgtcggccagggcgagacaacaaagcctgacgtgatcctgcggctggaacagggcaaagagccttggctggaagaggaagaggtgctcggatctggcagagccgagaagaatggcgatatcggcggacagatctggaagccaaaggatgtgaaagagagtctcggaagcggagctactaacttcagcctgctgaagcaggctggagacgtggaggagaaccctggacctatgcctgctgctaagagagtgaaactggatggatccaaccatgaccaggaatttgaccccccaaaggtttacccacctgtgccagctgagaagaggaagcccatccgcgtgctgtctctctttgatgggattgctacagggctcctggtgctgaaggacctgggcatccaagtggaccgctacattgcctccgaggtgtgtgaggactccatcacggtgggcatggtgcggcaccagggaaagatcatgtacgtcggggacgtccgcagcgtcacacagaagcatatccaggagtggggcccattcgacctggtgattggaggcagtccctgcaatgacctctccattgtcaaccctgcccgcaagggactttatgagggtactggccgcctcttctttgagttctaccgcctcctgcatgatgcgcggcccaaggagggagatgatcgccccttcttctggctctttgagaatgtggtggccatgggcgttagtgacaagagggacatctcgcgatttcttgagtctaaccccgtgatgattgacgccaaagaagtgtctgctgcacacagggcccgttacttctggggtaaccttcctggcatgaacaggcctttggcatccactgtgaatgataagctggagctgcaagagtgtctggagcacggcagaatagccaagttcagcaaagtgaggaccattaccaccaggtcaaactctataaagcagggcaaagaccagcatttccccgtgttcatgaacgagaaggaggacatcctgtggtgcactgaaatggaaagggtgtttggcttccccgtccactacacagacgtctccaacatgagccgcttggcgaggcagagactgctgggccgatcgtggagcgtgccggtcatccgccacctcttcgctccgctgaaggaatattttgcttgtgtgtctagcggcaatagtaacgctaacagccgcgggccgagcttcagcagcggcctggtgccgttaagcttgcgcggcagccatatgttcgaaaccgtgcctgtgtggaggagacagccagtccgggtgctgtccctttttgaagacatcaagaaagagctgacgagtttgggctttttggaaagtggttctgacccgggacaactgaagcatgtggttgatgtcacagacacagtgaggaaggatgtggaggagtggggacccttcgatcttgtgtacggcgccacacctcccctgggccacacctgtgaccgtcctcccagctggtacctgttccagttccaccggctcctgcagtacgcacggcccaagccaggcagccccaggcccttcttctggatgttcgtggacaatctggtgctgaacaaggaagacctggacgtcgcatctcgcttcctggagatggagccagtcaccatcccagatgtccacggcggatccttgcagaatgctgtccgcgtgtggagcaacatcccagccataaggagcagcaggcactgggctctggtttcggaagaagaattgtccctgctggcccagaacaagcagagctcgaagctcgcggccaagtggcccaccaagctggtgaagaactgctttctccccctaagagaatatttcaagtatttttcaggagggccgagctctggcgcacccccaccaagtggagggtctcctgccgggtccccaacatctactgaagaaggcaccagcgaatccgcaacgcccgagtcaggccctggtacctccacagaaccatctgaaggtagtgcgcctggttccccagctggaagccctacttccaccgaagaaggcacgtcaaccgaaccaagtgaaggatctgcccctgggaccagcactgaaccatctgagccaaaaaagaagagaaaggtaatggacaagaagtacagcatcggcctggccatcggcaccaactctgtgggctgggccgtgatcaccgacgagtacaaggtgcccagcaagaaattcaaggtgctgggcaacaccgaccggcacagcatcaagaagaacctgatcggcgccctgctgttcgacagcggagaaacagccgaggccacccggctgaagagaaccgccagaagaagatacaccagacggaagaaccggatctgctatctgcaagagatcttcagcaacgagatggccaaggtggacgacagcttcttccacagactggaagagtccttcctggtggaagaggataagaagcacgagcggcaccccatcttcggcaacatcgtggacgaggtggcctaccacgagaagtaccccaccatctaccacctgagaaagaaactggtggacagcaccgacaaggccgacctgcggctgatctatctggccctggcccacatgatcaagttccggggccacttcctgatcgagggcgacctgaaccccgacaacagcgacgtggacaagctgttcatccagctggtgcagacctacaaccagctgttcgaggaaaaccccatcaacgccagcggcgtggacgccaaggccatcctgtctgccagactgagcaagagcagacggctggaaaatctgatcgcccagctgcccggcgagaagaagaatggcctgttcggcaacctgattgccctgagcctgggcctgacccccaacttcaagagcaacttcgacctggccgaggatgccaaactgcagctgagcaaggacacctacgacgacgacctggacaacctgctggcccagatcggcgaccagtacgccgacctgtttctggccgccaagaacctgtccgacgccatcctgctgagcgacatcctgagagtgaacaccgagatcaccaaggcccccctgagcgcctctatgatcaagagatacgacgagcaccaccaggacctgaccctgctgaaagctctcgtgcggcagcagctgcctgagaagtacaaagagattttcttcgaccagagcaagaacggctacgccggctacatcgatggcggagccagccaggaagagttctacaagttcatcaagcccatcctggaaaagatggacggcaccgaggaactgctcgtgaagctgaacagagaggacctgctgcggaagcagcggaccttcgacaacggcagcatcccccaccagatccacctgggagagctgcacgccattctgcggcggcaggaagatttttacccattcctgaaggacaaccgggaaaagatcgagaagatcctgaccttccgcatcccctactacgtgggccctctggccaggggaaacagcagattcgcctggatgaccagaaagagcgaggaaaccatcaccccctggaacttcgaggaagtggtggacaagggcgccagcgcccagagcttcatcgagcggatgaccaacttcgataagaacctgcccaacgagaaggtgctgcccaagcacagcctgctgtacgagtacttcaccgtgtacaacgagctgaccaaagtgaaatacgtgaccgagggaatgagaaagcccgccttcctgagcggcgagcagaaaaaagccatcgtggacctgctgttcaagaccaaccggaaagtgaccgtgaagcagctgaaagaggactacttcaagaaaatcgagtgcttcgactccgtggaaatctccggcgtggaagatcggttcaacgcctccctgggcacataccacgatctgctgaaaattatcaaggacaaggacttcctggacaatgaggaaaacgaggacattctggaagatatcgtgctgaccctgacactgtttgaggacagagagatgatcgaggaacggctgaaaacctatgcccacctgttcgacgacaaagtgatgaagcagctgaagcggcggagatacaccggctggggcaggctgagccggaagctgatcaacggcatccgggacaagcagtccggcaagacaatcctggatttcctgaagtccgacggcttcgccaacagaaacttcatgcagctgatccacgacgacagcctgacctttaaagaggacatccagaaagcccaggtgtccggccagggcgatagcctgcacgagcacattgccaatctggccggcagccccgccattaagaagggcatcctgcagacagtgaaggtggtggacgagctcgtgaaagtgatgggccggcacaagcccgagaacatcgtgatcgaaatggccagagagaaccagaccacccagaagggacagaagaacagccgcgagagaatgaagcggatcgaagagggcatcaaagagctgggcagccagatcctgaaagaacaccccgtggaaaacacccagctgcagaacgagaagctgtacctgtactacctgcagaatgggcgggatatgtacgtggaccaggaactggacatcaaccggctgtccgactacgatgtggacgctatcgtgcctcagagctttctgaaggacgactccatcgataacaaagtgctgactcggagcgacaagaaccggggcaagagcgacaacgtgccctccgaagaggtcgtgaagaagatgaagaactactggcgccagctgctgaatgccaagctgattacccagaggaagttcgacaatctgaccaaggccgagagaggcggcctgagcgaactggataaggccggcttcatcaagagacagctggtggaaacccggcagatcacaaagcacgtggcacagatcctggactcccggatgaacactaagtacgacgagaacgacaaactgatccgggaagtgaaagtgatcaccctgaagtccaagctggtgtccgatttccggaaggatttccagttttacaaagtgcgcgagatcaacaactaccaccacgcccacgacgcctacctgaacgccgtcgtgggaaccgccctgatcaaaaagtaccctaagctggaaagcgagttcgtgtacggcgactacaaggtgtacgacgtgcggaagatgatcgccaagagcgagcaggaaatcggcaaggctaccgccaagtacttcttctacagcaacatcatgaactttttcaagaccgagattaccctggccaacggcgagatccggaagcggcctctgatcgagacaaacggcgaaacaggcgagatcgtgtgggataagggccgggactttgccaccgtgcggaaagtgctgtctatgccccaagtgaatatcgtgaaaaagaccgaggtgcagacaggcggcttcagcaaagagtctatcctgcccaagaggaacagcgacaagctgatcgccagaaagaaggactgggaccctaagaagtacggcggcttcgacagccccaccgtggcctattctgtgctggtggtggccaaagtggaaaagggcaagtccaagaaactgaagagtgtgaaagagctgctggggatcaccatcatggaaagaagcagcttcgagaagaatcccatcgactttctggaagccaagggctacaaagaagtgaaaaaggacctgatcatcaagctgcctaagtactccctgttcgagctggaaaacggccggaagagaatgctggcctctgccggcgaactgcagaagggaaacgaactggccctgccctccaaatatgtgaacttcctgtacctggccagccactatgagaagctgaagggctcccccgaggataatgagcagaaacagctgtttgtggaacagcacaaacactacctggacgagatcatcgagcagatcagcgagttctccaagagagtgatcctggccgacgctaatctggacaaggtgctgagcgcctacaacaagcacagagacaagcctatcagagagcaggccgagaatatcatccacctgtttaccctgaccaatctgggagcccctgccgccttcaagtactttgacaccaccatcgaccggaagaggtacaccagcaccaaagaggtgctggacgccaccctgatccaccagagcatcaccggcctgtacgagacacggatcgacctgtctcagctgggaggcgacgcctatccctatgacgtgcccgattatgccagcctgggcagcggctcccccaagaaaaaacgcaaggtggaagatcctaagaaaaagcggaaagtggacggcattggtagtgggagcggccccgacatcgtgatgacccagagccccagcagcctgagcgccagcgtgggcgaccgcgtgaccatcacctgccgcagcagcaccggcgccgtgaccaccagcaactacgccagctgggtgcaggagaagcccggcaagctgttcaagggcctgatcggcggcaccaacaaccgcgcccccggcgtgcccagccgcttcagcggcagcctgatcggcgacaaggccaccctgaccatcagcagcctgcagcccgaggacttcgccacctacttctgcgccctgtggtacagcaaccactgggtgttcggccagggcaccaaggtggagctgaagcgcggcggcggcggcagcggcggcggcggcagcggcggcggcggcagcagcggcggcggcagcgaggtgaagctgctggagagcggcggcggcctggtgcagcccggcggcagcctgaagctgagctgcgccgtgagcggcttcagcctgaccgactacggcgtgaactgggtgcgccaggcccccggccgcggcctggagtggatcggcgtgatctggggcgacggcatcaccgactacaacagcgccctgaaggaccgcttcatcatcagcaaggacaacggcaagaacaccgtgtacctgcagatgagcaaggtgcgcagcgacgacaccgccctgtactactgcgtgaccggcctgttcgactactggggccagggcaccctggtgaccgtgagcagctacccatacgatgttccagattacgctggtggaggcggaggttctgggggaggaggtagtggcggtggtggttcaggaggcggcggaagctagtgagatcccaagcacgcagcaatgcagctcaaaacgcttagcctagccacacccccacgggaaacagcagtgattaacctttagcaataaacgaaagtttaactaagctatactaaccccagggttggtcaatttcgtgccagccacaccctggtactgcatgcacgcaatgctagctgcccctttcccgtcctgggcaccccgagtctcccccgaccccgggtcccaggtatgctcccacctccacctgccccactcaccacctctgctagttccagacacctccgagacgaggaaaaaaaaaaaaaaaaaaaaaaaaaaaaaaaaaaaaaaaaaaaaaaaaaaaaaaaaaaaaaaaaaaaaaaaaaaaaaaaaaaaaaaaaaaaaaaaaaaaaaaaaaaaaaaaaaaaaaaaa

SEQ ID NO: 274 - RNA, 7894 nt, synthetic construct
  misc_feature 1..7894: note = mRNA of V33_KRAB-1xGCN4-2a-D3a-hD3l-dCas9-scFv
  source 1..7894: mol_type = other RNA
aggactcactatttgttttcgcgcccagttgcaaaaagtgtcgacatttgcttctgacacaactgtgttcactagcaacctcaaacagacaccgccaccatgcctgctgctaagagagtgaaactggatggatcccggacactggtgaccttcaaggatgtatttgtggacttcaccagggaggagtggaagctgctggacactgctcagcagatcgtgtacagaaatgtgatgctggagaactataagaacctggtttccttgggttatcagcttactaagccagatgtgatcctccggttggagaagggagaagagcccggaagcggaatggaggaactgctgagcaagaactaccacctggaaaacgaggtggccagactgaagaaaggctctggctctggcggaagcggttctggcggatcaggatctggaagtggcggctctggaagcggaggttctggatctggcggaagcggagctactaacttcagcctgctgaagcaggctggagacgtggaggagaaccctggacctatgcctgctgctaagagagtgaaactggatggatccaaccatgaccaggaatttgaccccccaaaggtttacccacctgtgccagctgagaagaggaagcccatccgcgtgctgtctctctttgatgggattgctacagggctcctggtgctgaaggacctgggcatccaagtggaccgctacattgcctccgaggtgtgtgaggactccatcacggtgggcatggtgcggcaccagggaaagatcatgtacgtcggggacgtccgcagcgtcacacagaagcatatccaggagtggggcccattcgacctggtgattggaggcagtccctgcaatgacctctccattgtcaaccctgcccgcaagggactttatgagggtactggccgcctcttctttgagttctaccgcctcctgcatgatgcgcggcccaaggagggagatgatcgccccttcttctggctctttgagaatgtggtggccatgggcgttagtgacaagagggacatctcgcgatttcttgagtctaaccccgtgatgattgacgccaaagaagtgtctgctgcacacagggcccgttacttctggggtaaccttcctggcatgaacaggcctttggcatccactgtgaatgataagctggagctgcaagagtgtctggagcacggcagaatagccaagttcagcaaagtgaggaccattaccaccaggtcaaactctataaagcagggcaaagaccagcatttccccgtgttcatgaacgagaaggaggacatcctgtggtgcactgaaatggaaagggtgtttggcttccccgtccactacacagacgtctccaacatgagccgcttggcgaggcagagactgctgggccgatcgtggagcgtgccggtcatccgccacctcttcgctccgctgaaggaatattttgcttgtgtgtctagcggcaatagtaacgctaacagccgcgggccgagcttcagcagcggcctggtgccgttaagcttgcgcggcagccatatgttcgaaaccgtgcctgtgtggaggagacagccagtccgggtgctgtccctttttgaagacatcaagaaagagctgacgagtttgggctttttggaaagtggttctgacccgggacaactgaagcatgtggttgatgtcacagacacagtgaggaaggatgtggaggagtggggacccttcgatcttgtgtacggcgccacacctcccctgggccacacctgtgaccgtcctcccagctggtacctgttccagttccaccggctcctgcagtacgcacggcccaagccaggcagccccaggcccttcttctggatgttcgtggacaatctggtgctgaacaaggaagacctggacgtcgcatctcgcttcctggagatggagccagtcaccatcccagatgtccacggcggatccttgcagaatgctgtccgcgtgtggagcaacatcccagccataaggagcagcaggcactgggctctggtttcggaagaagaattgtccctgctggcccagaacaagcagagctcgaagctcgcggccaagtggcccaccaagctggtgaagaactgctttctccccctaagagaatatttcaagtatttttcaggagggccgagctctggcgcacccccaccaagtggagggtctcctgccgggtccccaacatctactgaagaaggcaccagcgaatccgcaacgcccgagtcaggccctggtacctccacagaaccatctgaaggtagtgcgcctggttccccagctggaagccctacttccaccgaagaaggcacgtcaaccgaaccaagtgaaggatctgcccctgggaccagcactgaaccatctgagccaaaaaagaagagaaaggtaatggacaagaagtacagcatcggcctggccatcggcaccaactctgtgggctgggccgtgatcaccgacgagtacaaggtgcccagcaagaaattcaaggtgctgggcaacaccgaccggcacagcatcaagaagaacctgatcggcgccctgctgttcgacagcggagaaacagccgaggccacccggctgaagagaaccgccagaagaagatacaccagacggaagaaccggatctgctatctgcaagagatcttcagcaacgagatggccaaggtggacgacagcttcttccacagactggaagagtccttcctggtggaagaggataagaagcacgagcggcaccccatcttcggcaacatcgtggacgaggtggcctaccacgagaagtaccccaccatctaccacctgagaaagaaactggtggacagcaccgacaaggccgacctgcggctgatctatctggccctggcccacatgatcaagttccggggccacttcctgatcgagggcgacctgaaccccgacaacagcgacgtggacaagctgttcatccagctggtgcagacctacaaccagctgttcgaggaaaaccccatcaacgccagcggcgtggacgccaaggccatcctgtctgccagactgagcaagagcagacggctggaaaatctgatcgcccagctgcccggcgagaagaagaatggcctgttcggcaacctgattgccctgagcctgggcctgacccccaacttcaagagcaacttcgacctggccgaggatgccaaactgcagctgagcaaggacacctacgacgacgacctggacaacctgctggcccagatcggcgaccagtacgccgacctgtttctggccgccaagaacctgtccgacgccatcctgctgagcgacatcctgagagtgaacaccgagatcaccaaggcccccctgagcgcctctatgatcaagagatacgacgagcaccaccaggacctgaccctgctgaaagctctcgtgcggcagcagctgcctgagaagtacaaagagattttcttcgaccagagcaagaacggctacgccggctacatcgatggcggagccagccaggaagagttctacaagttcatcaagcccatcctggaaaagatggacggcaccgaggaactgctcgtgaagctgaacagagaggacctgctgcggaagcagcggaccttcgacaacggcagcatcccccaccagatccacctgggagagctgcacgccattctgcggcggcaggaagatttttacccattcctgaaggacaaccgggaaaagatcgagaagatcctgaccttccgcatcccctactacgtgggccctctggccaggggaaacagcagattcgcctggatgaccagaaagagcgaggaaaccatcaccccctggaacttcgaggaagtggtggacaagggcgccagcgcccagagcttcatcgagcggatgaccaacttcgataagaacctgcccaacgagaaggtgctgcccaagcacagcctgctgtacgagtacttcaccgtgtacaacgagctgaccaaagtgaaatacgtgaccgagggaatgagaaagcccgccttcctgagcggcgagcagaaaaaagccatcgtggacctgctgttcaagaccaaccggaaagtgaccgtgaagcagctgaaagaggactacttcaagaaaatcgagtgcttcgactccgtggaaatctccggcgtggaagatcggttcaacgcctccctgggcacataccacgatctgctgaaaattatcaaggacaaggacttcctggacaatgaggaaaacgaggacattctggaagatatcgtgctgaccctgacactgtttgaggacagagagatgatcgaggaacggctgaaaacctatgcccacctgttcgacgacaaagtgatgaagcagctgaagcggcggagatacaccggctggggcaggctgagccggaagctgatcaacggcatccgggacaagcagtccggcaagacaatcctggatttcctgaagtccgacggcttcgccaacagaaacttcatgcagctgatccacgacgacagcctgacctttaaagaggacatccagaaagcccaggtgtccggccagggcgatagcctgcacgagcacattgccaatctggccggcagccccgccattaagaagggcatcctgcagacagtgaaggtggtggacgagctcgtgaaagtgatgggccggcacaagcccgagaacatcgtgatcgaaatggccagagagaaccagaccacccagaagggacagaagaacagccgcgagagaatgaagcggatcgaagagggcatcaaagagctgggcagccagatcctgaaagaacaccccgtggaaaacacccagctgcagaacgagaagctgtacctgtactacctgcagaatgggcgggatatgtacgtggaccaggaactggacatcaaccggctgtccgactacgatgtggacgctatcgtgcctcagagctttctgaaggacgactccatcgataacaaagtgctgactcggagcgacaagaaccggggcaagagcgacaacgtgccctccgaagaggtcgtgaagaagatgaagaactactggcgccagctgctgaatgccaagctgattacccagaggaagttcgacaatctgaccaaggccgagagaggcggcctgagcgaactggataaggccggcttcatcaagagacagctggtggaaacccggcagatcacaaagcacgtggcacagatcctggactcccggatgaacactaagtacgacgagaacgacaaactgatccgggaagtgaaagtgatcaccctgaagtccaagctggtgtccgatttccggaaggatttccagttttacaaagtgcgcgagatcaacaactaccaccacgcccacgacgcctacctgaacgccgtcgtgggaaccgccctgatcaaaaagtaccctaagctggaaagcgagttcgtgtacggcgactacaaggtgtacgacgtgcggaagatgatcgccaagagcgagcaggaaatcggcaaggctaccgccaagtacttcttctacagcaacatcatgaactttttcaagaccgagattaccctggccaacggcgagatccggaagcggcctctgatcgagacaaacggcgaaacaggcgagatcgtgtgggataagggccgggactttgccaccgtgcggaaagtgctgtctatgccccaagtgaatatcgtgaaaaagaccgaggtgcagacaggcggcttcagcaaagagtctatcctgcccaagaggaacagcgacaagctgatcgccagaaagaaggactgggaccctaagaagtacggcggcttcgacagccccaccgtggcctattctgtgctggtggtggccaaagtggaaaagggcaagtccaagaaactgaagagtgtgaaagagctgctggggatcaccatcatggaaagaagcagcttcgagaagaatcccatcgactttctggaagccaagggctacaaagaagtgaaaaaggacctgatcatcaagctgcctaagtactccctgttcgagctggaaaacggccggaagagaatgctggcctctgccggcgaactgcagaagggaaacgaactggccctgccctccaaatatgtgaacttcctgtacctggccagccactatgagaagctgaagggctcccccgaggataatgagcagaaacagctgtttgtggaacagcacaaacactacctggacgagatcatcgagcagatcagcgagttctccaagagagtgatcctggccgacgctaatctggacaaggtgctgagcgcctacaacaagcacagagacaagcctatcagagagcaggccgagaatatcatccacctgtttaccctgaccaatctgggagcccctgccgccttcaagtactttgacaccaccatcgaccggaagaggtacaccagcaccaaagaggtgctggacgccaccctgatccaccagagcatcaccggcctgtacgagacacggatcgacctgtctcagctgggaggcgacgcctatccctatgacgtgcccgattatgccagcctgggcagcggctcccccaagaaaaaacgcaaggtggaagatcctaagaaaaagcggaaagtggacggcattggtagtgggagcggccccgacatcgtgatgacccagagccccagcagcctgagcgccagcgtgggcgaccgcgtgaccatcacctgccgcagcagcaccggcgccgtgaccaccagcaactacgccagctgggtgcaggagaagcccggcaagctgttcaagggcctgatcggcggcaccaacaaccgcgcccccggcgtgcccagccgcttcagcggcagcctgatcggcgacaaggccaccctgaccatcagcagcctgcagcccgaggacttcgccacctacttctgcgccctgtggtacagcaaccactgggtgttcggccagggcaccaaggtggagctgaagcgcggcggcggcggcagcggcggcggcggcagcggcggcggcggcagcagcggcggcggcagcgaggtgaagctgctggagagcggcggcggcctggtgcagcccggcggcagcctgaagctgagctgcgccgtgagcggcttcagcctgaccgactacggcgtgaactgggtgcgccaggcccccggccgcggcctggagtggatcggcgtgatctggggcgacggcatcaccgactacaacagcgccctgaaggaccgcttcatcatcagcaaggacaacggcaagaacaccgtgtacctgcagatgagcaaggtgcgcagcgacgacaccgccctgtactactgcgtgaccggcctgttcgactactggggccagggcaccctggtgaccgtgagcagctacccatacgatgttccagattacgctggtggaggcggaggttctgggggaggaggtagtggcggtggtggttcaggaggcggcggaagctagtgagatcccaagcacgcagcaatgcagctcaaaacgcttagcctagccacacccccacgggaaacagcagtgattaacctttagcaataaacgaaagtttaactaagctatactaaccccagggttggtcaatttcgtgccagccacaccctggtactgcatgcacgcaatgctagctgcccctttcccgtcctgggcaccccgagtctcccccgaccccgggtcccaggtatgctcccacctccacctgccccactcaccacctctgctagttccagacacctccgagacgaggaaaaaaaaaaaaaaaaaaaaaaaaaaaaaaaaaaaaaaaaaaaaaaaaaaaaaaaaaaaaaaaaaaaaaaaaaaaaaaaaaaaaaaaaaaaaaaaaaaaaaaaaaaaaaaaaaaaaaaaa

SEQ ID NO: 275 - RNA, 7912 nt, synthetic construct
  misc_feature 1..7912: note = mRNA of V34_D3a-D3l-1xGCN4-2a-scFv-dCas9-KRAB
  source 1..7912: mol_type = other RNA
aggactcactatttgttttcgcgcccagttgcaaaaagtgtcgacatttgcttctgacacaactgtgttcactagcaacctcaaacagacaccgccaccatgcctgctgctaagagagtgaaactggatggatccaaccatgaccaggaatttgaccccccaaaggtttacccacctgtgccagctgagaagaggaagcccatccgcgtgctgtctctctttgatgggattgctacagggctcctggtgctgaaggacctgggcatccaagtggaccgctacattgcctccgaggtgtgtgaggactccatcacggtgggcatggtgcggcaccagggaaagatcatgtacgtcggggacgtccgcagcgtcacacagaagcatatccaggagtggggcccattcgacctggtgattggaggcagtccctgcaatgacctctccattgtcaaccctgcccgcaagggactttatgagggtactggccgcctcttctttgagttctaccgcctcctgcatgatgcgcggcccaaggagggagatgatcgccccttcttctggctctttgagaatgtggtggccatgggcgttagtgacaagagggacatctcgcgatttcttgagtctaaccccgtgatgattgacgccaaagaagtgtctgctgcacacagggcccgttacttctggggtaaccttcctggcatgaacaggcctttggcatccactgtgaatgataagctggagctgcaagagtgtctggagcacggcagaatagccaagttcagcaaagtgaggaccattaccaccaggtcaaactctataaagcagggcaaagaccagcatttccccgtgttcatgaacgagaaggaggacatcctgtggtgcactgaaatggaaagggtgtttggcttccccgtccactacacagacgtctccaacatgagccgcttggcgaggcagagactgctgggccgatcgtggagcgtgccggtcatccgccacctcttcgctccgctgaaggaatattttgcttgtgtgtctagcggcaatagtaacgctaacagccgcgggccgagcttcagcagcggcctggtgccgttaagcttgcgcggcagccatatgggccctatggagatatacaagacagtgtctgcatggaagagacagccagtgcgggtactgagcctcttcagaaacatcgacaaggtactaaagagtttgggcttcttggaaagcggttctggttctgggggaggaacgctgaagtacgtggaagatgtcacaaatgtcgtgaggagagacgtggagaaatggggcccctttgacctggtgtacggctcgacgcagcccctaggcagctcttgtgatcgctgtcccggctggtacatgttccagttccaccggatcctgcagtatgcgctgcctcgccaggagagtcagcggcccttcttctggatattcatggacaatctgctgctgactgaggatgaccaagagacaactacccgcttccttcagacagaggctgtgaccctccaggatgtccgtggcagagactaccagaatgctatgcgggtgtggagcaacattccagggctgaagagcaagcatgcgcccctgaccccaaaggaagaagagtatctgcaagcccaagtcagaagcaggagcaagctggacgccccgaaagttgacctcctggtgaagaactgccttctcccgctgagagagtacttcaagtatttttctcaaaactcacttcctcttggagggccgagctctggcgcacccccaccaagtggagggtctcctgccgggtccccaacatctactgaagaaggcaccagcgaatccgcaacgggcagtggcagcggaggaagtggatccggcggtagtggtagtggaagcggcggatccggctcaggcggatctggttcaggggaagaactcctctccaaaaactaccatctcgagaatgaggtcgcccgcctgaaaaaaggatcaggttccggtggttctggcagcggtggttcaggctcaggcagcggcggtagcggtagcggtggaagcggaagcggaccaaaaaagaagagaaaggtaggaagcggagctactaacttcagcctgctgaagcaggctggagacgtggaggagaaccctggacctatgcctgctgctaagagagtgaaactggatggatccggccccgacatcgtgatgacccagagccccagcagcctgagcgccagcgtgggcgaccgcgtgaccatcacctgccgcagcagcaccggcgccgtgaccaccagcaactacgccagctgggtgcaggagaagcccggcaagctgttcaagggcctgatcggcggcaccaacaaccgcgcccccggcgtgcccagccgcttcagcggcagcctgatcggcgacaaggccaccctgaccatcagcagcctgcagcccgaggacttcgccacctacttctgcgccctgtggtacagcaaccactgggtgttcggccagggcaccaaggtggagctgaagcgcggcggcggcggcagcggcggcggcggcagcggcggcggcggcagcagcggcggcggcagcgaggtgaagctgctggagagcggcggcggcctggtgcagcccggcggcagcctgaagctgagctgcgccgtgagcggcttcagcctgaccgactacggcgtgaactgggtgcgccaggcccccggccgcggcctggagtggatcggcgtgatctggggcgacggcatcaccgactacaacagcgccctgaaggaccgcttcatcatcagcaaggacaacggcaagaacaccgtgtacctgcagatgagcaaggtgcgcagcgacgacaccgccctgtactactgcgtgaccggcctgttcgactactggggccagggcaccctggtgaccgtgagcagctacccatacgatgttccagattacgctggtggaggcggaggttctgggggaggaggtagtggcggtggtggttcaggaggcggcggaagcggaagcggaccaaaaaagaagagaaaggtaatggacaagaagtacagcatcggcctggccatcggcaccaactctgtgggctgggccgtgatcaccgacgagtacaaggtgcccagcaagaaattcaaggtgctgggcaacaccgaccggcacagcatcaagaagaacctgatcggcgccctgctgttcgacagcggagaaacagccgaggccacccggctgaagagaaccgccagaagaagatacaccagacggaagaaccggatctgctatctgcaagagatcttcagcaacgagatggccaaggtggacgacagcttcttccacagactggaagagtccttcctggtggaagaggataagaagcacgagcggcaccccatcttcggcaacatcgtggacgaggtggcctaccacgagaagtaccccaccatctaccacctgagaaagaaactggtggacagcaccgacaaggccgacctgcggctgatctatctggccctggcccacatgatcaagttccggggccacttcctgatcgagggcgacctgaaccccgacaacagcgacgtggacaagctgttcatccagctggtgcagacctacaaccagctgttcgaggaaaaccccatcaacgccagcggcgtggacgccaaggccatcctgtctgccagactgagcaagagcagacggctggaaaatctgatcgcccagctgcccggcgagaagaagaatggcctgttcggcaacctgattgccctgagcctgggcctgacccccaacttcaagagcaacttcgacctggccgaggatgccaaactgcagctgagcaaggacacctacgacgacgacctggacaacctgctggcccagatcggcgaccagtacgccgacctgtttctggccgccaagaacctgtccgacgccatcctgctgagcgacatcctgagagtgaacaccgagatcaccaaggcccccctgagcgcctctatgatcaagagatacgacgagcaccaccaggacctgaccctgctgaaagctctcgtgcggcagcagctgcctgagaagtacaaagagattttcttcgaccagagcaagaacggctacgccggctacatcgatggcggagccagccaggaagagttctacaagttcatcaagcccatcctggaaaagatggacggcaccgaggaactgctcgtgaagctgaacagagaggacctgctgcggaagcagcggaccttcgacaacggcagcatcccccaccagatccacctgggagagctgcacgccattctgcggcggcaggaagatttttacccattcctgaaggacaaccgggaaaagatcgagaagatcctgaccttccgcatcccctactacgtgggccctctggccaggggaaacagcagattcgcctggatgaccagaaagagcgaggaaaccatcaccccctggaacttcgaggaagtggtggacaagggcgccagcgcccagagcttcatcgagcggatgaccaacttcgataagaacctgcccaacgagaaggtgctgcccaagcacagcctgctgtacgagtacttcaccgtgtacaacgagctgaccaaagtgaaatacgtgaccgagggaatgagaaagcccgccttcctgagcggcgagcagaaaaaagccatcgtggacctgctgttcaagaccaaccggaaagtgaccgtgaagcagctgaaagaggactacttcaagaaaatcgagtgcttcgactccgtggaaatctccggcgtggaagatcggttcaacgcctccctgggcacataccacgatctgctgaaaattatcaaggacaaggacttcctggacaatgaggaaaacgaggacattctggaagatatcgtgctgaccctgacactgtttgaggacagagagatgatcgaggaacggctgaaaacctatgcccacctgttcgacgacaaagtgatgaagcagctgaagcggcggagatacaccggctggggcaggctgagccggaagctgatcaacggcatccgggacaagcagtccggcaagacaatcctggatttcctgaagtccgacggcttcgccaacagaaacttcatgcagctgatccacgacgacagcctgacctttaaagaggacatccagaaagcccaggtgtccggccagggcgatagcctgcacgagcacattgccaatctggccggcagccccgccattaagaagggcatcctgcagacagtgaaggtggtggacgagctcgtgaaagtgatgggccggcacaagcccgagaacatcgtgatcgaaatggccagagagaaccagaccacccagaagggacagaagaacagccgcgagagaatgaagcggatcgaagagggcatcaaagagctgggcagccagatcctgaaagaacaccccgtggaaaacacccagctgcagaacgagaagctgtacctgtactacctgcagaatgggcgggatatgtacgtggaccaggaactggacatcaaccggctgtccgactacgatgtggacgctatcgtgcctcagagctttctgaaggacgactccatcgataacaaagtgctgactcggagcgacaagaaccggggcaagagcgacaacgtgccctccgaagaggtcgtgaagaagatgaagaactactggcgccagctgctgaatgccaagctgattacccagaggaagttcgacaatctgaccaaggccgagagaggcggcctgagcgaactggataaggccggcttcatcaagagacagctggtggaaacccggcagatcacaaagcacgtggcacagatcctggactcccggatgaacactaagtacgacgagaacgacaaactgatccgggaagtgaaagtgatcaccctgaagtccaagctggtgtccgatttccggaaggatttccagttttacaaagtgcgcgagatcaacaactaccaccacgcccacgacgcctacctgaacgccgtcgtgggaaccgccctgatcaaaaagtaccctaagctggaaagcgagttcgtgtacggcgactacaaggtgtacgacgtgcggaagatgatcgccaagagcgagcaggaaatcggcaaggctaccgccaagtacttcttctacagcaacatcatgaactttttcaagaccgagattaccctggccaacggcgagatccggaagcggcctctgatcgagacaaacggcgaaacaggcgagatcgtgtgggataagggccgggactttgccaccgtgcggaaagtgctgtctatgccccaagtgaatatcgtgaaaaagaccgaggtgcagacaggcggcttcagcaaagagtctatcctgcccaagaggaacagcgacaagctgatcgccagaaagaaggactgggaccctaagaagtacggcggcttcgacagccccaccgtggcctattctgtgctggtggtggccaaagtggaaaagggcaagtccaagaaactgaagagtgtgaaagagctgctggggatcaccatcatggaaagaagcagcttcgagaagaatcccatcgactttctggaagccaagggctacaaagaagtgaaaaaggacctgatcatcaagctgcctaagtactccctgttcgagctggaaaacggccggaagagaatgctggcctctgccggcgaactgcagaagggaaacgaactggccctgccctccaaatatgtgaacttcctgtacctggccagccactatgagaagctgaagggctcccccgaggataatgagcagaaacagctgtttgtggaacagcacaaacactacctggacgagatcatcgagcagatcagcgagttctccaagagagtgatcctggccgacgctaatctggacaaggtgctgagcgcctacaacaagcacagagacaagcctatcagagagcaggccgagaatatcatccacctgtttaccctgaccaatctgggagcccctgccgccttcaagtactttgacaccaccatcgaccggaagaggtacaccagcaccaaagaggtgctggacgccaccctgatccaccagagcatcaccggcctgtacgagacacggatcgacctgtctcagctgggaggcgacgcctatccctatgacgtgcccgattatgccagcctgggcagcggctcccccaagaaaaaacgcaaggtggaagatcctaagaaaaagcggaaagtggacggcagcggcagcgagacccccggtaccagcgagagcgccacccccgagagccggacactggtgaccttcaaggatgtatttgtggacttcaccagggaggagtggaagctgctggacactgctcagcagatcgtgtacagaaatgtgatgctggagaactataagaacctggtttccttgggttatcagcttactaagccagatgtgatcctccggttggagaagggagaagagccctgagatcccaagcacgcagcaatgcagctcaaaacgcttagcctagccacacccccacgggaaacagcagtgattaacctttagcaataaacgaaagtttaactaagctatactaaccccagggttggtcaatttcgtgccagccacaccctggtactgcatgcacgcaatgctagctgcccctttcccgtcctgggcaccccgagtctcccccgaccccgggtcccaggtatgctcccacctccacctgccccactcaccacctctgctagttccagacacctccgagacgaggaaaaaaaaaaaaaaaaaaaaaaaaaaaaaaaaaaaaaaaaaaaaaaaaaaaaaaaaaaaaaaaaaaaaaaaaaaaaaaaaaaaaaaaaaaaaaaaaaaaaaaaaaaaaaaaaaaaaaaaa

SEQ ID NO: 276 - RNA, 8077 nt, synthetic construct
  misc_feature 1..8077: note = mRNA of V35_scFv-dCas9-KRAB-2a-1xGCN4-D3l-D3a
  source 1..8077: mol_type = other RNA
aggactcactatttgttttcgcgcccagttgcaaaaagtgtcgacatttgcttctgacacaactgtgttcactagcaacctcaaacagacaccgccaccatgcctgctgctaagagagtgaaactggatggatccggccccgacatcgtgatgacccagagccccagcagcctgagcgccagcgtgggcgaccgcgtgaccatcacctgccgcagcagcaccggcgccgtgaccaccagcaactacgccagctgggtgcaggagaagcccggcaagctgttcaagggcctgatcggcggcaccaacaaccgcgcccccggcgtgcccagccgcttcagcggcagcctgatcggcgacaaggccaccctgaccatcagcagcctgcagcccgaggacttcgccacctacttctgcgccctgtggtacagcaaccactgggtgttcggccagggcaccaaggtggagctgaagcgcggcggcggcggcagcggcggcggcggcagcggcggcggcggcagcagcggcggcggcagcgaggtgaagctgctggagagcggcggcggcctggtgcagcccggcggcagcctgaagctgagctgcgccgtgagcggcttcagcctgaccgactacggcgtgaactgggtgcgccaggcccccggccgcggcctggagtggatcggcgtgatctggggcgacggcatcaccgactacaacagcgccctgaaggaccgcttcatcatcagcaaggacaacggcaagaacaccgtgtacctgcagatgagcaaggtgcgcagcgacgacaccgccctgtactactgcgtgaccggcctgttcgactactggggccagggcaccctggtgaccgtgagcagctacccatacgatgttccagattacgctggtggaggcggaggttctgggggaggaggtagtggcggtggtggttcaggaggcggcggaagcggaagcggaccaaaaaagaagagaaaggtaatggacaagaagtacagcatcggcctggccatcggcaccaactctgtgggctgggccgtgatcaccgacgagtacaaggtgcccagcaagaaattcaaggtgctgggcaacaccgaccggcacagcatcaagaagaacctgatcggcgccctgctgttcgacagcggagaaacagccgaggccacccggctgaagagaaccgccagaagaagatacaccagacggaagaaccggatctgctatctgcaagagatcttcagcaacgagatggccaaggtggacgacagcttcttccacagactggaagagtccttcctggtggaagaggataagaagcacgagcggcaccccatcttcggcaacatcgtggacgaggtggcctaccacgagaagtaccccaccatctaccacctgagaaagaaactggtggacagcaccgacaaggccgacctgcggctgatctatctggccctggcccacatgatcaagttccggggccacttcctgatcgagggcgacctgaaccccgacaacagcgacgtggacaagctgttcatccagctggtgcagacctacaaccagctgttcgaggaaaaccccatcaacgccagcggcgtggacgccaaggccatcctgtctgccagactgagcaagagcagacggctggaaaatctgatcgcccagctgcccggcgagaagaagaatggcctgttcggcaacctgattgccctgagcctgggcctgacccccaacttcaagagcaacttcgacctggccgaggatgccaaactgcagctgagcaaggacacctacgacgacgacctggacaacctgctggcccagatcggcgaccagtacgccgacctgtttctggccgccaagaacctgtccgacgccatcctgctgagcgacatcctgagagtgaacaccgagatcaccaaggcccccctgagcgcctctatgatcaagagatacgacgagcaccaccaggacctgaccctgctgaaagctctcgtgcggcagcagctgcctgagaagtacaaagagattttcttcgaccagagcaagaacggctacgccggctacatcgatggcggagccagccaggaagagttctacaagttcatcaagcccatcctggaaaagatggacggcaccgaggaactgctcgtgaagctgaacagagaggacctgctgcggaagcagcggaccttcgacaacggcagcatcccccaccagatccacctgggagagctgcacgccattctgcggcggcaggaagatttttacccattcctgaaggacaaccgggaaaagatcgagaagatcctgaccttccgcatcccctactacgtgggccctctggccaggggaaacagcagattcgcctggatgaccagaaagagcgaggaaaccatcaccccctggaacttcgaggaagtggtggacaagggcgccagcgcccagagcttcatcgagcggatgaccaacttcgataagaacctgcccaacgagaaggtgctgcccaagcacagcctgctgtacgagtacttcaccgtgtacaacgagctgaccaaagtgaaatacgtgaccgagggaatgagaaagcccgccttcctgagcggcgagcagaaaaaagccatcgtggacctgctgttcaagaccaaccggaaagtgaccgtgaagcagctgaaagaggactacttcaagaaaatcgagtgcttcgactccgtggaaatctccggcgtggaagatcggttcaacgcctccctgggcacataccacgatctgctgaaaattatcaaggacaaggacttcctggacaatgaggaaaacgaggacattctggaagatatcgtgctgaccctgacactgtttgaggacagagagatgatcgaggaacggctgaaaacctatgcccacctgttcgacgacaaagtgatgaagcagctgaagcggcggagatacaccggctggggcaggctgagccggaagctgatcaacggcatccgggacaagcagtccggcaagacaatcctggatttcctgaagtccgacggcttcgccaacagaaacttcatgcagctgatccacgacgacagcctgacctttaaagaggacatccagaaagcccaggtgtccggccagggcgatagcctgcacgagcacattgccaatctggccggcagccccgccattaagaagggcatcctgcagacagtgaaggtggtggacgagctcgtgaaagtgatgggccggcacaagcccgagaacatcgtgatcgaaatggccagagagaaccagaccacccagaagggacagaagaacagccgcgagagaatgaagcggatcgaagagggcatcaaagagctgggcagccagatcctgaaagaacaccccgtggaaaacacccagctgcagaacgagaagctgtacctgtactacctgcagaatgggcgggatatgtacgtggaccaggaactggacatcaaccggctgtccgactacgatgtggacgctatcgtgcctcagagctttctgaaggacgactccatcgataacaaagtgctgactcggagcgacaagaaccggggcaagagcgacaacgtgccctccgaagaggtcgtgaagaagatgaagaactactggcgccagctgctgaatgccaagctgattacccagaggaagttcgacaatctgaccaaggccgagagaggcggcctgagcgaactggataaggccggcttcatcaagagacagctggtggaaacccggcagatcacaaagcacgtggcacagatcctggactcccggatgaacactaagtacgacgagaacgacaaactgatccgggaagtgaaagtgatcaccctgaagtccaagctggtgtccgatttccggaaggatttccagttttacaaagtgcgcgagatcaacaactaccaccacgcccacgacgcctacctgaacgccgtcgtgggaaccgccctgatcaaaaagtaccctaagctggaaagcgagttcgtgtacggcgactacaaggtgtacgacgtgcggaagatgatcgccaagagcgagcaggaaatcggcaaggctaccgccaagtacttcttctacagcaacatcatgaactttttcaagaccgagattaccctggccaacggcgagatccggaagcggcctctgatcgagacaaacggcgaaacaggcgagatcgtgtgggataagggccgggactttgccaccgtgcggaaagtgctgtctatgccccaagtgaatatcgtgaaaaagaccgaggtgcagacaggcggcttcagcaaagagtctatcctgcccaagaggaacagcgacaagctgatcgccagaaagaaggactgggaccctaagaagtacggcggcttcgacagccccaccgtggcctattctgtgctggtggtggccaaagtggaaaagggcaagtccaagaaactgaagagtgtgaaagagctgctggggatcaccatcatggaaagaagcagcttcgagaagaatcccatcgactttctggaagccaagggctacaaagaagtgaaaaaggacctgatcatcaagctgcctaagtactccctgttcgagctggaaaacggccggaagagaatgctggcctctgccggcgaactgcagaagggaaacgaactggccctgccctccaaatatgtgaacttcctgtacctggccagccactatgagaagctgaagggctcccccgaggataatgagcagaaacagctgtttgtggaacagcacaaacactacctggacgagatcatcgagcagatcagcgagttctccaagagagtgatcctggccgacgctaatctggacaaggtgctgagcgcctacaacaagcacagagacaagcctatcagagagcaggccgagaatatcatccacctgtttaccctgaccaatctgggagcccctgccgccttcaagtactttgacaccaccatcgaccggaagaggtacaccagcaccaaagaggtgctggacgccaccctgatccaccagagcatcaccggcctgtacgagacacggatcgacctgtctcagctgggaggcgacgcctatccctatgacgtgcccgattatgccagcctgggcagcggctcccccaagaaaaaacgcaaggtggaagatcctaagaaaaagcggaaagtggacggcagcggcagcgagacccccggtaccagcgagagcgccacccccgagagccggacactggtgaccttcaaggatgtatttgtggacttcaccagggaggagtggaagctgctggacactgctcagcagatcgtgtacagaaatgtgatgctggagaactataagaacctggtttccttgggttatcagcttactaagccagatgtgatcctccggttggagaagggagaagagcccggaagcggagctactaacttcagcctgctgaagcaggctggagacgtggaggagaaccctggacctatgcctgctgctaagagagtgaaactggatggatccggctcaggcggatctggttcaggggaagaactcctctccaaaaactaccatctcgagaatgaggtcgcccgcctgaaaaaaggatcaggttccggtggttctggcagcggtggttcaggctcaggcagcggcggtagcggtagcggtggaagcggaagcggaacccccggtaccagcgagggcggccctagcagcggcgcccctccccctagcggcggcagccctgccggatcccctacaagcaccgaagaaggcacaagcgagtccgctacccctgagtccggccctggcacctccacagagcctagcgagggatccgctcctggatcccctgccggaagccctacctccaccgaggagggcacaagcaccgagccttccgagggcagcgcccccggaacaagcaccgaacctagcgagagcgccacccccgagagcatgttcgaaaccgtgcctgtgtggaggagacagccagtccgggtgctgtccctttttgaagacatcaagaaagagctgacgagtttgggctttttggaaagtggttctgacccgggacaactgaagcatgtggttgatgtcacagacacagtgaggaaggatgtggaggagtggggacccttcgatcttgtgtacggcgccacacctcccctgggccacacctgtgaccgtcctcccagctggtacctgttccagttccaccggctcctgcagtacgcacggcccaagccaggcagccccaggcccttcttctggatgttcgtggacaatctggtgctgaacaaggaagacctggacgtcgcatctcgcttcctggagatggagccagtcaccatcccagatgtccacggcggatccttgcagaatgctgtccgcgtgtggagcaacatcccagccataaggagcagcaggcactgggctctggtttcggaagaagaattgtccctgctggcccagaacaagcagagctcgaagctcgcggccaagtggcccaccaagctggtgaagaactgctttctccccctaagagaatatttcaagtatttttcaacagaactcacttcctctttatctagcggcaatagtaacgctaacagccgcgggccgagcttcagcagcggcctggtgccgttaagcttgcgcggcagccatatgaaccatgaccaggaatttgaccccccaaaggtttacccacctgtgccagctgagaagaggaagcccatccgcgtgctgtctctctttgatgggattgctacagggctcctggtgctgaaggacctgggcatccaagtggaccgctacattgcctccgaggtgtgtgaggactccatcacggtgggcatggtgcggcaccagggaaagatcatgtacgtcggggacgtccgcagcgtcacacagaagcatatccaggagtggggcccattcgacctggtgattggaggcagtccctgcaatgacctctccattgtcaaccctgcccgcaagggactttatgagggtactggccgcctcttctttgagttctaccgcctcctgcatgatgcgcggcccaaggagggagatgatcgccccttcttctggctctttgagaatgtggtggccatgggcgttagtgacaagagggacatctcgcgatttcttgagtctaaccccgtgatgattgacgccaaagaagtgtctgctgcacacagggcccgttacttctggggtaaccttcctggcatgaacaggcctttggcatccactgtgaatgataagctggagctgcaagagtgtctggagcacggcagaatagccaagttcagcaaagtgaggaccattaccaccaggtcaaactctataaagcagggcaaagaccagcatttccccgtcttcatgaacgagaaggaggacatcctgtggtgcactgaaatggaaagggtgtttggcttccccgtccactacacagacgtctccaacatgagccgcttggcgaggcagagactgctgggccgatcgtggagcgtgccggtcatccgccacctcttcgctccgctgaaggaatattttgcttgtgtgctcgaggctactaacttcagcctgctgaagcaggctggagacgtggaggagaaccctggacctatgcattaatgagatcccaagcacgcagcaatgcagctcaaaacgcttagcctagccacacccccacgggaaacagcagtgattaacctttagcaataaacgaaagtttaactaagctatactaaccccagggttggtcaatttcgtgccagccacaccctggtactgcatgcacgcaatgctagctgcccctttcccgtcctgggcaccccgagtctcccccgaccccgggtcccaggtatgctcccacctccacctgccccactcaccacctctgctagttccagacacctccgagacgaggaaaaaaaaaaaaaaaaaaaaaaaaaaaaaaaaaaaaaaaaaaaaaaaaaaaaaaaaaaaaaaaaaaaaaaaaaaaaaaaaaaaaaaaaaaaaaaaaaaaaaaaaaaaaaaaaaaaaaaaa

SEQ ID NO: 277 - RNA, 8473 nt, synthetic construct
  misc_feature 1..8473: note = mRNA of V36_scFv-dCas9-HP1a-2a-1xGCN4-D3l-D3a
  source 1..8473: mol_type = other RNA
aggactcactatttgttttcgcgcccagttgcaaaaagtgtcgacatttgcttctgacacaactgtgttcactagcaacctcaaacagacaccgccaccatgcctgctgctaagagagtgaaactggatggatccggccccgacatcgtgatgacccagagccccagcagcctgagcgccagcgtgggcgaccgcgtgaccatcacctgccgcagcagcaccggcgccgtgaccaccagcaactacgccagctgggtgcaggagaagcccggcaagctgttcaagggcctgatcggcggcaccaacaaccgcgcccccggcgtgcccagccgcttcagcggcagcctgatcggcgacaaggccaccctgaccatcagcagcctgcagcccgaggacttcgccacctacttctgcgccctgtggtacagcaaccactgggtgttcggccagggcaccaaggtggagctgaagcgcggcggcggcggcagcggcggcggcggcagcggcggcggcggcagcagcggcggcggcagcgaggtgaagctgctggagagcggcggcggcctggtgcagcccggcggcagcctgaagctgagctgcgccgtgagcggcttcagcctgaccgactacggcgtgaactgggtgcgccaggcccccggccgcggcctggagtggatcggcgtgatctggggcgacggcatcaccgactacaacagcgccctgaaggaccgcttcatcatcagcaaggacaacggcaagaacaccgtgtacctgcagatgagcaaggtgcgcagcgacgacaccgccctgtactactgcgtgaccggcctgttcgactactggggccagggcaccctggtgaccgtgagcagctacccatacgatgttccagattacgctggtggaggcggaggttctgggggaggaggtagtggcggtggtggttcaggaggcggcggaagcggaagcggaccaaaaaagaagagaaaggtaatggacaagaagtacagcatcggcctggccatcggcaccaactctgtgggctgggccgtgatcaccgacgagtacaaggtgcccagcaagaaattcaaggtgctgggcaacaccgaccggcacagcatcaagaagaacctgatcggcgccctgctgttcgacagcggagaaacagccgaggccacccggctgaagagaaccgccagaagaagatacaccagacggaagaaccggatctgctatctgcaagagatcttcagcaacgagatggccaaggtggacgacagcttcttccacagactggaagagtccttcctggtggaagaggataagaagcacgagcggcaccccatcttcggcaacatcgtggacgaggtggcctaccacgagaagtaccccaccatctaccacctgagaaagaaactggtggacagcaccgacaaggccgacctgcggctgatctatctggccctggcccacatgatcaagttccggggccacttcctgatcgagggcgacctgaaccccgacaacagcgacgtggacaagctgttcatccagctggtgcagacctacaaccagctgttcgaggaaaaccccatcaacgccagcggcgtggacgccaaggccatcctgtctgccagactgagcaagagcagacggctggaaaatctgatcgcccagctgcccggcgagaagaagaatggcctgttcggcaacctgattgccctgagcctgggcctgacccccaacttcaagagcaacttcgacctggccgaggatgccaaactgcagctgagcaaggacacctacgacgacgacctggacaacctgctggcccagatcggcgaccagtacgccgacctgtttctggccgccaagaacctgtccgacgccatcctgctgagcgacatcctgagagtgaacaccgagatcaccaaggcccccctgagcgcctctatgatcaagagatacgacgagcaccaccaggacctgaccctgctgaaagctctcgtgcggcagcagctgcctgagaagtacaaagagattttcttcgaccagagcaagaacggctacgccggctacatcgatggcggagccagccaggaagagttctacaagttcatcaagcccatcctggaaaagatggacggcaccgaggaactgctcgtgaagctgaacagagaggacctgctgcggaagcagcggaccttcgacaacggcagcatcccccaccagatccacctgggagagctgcacgccattctgcggcggcaggaagatttttacccattcctgaaggacaaccgggaaaagatcgagaagatcctgaccttccgcatcccctactacgtgggccctctggccaggggaaacagcagattcgcctggatgaccagaaagagcgaggaaaccatcaccccctggaacttcgaggaagtggtggacaagggcgccagcgcccagagcttcatcgagcggatgaccaacttcgataagaacctgcccaacgagaaggtgctgcccaagcacagcctgctgtacgagtacttcaccgtgtacaacgagctgaccaaagtgaaatacgtgaccgagggaatgagaaagcccgccttcctgagcggcgagcagaaaaaagccatcgtggacctgctgttcaagaccaaccggaaagtgaccgtgaagcagctgaaagaggactacttcaagaaaatcgagtgcttcgactccgtggaaatctccggcgtggaagatcggttcaacgcctccctgggcacataccacgatctgctgaaaattatcaaggacaaggacttcctggacaatgaggaaaacgaggacattctggaagatatcgtgctgaccctgacactgtttgaggacagagagatgatcgaggaacggctgaaaacctatgcccacctgttcgacgacaaagtgatgaagcagctgaagcggcggagatacaccggctggggcaggctgagccggaagctgatcaacggcatccgggacaagcagtccggcaagacaatcctggatttcctgaagtccgacggcttcgccaacagaaacttcatgcagctgatccacgacgacagcctgacctttaaagaggacatccagaaagcccaggtgtccggccagggcgatagcctgcacgagcacattgccaatctggccggcagccccgccattaagaagggcatcctgcagacagtgaaggtggtggacgagctcgtgaaagtgatgggccggcacaagcccgagaacatcgtgatcgaaatggccagagagaaccagaccacccagaagggacagaagaacagccgcgagagaatgaagcggatcgaagagggcatcaaagagctgggcagccagatcctgaaagaacaccccgtggaaaacacccagctgcagaacgagaagctgtacctgtactacctgcagaatgggcgggatatgtacgtggaccaggaactggacatcaaccggctgtccgactacgatgtggacgctatcgtgcctcagagctttctgaaggacgactccatcgataacaaagtgctgactcggagcgacaagaaccggggcaagagcgacaacgtgccctccgaagaggtcgtgaagaagatgaagaactactggcgccagctgctgaatgccaagctgattacccagaggaagttcgacaatctgaccaaggccgagagaggcggcctgagcgaactggataaggccggcttcatcaagagacagctggtggaaacccggcagatcacaaagcacgtggcacagatcctggactcccggatgaacactaagtacgacgagaacgacaaactgatccgggaagtgaaagtgatcaccctgaagtccaagctggtgtccgatttccggaaggatttccagttttacaaagtgcgcgagatcaacaactaccaccacgcccacgacgcctacctgaacgccgtcgtgggaaccgccctgatcaaaaagtaccctaagctggaaagcgagttcgtgtacggcgactacaaggtgtacgacgtgcggaagatgatcgccaagagcgagcaggaaatcggcaaggctaccgccaagtacttcttctacagcaacatcatgaactttttcaagaccgagattaccctggccaacggcgagatccggaagcggcctctgatcgagacaaacggcgaaacaggcgagatcgtgtgggataagggccgggactttgccaccgtgcggaaagtgctgtctatgccccaagtgaatatcgtgaaaaagaccgaggtgcagacaggcggcttcagcaaagagtctatcctgcccaagaggaacagcgacaagctgatcgccagaaagaaggactgggaccctaagaagtacggcggcttcgacagccccaccgtggcctattctgtgctggtggtggccaaagtggaaaagggcaagtccaagaaactgaagagtgtgaaagagctgctggggatcaccatcatggaaagaagcagcttcgagaagaatcccatcgactttctggaagccaagggctacaaagaagtgaaaaaggacctgatcatcaagctgcctaagtactccctgttcgagctggaaaacggccggaagagaatgctggcctctgccggcgaactgcagaagggaaacgaactggccctgccctccaaatatgtgaacttcctgtacctggccagccactatgagaagctgaagggctcccccgaggataatgagcagaaacagctgtttgtggaacagcacaaacactacctggacgagatcatcgagcagatcagcgagttctccaagagagtgatcctggccgacgctaatctggacaaggtgctgagcgcctacaacaagcacagagacaagcctatcagagagcaggccgagaatatcatccacctgtttaccctgaccaatctgggagcccctgccgccttcaagtactttgacaccaccatcgaccggaagaggtacaccagcaccaaagaggtgctggacgccaccctgatccaccagagcatcaccggcctgtacgagacacggatcgacctgtctcagctgggaggcgacgcctatccctatgacgtgcccgattatgccagcctgggcagcggctcccccaagaaaaaacgcaaggtggaagatcctaagaaaaagcggaaagtggacggcagcggcagcgagacccccggtaccagcgagagcgccacccccgagagccggacactcggaaagaaaaccaagcggacagctgacagttcttcttcagaggatgaggaggagtatgttgtggagaaggtgctagacaggcgcgtggttaagggacaagtggaatatctactgaagtggaaaggcttttctgaggagcacaatacttgggaacctgagaaaaacttggattgccctgagctaatttctgaatttatgaaaaagtataagaagatgaaggagggtgaaaataataaacccagggagaagtcagaaagtaacaagaggaaatccaatttctcaaacagtgccgatgacatcaaatctaaaaaaaagagagagcagagcaatgatatcgctcggggctttgagagaggactggaaccagaaaagatcattggggcaacagattcctgtggtgatttaatgttcctaatgaaatggaaagacacagatgaagctgacctggttcttgcaaaagaagctaatgtgaaatgtccacaaattgtgatagcattttatgaagagagactgacatggcatgcatatcctgaggatgcggaaaacaaagagaaagaaacagcaaagagcgagggcagcggcgctactaacttcagcctgctgaagcaggctggagacgtggaggagaaccctggacctatgcctgctgctaagagagtgaaactggatggatccggctcaggcggatctggttcaggggaagaactcctctccaaaaactaccatctcgagaatgaggtcgcccgcctgaaaaaaggatcaggttccggtggttctggcagcggtggttcaggctcaggcagcggcggtagcggtagcggtggaagcggaagcggaacccccggtaccagcgagggcggccctagcagcggcgcccctccccctagcggcggcagccctgccggatcccctacaagcaccgaagaaggcacaagcgagtccgctacccctgagtccggccctggcacctccacagagcctagcgagggatccgctcctggatcccctgccggaagccctacctccaccgaggagggcacaagcaccgagccttccgagggcagcgcccccggaacaagcaccgaacctagcgagagcgccacccccgagagcatgttcgaaaccgtgcctgtgtggaggagacagccagtccgggtgctgtccctttttgaagacatcaagaaagagctgacgagtttgggctttttggaaagtggttctgacccgggacaactgaagcatgtggttgatgtcacagacacagtgaggaaggatgtggaggagtggggacccttcgatcttgtgtacggcgccacacctcccctgggccacacctgtgaccgtcctcccagctggtacctgttccagttccaccggctcctgcagtacgcacggcccaagccaggcagccccaggcccttcttctggatgttcgtggacaatctggtgctgaacaaggaagacctggacgtcgcatctcgcttcctggagatggagccagtcaccatcccagatgtccacggcggatccttgcagaatgctgtccgcgtgtggagcaacatcccagccataaggagcagcaggcactgggctctggtttcggaagaagaattgtccctgctggcccagaacaagcagagctcgaagctcgcggccaagtggcccaccaagctggtgaagaactgctttctccccctaagagaatatttcaagtatttttcaacagaactcacttcctctttatctagcggcaatagtaacgctaacagccgcgggccgagcttcagcagcggcctggtgccgttaagcttgcgcggcagccatatgaaccatgaccaggaatttgaccccccaaaggtttacccacctgtgccagctgagaagaggaagcccatccgcgtgctgtctctctttgatgggattgctacagggctcctggtgctgaaggacctgggcatccaagtggaccgctacattgcctccgaggtgtgtgaggactccatcacggtgggcatggtgcggcaccagggaaagatcatgtacgtcggggacgtccgcagcgtcacacagaagcatatccaggagtggggcccattcgacctggtgattggaggcagtccctgcaatgacctctccattgtcaaccctgcccgcaagggactttatgagggtactggccgcctcttctttgagttctaccgcctcctgcatgatgcgcggcccaaggagggagatgatcgccccttcttctggctctttgagaatgtggtggccatgggcgttagtgacaagagggacatctcgcgatttcttgagtctaaccccgtgatgattgacgccaaagaagtgtctgctgcacacagggcccgttacttctggggtaaccttcctggcatgaacaggcctttggcatccactgtgaatgataagctggagctgcaagagtgtctggagcacggcagaatagccaagttcagcaaagtgaggaccattaccaccaggtcaaactctataaagcagggcaaagaccagcatttccccgtcttcatgaacgagaaggaggacatcctgtggtgcactgaaatggaaagggtgtttggcttccccgtccactacacagacgtctccaacatgagccgcttggcgaggcagagactgctgggccgatcgtggagcgtgccggtcatccgccacctcttcgctccgctgaaggaatattttgcttgtgtgctcgaggctactaacttcagcctgctgaagcaggctggagacgtggaggagaaccctggacctatgcattaatgagatcccaagcacgcagcaatgcagctcaaaacgcttagcctagccacacccccacgggaaacagcagtgattaacctttagcaataaacgaaagtttaactaagctatactaaccccagggttggtcaatttcgtgccagccacaccctggtactgcatgcacgcaatgctagctgcccctttcccgtcctgggcaccccgagtctcccccgaccccgggtcccaggtatgctcccacctccacctgccccactcaccacctctgctagttccagacacctccgagacgaggaaaaaaaaaaaaaaaaaaaaaaaaaaaaaaaaaaaaaaaaaaaaaaaaaaaaaaaaaaaaaaaaaaaaaaaaaaaaaaaaaaaaaaaaaaaaaaaaaaaaaaaaaaaaaaaaaaaaaaaa

SEQ ID NO: 278 - RNA, 8224 nt, synthetic construct
  misc_feature 1..8224: note = mRNA of V37_GFP1-10-KRAB-2a-D3a-D3l-dCas9-7xGFP11
  source 1..8224: mol_type = other RNA
aggactcactatttgttttcgcgcccagttgcaaaaagtgtcgacatttgcttctgacacaactgtgttcactagcaacctcaaacagacaccgccaccatgtccaagggagaggagctgttcaccggagtggtgccaatcctggtggagctggacggcgatgtgaacggccacaagttttctgtgcgcggagagggagagggcgacgcaaccatcggcaagctgacactgaagttcatctgcaccacaggcaagctgcccgtgccttggccaaccctggtgaccacactgacatacggcgtgcagtgtttctctaggtatccagaccacatgaagagacacgatttctttaagagcgccatgccagagggatacgtgcaggagcggaccatctccttcaaggacgatggcaagtataagacccgcgccgtggtgaagtttgagggcgatacactggtgaacaggatcgagctgaagggcaccgacttcaaggaggatggcaatatcctgggccacaagctggagtacaactttaatagccacaacgtgtatatcacagccgacaagcagaagaacggcatcaaggccaacttcaccgtgaggcacaatgtggaggacggctccgtgcagctggccgatcactaccagcagaacacacctatcggcgacggacccgtgctgctgcctgataatcactatctgtccacccagacagtgctgtctaaggacccaaacgagaagttggatccaggtggaggtggaagcggtcggacactggtgaccttcaaggatgtatttgtggacttcaccagggaggagtggaagctgctggacactgctcagcagatcgtgtacagaaatgtgatgctggagaactataagaacctggtttccttgggttatcagcttactaagccagatgtgatcctccggttggagaagggagaagagcccggaagcggaaagcgcaccgccgatggttccgagttcgaaagccccaaaaaaaagcgcaaggtcggaagcggagctactaacttcagcctgctgaagcaggctggagacgtggaggagaaccctggacctcctgctgctaagagagtgaaactggatggatccaaccatgaccaggaatttgaccccccaaaggtttacccacctgtgccagctgagaagaggaagcccatccgcgtgctgtctctctttgatgggattgctacagggctcctggtgctgaaggacctgggcatccaagtggaccgctacattgcctccgaggtgtgtgaggactccatcacggtgggcatggtgcggcaccagggaaagatcatgtacgtcggggacgtccgcagcgtcacacagaagcatatccaggagtggggcccattcgacctggtgattggaggcagtccctgcaatgacctctccattgtcaaccctgcccgcaagggactttatgagggtactggccgcctcttctttgagttctaccgcctcctgcatgatgcgcggcccaaggagggagatgatcgccccttcttctggctctttgagaatgtggtggccatgggcgttagtgacaagagggacatctcgcgatttcttgagtctaaccccgtgatgattgacgccaaagaagtgtctgctgcacacagggcccgttacttctggggtaaccttcctggcatgaacaggcctttggcatccactgtgaatgataagctggagctgcaagagtgtctggagcacggcagaatagccaagttcagcaaagtgaggaccattaccaccaggtcaaactctataaagcagggcaaagaccagcatttccccgtgttcatgaacgagaaggaggacatcctgtggtgcactgaaatggaaagggtgtttggcttccccgtccactacacagacgtctccaacatgagccgcttggcgaggcagagactgctgggccgatcgtggagcgtgccggtcatccgccacctcttcgctccgctgaaggaatattttgcttgtgtgtctagcggcaatagtaacgctaacagccgcgggccgagcttcagcagcggcctggtgccgttaagcttgcgcggcagccatatgggccctatggagatatacaagacagtgtctgcatggaagagacagccagtgcgggtactgagcctcttcagaaacatcgacaaggtactaaagagtttgggcttcttggaaagcggttctggttctgggggaggaacgctgaagtacgtggaagatgtcacaaatgtcgtgaggagagacgtggagaaatggggcccctttgacctggtgtacggctcgacgcagcccctaggcagctcttgtgatcgctgtcccggctggtacatgttccagttccaccggatcctgcagtatgcgctgcctcgccaggagagtcagcggcccttcttctggatattcatggacaatctgctgctgactgaggatgaccaagagacaactacccgcttccttcagacagaggctgtgaccctccaggatgtccgtggcagagactaccagaatgctatgcgggtgtggagcaacattccagggctgaagagcaagcatgcgcccctgaccccaaaggaagaagagtatctgcaagcccaagtcagaagcaggagcaagctggacgccccgaaagttgacctcctggtgaagaactgccttctcccgctgagagagtacttcaagtatttttctcaaaactcacttcctcttggagggccgagctctggcgcacccccaccaagtggagggtctcctgccgggtccccaacatctactgaagaaggcaccagcgaatccgcaacgcccgagtcaggccctggtacctccacagaaccatctgaaggtagtgcgcctggttccccagctggaagccctacttccaccgaagaaggcacgtcaaccgaaccaagtgaaggatctgcccctgggaccagcactgaaccatctgagccaaaaaagaagagaaaggtaatggacaagaagtacagcatcggcctggccatcggcaccaactctgtgggctgggccgtgatcaccgacgagtacaaggtgcccagcaagaaattcaaggtgctgggcaacaccgaccggcacagcatcaagaagaacctgatcggcgccctgctgttcgacagcggagaaacagccgaggccacccggctgaagagaaccgccagaagaagatacaccagacggaagaaccggatctgctatctgcaagagatcttcagcaacgagatggccaaggtggacgacagcttcttccacagactggaagagtccttcctggtggaagaggataagaagcacgagcggcaccccatcttcggcaacatcgtggacgaggtggcctaccacgagaagtaccccaccatctaccacctgagaaagaaactggtggacagcaccgacaaggccgacctgcggctgatctatctggccctggcccacatgatcaagttccggggccacttcctgatcgagggcgacctgaaccccgacaacagcgacgtggacaagctgttcatccagctggtgcagacctacaaccagctgttcgaggaaaaccccatcaacgccagcggcgtggacgccaaggccatcctgtctgccagactgagcaagagcagacggctggaaaatctgatcgcccagctgcccggcgagaagaagaatggcctgttcggcaacctgattgccctgagcctgggcctgacccccaacttcaagagcaacttcgacctggccgaggatgccaaactgcagctgagcaaggacacctacgacgacgacctggacaacctgctggcccagatcggcgaccagtacgccgacctgtttctggccgccaagaacctgtccgacgccatcctgctgagcgacatcctgagagtgaacaccgagatcaccaaggcccccctgagcgcctctatgatcaagagatacgacgagcaccaccaggacctgaccctgctgaaagctctcgtgcggcagcagctgcctgagaagtacaaagagattttcttcgaccagagcaagaacggctacgccggctacatcgatggcggagccagccaggaagagttctacaagttcatcaagcccatcctggaaaagatggacggcaccgaggaactgctcgtgaagctgaacagagaggacctgctgcggaagcagcggaccttcgacaacggcagcatcccccaccagatccacctgggagagctgcacgccattctgcggcggcaggaagatttttacccattcctgaaggacaaccgggaaaagatcgagaagatcctgaccttccgcatcccctactacgtgggccctctggccaggggaaacagcagattcgcctggatgaccagaaagagcgaggaaaccatcaccccctggaacttcgaggaagtggtggacaagggcgccagcgcccagagcttcatcgagcggatgaccaacttcgataagaacctgcccaacgagaaggtgctgcccaagcacagcctgctgtacgagtacttcaccgtgtacaacgagctgaccaaagtgaaatacgtgaccgagggaatgagaaagcccgccttcctgagcggcgagcagaaaaaagccatcgtggacctgctgttcaagaccaaccggaaagtgaccgtgaagcagctgaaagaggactacttcaagaaaatcgagtgcttcgactccgtggaaatctccggcgtggaagatcggttcaacgcctccctgggcacataccacgatctgctgaaaattatcaaggacaaggacttcctggacaatgaggaaaacgaggacattctggaagatatcgtgctgaccctgacactgtttgaggacagagagatgatcgaggaacggctgaaaacctatgcccacctgttcgacgacaaagtgatgaagcagctgaagcggcggagatacaccggctggggcaggctgagccggaagctgatcaacggcatccgggacaagcagtccggcaagacaatcctggatttcctgaagtccgacggcttcgccaacagaaacttcatgcagctgatccacgacgacagcctgacctttaaagaggacatccagaaagcccaggtgtccggccagggcgatagcctgcacgagcacattgccaatctggccggcagccccgccattaagaagggcatcctgcagacagtgaaggtggtggacgagctcgtgaaagtgatgggccggcacaagcccgagaacatcgtgatcgaaatggccagagagaaccagaccacccagaagggacagaagaacagccgcgagagaatgaagcggatcgaagagggcatcaaagagctgggcagccagatcctgaaagaacaccccgtggaaaacacccagctgcagaacgagaagctgtacctgtactacctgcagaatgggcgggatatgtacgtggaccaggaactggacatcaaccggctgtccgactacgatgtggacgctatcgtgcctcagagctttctgaaggacgactccatcgataacaaagtgctgactcggagcgacaagaaccggggcaagagcgacaacgtgccctccgaagaggtcgtgaagaagatgaagaactactggcgccagctgctgaatgccaagctgattacccagaggaagttcgacaatctgaccaaggccgagagaggcggcctgagcgaactggataaggccggcttcatcaagagacagctggtggaaacccggcagatcacaaagcacgtggcacagatcctggactcccggatgaacactaagtacgacgagaacgacaaactgatccgggaagtgaaagtgatcaccctgaagtccaagctggtgtccgatttccggaaggatttccagttttacaaagtgcgcgagatcaacaactaccaccacgcccacgacgcctacctgaacgccgtcgtgggaaccgccctgatcaaaaagtaccctaagctggaaagcgagttcgtgtacggcgactacaaggtgtacgacgtgcggaagatgatcgccaagagcgagcaggaaatcggcaaggctaccgccaagtacttcttctacagcaacatcatgaactttttcaagaccgagattaccctggccaacggcgagatccggaagcggcctctgatcgagacaaacggcgaaacaggcgagatcgtgtgggataagggccgggactttgccaccgtgcggaaagtgctgtctatgccccaagtgaatatcgtgaaaaagaccgaggtgcagacaggcggcttcagcaaagagtctatcctgcccaagaggaacagcgacaagctgatcgccagaaagaaggactgggaccctaagaagtacggcggcttcgacagccccaccgtggcctattctgtgctggtggtggccaaagtggaaaagggcaagtccaagaaactgaagagtgtgaaagagctgctggggatcaccatcatggaaagaagcagcttcgagaagaatcccatcgactttctggaagccaagggctacaaagaagtgaaaaaggacctgatcatcaagctgcctaagtactccctgttcgagctggaaaacggccggaagagaatgctggcctctgccggcgaactgcagaagggaaacgaactggccctgccctccaaatatgtgaacttcctgtacctggccagccactatgagaagctgaagggctcccccgaggataatgagcagaaacagctgtttgtggaacagcacaaacactacctggacgagatcatcgagcagatcagcgagttctccaagagagtgatcctggccgacgctaatctggacaaggtgctgagcgcctacaacaagcacagagacaagcctatcagagagcaggccgagaatatcatccacctgtttaccctgaccaatctgggagcccctgccgccttcaagtactttgacaccaccatcgaccggaagaggtacaccagcaccaaagaggtgctggacgccaccctgatccaccagagcatcaccggcctgtacgagacacggatcgacctgtctcagctgggaggcgacgcctatccctatgacgtgcccgattatgccagcctgggcagcggctcccccaagaaaaaacgcaaggtggaagatcctaagaaaaagcggaaagtggacggcagcggcagcgagacccccggtaccagcgagagcgccacccccgagagcggtagtgggagcaacggcagcagcggatccatgcgtgaccacatggtccttcatgagtatgtaaatgctgctgggattacaggtggctctggaggtagagatcatatggttctccacgaatacgttaacgccgcaggcatcactggcggtagtggaggacgcgaccatatggtactacatgaatatgtcaatgcagccggaataaccggagggtccggaggccgggatcacatggtgctgcatgagtatgtgaacgcggcgggtataactggtgggtcgggcggacgagaccatatggtgcttcacgaatacgtaaacgcagctggcattactggcggatcaggtggcagggatcacatggtactccatgagtacgtgaacgctgctggaatcacaggcggtagcggcggtcgggaccatatggtcctgcacgaatatgtcaatgctgccggtatcaccgcggccgcaaggtcaggctccggccagcggggaagcaagcgcaccgccgatggttccgagttcgaaagccccaaaaaaaagcgcaaggtctgagatcccaagcacgcagcaatgcagctcaaaacgcttagcctagccacacccccacgggaaacagcagtgattaacctttagcaataaacgaaagtttaactaagctatactaaccccagggttggtcaatttcgtgccagccacaccctggtactgcatgcacgcaatgctagctgcccctttcccgtcctgggcaccccgagtctcccccgaccccgggtcccaggtatgctcccacctccacctgccccactcaccacctctgctagttccagacacctccgagacgaggaaaaaaaaaaaaaaaaaaaaaaaaaaaaaaaaaaaaaaaaaaaaaaaaaaaaaaaaaaaaaaaaaaaaaaaaaaaaaaaaaaaaaaaaaaaaaaaaaaaaaaaaaaaaaaaaaaaaaaaa

SEQ ID NO: 279 - RNA, 7846 nt, synthetic construct
  misc_feature 1..7846: note = mRNA of V38_GFP1-10-KRAB-2a-D3a-D3l-dCas9-1xGFP11
  source 1..7846: mol_type = other RNA
aggactcactatttgttttcgcgcccagttgcaaaaagtgtcgacatttgcttctgacacaactgtgttcactagcaacctcaaacagacaccgccaccatgtccaagggagaggagctgttcaccggagtggtgccaatcctggtggagctggacggcgatgtgaacggccacaagttttctgtgcgcggagagggagagggcgacgcaaccatcggcaagctgacactgaagttcatctgcaccacaggcaagctgcccgtgccttggccaaccctggtgaccacactgacatacggcgtgcagtgtttctctaggtatccagaccacatgaagagacacgatttctttaagagcgccatgccagagggatacgtgcaggagcggaccatctccttcaaggacgatggcaagtataagacccgcgccgtggtgaagtttgagggcgatacactggtgaacaggatcgagctgaagggcaccgacttcaaggaggatggcaatatcctgggccacaagctggagtacaactttaatagccacaacgtgtatatcacagccgacaagcagaagaacggcatcaaggccaacttcaccgtgaggcacaatgtggaggacggctccgtgcagctggccgatcactaccagcagaacacacctatcggcgacggacccgtgctgctgcctgataatcactatctgtccacccagacagtgctgtctaaggacccaaacgagaagttggatccaggtggaggtggaagcggtcggacactggtgaccttcaaggatgtatttgtggacttcaccagggaggagtggaagctgctggacactgctcagcagatcgtgtacagaaatgtgatgctggagaactataagaacctggtttccttgggttatcagcttactaagccagatgtgatcctccggttggagaagggagaagagcccggaagcggaaagcgcaccgccgatggttccgagttcgaaagccccaaaaaaaagcgcaaggtcggaagcggagctactaacttcagcctgctgaagcaggctggagacgtggaggagaaccctggacctcctgctgctaagagagtgaaactggatggatccaaccatgaccaggaatttgaccccccaaaggtttacccacctgtgccagctgagaagaggaagcccatccgcgtgctgtctctctttgatgggattgctacagggctcctggtgctgaaggacctgggcatccaagtggaccgctacattgcctccgaggtgtgtgaggactccatcacggtgggcatggtgcggcaccagggaaagatcatgtacgtcggggacgtccgcagcgtcacacagaagcatatccaggagtggggcccattcgacctggtgattggaggcagtccctgcaatgacctctccattgtcaaccctgcccgcaagggactttatgagggtactggccgcctcttctttgagttctaccgcctcctgcatgatgcgcggcccaaggagggagatgatcgccccttcttctggctctttgagaatgtggtggccatgggcgttagtgacaagagggacatctcgcgatttcttgagtctaaccccgtgatgattgacgccaaagaagtgtctgctgcacacagggcccgttacttctggggtaaccttcctggcatgaacaggcctttggcatccactgtgaatgataagctggagctgcaagagtgtctggagcacggcagaatagccaagttcagcaaagtgaggaccattaccaccaggtcaaactctataaagcagggcaaagaccagcatttccccgtgttcatgaacgagaaggaggacatcctgtggtgcactgaaatggaaagggtgtttggcttccccgtccactacacagacgtctccaacatgagccgcttggcgaggcagagactgctgggccgatcgtggagcgtgccggtcatccgccacctcttcgctccgctgaaggaatattttgcttgtgtgtctagcggcaatagtaacgctaacagccgcgggccgagcttcagcagcggcctggtgccgttaagcttgcgcggcagccatatgggccctatggagatatacaagacagtgtctgcatggaagagacagccagtgcgggtactgagcctcttcagaaacatcgacaaggtactaaagagtttgggcttcttggaaagcggttctggttctgggggaggaacgctgaagtacgtggaagatgtcacaaatgtcgtgaggagagacgtggagaaatggggcccctttgacctggtgtacggctcgacgcagcccctaggcagctcttgtgatcgctgtcccggctggtacatgttccagttccaccggatcctgcagtatgcgctgcctcgccaggagagtcagcggcccttcttctggatattcatggacaatctgctgctgactgaggatgaccaagagacaactacccgcttccttcagacagaggctgtgaccctccaggatgtccgtggcagagactaccagaatgctatgcgggtgtggagcaacattccagggctgaagagcaagcatgcgcccctgaccccaaaggaagaagagtatctgcaagcccaagtcagaagcaggagcaagctggacgccccgaaagttgacctcctggtgaagaactgccttctcccgctgagagagtacttcaagtatttttctcaaaactcacttcctcttggagggccgagctctggcgcacccccaccaagtggagggtctcctgccgggtccccaacatctactgaagaaggcaccagcgaatccgcaacgcccgagtcaggccctggtacctccacagaaccatctgaaggtagtgcgcctggttccccagctggaagccctacttccaccgaagaaggcacgtcaaccgaaccaagtgaaggatctgcccctgggaccagcactgaaccatctgagccaaaaaagaagagaaaggtaatggacaagaagtacagcatcggcctggccatcggcaccaactctgtgggctgggccgtgatcaccgacgagtacaaggtgcccagcaagaaattcaaggtgctgggcaacaccgaccggcacagcatcaagaagaacctgatcggcgccctgctgttcgacagcggagaaacagccgaggccacccggctgaagagaaccgccagaagaagatacaccagacggaagaaccggatctgctatctgcaagagatcttcagcaacgagatggccaaggtggacgacagcttcttccacagactggaagagtccttcctggtggaagaggataagaagcacgagcggcaccccatcttcggcaacatcgtggacgaggtggcctaccacgagaagtaccccaccatctaccacctgagaaagaaactggtggacagcaccgacaaggccgacctgcggctgatctatctggccctggcccacatgatcaagttccggggccacttcctgatcgagggcgacctgaaccccgacaacagcgacgtggacaagctgttcatccagctggtgcagacctacaaccagctgttcgaggaaaaccccatcaacgccagcggcgtggacgccaaggccatcctgtctgccagactgagcaagagcagacggctggaaaatctgatcgcccagctgcccggcgagaagaagaatggcctgttcggcaacctgattgccctgagcctgggcctgacccccaacttcaagagcaacttcgacctggccgaggatgccaaactgcagctgagcaaggacacctacgacgacgacctggacaacctgctggcccagatcggcgaccagtacgccgacctgtttctggccgccaagaacctgtccgacgccatcctgctgagcgacatcctgagagtgaacaccgagatcaccaaggcccccctgagcgcctctatgatcaagagatacgacgagcaccaccaggacctgaccctgctgaaagctctcgtgcggcagcagctgcctgagaagtacaaagagattttcttcgaccagagcaagaacggctacgccggctacatcgatggcggagccagccaggaagagttctacaagttcatcaagcccatcctggaaaagatggacggcaccgaggaactgctcgtgaagctgaacagagaggacctgctgcggaagcagcggaccttcgacaacggcagcatcccccaccagatccacctgggagagctgcacgccattctgcggcggcaggaagatttttacccattcctgaaggacaaccgggaaaagatcgagaagatcctgaccttccgcatcccctactacgtgggccctctggccaggggaaacagcagattcgcctggatgaccagaaagagcgaggaaaccatcaccccctggaacttcgaggaagtggtggacaagggcgccagcgcccagagcttcatcgagcggatgaccaacttcgataagaacctgcccaacgagaaggtgctgcccaagcacagcctgctgtacgagtacttcaccgtgtacaacgagctgaccaaagtgaaatacgtgaccgagggaatgagaaagcccgccttcctgagcggcgagcagaaaaaagccatcgtggacctgctgttcaagaccaaccggaaagtgaccgtgaagcagctgaaagaggactacttcaagaaaatcgagtgcttcgactccgtggaaatctccggcgtggaagatcggttcaacgcctccctgggcacataccacgatctgctgaaaattatcaaggacaaggacttcctggacaatgaggaaaacgaggacattctggaagatatcgtgctgaccctgacactgtttgaggacagagagatgatcgaggaacggctgaaaacctatgcccacctgttcgacgacaaagtgatgaagcagctgaagcggcggagatacaccggctggggcaggctgagccggaagctgatcaacggcatccgggacaagcagtccggcaagacaatcctggatttcctgaagtccgacggcttcgccaacagaaacttcatgcagctgatccacgacgacagcctgacctttaaagaggacatccagaaagcccaggtgtccggccagggcgatagcctgcacgagcacattgccaatctggccggcagccccgccattaagaagggcatcctgcagacagtgaaggtggtggacgagctcgtgaaagtgatgggccggcacaagcccgagaacatcgtgatcgaaatggccagagagaaccagaccacccagaagggacagaagaacagccgcgagagaatgaagcggatcgaagagggcatcaaagagctgggcagccagatcctgaaagaacaccccgtggaaaacacccagctgcagaacgagaagctgtacctgtactacctgcagaatgggcgggatatgtacgtggaccaggaactggacatcaaccggctgtccgactacgatgtggacgctatcgtgcctcagagctttctgaaggacgactccatcgataacaaagtgctgactcggagcgacaagaaccggggcaagagcgacaacgtgccctccgaagaggtcgtgaagaagatgaagaactactggcgccagctgctgaatgccaagctgattacccagaggaagttcgacaatctgaccaaggccgagagaggcggcctgagcgaactggataaggccggcttcatcaagagacagctggtggaaacccggcagatcacaaagcacgtggcacagatcctggactcccggatgaacactaagtacgacgagaacgacaaactgatccgggaagtgaaagtgatcaccctgaagtccaagctggtgtccgatttccggaaggatttccagttttacaaagtgcgcgagatcaacaactaccaccacgcccacgacgcctacctgaacgccgtcgtgggaaccgccctgatcaaaaagtaccctaagctggaaagcgagttcgtgtacggcgactacaaggtgtacgacgtgcggaagatgatcgccaagagcgagcaggaaatcggcaaggctaccgccaagtacttcttctacagcaacatcatgaactttttcaagaccgagattaccctggccaacggcgagatccggaagcggcctctgatcgagacaaacggcgaaacaggcgagatcgtgtgggataagggccgggactttgccaccgtgcggaaagtgctgtctatgccccaagtgaatatcgtgaaaaagaccgaggtgcagacaggcggcttcagcaaagagtctatcctgcccaagaggaacagcgacaagctgatcgccagaaagaaggactgggaccctaagaagtacggcggcttcgacagccccaccgtggcctattctgtgctggtggtggccaaagtggaaaagggcaagtccaagaaactgaagagtgtgaaagagctgctggggatcaccatcatggaaagaagcagcttcgagaagaatcccatcgactttctggaagccaagggctacaaagaagtgaaaaaggacctgatcatcaagctgcctaagtactccctgttcgagctggaaaacggccggaagagaatgctggcctctgccggcgaactgcagaagggaaacgaactggccctgccctccaaatatgtgaacttcctgtacctggccagccactatgagaagctgaagggctcccccgaggataatgagcagaaacagctgtttgtggaacagcacaaacactacctggacgagatcatcgagcagatcagcgagttctccaagagagtgatcctggccgacgctaatctggacaaggtgctgagcgcctacaacaagcacagagacaagcctatcagagagcaggccgagaatatcatccacctgtttaccctgaccaatctgggagcccctgccgccttcaagtactttgacaccaccatcgaccggaagaggtacaccagcaccaaagaggtgctggacgccaccctgatccaccagagcatcaccggcctgtacgagacacggatcgacctgtctcagctgggaggcgacgcctatccctatgacgtgcccgattatgccagcctgggcagcggctcccccaagaaaaaacgcaaggtggaagatcctaagaaaaagcggaaagtggacggcagcggcagcgagacccccggtaccagcgagagcgccacccccgagagcggtagtgggagcaacggcagcagcggatccatgcgtgaccacatggtccttcatgagtatgtaaatgctgctgggattacagcggccgcaaggtcaggctccggccagcggggaagcaagcgcaccgccgatggttccgagttcgaaagccccaaaaaaaagcgcaaggtctgagatcccaagcacgcagcaatgcagctcaaaacgcttagcctagccacacccccacgggaaacagcagtgattaacctttagcaataaacgaaagtttaactaagctatactaaccccagggttggtcaatttcgtgccagccacaccctggtactgcatgcacgcaatgctagctgcccctttcccgtcctgggcaccccgagtctcccccgaccccgggtcccaggtatgctcccacctccacctgccccactcaccacctctgctagttccagacacctccgagacgaggaaaaaaaaaaaaaaaaaaaaaaaaaaaaaaaaaaaaaaaaaaaaaaaaaaaaaaaaaaaaaaaaaaaaaaaaaaaaaaaaaaaaaaaaaaaaaaaaaaaaaaaaaaaaaaaaaaaaaaaa

SEQ ID NO: 280 - RNA, 7864 nt, synthetic construct
  misc_feature 1..7864: note = mRNA of V39_GFP1-10-ZIM3-2a-D3a-hD3L-dCas9-1xGFP11
  source 1..7864: mol_type = other RNA
aggactcactatttgttttcgcgcccagttgcaaaaagtgtcgacatttgcttctgacacaactgtgttcactagcaacctcaaacagacaccgccaccatgtccaagggagaggagctgttcaccggagtggtgccaatcctggtggagctggacggcgatgtgaacggccacaagttttctgtgcgcggagagggagagggcgacgcaaccatcggcaagctgacactgaagttcatctgcaccacaggcaagctgcccgtgccttggccaaccctggtgaccacactgacatacggcgtgcagtgtttctctaggtatccagaccacatgaagagacacgatttctttaagagcgccatgccagagggatacgtgcaggagcggaccatctccttcaaggacgatggcaagtataagacccgcgccgtggtgaagtttgagggcgatacactggtgaacaggatcgagctgaagggcaccgacttcaaggaggatggcaatatcctgggccacaagctggagtacaactttaatagccacaacgtgtatatcacagccgacaagcagaagaacggcatcaaggccaacttcaccgtgaggcacaatgtggaggacggctccgtgcagctggccgatcactaccagcagaacacacctatcggcgacggacccgtgctgctgcctgataatcactatctgtccacccagacagtgctgtctaaggacccaaacgagaagttggatccaggtggaggtggaagcggtatgaacaattcccagggaagagtgaccttcgaggacgtgaccgtgaacttcacccaaggcgagtggcagagactgaaccccgagcagagaaacctgtaccgggacgtgatgctggaaaactacagcaacctggtgtccgtcggccagggcgagacaacaaagcctgacgtgatcctgcggctggaacagggcaaagagccttggctggaagaggaagaggtgctcggatctggcagagccgagaagaatggcgatatcggcggacagatctggaagccaaaggatgtgaaagagagtctcggaagcggagctactaacttcagcctgctgaagcaggctggagacgtggaggagaaccctggacctatgcctgctgctaagagagtgaaactggatggatccaaccatgaccaggaatttgaccccccaaaggtttacccacctgtgccagctgagaagaggaagcccatccgcgtgctgtctctctttgatgggattgctacagggctcctggtgctgaaggacctgggcatccaagtggaccgctacattgcctccgaggtgtgtgaggactccatcacggtgggcatggtgcggcaccagggaaagatcatgtacgtcggggacgtccgcagcgtcacacagaagcatatccaggagtggggcccattcgacctggtgattggaggcagtccctgcaatgacctctccattgtcaaccctgcccgcaagggactttatgagggtactggccgcctcttctttgagttctaccgcctcctgcatgatgcgcggcccaaggagggagatgatcgccccttcttctggctctttgagaatgtggtggccatgggcgttagtgacaagagggacatctcgcgatttcttgagtctaaccccgtgatgattgacgccaaagaagtgtctgctgcacacagggcccgttacttctggggtaaccttcctggcatgaacaggcctttggcatccactgtgaatgataagctggagctgcaagagtgtctggagcacggcagaatagccaagttcagcaaagtgaggaccattaccaccaggtcaaactctataaagcagggcaaagaccagcatttccccgtgttcatgaacgagaaggaggacatcctgtggtgcactgaaatggaaagggtgtttggcttccccgtccactacacagacgtctccaacatgagccgcttggcgaggcagagactgctgggccgatcgtggagcgtgccggtcatccgccacctcttcgctccgctgaaggaatattttgcttgtgtgtctagcggcaatagtaacgctaacagccgcgggccgagcttcagcagcggcctggtgccgttaagcttgcgcggcagccatatgttcgaaaccgtgcctgtgtggaggagacagccagtccgggtgctgtccctttttgaagacatcaagaaagagctgacgagtttgggctttttggaaagtggttctgacccgggacaactgaagcatgtggttgatgtcacagacacagtgaggaaggatgtggaggagtggggacccttcgatcttgtgtacggcgccacacctcccctgggccacacctgtgaccgtcctcccagctggtacctgttccagttccaccggctcctgcagtacgcacggcccaagccaggcagccccaggcccttcttctggatgttcgtggacaatctggtgctgaacaaggaagacctggacgtcgcatctcgcttcctggagatggagccagtcaccatcccagatgtccacggcggatccttgcagaatgctgtccgcgtgtggagcaacatcccagccataaggagcagcaggcactgggctctggtttcggaagaagaattgtccctgctggcccagaacaagcagagctcgaagctcgcggccaagtggcccaccaagctggtgaagaactgctttctccccctaagagaatatttcaagtatttttcaggagggccgagctctggcgcacccccaccaagtggagggtctcctgccgggtccccaacatctactgaagaaggcaccagcgaatccgcaacgcccgagtcaggccctggtacctccacagaaccatctgaaggtagtgcgcctggttccccagctggaagccctacttccaccgaagaaggcacgtcaaccgaaccaagtgaaggatctgcccctgggaccagcactgaaccatctgagccaaaaaagaagagaaaggtaatggacaagaagtacagcatcggcctggccatcggcaccaactctgtgggctgggccgtgatcaccgacgagtacaaggtgcccagcaagaaattcaaggtgctgggcaacaccgaccggcacagcatcaagaagaacctgatcggcgccctgctgttcgacagcggagaaacagccgaggccacccggctgaagagaaccgccagaagaagatacaccagacggaagaaccggatctgctatctgcaagagatcttcagcaacgagatggccaaggtggacgacagcttcttccacagactggaagagtccttcctggtggaagaggataagaagcacgagcggcaccccatcttcggcaacatcgtggacgaggtggcctaccacgagaagtaccccaccatctaccacctgagaaagaaactggtggacagcaccgacaaggccgacctgcggctgatctatctggccctggcccacatgatcaagttccggggccacttcctgatcgagggcgacctgaaccccgacaacagcgacgtggacaagctgttcatccagctggtgcagacctacaaccagctgttcgaggaaaaccccatcaacgccagcggcgtggacgccaaggccatcctgtctgccagactgagcaagagcagacggctggaaaatctgatcgcccagctgcccggcgagaagaagaatggcctgttcggcaacctgattgccctgagcctgggcctgacccccaacttcaagagcaacttcgacctggccgaggatgccaaactgcagctgagcaaggacacctacgacgacgacctggacaacctgctggcccagatcggcgaccagtacgccgacctgtttctggccgccaagaacctgtccgacgccatcctgctgagcgacatcctgagagtgaacaccgagatcaccaaggcccccctgagcgcctctatgatcaagagatacgacgagcaccaccaggacctgaccctgctgaaagctctcgtgcggcagcagctgcctgagaagtacaaagagattttcttcgaccagagcaagaacggctacgccggctacatcgatggcggagccagccaggaagagttctacaagttcatcaagcccatcctggaaaagatggacggcaccgaggaactgctcgtgaagctgaacagagaggacctgctgcggaagcagcggaccttcgacaacggcagcatcccccaccagatccacctgggagagctgcacgccattctgcggcggcaggaagatttttacccattcctgaaggacaaccgggaaaagatcgagaagatcctgaccttccgcatcccctactacgtgggccctctggccaggggaaacagcagattcgcctggatgaccagaaagagcgaggaaaccatcaccccctggaacttcgaggaagtggtggacaagggcgccagcgcccagagcttcatcgagcggatgaccaacttcgataagaacctgcccaacgagaaggtgctgcccaagcacagcctgctgtacgagtacttcaccgtgtacaacgagctgaccaaagtgaaatacgtgaccgagggaatgagaaagcccgccttcctgagcggcgagcagaaaaaagccatcgtggacctgctgttcaagaccaaccggaaagtgaccgtgaagcagctgaaagaggactacttcaagaaaatcgagtgcttcgactccgtggaaatctccggcgtggaagatcggttcaacgcctccctgggcacataccacgatctgctgaaaattatcaaggacaaggacttcctggacaatgaggaaaacgaggacattctggaagatatcgtgctgaccctgacactgtttgaggacagagagatgatcgaggaacggctgaaaacctatgcccacctgttcgacgacaaagtgatgaagcagctgaagcggcggagatacaccggctggggcaggctgagccggaagctgatcaacggcatccgggacaagcagtccggcaagacaatcctggatttcctgaagtccgacggcttcgccaacagaaacttcatgcagctgatccacgacgacagcctgacctttaaagaggacatccagaaagcccaggtgtccggccagggcgatagcctgcacgagcacattgccaatctggccggcagccccgccattaagaagggcatcctgcagacagtgaaggtggtggacgagctcgtgaaagtgatgggccggcacaagcccgagaacatcgtgatcgaaatggccagagagaaccagaccacccagaagggacagaagaacagccgcgagagaatgaagcggatcgaagagggcatcaaagagctgggcagccagatcctgaaagaacaccccgtggaaaacacccagctgcagaacgagaagctgtacctgtactacctgcagaatgggcgggatatgtacgtggaccaggaactggacatcaaccggctgtccgactacgatgtggacgctatcgtgcctcagagctttctgaaggacgactccatcgataacaaagtgctgactcggagcgacaagaaccggggcaagagcgacaacgtgccctccgaagaggtcgtgaagaagatgaagaactactggcgccagctgctgaatgccaagctgattacccagaggaagttcgacaatctgaccaaggccgagagaggcggcctgagcgaactggataaggccggcttcatcaagagacagctggtggaaacccggcagatcacaaagcacgtggcacagatcctggactcccggatgaacactaagtacgacgagaacgacaaactgatccgggaagtgaaagtgatcaccctgaagtccaagctggtgtccgatttccggaaggatttccagttttacaaagtgcgcgagatcaacaactaccaccacgcccacgacgcctacctgaacgccgtcgtgggaaccgccctgatcaaaaagtaccctaagctggaaagcgagttcgtgtacggcgactacaaggtgtacgacgtgcggaagatgatcgccaagagcgagcaggaaatcggcaaggctaccgccaagtacttcttctacagcaacatcatgaactttttcaagaccgagattaccctggccaacggcgagatccggaagcggcctctgatcgagacaaacggcgaaacaggcgagatcgtgtgggataagggccgggactttgccaccgtgcggaaagtgctgtctatgccccaagtgaatatcgtgaaaaagaccgaggtgcagacaggcggcttcagcaaagagtctatcctgcccaagaggaacagcgacaagctgatcgccagaaagaaggactgggaccctaagaagtacggcggcttcgacagccccaccgtggcctattctgtgctggtggtggccaaagtggaaaagggcaagtccaagaaactgaagagtgtgaaagagctgctggggatcaccatcatggaaagaagcagcttcgagaagaatcccatcgactttctggaagccaagggctacaaagaagtgaaaaaggacctgatcatcaagctgcctaagtactccctgttcgagctggaaaacggccggaagagaatgctggcctctgccggcgaactgcagaagggaaacgaactggccctgccctccaaatatgtgaacttcctgtacctggccagccactatgagaagctgaagggctcccccgaggataatgagcagaaacagctgtttgtggaacagcacaaacactacctggacgagatcatcgagcagatcagcgagttctccaagagagtgatcctggccgacgctaatctggacaaggtgctgagcgcctacaacaagcacagagacaagcctatcagagagcaggccgagaatatcatccacctgtttaccctgaccaatctgggagcccctgccgccttcaagtactttgacaccaccatcgaccggaagaggtacaccagcaccaaagaggtgctggacgccaccctgatccaccagagcatcaccggcctgtacgagacacggatcgacctgtctcagctgggaggcgacgcctatccctatgacgtgcccgattatgccagcctgggcagcggctcccccaagaaaaaacgcaaggtggaagatcctaagaaaaagcggaaagtggacggcagcggcagcgagacccccggtaccagcgagagcgccacccccgagagcggtagtgggagcaacggcagcagcggatccatgcgtgaccacatggtccttcatgagtatgtaaatgctgctgggattacagcggccgcaaggtcaggctccggccagcggggaagcaagcgcaccgccgatggttccgagttcgaaagccccaaaaaaaagcgcaaggtctgagatcccaagcacgcagcaatgcagctcaaaacgcttagcctagccacacccccacgggaaacagcagtgattaacctttagcaataaacgaaagtttaactaagctatactaaccccagggttggtcaatttcgtgccagccacaccctggtactgcatgcacgcaatgctagctgcccctttcccgtcctgggcaccccgagtctcccccgaccccgggtcccaggtatgctcccacctccacctgccccactcaccacctctgctagttccagacacctccgagacgaggaaaaaaaaaaaaaaaaaaaaaaaaaaaaaaaaaaaaaaaaaaaaaaaaaaaaaaaaaaaaaaaaaaaaaaaaaaaaaaaaaaaaaaaaaaaaaaaaaaaaaaaaaaaaaaaaaaaaaaaa

SEQ ID NO: 281 - RNA, 9010 nt, synthetic construct
  misc_feature 1..9010: note = mRNA of V40_GFP1-10-HDAC1-2a-D3a-hD3L-dCas9-1xGFP11
  source 1..9010: mol_type = other RNA
aggactcactatttgttttcgcgcccagttgcaaaaagtgtcgacatttgcttctgacacaactgtgttcactagcaacctcaaacagacaccgccaccatgtccaagggagaggagctgttcaccggagtggtgccaatcctggtggagctggacggcgatgtgaacggccacaagttttctgtgcgcggagagggagagggcgacgcaaccatcggcaagctgacactgaagttcatctgcaccacaggcaagctgcccgtgccttggccaaccctggtgaccacactgacatacggcgtgcagtgtttctctaggtatccagaccacatgaagagacacgatttctttaagagcgccatgccagagggatacgtgcaggagcggaccatctccttcaaggacgatggcaagtataagacccgcgccgtggtgaagtttgagggcgatacactggtgaacaggatcgagctgaagggcaccgacttcaaggaggatggcaatatcctgggccacaagctggagtacaactttaatagccacaacgtgtatatcacagccgacaagcagaagaacggcatcaaggccaacttcaccgtgaggcacaatgtggaggacggctccgtgcagctggccgatcactaccagcagaacacacctatcggcgacggacccgtgctgctgcctgataatcactatctgtccacccagacagtgctgtctaaggacccaaacgagaagttggatccaggtggaggtggaagcggtatggcgcagacgcagggcacccggaggaaagtctgttactactacgacggggatgttggaaattactattatggacaaggccacccaatgaagcctcaccgaatccgcatgactcataatttgctgctcaactatggtctctaccgaaaaatggaaatctatcgccctcacaaagccaatgctgaggagatgaccaagtaccacagcgatgactacattaaattcttgcgctccatccgtccagataacatgtcggagtacagcaagcagatgcagagattcaacgttggtgaggactgtccagtattcgatggcctgtttgagttctgtcagttgtctactggtggttctgtggcaagtgctgtgaaacttaataagcagcagacggacatcgctgtgaattgggctgggggcctgcaccatgcaaagaagtccgaggcatctggcttctgttacgtcaatgatatcgtcttggccatcctggaactgctaaagtatcaccagagggtgctgtacattgacattgatattcaccatggtgacggcgtggaagaggccttctacaccacggaccgggtcatgactgtgtcctttcataagtatggagagtacttcccaggaactggggacctacgggatatcggggctggcaaaggcaagtattatgctgttaactacccgctccgagacgggattgatgacgagtcctatgaggccattttcaagccggtcatgtccaaagtaatggagatgttccagcctagtgcggtggtcttacagtgtggctcagactccctatctggggatcggttaggttgcttcaatctaactatcaaaggacacgccaagtgtgtggaatttgtcaagagctttaacctgcctatgctgatgctgggaggcggtggttacaccattcgtaacgttgcccggtgctggacatatgagacagctgtggccctggatacggagatccctaatgagcttccatacaatgactactttgaatactttggaccagatttcaagctccacatcagtccttccaatatgactaaccagaacacgaatgagtacctggagaagatcaaacagcgactgtttgagaaccttagaatgctgccgcacgcacctggggtccaaatgcaggcgattcctgaggacgccatccctgaggagagtggcgatgaggacgaagacgaccctgacaagcgcatctcgatctgctcctctgacaaacgaattgcctgtgaggaagagttctccgattctgaagaggagggagaggggggccgcaagaactcttccaacttcaaaaaagccaagagagtcaaaacagaggatgaaaaagagaaagacccagaggagaagaaagaagtcaccgaagaggagaaaaccaaggaggagaagccagaagccaaaggggtcaaggaggaggtcaagttggccggaagcggagctactaacttcagcctgctgaagcaggctggagacgtggaggagaaccctggacctatgcctgctgctaagagagtgaaactggatggatccaaccatgaccaggaatttgaccccccaaaggtttacccacctgtgccagctgagaagaggaagcccatccgcgtgctgtctctctttgatgggattgctacagggctcctggtgctgaaggacctgggcatccaagtggaccgctacattgcctccgaggtgtgtgaggactccatcacggtgggcatggtgcggcaccagggaaagatcatgtacgtcggggacgtccgcagcgtcacacagaagcatatccaggagtggggcccattcgacctggtgattggaggcagtccctgcaatgacctctccattgtcaaccctgcccgcaagggactttatgagggtactggccgcctcttctttgagttctaccgcctcctgcatgatgcgcggcccaaggagggagatgatcgccccttcttctggctctttgagaatgtggtggccatgggcgttagtgacaagagggacatctcgcgatttcttgagtctaaccccgtgatgattgacgccaaagaagtgtctgctgcacacagggcccgttacttctggggtaaccttcctggcatgaacaggcctttggcatccactgtgaatgataagctggagctgcaagagtgtctggagcacggcagaatagccaagttcagcaaagtgaggaccattaccaccaggtcaaactctataaagcagggcaaagaccagcatttccccgtgttcatgaacgagaaggaggacatcctgtggtgcactgaaatggaaagggtgtttggcttccccgtccactacacagacgtctccaacatgagccgcttggcgaggcagagactgctgggccgatcgtggagcgtgccggtcatccgccacctcttcgctccgctgaaggaatattttgcttgtgtgtctagcggcaatagtaacgctaacagccgcgggccgagcttcagcagcggcctggtgccgttaagcttgcgcggcagccatatgttcgaaaccgtgcctgtgtggaggagacagccagtccgggtgctgtccctttttgaagacatcaagaaagagctgacgagtttgggctttttggaaagtggttctgacccgggacaactgaagcatgtggttgatgtcacagacacagtgaggaaggatgtggaggagtggggacccttcgatcttgtgtacggcgccacacctcccctgggccacacctgtgaccgtcctcccagctggtacctgttccagttccaccggctcctgcagtacgcacggcccaagccaggcagccccaggcccttcttctggatgttcgtggacaatctggtgctgaacaaggaagacctggacgtcgcatctcgcttcctggagatggagccagtcaccatcccagatgtccacggcggatccttgcagaatgctgtccgcgtgtggagcaacatcccagccataaggagcagcaggcactgggctctggtttcggaagaagaattgtccctgctggcccagaacaagcagagctcgaagctcgcggccaagtggcccaccaagctggtgaagaactgctttctccccctaagagaatatttcaagtatttttcaggagggccgagctctggcgcacccccaccaagtggagggtctcctgccgggtccccaacatctactgaagaaggcaccagcgaatccgcaacgcccgagtcaggccctggtacctccacagaaccatctgaaggtagtgcgcctggttccccagctggaagccctacttccaccgaagaaggcacgtcaaccgaaccaagtgaaggatctgcccctgggaccagcactgaaccatctgagccaaaaaagaagagaaaggtaatggacaagaagtacagcatcggcctggccatcggcaccaactctgtgggctgggccgtgatcaccgacgagtacaaggtgcccagcaagaaattcaaggtgctgggcaacaccgaccggcacagcatcaagaagaacctgatcggcgccctgctgttcgacagcggagaaacagccgaggccacccggctgaagagaaccgccagaagaagatacaccagacggaagaaccggatctgctatctgcaagagatcttcagcaacgagatggccaaggtggacgacagcttcttccacagactggaagagtccttcctggtggaagaggataagaagcacgagcggcaccccatcttcggcaacatcgtggacgaggtggcctaccacgagaagtaccccaccatctaccacctgagaaagaaactggtggacagcaccgacaaggccgacctgcggctgatctatctggccctggcccacatgatcaagttccggggccacttcctgatcgagggcgacctgaaccccgacaacagcgacgtggacaagctgttcatccagctggtgcagacctacaaccagctgttcgaggaaaaccccatcaacgccagcggcgtggacgccaaggccatcctgtctgccagactgagcaagagcagacggctggaaaatctgatcgcccagctgcccggcgagaagaagaatggcctgttcggcaacctgattgccctgagcctgggcctgacccccaacttcaagagcaacttcgacctggccgaggatgccaaactgcagctgagcaaggacacctacgacgacgacctggacaacctgctggcccagatcggcgaccagtacgccgacctgtttctggccgccaagaacctgtccgacgccatcctgctgagcgacatcctgagagtgaacaccgagatcaccaaggcccccctgagcgcctctatgatcaagagatacgacgagcaccaccaggacctgaccctgctgaaagctctcgtgcggcagcagctgcctgagaagtacaaagagattttcttcgaccagagcaagaacggctacgccggctacatcgatggcggagccagccaggaagagttctacaagttcatcaagcccatcctggaaaagatggacggcaccgaggaactgctcgtgaagctgaacagagaggacctgctgcggaagcagcggaccttcgacaacggcagcatcccccaccagatccacctgggagagctgcacgccattctgcggcggcaggaagatttttacccattcctgaaggacaaccgggaaaagatcgagaagatcctgaccttccgcatcccctactacgtgggccctctggccaggggaaacagcagattcgcctggatgaccagaaagagcgaggaaaccatcaccccctggaacttcgaggaagtggtggacaagggcgccagcgcccagagcttcatcgagcggatgaccaacttcgataagaacctgcccaacgagaaggtgctgcccaagcacagcctgctgtacgagtacttcaccgtgtacaacgagctgaccaaagtgaaatacgtgaccgagggaatgagaaagcccgccttcctgagcggcgagcagaaaaaagccatcgtggacctgctgttcaagaccaaccggaaagtgaccgtgaagcagctgaaagaggactacttcaagaaaatcgagtgcttcgactccgtggaaatctccggcgtggaagatcggttcaacgcctccctgggcacataccacgatctgctgaaaattatcaaggacaaggacttcctggacaatgaggaaaacgaggacattctggaagatatcgtgctgaccctgacactgtttgaggacagagagatgatcgaggaacggctgaaaacctatgcccacctgttcgacgacaaagtgatgaagcagctgaagcggcggagatacaccggctggggcaggctgagccggaagctgatcaacggcatccgggacaagcagtccggcaagacaatcctggatttcctgaagtccgacggcttcgccaacagaaacttcatgcagctgatccacgacgacagcctgacctttaaagaggacatccagaaagcccaggtgtccggccagggcgatagcctgcacgagcacattgccaatctggccggcagccccgccattaagaagggcatcctgcagacagtgaaggtggtggacgagctcgtgaaagtgatgggccggcacaagcccgagaacatcgtgatcgaaatggccagagagaaccagaccacccagaagggacagaagaacagccgcgagagaatgaagcggatcgaagagggcatcaaagagctgggcagccagatcctgaaagaacaccccgtggaaaacacccagctgcagaacgagaagctgtacctgtactacctgcagaatgggcgggatatgtacgtggaccaggaactggacatcaaccggctgtccgactacgatgtggacgctatcgtgcctcagagctttctgaaggacgactccatcgataacaaagtgctgactcggagcgacaagaaccggggcaagagcgacaacgtgccctccgaagaggtcgtgaagaagatgaagaactactggcgccagctgctgaatgccaagctgattacccagaggaagttcgacaatctgaccaaggccgagagaggcggcctgagcgaactggataaggccggcttcatcaagagacagctggtggaaacccggcagatcacaaagcacgtggcacagatcctggactcccggatgaacactaagtacgacgagaacgacaaactgatccgggaagtgaaagtgatcaccctgaagtccaagctggtgtccgatttccggaaggatttccagttttacaaagtgcgcgagatcaacaactaccaccacgcccacgacgcctacctgaacgccgtcgtgggaaccgccctgatcaaaaagtaccctaagctggaaagcgagttcgtgtacggcgactacaaggtgtacgacgtgcggaagatgatcgccaagagcgagcaggaaatcggcaaggctaccgccaagtacttcttctacagcaacatcatgaactttttcaagaccgagattaccctggccaacggcgagatccggaagcggcctctgatcgagacaaacggcgaaacaggcgagatcgtgtgggataagggccgggactttgccaccgtgcggaaagtgctgtctatgccccaagtgaatatcgtgaaaaagaccgaggtgcagacaggcggcttcagcaaagagtctatcctgcccaagaggaacagcgacaagctgatcgccagaaagaaggactgggaccctaagaagtacggcggcttcgacagccccaccgtggcctattctgtgctggtggtggccaaagtggaaaagggcaagtccaagaaactgaagagtgtgaaagagctgctggggatcaccatcatggaaagaagcagcttcgagaagaatcccatcgactttctggaagccaagggctacaaagaagtgaaaaaggacctgatcatcaagctgcctaagtactccctgttcgagctggaaaacggccggaagagaatgctggcctctgccggcgaactgcagaagggaaacgaactggccctgccctccaaatatgtgaacttcctgtacctggccagccactatgagaagctgaagggctcccccgaggataatgagcagaaacagctgtttgtggaacagcacaaacactacctggacgagatcatcgagcagatcagcgagttctccaagagagtgatcctggccgacgctaatctggacaaggtgctgagcgcctacaacaagcacagagacaagcctatcagagagcaggccgagaatatcatccacctgtttaccctgaccaatctgggagcccctgccgccttcaagtactttgacaccaccatcgaccggaagaggtacaccagcaccaaagaggtgctggacgccaccctgatccaccagagcatcaccggcctgtacgagacacggatcgacctgtctcagctgggaggcgacgcctatccctatgacgtgcccgattatgccagcctgggcagcggctcccccaagaaaaaacgcaaggtggaagatcctaagaaaaagcggaaagtggacggcagcggcagcgagacccccggtaccagcgagagcgccacccccgagagcggtagtgggagcaacggcagcagcggatccatgcgtgaccacatggtccttcatgagtatgtaaatgctgctgggattacagcggccgcaaggtcaggctccggccagcggggaagcaagcgcaccgccgatggttccgagttcgaaagccccaaaaaaaagcgcaaggtctgagatcccaagcacgcagcaatgcagctcaaaacgcttagcctagccacacccccacgggaaacagcagtgattaacctttagcaataaacgaaagtttaactaagctatactaaccccagggttggtcaatttcgtgccagccacaccctggtactgcatgcacgcaatgctagctgcccctttcccgtcctgggcaccccgagtctcccccgaccccgggtcccaggtatgctcccacctccacctgccccactcaccacctctgctagttccagacacctccgagacgaggaaaaaaaaaaaaaaaaaaaaaaaaaaaaaaaaaaaaaaaaaaaaaaaaaaaaaaaaaaaaaaaaaaaaaaaaaaaaaaaaaaaaaaaaaaaaaaaaaaaaaaaaaaaaaaaaaaaaaaaa

SEQ ID NO: 282 - RNA, 7444 nt, synthetic construct
  misc_feature 1..7444: note = mRNA of V41_GFP1-10-ZIM3-2a-D3a-hD3L-dCas12a-1xGFP11
  source 1..7444: mol_type = other RNA
aggactcactatttgttttcgcgcccagttgcaaaaagtgtcgacatttgcttctgacacaactgtgttcactagcaacctcaaacagacaccgccaccatgtccaagggagaggagctgttcaccggagtggtgccaatcctggtggagctggacggcgatgtgaacggccacaagttttctgtgcgcggagagggagagggcgacgcaaccatcggcaagctgacactgaagttcatctgcaccacaggcaagctgcccgtgccttggccaaccctggtgaccacactgacatacggcgtgcagtgtttctctaggtatccagaccacatgaagagacacgatttctttaagagcgccatgccagagggatacgtgcaggagcggaccatctccttcaaggacgatggcaagtataagacccgcgccgtggtgaagtttgagggcgatacactggtgaacaggatcgagctgaagggcaccgacttcaaggaggatggcaatatcctgggccacaagctggagtacaactttaatagccacaacgtgtatatcacagccgacaagcagaagaacggcatcaaggccaacttcaccgtgaggcacaatgtggaggacggctccgtgcagctggccgatcactaccagcagaacacacctatcggcgacggacccgtgctgctgcctgataatcactatctgtccacccagacagtgctgtctaaggacccaaacgagaagttggatccaggtggaggtggaagcggtatgaacaattcccagggaagagtgaccttcgaggacgtgaccgtgaacttcacccaaggcgagtggcagagactgaaccccgagcagagaaacctgtaccgggacgtgatgctggaaaactacagcaacctggtgtccgtcggccagggcgagacaacaaagcctgacgtgatcctgcggctggaacagggcaaagagccttggctggaagaggaagaggtgctcggatctggcagagccgagaagaatggcgatatcggcggacagatctggaagccaaaggatgtgaaagagagtctcggaagcggagctactaacttcagcctgctgaagcaggctggagacgtggaggagaaccctggacctatgcctgctgctaagagagtgaaactggatggatccaaccatgaccaggaatttgaccccccaaaggtttacccacctgtgccagctgagaagaggaagcccatccgcgtgctgtctctctttgatgggattgctacagggctcctggtgctgaaggacctgggcatccaagtggaccgctacattgcctccgaggtgtgtgaggactccatcacggtgggcatggtgcggcaccagggaaagatcatgtacgtcggggacgtccgcagcgtcacacagaagcatatccaggagtggggcccattcgacctggtgattggaggcagtccctgcaatgacctctccattgtcaaccctgcccgcaagggactttatgagggtactggccgcctcttctttgagttctaccgcctcctgcatgatgcgcggcccaaggagggagatgatcgccccttcttctggctctttgagaatgtggtggccatgggcgttagtgacaagagggacatctcgcgatttcttgagtctaaccccgtgatgattgacgccaaagaagtgtctgctgcacacagggcccgttacttctggggtaaccttcctggcatgaacaggcctttggcatccactgtgaatgataagctggagctgcaagagtgtctggagcacggcagaatagccaagttcagcaaagtgaggaccattaccaccaggtcaaactctataaagcagggcaaagaccagcatttccccgtgttcatgaacgagaaggaggacatcctgtggtgcactgaaatggaaagggtgtttggcttccccgtccactacacagacgtctccaacatgagccgcttggcgaggcagagactgctgggccgatcgtggagcgtgccggtcatccgccacctcttcgctccgctgaaggaatattttgcttgtgtgtctagcggcaatagtaacgctaacagccgcgggccgagcttcagcagcggcctggtgccgttaagcttgcgcggcagccatatgttcgaaaccgtgcctgtgtggaggagacagccagtccgggtgctgtccctttttgaagacatcaagaaagagctgacgagtttgggctttttggaaagtggttctgacccgggacaactgaagcatgtggttgatgtcacagacacagtgaggaaggatgtggaggagtggggacccttcgatcttgtgtacggcgccacacctcccctgggccacacctgtgaccgtcctcccagctggtacctgttccagttccaccggctcctgcagtacgcacggcccaagccaggcagccccaggcccttcttctggatgttcgtggacaatctggtgctgaacaaggaagacctggacgtcgcatctcgcttcctggagatggagccagtcaccatcccagatgtccacggcggatccttgcagaatgctgtccgcgtgtggagcaacatcccagccataaggagcagcaggcactgggctctggtttcggaagaagaattgtccctgctggcccagaacaagcagagctcgaagctcgcggccaagtggcccaccaagctggtgaagaactgctttctccccctaagagaatatttcaagtatttttcaggagggccgagctctggcgcacccccaccaagtggagggtctcctgccgggtccccaacatctactgaagaaggcaccagcgaatccgcaacgcccgagtcaggccctggtacctccacagaaccatctgaaggtagtgcgcctggttccccagctggaagccctacttccaccgaagaaggcacgtcaaccgaaccaagtgaaggatctgcccctgggaccagcactgaaccatctgagccaaaaaagaagagaaaggtaatgtcaaagctggagaaattcaccaactgttatagcctgtctaagaccctgcgcttcaaggcaatcccagtgggcaagacacaagagaacattgacaacaaacggctcctggtggaggatgagaagagggctgaagattacaagggcgttaagaagctgctggataggtactatctgtcattcatcaacgatgtcctccacagtatcaagctgaagaatctgaacaattacatttctctgttccggaagaagacacggaccgagaaggagaacaaagagctggagaatctggagatcaacctgaggaaagaaatagctaaggctttcaaagggaacgagggttacaagtccctgttcaagaaagacattatcgagactattctgcctgagttcctggacgataaagatgagatcgccctcgtcaattccttcaatgggtttaccacagcctttaccggcttcttcgacaatagagagaatatgttctctgaagaggccaaatccactagcatcgcctttcgctgcataaacgagaacctgactaggtacatcagcaatatggacatctttgagaaagtcgatgccatattcgacaaacatgaggtgcaggagattaaggagaagatcctgaactcagattacgatgtcgaagatttcttcgagggagagttcttcaacttcgtgctcacacaagagggcattgatgtgtacaatgcaatcattggagggttcgtgacagagagtggcgagaagataaagggcctgaacgagtatatcaacctctacaaccagaaaaccaagcagaaactgcctaagttcaagccactgtacaaacaagtgctctcagatagggaaagcctgagcttctacggtgaagggtatacatcagatgaagaagtgctcgaagtgttccgcaacaccctcaataagaacagtgaaatcttctcttcaatcaagaagctggagaaactgttcaagaatttcgatgagtactcctctgccggaatctttgtgaagaatggccctgcaatatccactattagcaaagacatctttggcgagtggaacgttatcagggataagtggaatgccgagtacgatgatattcatctcaagaagaaagccgtggttacagagaaatacgaggatgatagacgcaagagctttaagaagattggtagcttctctctcgaacagctgcaggagtacgccgacgctgacctgtcagtcgtggagaaactcaaggagatcataatccagaaggtggatgaaatctacaaagtgtatggaagctctgagaaactcttcgatgcagactttgttctggagaagagtctgaagaagaacgacgcagtggttgctatcatgaaggacctgctggattctgttaagtctttcgagaattacattaaggcattctttggtgaagggaaggagacaaatagggacgagagcttctatggcgactttgttctggcctacgacatcctcctcaaggttgaccacatctatgacgctatacggaattacgttacccagaagccctatagcaaagacaagttcaagctgtatttccagaatccacagtttatgggtgggtgggataaagacaaagaaacagattacagggccactatcctgcggtacggcagcaaatactatctggctatcatggataagaagtacgccaaatgcctccagaagatcgacaaggacgacgtgaacggtaactacgagaagatcaattacaagctcctgccaggacctaacaagatgctgcccaaggtgttcttctccaagaaatggatggcctactataacccaagcgaggacattcagaagatatacaagaatgggacattcaagaagggcgatatgttcaacctcaacgactgccacaagctgattgatttcttcaaggatagcatttctcgctatcccaagtggtctaatgcatacgatttcaacttcagcgagactgagaagtacaaagacatcgctggcttctaccgggaggtggaagagcaaggctataaggtgtcattcgaatccgcttctaagaaggaagtggataagctcgtggaagagggtaagctgtacatgttccagatatacaacaaagacttcagcgataagagccacggcactccaaacctccatactatgtatttcaagctgctgtttgacgagaacaaccacggacagattaggctgtcaggaggcgcagaactcttcatgcgcagagcttcactgaagaaggaggaactcgttgtccacccagccaatagccctatagccaataagaatccagacaatcctaagaaaaccactactctgtcttacgatgtgtataaggataagagattctctgaagatcagtacgaactgcacatacccattgccattaacaagtgccctaagaacatcttcaagattaacacagaggttagagtgctcctgaaacacgacgataacccttatgttataggcattgctcgcggagagagaaacctgctgtacatcgtcgtggtggacggcaaaggcaacatcgtggaacagtacagtctcaatgaaatcattaacaatttcaacggaatccgcattaagaccgactaccattctctcctcgacaagaaggagaaagaaaggttcgaagcaagacagaattggacaagtatagagaatatcaaagaactgaaggctgggtacatctctcaggttgtgcacaagatatgtgagctggtggagaagtacgacgctgttatcgccctcgcggacctgaatagcggcttcaagaactccagggtgaaggtggagaagcaggtgtatcagaagttcgagaagatgctgatcgacaagctcaactatatggtggacaagaaatccaatccttgcgctactggtggagccctgaagggctatcaaatcaccaataagttcgaatctttcaagtctatgagcacccagaatggcttcatcttctacatacccgcatggctgacatccaagattgatccctctaccggatttgttaatctgctcaagactaagtacacctctattgctgactcaaagaagttcatatcatcatttgaccgcatcatgtacgtgccagaagaggacctgttcgagtttgccctggattacaagaatttctctcggactgacgccgactacatcaagaagtggaagctctactcttatggtaatcggattcgcatattccgcaatcccaagaagaataacgtgttcgattgggaggaagtttgcctcaccagcgcttacaaggagctgttcaataagtatgggattaactaccagcagggcgacataagagccctgctgtgcgaacaatctgataaggcattctattcctctttcatggcactgatgtcactgatgctgcaaatgcgcaattccatcaccggaagaacagacgtggcctttctgatctctcctgtcaagaactcagatggcatcttctacgattcccgcaactatgaagcacaggagaatgctatcctgcctaagaatgccgatgcaaatggagcctataacatcgccagaaaggtcctctgggccataggacaattcaagaaagctgaagatgagaagctggacaaggtgaagatcgccatttcaaacaaagagtggctcgaatatgctcagacctcagtgaagcatgcctatccctatgacgtgcccgattatgccagcctgggcagcggctcccccaagaaaaaacgcaaggtggaagatcctaagaaaaagcggaaagtggacggcagcggcagcgagacccccggtaccagcgagagcgccacccccgagagcggtagtgggagcaacggcagcagcggatccatgcgtgaccacatggtccttcatgagtatgtaaatgctgctgggattacagcggccgcaaggtcaggctccggccagcggggaagcaagcgcaccgccgatggttccgagttcgaaagccccaaaaaaaagcgcaaggtctgagatcccaagcacgcagcaatgcagctcaaaacgcttagcctagccacacccccacgggaaacagcagtgattaacctttagcaataaacgaaagtttaactaagctatactaaccccagggttggtcaatttcgtgccagccacaccctggtactgcatgcacgcaatgctagctgcccctttcccgtcctgggcaccccgagtctcccccgaccccgggtcccaggtatgctcccacctccacctgccccactcaccacctctgctagttccagacacctccgagacgaggaaaaaaaaaaaaaaaaaaaaaaaaaaaaaaaaaaaaaaaaaaaaaaaaaaaaaaaaaaaaaaaaaaaaaaaaaaaaaaaaaaaaaaaaaaaaaaaaaaaaaaaaaaaaaaaaaaaaaaaa

SEQ ID NO: 283 - RNA, 6793 nt, synthetic construct
  misc_feature 1..6793: note = mRNA of V42_GFP1-10-ZIM3-2a-D3a-hD3L-dCas12i-1xGFP11
  source 1..6793: mol_type = other RNA
aggactcactatttgttttcgcgcccagttgcaaaaagtgtcgacatttgcttctgacacaactgtgttcactagcaacctcaaacagacaccgccaccatgtccaagggagaggagctgttcaccggagtggtgccaatcctggtggagctggacggcgatgtgaacggccacaagttttctgtgcgcggagagggagagggcgacgcaaccatcggcaagctgacactgaagttcatctgcaccacaggcaagctgcccgtgccttggccaaccctggtgaccacactgacatacggcgtgcagtgtttctctaggtatccagaccacatgaagagacacgatttctttaagagcgccatgccagagggatacgtgcaggagcggaccatctccttcaaggacgatggcaagtataagacccgcgccgtggtgaagtttgagggcgatacactggtgaacaggatcgagctgaagggcaccgacttcaaggaggatggcaatatcctgggccacaagctggagtacaactttaatagccacaacgtgtatatcacagccgacaagcagaagaacggcatcaaggccaacttcaccgtgaggcacaatgtggaggacggctccgtgcagctggccgatcactaccagcagaacacacctatcggcgacggacccgtgctgctgcctgataatcactatctgtccacccagacagtgctgtctaaggacccaaacgagaagttggatccaggtggaggtggaagcggtatgaacaattcccagggaagagtgaccttcgaggacgtgaccgtgaacttcacccaaggcgagtggcagagactgaaccccgagcagagaaacctgtaccgggacgtgatgctggaaaactacagcaacctggtgtccgtcggccagggcgagacaacaaagcctgacgtgatcctgcggctggaacagggcaaagagccttggctggaagaggaagaggtgctcggatctggcagagccgagaagaatggcgatatcggcggacagatctggaagccaaaggatgtgaaagagagtctcggaagcggagctactaacttcagcctgctgaagcaggctggagacgtggaggagaaccctggacctatgcctgctgctaagagagtgaaactggatggatccaaccatgaccaggaatttgaccccccaaaggtttacccacctgtgccagctgagaagaggaagcccatccgcgtgctgtctctctttgatgggattgctacagggctcctggtgctgaaggacctgggcatccaagtggaccgctacattgcctccgaggtgtgtgaggactccatcacggtgggcatggtgcggcaccagggaaagatcatgtacgtcggggacgtccgcagcgtcacacagaagcatatccaggagtggggcccattcgacctggtgattggaggcagtccctgcaatgacctctccattgtcaaccctgcccgcaagggactttatgagggtactggccgcctcttctttgagttctaccgcctcctgcatgatgcgcggcccaaggagggagatgatcgccccttcttctggctctttgagaatgtggtggccatgggcgttagtgacaagagggacatctcgcgatttcttgagtctaaccccgtgatgattgacgccaaagaagtgtctgctgcacacagggcccgttacttctggggtaaccttcctggcatgaacaggcctttggcatccactgtgaatgataagctggagctgcaagagtgtctggagcacggcagaatagccaagttcagcaaagtgaggaccattaccaccaggtcaaactctataaagcagggcaaagaccagcatttccccgtgttcatgaacgagaaggaggacatcctgtggtgcactgaaatggaaagggtgtttggcttccccgtccactacacagacgtctccaacatgagccgcttggcgaggcagagactgctgggccgatcgtggagcgtgccggtcatccgccacctcttcgctccgctgaaggaatattttgcttgtgtgtctagcggcaatagtaacgctaacagccgcgggccgagcttcagcagcggcctggtgccgttaagcttgcgcggcagccatatgttcgaaaccgtgcctgtgtggaggagacagccagtccgggtgctgtccctttttgaagacatcaagaaagagctgacgagtttgggctttttggaaagtggttctgacccgggacaactgaagcatgtggttgatgtcacagacacagtgaggaaggatgtggaggagtggggacccttcgatcttgtgtacggcgccacacctcccctgggccacacctgtgaccgtcctcccagctggtacctgttccagttccaccggctcctgcagtacgcacggcccaagccaggcagccccaggcccttcttctggatgttcgtggacaatctggtgctgaacaaggaagacctggacgtcgcatctcgcttcctggagatggagccagtcaccatcccagatgtccacggcggatccttgcagaatgctgtccgcgtgtggagcaacatcccagccataaggagcagcaggcactgggctctggtttcggaagaagaattgtccctgctggcccagaacaagcagagctcgaagctcgcggccaagtggcccaccaagctggtgaagaactgctttctccccctaagagaatatttcaagtatttttcaggagggccgagctctggcgcacccccaccaagtggagggtctcctgccgggtccccaacatctactgaagaaggcaccagcgaatccgcaacgcccgagtcaggccctggtacctccacagaaccatctgaaggtagtgcgcctggttccccagctggaagccctacttccaccgaagaaggcacgtcaaccgaaccaagtgaaggatctgcccctgggaccagcactgaaccatctgagccaaaaaagaagagaaaggtaatgggcatcaccatgagcgacaccaccttcagaccctacaagagcaagctgaaccccaacgagcggaagatgcctatggtggtggacaccatgaattggtgcgacaacgcctgcagcgtgttcttcgatctgttcgtgggcctgtacggcggcgtgaagatcggcgacgtgaccaatttcctgaccgagaagcaggacaccaccaccgatgccgatctgctgtgcgccatcaactggttcagagccatgcctgtgtctaaccccgatgccgttgtgggacctgagcagctggttgtgcggttcagagactacagcggccacaatccatctccaatggccagcatgtacctgagcgcccctgtgaaccctagatacacctgggtcgactgccggttcctgtaccagcagatgtgtcagaccctgggcgccaacctggatgtggacatctctaccctggtgcagaccggcctgctgcctatccagaaggatacacagctgaacgcctacagcttctgcagcaacgtgttcggcgagggcgtgaaagaagatcccagcgccaaagtgaccagctacacagccgctgccaatgctctgagcggcgccaccaatcctatcatcacctacgaggactaccggcagatcctgtccagcgccatcaccaacagacccagcagaaagggcgccaaggatattctggccgccgatctggatagcaccaagacaggtgttctgcccggcaactacgtgtcccagagaatcgccatgtaccaggcctctgccgcctctaaagctagaggcgtggtgctgcccaaccggctgagagtgaaagcctacctgcagaacctcgtgggactgaactacatctgcaccacctgggccgctcctatgctgagagccgtgggcgacatcaagagcaagaacagcaacaactaccgcttcgtgggcgagagactggaacggcagcaagagatcgataacctgctggccgtgtccaacatcagaagcgcccaggccatcctgcagcagttcagggccaatgagagcaaccagttctacatcaagaagcggcacatcggcaagggcctgcctagcctgtacgacatgtgggatctgatggacgagaaagagggcatcgacaactacatccagagcctgaagggcgacaagaccgagaggctgccaatcagagagctgctgcagatcatctaccctcacagaaagagcgtgtccgccgagctgtttctgtctgccgccgaactgaccgacgtggaagatagacagaaccggtgcatggtgcaccctacagtgcggggctctctggtcatcaacttcggcaagagcagcaccatcttcggcgctatcacccctcctgacacactgatcaagttccggggcgaaatggtgcctgctggacagacaggcatgatctggttcacaatgcacctggtggacggcggcaaatgggtcaagcaccacattccttgccacagcagccggtacttcgaggaaatctacgcctggaagaaggacctgcctacactgccctttccacggcggagcctgtatggctatgccatcggcaacaagatcagcgacacccggaagatcgacctgcggagaaagaaggccagcaagcagtacctgcggaccctggaaaacatgacccacaacgtggaatttgaccccaccacacagttcatggtggaccaagagctgaacgtgaccatcaccgccagagtgaagaaaatccctcctgtgcgggatgtgcccgtgggcagcagaattatgggcctgaacaagaaccagaccatccgggactgctacagcatctgggagagagtggaagccaacaccagcggcagctttcagcatcccgtggtccaggatgtgtggctgagactggtggccgatggccacgtgacctctacagtgaatggccccaacggccagatcgaccagatgagctactctggccccgatgtggccaactgcggcaactggatgcaagagcggagcaacttcatcaccagcgtggacgacgccgaccagtctatcatgaagcactttctgtggaacaaccgcgtgaagctgtatgcctggaactgcgtgtacgccggcacactgatgaaggccatctctaagcagatgaccaccgccaaccggaacctgttcagaaacgagatcctgagcttcgttggcggcagattcggctgcagactgggatctctggcccaggtttcactggacctgctgcggaggatgaagtccgtgatcagctgctacttcagccggaacaacgccttcaccatcgaggaaagaagcgccttcgacaaagaactgatggaactgttcgagagcctggacaacaagatgaacaacaagcggaaagagaaagtcaaccggacactcagcagcatcttccaggtggccaagcagcacaatgttgtgcggctggtggtcaccaagaacctgcagacccctgatgccaatgtgcggagcgtgatgaatcagagatccgtggattggtgcgctcggaagattgaagagaagatcgtggacctgggcaacgtgatcggaatctatgtggatctggtggaagccctggatctgagccatctggaccccttcatctatatcgccaagggcgacgtgggcaaagagtgccagtttgacgaggtggaaagcagctccctgctgccaattcacaccagcatgtttcgcgactggcacggcctggttaacaagggcagaaccaccacacctatctaccacagcgccctgaggagcttcgccagccactacggcctgagattcgatgacctggccagaatcaaggccgctgagctggccaaaatgctgccagaccagaaggtgttcatcccacacagaggcggacggttcttcatgagcacataccccgtgaccagcaccagcagacccgtgtcttatgatggccggcagcggttcctgaacagcggcgatatggtggccccagtgaacaccatgctgcgcggattcagaagggccagatctgcctatccctatgacgtgcccgattatgccagcctgggcagcggctcccccaagaaaaaacgcaaggtggaagatcctaagaaaaagcggaaagtggacggcagcggcagcgagacccccggtaccagcgagagcgccacccccgagagcggtagtgggagcaacggcagcagcggatccatgcgtgaccacatggtccttcatgagtatgtaaatgctgctgggattacagcggccgcaaggtcaggctccggccagcggggaagcaagcgcaccgccgatggttccgagttcgaaagccccaaaaaaaagcgcaaggtctgagatcccaagcacgcagcaatgcagctcaaaacgcttagcctagccacacccccacgggaaacagcagtgattaacctttagcaataaacgaaagtttaactaagctatactaaccccagggttggtcaatttcgtgccagccacaccctggtactgcatgcacgcaatgctagctgcccctttcccgtcctgggcaccccgagtctcccccgaccccgggtcccaggtatgctcccacctccacctgccccactcaccacctctgctagttccagacacctccgagacgaggaaaaaaaaaaaaaaaaaaaaaaaaaaaaaaaaaaaaaaaaaaaaaaaaaaaaaaaaaaaaaaaaaaaaaaaaaaaaaaaaaaaaaaaaaaaaaaaaaaaaaaaaaaaaaaaaaaaaaaaa

SEQ ID NO: 284 - RNA, 7687 nt, synthetic construct
  misc_feature 1..7687: note = mRNA of V43_D3a-D3l-GFP1-10-2a-1xGFP11-dCas9-KRAB
  source 1..7687: mol_type = other RNA
aggactcactatttgttttcgcgcccagttgcaaaaagtgtcgacatttgcttctgacacaactgtgttcactagcaacctcaaacagacaccgccaccatgcctgctgctaagagagtgaaactggatggatccaaccatgaccaggaatttgaccccccaaaggtttacccacctgtgccagctgagaagaggaagcccatccgcgtgctgtctctctttgatgggattgctacagggctcctggtgctgaaggacctgggcatccaagtggaccgctacattgcctccgaggtgtgtgaggactccatcacggtgggcatggtgcggcaccagggaaagatcatgtacgtcggggacgtccgcagcgtcacacagaagcatatccaggagtggggcccattcgacctggtgattggaggcagtccctgcaatgacctctccattgtcaaccctgcccgcaagggactttatgagggtactggccgcctcttctttgagttctaccgcctcctgcatgatgcgcggcccaaggagggagatgatcgccccttcttctggctctttgagaatgtggtggccatgggcgttagtgacaagagggacatctcgcgatttcttgagtctaaccccgtgatgattgacgccaaagaagtgtctgctgcacacagggcccgttacttctggggtaaccttcctggcatgaacaggcctttggcatccactgtgaatgataagctggagctgcaagagtgtctggagcacggcagaatagccaagttcagcaaagtgaggaccattaccaccaggtcaaactctataaagcagggcaaagaccagcatttccccgtgttcatgaacgagaaggaggacatcctgtggtgcactgaaatggaaagggtgtttggcttccccgtccactacacagacgtctccaacatgagccgcttggcgaggcagagactgctgggccgatcgtggagcgtgccggtcatccgccacctcttcgctccgctgaaggaatattttgcttgtgtgtctagcggcaatagtaacgctaacagccgcgggccgagcttcagcagcggcctggtgccgttaagcttgcgcggcagccatatgggccctatggagatatacaagacagtgtctgcatggaagagacagccagtgcgggtactgagcctcttcagaaacatcgacaaggtactaaagagtttgggcttcttggaaagcggttctggttctgggggaggaacgctgaagtacgtggaagatgtcacaaatgtcgtgaggagagacgtggagaaatggggcccctttgacctggtgtacggctcgacgcagcccctaggcagctcttgtgatcgctgtcccggctggtacatgttccagttccaccggatcctgcagtatgcgctgcctcgccaggagagtcagcggcccttcttctggatattcatggacaatctgctgctgactgaggatgaccaagagacaactacccgcttccttcagacagaggctgtgaccctccaggatgtccgtggcagagactaccagaatgctatgcgggtgtggagcaacattccagggctgaagagcaagcatgcgcccctgaccccaaaggaagaagagtatctgcaagcccaagtcagaagcaggagcaagctggacgccccgaaagttgacctcctggtgaagaactgccttctcccgctgagagagtacttcaagtatttttctcaaaactcacttcctcttggagggccgagctctggcgcacccccaccaagtggagggtctcctgccgggtccccaacatctactgaagaaggcaccagcgaatccgcaacgatgtccaagggagaggagctgttcaccggagtggtgccaatcctggtggagctggacggcgatgtgaacggccacaagttttctgtgcgcggagagggagagggcgacgcaaccatcggcaagctgacactgaagttcatctgcaccacaggcaagctgcccgtgccttggccaaccctggtgaccacactgacatacggcgtgcagtgtttctctaggtatccagaccacatgaagagacacgatttctttaagagcgccatgccagagggatacgtgcaggagcggaccatctccttcaaggacgatggcaagtataagacccgcgccgtggtgaagtttgagggcgatacactggtgaacaggatcgagctgaagggcaccgacttcaaggaggatggcaatatcctgggccacaagctggagtacaactttaatagccacaacgtgtatatcacagccgacaagcagaagaacggcatcaaggccaacttcaccgtgaggcacaatgtggaggacggctccgtgcagctggccgatcactaccagcagaacacacctatcggcgacggacccgtgctgctgcctgataatcactatctgtccacccagacagtgctgtctaaggacccaaacgagaagttggatccaggtggaggtggaagcggaagcggagctactaacttcagcctgctgaagcaggctggagacgtggaggagaaccctggacctatgcctgctgctaagagagtgaaactggatggatccggccccgacatcgtgatcggtagcggcggtcgggaccatatggtcctgcacgaatatgtcaatgctgccggtatcaccgcggccgcaaggtcaggctccggccagcggggaagcaagcgcaccgccgatggttccgagttcgaaagccccaaaaaaaagcgcaaggtcggcggaagcggaagcggaccaaaaaagaagagaaaggtaatggacaagaagtacagcatcggcctggccatcggcaccaactctgtgggctgggccgtgatcaccgacgagtacaaggtgcccagcaagaaattcaaggtgctgggcaacaccgaccggcacagcatcaagaagaacctgatcggcgccctgctgttcgacagcggagaaacagccgaggccacccggctgaagagaaccgccagaagaagatacaccagacggaagaaccggatctgctatctgcaagagatcttcagcaacgagatggccaaggtggacgacagcttcttccacagactggaagagtccttcctggtggaagaggataagaagcacgagcggcaccccatcttcggcaacatcgtggacgaggtggcctaccacgagaagtaccccaccatctaccacctgagaaagaaactggtggacagcaccgacaaggccgacctgcggctgatctatctggccctggcccacatgatcaagttccggggccacttcctgatcgagggcgacctgaaccccgacaacagcgacgtggacaagctgttcatccagctggtgcagacctacaaccagctgttcgaggaaaaccccatcaacgccagcggcgtggacgccaaggccatcctgtctgccagactgagcaagagcagacggctggaaaatctgatcgcccagctgcccggcgagaagaagaatggcctgttcggcaacctgattgccctgagcctgggcctgacccccaacttcaagagcaacttcgacctggccgaggatgccaaactgcagctgagcaaggacacctacgacgacgacctggacaacctgctggcccagatcggcgaccagtacgccgacctgtttctggccgccaagaacctgtccgacgccatcctgctgagcgacatcctgagagtgaacaccgagatcaccaaggcccccctgagcgcctctatgatcaagagatacgacgagcaccaccaggacctgaccctgctgaaagctctcgtgcggcagcagctgcctgagaagtacaaagagattttcttcgaccagagcaagaacggctacgccggctacatcgatggcggagccagccaggaagagttctacaagttcatcaagcccatcctggaaaagatggacggcaccgaggaactgctcgtgaagctgaacagagaggacctgctgcggaagcagcggaccttcgacaacggcagcatcccccaccagatccacctgggagagctgcacgccattctgcggcggcaggaagatttttacccattcctgaaggacaaccgggaaaagatcgagaagatcctgaccttccgcatcccctactacgtgggccctctggccaggggaaacagcagattcgcctggatgaccagaaagagcgaggaaaccatcaccccctggaacttcgaggaagtggtggacaagggcgccagcgcccagagcttcatcgagcggatgaccaacttcgataagaacctgcccaacgagaaggtgctgcccaagcacagcctgctgtacgagtacttcaccgtgtacaacgagctgaccaaagtgaaatacgtgaccgagggaatgagaaagcccgccttcctgagcggcgagcagaaaaaagccatcgtggacctgctgttcaagaccaaccggaaagtgaccgtgaagcagctgaaagaggactacttcaagaaaatcgagtgcttcgactccgtggaaatctccggcgtggaagatcggttcaacgcctccctgggcacataccacgatctgctgaaaattatcaaggacaaggacttcctggacaatgaggaaaacgaggacattctggaagatatcgtgctgaccctgacactgtttgaggacagagagatgatcgaggaacggctgaaaacctatgcccacctgttcgacgacaaagtgatgaagcagctgaagcggcggagatacaccggctggggcaggctgagccggaagctgatcaacggcatccgggacaagcagtccggcaagacaatcctggatttcctgaagtccgacggcttcgccaacagaaacttcatgcagctgatccacgacgacagcctgacctttaaagaggacatccagaaagcccaggtgtccggccagggcgatagcctgcacgagcacattgccaatctggccggcagccccgccattaagaagggcatcctgcagacagtgaaggtggtggacgagctcgtgaaagtgatgggccggcacaagcccgagaacatcgtgatcgaaatggccagagagaaccagaccacccagaagggacagaagaacagccgcgagagaatgaagcggatcgaagagggcatcaaagagctgggcagccagatcctgaaagaacaccccgtggaaaacacccagctgcagaacgagaagctgtacctgtactacctgcagaatgggcgggatatgtacgtggaccaggaactggacatcaaccggctgtccgactacgatgtggacgctatcgtgcctcagagctttctgaaggacgactccatcgataacaaagtgctgactcggagcgacaagaaccggggcaagagcgacaacgtgccctccgaagaggtcgtgaagaagatgaagaactactggcgccagctgctgaatgccaagctgattacccagaggaagttcgacaatctgaccaaggccgagagaggcggcctgagcgaactggataaggccggcttcatcaagagacagctggtggaaacccggcagatcacaaagcacgtggcacagatcctggactcccggatgaacactaagtacgacgagaacgacaaactgatccgggaagtgaaagtgatcaccctgaagtccaagctggtgtccgatttccggaaggatttccagttttacaaagtgcgcgagatcaacaactaccaccacgcccacgacgcctacctgaacgccgtcgtgggaaccgccctgatcaaaaagtaccctaagctggaaagcgagttcgtgtacggcgactacaaggtgtacgacgtgcggaagatgatcgccaagagcgagcaggaaatcggcaaggctaccgccaagtacttcttctacagcaacatcatgaactttttcaagaccgagattaccctggccaacggcgagatccggaagcggcctctgatcgagacaaacggcgaaacaggcgagatcgtgtgggataagggccgggactttgccaccgtgcggaaagtgctgtctatgccccaagtgaatatcgtgaaaaagaccgaggtgcagacaggcggcttcagcaaagagtctatcctgcccaagaggaacagcgacaagctgatcgccagaaagaaggactgggaccctaagaagtacggcggcttcgacagccccaccgtggcctattctgtgctggtggtggccaaagtggaaaagggcaagtccaagaaactgaagagtgtgaaagagctgctggggatcaccatcatggaaagaagcagcttcgagaagaatcccatcgactttctggaagccaagggctacaaagaagtgaaaaaggacctgatcatcaagctgcctaagtactccctgttcgagctggaaaacggccggaagagaatgctggcctctgccggcgaactgcagaagggaaacgaactggccctgccctccaaatatgtgaacttcctgtacctggccagccactatgagaagctgaagggctcccccgaggataatgagcagaaacagctgtttgtggaacagcacaaacactacctggacgagatcatcgagcagatcagcgagttctccaagagagtgatcctggccgacgctaatctggacaaggtgctgagcgcctacaacaagcacagagacaagcctatcagagagcaggccgagaatatcatccacctgtttaccctgaccaatctgggagcccctgccgccttcaagtactttgacaccaccatcgaccggaagaggtacaccagcaccaaagaggtgctggacgccaccctgatccaccagagcatcaccggcctgtacgagacacggatcgacctgtctcagctgggaggcgacgcctatccctatgacgtgcccgattatgccagcctgggcagcggctcccccaagaaaaaacgcaaggtggaagatcctaagaaaaagcggaaagtggacggcagcggcagcgagacccccggtaccagcgagagcgccacccccgagagccggacactggtgaccttcaaggatgtatttgtggacttcaccagggaggagtggaagctgctggacactgctcagcagatcgtgtacagaaatgtgatgctggagaactataagaacctggtttccttgggttatcagcttactaagccagatgtgatcctccggttggagaagggagaagagccctgagatcccaagcacgcagcaatgcagctcaaaacgcttagcctagccacacccccacgggaaacagcagtgattaacctttagcaataaacgaaagtttaactaagctatactaaccccagggttggtcaatttcgtgccagccacaccctggtactgcatgcacgcaatgctagctgcccctttcccgtcctgggcaccccgagtctcccccgaccccgggtcccaggtatgctcccacctccacctgccccactcaccacctctgctagttccagacacctccgagacgaggaaaaaaaaaaaaaaaaaaaaaaaaaaaaaaaaaaaaaaaaaaaaaaaaaaaaaaaaaaaaaaaaaaaaaaaaaaaaaaaaaaaaaaaaaaaaaaaaaaaaaaaaaaaaaaaaaaaaaaaa

SEQ ID NO: 285 - RNA, 8281 nt, synthetic construct
  misc_feature 1..8281: note = mRNA of V44_7xGFP11-dCas9-ZIM3-2a-D3a-hD3L-GFP1-10
  source 1..8281: mol_type = other RNA
aggactcactatttgttttcgcgcccagttgcaaaaagtgtcgacatttgcttctgacacaactgtgttcactagcaacctcaaacagacaccgccaccatgcctgctgctaagagagtgaaactggatggatccatgcgtgaccacatggtccttcatgagtatgtaaatgctgctgggattacaggtggctctggaggtagagatcatatggttctccacgaatacgttaacgccgcaggcatcactggcggtagtggaggacgcgaccatatggtactacatgaatatgtcaatgcagccggaataaccggagggtccggaggccgggatcacatggtgctgcatgagtatgtgaacgcggcgggtataactggtgggtcgggcggacgagaccatatggtgcttcacgaatacgtaaacgcagctggcattactggcggatcaggtggcagggatcacatggtactccatgagtacgtgaacgctgctggaatcacaggcggtagcggcggtcgggaccatatggtcctgcacgaatatgtcaatgctgccggtatcaccgcggccgcaaggtcaggctccggccagcggggaagcaagcgcaccgccgatggttccgagttcgaaagccccaaaaaaaagcgcaaggtcggcggaagcggaagcggaccaaaaaagaagagaaaggtaatggacaagaagtacagcatcggcctggccatcggcaccaactctgtgggctgggccgtgatcaccgacgagtacaaggtgcccagcaagaaattcaaggtgctgggcaacaccgaccggcacagcatcaagaagaacctgatcggcgccctgctgttcgacagcggagaaacagccgaggccacccggctgaagagaaccgccagaagaagatacaccagacggaagaaccggatctgctatctgcaagagatcttcagcaacgagatggccaaggtggacgacagcttcttccacagactggaagagtccttcctggtggaagaggataagaagcacgagcggcaccccatcttcggcaacatcgtggacgaggtggcctaccacgagaagtaccccaccatctaccacctgagaaagaaactggtggacagcaccgacaaggccgacctgcggctgatctatctggccctggcccacatgatcaagttccggggccacttcctgatcgagggcgacctgaaccccgacaacagcgacgtggacaagctgttcatccagctggtgcagacctacaaccagctgttcgaggaaaaccccatcaacgccagcggcgtggacgccaaggccatcctgtctgccagactgagcaagagcagacggctggaaaatctgatcgcccagctgcccggcgagaagaagaatggcctgttcggcaacctgattgccctgagcctgggcctgacccccaacttcaagagcaacttcgacctggccgaggatgccaaactgcagctgagcaaggacacctacgacgacgacctggacaacctgctggcccagatcggcgaccagtacgccgacctgtttctggccgccaagaacctgtccgacgccatcctgctgagcgacatcctgagagtgaacaccgagatcaccaaggcccccctgagcgcctctatgatcaagagatacgacgagcaccaccaggacctgaccctgctgaaagctctcgtgcggcagcagctgcctgagaagtacaaagagattttcttcgaccagagcaagaacggctacgccggctacatcgatggcggagccagccaggaagagttctacaagttcatcaagcccatcctggaaaagatggacggcaccgaggaactgctcgtgaagctgaacagagaggacctgctgcggaagcagcggaccttcgacaacggcagcatcccccaccagatccacctgggagagctgcacgccattctgcggcggcaggaagatttttacccattcctgaaggacaaccgggaaaagatcgagaagatcctgaccttccgcatcccctactacgtgggccctctggccaggggaaacagcagattcgcctggatgaccagaaagagcgaggaaaccatcaccccctggaacttcgaggaagtggtggacaagggcgccagcgcccagagcttcatcgagcggatgaccaacttcgataagaacctgcccaacgagaaggtgctgcccaagcacagcctgctgtacgagtacttcaccgtgtacaacgagctgaccaaagtgaaatacgtgaccgagggaatgagaaagcccgccttcctgagcggcgagcagaaaaaagccatcgtggacctgctgttcaagaccaaccggaaagtgaccgtgaagcagctgaaagaggactacttcaagaaaatcgagtgcttcgactccgtggaaatctccggcgtggaagatcggttcaacgcctccctgggcacataccacgatctgctgaaaattatcaaggacaaggacttcctggacaatgaggaaaacgaggacattctggaagatatcgtgctgaccctgacactgtttgaggacagagagatgatcgaggaacggctgaaaacctatgcccacctgttcgacgacaaagtgatgaagcagctgaagcggcggagatacaccggctggggcaggctgagccggaagctgatcaacggcatccgggacaagcagtccggcaagacaatcctggatttcctgaagtccgacggcttcgccaacagaaacttcatgcagctgatccacgacgacagcctgacctttaaagaggacatccagaaagcccaggtgtccggccagggcgatagcctgcacgagcacattgccaatctggccggcagccccgccattaagaagggcatcctgcagacagtgaaggtggtggacgagctcgtgaaagtgatgggccggcacaagcccgagaacatcgtgatcgaaatggccagagagaaccagaccacccagaagggacagaagaacagccgcgagagaatgaagcggatcgaagagggcatcaaagagctgggcagccagatcctgaaagaacaccccgtggaaaacacccagctgcagaacgagaagctgtacctgtactacctgcagaatgggcgggatatgtacgtggaccaggaactggacatcaaccggctgtccgactacgatgtggacgctatcgtgcctcagagctttctgaaggacgactccatcgataacaaagtgctgactcggagcgacaagaaccggggcaagagcgacaacgtgccctccgaagaggtcgtgaagaagatgaagaactactggcgccagctgctgaatgccaagctgattacccagaggaagttcgacaatctgaccaaggccgagagaggcggcctgagcgaactggataaggccggcttcatcaagagacagctggtggaaacccggcagatcacaaagcacgtggcacagatcctggactcccggatgaacactaagtacgacgagaacgacaaactgatccgggaagtgaaagtgatcaccctgaagtccaagctggtgtccgatttccggaaggatttccagttttacaaagtgcgcgagatcaacaactaccaccacgcccacgacgcctacctgaacgccgtcgtgggaaccgccctgatcaaaaagtaccctaagctggaaagcgagttcgtgtacggcgactacaaggtgtacgacgtgcggaagatgatcgccaagagcgagcaggaaatcggcaaggctaccgccaagtacttcttctacagcaacatcatgaactttttcaagaccgagattaccctggccaacggcgagatccggaagcggcctctgatcgagacaaacggcgaaacaggcgagatcgtgtgggataagggccgggactttgccaccgtgcggaaagtgctgtctatgccccaagtgaatatcgtgaaaaagaccgaggtgcagacaggcggcttcagcaaagagtctatcctgcccaagaggaacagcgacaagctgatcgccagaaagaaggactgggaccctaagaagtacggcggcttcgacagccccaccgtggcctattctgtgctggtggtggccaaagtggaaaagggcaagtccaagaaactgaagagtgtgaaagagctgctggggatcaccatcatggaaagaagcagcttcgagaagaatcccatcgactttctggaagccaagggctacaaagaagtgaaaaaggacctgatcatcaagctgcctaagtactccctgttcgagctggaaaacggccggaagagaatgctggcctctgccggcgaactgcagaagggaaacgaactggccctgccctccaaatatgtgaacttcctgtacctggccagccactatgagaagctgaagggctcccccgaggataatgagcagaaacagctgtttgtggaacagcacaaacactacctggacgagatcatcgagcagatcagcgagttctccaagagagtgatcctggccgacgctaatctggacaaggtgctgagcgcctacaacaagcacagagacaagcctatcagagagcaggccgagaatatcatccacctgtttaccctgaccaatctgggagcccctgccgccttcaagtactttgacaccaccatcgaccggaagaggtacaccagcaccaaagaggtgctggacgccaccctgatccaccagagcatcaccggcctgtacgagacacggatcgacctgtctcagctgggaggcgacgcctatccctatgacgtgcccgattatgccagcctgggcagcggctcccccaagaaaaaacgcaaggtggaagatcctaagaaaaagcggaaagtggacggcagcggcagcgagacccccggtaccagcgagagcgccacccccgagagcatgaacaattcccagggaagagtgaccttcgaggatgtcactgtgaacttcacccagggggagtggcagcggctgaatcccgaacagagaaacttgtacagggatgtgatgctggagaattacagcaaccttgtctctgtgggacaaggggaaaccaccaaacccgatgtgatcttgaggttggaacaaggaaaggagccatggttggaggaagaggaagtgctgggaagtggccgtgcagaaaaaaatggggacattggagggcagatttggaagccaaaggatgtgaaagagagtctcctcgagggaagcggagctactaacttcagcctgctgaagcaggctggagacgtggaggagaaccctggacctatgcctgctgctaagagagtgaaactggatggatccaaccatgaccaggaatttgaccccccaaaggtttacccacctgtgccagctgagaagaggaagcccatccgcgtgctgtctctctttgatgggattgctacagggctcctggtgctgaaggacctgggcatccaagtggaccgctacattgcctccgaggtgtgtgaggactccatcacggtgggcatggtgcggcaccagggaaagatcatgtacgtcggggacgtccgcagcgtcacacagaagcatatccaggagtggggcccattcgacctggtgattggaggcagtccctgcaatgacctctccattgtcaaccctgcccgcaagggactttatgagggtactggccgcctcttctttgagttctaccgcctcctgcatgatgcgcggcccaaggagggagatgatcgccccttcttctggctctttgagaatgtggtggccatgggcgttagtgacaagagggacatctcgcgatttcttgagtctaaccccgtgatgattgacgccaaagaagtgtctgctgcacacagggcccgttacttctggggtaaccttcctggcatgaacaggcctttggcatccactgtgaatgataagctggagctgcaagagtgtctggagcacggcagaatagccaagttcagcaaagtgaggaccattaccaccaggtcaaactctataaagcagggcaaagaccagcatttccccgtgttcatgaacgagaaggaggacatcctgtggtgcactgaaatggaaagggtgtttggcttccccgtccactacacagacgtctccaacatgagccgcttggcgaggcagagactgctgggccgatcgtggagcgtgccggtcatccgccacctcttcgctccgctgaaggaatattttgcttgtgtgtctagcggcaatagtaacgctaacagccgcgggccgagcttcagcagcggcctggtgccgttaagcttgcgcggcagccatatgttcgaaaccgtgcctgtgtggaggagacagccagtccgggtgctgtccctttttgaagacatcaagaaagagctgacgagtttgggctttttggaaagtggttctgacccgggacaactgaagcatgtggttgatgtcacagacacagtgaggaaggatgtggaggagtggggacccttcgatcttgtgtacggcgccacacctcccctgggccacacctgtgaccgtcctcccagctggtacctgttccagttccaccggctcctgcagtacgcacggcccaagccaggcagccccaggcccttcttctggatgttcgtggacaatctggtgctgaacaaggaagacctggacgtcgcatctcgcttcctggagatggagccagtcaccatcccagatgtccacggcggatccttgcagaatgctgtccgcgtgtggagcaacatcccagccataaggagcagcaggcactgggctctggtttcggaagaagaattgtccctgctggcccagaacaagcagagctcgaagctcgcggccaagtggcccaccaagctggtgaagaactgctttctccccctaagagaatatttcaagtatttttcaggagggccgagctctggcgcacccccaccaagtggagggtctcctgccgggtccccaacatctactgaagaaggcaccagcgaatccgcaacgcccgagtcaggccctggtacctccacagaaccatctgaaggtagtgcgcctggttccccagctggaagccctacttccaccgaagaaggcacgtcaaccgaaccaagtgaaggatctgcccctgggaccagcactgaaccatctgagccaaaaaagaagagaaaggtaccatctgagatgtccaagggagaggagctgttcaccggagtggtgccaatcctggtggagctggacggcgatgtgaacggccacaagttttctgtgcgcggagagggagagggcgacgcaaccatcggcaagctgacactgaagttcatctgcaccacaggcaagctgcccgtgccttggccaaccctggtgaccacactgacatacggcgtgcagtgtttctctaggtatccagaccacatgaagagacacgatttctttaagagcgccatgccagagggatacgtgcaggagcggaccatctccttcaaggacgatggcaagtataagacccgcgccgtggtgaagtttgagggcgatacactggtgaacaggatcgagctgaagggcaccgacttcaaggaggatggcaatatcctgggccacaagctggagtacaactttaatagccacaacgtgtatatcacagccgacaagcagaagaacggcatcaaggccaacttcaccgtgaggcacaatgtggaggacggctccgtgcagctggccgatcactaccagcagaacacacctatcggcgacggacccgtgctgctgcctgataatcactatctgtccacccagacagtgctgtctaaggacccaaacgagaagtgataataggatcccaagcacgcagcaatgcagctcaaaacgcttagcctagccacacccccacgggaaacagcagtgattaacctttagcaataaacgaaagtttaactaagctatactaaccccagggttggtcaatttcgtgccagccacaccctggtactgcatgcacgcaatgctagctgcccctttcccgtcctgggcaccccgagtctcccccgaccccgggtcccaggtatgctcccacctccacctgccccactcaccacctctgctagttccagacacctccgagacgaggaaaaaaaaaaaaaaaaaaaaaaaaaaaaaaaaaaaaaaaaaaaaaaaaaaaaaaaaaaaaaaaaaaaaaaaaaaaaaaaaaaaaaaaaaaaaaaaaaaaaaaaaaaaaaaaaaaaaaaaa

SEQ ID NO: 286 - RNA, 7678 nt, synthetic construct
  misc_feature 1..7678: note = mRNA of V45_D3a-D3l-1xGFP11-2a-GFP1-10-dCas9-KRAB
  source 1..7678: mol_type = other RNA
aggactcactatttgttttcgcgcccagttgcaaaaagtgtcgacatttgcttctgacacaactgtgttcactagcaacctcaaacagacaccgccaccatgcctgctgctaagagagtgaaactggatggatccaaccatgaccaggaatttgaccccccaaaggtttacccacctgtgccagctgagaagaggaagcccatccgcgtgctgtctctctttgatgggattgctacagggctcctggtgctgaaggacctgggcatccaagtggaccgctacattgcctccgaggtgtgtgaggactccatcacggtgggcatggtgcggcaccagggaaagatcatgtacgtcggggacgtccgcagcgtcacacagaagcatatccaggagtggggcccattcgacctggtgattggaggcagtccctgcaatgacctctccattgtcaaccctgcccgcaagggactttatgagggtactggccgcctcttctttgagttctaccgcctcctgcatgatgcgcggcccaaggagggagatgatcgccccttcttctggctctttgagaatgtggtggccatgggcgttagtgacaagagggacatctcgcgatttcttgagtctaaccccgtgatgattgacgccaaagaagtgtctgctgcacacagggcccgttacttctggggtaaccttcctggcatgaacaggcctttggcatccactgtgaatgataagctggagctgcaagagtgtctggagcacggcagaatagccaagttcagcaaagtgaggaccattaccaccaggtcaaactctataaagcagggcaaagaccagcatttccccgtgttcatgaacgagaaggaggacatcctgtggtgcactgaaatggaaagggtgtttggcttccccgtccactacacagacgtctccaacatgagccgcttggcgaggcagagactgctgggccgatcgtggagcgtgccggtcatccgccacctcttcgctccgctgaaggaatattttgcttgtgtgtctagcggcaatagtaacgctaacagccgcgggccgagcttcagcagcggcctggtgccgttaagcttgcgcggcagccatatgggccctatggagatatacaagacagtgtctgcatggaagagacagccagtgcgggtactgagcctcttcagaaacatcgacaaggtactaaagagtttgggcttcttggaaagcggttctggttctgggggaggaacgctgaagtacgtggaagatgtcacaaatgtcgtgaggagagacgtggagaaatggggcccctttgacctggtgtacggctcgacgcagcccctaggcagctcttgtgatcgctgtcccggctggtacatgttccagttccaccggatcctgcagtatgcgctgcctcgccaggagagtcagcggcccttcttctggatattcatggacaatctgctgctgactgaggatgaccaagagacaactacccgcttccttcagacagaggctgtgaccctccaggatgtccgtggcagagactaccagaatgctatgcgggtgtggagcaacattccagggctgaagagcaagcatgcgcccctgaccccaaaggaagaagagtatctgcaagcccaagtcagaagcaggagcaagctggacgccccgaaagttgacctcctggtgaagaactgccttctcccgctgagagagtacttcaagtatttttctcaaaactcacttcctcttggagggccgagctctggcgcacccccaccaagtggagggtctcctgccgggtccccaacatctactgaagaaggcaccagcgaatccgcaacgggcggtagcggcggtcgggaccatatggtcctgcacgaatatgtcaatgctgccggtatcaccgcggccgcaaggtcaggctccggccagcggggaagcaagcgcaccgccgatggttccgagttcgaaagccccaaaaaaaagcgcaaggtcggaagcggagctactaacttcagcctgctgaagcaggctggagacgtggaggagaaccctggacctatgcctgctgctaagagagtgaaactggatggatccggccccgacatcgtgatgtccaagggagaggagctgttcaccggagtggtgccaatcctggtggagctggacggcgatgtgaacggccacaagttttctgtgcgcggagagggagagggcgacgcaaccatcggcaagctgacactgaagttcatctgcaccacaggcaagctgcccgtgccttggccaaccctggtgaccacactgacatacggcgtgcagtgtttctctaggtatccagaccacatgaagagacacgatttctttaagagcgccatgccagagggatacgtgcaggagcggaccatctccttcaaggacgatggcaagtataagacccgcgccgtggtgaagtttgagggcgatacactggtgaacaggatcgagctgaagggcaccgacttcaaggaggatggcaatatcctgggccacaagctggagtacaactttaatagccacaacgtgtatatcacagccgacaagcagaagaacggcatcaaggccaacttcaccgtgaggcacaatgtggaggacggctccgtgcagctggccgatcactaccagcagaacacacctatcggcgacggacccgtgctgctgcctgataatcactatctgtccacccagacagtgctgtctaaggacccaaacgagaagttggatccaggtggaggcggaagcggaagcggaccaaaaaagaagagaaaggtaatggacaagaagtacagcatcggcctggccatcggcaccaactctgtgggctgggccgtgatcaccgacgagtacaaggtgcccagcaagaaattcaaggtgctgggcaacaccgaccggcacagcatcaagaagaacctgatcggcgccctgctgttcgacagcggagaaacagccgaggccacccggctgaagagaaccgccagaagaagatacaccagacggaagaaccggatctgctatctgcaagagatcttcagcaacgagatggccaaggtggacgacagcttcttccacagactggaagagtccttcctggtggaagaggataagaagcacgagcggcaccccatcttcggcaacatcgtggacgaggtggcctaccacgagaagtaccccaccatctaccacctgagaaagaaactggtggacagcaccgacaaggccgacctgcggctgatctatctggccctggcccacatgatcaagttccggggccacttcctgatcgagggcgacctgaaccccgacaacagcgacgtggacaagctgttcatccagctggtgcagacctacaaccagctgttcgaggaaaaccccatcaacgccagcggcgtggacgccaaggccatcctgtctgccagactgagcaagagcagacggctggaaaatctgatcgcccagctgcccggcgagaagaagaatggcctgttcggcaacctgattgccctgagcctgggcctgacccccaacttcaagagcaacttcgacctggccgaggatgccaaactgcagctgagcaaggacacctacgacgacgacctggacaacctgctggcccagatcggcgaccagtacgccgacctgtttctggccgccaagaacctgtccgacgccatcctgctgagcgacatcctgagagtgaacaccgagatcaccaaggcccccctgagcgcctctatgatcaagagatacgacgagcaccaccaggacctgaccctgctgaaagctctcgtgcggcagcagctgcctgagaagtacaaagagattttcttcgaccagagcaagaacggctacgccggctacatcgatggcggagccagccaggaagagttctacaagttcatcaagcccatcctggaaaagatggacggcaccgaggaactgctcgtgaagctgaacagagaggacctgctgcggaagcagcggaccttcgacaacggcagcatcccccaccagatccacctgggagagctgcacgccattctgcggcggcaggaagatttttacccattcctgaaggacaaccgggaaaagatcgagaagatcctgaccttccgcatcccctactacgtgggccctctggccaggggaaacagcagattcgcctggatgaccagaaagagcgaggaaaccatcaccccctggaacttcgaggaagtggtggacaagggcgccagcgcccagagcttcatcgagcggatgaccaacttcgataagaacctgcccaacgagaaggtgctgcccaagcacagcctgctgtacgagtacttcaccgtgtacaacgagctgaccaaagtgaaatacgtgaccgagggaatgagaaagcccgccttcctgagcggcgagcagaaaaaagccatcgtggacctgctgttcaagaccaaccggaaagtgaccgtgaagcagctgaaagaggactacttcaagaaaatcgagtgcttcgactccgtggaaatctccggcgtggaagatcggttcaacgcctccctgggcacataccacgatctgctgaaaattatcaaggacaaggacttcctggacaatgaggaaaacgaggacattctggaagatatcgtgctgaccctgacactgtttgaggacagagagatgatcgaggaacggctgaaaacctatgcccacctgttcgacgacaaagtgatgaagcagctgaagcggcggagatacaccggctggggcaggctgagccggaagctgatcaacggcatccgggacaagcagtccggcaagacaatcctggatttcctgaagtccgacggcttcgccaacagaaacttcatgcagctgatccacgacgacagcctgacctttaaagaggacatccagaaagcccaggtgtccggccagggcgatagcctgcacgagcacattgccaatctggccggcagccccgccattaagaagggcatcctgcagacagtgaaggtggtggacgagctcgtgaaagtgatgggccggcacaagcccgagaacatcgtgatcgaaatggccagagagaaccagaccacccagaagggacagaagaacagccgcgagagaatgaagcggatcgaagagggcatcaaagagctgggcagccagatcctgaaagaacaccccgtggaaaacacccagctgcagaacgagaagctgtacctgtactacctgcagaatgggcgggatatgtacgtggaccaggaactggacatcaaccggctgtccgactacgatgtggacgctatcgtgcctcagagctttctgaaggacgactccatcgataacaaagtgctgactcggagcgacaagaaccggggcaagagcgacaacgtgccctccgaagaggtcgtgaagaagatgaagaactactggcgccagctgctgaatgccaagctgattacccagaggaagttcgacaatctgaccaaggccgagagaggcggcctgagcgaactggataaggccggcttcatcaagagacagctggtggaaacccggcagatcacaaagcacgtggcacagatcctggactcccggatgaacactaagtacgacgagaacgacaaactgatccgggaagtgaaagtgatcaccctgaagtccaagctggtgtccgatttccggaaggatttccagttttacaaagtgcgcgagatcaacaactaccaccacgcccacgacgcctacctgaacgccgtcgtgggaaccgccctgatcaaaaagtaccctaagctggaaagcgagttcgtgtacggcgactacaaggtgtacgacgtgcggaagatgatcgccaagagcgagcaggaaatcggcaaggctaccgccaagtacttcttctacagcaacatcatgaactttttcaagaccgagattaccctggccaacggcgagatccggaagcggcctctgatcgagacaaacggcgaaacaggcgagatcgtgtgggataagggccgggactttgccaccgtgcggaaagtgctgtctatgccccaagtgaatatcgtgaaaaagaccgaggtgcagacaggcggcttcagcaaagagtctatcctgcccaagaggaacagcgacaagctgatcgccagaaagaaggactgggaccctaagaagtacggcggcttcgacagccccaccgtggcctattctgtgctggtggtggccaaagtggaaaagggcaagtccaagaaactgaagagtgtgaaagagctgctggggatcaccatcatggaaagaagcagcttcgagaagaatcccatcgactttctggaagccaagggctacaaagaagtgaaaaaggacctgatcatcaagctgcctaagtactccctgttcgagctggaaaacggccggaagagaatgctggcctctgccggcgaactgcagaagggaaacgaactggccctgccctccaaatatgtgaacttcctgtacctggccagccactatgagaagctgaagggctcccccgaggataatgagcagaaacagctgtttgtggaacagcacaaacactacctggacgagatcatcgagcagatcagcgagttctccaagagagtgatcctggccgacgctaatctggacaaggtgctgagcgcctacaacaagcacagagacaagcctatcagagagcaggccgagaatatcatccacctgtttaccctgaccaatctgggagcccctgccgccttcaagtactttgacaccaccatcgaccggaagaggtacaccagcaccaaagaggtgctggacgccaccctgatccaccagagcatcaccggcctgtacgagacacggatcgacctgtctcagctgggaggcgacgcctatccctatgacgtgcccgattatgccagcctgggcagcggctcccccaagaaaaaacgcaaggtggaagatcctaagaaaaagcggaaagtggacggcagcggcagcgagacccccggtaccagcgagagcgccacccccgagagccggacactggtgaccttcaaggatgtatttgtggacttcaccagggaggagtggaagctgctggacactgctcagcagatcgtgtacagaaatgtgatgctggagaactataagaacctggtttccttgggttatcagcttactaagccagatgtgatcctccggttggagaagggagaagagccctgagatcccaagcacgcagcaatgcagctcaaaacgcttagcctagccacacccccacgggaaacagcagtgattaacctttagcaataaacgaaagtttaactaagctatactaaccccagggttggtcaatttcgtgccagccacaccctggtactgcatgcacgcaatgctagctgcccctttcccgtcctgggcaccccgagtctcccccgaccccgggtcccaggtatgctcccacctccacctgccccactcaccacctctgctagttccagacacctccgagacgaggaaaaaaaaaaaaaaaaaaaaaaaaaaaaaaaaaaaaaaaaaaaaaaaaaaaaaaaaaaaaaaaaaaaaaaaaaaaaaaaaaaaaaaaaaaaaaaaaaaaaaaaaaaaaaaaaaaaaaaaa

SEQ ID NO: 287 - RNA, 8485 nt, synthetic construct
  misc_feature 1..8485: note = mRNA of V46_10xGFP11-dCas9-ZIM3-2a-D3a-hD3L-GFP1-10
  source 1..8485: mol_type = other RNA
aggactcactatttgttttcgcgcccagttgcaaaaagtgtcgacatttgcttctgacacaactgtgttcactagcaacctcaaacagacaccgccaccatgcctgctgctaagagagtgaaactggatggatccatgcgtgaccacatggtccttcatgagtatgtaaatgctgctgggattacaggtggctctggaggtagagatcatatggttctccacgaatacgttaacgccgcaggcatcactggcggtagtggaggacgcgaccatatggtactacatgaatatgtcaatgcagccggaataaccggagggtccggaggccgggatcacatggtgctgcatgagtatgtgaacgcggcgggtataactggtgggtcgggcggacgagaccatatggtgcttcacgaatacgtaaacgcagctggcattactggcggatcaggtggcagggatcacatggtactccatgagtacgtgaacgctgctggaatcacaggcggtagcggcggtcgggaccatatggtcctgcacgaatatgtcaatgctgccggtatcaccgcggccgcaggtggctctggaggtagagatcatatggttctccacgaatacgttaacgccgcaggcatcactggcggtagtggaggacgcgaccatatggtactacatgaatatgtcaatgcagccggaataaccggagggtccggaggccgggatcacatggtgctgcatgagtatgtgaacgcggcgggtataactggtgggtcgggcggaaggtcaggctccggccagcggggaagcaagcgcaccgccgatggttccgagttcgaaagccccaaaaaaaagcgcaaggtcggcggaagcggaagcggaccaaaaaagaagagaaaggtaatggacaagaagtacagcatcggcctggccatcggcaccaactctgtgggctgggccgtgatcaccgacgagtacaaggtgcccagcaagaaattcaaggtgctgggcaacaccgaccggcacagcatcaagaagaacctgatcggcgccctgctgttcgacagcggagaaacagccgaggccacccggctgaagagaaccgccagaagaagatacaccagacggaagaaccggatctgctatctgcaagagatcttcagcaacgagatggccaaggtggacgacagcttcttccacagactggaagagtccttcctggtggaagaggataagaagcacgagcggcaccccatcttcggcaacatcgtggacgaggtggcctaccacgagaagtaccccaccatctaccacctgagaaagaaactggtggacagcaccgacaaggccgacctgcggctgatctatctggccctggcccacatgatcaagttccggggccacttcctgatcgagggcgacctgaaccccgacaacagcgacgtggacaagctgttcatccagctggtgcagacctacaaccagctgttcgaggaaaaccccatcaacgccagcggcgtggacgccaaggccatcctgtctgccagactgagcaagagcagacggctggaaaatctgatcgcccagctgcccggcgagaagaagaatggcctgttcggcaacctgattgccctgagcctgggcctgacccccaacttcaagagcaacttcgacctggccgaggatgccaaactgcagctgagcaaggacacctacgacgacgacctggacaacctgctggcccagatcggcgaccagtacgccgacctgtttctggccgccaagaacctgtccgacgccatcctgctgagcgacatcctgagagtgaacaccgagatcaccaaggcccccctgagcgcctctatgatcaagagatacgacgagcaccaccaggacctgaccctgctgaaagctctcgtgcggcagcagctgcctgagaagtacaaagagattttcttcgaccagagcaagaacggctacgccggctacatcgatggcggagccagccaggaagagttctacaagttcatcaagcccatcctggaaaagatggacggcaccgaggaactgctcgtgaagctgaacagagaggacctgctgcggaagcagcggaccttcgacaacggcagcatcccccaccagatccacctgggagagctgcacgccattctgcggcggcaggaagatttttacccattcctgaaggacaaccgggaaaagatcgagaagatcctgaccttccgcatcccctactacgtgggccctctggccaggggaaacagcagattcgcctggatgaccagaaagagcgaggaaaccatcaccccctggaacttcgaggaagtggtggacaagggcgccagcgcccagagcttcatcgagcggatgaccaacttcgataagaacctgcccaacgagaaggtgctgcccaagcacagcctgctgtacgagtacttcaccgtgtacaacgagctgaccaaagtgaaatacgtgaccgagggaatgagaaagcccgccttcctgagcggcgagcagaaaaaagccatcgtggacctgctgttcaagaccaaccggaaagtgaccgtgaagcagctgaaagaggactacttcaagaaaatcgagtgcttcgactccgtggaaatctccggcgtggaagatcggttcaacgcctccctgggcacataccacgatctgctgaaaattatcaaggacaaggacttcctggacaatgaggaaaacgaggacattctggaagatatcgtgctgaccctgacactgtttgaggacagagagatgatcgaggaacggctgaaaacctatgcccacctgttcgacgacaaagtgatgaagcagctgaagcggcggagatacaccggctggggcaggctgagccggaagctgatcaacggcatccgggacaagcagtccggcaagacaatcctggatttcctgaagtccgacggcttcgccaacagaaacttcatgcagctgatccacgacgacagcctgacctttaaagaggacatccagaaagcccaggtgtccggccagggcgatagcctgcacgagcacattgccaatctggccggcagccccgccattaagaagggcatcctgcagacagtgaaggtggtggacgagctcgtgaaagtgatgggccggcacaagcccgagaacatcgtgatcgaaatggccagagagaaccagaccacccagaagggacagaagaacagccgcgagagaatgaagcggatcgaagagggcatcaaagagctgggcagccagatcctgaaagaacaccccgtggaaaacacccagctgcagaacgagaagctgtacctgtactacctgcagaatgggcgggatatgtacgtggaccaggaactggacatcaaccggctgtccgactacgatgtggacgctatcgtgcctcagagctttctgaaggacgactccatcgataacaaagtgctgactcggagcgacaagaaccggggcaagagcgacaacgtgccctccgaagaggtcgtgaagaagatgaagaactactggcgccagctgctgaatgccaagctgattacccagaggaagttcgacaatctgaccaaggccgagagaggcggcctgagcgaactggataaggccggcttcatcaagagacagctggtggaaacccggcagatcacaaagcacgtggcacagatcctggactcccggatgaacactaagtacgacgagaacgacaaactgatccgggaagtgaaagtgatcaccctgaagtccaagctggtgtccgatttccggaaggatttccagttttacaaagtgcgcgagatcaacaactaccaccacgcccacgacgcctacctgaacgccgtcgtgggaaccgccctgatcaaaaagtaccctaagctggaaagcgagttcgtgtacggcgactacaaggtgtacgacgtgcggaagatgatcgccaagagcgagcaggaaatcggcaaggctaccgccaagtacttcttctacagcaacatcatgaactttttcaagaccgagattaccctggccaacggcgagatccggaagcggcctctgatcgagacaaacggcgaaacaggcgagatcgtgtgggataagggccgggactttgccaccgtgcggaaagtgctgtctatgccccaagtgaatatcgtgaaaaagaccgaggtgcagacaggcggcttcagcaaagagtctatcctgcccaagaggaacagcgacaagctgatcgccagaaagaaggactgggaccctaagaagtacggcggcttcgacagccccaccgtggcctattctgtgctggtggtggccaaagtggaaaagggcaagtccaagaaactgaagagtgtgaaagagctgctggggatcaccatcatggaaagaagcagcttcgagaagaatcccatcgactttctggaagccaagggctacaaagaagtgaaaaaggacctgatcatcaagctgcctaagtactccctgttcgagctggaaaacggccggaagagaatgctggcctctgccggcgaactgcagaagggaaacgaactggccctgccctccaaatatgtgaacttcctgtacctggccagccactatgagaagctgaagggctcccccgaggataatgagcagaaacagctgtttgtggaacagcacaaacactacctggacgagatcatcgagcagatcagcgagttctccaagagagtgatcctggccgacgctaatctggacaaggtgctgagcgcctacaacaagcacagagacaagcctatcagagagcaggccgagaatatcatccacctgtttaccctgaccaatctgggagcccctgccgccttcaagtactttgacaccaccatcgaccggaagaggtacaccagcaccaaagaggtgctggacgccaccctgatccaccagagcatcaccggcctgtacgagacacggatcgacctgtctcagctgggaggcgacgcctatccctatgacgtgcccgattatgccagcctgggcagcggctcccccaagaaaaaacgcaaggtggaagatcctaagaaaaagcggaaagtggacggcagcggcagcgagacccccggtaccagcgagagcgccacccccgagagcatgaacaattcccagggaagagtgaccttcgaggatgtcactgtgaacttcacccagggggagtggcagcggctgaatcccgaacagagaaacttgtacagggatgtgatgctggagaattacagcaaccttgtctctgtgggacaaggggaaaccaccaaacccgatgtgatcttgaggttggaacaaggaaaggagccatggttggaggaagaggaagtgctgggaagtggccgtgcagaaaaaaatggggacattggagggcagatttggaagccaaaggatgtgaaagagagtctcctcgagggaagcggagctactaacttcagcctgctgaagcaggctggagacgtggaggagaaccctggacctatgcctgctgctaagagagtgaaactggatggatccaaccatgaccaggaatttgaccccccaaaggtttacccacctgtgccagctgagaagaggaagcccatccgcgtgctgtctctctttgatgggattgctacagggctcctggtgctgaaggacctgggcatccaagtggaccgctacattgcctccgaggtgtgtgaggactccatcacggtgggcatggtgcggcaccagggaaagatcatgtacgtcggggacgtccgcagcgtcacacagaagcatatccaggagtggggcccattcgacctggtgattggaggcagtccctgcaatgacctctccattgtcaaccctgcccgcaagggactttatgagggtactggccgcctcttctttgagttctaccgcctcctgcatgatgcgcggcccaaggagggagatgatcgccccttcttctggctctttgagaatgtggtggccatgggcgttagtgacaagagggacatctcgcgatttcttgagtctaaccccgtgatgattgacgccaaagaagtgtctgctgcacacagggcccgttacttctggggtaaccttcctggcatgaacaggcctttggcatccactgtgaatgataagctggagctgcaagagtgtctggagcacggcagaatagccaagttcagcaaagtgaggaccattaccaccaggtcaaactctataaagcagggcaaagaccagcatttccccgtgttcatgaacgagaaggaggacatcctgtggtgcactgaaatggaaagggtgtttggcttccccgtccactacacagacgtctccaacatgagccgcttggcgaggcagagactgctgggccgatcgtggagcgtgccggtcatccgccacctcttcgctccgctgaaggaatattttgcttgtgtgtctagcggcaatagtaacgctaacagccgcgggccgagcttcagcagcggcctggtgccgttaagcttgcgcggcagccatatgttcgaaaccgtgcctgtgtggaggagacagccagtccgggtgctgtccctttttgaagacatcaagaaagagctgacgagtttgggctttttggaaagtggttctgacccgggacaactgaagcatgtggttgatgtcacagacacagtgaggaaggatgtggaggagtggggacccttcgatcttgtgtacggcgccacacctcccctgggccacacctgtgaccgtcctcccagctggtacctgttccagttccaccggctcctgcagtacgcacggcccaagccaggcagccccaggcccttcttctggatgttcgtggacaatctggtgctgaacaaggaagacctggacgtcgcatctcgcttcctggagatggagccagtcaccatcccagatgtccacggcggatccttgcagaatgctgtccgcgtgtggagcaacatcccagccataaggagcagcaggcactgggctctggtttcggaagaagaattgtccctgctggcccagaacaagcagagctcgaagctcgcggccaagtggcccaccaagctggtgaagaactgctttctccccctaagagaatatttcaagtatttttcaggagggccgagctctggcgcacccccaccaagtggagggtctcctgccgggtccccaacatctactgaagaaggcaccagcgaatccgcaacgcccgagtcaggccctggtacctccacagaaccatctgaaggtagtgcgcctggttccccagctggaagccctacttccaccgaagaaggcacgtcaaccgaaccaagtgaaggatctgcccctgggaccagcactgaaccatctgagccaaaaaagaagagaaaggtaccatctgagatgtccaagggagaggagctgttcaccggagtggtgccaatcctggtggagctggacggcgatgtgaacggccacaagttttctgtgcgcggagagggagagggcgacgcaaccatcggcaagctgacactgaagttcatctgcaccacaggcaagctgcccgtgccttggccaaccctggtgaccacactgacatacggcgtgcagtgtttctctaggtatccagaccacatgaagagacacgatttctttaagagcgccatgccagagggatacgtgcaggagcggaccatctccttcaaggacgatggcaagtataagacccgcgccgtggtgaagtttgagggcgatacactggtgaacaggatcgagctgaagggcaccgacttcaaggaggatggcaatatcctgggccacaagctggagtacaactttaatagccacaacgtgtatatcacagccgacaagcagaagaacggcatcaaggccaacttcaccgtgaggcacaatgtggaggacggctccgtgcagctggccgatcactaccagcagaacacacctatcggcgacggacccgtgctgctgcctgataatcactatctgtccacccagacagtgctgtctaaggacccaaacgagaagtgataataggatcccaagcacgcagcaatgcagctcaaaacgcttagcctagccacacccccacgggaaacagcagtgattaacctttagcaataaacgaaagtttaactaagctatactaaccccagggttggtcaatttcgtgccagccacaccctggtactgcatgcacgcaatgctagctgcccctttcccgtcctgggcaccccgagtctcccccgaccccgggtcccaggtatgctcccacctccacctgccccactcaccacctctgctagttccagacacctccgagacgaggaaaaaaaaaaaaaaaaaaaaaaaaaaaaaaaaaaaaaaaaaaaaaaaaaaaaaaaaaaaaaaaaaaaaaaaaaaaaaaaaaaaaaaaaaaaaaaaaaaaaaaaaaaaaaaaaaaaaaaaa

SEQ ID NO: 288 - RNA, 8155 nt, synthetic construct
  misc_feature 1..8155: note = mRNA of V47_scFv-ZIM3-2a-D3a-hD3L-dCas9-1xGCN4
  source 1..8155: mol_type = other RNA
aggactcactatttgttttcgcgcccagttgcaaaaagtgtcgacatttgcttctgacacaactgtgttcactagcaacctcaaacagacaccgccaccatggtgcctgccgccaagagagtgaagctggacggaagcggccctgacatcgtgatgacacagagcccttctagcctgagcgccagcgtgggagacagagtgaccatcacctgtagaagcagcacaggcgccgtgaccaccagcaattatgccagctgggtgcaagagaagcccggcaagctgttcaagggactgatcggcggcaccaacaatagagcacctggcgtgccaagcagattcagcggctctctgatcggagacaaggccacactgaccataagcagcctgcagcctgaggacttcgccacctacttttgcgccctgtggtacagcaaccactgggtgttcggccagggcaccaaggtggaactgaaaagaggcggcggaggatctggcggaggtggaagcggaggcggaggttctagtggtggtggcagcgaagtgaaactgctggaaagtggtggcggcctggttcagcctggcggatctctgaaactgagctgtgccgtgtccggcttcagcctgacagattacggcgtgaactgggtccgacaggcccctggaagaggactggaatggatcggagtgatctggggcgacggcatcaccgactacaatagcgccctgaaggaccggttcatcatcagcaaggacaacggcaagaacaccgtgtacctgcagatgagcaaagtgcggagcgacgacacagccctgtactactgtgtgaccggcctgttcgattactggggccagggaacactggtcaccgtgtctagctacccctacgacgtgccagattatgctggtggcggtggtggtagtggtggcggaggaagcggcggaggcggttctggtggcggcggttctcttgatcctggcggtggcggcagcggcatgaacaattctcagggcagagtgacattcgaggacgtgaccgtgaacttcacccaaggcgagtggcagagactgaaccccgagcagagaaacctgtaccgggacgtgatgctggaaaactactccaacctggtgtccgttggccagggcgaaaccaccaagcctgacgtgatcctgagactggaacagggcaaagagccctggctcgaagaggaagaggtgctcggatctggcagagccgagaagaatggcgatattggcggacagatctggaagcccaaggacgtgaaagagagccttggcagcggcgccaccaatttcagcctgctgaaacaggctggcgacgtggaagagaaccccggacctatgcctgccgccaagagagtgaagctggacggcagcaaccacgaccaagagttcgaccctcctaaggtgtaccctcctgtgccagccgagaagcggaagcctatcagagtgctgagcctgttcgacggaatcgccacaggactgctggtgctgaaggatctgggaatccaggtggaccggtatatcgccagcgaagtgtgcgaggacagcatcacagttggcatggttcgacaccagggcaagattatgtacgtgggcgacgtgcggagcgtgacccagaaacacattcaagagtggggccccttcgacctggttatcggcggcagcccttgcaacgatctgagcatcgtgaaccccgccagaaagggcctgtatgaaggcaccggcagactgttcttcgagttctacagactgctgcacgacgccagacctaaagagggcgacgacagaccattcttctggctgttcgagaacgtggtggctatgggcgtgtccgacaagcgggacatcagccggtttctggaaagcaaccccgtgatgatcgacgccaaagaggtgtccgctgctcaccgggccagatacttttggggcaatctgcccggcatgaacagacctctggccagcaccgtgaacgacaagctggaactgcaagagtgcctggaacacggccggatcgccaagtttagcaaagtgcggaccatcaccaccaggtccaacagcatcaagcagggcaaagaccagcacttccccgtgttcatgaatgagaaagaggacatcctgtggtgcaccgagatggaaagagtgttcggcttccctgtgcactacaccgacgtgtccaacatgagcagactggccagacagaggctgctgggcagatcttggagcgtgccagtgatcagacacctgttcgcccctctgaaagaatacttcgcctgcgtgtccagcggcaacagcaacgccaatagcagaggccctagcttcagctctggactggtgcctttgagcctgagaggcagccacatgttcgagacagtgcctgtgtggcggagacagcccgttagagtgctgtccctgtttgaggacatcaagaaagagctgaccagcctgggcttcctggaaagcggatctgatcctggccagctgaagcacgtggtggacgtgaccgataccgtgcggaaggatgtggaagaatggggcccttttgatctggtgtacggcgccacacctcctctgggccacacatgtgatagacctccaagctggtatctgttccagttccaccggctgctgcagtacgctagacccaagcctggaagccccaggcctttcttttggatgttcgtggacaacctggtcctgaacaaagaggacctggacgtcgccagccggttcctcgaaatggaacctgtgacaatccccgacgtgcacggcggatctctgcagaatgctgtcagagtgtggtctaacatccccgccatcagaagcagcagacactgggcccttgtgtccgaggaagaactgtctctgctggcccagaacaagcagagcagcaagctggccgccaagtggcctacaaagctggtcaagaactgcttcctgcctctgcgcgagtacttcaagtatttcagcggcggacctagctctggcgcccctccacctagcggaggatctccagcaggatctcctaccagcaccgaggaaggcacaagcgagtctgccacacctgagtctggccctggcacatctacagagcctagcgagggatctgcccctggatctcctgctggcagccctacatctaccgaagagggaaccagcacagagccttccgaaggttctgctcctggcacaagcaccgagccaagcgagcctaagaagaagagaaaagtcggcagcgacaagaagtacagcatcggcctggccatcggcaccaactctgtgggctgggccgtgatcaccgacgagtacaaggtgcccagcaagaaattcaaggtgctgggcaacaccgaccggcacagcatcaagaagaacctgatcggcgccctgctgttcgacagcggagaaacagccgaggccacccggctgaagagaaccgccagaagaagatacaccagacggaagaaccggatctgctatctgcaagagatcttcagcaacgagatggccaaggtggacgacagcttcttccacagactggaagagtccttcctggtggaagaggataagaagcacgagcggcaccccatcttcggcaacatcgtggacgaggtggcctaccacgagaagtaccccaccatctaccacctgagaaagaaactggtggacagcaccgacaaggccgacctgcggctgatctatctggccctggcccacatgatcaagttccggggccacttcctgatcgagggcgacctgaaccccgacaacagcgacgtggacaagctgttcatccagctggtgcagacctacaaccagctgttcgaggaaaaccccatcaacgccagcggcgtggacgccaaggccatcctgtctgccagactgagcaagagcagacggctggaaaatctgatcgcccagctgcccggcgagaagaagaatggcctgttcggcaacctgattgccctgagcctgggcctgacccccaacttcaagagcaacttcgacctggccgaggatgccaaactgcagctgagcaaggacacctacgacgacgacctggacaacctgctggcccagatcggcgaccagtacgccgacctgtttctggccgccaagaacctgtccgacgccatcctgctgagcgacatcctgagagtgaacaccgagatcaccaaggcccccctgagcgcctctatgatcaagagatacgacgagcaccaccaggacctgaccctgctgaaagctctcgtgcggcagcagctgcctgagaagtacaaagagattttcttcgaccagagcaagaacggctacgccggctacatcgatggcggagccagccaggaagagttctacaagttcatcaagcccatcctggaaaagatggacggcaccgaggaactgctcgtgaagctgaacagagaggacctgctgcggaagcagcggaccttcgacaacggcagcatcccccaccagatccacctgggagagctgcacgccattctgcggcggcaggaagatttttacccattcctgaaggacaaccgggaaaagatcgagaagatcctgaccttccgcatcccctactacgtgggccctctggccaggggaaacagcagattcgcctggatgaccagaaagagcgaggaaaccatcaccccctggaacttcgaggaagtggtggacaagggcgccagcgcccagagcttcatcgagcggatgaccaacttcgataagaacctgcccaacgagaaggtgctgcccaagcacagcctgctgtacgagtacttcaccgtgtacaacgagctgaccaaagtgaaatacgtgaccgagggaatgagaaagcccgccttcctgagcggcgagcagaaaaaagccatcgtggacctgctgttcaagaccaaccggaaagtgaccgtgaagcagctgaaagaggactacttcaagaaaatcgagtgcttcgactccgtggaaatctccggcgtggaagatcggttcaacgcctccctgggcacataccacgatctgctgaaaattatcaaggacaaggacttcctggacaatgaggaaaacgaggacattctggaagatatcgtgctgaccctgacactgtttgaggacagagagatgatcgaggaacggctgaaaacctatgcccacctgttcgacgacaaagtgatgaagcagctgaagcggcggagatacaccggctggggcaggctgagccggaagctgatcaacggcatccgggacaagcagtccggcaagacaatcctggatttcctgaagtccgacggcttcgccaacagaaacttcatgcagctgatccacgacgacagcctgacctttaaagaggacatccagaaagcccaggtgtccggccagggcgatagcctgcacgagcacattgccaatctggccggcagccccgccattaagaagggcatcctgcagacagtgaaggtggtggacgagctcgtgaaagtgatgggccggcacaagcccgagaacatcgtgatcgaaatggccagagagaaccagaccacccagaagggacagaagaacagccgcgagagaatgaagcggatcgaagagggcatcaaagagctgggcagccagatcctgaaagaacaccccgtggaaaacacccagctgcagaacgagaagctgtacctgtactacctgcagaatgggcgggatatgtacgtggaccaggaactggacatcaaccggctgtccgactacgatgtggacgctatcgtgcctcagagctttctgaaggacgactccatcgataacaaagtgctgactcggagcgacaagaaccggggcaagagcgacaacgtgccctccgaagaggtcgtgaagaagatgaagaactactggcgccagctgctgaatgccaagctgattacccagaggaagttcgacaatctgaccaaggccgagagaggcggcctgagcgaactggataaggccggcttcatcaagagacagctggtggaaacccggcagatcacaaagcacgtggcacagatcctggactcccggatgaacactaagtacgacgagaacgacaaactgatccgggaagtgaaagtgatcaccctgaagtccaagctggtgtccgatttccggaaggatttccagttttacaaagtgcgcgagatcaacaactaccaccacgcccacgacgcctacctgaacgccgtcgtgggaaccgccctgatcaaaaagtaccctaagctggaaagcgagttcgtgtacggcgactacaaggtgtacgacgtgcggaagatgatcgccaagagcgagcaggaaatcggcaaggctaccgccaagtacttcttctacagcaacatcatgaactttttcaagaccgagattaccctggccaacggcgagatccggaagcggcctctgatcgagacaaacggcgaaacaggcgagatcgtgtgggataagggccgggactttgccaccgtgcggaaagtgctgtctatgccccaagtgaatatcgtgaaaaagaccgaggtgcagacaggcggcttcagcaaagagtctatcctgcccaagaggaacagcgacaagctgatcgccagaaagaaggactgggaccctaagaagtacggcggcttcgacagccccaccgtggcctattctgtgctggtggtggccaaagtggaaaagggcaagtccaagaaactgaagagtgtgaaagagctgctggggatcaccatcatggaaagaagcagcttcgagaagaatcccatcgactttctggaagccaagggctacaaagaagtgaaaaaggacctgatcatcaagctgcctaagtactccctgttcgagctggaaaacggccggaagagaatgctggcctctgccggcgaactgcagaagggaaacgaactggccctgccctccaaatatgtgaacttcctgtacctggccagccactatgagaagctgaagggctcccccgaggataatgagcagaaacagctgtttgtggaacagcacaaacactacctggacgagatcatcgagcagatcagcgagttctccaagagagtgatcctggccgacgctaatctggacaaggtgctgagcgcctacaacaagcacagagacaagcctatcagagagcaggccgagaatatcatccacctgtttaccctgaccaatctgggagcccctgccgccttcaagtactttgacaccaccatcgaccggaagaggtacaccagcaccaaagaggtgctggacgccaccctgatccaccagagcatcaccggcctgtacgagacacggatcgacctgtctcagctgggaggcgacgcctatccctatgacgtgcccgattatgccagcctgggcagcggctcccccaagaaaaaacgcaaggtggaagatcctaagaaaaagcggaaagtggacggcatcggctccggctctaatggatctagcggagaggaactcctgtccaagaactaccaccttgagaacgaagtggcccgactcaagaaaggctctggtagcggaggctcaggttccggcggatcaggcagtggttctggcggttccggctcaggcggtagtggcagtggcgaagaacttctgagcaaaaactaccacggctctggctccggacagcggggctctaaaagaacagccgacggcagcgagtttgagagccctaaaaagaaaagaaaagtgtgataatagggatcccaagcacgcagcaatgcagctcaaaacgcttagcctagccacacccccacgggaaacagcagtgattaacctttagcaataaacgaaagtttaactaagctatactaaccccagggttggtcaatttcgtgccagccacaccctggtactgcatgcacgcaatgctagctgcccctttcccgtcctgggcaccccgagtctcccccgaccccgggtcccaggtatgctcccacctccacctgccccactcaccacctctgctagttccagacacctccgaagatggaaaaaaaaaaaaaaaaaaaaaaaaaaaaaaaaaaaaaaaaaaaaaaaaaaaaaaaaaaaaaaaaaaaaaaaaaaaaaaaaaaaaaaaaaaaaaaaaaaaaaaaaaaaaaaaaaaaaaaaa

SEQ ID NO: 289 - DNA, 5175 bp, synthetic construct
  misc_feature 1..5175: note = CDS of V1_3xGCN4-dCas9-3xGCN4
  source 1..5175: mol_type = other DNA
atgcctgctgctaagagagtgaaactggatggatccgaggaactgctgagcaagaactaccacctggaaaacgaggtggccagactgaagaaaggctctggctctggcggaagcggttctggcggatcaggatctggaagtggcggctctggaagcggaggttctggatctggcgaagaactgctgtctaagaattatcacctcgagaacgaagtggctcggctcaagaaaggcagtggcagcggaggaagtggatccggcggtagtggtagtggaagcggcggatccggctcaggcggatctggttcaggggaagaactcctctccaaaaactaccatctcgagaatgaggtcgcccgcctgaaaaaaggatcaggttccggtggttctggcagcggtggttcaggctcaggcagcggcggtagcggtagcggtggaagcggaagcggaccaaaaaagaagagaaaggtaatggacaagaagtacagcatcggcctggccatcggcaccaactctgtgggctgggccgtgatcaccgacgagtacaaggtgcccagcaagaaattcaaggtgctgggcaacaccgaccggcacagcatcaagaagaacctgatcggcgccctgctgttcgacagcggagaaacagccgaggccacccggctgaagagaaccgccagaagaagatacaccagacggaagaaccggatctgctatctgcaagagatcttcagcaacgagatggccaaggtggacgacagcttcttccacagactggaagagtccttcctggtggaagaggataagaagcacgagcggcaccccatcttcggcaacatcgtggacgaggtggcctaccacgagaagtaccccaccatctaccacctgagaaagaaactggtggacagcaccgacaaggccgacctgcggctgatctatctggccctggcccacatgatcaagttccggggccacttcctgatcgagggcgacctgaaccccgacaacagcgacgtggacaagctgttcatccagctggtgcagacctacaaccagctgttcgaggaaaaccccatcaacgccagcggcgtggacgccaaggccatcctgtctgccagactgagcaagagcagacggctggaaaatctgatcgcccagctgcccggcgagaagaagaatggcctgttcggcaacctgattgccctgagcctgggcctgacccccaacttcaagagcaacttcgacctggccgaggatgccaaactgcagctgagcaaggacacctacgacgacgacctggacaacctgctggcccagatcggcgaccagtacgccgacctgtttctggccgccaagaacctgtccgacgccatcctgctgagcgacatcctgagagtgaacaccgagatcaccaaggcccccctgagcgcctctatgatcaagagatacgacgagcaccaccaggacctgaccctgctgaaagctctcgtgcggcagcagctgcctgagaagtacaaagagattttcttcgaccagagcaagaacggctacgccggctacatcgatggcggagccagccaggaagagttctacaagttcatcaagcccatcctggaaaagatggacggcaccgaggaactgctcgtgaagctgaacagagaggacctgctgcggaagcagcggaccttcgacaacggcagcatcccccaccagatccacctgggagagctgcacgccattctgcggcggcaggaagatttttacccattcctgaaggacaaccgggaaaagatcgagaagatcctgaccttccgcatcccctactacgtgggccctctggccaggggaaacagcagattcgcctggatgaccagaaagagcgaggaaaccatcaccccctggaacttcgaggaagtggtggacaagggcgccagcgcccagagcttcatcgagcggatgaccaacttcgataagaacctgcccaacgagaaggtgctgcccaagcacagcctgctgtacgagtacttcaccgtgtacaacgagctgaccaaagtgaaatacgtgaccgagggaatgagaaagcccgccttcctgagcggcgagcagaaaaaagccatcgtggacctgctgttcaagaccaaccggaaagtgaccgtgaagcagctgaaagaggactacttcaagaaaatcgagtgcttcgactccgtggaaatctccggcgtggaagatcggttcaacgcctccctgggcacataccacgatctgctgaaaattatcaaggacaaggacttcctggacaatgaggaaaacgaggacattctggaagatatcgtgctgaccctgacactgtttgaggacagagagatgatcgaggaacggctgaaaacctatgcccacctgttcgacgacaaagtgatgaagcagctgaagcggcggagatacaccggctggggcaggctgagccggaagctgatcaacggcatccgggacaagcagtccggcaagacaatcctggatttcctgaagtccgacggcttcgccaacagaaacttcatgcagctgatccacgacgacagcctgacctttaaagaggacatccagaaagcccaggtgtccggccagggcgatagcctgcacgagcacattgccaatctggccggcagccccgccattaagaagggcatcctgcagacagtgaaggtggtggacgagctcgtgaaagtgatgggccggcacaagcccgagaacatcgtgatcgaaatggccagagagaaccagaccacccagaagggacagaagaacagccgcgagagaatgaagcggatcgaagagggcatcaaagagctgggcagccagatcctgaaagaacaccccgtggaaaacacccagctgcagaacgagaagctgtacctgtactacctgcagaatgggcgggatatgtacgtggaccaggaactggacatcaaccggctgtccgactacgatgtggacgctatcgtgcctcagagctttctgaaggacgactccatcgataacaaagtgctgactcggagcgacaagaaccggggcaagagcgacaacgtgccctccgaagaggtcgtgaagaagatgaagaactactggcgccagctgctgaatgccaagctgattacccagaggaagttcgacaatctgaccaaggccgagagaggcggcctgagcgaactggataaggccggcttcatcaagagacagctggtggaaacccggcagatcacaaagcacgtggcacagatcctggactcccggatgaacactaagtacgacgagaacgacaaactgatccgggaagtgaaagtgatcaccctgaagtccaagctggtgtccgatttccggaaggatttccagttttacaaagtgcgcgagatcaacaactaccaccacgcccacgacgcctacctgaacgccgtcgtgggaaccgccctgatcaaaaagtaccctaagctggaaagcgagttcgtgtacggcgactacaaggtgtacgacgtgcggaagatgatcgccaagagcgagcaggaaatcggcaaggctaccgccaagtacttcttctacagcaacatcatgaactttttcaagaccgagattaccctggccaacggcgagatccggaagcggcctctgatcgagacaaacggcgaaacaggcgagatcgtgtgggataagggccgggactttgccaccgtgcggaaagtgctgtctatgccccaagtgaatatcgtgaaaaagaccgaggtgcagacaggcggcttcagcaaagagtctatcctgcccaagaggaacagcgacaagctgatcgccagaaagaaggactgggaccctaagaagtacggcggcttcgacagccccaccgtggcctattctgtgctggtggtggccaaagtggaaaagggcaagtccaagaaactgaagagtgtgaaagagctgctggggatcaccatcatggaaagaagcagcttcgagaagaatcccatcgactttctggaagccaagggctacaaagaagtgaaaaaggacctgatcatcaagctgcctaagtactccctgttcgagctggaaaacggccggaagagaatgctggcctctgccggcgaactgcagaagggaaacgaactggccctgccctccaaatatgtgaacttcctgtacctggccagccactatgagaagctgaagggctcccccgaggataatgagcagaaacagctgtttgtggaacagcacaaacactacctggacgagatcatcgagcagatcagcgagttctccaagagagtgatcctggccgacgctaatctggacaaggtgctgagcgcctacaacaagcacagagacaagcctatcagagagcaggccgagaatatcatccacctgtttaccctgaccaatctgggagcccctgccgccttcaagtactttgacaccaccatcgaccggaagaggtacaccagcaccaaagaggtgctggacgccaccctgatccaccagagcatcaccggcctgtacgagacacggatcgacctgtctcagctgggaggcgacgcctatccctatgacgtgcccgattatgccagcctgggcagcggctcccccaagaaaaaacgcaaggtggaagatcctaagaaaaagcggaaagtggacggcagcggcagcgagacccccggtaccagtggcggatctggctccggtagcggaggatcaggatccggcggaagcggatcaggcgaggaactgctttccaaaaattaccaccttgaaaacgaagtcgcccgcctcaagaaaggttctggcagcggaggctctggcagtggtggtagcggaagtggaagtggtggcagtggtagcggtggatctggaagcggcgaggaactcctgtcaaagaattaccatctcgaaaacgaggtcgcaaggctcaagaaaggctcaggatcaggcggctctggatccggcggttctggttccggctcaggtggaagtggatctggcggctcaggttccggcgaagaattgctttccaagaactaccatttggaaaatgaagtcgctcgtttgaagaaaggttcaggctccggccagcggggaagcaagcgcaccgccgatggttccgagttcgaaagccccaaaaaaaagcgcaaggtctga

SEQ ID NO: 290 - DNA, 1080 bp, synthetic construct
  misc_feature 1..1080: note = CDS of V2_scFv-KRAB
  source 1..1080: mol_type = other DNA
atgcctgctgctaagagagtgaaactggatggatccggccccgacatcgtgatgacccagagccccagcagcctgagcgccagcgtgggcgaccgcgtgaccatcacctgccgcagcagcaccggcgccgtgaccaccagcaactacgccagctgggtgcaggagaagcccggcaagctgttcaagggcctgatcggcggcaccaacaaccgcgcccccggcgtgcccagccgcttcagcggcagcctgatcggcgacaaggccaccctgaccatcagcagcctgcagcccgaggacttcgccacctacttctgcgccctgtggtacagcaaccactgggtgttcggccagggcaccaaggtggagctgaagcgcggcggcggcggcagcggcggcggcggcagcggcggcggcggcagcagcggcggcggcagcgaggtgaagctgctggagagcggcggcggcctggtgcagcccggcggcagcctgaagctgagctgcgccgtgagcggcttcagcctgaccgactacggcgtgaactgggtgcgccaggcccccggccgcggcctggagtggatcggcgtgatctggggcgacggcatcaccgactacaacagcgccctgaaggaccgcttcatcatcagcaaggacaacggcaagaacaccgtgtacctgcagatgagcaaggtgcgcagcgacgacaccgccctgtactactgcgtgaccggcctgttcgactactggggccagggcaccctggtgaccgtgagcagctacccatacgatgttccagattacgctggtggaggcggaggttctgggggaggaggtagtggcggtggtggttcaggaggcggcggaagcttggatccaggtggaggtggaagcggtcggacactggtgaccttcaaggatgtatttgtggacttcaccagggaggagtggaagctgctggacactgctcagcagatcgtgtacagaaatgtgatgctggagaactataagaacctggtttccttgggttatcagcttactaagccagatgtgatcctccggttggagaagggagaagagccctag

SEQ ID NO: 291 - DNA, 6411 bp, synthetic construct
  misc_feature 1..6411: note = CDS of V3_D3a-D3l-dCas9-1xGCN4
  source 1..6411: mol_type = other DNA
atgcctgctgctaagagagtgaaactggatggatccaaccatgaccaggaatttgaccccccaaaggtttacccacctgtgccagctgagaagaggaagcccatccgcgtgctgtctctctttgatgggattgctacagggctcctggtgctgaaggacctgggcatccaagtggaccgctacattgcctccgaggtgtgtgaggactccatcacggtgggcatggtgcggcaccagggaaagatcatgtacgtcggggacgtccgcagcgtcacacagaagcatatccaggagtggggcccattcgacctggtgattggaggcagtccctgcaatgacctctccattgtcaaccctgcccgcaagggactttatgagggtactggccgcctcttctttgagttctaccgcctcctgcatgatgcgcggcccaaggagggagatgatcgccccttcttctggctctttgagaatgtggtggccatgggcgttagtgacaagagggacatctcgcgatttcttgagtctaaccccgtgatgattgacgccaaagaagtgtctgctgcacacagggcccgttacttctggggtaaccttcctggcatgaacaggcctttggcatccactgtgaatgataagctggagctgcaagagtgtctggagcacggcagaatagccaagttcagcaaagtgaggaccattaccaccaggtcaaactctataaagcagggcaaagaccagcatttccccgtcttcatgaacgagaaggaggacatcctgtggtgcactgaaatggaaagggtgtttggcttccccgtccactacacagacgtctccaacatgagccgcttggcgaggcagagactgctgggccgatcgtggagcgtgccggtcatccgccacctcttcgctccgctgaaggaatattttgcttgtgtgtctagcggcaatagtaacgctaacagccgcgggccgagcttcagcagcggcctggtgccgttaagcttgcgcggcagccatatgggccctatggagatatacaagacagtgtctgcatggaagagacagccagtgcgggtactgagcctcttcagaaacatcgacaaggtactaaagagtttgggcttcttggaaagcggttctggttctgggggaggaacgctgaagtacgtggaagatgtcacaaatgtcgtgaggagagacgtggagaaatggggcccctttgacctggtgtacggctcgacgcagcccctaggcagctcttgtgatcgctgtcccggctggtacatgttccagttccaccggatcctgcagtatgcgctgcctcgccaggagagtcagcggcccttcttctggatattcatggacaatctgctgctgactgaggatgaccaagagacaactacccgcttccttcagacagaggctgtgaccctccaggatgtccgtggcagagactaccagaatgctatgcgggtgtggagcaacattccagggctgaagagcaagcatgcgcccctgaccccaaaggaagaagagtatctgcaagcccaagtcagaagcaggagcaagctggacgccccgaaagttgacctcctggtgaagaactgccttctcccgctgagagagtacttcaagtatttttctcaaaactcacttcctcttggagggccgagctctggcgcacccccaccaagtggagggtctcctgccgggtccccaacatctactgaagaaggcaccagcgaatccgcaacgcccgagtcaggccctggtacctccacagaaccatctgaaggtagtgcgcctggttccccagctggaagccctacttccaccgaagaaggcacgtcaaccgaaccaagtgaaggatctgcccctgggaccagcactgaaccatctgagccaaaaaagaagagaaaggtaatggacaagaagtacagcatcggcctggccatcggcaccaactctgtgggctgggccgtgatcaccgacgagtacaaggtgcccagcaagaaattcaaggtgctgggcaacaccgaccggcacagcatcaagaagaacctgatcggcgccctgctgttcgacagcggagaaacagccgaggccacccggctgaagagaaccgccagaagaagatacaccagacggaagaaccggatctgctatctgcaagagatcttcagcaacgagatggccaaggtggacgacagcttcttccacagactggaagagtccttcctggtggaagaggataagaagcacgagcggcaccccatcttcggcaacatcgtggacgaggtggcctaccacgagaagtaccccaccatctaccacctgagaaagaaactggtggacagcaccgacaaggccgacctgcggctgatctatctggccctggcccacatgatcaagttccggggccacttcctgatcgagggcgacctgaaccccgacaacagcgacgtggacaagctgttcatccagctggtgcagacctacaaccagctgttcgaggaaaaccccatcaacgccagcggcgtggacgccaaggccatcctgtctgccagactgagcaagagcagacggctggaaaatctgatcgcccagctgcccggcgagaagaagaatggcctgttcggcaacctgattgccctgagcctgggcctgacccccaacttcaagagcaacttcgacctggccgaggatgccaaactgcagctgagcaaggacacctacgacgacgacctggacaacctgctggcccagatcggcgaccagtacgccgacctgtttctggccgccaagaacctgtccgacgccatcctgctgagcgacatcctgagagtgaacaccgagatcaccaaggcccccctgagcgcctctatgatcaagagatacgacgagcaccaccaggacctgaccctgctgaaagctctcgtgcggcagcagctgcctgagaagtacaaagagattttcttcgaccagagcaagaacggctacgccggctacatcgatggcggagccagccaggaagagttctacaagttcatcaagcccatcctggaaaagatggacggcaccgaggaactgctcgtgaagctgaacagagaggacctgctgcggaagcagcggaccttcgacaacggcagcatcccccaccagatccacctgggagagctgcacgccattctgcggcggcaggaagatttttacccattcctgaaggacaaccgggaaaagatcgagaagatcctgaccttccgcatcccctactacgtgggccctctggccaggggaaacagcagattcgcctggatgaccagaaagagcgaggaaaccatcaccccctggaacttcgaggaagtggtggacaagggcgccagcgcccagagcttcatcgagcggatgaccaacttcgataagaacctgcccaacgagaaggtgctgcccaagcacagcctgctgtacgagtacttcaccgtgtacaacgagctgaccaaagtgaaatacgtgaccgagggaatgagaaagcccgccttcctgagcggcgagcagaaaaaagccatcgtggacctgctgttcaagaccaaccggaaagtgaccgtgaagcagctgaaagaggactacttcaagaaaatcgagtgcttcgactccgtggaaatctccggcgtggaagatcggttcaacgcctccctgggcacataccacgatctgctgaaaattatcaaggacaaggacttcctggacaatgaggaaaacgaggacattctggaagatatcgtgctgaccctgacactgtttgaggacagagagatgatcgaggaacggctgaaaacctatgcccacctgttcgacgacaaagtgatgaagcagctgaagcggcggagatacaccggctggggcaggctgagccggaagctgatcaacggcatccgggacaagcagtccggcaagacaatcctggatttcctgaagtccgacggcttcgccaacagaaacttcatgcagctgatccacgacgacagcctgacctttaaagaggacatccagaaagcccaggtgtccggccagggcgatagcctgcacgagcacattgccaatctggccggcagccccgccattaagaagggcatcctgcagacagtgaaggtggtggacgagctcgtgaaagtgatgggccggcacaagcccgagaacatcgtgatcgaaatggccagagagaaccagaccacccagaagggacagaagaacagccgcgagagaatgaagcggatcgaagagggcatcaaagagctgggcagccagatcctgaaagaacaccccgtggaaaacacccagctgcagaacgagaagctgtacctgtactacctgcagaatgggcgggatatgtacgtggaccaggaactggacatcaaccggctgtccgactacgatgtggacgctatcgtgcctcagagctttctgaaggacgactccatcgataacaaagtgctgactcggagcgacaagaaccggggcaagagcgacaacgtgccctccgaagaggtcgtgaagaagatgaagaactactggcgccagctgctgaatgccaagctgattacccagaggaagttcgacaatctgaccaaggccgagagaggcggcctgagcgaactggataaggccggcttcatcaagagacagctggtggaaacccggcagatcacaaagcacgtggcacagatcctggactcccggatgaacactaagtacgacgagaacgacaaactgatccgggaagtgaaagtgatcaccctgaagtccaagctggtgtccgatttccggaaggatttccagttttacaaagtgcgcgagatcaacaactaccaccacgcccacgacgcctacctgaacgccgtcgtgggaaccgccctgatcaaaaagtaccctaagctggaaagcgagttcgtgtacggcgactacaaggtgtacgacgtgcggaagatgatcgccaagagcgagcaggaaatcggcaaggctaccgccaagtacttcttctacagcaacatcatgaactttttcaagaccgagattaccctggccaacggcgagatccggaagcggcctctgatcgagacaaacggcgaaacaggcgagatcgtgtgggataagggccgggactttgccaccgtgcggaaagtgctgtctatgccccaagtgaatatcgtgaaaaagaccgaggtgcagacaggcggcttcagcaaagagtctatcctgcccaagaggaacagcgacaagctgatcgccagaaagaaggactgggaccctaagaagtacggcggcttcgacagccccaccgtggcctattctgtgctggtggtggccaaagtggaaaagggcaagtccaagaaactgaagagtgtgaaagagctgctggggatcaccatcatggaaagaagcagcttcgagaagaatcccatcgactttctggaagccaagggctacaaagaagtgaaaaaggacctgatcatcaagctgcctaagtactccctgttcgagctggaaaacggccggaagagaatgctggcctctgccggcgaactgcagaagggaaacgaactggccctgccctccaaatatgtgaacttcctgtacctggccagccactatgagaagctgaagggctcccccgaggataatgagcagaaacagctgtttgtggaacagcacaaacactacctggacgagatcatcgagcagatcagcgagttctccaagagagtgatcctggccgacgctaatctggacaaggtgctgagcgcctacaacaagcacagagacaagcctatcagagagcaggccgagaatatcatccacctgtttaccctgaccaatctgggagcccctgccgccttcaagtactttgacaccaccatcgaccggaagaggtacaccagcaccaaagaggtgctggacgccaccctgatccaccagagcatcaccggcctgtacgagacacggatcgacctgtctcagctgggaggcgacgcctatccctatgacgtgcccgattatgccagcctgggcagcggctcccccaagaaaaaacgcaaggtggaagatcctaagaaaaagcggaaagtggacggcattggtagtgggagcaacggcagcagcggagaggaactgctgagcaagaactaccacctggaaaacgaggtggccagactgaagaaaggctctggctctggcggaagcggttctggcggatcaggatctggaagtggcggctctggaagcggaggttctggatctggcgaagaactgctgtctaagaattatcacggttcaggctccggccagcggggaagcaagcgcaccgccgatggttccgagttcgaaagccccaaaaaaaagcgcaaggtctga

SEQ ID NO: 292 - DNA, 6441 bp, synthetic construct
  misc_feature 1..6441: note = CDS of V4_D3a-D3l-dCas9-2xGCN4
  source 1..6441: mol_type = other DNA
atgcctgctgctaagagagtgaaactggatggatccaaccatgaccaggaatttgaccccccaaaggtttacccacctgtgccagctgagaagaggaagcccatccgcgtgctgtctctctttgatgggattgctacagggctcctggtgctgaaggacctgggcatccaagtggaccgctacattgcctccgaggtgtgtgaggactccatcacggtgggcatggtgcggcaccagggaaagatcatgtacgtcggggacgtccgcagcgtcacacagaagcatatccaggagtggggcccattcgacctggtgattggaggcagtccctgcaatgacctctccattgtcaaccctgcccgcaagggactttatgagggtactggccgcctcttctttgagttctaccgcctcctgcatgatgcgcggcccaaggagggagatgatcgccccttcttctggctctttgagaatgtggtggccatgggcgttagtgacaagagggacatctcgcgatttcttgagtctaaccccgtgatgattgacgccaaagaagtgtctgctgcacacagggcccgttacttctggggtaaccttcctggcatgaacaggcctttggcatccactgtgaatgataagctggagctgcaagagtgtctggagcacggcagaatagccaagttcagcaaagtgaggaccattaccaccaggtcaaactctataaagcagggcaaagaccagcatttccccgtcttcatgaacgagaaggaggacatcctgtggtgcactgaaatggaaagggtgtttggcttccccgtccactacacagacgtctccaacatgagccgcttggcgaggcagagactgctgggccgatcgtggagcgtgccggtcatccgccacctcttcgctccgctgaaggaatattttgcttgtgtgtctagcggcaatagtaacgctaacagccgcgggccgagcttcagcagcggcctggtgccgttaagcttgcgcggcagccatatgggccctatggagatatacaagacagtgtctgcatggaagagacagccagtgcgggtactgagcctcttcagaaacatcgacaaggtactaaagagtttgggcttcttggaaagcggttctggttctgggggaggaacgctgaagtacgtggaagatgtcacaaatgtcgtgaggagagacgtggagaaatggggcccctttgacctggtgtacggctcgacgcagcccctaggcagctcttgtgatcgctgtcccggctggtacatgttccagttccaccggatcctgcagtatgcgctgcctcgccaggagagtcagcggcccttcttctggatattcatggacaatctgctgctgactgaggatgaccaagagacaactacccgcttccttcagacagaggctgtgaccctccaggatgtccgtggcagagactaccagaatgctatgcgggtgtggagcaacattccagggctgaagagcaagcatgcgcccctgaccccaaaggaagaagagtatctgcaagcccaagtcagaagcaggagcaagctggacgccccgaaagttgacctcctggtgaagaactgccttctcccgctgagagagtacttcaagtatttttctcaaaactcacttcctcttggagggccgagctctggcgcacccccaccaagtggagggtctcctgccgggtccccaacatctactgaagaaggcaccagcgaatccgcaacgcccgagtcaggccctggtacctccacagaaccatctgaaggtagtgcgcctggttccccagctggaagccctacttccaccgaagaaggcacgtcaaccgaaccaagtgaaggatctgcccctgggaccagcactgaaccatctgagccaaaaaagaagagaaaggtaatggacaagaagtacagcatcggcctggccatcggcaccaactctgtgggctgggccgtgatcaccgacgagtacaaggtgcccagcaagaaattcaaggtgctgggcaacaccgaccggcacagcatcaagaagaacctgatcggcgccctgctgttcgacagcggagaaacagccgaggccacccggctgaagagaaccgccagaagaagatacaccagacggaagaaccggatctgctatctgcaagagatcttcagcaacgagatggccaaggtggacgacagcttcttccacagactggaagagtccttcctggtggaagaggataagaagcacgagcggcaccccatcttcggcaacatcgtggacgaggtggcctaccacgagaagtaccccaccatctaccacctgagaaagaaactggtggacagcaccgacaaggccgacctgcggctgatctatctggccctggcccacatgatcaagttccggggccacttcctgatcgagggcgacctgaaccccgacaacagcgacgtggacaagctgttcatccagctggtgcagacctacaaccagctgttcgaggaaaaccccatcaacgccagcggcgtggacgccaaggccatcctgtctgccagactgagcaagagcagacggctggaaaatctgatcgcccagctgcccggcgagaagaagaatggcctgttcggcaacctgattgccctgagcctgggcctgacccccaacttcaagagcaacttcgacctggccgaggatgccaaactgcagctgagcaaggacacctacgacgacgacctggacaacctgctggcccagatcggcgaccagtacgccgacctgtttctggccgccaagaacctgtccgacgccatcctgctgagcgacatcctgagagtgaacaccgagatcaccaaggcccccctgagcgcctctatgatcaagagatacgacgagcaccaccaggacctgaccctgctgaaagctctcgtgcggcagcagctgcctgagaagtacaaagagattttcttcgaccagagcaagaacggctacgccggctacatcgatggcggagccagccaggaagagttctacaagttcatcaagcccatcctggaaaagatggacggcaccgaggaactgctcgtgaagctgaacagagaggacctgctgcggaagcagcggaccttcgacaacggcagcatcccccaccagatccacctgggagagctgcacgccattctgcggcggcaggaagatttttacccattcctgaaggacaaccgggaaaagatcgagaagatcctgaccttccgcatcccctactacgtgggccctctggccaggggaaacagcagattcgcctggatgaccagaaagagcgaggaaaccatcaccccctggaacttcgaggaagtggtggacaagggcgccagcgcccagagcttcatcgagcggatgaccaacttcgataagaacctgcccaacgagaaggtgctgcccaagcacagcctgctgtacgagtacttcaccgtgtacaacgagctgaccaaagtgaaatacgtgaccgagggaatgagaaagcccgccttcctgagcggcgagcagaaaaaagccatcgtggacctgctgttcaagaccaaccggaaagtgaccgtgaagcagctgaaagaggactacttcaagaaaatcgagtgcttcgactccgtggaaatctccggcgtggaagatcggttcaacgcctccctgggcacataccacgatctgctgaaaattatcaaggacaaggacttcctggacaatgaggaaaacgaggacattctggaagatatcgtgctgaccctgacactgtttgaggacagagagatgatcgaggaacggctgaaaacctatgcccacctgttcgacgacaaagtgatgaagcagctgaagcggcggagatacaccggctggggcaggctgagccggaagctgatcaacggcatccgggacaagcagtccggcaagacaatcctggatttcctgaagtccgacggcttcgccaacagaaacttcatgcagctgatccacgacgacagcctgacctttaaagaggacatccagaaagcccaggtgtccggccagggcgatagcctgcacgagcacattgccaatctggccggcagccccgccattaagaagggcatcctgcagacagtgaaggtggtggacgagctcgtgaaagtgatgggccggcacaagcccgagaacatcgtgatcgaaatggccagagagaaccagaccacccagaagggacagaagaacagccgcgagagaatgaagcggatcgaagagggcatcaaagagctgggcagccagatcctgaaagaacaccccgtggaaaacacccagctgcagaacgagaagctgtacctgtactacctgcagaatgggcgggatatgtacgtggaccaggaactggacatcaaccggctgtccgactacgatgtggacgctatcgtgcctcagagctttctgaaggacgactccatcgataacaaagtgctgactcggagcgacaagaaccggggcaagagcgacaacgtgccctccgaagaggtcgtgaagaagatgaagaactactggcgccagctgctgaatgccaagctgattacccagaggaagttcgacaatctgaccaaggccgagagaggcggcctgagcgaactggataaggccggcttcatcaagagacagctggtggaaacccggcagatcacaaagcacgtggcacagatcctggactcccggatgaacactaagtacgacgagaacgacaaactgatccgggaagtgaaagtgatcaccctgaagtccaagctggtgtccgatttccggaaggatttccagttttacaaagtgcgcgagatcaacaactaccaccacgcccacgacgcctacctgaacgccgtcgtgggaaccgccctgatcaaaaagtaccctaagctggaaagcgagttcgtgtacggcgactacaaggtgtacgacgtgcggaagatgatcgccaagagcgagcaggaaatcggcaaggctaccgccaagtacttcttctacagcaacatcatgaactttttcaagaccgagattaccctggccaacggcgagatccggaagcggcctctgatcgagacaaacggcgaaacaggcgagatcgtgtgggataagggccgggactttgccaccgtgcggaaagtgctgtctatgccccaagtgaatatcgtgaaaaagaccgaggtgcagacaggcggcttcagcaaagagtctatcctgcccaagaggaacagcgacaagctgatcgccagaaagaaggactgggaccctaagaagtacggcggcttcgacagccccaccgtggcctattctgtgctggtggtggccaaagtggaaaagggcaagtccaagaaactgaagagtgtgaaagagctgctggggatcaccatcatggaaagaagcagcttcgagaagaatcccatcgactttctggaagccaagggctacaaagaagtgaaaaaggacctgatcatcaagctgcctaagtactccctgttcgagctggaaaacggccggaagagaatgctggcctctgccggcgaactgcagaagggaaacgaactggccctgccctccaaatatgtgaacttcctgtacctggccagccactatgagaagctgaagggctcccccgaggataatgagcagaaacagctgtttgtggaacagcacaaacactacctggacgagatcatcgagcagatcagcgagttctccaagagagtgatcctggccgacgctaatctggacaaggtgctgagcgcctacaacaagcacagagacaagcctatcagagagcaggccgagaatatcatccacctgtttaccctgaccaatctgggagcccctgccgccttcaagtactttgacaccaccatcgaccggaagaggtacaccagcaccaaagaggtgctggacgccaccctgatccaccagagcatcaccggcctgtacgagacacggatcgacctgtctcagctgggaggcgacgcctatccctatgacgtgcccgattatgccagcctgggcagcggctcccccaagaaaaaacgcaaggtggaagatcctaagaaaaagcggaaagtggacggcattggtagtgggagcaacggcagcagcggagaggaactgctgagcaagaactaccacctggaaaacgaggtggccagactgaagaaaggctctggctctggcggaagcggttctggcggatcaggatctggaagtggcggctctggaagcggaggttctggatctggcgaagaactgctgtctaagaattatcacctcgagaatgaagtcgctcgtttgaagaaaggttcaggctccggccagcggggaagcaagcgcaccgccgatggttccgagttcgaaagccccaaaaaaaagcgcaaggtctga

SEQ ID NO: 293 - DNA, 6717 bp, synthetic construct
  misc_feature 1..6717: note = CDS of V5_D3a-D3l-dCas9-4xGCN4
  source 1..6717: mol_type = other DNA
atgcctgctgctaagagagtgaaactggatggatccaaccatgaccaggaatttgaccccccaaaggtttacccacctgtgccagctgagaagaggaagcccatccgcgtgctgtctctctttgatgggattgctacagggctcctggtgctgaaggacctgggcatccaagtggaccgctacattgcctccgaggtgtgtgaggactccatcacggtgggcatggtgcggcaccagggaaagatcatgtacgtcggggacgtccgcagcgtcacacagaagcatatccaggagtggggcccattcgacctggtgattggaggcagtccctgcaatgacctctccattgtcaaccctgcccgcaagggactttatgagggtactggccgcctcttctttgagttctaccgcctcctgcatgatgcgcggcccaaggagggagatgatcgccccttcttctggctctttgagaatgtggtggccatgggcgttagtgacaagagggacatctcgcgatttcttgagtctaaccccgtgatgattgacgccaaagaagtgtctgctgcacacagggcccgttacttctggggtaaccttcctggcatgaacaggcctttggcatccactgtgaatgataagctggagctgcaagagtgtctggagcacggcagaatagccaagttcagcaaagtgaggaccattaccaccaggtcaaactctataaagcagggcaaagaccagcatttccccgtcttcatgaacgagaaggaggacatcctgtggtgcactgaaatggaaagggtgtttggcttccccgtccactacacagacgtctccaacatgagccgcttggcgaggcagagactgctgggccgatcgtggagcgtgccggtcatccgccacctcttcgctccgctgaaggaatattttgcttgtgtgtctagcggcaatagtaacgctaacagccgcgggccgagcttcagcagcggcctggtgccgttaagcttgcgcggcagccatatgggccctatggagatatacaagacagtgtctgcatggaagagacagccagtgcgggtactgagcctcttcagaaacatcgacaaggtactaaagagtttgggcttcttggaaagcggttctggttctgggggaggaacgctgaagtacgtggaagatgtcacaaatgtcgtgaggagagacgtggagaaatggggcccctttgacctggtgtacggctcgacgcagcccctaggcagctcttgtgatcgctgtcccggctggtacatgttccagttccaccggatcctgcagtatgcgctgcctcgccaggagagtcagcggcccttcttctggatattcatggacaatctgctgctgactgaggatgaccaagagacaactacccgcttccttcagacagaggctgtgaccctccaggatgtccgtggcagagactaccagaatgctatgcgggtgtggagcaacattccagggctgaagagcaagcatgcgcccctgaccccaaaggaagaagagtatctgcaagcccaagtcagaagcaggagcaagctggacgccccgaaagttgacctcctggtgaagaactgccttctcccgctgagagagtacttcaagtatttttctcaaaactcacttcctcttggagggccgagctctggcgcacccccaccaagtggagggtctcctgccgggtccccaacatctactgaagaaggcaccagcgaatccgcaacgcccgagtcaggccctggtacctccacagaaccatctgaaggtagtgcgcctggttccccagctggaagccctacttccaccgaagaaggcacgtcaaccgaaccaagtgaaggatctgcccctgggaccagcactgaaccatctgagccaaaaaagaagagaaaggtaatggacaagaagtacagcatcggcctggccatcggcaccaactctgtgggctgggccgtgatcaccgacgagtacaaggtgcccagcaagaaattcaaggtgctgggcaacaccgaccggcacagcatcaagaagaacctgatcggcgccctgctgttcgacagcggagaaacagccgaggccacccggctgaagagaaccgccagaagaagatacaccagacggaagaaccggatctgctatctgcaagagatcttcagcaacgagatggccaaggtggacgacagcttcttccacagactggaagagtccttcctggtggaagaggataagaagcacgagcggcaccccatcttcggcaacatcgtggacgaggtggcctaccacgagaagtaccccaccatctaccacctgagaaagaaactggtggacagcaccgacaaggccgacctgcggctgatctatctggccctggcccacatgatcaagttccggggccacttcctgatcgagggcgacctgaaccccgacaacagcgacgtggacaagctgttcatccagctggtgcagacctacaaccagctgttcgaggaaaaccccatcaacgccagcggcgtggacgccaaggccatcctgtctgccagactgagcaagagcagacggctggaaaatctgatcgcccagctgcccggcgagaagaagaatggcctgttcggcaacctgattgccctgagcctgggcctgacccccaacttcaagagcaacttcgacctggccgaggatgccaaactgcagctgagcaaggacacctacgacgacgacctggacaacctgctggcccagatcggcgaccagtacgccgacctgtttctggccgccaagaacctgtccgacgccatcctgctgagcgacatcctgagagtgaacaccgagatcaccaaggcccccctgagcgcctctatgatcaagagatacgacgagcaccaccaggacctgaccctgctgaaagctctcgtgcggcagcagctgcctgagaagtacaaagagattttcttcgaccagagcaagaacggctacgccggctacatcgatggcggagccagccaggaagagttctacaagttcatcaagcccatcctggaaaagatggacggcaccgaggaactgctcgtgaagctgaacagagaggacctgctgcggaagcagcggaccttcgacaacggcagcatcccccaccagatccacctgggagagctgcacgccattctgcggcggcaggaagatttttacccattcctgaaggacaaccgggaaaagatcgagaagatcctgaccttccgcatcccctactacgtgggccctctggccaggggaaacagcagattcgcctggatgaccagaaagagcgaggaaaccatcaccccctggaacttcgaggaagtggtggacaagggcgccagcgcccagagcttcatcgagcggatgaccaacttcgataagaacctgcccaacgagaaggtgctgcccaagcacagcctgctgtacgagtacttcaccgtgtacaacgagctgaccaaagtgaaatacgtgaccgagggaatgagaaagcccgccttcctgagcggcgagcagaaaaaagccatcgtggacctgctgttcaagaccaaccggaaagtgaccgtgaagcagctgaaagaggactacttcaagaaaatcgagtgcttcgactccgtggaaatctccggcgtggaagatcggttcaacgcctccctgggcacataccacgatctgctgaaaattatcaaggacaaggacttcctggacaatgaggaaaacgaggacattctggaagatatcgtgctgaccctgacactgtttgaggacagagagatgatcgaggaacggctgaaaacctatgcccacctgttcgacgacaaagtgatgaagcagctgaagcggcggagatacaccggctggggcaggctgagccggaagctgatcaacggcatccgggacaagcagtccggcaagacaatcctggatttcctgaagtccgacggcttcgccaacagaaacttcatgcagctgatccacgacgacagcctgacctttaaagaggacatccagaaagcccaggtgtccggccagggcgatagcctgcacgagcacattgccaatctggccggcagccccgccattaagaagggcatcctgcagacagtgaaggtggtggacgagctcgtgaaagtgatgggccggcacaagcccgagaacatcgtgatcgaaatggccagagagaaccagaccacccagaagggacagaagaacagccgcgagagaatgaagcggatcgaagagggcatcaaagagctgggcagccagatcctgaaagaacaccccgtggaaaacacccagctgcagaacgagaagctgtacctgtactacctgcagaatgggcgggatatgtacgtggaccaggaactggacatcaaccggctgtccgactacgatgtggacgctatcgtgcctcagagctttctgaaggacgactccatcgataacaaagtgctgactcggagcgacaagaaccggggcaagagcgacaacgtgccctccgaagaggtcgtgaagaagatgaagaactactggcgccagctgctgaatgccaagctgattacccagaggaagttcgacaatctgaccaaggccgagagaggcggcctgagcgaactggataaggccggcttcatcaagagacagctggtggaaacccggcagatcacaaagcacgtggcacagatcctggactcccggatgaacactaagtacgacgagaacgacaaactgatccgggaagtgaaagtgatcaccctgaagtccaagctggtgtccgatttccggaaggatttccagttttacaaagtgcgcgagatcaacaactaccaccacgcccacgacgcctacctgaacgccgtcgtgggaaccgccctgatcaaaaagtaccctaagctggaaagcgagttcgtgtacggcgactacaaggtgtacgacgtgcggaagatgatcgccaagagcgagcaggaaatcggcaaggctaccgccaagtacttcttctacagcaacatcatgaactttttcaagaccgagattaccctggccaacggcgagatccggaagcggcctctgatcgagacaaacggcgaaacaggcgagatcgtgtgggataagggccgggactttgccaccgtgcggaaagtgctgtctatgccccaagtgaatatcgtgaaaaagaccgaggtgcagacaggcggcttcagcaaagagtctatcctgcccaagaggaacagcgacaagctgatcgccagaaagaaggactgggaccctaagaagtacggcggcttcgacagccccaccgtggcctattctgtgctggtggtggccaaagtggaaaagggcaagtccaagaaactgaagagtgtgaaagagctgctggggatcaccatcatggaaagaagcagcttcgagaagaatcccatcgactttctggaagccaagggctacaaagaagtgaaaaaggacctgatcatcaagctgcctaagtactccctgttcgagctggaaaacggccggaagagaatgctggcctctgccggcgaactgcagaagggaaacgaactggccctgccctccaaatatgtgaacttcctgtacctggccagccactatgagaagctgaagggctcccccgaggataatgagcagaaacagctgtttgtggaacagcacaaacactacctggacgagatcatcgagcagatcagcgagttctccaagagagtgatcctggccgacgctaatctggacaaggtgctgagcgcctacaacaagcacagagacaagcctatcagagagcaggccgagaatatcatccacctgtttaccctgaccaatctgggagcccctgccgccttcaagtactttgacaccaccatcgaccggaagaggtacaccagcaccaaagaggtgctggacgccaccctgatccaccagagcatcaccggcctgtacgagacacggatcgacctgtctcagctgggaggcgacgcctatccctatgacgtgcccgattatgccagcctgggcagcggctcccccaagaaaaaacgcaaggtggaagatcctaagaaaaagcggaaagtggacggcattggtagtgggagcaacggcagcagcggagaggaactgctgagcaagaactaccacctggaaaacgaggtggccagactgaagaaaggctctggctctggcggaagcggttctggcggatcaggatctggaagtggcggctctggaagcggaggttctggatctggcgaagaactgctgtctaagaattatcacctcgagaacgaagtcgcccgcctcaagaaaggttctggcagcggaggctctggcagtggtggtagcggaagtggaagtggtggcagtggtagcggtggatctggaagcggcgaggaactcctgtcaaagaattaccatctcgaaaacgaggtcgcaaggctcaagaaaggctcaggatcaggcggctctggatccggcggttctggttccggctcaggtggaagtggatctggcggctcaggttccggcgaagaattgctttccaagaactaccatttggaaaatgaagtcgctcgtttgaagaaaggttcaggctccggccagcggggaagcaagcgcaccgccgatggttccgagttcgaaagccccaaaaaaaagcgcaaggtctga

SEQ ID NO: 294 - DNA, 7545 bp, synthetic construct
  misc_feature 1..7545: note = CDS of V6_D3a-D3l-dCas9-10xGCN4
  source 1..7545: mol_type = other DNA
atgcctgctgctaagagagtgaaactggatggatccaaccatgaccaggaatttgaccccccaaaggtttacccacctgtgccagctgagaagaggaagcccatccgcgtgctgtctctctttgatgggattgctacagggctcctggtgctgaaggacctgggcatccaagtggaccgctacattgcctccgaggtgtgtgaggactccatcacggtgggcatggtgcggcaccagggaaagatcatgtacgtcggggacgtccgcagcgtcacacagaagcatatccaggagtggggcccattcgacctggtgattggaggcagtccctgcaatgacctctccattgtcaaccctgcccgcaagggactttatgagggtactggccgcctcttctttgagttctaccgcctcctgcatgatgcgcggcccaaggagggagatgatcgccccttcttctggctctttgagaatgtggtggccatgggcgttagtgacaagagggacatctcgcgatttcttgagtctaaccccgtgatgattgacgccaaagaagtgtctgctgcacacagggcccgttacttctggggtaaccttcctggcatgaacaggcctttggcatccactgtgaatgataagctggagctgcaagagtgtctggagcacggcagaatagccaagttcagcaaagtgaggaccattaccaccaggtcaaactctataaagcagggcaaagaccagcatttccccgtcttcatgaacgagaaggaggacatcctgtggtgcactgaaatggaaagggtgtttggcttccccgtccactacacagacgtctccaacatgagccgcttggcgaggcagagactgctgggccgatcgtggagcgtgccggtcatccgccacctcttcgctccgctgaaggaatattttgcttgtgtgtctagcggcaatagtaacgctaacagccgcgggccgagcttcagcagcggcctggtgccgttaagcttgcgcggcagccatatgggccctatggagatatacaagacagtgtctgcatggaagagacagccagtgcgggtactgagcctcttcagaaacatcgacaaggtactaaagagtttgggcttcttggaaagcggttctggttctgggggaggaacgctgaagtacgtggaagatgtcacaaatgtcgtgaggagagacgtggagaaatggggcccctttgacctggtgtacggctcgacgcagcccctaggcagctcttgtgatcgctgtcccggctggtacatgttccagttccaccggatcctgcagtatgcgctgcctcgccaggagagtcagcggcccttcttctggatattcatggacaatctgctgctgactgaggatgaccaagagacaactacccgcttccttcagacagaggctgtgaccctccaggatgtccgtggcagagactaccagaatgctatgcgggtgtggagcaacattccagggctgaagagcaagcatgcgcccctgaccccaaaggaagaagagtatctgcaagcccaagtcagaagcaggagcaagctggacgccccgaaagttgacctcctggtgaagaactgccttctcccgctgagagagtacttcaagtatttttctcaaaactcacttcctcttggagggccgagctctggcgcacccccaccaagtggagggtctcctgccgggtccccaacatctactgaagaaggcaccagcgaatccgcaacgcccgagtcaggccctggtacctccacagaaccatctgaaggtagtgcgcctggttccccagctggaagccctacttccaccgaagaaggcacgtcaaccgaaccaagtgaaggatctgcccctgggaccagcactgaaccatctgagccaaaaaagaagagaaaggtaatggacaagaagtacagcatcggcctggccatcggcaccaactctgtgggctgggccgtgatcaccgacgagtacaaggtgcccagcaagaaattcaaggtgctgggcaacaccgaccggcacagcatcaagaagaacctgatcggcgccctgctgttcgacagcggagaaacagccgaggccacccggctgaagagaaccgccagaagaagatacaccagacggaagaaccggatctgctatctgcaagagatcttcagcaacgagatggccaaggtggacgacagcttcttccacagactggaagagtccttcctggtggaagaggataagaagcacgagcggcaccccatcttcggcaacatcgtggacgaggtggcctaccacgagaagtaccccaccatctaccacctgagaaagaaactggtggacagcaccgacaaggccgacctgcggctgatctatctggccctggcccacatgatcaagttccggggccacttcctgatcgagggcgacctgaaccccgacaacagcgacgtggacaagctgttcatccagctggtgcagacctacaaccagctgttcgaggaaaaccccatcaacgccagcggcgtggacgccaaggccatcctgtctgccagactgagcaagagcagacggctggaaaatctgatcgcccagctgcccggcgagaagaagaatggcctgttcggcaacctgattgccctgagcctgggcctgacccccaacttcaagagcaacttcgacctggccgaggatgccaaactgcagctgagcaaggacacctacgacgacgacctggacaacctgctggcccagatcggcgaccagtacgccgacctgtttctggccgccaagaacctgtccgacgccatcctgctgagcgacatcctgagagtgaacaccgagatcaccaaggcccccctgagcgcctctatgatcaagagatacgacgagcaccaccaggacctgaccctgctgaaagctctcgtgcggcagcagctgcctgagaagtacaaagagattttcttcgaccagagcaagaacggctacgccggctacatcgatggcggagccagccaggaagagttctacaagttcatcaagcccatcctggaaaagatggacggcaccgaggaactgctcgtgaagctgaacagagaggacctgctgcggaagcagcggaccttcgacaacggcagcatcccccaccagatccacctgggagagctgcacgccattctgcggcggcaggaagatttttacccattcctgaaggacaaccgggaaaagatcgagaagatcctgaccttccgcatcccctactacgtgggccctctggccaggggaaacagcagattcgcctggatgaccagaaagagcgaggaaaccatcaccccctggaacttcgaggaagtggtggacaagggcgccagcgcccagagcttcatcgagcggatgaccaacttcgataagaacctgcccaacgagaaggtgctgcccaagcacagcctgctgtacgagtacttcaccgtgtacaacgagctgaccaaagtgaaatacgtgaccgagggaatgagaaagcccgccttcctgagcggcgagcagaaaaaagccatcgtggacctgctgttcaagaccaaccggaaagtgaccgtgaagcagctgaaagaggactacttcaagaaaatcgagtgcttcgactccgtggaaatctccggcgtggaagatcggttcaacgcctccctgggcacataccacgatctgctgaaaattatcaaggacaaggacttcctggacaatgaggaaaacgaggacattctggaagatatcgtgctgaccctgacactgtttgaggacagagagatgatcgaggaacggctgaaaacctatgcccacctgttcgacgacaaagtgatgaagcagctgaagcggcggagatacaccggctggggcaggctgagccggaagctgatcaacggcatccgggacaagcagtccggcaagacaatcctggatttcctgaagtccgacggcttcgccaacagaaacttcatgcagctgatccacgacgacagcctgacctttaaagaggacatccagaaagcccaggtgtccggccagggcgatagcctgcacgagcacattgccaatctggccggcagccccgccattaagaagggcatcctgcagacagtgaaggtggtggacgagctcgtgaaagtgatgggccggcacaagcccgagaacatcgtgatcgaaatggccagagagaaccagaccacccagaagggacagaagaacagccgcgagagaatgaagcggatcgaagagggcatcaaagagctgggcagccagatcctgaaagaacaccccgtggaaaacacccagctgcagaacgagaagctgtacctgtactacctgcagaatgggcgggatatgtacgtggaccaggaactggacatcaaccggctgtccgactacgatgtggacgctatcgtgcctcagagctttctgaaggacgactccatcgataacaaagtgctgactcggagcgacaagaaccggggcaagagcgacaacgtgccctccgaagaggtcgtgaagaagatgaagaactactggcgccagctgctgaatgccaagctgattacccagaggaagttcgacaatctgaccaaggccgagagaggcggcctgagcgaactggataaggccggcttcatcaagagacagctggtggaaacccggcagatcacaaagcacgtggcacagatcctggactcccggatgaacactaagtacgacgagaacgacaaactgatccgggaagtgaaagtgatcaccctgaagtccaagctggtgtccgatttccggaaggatttccagttttacaaagtgcgcgagatcaacaactaccaccacgcccacgacgcctacctgaacgccgtcgtgggaaccgccctgatcaaaaagtaccctaagctggaaagcgagttcgtgtacggcgactacaaggtgtacgacgtgcggaagatgatcgccaagagcgagcaggaaatcggcaaggctaccgccaagtacttcttctacagcaacatcatgaactttttcaagaccgagattaccctggccaacggcgagatccggaagcggcctctgatcgagacaaacggcgaaacaggcgagatcgtgtgggataagggccgggactttgccaccgtgcggaaagtgctgtctatgccccaagtgaatatcgtgaaaaagaccgaggtgcagacaggcggcttcagcaaagagtctatcctgcccaagaggaacagcgacaagctgatcgccagaaagaaggactgggaccctaagaagtacggcggcttcgacagccccaccgtggcctattctgtgctggtggtggccaaagtggaaaagggcaagtccaagaaactgaagagtgtgaaagagctgctggggatcaccatcatggaaagaagcagcttcgagaagaatcccatcgactttctggaagccaagggctacaaagaagtgaaaaaggacctgatcatcaagctgcctaagtactccctgttcgagctggaaaacggccggaagagaatgctggcctctgccggcgaactgcagaagggaaacgaactggccctgccctccaaatatgtgaacttcctgtacctggccagccactatgagaagctgaagggctcccccgaggataatgagcagaaacagctgtttgtggaacagcacaaacactacctggacgagatcatcgagcagatcagcgagttctccaagagagtgatcctggccgacgctaatctggacaaggtgctgagcgcctacaacaagcacagagacaagcctatcagagagcaggccgagaatatcatccacctgtttaccctgaccaatctgggagcccctgccgccttcaagtactttgacaccaccatcgaccggaagaggtacaccagcaccaaagaggtgctggacgccaccctgatccaccagagcatcaccggcctgtacgagacacggatcgacctgtctcagctgggaggcgacgcctatccctatgacgtgcccgattatgccagcctgggcagcggctcccccaagaaaaaacgcaaggtggaagatcctaagaaaaagcggaaagtggacggcattggtagtgggagcaacggcagcagcggagaggaactgctgagcaagaactaccacctggaaaacgaggtggccagactgaagaaaggctctggctctggcggaagcggttctggcggatcaggatctggaagtggcggctctggaagcggaggttctggatctggcgaagaactgctgtctaagaattatcacctcgagaacgaagtggctcggctcaagaaaggcagtggcagcggaggaagtggatccggcggtagtggtagtggaagcggcggatccggctcaggcggatctggttcaggggaagaactcctctccaaaaactaccatctcgagaatgaggtcgcccgcctgaaaaaaggatcaggttccggtggttctggcagcggtggttcaggctcaggcagcggcggtagcggtagcggtggaagcggaagcggagaagaacttctcagcaaaaattaccacttggagaatgaagttgcaagactcaaaaaaggttccggcagtggcggcagcggcagcggcggatctggtagtggatctggtggcagtggttcaggcggaagtggtagcggagaggaattgctctcaaagaactatcatttggagaacgaggttgcacgcttgaagaaaggcagcggatcaggcggatctggcagcggtggatctggttctggatccggcggctccggtagtggtggaagtggctctggggaagaattgcttagcaagaattatcatcttgaaaatgaggttgccaggcttaaaaaaggcagtggctccggcggatccggaagcggaggcagcggatctggatctggtggttcaggatctggcggttctggtagcggggaagaactgttgagtaaaaactatcaccttgagaacgaggtcgcaaggttgaaaaaaggatccggctctggcggctccggaagtggcggatctggctccggtagcggaggatcaggatccggcggaagcggatcaggcgaggaactgctttccaaaaattaccaccttgaaaacgaagtcgcccgcctcaagaaaggttctggcagcggaggctctggcagtggtggtagcggaagtggaagtggtggcagtggtagcggtggatctggaagcggcgaggaactcctgtcaaagaattaccatctcgaaaacgaggtcgcaaggctcaagaaaggctcaggatcaggcggctctggatccggcggttctggttccggctcaggtggaagtggatctggcggctcaggttccggcgaagaattgctttccaagaactaccatttggaaaatgaagtcgctcgtttgaagaaaggttcaggctccggccagcggggaagcaagcgcaccgccgatggttccgagttcgaaagccccaaaaaaaagcgcaaggtctga

SEQ ID NO: 295 - DNA, 2736 bp, synthetic construct
  misc_feature 1..2736: note = CDS of V7_D3a-D3l-scFv
  source 1..2736: mol_type = other DNA
atgcctgctgctaagagagtgaaactggatggatccaaccatgaccaggaatttgaccccccaaaggtttacccacctgtgccagctgagaagaggaagcccatccgcgtgctgtctctctttgatgggattgctacagggctcctggtgctgaaggacctgggcatccaagtggaccgctacattgcctccgaggtgtgtgaggactccatcacggtgggcatggtgcggcaccagggaaagatcatgtacgtcggggacgtccgcagcgtcacacagaagcatatccaggagtggggcccattcgacctggtgattggaggcagtccctgcaatgacctctccattgtcaaccctgcccgcaagggactttatgagggtactggccgcctcttctttgagttctaccgcctcctgcatgatgcgcggcccaaggagggagatgatcgccccttcttctggctctttgagaatgtggtggccatgggcgttagtgacaagagggacatctcgcgatttcttgagtctaaccccgtgatgattgacgccaaagaagtgtctgctgcacacagggcccgttacttctggggtaaccttcctggcatgaacaggcctttggcatccactgtgaatgataagctggagctgcaagagtgtctggagcacggcagaatagccaagttcagcaaagtgaggaccattaccaccaggtcaaactctataaagcagggcaaagaccagcatttccccgtgttcatgaacgagaaggaggacatcctgtggtgcactgaaatggaaagggtgtttggcttccccgtccactacacagacgtctccaacatgagccgcttggcgaggcagagactgctgggccgatcgtggagcgtgccggtcatccgccacctcttcgctccgctgaaggaatattttgcttgtgtgtctagcggcaatagtaacgctaacagccgcgggccgagcttcagcagcggcctggtgccgttaagcttgcgcggcagccatatgggccctatggagatatacaagacagtgtctgcatggaagagacagccagtgcgggtactgagcctcttcagaaacatcgacaaggtactaaagagtttgggcttcttggaaagcggttctggttctgggggaggaacgctgaagtacgtggaagatgtcacaaatgtcgtgaggagagacgtggagaaatggggcccctttgacctggtgtacggctcgacgcagcccctaggcagctcttgtgatcgctgtcccggctggtacatgttccagttccaccggatcctgcagtatgcgctgcctcgccaggagagtcagcggcccttcttctggatattcatggacaatctgctgctgactgaggatgaccaagagacaactacccgcttccttcagacagaggctgtgaccctccaggatgtccgtggcagagactaccagaatgctatgcgggtgtggagcaacattccagggctgaagagcaagcatgcgcccctgaccccaaaggaagaagagtatctgcaagcccaagtcagaagcaggagcaagctggacgccccgaaagttgacctcctggtgaagaactgccttctcccgctgagagagtacttcaagtatttttctcaaaactcacttcctcttggagggccgagctctggcgcacccccaccaagtggagggtctcctgccgggtccccaacatctactgaagaaggcaccagcgaatccgcaacgcccgagtcaggccctggtacctccacagaaccatctgaaggtagtgcgcctggttccccagctggaagccctacttccaccgaagaaggcacgtcaaccgaaccaagtgaaggatctgcccctgggaccagcactgaaccatctgagggccccgacatcgtgatgacccagagccccagcagcctgagcgccagcgtgggcgaccgcgtgaccatcacctgccgcagcagcaccggcgccgtgaccaccagcaactacgccagctgggtgcaggagaagcccggcaagctgttcaagggcctgatcggcggcaccaacaaccgcgcccccggcgtgcccagccgcttcagcggcagcctgatcggcgacaaggccaccctgaccatcagcagcctgcagcccgaggacttcgccacctacttctgcgccctgtggtacagcaaccactgggtgttcggccagggcaccaaggtggagctgaagcgcggcggcggcggcagcggcggcggcggcagcggcggcggcggcagcagcggcggcggcagcgaggtgaagctgctggagagcggcggcggcctggtgcagcccggcggcagcctgaagctgagctgcgccgtgagcggcttcagcctgaccgactacggcgtgaactgggtgcgccaggcccccggccgcggcctggagtggatcggcgtgatctggggcgacggcatcaccgactacaacagcgccctgaaggaccgcttcatcatcagcaaggacaacggcaagaacaccgtgtacctgcagatgagcaaggtgcgcagcgacgacaccgccctgtactactgcgtgaccggcctgttcgactactggggccagggcaccctggtgaccgtgagcagctacccatacgatgttccagattacgctggtggaggcggaggttctgggggaggaggtagtggcggtggtggttcaggaggcggcggaagctag

SEQ ID NO: 296 - DNA, 4914 bp, synthetic construct
  misc_feature 1..4914: note = CDS of V8_3xGCN4-dCas9-KRAB
  source 1..4914: mol_type = other DNA
atgcctgctgctaagagagtgaaactggatggatccgaggaactgctgagcaagaactaccacctggaaaacgaggtggccagactgaagaaaggctctggctctggcggaagcggttctggcggatcaggatctggaagtggcggctctggaagcggaggttctggatctggcgaagaactgctgtctaagaattatcacctcgagaacgaagtggctcggctcaagaaaggcagtggcagcggaggaagtggatccggcggtagtggtagtggaagcggcggatccggctcaggcggatctggttcaggggaagaactcctctccaaaaactaccatctcgagaatgaggtcgcccgcctgaaaaaaggatcaggttccggtggttctggcagcggtggttcaggctcaggcagcggcggtagcggtagcggtggaagcggaagcggaccaaaaaagaagagaaaggtaatggacaagaagtacagcatcggcctggccatcggcaccaactctgtgggctgggccgtgatcaccgacgagtacaaggtgcccagcaagaaattcaaggtgctgggcaacaccgaccggcacagcatcaagaagaacctgatcggcgccctgctgttcgacagcggagaaacagccgaggccacccggctgaagagaaccgccagaagaagatacaccagacggaagaaccggatctgctatctgcaagagatcttcagcaacgagatggccaaggtggacgacagcttcttccacagactggaagagtccttcctggtggaagaggataagaagcacgagcggcaccccatcttcggcaacatcgtggacgaggtggcctaccacgagaagtaccccaccatctaccacctgagaaagaaactggtggacagcaccgacaaggccgacctgcggctgatctatctggccctggcccacatgatcaagttccggggccacttcctgatcgagggcgacctgaaccccgacaacagcgacgtggacaagctgttcatccagctggtgcagacctacaaccagctgttcgaggaaaaccccatcaacgccagcggcgtggacgccaaggccatcctgtctgccagactgagcaagagcagacggctggaaaatctgatcgcccagctgcccggcgagaagaagaatggcctgttcggcaacctgattgccctgagcctgggcctgacccccaacttcaagagcaacttcgacctggccgaggatgccaaactgcagctgagcaaggacacctacgacgacgacctggacaacctgctggcccagatcggcgaccagtacgccgacctgtttctggccgccaagaacctgtccgacgccatcctgctgagcgacatcctgagagtgaacaccgagatcaccaaggcccccctgagcgcctctatgatcaagagatacgacgagcaccaccaggacctgaccctgctgaaagctctcgtgcggcagcagctgcctgagaagtacaaagagattttcttcgaccagagcaagaacggctacgccggctacatcgatggcggagccagccaggaagagttctacaagttcatcaagcccatcctggaaaagatggacggcaccgaggaactgctcgtgaagctgaacagagaggacctgctgcggaagcagcggaccttcgacaacggcagcatcccccaccagatccacctgggagagctgcacgccattctgcggcggcaggaagatttttacccattcctgaaggacaaccgggaaaagatcgagaagatcctgaccttccgcatcccctactacgtgggccctctggccaggggaaacagcagattcgcctggatgaccagaaagagcgaggaaaccatcaccccctggaacttcgaggaagtggtggacaagggcgccagcgcccagagcttcatcgagcggatgaccaacttcgataagaacctgcccaacgagaaggtgctgcccaagcacagcctgctgtacgagtacttcaccgtgtacaacgagctgaccaaagtgaaatacgtgaccgagggaatgagaaagcccgccttcctgagcggcgagcagaaaaaagccatcgtggacctgctgttcaagaccaaccggaaagtgaccgtgaagcagctgaaagaggactacttcaagaaaatcgagtgcttcgactccgtggaaatctccggcgtggaagatcggttcaacgcctccctgggcacataccacgatctgctgaaaattatcaaggacaaggacttcctggacaatgaggaaaacgaggacattctggaagatatcgtgctgaccctgacactgtttgaggacagagagatgatcgaggaacggctgaaaacctatgcccacctgttcgacgacaaagtgatgaagcagctgaagcggcggagatacaccggctggggcaggctgagccggaagctgatcaacggcatccgggacaagcagtccggcaagacaatcctggatttcctgaagtccgacggcttcgccaacagaaacttcatgcagctgatccacgacgacagcctgacctttaaagaggacatccagaaagcccaggtgtccggccagggcgatagcctgcacgagcacattgccaatctggccggcagccccgccattaagaagggcatcctgcagacagtgaaggtggtggacgagctcgtgaaagtgatgggccggcacaagcccgagaacatcgtgatcgaaatggccagagagaaccagaccacccagaagggacagaagaacagccgcgagagaatgaagcggatcgaagagggcatcaaagagctgggcagccagatcctgaaagaacaccccgtggaaaacacccagctgcagaacgagaagctgtacctgtactacctgcagaatgggcgggatatgtacgtggaccaggaactggacatcaaccggctgtccgactacgatgtggacgctatcgtgcctcagagctttctgaaggacgactccatcgataacaaagtgctgactcggagcgacaagaaccggggcaagagcgacaacgtgccctccgaagaggtcgtgaagaagatgaagaactactggcgccagctgctgaatgccaagctgattacccagaggaagttcgacaatctgaccaaggccgagagaggcggcctgagcgaactggataaggccggcttcatcaagagacagctggtggaaacccggcagatcacaaagcacgtggcacagatcctggactcccggatgaacactaagtacgacgagaacgacaaactgatccgggaagtgaaagtgatcaccctgaagtccaagctggtgtccgatttccggaaggatttccagttttacaaagtgcgcgagatcaacaactaccaccacgcccacgacgcctacctgaacgccgtcgtgggaaccgccctgatcaaaaagtaccctaagctggaaagcgagttcgtgtacggcgactacaaggtgtacgacgtgcggaagatgatcgccaagagcgagcaggaaatcggcaaggctaccgccaagtacttcttctacagcaacatcatgaactttttcaagaccgagattaccctggccaacggcgagatccggaagcggcctctgatcgagacaaacggcgaaacaggcgagatcgtgtgggataagggccgggactttgccaccgtgcggaaagtgctgtctatgccccaagtgaatatcgtgaaaaagaccgaggtgcagacaggcggcttcagcaaagagtctatcctgcccaagaggaacagcgacaagctgatcgccagaaagaaggactgggaccctaagaagtacggcggcttcgacagccccaccgtggcctattctgtgctggtggtggccaaagtggaaaagggcaagtccaagaaactgaagagtgtgaaagagctgctggggatcaccatcatggaaagaagcagcttcgagaagaatcccatcgactttctggaagccaagggctacaaagaagtgaaaaaggacctgatcatcaagctgcctaagtactccctgttcgagctggaaaacggccggaagagaatgctggcctctgccggcgaactgcagaagggaaacgaactggccctgccctccaaatatgtgaacttcctgtacctggccagccactatgagaagctgaagggctcccccgaggataatgagcagaaacagctgtttgtggaacagcacaaacactacctggacgagatcatcgagcagatcagcgagttctccaagagagtgatcctggccgacgctaatctggacaaggtgctgagcgcctacaacaagcacagagacaagcctatcagagagcaggccgagaatatcatccacctgtttaccctgaccaatctgggagcccctgccgccttcaagtactttgacaccaccatcgaccggaagaggtacaccagcaccaaagaggtgctggacgccaccctgatccaccagagcatcaccggcctgtacgagacacggatcgacctgtctcagctgggaggcgacgcctatccctatgacgtgcccgattatgccagcctgggcagcggctcccccaagaaaaaacgcaaggtggaagatcctaagaaaaagcggaaagtggacggcagcggcagcgagacccccggtaccagcgagagcgccacccccgagagccggacactggtgaccttcaaggatgtatttgtggacttcaccagggaggagtggaagctgctggacactgctcagcagatcgtgtacagaaatgtgatgctggagaactataagaacctggtttccttgggttatcagcttactaagccagatgtgatcctccggttggagaagggagaagagccctga

SEQ ID NO: 297 - DNA, 891 bp, synthetic construct
  misc_feature 1..891: note = CDS of V9_GFP1-10-KRAB
  source 1..891: mol_type = other DNA
atgcctgctgctaagagagtgaaactggatggatcctccaagggagaggagctgttcaccggagtggtgccaatcctggtggagctggacggcgatgtgaacggccacaagttttctgtgcgcggagagggagagggcgacgcaaccatcggcaagctgacactgaagttcatctgcaccacaggcaagctgcccgtgccttggccaaccctggtgaccacactgacatacggcgtgcagtgtttctctaggtatccagaccacatgaagagacacgatttctttaagagcgccatgccagagggatacgtgcaggagcggaccatctccttcaaggacgatggcaagtataagacccgcgccgtggtgaagtttgagggcgatacactggtgaacaggatcgagctgaagggcaccgacttcaaggaggatggcaatatcctgggccacaagctggagtacaactttaatagccacaacgtgtatatcacagccgacaagcagaagaacggcatcaaggccaacttcaccgtgaggcacaatgtggaggacggctccgtgcagctggccgatcactaccagcagaacacacctatcggcgacggacccgtgctgctgcctgataatcactatctgtccacccagacagtgctgtctaaggacccaaacgagaagttggatccaggtggaggtggaagcggtcggacactggtgaccttcaaggatgtatttgtggacttcaccagggaggagtggaagctgctggacactgctcagcagatcgtgtacagaaatgtgatgctggagaactataagaacctggtttccttgggttatcagcttactaagccagatgtgatcctccggttggagaagggagaagagccctga

SEQ ID NO: 298 - DNA, 6369 bp, synthetic construct
  misc_feature 1..6369: note = CDS of V10_D3a-D3l-dCas9-1xGFP11
  source 1..6369: mol_type = other DNA
atgcctgctgctaagagagtgaaactggatggatccaaccatgaccaggaatttgaccccccaaaggtttacccacctgtgccagctgagaagaggaagcccatccgcgtgctgtctctctttgatgggattgctacagggctcctggtgctgaaggacctgggcatccaagtggaccgctacattgcctccgaggtgtgtgaggactccatcacggtgggcatggtgcggcaccagggaaagatcatgtacgtcggggacgtccgcagcgtcacacagaagcatatccaggagtggggcccattcgacctggtgattggaggcagtccctgcaatgacctctccattgtcaaccctgcccgcaagggactttatgagggtactggccgcctcttctttgagttctaccgcctcctgcatgatgcgcggcccaaggagggagatgatcgccccttcttctggctctttgagaatgtggtggccatgggcgttagtgacaagagggacatctcgcgatttcttgagtctaaccccgtgatgattgacgccaaagaagtgtctgctgcacacagggcccgttacttctggggtaaccttcctggcatgaacaggcctttggcatccactgtgaatgataagctggagctgcaagagtgtctggagcacggcagaatagccaagttcagcaaagtgaggaccattaccaccaggtcaaactctataaagcagggcaaagaccagcatttccccgtgttcatgaacgagaaggaggacatcctgtggtgcactgaaatggaaagggtgtttggcttccccgtccactacacagacgtctccaacatgagccgcttggcgaggcagagactgctgggccgatcgtggagcgtgccggtcatccgccacctcttcgctccgctgaaggaatattttgcttgtgtgtctagcggcaatagtaacgctaacagccgcgggccgagcttcagcagcggcctggtgccgttaagcttgcgcggcagccatatgggccctatggagatatacaagacagtgtctgcatggaagagacagccagtgcgggtactgagcctcttcagaaacatcgacaaggtactaaagagtttgggcttcttggaaagcggttctggttctgggggaggaacgctgaagtacgtggaagatgtcacaaatgtcgtgaggagagacgtggagaaatggggcccctttgacctggtgtacggctcgacgcagcccctaggcagctcttgtgatcgctgtcccggctggtacatgttccagttccaccggatcctgcagtatgcgctgcctcgccaggagagtcagcggcccttcttctggatattcatggacaatctgctgctgactgaggatgaccaagagacaactacccgcttccttcagacagaggctgtgaccctccaggatgtccgtggcagagactaccagaatgctatgcgggtgtggagcaacattccagggctgaagagcaagcatgcgcccctgaccccaaaggaagaagagtatctgcaagcccaagtcagaagcaggagcaagctggacgccccgaaagttgacctcctggtgaagaactgccttctcccgctgagagagtacttcaagtatttttctcaaaactcacttcctcttggagggccgagctctggcgcacccccaccaagtggagggtctcctgccgggtccccaacatctactgaagaaggcaccagcgaatccgcaacgcccgagtcaggccctggtacctccacagaaccatctgaaggtagtgcgcctggttccccagctggaagccctacttccaccgaagaaggcacgtcaaccgaaccaagtgaaggatctgcccctgggaccagcactgaaccatctgagccaaaaaagaagagaaaggtaatggacaagaagtacagcatcggcctggccatcggcaccaactctgtgggctgggccgtgatcaccgacgagtacaaggtgcccagcaagaaattcaaggtgctgggcaacaccgaccggcacagcatcaagaagaacctgatcggcgccctgctgttcgacagcggagaaacagccgaggccacccggctgaagagaaccgccagaagaagatacaccagacggaagaaccggatctgctatctgcaagagatcttcagcaacgagatggccaaggtggacgacagcttcttccacagactggaagagtccttcctggtggaagaggataagaagcacgagcggcaccccatcttcggcaacatcgtggacgaggtggcctaccacgagaagtaccccaccatctaccacctgagaaagaaactggtggacagcaccgacaaggccgacctgcggctgatctatctggccctggcccacatgatcaagttccggggccacttcctgatcgagggcgacctgaaccccgacaacagcgacgtggacaagctgttcatccagctggtgcagacctacaaccagctgttcgaggaaaaccccatcaacgccagcggcgtggacgccaaggccatcctgtctgccagactgagcaagagcagacggctggaaaatctgatcgcccagctgcccggcgagaagaagaatggcctgttcggcaacctgattgccctgagcctgggcctgacccccaacttcaagagcaacttcgacctggccgaggatgccaaactgcagctgagcaaggacacctacgacgacgacctggacaacctgctggcccagatcggcgaccagtacgccgacctgtttctggccgccaagaacctgtccgacgccatcctgctgagcgacatcctgagagtgaacaccgagatcaccaaggcccccctgagcgcctctatgatcaagagatacgacgagcaccaccaggacctgaccctgctgaaagctctcgtgcggcagcagctgcctgagaagtacaaagagattttcttcgaccagagcaagaacggctacgccggctacatcgatggcggagccagccaggaagagttctacaagttcatcaagcccatcctggaaaagatggacggcaccgaggaactgctcgtgaagctgaacagagaggacctgctgcggaagcagcggaccttcgacaacggcagcatcccccaccagatccacctgggagagctgcacgccattctgcggcggcaggaagatttttacccattcctgaaggacaaccgggaaaagatcgagaagatcctgaccttccgcatcccctactacgtgggccctctggccaggggaaacagcagattcgcctggatgaccagaaagagcgaggaaaccatcaccccctggaacttcgaggaagtggtggacaagggcgccagcgcccagagcttcatcgagcggatgaccaacttcgataagaacctgcccaacgagaaggtgctgcccaagcacagcctgctgtacgagtacttcaccgtgtacaacgagctgaccaaagtgaaatacgtgaccgagggaatgagaaagcccgccttcctgagcggcgagcagaaaaaagccatcgtggacctgctgttcaagaccaaccggaaagtgaccgtgaagcagctgaaagaggactacttcaagaaaatcgagtgcttcgactccgtggaaatctccggcgtggaagatcggttcaacgcctccctgggcacataccacgatctgctgaaaattatcaaggacaaggacttcctggacaatgaggaaaacgaggacattctggaagatatcgtgctgaccctgacactgtttgaggacagagagatgatcgaggaacggctgaaaacctatgcccacctgttcgacgacaaagtgatgaagcagctgaagcggcggagatacaccggctggggcaggctgagccggaagctgatcaacggcatccgggacaagcagtccggcaagacaatcctggatttcctgaagtccgacggcttcgccaacagaaacttcatgcagctgatccacgacgacagcctgacctttaaagaggacatccagaaagcccaggtgtccggccagggcgatagcctgcacgagcacattgccaatctggccggcagccccgccattaagaagggcatcctgcagacagtgaaggtggtggacgagctcgtgaaagtgatgggccggcacaagcccgagaacatcgtgatcgaaatggccagagagaaccagaccacccagaagggacagaagaacagccgcgagagaatgaagcggatcgaagagggcatcaaagagctgggcagccagatcctgaaagaacaccccgtggaaaacacccagctgcagaacgagaagctgtacctgtactacctgcagaatgggcgggatatgtacgtggaccaggaactggacatcaaccggctgtccgactacgatgtggacgctatcgtgcctcagagctttctgaaggacgactccatcgataacaaagtgctgactcggagcgacaagaaccggggcaagagcgacaacgtgccctccgaagaggtcgtgaagaagatgaagaactactggcgccagctgctgaatgccaagctgattacccagaggaagttcgacaatctgaccaaggccgagagaggcggcctgagcgaactggataaggccggcttcatcaagagacagctggtggaaacccggcagatcacaaagcacgtggcacagatcctggactcccggatgaacactaagtacgacgagaacgacaaactgatccgggaagtgaaagtgatcaccctgaagtccaagctggtgtccgatttccggaaggatttccagttttacaaagtgcgcgagatcaacaactaccaccacgcccacgacgcctacctgaacgccgtcgtgggaaccgccctgatcaaaaagtaccctaagctggaaagcgagttcgtgtacggcgactacaaggtgtacgacgtgcggaagatgatcgccaagagcgagcaggaaatcggcaaggctaccgccaagtacttcttctacagcaacatcatgaactttttcaagaccgagattaccctggccaacggcgagatccggaagcggcctctgatcgagacaaacggcgaaacaggcgagatcgtgtgggataagggccgggactttgccaccgtgcggaaagtgctgtctatgccccaagtgaatatcgtgaaaaagaccgaggtgcagacaggcggcttcagcaaagagtctatcctgcccaagaggaacagcgacaagctgatcgccagaaagaaggactgggaccctaagaagtacggcggcttcgacagccccaccgtggcctattctgtgctggtggtggccaaagtggaaaagggcaagtccaagaaactgaagagtgtgaaagagctgctggggatcaccatcatggaaagaagcagcttcgagaagaatcccatcgactttctggaagccaagggctacaaagaagtgaaaaaggacctgatcatcaagctgcctaagtactccctgttcgagctggaaaacggccggaagagaatgctggcctctgccggcgaactgcagaagggaaacgaactggccctgccctccaaatatgtgaacttcctgtacctggccagccactatgagaagctgaagggctcccccgaggataatgagcagaaacagctgtttgtggaacagcacaaacactacctggacgagatcatcgagcagatcagcgagttctccaagagagtgatcctggccgacgctaatctggacaaggtgctgagcgcctacaacaagcacagagacaagcctatcagagagcaggccgagaatatcatccacctgtttaccctgaccaatctgggagcccctgccgccttcaagtactttgacaccaccatcgaccggaagaggtacaccagcaccaaagaggtgctggacgccaccctgatccaccagagcatcaccggcctgtacgagacacggatcgacctgtctcagctgggaggcgacgcctatccctatgacgtgcccgattatgccagcctgggcagcggctcccccaagaaaaaacgcaaggtggaagatcctaagaaaaagcggaaagtggacggcagcggcagcgagacccccggtaccagcgagagcgccacccccgagagcggtagtgggagcaacggcagcagcggatccatgcgtgaccacatggtccttcatgagtatgtaaatgctgctgggattacaggtggctctggaggtgcggccgcaaggtcaggctccggccagcggggaagcaagcgcaccgccgatggttccgagttcgaaagccccaaaaaaaagcgcaaggtctga

SEQ ID NO: 299 - DNA, 6732 bp, synthetic construct
  misc_feature 1..6732: note = CDS of V11_D3a-D3l-dCas9-8xGFP11
  source 1..6732: mol_type = other DNA
atgcctgctgctaagagagtgaaactggatggatccaaccatgaccaggaatttgaccccccaaaggtttacccacctgtgccagctgagaagaggaagcccatccgcgtgctgtctctctttgatgggattgctacagggctcctggtgctgaaggacctgggcatccaagtggaccgctacattgcctccgaggtgtgtgaggactccatcacggtgggcatggtgcggcaccagggaaagatcatgtacgtcggggacgtccgcagcgtcacacagaagcatatccaggagtggggcccattcgacctggtgattggaggcagtccctgcaatgacctctccattgtcaaccctgcccgcaagggactttatgagggtactggccgcctcttctttgagttctaccgcctcctgcatgatgcgcggcccaaggagggagatgatcgccccttcttctggctctttgagaatgtggtggccatgggcgttagtgacaagagggacatctcgcgatttcttgagtctaaccccgtgatgattgacgccaaagaagtgtctgctgcacacagggcccgttacttctggggtaaccttcctggcatgaacaggcctttggcatccactgtgaatgataagctggagctgcaagagtgtctggagcacggcagaatagccaagttcagcaaagtgaggaccattaccaccaggtcaaactctataaagcagggcaaagaccagcatttccccgtgttcatgaacgagaaggaggacatcctgtggtgcactgaaatggaaagggtgtttggcttccccgtccactacacagacgtctccaacatgagccgcttggcgaggcagagactgctgggccgatcgtggagcgtgccggtcatccgccacctcttcgctccgctgaaggaatattttgcttgtgtgtctagcggcaatagtaacgctaacagccgcgggccgagcttcagcagcggcctggtgccgttaagcttgcgcggcagccatatgggccctatggagatatacaagacagtgtctgcatggaagagacagccagtgcgggtactgagcctcttcagaaacatcgacaaggtactaaagagtttgggcttcttggaaagcggttctggttctgggggaggaacgctgaagtacgtggaagatgtcacaaatgtcgtgaggagagacgtggagaaatggggcccctttgacctggtgtacggctcgacgcagcccctaggcagctcttgtgatcgctgtcccggctggtacatgttccagttccaccggatcctgcagtatgcgctgcctcgccaggagagtcagcggcccttcttctggatattcatggacaatctgctgctgactgaggatgaccaagagacaactacccgcttccttcagacagaggctgtgaccctccaggatgtccgtggcagagactaccagaatgctatgcgggtgtggagcaacattccagggctgaagagcaagcatgcgcccctgaccccaaaggaagaagagtatctgcaagcccaagtcagaagcaggagcaagctggacgccccgaaagttgacctcctggtgaagaactgccttctcccgctgagagagtacttcaagtatttttctcaaaactcacttcctcttggagggccgagctctggcgcacccccaccaagtggagggtctcctgccgggtccccaacatctactgaagaaggcaccagcgaatccgcaacgcccgagtcaggccctggtacctccacagaaccatctgaaggtagtgcgcctggttccccagctggaagccctacttccaccgaagaaggcacgtcaaccgaaccaagtgaaggatctgcccctgggaccagcactgaaccatctgagccaaaaaagaagagaaaggtaatggacaagaagtacagcatcggcctggccatcggcaccaactctgtgggctgggccgtgatcaccgacgagtacaaggtgcccagcaagaaattcaaggtgctgggcaacaccgaccggcacagcatcaagaagaacctgatcggcgccctgctgttcgacagcggagaaacagccgaggccacccggctgaagagaaccgccagaagaagatacaccagacggaagaaccggatctgctatctgcaagagatcttcagcaacgagatggccaaggtggacgacagcttcttccacagactggaagagtccttcctggtggaagaggataagaagcacgagcggcaccccatcttcggcaacatcgtggacgaggtggcctaccacgagaagtaccccaccatctaccacctgagaaagaaactggtggacagcaccgacaaggccgacctgcggctgatctatctggccctggcccacatgatcaagttccggggccacttcctgatcgagggcgacctgaaccccgacaacagcgacgtggacaagctgttcatccagctggtgcagacctacaaccagctgttcgaggaaaaccccatcaacgccagcggcgtggacgccaaggccatcctgtctgccagactgagcaagagcagacggctggaaaatctgatcgcccagctgcccggcgagaagaagaatggcctgttcggcaacctgattgccctgagcctgggcctgacccccaacttcaagagcaacttcgacctggccgaggatgccaaactgcagctgagcaaggacacctacgacgacgacctggacaacctgctggcccagatcggcgaccagtacgccgacctgtttctggccgccaagaacctgtccgacgccatcctgctgagcgacatcctgagagtgaacaccgagatcaccaaggcccccctgagcgcctctatgatcaagagatacgacgagcaccaccaggacctgaccctgctgaaagctctcgtgcggcagcagctgcctgagaagtacaaagagattttcttcgaccagagcaagaacggctacgccggctacatcgatggcggagccagccaggaagagttctacaagttcatcaagcccatcctggaaaagatggacggcaccgaggaactgctcgtgaagctgaacagagaggacctgctgcggaagcagcggaccttcgacaacggcagcatcccccaccagatccacctgggagagctgcacgccattctgcggcggcaggaagatttttacccattcctgaaggacaaccgggaaaagatcgagaagatcctgaccttccgcatcccctactacgtgggccctctggccaggggaaacagcagattcgcctggatgaccagaaagagcgaggaaaccatcaccccctggaacttcgaggaagtggtggacaagggcgccagcgcccagagcttcatcgagcggatgaccaacttcgataagaacctgcccaacgagaaggtgctgcccaagcacagcctgctgtacgagtacttcaccgtgtacaacgagctgaccaaagtgaaatacgtgaccgagggaatgagaaagcccgccttcctgagcggcgagcagaaaaaagccatcgtggacctgctgttcaagaccaaccggaaagtgaccgtgaagcagctgaaagaggactacttcaagaaaatcgagtgcttcgactccgtggaaatctccggcgtggaagatcggttcaacgcctccctgggcacataccacgatctgctgaaaattatcaaggacaaggacttcctggacaatgaggaaaacgaggacattctggaagatatcgtgctgaccctgacactgtttgaggacagagagatgatcgaggaacggctgaaaacctatgcccacctgttcgacgacaaagtgatgaagcagctgaagcggcggagatacaccggctggggcaggctgagccggaagctgatcaacggcatccgggacaagcagtccggcaagacaatcctggatttcctgaagtccgacggcttcgccaacagaaacttcatgcagctgatccacgacgacagcctgacctttaaagaggacatccagaaagcccaggtgtccggccagggcgatagcctgcacgagcacattgccaatctggccggcagccccgccattaagaagggcatcctgcagacagtgaaggtggtggacgagctcgtgaaagtgatgggccggcacaagcccgagaacatcgtgatcgaaatggccagagagaaccagaccacccagaagggacagaagaacagccgcgagagaatgaagcggatcgaagagggcatcaaagagctgggcagccagatcctgaaagaacaccccgtggaaaacacccagctgcagaacgagaagctgtacctgtactacctgcagaatgggcgggatatgtacgtggaccaggaactggacatcaaccggctgtccgactacgatgtggacgctatcgtgcctcagagctttctgaaggacgactccatcgataacaaagtgctgactcggagcgacaagaaccggggcaagagcgacaacgtgccctccgaagaggtcgtgaagaagatgaagaactactggcgccagctgctgaatgccaagctgattacccagaggaagttcgacaatctgaccaaggccgagagaggcggcctgagcgaactggataaggccggcttcatcaagagacagctggtggaaacccggcagatcacaaagcacgtggcacagatcctggactcccggatgaacactaagtacgacgagaacgacaaactgatccgggaagtgaaagtgatcaccctgaagtccaagctggtgtccgatttccggaaggatttccagttttacaaagtgcgcgagatcaacaactaccaccacgcccacgacgcctacctgaacgccgtcgtgggaaccgccctgatcaaaaagtaccctaagctggaaagcgagttcgtgtacggcgactacaaggtgtacgacgtgcggaagatgatcgccaagagcgagcaggaaatcggcaaggctaccgccaagtacttcttctacagcaacatcatgaactttttcaagaccgagattaccctggccaacggcgagatccggaagcggcctctgatcgagacaaacggcgaaacaggcgagatcgtgtgggataagggccgggactttgccaccgtgcggaaagtgctgtctatgccccaagtgaatatcgtgaaaaagaccgaggtgcagacaggcggcttcagcaaagagtctatcctgcccaagaggaacagcgacaagctgatcgccagaaagaaggactgggaccctaagaagtacggcggcttcgacagccccaccgtggcctattctgtgctggtggtggccaaagtggaaaagggcaagtccaagaaactgaagagtgtgaaagagctgctggggatcaccatcatggaaagaagcagcttcgagaagaatcccatcgactttctggaagccaagggctacaaagaagtgaaaaaggacctgatcatcaagctgcctaagtactccctgttcgagctggaaaacggccggaagagaatgctggcctctgccggcgaactgcagaagggaaacgaactggccctgccctccaaatatgtgaacttcctgtacctggccagccactatgagaagctgaagggctcccccgaggataatgagcagaaacagctgtttgtggaacagcacaaacactacctggacgagatcatcgagcagatcagcgagttctccaagagagtgatcctggccgacgctaatctggacaaggtgctgagcgcctacaacaagcacagagacaagcctatcagagagcaggccgagaatatcatccacctgtttaccctgaccaatctgggagcccctgccgccttcaagtactttgacaccaccatcgaccggaagaggtacaccagcaccaaagaggtgctggacgccaccctgatccaccagagcatcaccggcctgtacgagacacggatcgacctgtctcagctgggaggcgacgcctatccctatgacgtgcccgattatgccagcctgggcagcggctcccccaagaaaaaacgcaaggtggaagatcctaagaaaaagcggaaagtggacggcagcggcagcgagacccccggtaccagcgagagcgccacccccgagagcggtagtgggagcaacggcagcagcggatccatgcgtgaccacatggtccttcatgagtatgtaaatgctgctgggattacaggtggctctggaggtagagatcatatggttctccacgaatacgttaacgccgcaggcatcactggcggtagtggaggacgcgaccatatggtactacatgaatatgtcaatgcagccggaataaccggagggtccggaggccgggatcacatggtgctgcatgagtatgtgaacgcggcgggtataactggtgggtcgggcggacgagaccatatggtgcttcacgaatacgtaaacgcagctggcattactggcggatcaggtggcagggatcacatggtactccatgagtacgtgaacgctgctggaatcacaggcggtagcggcggtcgggaccatatggtcctgcacgaatatgtcaatgctgccggtatcaccgcggccgcaaggtcaggctccggccagcggggaagcaagcgcaccgccgatggttccgagttcgaaagccccaaaaaaaagcgcaaggtctga

SEQ ID NO: 300 - DNA, 7551 bp, synthetic construct
  misc_feature 1..7551: note = CDS of V12_scFv-KRAB-2a-D3a-D3l-dCas9-1xGCN4
  source 1..7551: mol_type = other DNA
atgggccccgacatcgtgatgacccagagccccagcagcctgagcgccagcgtgggcgaccgcgtgaccatcacctgccgcagcagcaccggcgccgtgaccaccagcaactacgccagctgggtgcaggagaagcccggcaagctgttcaagggcctgatcggcggcaccaacaaccgcgcccccggcgtgcccagccgcttcagcggcagcctgatcggcgacaaggccaccctgaccatcagcagcctgcagcccgaggacttcgccacctacttctgcgccctgtggtacagcaaccactgggtgttcggccagggcaccaaggtggagctgaagcgcggcggcggcggcagcggcggcggcggcagcggcggcggcggcagcagcggcggcggcagcgaggtgaagctgctggagagcggcggcggcctggtgcagcccggcggcagcctgaagctgagctgcgccgtgagcggcttcagcctgaccgactacggcgtgaactgggtgcgccaggcccccggccgcggcctggagtggatcggcgtgatctggggcgacggcatcaccgactacaacagcgccctgaaggaccgcttcatcatcagcaaggacaacggcaagaacaccgtgtacctgcagatgagcaaggtgcgcagcgacgacaccgccctgtactactgcgtgaccggcctgttcgactactggggccagggcaccctggtgaccgtgagcagctacccatacgatgttccagattacgctggtggaggcggaggttctgggggaggaggtagtggcggtggtggttcaggaggcggcggaagcttggatccaggtggaggtggaagcggtcggacactggtgaccttcaaggatgtatttgtggacttcaccagggaggagtggaagctgctggacactgctcagcagatcgtgtacagaaatgtgatgctggagaactataagaacctggtttccttgggttatcagcttactaagccagatgtgatcctccggttggagaagggagaagagcccggaagcggaaagcgcaccgccgatggttccgagttcgaaagccccaaaaaaaagcgcaaggtcggaagcggagctactaacttcagcctgctgaagcaggctggagacgtggaggagaaccctggacctatgaaccatgaccaggaatttgaccccccaaaggtttacccacctgtgccagctgagaagaggaagcccatccgcgtgctgtctctctttgatgggattgctacagggctcctggtgctgaaggacctgggcatccaagtggaccgctacattgcctccgaggtgtgtgaggactccatcacggtgggcatggtgcggcaccagggaaagatcatgtacgtcggggacgtccgcagcgtcacacagaagcatatccaggagtggggcccattcgacctggtgattggaggcagtccctgcaatgacctctccattgtcaaccctgcccgcaagggactttatgagggtactggccgcctcttctttgagttctaccgcctcctgcatgatgcgcggcccaaggagggagatgatcgccccttcttctggctctttgagaatgtggtggccatgggcgttagtgacaagagggacatctcgcgatttcttgagtctaaccccgtgatgattgacgccaaagaagtgtctgctgcacacagggcccgttacttctggggtaaccttcctggcatgaacaggcctttggcatccactgtgaatgataagctggagctgcaagagtgtctggagcacggcagaatagccaagttcagcaaagtgaggaccattaccaccaggtcaaactctataaagcagggcaaagaccagcatttccccgtcttcatgaacgagaaggaggacatcctgtggtgcactgaaatggaaagggtgtttggcttccccgtccactacacagacgtctccaacatgagccgcttggcgaggcagagactgctgggccgatcgtggagcgtgccggtcatccgccacctcttcgctccgctgaaggaatattttgcttgtgtgtctagcggcaatagtaacgctaacagccgcgggccgagcttcagcagcggcctggtgccgttaagcttgcgcggcagccatatgggccctatggagatatacaagacagtgtctgcatggaagagacagccagtgcgggtactgagcctcttcagaaacatcgacaaggtactaaagagtttgggcttcttggaaagcggttctggttctgggggaggaacgctgaagtacgtggaagatgtcacaaatgtcgtgaggagagacgtggagaaatggggcccctttgacctggtgtacggctcgacgcagcccctaggcagctcttgtgatcgctgtcccggctggtacatgttccagttccaccggatcctgcagtatgcgctgcctcgccaggagagtcagcggcccttcttctggatattcatggacaatctgctgctgactgaggatgaccaagagacaactacccgcttccttcagacagaggctgtgaccctccaggatgtccgtggcagagactaccagaatgctatgcgggtgtggagcaacattccagggctgaagagcaagcatgcgcccctgaccccaaaggaagaagagtatctgcaagcccaagtcagaagcaggagcaagctggacgccccgaaagttgacctcctggtgaagaactgccttctcccgctgagagagtacttcaagtatttttctcaaaactcacttcctcttggagggccgagctctggcgcacccccaccaagtggagggtctcctgccgggtccccaacatctactgaagaaggcaccagcgaatccgcaacgcccgagtcaggccctggtacctccacagaaccatctgaaggtagtgcgcctggttccccagctggaagccctacttccaccgaagaaggcacgtcaaccgaaccaagtgaaggatctgcccctgggaccagcactgaaccatctgagccaaaaaagaagagaaaggtaatggacaagaagtacagcatcggcctggccatcggcaccaactctgtgggctgggccgtgatcaccgacgagtacaaggtgcccagcaagaaattcaaggtgctgggcaacaccgaccggcacagcatcaagaagaacctgatcggcgccctgctgttcgacagcggagaaacagccgaggccacccggctgaagagaaccgccagaagaagatacaccagacggaagaaccggatctgctatctgcaagagatcttcagcaacgagatggccaaggtggacgacagcttcttccacagactggaagagtccttcctggtggaagaggataagaagcacgagcggcaccccatcttcggcaacatcgtggacgaggtggcctaccacgagaagtaccccaccatctaccacctgagaaagaaactggtggacagcaccgacaaggccgacctgcggctgatctatctggccctggcccacatgatcaagttccggggccacttcctgatcgagggcgacctgaaccccgacaacagcgacgtggacaagctgttcatccagctggtgcagacctacaaccagctgttcgaggaaaaccccatcaacgccagcggcgtggacgccaaggccatcctgtctgccagactgagcaagagcagacggctggaaaatctgatcgcccagctgcccggcgagaagaagaatggcctgttcggcaacctgattgccctgagcctgggcctgacccccaacttcaagagcaacttcgacctggccgaggatgccaaactgcagctgagcaaggacacctacgacgacgacctggacaacctgctggcccagatcggcgaccagtacgccgacctgtttctggccgccaagaacctgtccgacgccatcctgctgagcgacatcctgagagtgaacaccgagatcaccaaggcccccctgagcgcctctatgatcaagagatacgacgagcaccaccaggacctgaccctgctgaaagctctcgtgcggcagcagctgcctgagaagtacaaagagattttcttcgaccagagcaagaacggctacgccggctacatcgatggcggagccagccaggaagagttctacaagttcatcaagcccatcctggaaaagatggacggcaccgaggaactgctcgtgaagctgaacagagaggacctgctgcggaagcagcggaccttcgacaacggcagcatcccccaccagatccacctgggagagctgcacgccattctgcggcggcaggaagatttttacccattcctgaaggacaaccgggaaaagatcgagaagatcctgaccttccgcatcccctactacgtgggccctctggccaggggaaacagcagattcgcctggatgaccagaaagagcgaggaaaccatcaccccctggaacttcgaggaagtggtggacaagggcgccagcgcccagagcttcatcgagcggatgaccaacttcgataagaacctgcccaacgagaaggtgctgcccaagcacagcctgctgtacgagtacttcaccgtgtacaacgagctgaccaaagtgaaatacgtgaccgagggaatgagaaagcccgccttcctgagcggcgagcagaaaaaagccatcgtggacctgctgttcaagaccaaccggaaagtgaccgtgaagcagctgaaagaggactacttcaagaaaatcgagtgcttcgactccgtggaaatctccggcgtggaagatcggttcaacgcctccctgggcacataccacgatctgctgaaaattatcaaggacaaggacttcctggacaatgaggaaaacgaggacattctggaagatatcgtgctgaccctgacactgtttgaggacagagagatgatcgaggaacggctgaaaacctatgcccacctgttcgacgacaaagtgatgaagcagctgaagcggcggagatacaccggctggggcaggctgagccggaagctgatcaacggcatccgggacaagcagtccggcaagacaatcctggatttcctgaagtccgacggcttcgccaacagaaacttcatgcagctgatccacgacgacagcctgacctttaaagaggacatccagaaagcccaggtgtccggccagggcgatagcctgcacgagcacattgccaatctggccggcagccccgccattaagaagggcatcctgcagacagtgaaggtggtggacgagctcgtgaaagtgatgggccggcacaagcccgagaacatcgtgatcgaaatggccagagagaaccagaccacccagaagggacagaagaacagccgcgagagaatgaagcggatcgaagagggcatcaaagagctgggcagccagatcctgaaagaacaccccgtggaaaacacccagctgcagaacgagaagctgtacctgtactacctgcagaatgggcgggatatgtacgtggaccaggaactggacatcaaccggctgtccgactacgatgtggacgctatcgtgcctcagagctttctgaaggacgactccatcgataacaaagtgctgactcggagcgacaagaaccggggcaagagcgacaacgtgccctccgaagaggtcgtgaagaagatgaagaactactggcgccagctgctgaatgccaagctgattacccagaggaagttcgacaatctgaccaaggccgagagaggcggcctgagcgaactggataaggccggcttcatcaagagacagctggtggaaacccggcagatcacaaagcacgtggcacagatcctggactcccggatgaacactaagtacgacgagaacgacaaactgatccgggaagtgaaagtgatcaccctgaagtccaagctggtgtccgatttccggaaggatttccagttttacaaagtgcgcgagatcaacaactaccaccacgcccacgacgcctacctgaacgccgtcgtgggaaccgccctgatcaaaaagtaccctaagctggaaagcgagttcgtgtacggcgactacaaggtgtacgacgtgcggaagatgatcgccaagagcgagcaggaaatcggcaaggctaccgccaagtacttcttctacagcaacatcatgaactttttcaagaccgagattaccctggccaacggcgagatccggaagcggcctctgatcgagacaaacggcgaaacaggcgagatcgtgtgggataagggccgggactttgccaccgtgcggaaagtgctgtctatgccccaagtgaatatcgtgaaaaagaccgaggtgcagacaggcggcttcagcaaagagtctatcctgcccaagaggaacagcgacaagctgatcgccagaaagaaggactgggaccctaagaagtacggcggcttcgacagccccaccgtggcctattctgtgctggtggtggccaaagtggaaaagggcaagtccaagaaactgaagagtgtgaaagagctgctggggatcaccatcatggaaagaagcagcttcgagaagaatcccatcgactttctggaagccaagggctacaaagaagtgaaaaaggacctgatcatcaagctgcctaagtactccctgttcgagctggaaaacggccggaagagaatgctggcctctgccggcgaactgcagaagggaaacgaactggccctgccctccaaatatgtgaacttcctgtacctggccagccactatgagaagctgaagggctcccccgaggataatgagcagaaacagctgtttgtggaacagcacaaacactacctggacgagatcatcgagcagatcagcgagttctccaagagagtgatcctggccgacgctaatctggacaaggtgctgagcgcctacaacaagcacagagacaagcctatcagagagcaggccgagaatatcatccacctgtttaccctgaccaatctgggagcccctgccgccttcaagtactttgacaccaccatcgaccggaagaggtacaccagcaccaaagaggtgctggacgccaccctgatccaccagagcatcaccggcctgtacgagacacggatcgacctgtctcagctgggaggcgacgcctatccctatgacgtgcccgattatgccagcctgggcagcggctcccccaagaaaaaacgcaaggtggaagatcctaagaaaaagcggaaagtggacggcattggtagtgggagcaacggcagcagcggagaggaactgctgagcaagaactaccacctggaaaacgaggtggccagactgaagaaaggctctggctctggcggaagcggttctggcggatcaggatctggaagtggcggctctggaagcggaggttctggatctggcgaagaactgctgtctaagaattatcacggttcaggctccggccagcggggaagcaagcgcaccgccgatggttccgagttcgaaagccccaaaaaaaagcgcaaggtctga

SEQ ID NO: 301 - DNA, 7581 bp, synthetic construct
  misc_feature 1..7581: note = CDS of V13_scFv-KRAB-2a-D3a-D3l-dCas9-2xGCN4
  source 1..7581: mol_type = other DNA
atgggccccgacatcgtgatgacccagagccccagcagcctgagcgccagcgtgggcgaccgcgtgaccatcacctgccgcagcagcaccggcgccgtgaccaccagcaactacgccagctgggtgcaggagaagcccggcaagctgttcaagggcctgatcggcggcaccaacaaccgcgcccccggcgtgcccagccgcttcagcggcagcctgatcggcgacaaggccaccctgaccatcagcagcctgcagcccgaggacttcgccacctacttctgcgccctgtggtacagcaaccactgggtgttcggccagggcaccaaggtggagctgaagcgcggcggcggcggcagcggcggcggcggcagcggcggcggcggcagcagcggcggcggcagcgaggtgaagctgctggagagcggcggcggcctggtgcagcccggcggcagcctgaagctgagctgcgccgtgagcggcttcagcctgaccgactacggcgtgaactgggtgcgccaggcccccggccgcggcctggagtggatcggcgtgatctggggcgacggcatcaccgactacaacagcgccctgaaggaccgcttcatcatcagcaaggacaacggcaagaacaccgtgtacctgcagatgagcaaggtgcgcagcgacgacaccgccctgtactactgcgtgaccggcctgttcgactactggggccagggcaccctggtgaccgtgagcagctacccatacgatgttccagattacgctggtggaggcggaggttctgggggaggaggtagtggcggtggtggttcaggaggcggcggaagcttggatccaggtggaggtggaagcggtcggacactggtgaccttcaaggatgtatttgtggacttcaccagggaggagtggaagctgctggacactgctcagcagatcgtgtacagaaatgtgatgctggagaactataagaacctggtttccttgggttatcagcttactaagccagatgtgatcctccggttggagaagggagaagagcccggaagcggaaagcgcaccgccgatggttccgagttcgaaagccccaaaaaaaagcgcaaggtcggaagcggagctactaacttcagcctgctgaagcaggctggagacgtggaggagaaccctggacctatgaaccatgaccaggaatttgaccccccaaaggtttacccacctgtgccagctgagaagaggaagcccatccgcgtgctgtctctctttgatgggattgctacagggctcctggtgctgaaggacctgggcatccaagtggaccgctacattgcctccgaggtgtgtgaggactccatcacggtgggcatggtgcggcaccagggaaagatcatgtacgtcggggacgtccgcagcgtcacacagaagcatatccaggagtggggcccattcgacctggtgattggaggcagtccctgcaatgacctctccattgtcaaccctgcccgcaagggactttatgagggtactggccgcctcttctttgagttctaccgcctcctgcatgatgcgcggcccaaggagggagatgatcgccccttcttctggctctttgagaatgtggtggccatgggcgttagtgacaagagggacatctcgcgatttcttgagtctaaccccgtgatgattgacgccaaagaagtgtctgctgcacacagggcccgttacttctggggtaaccttcctggcatgaacaggcctttggcatccactgtgaatgataagctggagctgcaagagtgtctggagcacggcagaatagccaagttcagcaaagtgaggaccattaccaccaggtcaaactctataaagcagggcaaagaccagcatttccccgtcttcatgaacgagaaggaggacatcctgtggtgcactgaaatggaaagggtgtttggcttccccgtccactacacagacgtctccaacatgagccgcttggcgaggcagagactgctgggccgatcgtggagcgtgccggtcatccgccacctcttcgctccgctgaaggaatattttgcttgtgtgtctagcggcaatagtaacgctaacagccgcgggccgagcttcagcagcggcctggtgccgttaagcttgcgcggcagccatatgggccctatggagatatacaagacagtgtctgcatggaagagacagccagtgcgggtactgagcctcttcagaaacatcgacaaggtactaaagagtttgggcttcttggaaagcggttctggttctgggggaggaacgctgaagtacgtggaagatgtcacaaatgtcgtgaggagagacgtggagaaatggggcccctttgacctggtgtacggctcgacgcagcccctaggcagctcttgtgatcgctgtcccggctggtacatgttccagttccaccggatcctgcagtatgcgctgcctcgccaggagagtcagcggcccttcttctggatattcatggacaatctgctgctgactgaggatgaccaagagacaactacccgcttccttcagacagaggctgtgaccctccaggatgtccgtggcagagactaccagaatgctatgcgggtgtggagcaacattccagggctgaagagcaagcatgcgcccctgaccccaaaggaagaagagtatctgcaagcccaagtcagaagcaggagcaagctggacgccccgaaagttgacctcctggtgaagaactgccttctcccgctgagagagtacttcaagtatttttctcaaaactcacttcctcttggagggccgagctctggcgcacccccaccaagtggagggtctcctgccgggtccccaacatctactgaagaaggcaccagcgaatccgcaacgcccgagtcaggccctggtacctccacagaaccatctgaaggtagtgcgcctggttccccagctggaagccctacttccaccgaagaaggcacgtcaaccgaaccaagtgaaggatctgcccctgggaccagcactgaaccatctgagccaaaaaagaagagaaaggtaatggacaagaagtacagcatcggcctggccatcggcaccaactctgtgggctgggccgtgatcaccgacgagtacaaggtgcccagcaagaaattcaaggtgctgggcaacaccgaccggcacagcatcaagaagaacctgatcggcgccctgctgttcgacagcggagaaacagccgaggccacccggctgaagagaaccgccagaagaagatacaccagacggaagaaccggatctgctatctgcaagagatcttcagcaacgagatggccaaggtggacgacagcttcttccacagactggaagagtccttcctggtggaagaggataagaagcacgagcggcaccccatcttcggcaacatcgtggacgaggtggcctaccacgagaagtaccccaccatctaccacctgagaaagaaactggtggacagcaccgacaaggccgacctgcggctgatctatctggccctggcccacatgatcaagttccggggccacttcctgatcgagggcgacctgaaccccgacaacagcgacgtggacaagctgttcatccagctggtgcagacctacaaccagctgttcgaggaaaaccccatcaacgccagcggcgtggacgccaaggccatcctgtctgccagactgagcaagagcagacggctggaaaatctgatcgcccagctgcccggcgagaagaagaatggcctgttcggcaacctgattgccctgagcctgggcctgacccccaacttcaagagcaacttcgacctggccgaggatgccaaactgcagctgagcaaggacacctacgacgacgacctggacaacctgctggcccagatcggcgaccagtacgccgacctgtttctggccgccaagaacctgtccgacgccatcctgctgagcgacatcctgagagtgaacaccgagatcaccaaggcccccctgagcgcctctatgatcaagagatacgacgagcaccaccaggacctgaccctgctgaaagctctcgtgcggcagcagctgcctgagaagtacaaagagattttcttcgaccagagcaagaacggctacgccggctacatcgatggcggagccagccaggaagagttctacaagttcatcaagcccatcctggaaaagatggacggcaccgaggaactgctcgtgaagctgaacagagaggacctgctgcggaagcagcggaccttcgacaacggcagcatcccccaccagatccacctgggagagctgcacgccattctgcggcggcaggaagatttttacccattcctgaaggacaaccgggaaaagatcgagaagatcctgaccttccgcatcccctactacgtgggccctctggccaggggaaacagcagattcgcctggatgaccagaaagagcgaggaaaccatcaccccctggaacttcgaggaagtggtggacaagggcgccagcgcccagagcttcatcgagcggatgaccaacttcgataagaacctgcccaacgagaaggtgctgcccaagcacagcctgctgtacgagtacttcaccgtgtacaacgagctgaccaaagtgaaatacgtgaccgagggaatgagaaagcccgccttcctgagcggcgagcagaaaaaagccatcgtggacctgctgttcaagaccaaccggaaagtgaccgtgaagcagctgaaagaggactacttcaagaaaatcgagtgcttcgactccgtggaaatctccggcgtggaagatcggttcaacgcctccctgggcacataccacgatctgctgaaaattatcaaggacaaggacttcctggacaatgaggaaaacgaggacattctggaagatatcgtgctgaccctgacactgtttgaggacagagagatgatcgaggaacggctgaaaacctatgcccacctgttcgacgacaaagtgatgaagcagctgaagcggcggagatacaccggctggggcaggctgagccggaagctgatcaacggcatccgggacaagcagtccggcaagacaatcctggatttcctgaagtccgacggcttcgccaacagaaacttcatgcagctgatccacgacgacagcctgacctttaaagaggacatccagaaagcccaggtgtccggccagggcgatagcctgcacgagcacattgccaatctggccggcagccccgccattaagaagggcatcctgcagacagtgaaggtggtggacgagctcgtgaaagtgatgggccggcacaagcccgagaacatcgtgatcgaaatggccagagagaaccagaccacccagaagggacagaagaacagccgcgagagaatgaagcggatcgaagagggcatcaaagagctgggcagccagatcctgaaagaacaccccgtggaaaacacccagctgcagaacgagaagctgtacctgtactacctgcagaatgggcgggatatgtacgtggaccaggaactggacatcaaccggctgtccgactacgatgtggacgctatcgtgcctcagagctttctgaaggacgactccatcgataacaaagtgctgactcggagcgacaagaaccggggcaagagcgacaacgtgccctccgaagaggtcgtgaagaagatgaagaactactggcgccagctgctgaatgccaagctgattacccagaggaagttcgacaatctgaccaaggccgagagaggcggcctgagcgaactggataaggccggcttcatcaagagacagctggtggaaacccggcagatcacaaagcacgtggcacagatcctggactcccggatgaacactaagtacgacgagaacgacaaactgatccgggaagtgaaagtgatcaccctgaagtccaagctggtgtccgatttccggaaggatttccagttttacaaagtgcgcgagatcaacaactaccaccacgcccacgacgcctacctgaacgccgtcgtgggaaccgccctgatcaaaaagtaccctaagctggaaagcgagttcgtgtacggcgactacaaggtgtacgacgtgcggaagatgatcgccaagagcgagcaggaaatcggcaaggctaccgccaagtacttcttctacagcaacatcatgaactttttcaagaccgagattaccctggccaacggcgagatccggaagcggcctctgatcgagacaaacggcgaaacaggcgagatcgtgtgggataagggccgggactttgccaccgtgcggaaagtgctgtctatgccccaagtgaatatcgtgaaaaagaccgaggtgcagacaggcggcttcagcaaagagtctatcctgcccaagaggaacagcgacaagctgatcgccagaaagaaggactgggaccctaagaagtacggcggcttcgacagccccaccgtggcctattctgtgctggtggtggccaaagtggaaaagggcaagtccaagaaactgaagagtgtgaaagagctgctggggatcaccatcatggaaagaagcagcttcgagaagaatcccatcgactttctggaagccaagggctacaaagaagtgaaaaaggacctgatcatcaagctgcctaagtactccctgttcgagctggaaaacggccggaagagaatgctggcctctgccggcgaactgcagaagggaaacgaactggccctgccctccaaatatgtgaacttcctgtacctggccagccactatgagaagctgaagggctcccccgaggataatgagcagaaacagctgtttgtggaacagcacaaacactacctggacgagatcatcgagcagatcagcgagttctccaagagagtgatcctggccgacgctaatctggacaaggtgctgagcgcctacaacaagcacagagacaagcctatcagagagcaggccgagaatatcatccacctgtttaccctgaccaatctgggagcccctgccgccttcaagtactttgacaccaccatcgaccggaagaggtacaccagcaccaaagaggtgctggacgccaccctgatccaccagagcatcaccggcctgtacgagacacggatcgacctgtctcagctgggaggcgacgcctatccctatgacgtgcccgattatgccagcctgggcagcggctcccccaagaaaaaacgcaaggtggaagatcctaagaaaaagcggaaagtggacggcattggtagtgggagcaacggcagcagcggagaggaactgctgagcaagaactaccacctggaaaacgaggtggccagactgaagaaaggctctggctctggcggaagcggttctggcggatcaggatctggaagtggcggctctggaagcggaggttctggatctggcgaagaactgctgtctaagaattatcacctcgagaatgaagtcgctcgtttgaagaaaggttcaggctccggccagcggggaagcaagcgcaccgccgatggttccgagttcgaaagccccaaaaaaaagcgcaaggtctga

SEQ ID NO: 302 - DNA, 8685 bp, synthetic construct
  misc_feature 1..8685: note = CDS of V14-scFv-KRAB-2a-D3a-D3l-dCas9-10xGCN4
  source 1..8685: mol_type = other DNA
atgggccccgacatcgtgatgacccagagccccagcagcctgagcgccagcgtgggcgaccgcgtgaccatcacctgccgcagcagcaccggcgccgtgaccaccagcaactacgccagctgggtgcaggagaagcccggcaagctgttcaagggcctgatcggcggcaccaacaaccgcgcccccggcgtgcccagccgcttcagcggcagcctgatcggcgacaaggccaccctgaccatcagcagcctgcagcccgaggacttcgccacctacttctgcgccctgtggtacagcaaccactgggtgttcggccagggcaccaaggtggagctgaagcgcggcggcggcggcagcggcggcggcggcagcggcggcggcggcagcagcggcggcggcagcgaggtgaagctgctggagagcggcggcggcctggtgcagcccggcggcagcctgaagctgagctgcgccgtgagcggcttcagcctgaccgactacggcgtgaactgggtgcgccaggcccccggccgcggcctggagtggatcggcgtgatctggggcgacggcatcaccgactacaacagcgccctgaaggaccgcttcatcatcagcaaggacaacggcaagaacaccgtgtacctgcagatgagcaaggtgcgcagcgacgacaccgccctgtactactgcgtgaccggcctgttcgactactggggccagggcaccctggtgaccgtgagcagctacccatacgatgttccagattacgctggtggaggcggaggttctgggggaggaggtagtggcggtggtggttcaggaggcggcggaagcttggatccaggtggaggtggaagcggtcggacactggtgaccttcaaggatgtatttgtggacttcaccagggaggagtggaagctgctggacactgctcagcagatcgtgtacagaaatgtgatgctggagaactataagaacctggtttccttgggttatcagcttactaagccagatgtgatcctccggttggagaagggagaagagcccggaagcggaaagcgcaccgccgatggttccgagttcgaaagccccaaaaaaaagcgcaaggtcggaagcggagctactaacttcagcctgctgaagcaggctggagacgtggaggagaaccctggacctatgaaccatgaccaggaatttgaccccccaaaggtttacccacctgtgccagctgagaagaggaagcccatccgcgtgctgtctctctttgatgggattgctacagggctcctggtgctgaaggacctgggcatccaagtggaccgctacattgcctccgaggtgtgtgaggactccatcacggtgggcatggtgcggcaccagggaaagatcatgtacgtcggggacgtccgcagcgtcacacagaagcatatccaggagtggggcccattcgacctggtgattggaggcagtccctgcaatgacctctccattgtcaaccctgcccgcaagggactttatgagggtactggccgcctcttctttgagttctaccgcctcctgcatgatgcgcggcccaaggagggagatgatcgccccttcttctggctctttgagaatgtggtggccatgggcgttagtgacaagagggacatctcgcgatttcttgagtctaaccccgtgatgattgacgccaaagaagtgtctgctgcacacagggcccgttacttctggggtaaccttcctggcatgaacaggcctttggcatccactgtgaatgataagctggagctgcaagagtgtctggagcacggcagaatagccaagttcagcaaagtgaggaccattaccaccaggtcaaactctataaagcagggcaaagaccagcatttccccgtcttcatgaacgagaaggaggacatcctgtggtgcactgaaatggaaagggtgtttggcttccccgtccactacacagacgtctccaacatgagccgcttggcgaggcagagactgctgggccgatcgtggagcgtgccggtcatccgccacctcttcgctccgctgaaggaatattttgcttgtgtgtctagcggcaatagtaacgctaacagccgcgggccgagcttcagcagcggcctggtgccgttaagcttgcgcggcagccatatgggccctatggagatatacaagacagtgtctgcatggaagagacagccagtgcgggtactgagcctcttcagaaacatcgacaaggtactaaagagtttgggcttcttggaaagcggttctggttctgggggaggaacgctgaagtacgtggaagatgtcacaaatgtcgtgaggagagacgtggagaaatggggcccctttgacctggtgtacggctcgacgcagcccctaggcagctcttgtgatcgctgtcccggctggtacatgttccagttccaccggatcctgcagtatgcgctgcctcgccaggagagtcagcggcccttcttctggatattcatggacaatctgctgctgactgaggatgaccaagagacaactacccgcttccttcagacagaggctgtgaccctccaggatgtccgtggcagagactaccagaatgctatgcgggtgtggagcaacattccagggctgaagagcaagcatgcgcccctgaccccaaaggaagaagagtatctgcaagcccaagtcagaagcaggagcaagctggacgccccgaaagttgacctcctggtgaagaactgccttctcccgctgagagagtacttcaagtatttttctcaaaactcacttcctcttggagggccgagctctggcgcacccccaccaagtggagggtctcctgccgggtccccaacatctactgaagaaggcaccagcgaatccgcaacgcccgagtcaggccctggtacctccacagaaccatctgaaggtagtgcgcctggttccccagctggaagccctacttccaccgaagaaggcacgtcaaccgaaccaagtgaaggatctgcccctgggaccagcactgaaccatctgagccaaaaaagaagagaaaggtaatggacaagaagtacagcatcggcctggccatcggcaccaactctgtgggctgggccgtgatcaccgacgagtacaaggtgcccagcaagaaattcaaggtgctgggcaacaccgaccggcacagcatcaagaagaacctgatcggcgccctgctgttcgacagcggagaaacagccgaggccacccggctgaagagaaccgccagaagaagatacaccagacggaagaaccggatctgctatctgcaagagatcttcagcaacgagatggccaaggtggacgacagcttcttccacagactggaagagtccttcctggtggaagaggataagaagcacgagcggcaccccatcttcggcaacatcgtggacgaggtggcctaccacgagaagtaccccaccatctaccacctgagaaagaaactggtggacagcaccgacaaggccgacctgcggctgatctatctggccctggcccacatgatcaagttccggggccacttcctgatcgagggcgacctgaaccccgacaacagcgacgtggacaagctgttcatccagctggtgcagacctacaaccagctgttcgaggaaaaccccatcaacgccagcggcgtggacgccaaggccatcctgtctgccagactgagcaagagcagacggctggaaaatctgatcgcccagctgcccggcgagaagaagaatggcctgttcggcaacctgattgccctgagcctgggcctgacccccaacttcaagagcaacttcgacctggccgaggatgccaaactgcagctgagcaaggacacctacgacgacgacctggacaacctgctggcccagatcggcgaccagtacgccgacctgtttctggccgccaagaacctgtccgacgccatcctgctgagcgacatcctgagagtgaacaccgagatcaccaaggcccccctgagcgcctctatgatcaagagatacgacgagcaccaccaggacctgaccctgctgaaagctctcgtgcggcagcagctgcctgagaagtacaaagagattttcttcgaccagagcaagaacggctacgccggctacatcgatggcggagccagccaggaagagttctacaagttcatcaagcccatcctggaaaagatggacggcaccgaggaactgctcgtgaagctgaacagagaggacctgctgcggaagcagcggaccttcgacaacggcagcatcccccaccagatccacctgggagagctgcacgccattctgcggcggcaggaagatttttacccattcctgaaggacaaccgggaaaagatcgagaagatcctgaccttccgcatcccctactacgtgggccctctggccaggggaaacagcagattcgcctggatgaccagaaagagcgaggaaaccatcaccccctggaacttcgaggaagtggtggacaagggcgccagcgcccagagcttcatcgagcggatgaccaacttcgataagaacctgcccaacgagaaggtgctgcccaagcacagcctgctgtacgagtacttcaccgtgtacaacgagctgaccaaagtgaaatacgtgaccgagggaatgagaaagcccgccttcctgagcggcgagcagaaaaaagccatcgtggacctgctgttcaagaccaaccggaaagtgaccgtgaagcagctgaaagaggactacttcaagaaaatcgagtgcttcgactccgtggaaatctccggcgtggaagatcggttcaacgcctccctgggcacataccacgatctgctgaaaattatcaaggacaaggacttcctggacaatgaggaaaacgaggacattctggaagatatcgtgctgaccctgacactgtttgaggacagagagatgatcgaggaacggctgaaaacctatgcccacctgttcgacgacaaagtgatgaagcagctgaagcggcggagatacaccggctggggcaggctgagccggaagctgatcaacggcatccgggacaagcagtccggcaagacaatcctggatttcctgaagtccgacggcttcgccaacagaaacttcatgcagctgatccacgacgacagcctgacctttaaagaggacatccagaaagcccaggtgtccggccagggcgatagcctgcacgagcacattgccaatctggccggcagccccgccattaagaagggcatcctgcagacagtgaaggtggtggacgagctcgtgaaagtgatgggccggcacaagcccgagaacatcgtgatcgaaatggccagagagaaccagaccacccagaagggacagaagaacagccgcgagagaatgaagcggatcgaagagggcatcaaagagctgggcagccagatcctgaaagaacaccccgtggaaaacacccagctgcagaacgagaagctgtacctgtactacctgcagaatgggcgggatatgtacgtggaccaggaactggacatcaaccggctgtccgactacgatgtggacgctatcgtgcctcagagctttctgaaggacgactccatcgataacaaagtgctgactcggagcgacaagaaccggggcaagagcgacaacgtgccctccgaagaggtcgtgaagaagatgaagaactactggcgccagctgctgaatgccaagctgattacccagaggaagttcgacaatctgaccaaggccgagagaggcggcctgagcgaactggataaggccggcttcatcaagagacagctggtggaaacccggcagatcacaaagcacgtggcacagatcctggactcccggatgaacactaagtacgacgagaacgacaaactgatccgggaagtgaaagtgatcaccctgaagtccaagctggtgtccgatttccggaaggatttccagttttacaaagtgcgcgagatcaacaactaccaccacgcccacgacgcctacctgaacgccgtcgtgggaaccgccctgatcaaaaagtaccctaagctggaaagcgagttcgtgtacggcgactacaaggtgtacgacgtgcggaagatgatcgccaagagcgagcaggaaatcggcaaggctaccgccaagtacttcttctacagcaacatcatgaactttttcaagaccgagattaccctggccaacggcgagatccggaagcggcctctgatcgagacaaacggcgaaacaggcgagatcgtgtgggataagggccgggactttgccaccgtgcggaaagtgctgtctatgccccaagtgaatatcgtgaaaaagaccgaggtgcagacaggcggcttcagcaaagagtctatcctgcccaagaggaacagcgacaagctgatcgccagaaagaaggactgggaccctaagaagtacggcggcttcgacagccccaccgtggcctattctgtgctggtggtggccaaagtggaaaagggcaagtccaagaaactgaagagtgtgaaagagctgctggggatcaccatcatggaaagaagcagcttcgagaagaatcccatcgactttctggaagccaagggctacaaagaagtgaaaaaggacctgatcatcaagctgcctaagtactccctgttcgagctggaaaacggccggaagagaatgctggcctctgccggcgaactgcagaagggaaacgaactggccctgccctccaaatatgtgaacttcctgtacctggccagccactatgagaagctgaagggctcccccgaggataatgagcagaaacagctgtttgtggaacagcacaaacactacctggacgagatcatcgagcagatcagcgagttctccaagagagtgatcctggccgacgctaatctggacaaggtgctgagcgcctacaacaagcacagagacaagcctatcagagagcaggccgagaatatcatccacctgtttaccctgaccaatctgggagcccctgccgccttcaagtactttgacaccaccatcgaccggaagaggtacaccagcaccaaagaggtgctggacgccaccctgatccaccagagcatcaccggcctgtacgagacacggatcgacctgtctcagctgggaggcgacgcctatccctatgacgtgcccgattatgccagcctgggcagcggctcccccaagaaaaaacgcaaggtggaagatcctaagaaaaagcggaaagtggacggcattggtagtgggagcaacggcagcagcggagaggaactgctgagcaagaactaccacctggaaaacgaggtggccagactgaagaaaggctctggctctggcggaagcggttctggcggatcaggatctggaagtggcggctctggaagcggaggttctggatctggcgaagaactgctgtctaagaattatcacctcgagaacgaagtggctcggctcaagaaaggcagtggcagcggaggaagtggatccggcggtagtggtagtggaagcggcggatccggctcaggcggatctggttcaggggaagaactcctctccaaaaactaccatctcgagaatgaggtcgcccgcctgaaaaaaggatcaggttccggtggttctggcagcggtggttcaggctcaggcagcggcggtagcggtagcggtggaagcggaagcggagaagaacttctcagcaaaaattaccacttggagaatgaagttgcaagactcaaaaaaggttccggcagtggcggcagcggcagcggcggatctggtagtggatctggtggcagtggttcaggcggaagtggtagcggagaggaattgctctcaaagaactatcatttggagaacgaggttgcacgcttgaagaaaggcagcggatcaggcggatctggcagcggtggatctggttctggatccggcggctccggtagtggtggaagtggctctggggaagaattgcttagcaagaattatcatcttgaaaatgaggttgccaggcttaaaaaaggcagtggctccggcggatccggaagcggaggcagcggatctggatctggtggttcaggatctggcggttctggtagcggggaagaactgttgagtaaaaactatcaccttgagaacgaggtcgcaaggttgaaaaaaggatccggctctggcggctccggaagtggcggatctggctccggtagcggaggatcaggatccggcggaagcggatcaggcgaggaactgctttccaaaaattaccaccttgaaaacgaagtcgcccgcctcaagaaaggttctggcagcggaggctctggcagtggtggtagcggaagtggaagtggtggcagtggtagcggtggatctggaagcggcgaggaactcctgtcaaagaattaccatctcgaaaacgaggtcgcaaggctcaagaaaggctcaggatcaggcggctctggatccggcggttctggttccggctcaggtggaagtggatctggcggctcaggttccggcgaagaattgctttccaagaactaccatttggaaaatgaagtcgctcgtttgaagaaaggttcaggctccggccagcggggaagcaagcgcaccgccgatggttccgagttcgaaagccccaaaaaaaagcgcaaggtctga

SEQ ID NO: 303 - DNA, 7632 bp, synthetic construct
  misc_feature 1..7632: note = CDS of V15_scFv-ZIM3-2a-D3a-hD3L-dCas9-1xGCN4
  source 1..7632: mol_type = other DNA
atgcctgctgctaagagagtgaaactggatggatccggccccgacatcgtgatgacccagagccccagcagcctgagcgccagcgtgggcgaccgcgtgaccatcacctgccgcagcagcaccggcgccgtgaccaccagcaactacgccagctgggtgcaggagaagcccggcaagctgttcaagggcctgatcggcggcaccaacaaccgcgcccccggcgtgcccagccgcttcagcggcagcctgatcggcgacaaggccaccctgaccatcagcagcctgcagcccgaggacttcgccacctacttctgcgccctgtggtacagcaaccactgggtgttcggccagggcaccaaggtggagctgaagcgcggcggcggcggcagcggcggcggcggcagcggcggcggcggcagcagcggcggcggcagcgaggtgaagctgctggagagcggcggcggcctggtgcagcccggcggcagcctgaagctgagctgcgccgtgagcggcttcagcctgaccgactacggcgtgaactgggtgcgccaggcccccggccgcggcctggagtggatcggcgtgatctggggcgacggcatcaccgactacaacagcgccctgaaggaccgcttcatcatcagcaaggacaacggcaagaacaccgtgtacctgcagatgagcaaggtgcgcagcgacgacaccgccctgtactactgcgtgaccggcctgttcgactactggggccagggcaccctggtgaccgtgagcagctacccatacgatgttccagattacgctggtggaggcggaggttctgggggaggaggtagtggcggtggtggttcaggaggcggcggaagcttggatccaggtggaggtggaagcggtatgaacaattcccagggaagagtgaccttcgaggacgtgaccgtgaacttcacccaaggcgagtggcagagactgaaccccgagcagagaaacctgtaccgggacgtgatgctggaaaactacagcaacctggtgtccgtcggccagggcgagacaacaaagcctgacgtgatcctgcggctggaacagggcaaagagccttggctggaagaggaagaggtgctcggatctggcagagccgagaagaatggcgatatcggcggacagatctggaagccaaaggatgtgaaagagagtctcggaagcggagctactaacttcagcctgctgaagcaggctggagacgtggaggagaaccctggacctatgcctgctgctaagagagtgaaactggatggatccaaccatgaccaggaatttgaccccccaaaggtttacccacctgtgccagctgagaagaggaagcccatccgcgtgctgtctctctttgatgggattgctacagggctcctggtgctgaaggacctgggcatccaagtggaccgctacattgcctccgaggtgtgtgaggactccatcacggtgggcatggtgcggcaccagggaaagatcatgtacgtcggggacgtccgcagcgtcacacagaagcatatccaggagtggggcccattcgacctggtgattggaggcagtccctgcaatgacctctccattgtcaaccctgcccgcaagggactttatgagggtactggccgcctcttctttgagttctaccgcctcctgcatgatgcgcggcccaaggagggagatgatcgccccttcttctggctctttgagaatgtggtggccatgggcgttagtgacaagagggacatctcgcgatttcttgagtctaaccccgtgatgattgacgccaaagaagtgtctgctgcacacagggcccgttacttctggggtaaccttcctggcatgaacaggcctttggcatccactgtgaatgataagctggagctgcaagagtgtctggagcacggcagaatagccaagttcagcaaagtgaggaccattaccaccaggtcaaactctataaagcagggcaaagaccagcatttccccgtgttcatgaacgagaaggaggacatcctgtggtgcactgaaatggaaagggtgtttggcttccccgtccactacacagacgtctccaacatgagccgcttggcgaggcagagactgctgggccgatcgtggagcgtgccggtcatccgccacctcttcgctccgctgaaggaatattttgcttgtgtgtctagcggcaatagtaacgctaacagccgcgggccgagcttcagcagcggcctggtgccgttaagcttgcgcggcagccatatgttcgaaaccgtgcctgtgtggaggagacagccagtccgggtgctgtccctttttgaagacatcaagaaagagctgacgagtttgggctttttggaaagtggttctgacccgggacaactgaagcatgtggttgatgtcacagacacagtgaggaaggatgtggaggagtggggacccttcgatcttgtgtacggcgccacacctcccctgggccacacctgtgaccgtcctcccagctggtacctgttccagttccaccggctcctgcagtacgcacggcccaagccaggcagccccaggcccttcttctggatgttcgtggacaatctggtgctgaacaaggaagacctggacgtcgcatctcgcttcctggagatggagccagtcaccatcccagatgtccacggcggatccttgcagaatgctgtccgcgtgtggagcaacatcccagccataaggagcagcaggcactgggctctggtttcggaagaagaattgtccctgctggcccagaacaagcagagctcgaagctcgcggccaagtggcccaccaagctggtgaagaactgctttctccccctaagagaatatttcaagtatttttcaggagggccgagctctggcgcacccccaccaagtggagggtctcctgccgggtccccaacatctactgaagaaggcaccagcgaatccgcaacgcccgagtcaggccctggtacctccacagaaccatctgaaggtagtgcgcctggttccccagctggaagccctacttccaccgaagaaggcacgtcaaccgaaccaagtgaaggatctgcccctgggaccagcactgaaccatctgagccaaaaaagaagagaaaggtaatggacaagaagtacagcatcggcctggccatcggcaccaactctgtgggctgggccgtgatcaccgacgagtacaaggtgcccagcaagaaattcaaggtgctgggcaacaccgaccggcacagcatcaagaagaacctgatcggcgccctgctgttcgacagcggagaaacagccgaggccacccggctgaagagaaccgccagaagaagatacaccagacggaagaaccggatctgctatctgcaagagatcttcagcaacgagatggccaaggtggacgacagcttcttccacagactggaagagtccttcctggtggaagaggataagaagcacgagcggcaccccatcttcggcaacatcgtggacgaggtggcctaccacgagaagtaccccaccatctaccacctgagaaagaaactggtggacagcaccgacaaggccgacctgcggctgatctatctggccctggcccacatgatcaagttccggggccacttcctgatcgagggcgacctgaaccccgacaacagcgacgtggacaagctgttcatccagctggtgcagacctacaaccagctgttcgaggaaaaccccatcaacgccagcggcgtggacgccaaggccatcctgtctgccagactgagcaagagcagacggctggaaaatctgatcgcccagctgcccggcgagaagaagaatggcctgttcggcaacctgattgccctgagcctgggcctgacccccaacttcaagagcaacttcgacctggccgaggatgccaaactgcagctgagcaaggacacctacgacgacgacctggacaacctgctggcccagatcggcgaccagtacgccgacctgtttctggccgccaagaacctgtccgacgccatcctgctgagcgacatcctgagagtgaacaccgagatcaccaaggcccccctgagcgcctctatgatcaagagatacgacgagcaccaccaggacctgaccctgctgaaagctctcgtgcggcagcagctgcctgagaagtacaaagagattttcttcgaccagagcaagaacggctacgccggctacatcgatggcggagccagccaggaagagttctacaagttcatcaagcccatcctggaaaagatggacggcaccgaggaactgctcgtgaagctgaacagagaggacctgctgcggaagcagcggaccttcgacaacggcagcatcccccaccagatccacctgggagagctgcacgccattctgcggcggcaggaagatttttacccattcctgaaggacaaccgggaaaagatcgagaagatcctgaccttccgcatcccctactacgtgggccctctggccaggggaaacagcagattcgcctggatgaccagaaagagcgaggaaaccatcaccccctggaacttcgaggaagtggtggacaagggcgccagcgcccagagcttcatcgagcggatgaccaacttcgataagaacctgcccaacgagaaggtgctgcccaagcacagcctgctgtacgagtacttcaccgtgtacaacgagctgaccaaagtgaaatacgtgaccgagggaatgagaaagcccgccttcctgagcggcgagcagaaaaaagccatcgtggacctgctgttcaagaccaaccggaaagtgaccgtgaagcagctgaaagaggactacttcaagaaaatcgagtgcttcgactccgtggaaatctccggcgtggaagatcggttcaacgcctccctgggcacataccacgatctgctgaaaattatcaaggacaaggacttcctggacaatgaggaaaacgaggacattctggaagatatcgtgctgaccctgacactgtttgaggacagagagatgatcgaggaacggctgaaaacctatgcccacctgttcgacgacaaagtgatgaagcagctgaagcggcggagatacaccggctggggcaggctgagccggaagctgatcaacggcatccgggacaagcagtccggcaagacaatcctggatttcctgaagtccgacggcttcgccaacagaaacttcatgcagctgatccacgacgacagcctgacctttaaagaggacatccagaaagcccaggtgtccggccagggcgatagcctgcacgagcacattgccaatctggccggcagccccgccattaagaagggcatcctgcagacagtgaaggtggtggacgagctcgtgaaagtgatgggccggcacaagcccgagaacatcgtgatcgaaatggccagagagaaccagaccacccagaagggacagaagaacagccgcgagagaatgaagcggatcgaagagggcatcaaagagctgggcagccagatcctgaaagaacaccccgtggaaaacacccagctgcagaacgagaagctgtacctgtactacctgcagaatgggcgggatatgtacgtggaccaggaactggacatcaaccggctgtccgactacgatgtggacgctatcgtgcctcagagctttctgaaggacgactccatcgataacaaagtgctgactcggagcgacaagaaccggggcaagagcgacaacgtgccctccgaagaggtcgtgaagaagatgaagaactactggcgccagctgctgaatgccaagctgattacccagaggaagttcgacaatctgaccaaggccgagagaggcggcctgagcgaactggataaggccggcttcatcaagagacagctggtggaaacccggcagatcacaaagcacgtggcacagatcctggactcccggatgaacactaagtacgacgagaacgacaaactgatccgggaagtgaaagtgatcaccctgaagtccaagctggtgtccgatttccggaaggatttccagttttacaaagtgcgcgagatcaacaactaccaccacgcccacgacgcctacctgaacgccgtcgtgggaaccgccctgatcaaaaagtaccctaagctggaaagcgagttcgtgtacggcgactacaaggtgtacgacgtgcggaagatgatcgccaagagcgagcaggaaatcggcaaggctaccgccaagtacttcttctacagcaacatcatgaactttttcaagaccgagattaccctggccaacggcgagatccggaagcggcctctgatcgagacaaacggcgaaacaggcgagatcgtgtgggataagggccgggactttgccaccgtgcggaaagtgctgtctatgccccaagtgaatatcgtgaaaaagaccgaggtgcagacaggcggcttcagcaaagagtctatcctgcccaagaggaacagcgacaagctgatcgccagaaagaaggactgggaccctaagaagtacggcggcttcgacagccccaccgtggcctattctgtgctggtggtggccaaagtggaaaagggcaagtccaagaaactgaagagtgtgaaagagctgctggggatcaccatcatggaaagaagcagcttcgagaagaatcccatcgactttctggaagccaagggctacaaagaagtgaaaaaggacctgatcatcaagctgcctaagtactccctgttcgagctggaaaacggccggaagagaatgctggcctctgccggcgaactgcagaagggaaacgaactggccctgccctccaaatatgtgaacttcctgtacctggccagccactatgagaagctgaagggctcccccgaggataatgagcagaaacagctgtttgtggaacagcacaaacactacctggacgagatcatcgagcagatcagcgagttctccaagagagtgatcctggccgacgctaatctggacaaggtgctgagcgcctacaacaagcacagagacaagcctatcagagagcaggccgagaatatcatccacctgtttaccctgaccaatctgggagcccctgccgccttcaagtactttgacaccaccatcgaccggaagaggtacaccagcaccaaagaggtgctggacgccaccctgatccaccagagcatcaccggcctgtacgagacacggatcgacctgtctcagctgggaggcgacgcctatccctatgacgtgcccgattatgccagcctgggcagcggctcccccaagaaaaaacgcaaggtggaagatcctaagaaaaagcggaaagtggacggcattggtagtgggagcaacggcagcagcggagaggaactgctgagcaagaactaccacctggaaaacgaggtggccagactgaagaaaggctctggctctggcggaagcggttctggcggatcaggatctggaagtggcggctctggaagcggaggttctggatctggcgaagaactgctgtctaagaattatcacggttcaggctccggccagcggggaagcaagcgcaccgccgatggttccgagttcgaaagccccaaaaaaaagcgcaaggtctga

SEQ ID NO: 304 - DNA, 7662 bp, synthetic construct
  misc_feature 1..7662: note = CDS of V16_scFv-ZIM3-2a-D3a-hD3L-dCas9-2xGCN4
  source 1..7662: mol_type = other DNA
atgcctgctgctaagagagtgaaactggatggatccggccccgacatcgtgatgacccagagccccagcagcctgagcgccagcgtgggcgaccgcgtgaccatcacctgccgcagcagcaccggcgccgtgaccaccagcaactacgccagctgggtgcaggagaagcccggcaagctgttcaagggcctgatcggcggcaccaacaaccgcgcccccggcgtgcccagccgcttcagcggcagcctgatcggcgacaaggccaccctgaccatcagcagcctgcagcccgaggacttcgccacctacttctgcgccctgtggtacagcaaccactgggtgttcggccagggcaccaaggtggagctgaagcgcggcggcggcggcagcggcggcggcggcagcggcggcggcggcagcagcggcggcggcagcgaggtgaagctgctggagagcggcggcggcctggtgcagcccggcggcagcctgaagctgagctgcgccgtgagcggcttcagcctgaccgactacggcgtgaactgggtgcgccaggcccccggccgcggcctggagtggatcggcgtgatctggggcgacggcatcaccgactacaacagcgccctgaaggaccgcttcatcatcagcaaggacaacggcaagaacaccgtgtacctgcagatgagcaaggtgcgcagcgacgacaccgccctgtactactgcgtgaccggcctgttcgactactggggccagggcaccctggtgaccgtgagcagctacccatacgatgttccagattacgctggtggaggcggaggttctgggggaggaggtagtggcggtggtggttcaggaggcggcggaagcttggatccaggtggaggtggaagcggtatgaacaattcccagggaagagtgaccttcgaggacgtgaccgtgaacttcacccaaggcgagtggcagagactgaaccccgagcagagaaacctgtaccgggacgtgatgctggaaaactacagcaacctggtgtccgtcggccagggcgagacaacaaagcctgacgtgatcctgcggctggaacagggcaaagagccttggctggaagaggaagaggtgctcggatctggcagagccgagaagaatggcgatatcggcggacagatctggaagccaaaggatgtgaaagagagtctcggaagcggagctactaacttcagcctgctgaagcaggctggagacgtggaggagaaccctggacctatgcctgctgctaagagagtgaaactggatggatccaaccatgaccaggaatttgaccccccaaaggtttacccacctgtgccagctgagaagaggaagcccatccgcgtgctgtctctctttgatgggattgctacagggctcctggtgctgaaggacctgggcatccaagtggaccgctacattgcctccgaggtgtgtgaggactccatcacggtgggcatggtgcggcaccagggaaagatcatgtacgtcggggacgtccgcagcgtcacacagaagcatatccaggagtggggcccattcgacctggtgattggaggcagtccctgcaatgacctctccattgtcaaccctgcccgcaagggactttatgagggtactggccgcctcttctttgagttctaccgcctcctgcatgatgcgcggcccaaggagggagatgatcgccccttcttctggctctttgagaatgtggtggccatgggcgttagtgacaagagggacatctcgcgatttcttgagtctaaccccgtgatgattgacgccaaagaagtgtctgctgcacacagggcccgttacttctggggtaaccttcctggcatgaacaggcctttggcatccactgtgaatgataagctggagctgcaagagtgtctggagcacggcagaatagccaagttcagcaaagtgaggaccattaccaccaggtcaaactctataaagcagggcaaagaccagcatttccccgtgttcatgaacgagaaggaggacatcctgtggtgcactgaaatggaaagggtgtttggcttccccgtccactacacagacgtctccaacatgagccgcttggcgaggcagagactgctgggccgatcgtggagcgtgccggtcatccgccacctcttcgctccgctgaaggaatattttgcttgtgtgtctagcggcaatagtaacgctaacagccgcgggccgagcttcagcagcggcctggtgccgttaagcttgcgcggcagccatatgttcgaaaccgtgcctgtgtggaggagacagccagtccgggtgctgtccctttttgaagacatcaagaaagagctgacgagtttgggctttttggaaagtggttctgacccgggacaactgaagcatgtggttgatgtcacagacacagtgaggaaggatgtggaggagtggggacccttcgatcttgtgtacggcgccacacctcccctgggccacacctgtgaccgtcctcccagctggtacctgttccagttccaccggctcctgcagtacgcacggcccaagccaggcagccccaggcccttcttctggatgttcgtggacaatctggtgctgaacaaggaagacctggacgtcgcatctcgcttcctggagatggagccagtcaccatcccagatgtccacggcggatccttgcagaatgctgtccgcgtgtggagcaacatcccagccataaggagcagcaggcactgggctctggtttcggaagaagaattgtccctgctggcccagaacaagcagagctcgaagctcgcggccaagtggcccaccaagctggtgaagaactgctttctccccctaagagaatatttcaagtatttttcaggagggccgagctctggcgcacccccaccaagtggagggtctcctgccgggtccccaacatctactgaagaaggcaccagcgaatccgcaacgcccgagtcaggccctggtacctccacagaaccatctgaaggtagtgcgcctggttccccagctggaagccctacttccaccgaagaaggcacgtcaaccgaaccaagtgaaggatctgcccctgggaccagcactgaaccatctgagccaaaaaagaagagaaaggtaatggacaagaagtacagcatcggcctggccatcggcaccaactctgtgggctgggccgtgatcaccgacgagtacaaggtgcccagcaagaaattcaaggtgctgggcaacaccgaccggcacagcatcaagaagaacctgatcggcgccctgctgttcgacagcggagaaacagccgaggccacccggctgaagagaaccgccagaagaagatacaccagacggaagaaccggatctgctatctgcaagagatcttcagcaacgagatggccaaggtggacgacagcttcttccacagactggaagagtccttcctggtggaagaggataagaagcacgagcggcaccccatcttcggcaacatcgtggacgaggtggcctaccacgagaagtaccccaccatctaccacctgagaaagaaactggtggacagcaccgacaaggccgacctgcggctgatctatctggccctggcccacatgatcaagttccggggccacttcctgatcgagggcgacctgaaccccgacaacagcgacgtggacaagctgttcatccagctggtgcagacctacaaccagctgttcgaggaaaaccccatcaacgccagcggcgtggacgccaaggccatcctgtctgccagactgagcaagagcagacggctggaaaatctgatcgcccagctgcccggcgagaagaagaatggcctgttcggcaacctgattgccctgagcctgggcctgacccccaacttcaagagcaacttcgacctggccgaggatgccaaactgcagctgagcaaggacacctacgacgacgacctggacaacctgctggcccagatcggcgaccagtacgccgacctgtttctggccgccaagaacctgtccgacgccatcctgctgagcgacatcctgagagtgaacaccgagatcaccaaggcccccctgagcgcctctatgatcaagagatacgacgagcaccaccaggacctgaccctgctgaaagctctcgtgcggcagcagctgcctgagaagtacaaagagattttcttcgaccagagcaagaacggctacgccggctacatcgatggcggagccagccaggaagagttctacaagttcatcaagcccatcctggaaaagatggacggcaccgaggaactgctcgtgaagctgaacagagaggacctgctgcggaagcagcggaccttcgacaacggcagcatcccccaccagatccacctgggagagctgcacgccattctgcggcggcaggaagatttttacccattcctgaaggacaaccgggaaaagatcgagaagatcctgaccttccgcatcccctactacgtgggccctctggccaggggaaacagcagattcgcctggatgaccagaaagagcgaggaaaccatcaccccctggaacttcgaggaagtggtggacaagggcgccagcgcccagagcttcatcgagcggatgaccaacttcgataagaacctgcccaacgagaaggtgctgcccaagcacagcctgctgtacgagtacttcaccgtgtacaacgagctgaccaaagtgaaatacgtgaccgagggaatgagaaagcccgccttcctgagcggcgagcagaaaaaagccatcgtggacctgctgttcaagaccaaccggaaagtgaccgtgaagcagctgaaagaggactacttcaagaaaatcgagtgcttcgactccgtggaaatctccggcgtggaagatcggttcaacgcctccctgggcacataccacgatctgctgaaaattatcaaggacaaggacttcctggacaatgaggaaaacgaggacattctggaagatatcgtgctgaccctgacactgtttgaggacagagagatgatcgaggaacggctgaaaacctatgcccacctgttcgacgacaaagtgatgaagcagctgaagcggcggagatacaccggctggggcaggctgagccggaagctgatcaacggcatccgggacaagcagtccggcaagacaatcctggatttcctgaagtccgacggcttcgccaacagaaacttcatgcagctgatccacgacgacagcctgacctttaaagaggacatccagaaagcccaggtgtccggccagggcgatagcctgcacgagcacattgccaatctggccggcagccccgccattaagaagggcatcctgcagacagtgaaggtggtggacgagctcgtgaaagtgatgggccggcacaagcccgagaacatcgtgatcgaaatggccagagagaaccagaccacccagaagggacagaagaacagccgcgagagaatgaagcggatcgaagagggcatcaaagagctgggcagccagatcctgaaagaacaccccgtggaaaacacccagctgcagaacgagaagctgtacctgtactacctgcagaatgggcgggatatgtacgtggaccaggaactggacatcaaccggctgtccgactacgatgtggacgctatcgtgcctcagagctttctgaaggacgactccatcgataacaaagtgctgactcggagcgacaagaaccggggcaagagcgacaacgtgccctccgaagaggtcgtgaagaagatgaagaactactggcgccagctgctgaatgccaagctgattacccagaggaagttcgacaatctgaccaaggccgagagaggcggcctgagcgaactggataaggccggcttcatcaagagacagctggtggaaacccggcagatcacaaagcacgtggcacagatcctggactcccggatgaacactaagtacgacgagaacgacaaactgatccgggaagtgaaagtgatcaccctgaagtccaagctggtgtccgatttccggaaggatttccagttttacaaagtgcgcgagatcaacaactaccaccacgcccacgacgcctacctgaacgccgtcgtgggaaccgccctgatcaaaaagtaccctaagctggaaagcgagttcgtgtacggcgactacaaggtgtacgacgtgcggaagatgatcgccaagagcgagcaggaaatcggcaaggctaccgccaagtacttcttctacagcaacatcatgaactttttcaagaccgagattaccctggccaacggcgagatccggaagcggcctctgatcgagacaaacggcgaaacaggcgagatcgtgtgggataagggccgggactttgccaccgtgcggaaagtgctgtctatgccccaagtgaatatcgtgaaaaagaccgaggtgcagacaggcggcttcagcaaagagtctatcctgcccaagaggaacagcgacaagctgatcgccagaaagaaggactgggaccctaagaagtacggcggcttcgacagccccaccgtggcctattctgtgctggtggtggccaaagtggaaaagggcaagtccaagaaactgaagagtgtgaaagagctgctggggatcaccatcatggaaagaagcagcttcgagaagaatcccatcgactttctggaagccaagggctacaaagaagtgaaaaaggacctgatcatcaagctgcctaagtactccctgttcgagctggaaaacggccggaagagaatgctggcctctgccggcgaactgcagaagggaaacgaactggccctgccctccaaatatgtgaacttcctgtacctggccagccactatgagaagctgaagggctcccccgaggataatgagcagaaacagctgtttgtggaacagcacaaacactacctggacgagatcatcgagcagatcagcgagttctccaagagagtgatcctggccgacgctaatctggacaaggtgctgagcgcctacaacaagcacagagacaagcctatcagagagcaggccgagaatatcatccacctgtttaccctgaccaatctgggagcccctgccgccttcaagtactttgacaccaccatcgaccggaagaggtacaccagcaccaaagaggtgctggacgccaccctgatccaccagagcatcaccggcctgtacgagacacggatcgacctgtctcagctgggaggcgacgcctatccctatgacgtgcccgattatgccagcctgggcagcggctcccccaagaaaaaacgcaaggtggaagatcctaagaaaaagcggaaagtggacggcattggtagtgggagcaacggcagcagcggagaggaactgctgagcaagaactaccacctggaaaacgaggtggccagactgaagaaaggctctggctctggcggaagcggttctggcggatcaggatctggaagtggcggctctggaagcggaggttctggatctggcgaagaactgctgtctaagaattatcacctcgagaatgaagtcgctcgtttgaagaaaggttcaggctccggccagcggggaagcaagcgcaccgccgatggttccgagttcgaaagccccaaaaaaaagcgcaaggtctga

SEQ ID NO: 305 - DNA, 8766 bp, synthetic construct
  misc_feature 1..8766: note = CDS of V17_scFv-ZIM3-2a-D3a-hD3L-dCas9-10xGCN4
  source 1..8766: mol_type = other DNA
atgcctgctgctaagagagtgaaactggatggatccggccccgacatcgtgatgacccagagccccagcagcctgagcgccagcgtgggcgaccgcgtgaccatcacctgccgcagcagcaccggcgccgtgaccaccagcaactacgccagctgggtgcaggagaagcccggcaagctgttcaagggcctgatcggcggcaccaacaaccgcgcccccggcgtgcccagccgcttcagcggcagcctgatcggcgacaaggccaccctgaccatcagcagcctgcagcccgaggacttcgccacctacttctgcgccctgtggtacagcaaccactgggtgttcggccagggcaccaaggtggagctgaagcgcggcggcggcggcagcggcggcggcggcagcggcggcggcggcagcagcggcggcggcagcgaggtgaagctgctggagagcggcggcggcctggtgcagcccggcggcagcctgaagctgagctgcgccgtgagcggcttcagcctgaccgactacggcgtgaactgggtgcgccaggcccccggccgcggcctggagtggatcggcgtgatctggggcgacggcatcaccgactacaacagcgccctgaaggaccgcttcatcatcagcaaggacaacggcaagaacaccgtgtacctgcagatgagcaaggtgcgcagcgacgacaccgccctgtactactgcgtgaccggcctgttcgactactggggccagggcaccctggtgaccgtgagcagctacccatacgatgttccagattacgctggtggaggcggaggttctgggggaggaggtagtggcggtggtggttcaggaggcggcggaagcttggatccaggtggaggtggaagcggtatgaacaattcccagggaagagtgaccttcgaggacgtgaccgtgaacttcacccaaggcgagtggcagagactgaaccccgagcagagaaacctgtaccgggacgtgatgctggaaaactacagcaacctggtgtccgtcggccagggcgagacaacaaagcctgacgtgatcctgcggctggaacagggcaaagagccttggctggaagaggaagaggtgctcggatctggcagagccgagaagaatggcgatatcggcggacagatctggaagccaaaggatgtgaaagagagtctcggaagcggagctactaacttcagcctgctgaagcaggctggagacgtggaggagaaccctggacctatgcctgctgctaagagagtgaaactggatggatccaaccatgaccaggaatttgaccccccaaaggtttacccacctgtgccagctgagaagaggaagcccatccgcgtgctgtctctctttgatgggattgctacagggctcctggtgctgaaggacctgggcatccaagtggaccgctacattgcctccgaggtgtgtgaggactccatcacggtgggcatggtgcggcaccagggaaagatcatgtacgtcggggacgtccgcagcgtcacacagaagcatatccaggagtggggcccattcgacctggtgattggaggcagtccctgcaatgacctctccattgtcaaccctgcccgcaagggactttatgagggtactggccgcctcttctttgagttctaccgcctcctgcatgatgcgcggcccaaggagggagatgatcgccccttcttctggctctttgagaatgtggtggccatgggcgttagtgacaagagggacatctcgcgatttcttgagtctaaccccgtgatgattgacgccaaagaagtgtctgctgcacacagggcccgttacttctggggtaaccttcctggcatgaacaggcctttggcatccactgtgaatgataagctggagctgcaagagtgtctggagcacggcagaatagccaagttcagcaaagtgaggaccattaccaccaggtcaaactctataaagcagggcaaagaccagcatttccccgtgttcatgaacgagaaggaggacatcctgtggtgcactgaaatggaaagggtgtttggcttccccgtccactacacagacgtctccaacatgagccgcttggcgaggcagagactgctgggccgatcgtggagcgtgccggtcatccgccacctcttcgctccgctgaaggaatattttgcttgtgtgtctagcggcaatagtaacgctaacagccgcgggccgagcttcagcagcggcctggtgccgttaagcttgcgcggcagccatatgttcgaaaccgtgcctgtgtggaggagacagccagtccgggtgctgtccctttttgaagacatcaagaaagagctgacgagtttgggctttttggaaagtggttctgacccgggacaactgaagcatgtggttgatgtcacagacacagtgaggaaggatgtggaggagtggggacccttcgatcttgtgtacggcgccacacctcccctgggccacacctgtgaccgtcctcccagctggtacctgttccagttccaccggctcctgcagtacgcacggcccaagccaggcagccccaggcccttcttctggatgttcgtggacaatctggtgctgaacaaggaagacctggacgtcgcatctcgcttcctggagatggagccagtcaccatcccagatgtccacggcggatccttgcagaatgctgtccgcgtgtggagcaacatcccagccataaggagcagcaggcactgggctctggtttcggaagaagaattgtccctgctggcccagaacaagcagagctcgaagctcgcggccaagtggcccaccaagctggtgaagaactgctttctccccctaagagaatatttcaagtatttttcaggagggccgagctctggcgcacccccaccaagtggagggtctcctgccgggtccccaacatctactgaagaaggcaccagcgaatccgcaacgcccgagtcaggccctggtacctccacagaaccatctgaaggtagtgcgcctggttccccagctggaagccctacttccaccgaagaaggcacgtcaaccgaaccaagtgaaggatctgcccctgggaccagcactgaaccatctgagccaaaaaagaagagaaaggtaatggacaagaagtacagcatcggcctggccatcggcaccaactctgtgggctgggccgtgatcaccgacgagtacaaggtgcccagcaagaaattcaaggtgctgggcaacaccgaccggcacagcatcaagaagaacctgatcggcgccctgctgttcgacagcggagaaacagccgaggccacccggctgaagagaaccgccagaagaagatacaccagacggaagaaccggatctgctatctgcaagagatcttcagcaacgagatggccaaggtggacgacagcttcttccacagactggaagagtccttcctggtggaagaggataagaagcacgagcggcaccccatcttcggcaacatcgtggacgaggtggcctaccacgagaagtaccccaccatctaccacctgagaaagaaactggtggacagcaccgacaaggccgacctgcggctgatctatctggccctggcccacatgatcaagttccggggccacttcctgatcgagggcgacctgaaccccgacaacagcgacgtggacaagctgttcatccagctggtgcagacctacaaccagctgttcgaggaaaaccccatcaacgccagcggcgtggacgccaaggccatcctgtctgccagactgagcaagagcagacggctggaaaatctgatcgcccagctgcccggcgagaagaagaatggcctgttcggcaacctgattgccctgagcctgggcctgacccccaacttcaagagcaacttcgacctggccgaggatgccaaactgcagctgagcaaggacacctacgacgacgacctggacaacctgctggcccagatcggcgaccagtacgccgacctgtttctggccgccaagaacctgtccgacgccatcctgctgagcgacatcctgagagtgaacaccgagatcaccaaggcccccctgagcgcctctatgatcaagagatacgacgagcaccaccaggacctgaccctgctgaaagctctcgtgcggcagcagctgcctgagaagtacaaagagattttcttcgaccagagcaagaacggctacgccggctacatcgatggcggagccagccaggaagagttctacaagttcatcaagcccatcctggaaaagatggacggcaccgaggaactgctcgtgaagctgaacagagaggacctgctgcggaagcagcggaccttcgacaacggcagcatcccccaccagatccacctgggagagctgcacgccattctgcggcggcaggaagatttttacccattcctgaaggacaaccgggaaaagatcgagaagatcctgaccttccgcatcccctactacgtgggccctctggccaggggaaacagcagattcgcctggatgaccagaaagagcgaggaaaccatcaccccctggaacttcgaggaagtggtggacaagggcgccagcgcccagagcttcatcgagcggatgaccaacttcgataagaacctgcccaacgagaaggtgctgcccaagcacagcctgctgtacgagtacttcaccgtgtacaacgagctgaccaaagtgaaatacgtgaccgagggaatgagaaagcccgccttcctgagcggcgagcagaaaaaagccatcgtggacctgctgttcaagaccaaccggaaagtgaccgtgaagcagctgaaagaggactacttcaagaaaatcgagtgcttcgactccgtggaaatctccggcgtggaagatcggttcaacgcctccctgggcacataccacgatctgctgaaaattatcaaggacaaggacttcctggacaatgaggaaaacgaggacattctggaagatatcgtgctgaccctgacactgtttgaggacagagagatgatcgaggaacggctgaaaacctatgcccacctgttcgacgacaaagtgatgaagcagctgaagcggcggagatacaccggctggggcaggctgagccggaagctgatcaacggcatccgggacaagcagtccggcaagacaatcctggatttcctgaagtccgacggcttcgccaacagaaacttcatgcagctgatccacgacgacagcctgacctttaaagaggacatccagaaagcccaggtgtccggccagggcgatagcctgcacgagcacattgccaatctggccggcagccccgccattaagaagggcatcctgcagacagtgaaggtggtggacgagctcgtgaaagtgatgggccggcacaagcccgagaacatcgtgatcgaaatggccagagagaaccagaccacccagaagggacagaagaacagccgcgagagaatgaagcggatcgaagagggcatcaaagagctgggcagccagatcctgaaagaacaccccgtggaaaacacccagctgcagaacgagaagctgtacctgtactacctgcagaatgggcgggatatgtacgtggaccaggaactggacatcaaccggctgtccgactacgatgtggacgctatcgtgcctcagagctttctgaaggacgactccatcgataacaaagtgctgactcggagcgacaagaaccggggcaagagcgacaacgtgccctccgaagaggtcgtgaagaagatgaagaactactggcgccagctgctgaatgccaagctgattacccagaggaagttcgacaatctgaccaaggccgagagaggcggcctgagcgaactggataaggccggcttcatcaagagacagctggtggaaacccggcagatcacaaagcacgtggcacagatcctggactcccggatgaacactaagtacgacgagaacgacaaactgatccgggaagtgaaagtgatcaccctgaagtccaagctggtgtccgatttccggaaggatttccagttttacaaagtgcgcgagatcaacaactaccaccacgcccacgacgcctacctgaacgccgtcgtgggaaccgccctgatcaaaaagtaccctaagctggaaagcgagttcgtgtacggcgactacaaggtgtacgacgtgcggaagatgatcgccaagagcgagcaggaaatcggcaaggctaccgccaagtacttcttctacagcaacatcatgaactttttcaagaccgagattaccctggccaacggcgagatccggaagcggcctctgatcgagacaaacggcgaaacaggcgagatcgtgtgggataagggccgggactttgccaccgtgcggaaagtgctgtctatgccccaagtgaatatcgtgaaaaagaccgaggtgcagacaggcggcttcagcaaagagtctatcctgcccaagaggaacagcgacaagctgatcgccagaaagaaggactgggaccctaagaagtacggcggcttcgacagccccaccgtggcctattctgtgctggtggtggccaaagtggaaaagggcaagtccaagaaactgaagagtgtgaaagagctgctggggatcaccatcatggaaagaagcagcttcgagaagaatcccatcgactttctggaagccaagggctacaaagaagtgaaaaaggacctgatcatcaagctgcctaagtactccctgttcgagctggaaaacggccggaagagaatgctggcctctgccggcgaactgcagaagggaaacgaactggccctgccctccaaatatgtgaacttcctgtacctggccagccactatgagaagctgaagggctcccccgaggataatgagcagaaacagctgtttgtggaacagcacaaacactacctggacgagatcatcgagcagatcagcgagttctccaagagagtgatcctggccgacgctaatctggacaaggtgctgagcgcctacaacaagcacagagacaagcctatcagagagcaggccgagaatatcatccacctgtttaccctgaccaatctgggagcccctgccgccttcaagtactttgacaccaccatcgaccggaagaggtacaccagcaccaaagaggtgctggacgccaccctgatccaccagagcatcaccggcctgtacgagacacggatcgacctgtctcagctgggaggcgacgcctatccctatgacgtgcccgattatgccagcctgggcagcggctcccccaagaaaaaacgcaaggtggaagatcctaagaaaaagcggaaagtggacggcattggtagtgggagcaacggcagcagcggagaggaactgctgagcaagaactaccacctggaaaacgaggtggccagactgaagaaaggctctggctctggcggaagcggttctggcggatcaggatctggaagtggcggctctggaagcggaggttctggatctggcgaagaactgctgtctaagaattatcacctcgagaacgaagtggctcggctcaagaaaggcagtggcagcggaggaagtggatccggcggtagtggtagtggaagcggcggatccggctcaggcggatctggttcaggggaagaactcctctccaaaaactaccatctcgagaatgaggtcgcccgcctgaaaaaaggatcaggttccggtggttctggcagcggtggttcaggctcaggcagcggcggtagcggtagcggtggaagcggaagcggagaagaacttctcagcaaaaattaccacttggagaatgaagttgcaagactcaaaaaaggttccggcagtggcggcagcggcagcggcggatctggtagtggatctggtggcagtggttcaggcggaagtggtagcggagaggaattgctctcaaagaactatcatttggagaacgaggttgcacgcttgaagaaaggcagcggatcaggcggatctggcagcggtggatctggttctggatccggcggctccggtagtggtggaagtggctctggggaagaattgcttagcaagaattatcatcttgaaaatgaggttgccaggcttaaaaaaggcagtggctccggcggatccggaagcggaggcagcggatctggatctggtggttcaggatctggcggttctggtagcggggaagaactgttgagtaaaaactatcaccttgagaacgaggtcgcaaggttgaaaaaaggatccggctctggcggctccggaagtggcggatctggctccggtagcggaggatcaggatccggcggaagcggatcaggcgaggaactgctttccaaaaattaccaccttgaaaacgaagtcgcccgcctcaagaaaggttctggcagcggaggctctggcagtggtggtagcggaagtggaagtggtggcagtggtagcggtggatctggaagcggcgaggaactcctgtcaaagaattaccatctcgaaaacgaggtcgcaaggctcaagaaaggctcaggatcaggcggctctggatccggcggttctggttccggctcaggtggaagtggatctggcggctcaggttccggcgaagaattgctttccaagaactaccatttggaaaatgaagtcgctcgtttgaagaaaggttcaggctccggccagcggggaagcaagcgcaccgccgatggttccgagttcgaaagccccaaaaaaaagcgcaaggtctga

SEQ ID NO: 306 - DNA, 7212 bp, synthetic construct
  misc_feature 1..7212: note = CDS of V18_scFv-ZIM3-2a-D3a-hD3L-dCas12a-1xGCN4
  source 1..7212: mol_type = other DNA
atgcctgctgctaagagagtgaaactggatggatccggccccgacatcgtgatgacccagagccccagcagcctgagcgccagcgtgggcgaccgcgtgaccatcacctgccgcagcagcaccggcgccgtgaccaccagcaactacgccagctgggtgcaggagaagcccggcaagctgttcaagggcctgatcggcggcaccaacaaccgcgcccccggcgtgcccagccgcttcagcggcagcctgatcggcgacaaggccaccctgaccatcagcagcctgcagcccgaggacttcgccacctacttctgcgccctgtggtacagcaaccactgggtgttcggccagggcaccaaggtggagctgaagcgcggcggcggcggcagcggcggcggcggcagcggcggcggcggcagcagcggcggcggcagcgaggtgaagctgctggagagcggcggcggcctggtgcagcccggcggcagcctgaagctgagctgcgccgtgagcggcttcagcctgaccgactacggcgtgaactgggtgcgccaggcccccggccgcggcctggagtggatcggcgtgatctggggcgacggcatcaccgactacaacagcgccctgaaggaccgcttcatcatcagcaaggacaacggcaagaacaccgtgtacctgcagatgagcaaggtgcgcagcgacgacaccgccctgtactactgcgtgaccggcctgttcgactactggggccagggcaccctggtgaccgtgagcagctacccatacgatgttccagattacgctggtggaggcggaggttctgggggaggaggtagtggcggtggtggttcaggaggcggcggaagcttggatccaggtggaggtggaagcggtatgaacaattcccagggaagagtgaccttcgaggacgtgaccgtgaacttcacccaaggcgagtggcagagactgaaccccgagcagagaaacctgtaccgggacgtgatgctggaaaactacagcaacctggtgtccgtcggccagggcgagacaacaaagcctgacgtgatcctgcggctggaacagggcaaagagccttggctggaagaggaagaggtgctcggatctggcagagccgagaagaatggcgatatcggcggacagatctggaagccaaaggatgtgaaagagagtctcggaagcggagctactaacttcagcctgctgaagcaggctggagacgtggaggagaaccctggacctatgcctgctgctaagagagtgaaactggatggatccaaccatgaccaggaatttgaccccccaaaggtttacccacctgtgccagctgagaagaggaagcccatccgcgtgctgtctctctttgatgggattgctacagggctcctggtgctgaaggacctgggcatccaagtggaccgctacattgcctccgaggtgtgtgaggactccatcacggtgggcatggtgcggcaccagggaaagatcatgtacgtcggggacgtccgcagcgtcacacagaagcatatccaggagtggggcccattcgacctggtgattggaggcagtccctgcaatgacctctccattgtcaaccctgcccgcaagggactttatgagggtactggccgcctcttctttgagttctaccgcctcctgcatgatgcgcggcccaaggagggagatgatcgccccttcttctggctctttgagaatgtggtggccatgggcgttagtgacaagagggacatctcgcgatttcttgagtctaaccccgtgatgattgacgccaaagaagtgtctgctgcacacagggcccgttacttctggggtaaccttcctggcatgaacaggcctttggcatccactgtgaatgataagctggagctgcaagagtgtctggagcacggcagaatagccaagttcagcaaagtgaggaccattaccaccaggtcaaactctataaagcagggcaaagaccagcatttccccgtgttcatgaacgagaaggaggacatcctgtggtgcactgaaatggaaagggtgtttggcttccccgtccactacacagacgtctccaacatgagccgcttggcgaggcagagactgctgggccgatcgtggagcgtgccggtcatccgccacctcttcgctccgctgaaggaatattttgcttgtgtgtctagcggcaatagtaacgctaacagccgcgggccgagcttcagcagcggcctggtgccgttaagcttgcgcggcagccatatgttcgaaaccgtgcctgtgtggaggagacagccagtccgggtgctgtccctttttgaagacatcaagaaagagctgacgagtttgggctttttggaaagtggttctgacccgggacaactgaagcatgtggttgatgtcacagacacagtgaggaaggatgtggaggagtggggacccttcgatcttgtgtacggcgccacacctcccctgggccacacctgtgaccgtcctcccagctggtacctgttccagttccaccggctcctgcagtacgcacggcccaagccaggcagccccaggcccttcttctggatgttcgtggacaatctggtgctgaacaaggaagacctggacgtcgcatctcgcttcctggagatggagccagtcaccatcccagatgtccacggcggatccttgcagaatgctgtccgcgtgtggagcaacatcccagccataaggagcagcaggcactgggctctggtttcggaagaagaattgtccctgctggcccagaacaagcagagctcgaagctcgcggccaagtggcccaccaagctggtgaagaactgctttctccccctaagagaatatttcaagtatttttcaggagggccgagctctggcgcacccccaccaagtggagggtctcctgccgggtccccaacatctactgaagaaggcaccagcgaatccgcaacgcccgagtcaggccctggtacctccacagaaccatctgaaggtagtgcgcctggttccccagctggaagccctacttccaccgaagaaggcacgtcaaccgaaccaagtgaaggatctgcccctgggaccagcactgaaccatctgagccaaaaaagaagagaaaggtaatgtcaaagctggagaaattcaccaactgttatagcctgtctaagaccctgcgcttcaaggcaatcccagtgggcaagacacaagagaacattgacaacaaacggctcctggtggaggatgagaagagggctgaagattacaagggcgttaagaagctgctggataggtactatctgtcattcatcaacgatgtcctccacagtatcaagctgaagaatctgaacaattacatttctctgttccggaagaagacacggaccgagaaggagaacaaagagctggagaatctggagatcaacctgaggaaagaaatagctaaggctttcaaagggaacgagggttacaagtccctgttcaagaaagacattatcgagactattctgcctgagttcctggacgataaagatgagatcgccctcgtcaattccttcaatgggtttaccacagcctttaccggcttcttcgacaatagagagaatatgttctctgaagaggccaaatccactagcatcgcctttcgctgcataaacgagaacctgactaggtacatcagcaatatggacatctttgagaaagtcgatgccatattcgacaaacatgaggtgcaggagattaaggagaagatcctgaactcagattacgatgtcgaagatttcttcgagggagagttcttcaacttcgtgctcacacaagagggcattgatgtgtacaatgcaatcattggagggttcgtgacagagagtggcgagaagataaagggcctgaacgagtatatcaacctctacaaccagaaaaccaagcagaaactgcctaagttcaagccactgtacaaacaagtgctctcagatagggaaagcctgagcttctacggtgaagggtatacatcagatgaagaagtgctcgaagtgttccgcaacaccctcaataagaacagtgaaatcttctcttcaatcaagaagctggagaaactgttcaagaatttcgatgagtactcctctgccggaatctttgtgaagaatggccctgcaatatccactattagcaaagacatctttggcgagtggaacgttatcagggataagtggaatgccgagtacgatgatattcatctcaagaagaaagccgtggttacagagaaatacgaggatgatagacgcaagagctttaagaagattggtagcttctctctcgaacagctgcaggagtacgccgacgctgacctgtcagtcgtggagaaactcaaggagatcataatccagaaggtggatgaaatctacaaagtgtatggaagctctgagaaactcttcgatgcagactttgttctggagaagagtctgaagaagaacgacgcagtggttgctatcatgaaggacctgctggattctgttaagtctttcgagaattacattaaggcattctttggtgaagggaaggagacaaatagggacgagagcttctatggcgactttgttctggcctacgacatcctcctcaaggttgaccacatctatgacgctatacggaattacgttacccagaagccctatagcaaagacaagttcaagctgtatttccagaatccacagtttatgggtgggtgggataaagacaaagaaacagattacagggccactatcctgcggtacggcagcaaatactatctggctatcatggataagaagtacgccaaatgcctccagaagatcgacaaggacgacgtgaacggtaactacgagaagatcaattacaagctcctgccaggacctaacaagatgctgcccaaggtgttcttctccaagaaatggatggcctactataacccaagcgaggacattcagaagatatacaagaatgggacattcaagaagggcgatatgttcaacctcaacgactgccacaagctgattgatttcttcaaggatagcatttctcgctatcccaagtggtctaatgcatacgatttcaacttcagcgagactgagaagtacaaagacatcgctggcttctaccgggaggtggaagagcaaggctataaggtgtcattcgaatccgcttctaagaaggaagtggataagctcgtggaagagggtaagctgtacatgttccagatatacaacaaagacttcagcgataagagccacggcactccaaacctccatactatgtatttcaagctgctgtttgacgagaacaaccacggacagattaggctgtcaggaggcgcagaactcttcatgcgcagagcttcactgaagaaggaggaactcgttgtccacccagccaatagccctatagccaataagaatccagacaatcctaagaaaaccactactctgtcttacgatgtgtataaggataagagattctctgaagatcagtacgaactgcacatacccattgccattaacaagtgccctaagaacatcttcaagattaacacagaggttagagtgctcctgaaacacgacgataacccttatgttataggcattgctcgcggagagagaaacctgctgtacatcgtcgtggtggacggcaaaggcaacatcgtggaacagtacagtctcaatgaaatcattaacaatttcaacggaatccgcattaagaccgactaccattctctcctcgacaagaaggagaaagaaaggttcgaagcaagacagaattggacaagtatagagaatatcaaagaactgaaggctgggtacatctctcaggttgtgcacaagatatgtgagctggtggagaagtacgacgctgttatcgccctcgcggacctgaatagcggcttcaagaactccagggtgaaggtggagaagcaggtgtatcagaagttcgagaagatgctgatcgacaagctcaactatatggtggacaagaaatccaatccttgcgctactggtggagccctgaagggctatcaaatcaccaataagttcgaatctttcaagtctatgagcacccagaatggcttcatcttctacatacccgcatggctgacatccaagattgatccctctaccggatttgttaatctgctcaagactaagtacacctctattgctgactcaaagaagttcatatcatcatttgaccgcatcatgtacgtgccagaagaggacctgttcgagtttgccctggattacaagaatttctctcggactgacgccgactacatcaagaagtggaagctctactcttatggtaatcggattcgcatattccgcaatcccaagaagaataacgtgttcgattgggaggaagtttgcctcaccagcgcttacaaggagctgttcaataagtatgggattaactaccagcagggcgacataagagccctgctgtgcgaacaatctgataaggcattctattcctctttcatggcactgatgtcactgatgctgcaaatgcgcaattccatcaccggaagaacagacgtggcctttctgatctctcctgtcaagaactcagatggcatcttctacgattcccgcaactatgaagcacaggagaatgctatcctgcctaagaatgccgatgcaaatggagcctataacatcgccagaaaggtcctctgggccataggacaattcaagaaagctgaagatgagaagctggacaaggtgaagatcgccatttcaaacaaagagtggctcgaatatgctcagacctcagtgaagcatgcctatccctatgacgtgcccgattatgccagcctgggcagcggctcccccaagaaaaaacgcaaggtggaagatcctaagaaaaagcggaaagtggacggcattggtagtgggagcaacggcagcagcggagaggaactgctgagcaagaactaccacctggaaaacgaggtggccagactgaagaaaggctctggctctggcggaagcggttctggcggatcaggatctggaagtggcggctctggaagcggaggttctggatctggcgaagaactgctgtctaagaattatcacggttcaggctccggccagcggggaagcaagcgcaccgccgatggttccgagttcgaaagccccaaaaaaaagcgcaaggtctga

SEQ ID NO: 307 - DNA, 6561 bp, synthetic construct
  misc_feature 1..6561: note = CDS of V19_scFv-ZIM3-2a-D3a-hD3L-dCas12i-1xGCN4
  source 1..6561: mol_type = other DNA
atgcctgctgctaagagagtgaaactggatggatccggccccgacatcgtgatgacccagagccccagcagcctgagcgccagcgtgggcgaccgcgtgaccatcacctgccgcagcagcaccggcgccgtgaccaccagcaactacgccagctgggtgcaggagaagcccggcaagctgttcaagggcctgatcggcggcaccaacaaccgcgcccccggcgtgcccagccgcttcagcggcagcctgatcggcgacaaggccaccctgaccatcagcagcctgcagcccgaggacttcgccacctacttctgcgccctgtggtacagcaaccactgggtgttcggccagggcaccaaggtggagctgaagcgcggcggcggcggcagcggcggcggcggcagcggcggcggcggcagcagcggcggcggcagcgaggtgaagctgctggagagcggcggcggcctggtgcagcccggcggcagcctgaagctgagctgcgccgtgagcggcttcagcctgaccgactacggcgtgaactgggtgcgccaggcccccggccgcggcctggagtggatcggcgtgatctggggcgacggcatcaccgactacaacagcgccctgaaggaccgcttcatcatcagcaaggacaacggcaagaacaccgtgtacctgcagatgagcaaggtgcgcagcgacgacaccgccctgtactactgcgtgaccggcctgttcgactactggggccagggcaccctggtgaccgtgagcagctacccatacgatgttccagattacgctggtggaggcggaggttctgggggaggaggtagtggcggtggtggttcaggaggcggcggaagcttggatccaggtggaggtggaagcggtatgaacaattcccagggaagagtgaccttcgaggacgtgaccgtgaacttcacccaaggcgagtggcagagactgaaccccgagcagagaaacctgtaccgggacgtgatgctggaaaactacagcaacctggtgtccgtcggccagggcgagacaacaaagcctgacgtgatcctgcggctggaacagggcaaagagccttggctggaagaggaagaggtgctcggatctggcagagccgagaagaatggcgatatcggcggacagatctggaagccaaaggatgtgaaagagagtctcggaagcggagctactaacttcagcctgctgaagcaggctggagacgtggaggagaaccctggacctatgcctgctgctaagagagtgaaactggatggatccaaccatgaccaggaatttgaccccccaaaggtttacccacctgtgccagctgagaagaggaagcccatccgcgtgctgtctctctttgatgggattgctacagggctcctggtgctgaaggacctgggcatccaagtggaccgctacattgcctccgaggtgtgtgaggactccatcacggtgggcatggtgcggcaccagggaaagatcatgtacgtcggggacgtccgcagcgtcacacagaagcatatccaggagtggggcccattcgacctggtgattggaggcagtccctgcaatgacctctccattgtcaaccctgcccgcaagggactttatgagggtactggccgcctcttctttgagttctaccgcctcctgcatgatgcgcggcccaaggagggagatgatcgccccttcttctggctctttgagaatgtggtggccatgggcgttagtgacaagagggacatctcgcgatttcttgagtctaaccccgtgatgattgacgccaaagaagtgtctgctgcacacagggcccgttacttctggggtaaccttcctggcatgaacaggcctttggcatccactgtgaatgataagctggagctgcaagagtgtctggagcacggcagaatagccaagttcagcaaagtgaggaccattaccaccaggtcaaactctataaagcagggcaaagaccagcatttccccgtgttcatgaacgagaaggaggacatcctgtggtgcactgaaatggaaagggtgtttggcttccccgtccactacacagacgtctccaacatgagccgcttggcgaggcagagactgctgggccgatcgtggagcgtgccggtcatccgccacctcttcgctccgctgaaggaatattttgcttgtgtgtctagcggcaatagtaacgctaacagccgcgggccgagcttcagcagcggcctggtgccgttaagcttgcgcggcagccatatgttcgaaaccgtgcctgtgtggaggagacagccagtccgggtgctgtccctttttgaagacatcaagaaagagctgacgagtttgggctttttggaaagtggttctgacccgggacaactgaagcatgtggttgatgtcacagacacagtgaggaaggatgtggaggagtggggacccttcgatcttgtgtacggcgccacacctcccctgggccacacctgtgaccgtcctcccagctggtacctgttccagttccaccggctcctgcagtacgcacggcccaagccaggcagccccaggcccttcttctggatgttcgtggacaatctggtgctgaacaaggaagacctggacgtcgcatctcgcttcctggagatggagccagtcaccatcccagatgtccacggcggatccttgcagaatgctgtccgcgtgtggagcaacatcccagccataaggagcagcaggcactgggctctggtttcggaagaagaattgtccctgctggcccagaacaagcagagctcgaagctcgcggccaagtggcccaccaagctggtgaagaactgctttctccccctaagagaatatttcaagtatttttcaggagggccgagctctggcgcacccccaccaagtggagggtctcctgccgggtccccaacatctactgaagaaggcaccagcgaatccgcaacgcccgagtcaggccctggtacctccacagaaccatctgaaggtagtgcgcctggttccccagctggaagccctacttccaccgaagaaggcacgtcaaccgaaccaagtgaaggatctgcccctgggaccagcactgaaccatctgagccaaaaaagaagagaaaggtaatgggcatcaccatgagcgacaccaccttcagaccctacaagagcaagctgaaccccaacgagcggaagatgcctatggtggtggacaccatgaattggtgcgacaacgcctgcagcgtgttcttcgatctgttcgtgggcctgtacggcggcgtgaagatcggcgacgtgaccaatttcctgaccgagaagcaggacaccaccaccgatgccgatctgctgtgcgccatcaactggttcagagccatgcctgtgtctaaccccgatgccgttgtgggacctgagcagctggttgtgcggttcagagactacagcggccacaatccatctccaatggccagcatgtacctgagcgcccctgtgaaccctagatacacctgggtcgactgccggttcctgtaccagcagatgtgtcagaccctgggcgccaacctggatgtggacatctctaccctggtgcagaccggcctgctgcctatccagaaggatacacagctgaacgcctacagcttctgcagcaacgtgttcggcgagggcgtgaaagaagatcccagcgccaaagtgaccagctacacagccgctgccaatgctctgagcggcgccaccaatcctatcatcacctacgaggactaccggcagatcctgtccagcgccatcaccaacagacccagcagaaagggcgccaaggatattctggccgccgatctggatagcaccaagacaggtgttctgcccggcaactacgtgtcccagagaatcgccatgtaccaggcctctgccgcctctaaagctagaggcgtggtgctgcccaaccggctgagagtgaaagcctacctgcagaacctcgtgggactgaactacatctgcaccacctgggccgctcctatgctgagagccgtgggcgacatcaagagcaagaacagcaacaactaccgcttcgtgggcgagagactggaacggcagcaagagatcgataacctgctggccgtgtccaacatcagaagcgcccaggccatcctgcagcagttcagggccaatgagagcaaccagttctacatcaagaagcggcacatcggcaagggcctgcctagcctgtacgacatgtgggatctgatggacgagaaagagggcatcgacaactacatccagagcctgaagggcgacaagaccgagaggctgccaatcagagagctgctgcagatcatctaccctcacagaaagagcgtgtccgccgagctgtttctgtctgccgccgaactgaccgacgtggaagatagacagaaccggtgcatggtgcaccctacagtgcggggctctctggtcatcaacttcggcaagagcagcaccatcttcggcgctatcacccctcctgacacactgatcaagttccggggcgaaatggtgcctgctggacagacaggcatgatctggttcacaatgcacctggtggacggcggcaaatgggtcaagcaccacattccttgccacagcagccggtacttcgaggaaatctacgcctggaagaaggacctgcctacactgccctttccacggcggagcctgtatggctatgccatcggcaacaagatcagcgacacccggaagatcgacctgcggagaaagaaggccagcaagcagtacctgcggaccctggaaaacatgacccacaacgtggaatttgaccccaccacacagttcatggtggaccaagagctgaacgtgaccatcaccgccagagtgaagaaaatccctcctgtgcgggatgtgcccgtgggcagcagaattatgggcctgaacaagaaccagaccatccgggactgctacagcatctgggagagagtggaagccaacaccagcggcagctttcagcatcccgtggtccaggatgtgtggctgagactggtggccgatggccacgtgacctctacagtgaatggccccaacggccagatcgaccagatgagctactctggccccgatgtggccaactgcggcaactggatgcaagagcggagcaacttcatcaccagcgtggacgacgccgaccagtctatcatgaagcactttctgtggaacaaccgcgtgaagctgtatgcctggaactgcgtgtacgccggcacactgatgaaggccatctctaagcagatgaccaccgccaaccggaacctgttcagaaacgagatcctgagcttcgttggcggcagattcggctgcagactgggatctctggcccaggtttcactggacctgctgcggaggatgaagtccgtgatcagctgctacttcagccggaacaacgccttcaccatcgaggaaagaagcgccttcgacaaagaactgatggaactgttcgagagcctggacaacaagatgaacaacaagcggaaagagaaagtcaaccggacactcagcagcatcttccaggtggccaagcagcacaatgttgtgcggctggtggtcaccaagaacctgcagacccctgatgccaatgtgcggagcgtgatgaatcagagatccgtggattggtgcgctcggaagattgaagagaagatcgtggacctgggcaacgtgatcggaatctatgtggatctggtggaagccctggatctgagccatctggaccccttcatctatatcgccaagggcgacgtgggcaaagagtgccagtttgacgaggtggaaagcagctccctgctgccaattcacaccagcatgtttcgcgactggcacggcctggttaacaagggcagaaccaccacacctatctaccacagcgccctgaggagcttcgccagccactacggcctgagattcgatgacctggccagaatcaaggccgctgagctggccaaaatgctgccagaccagaaggtgttcatcccacacagaggcggacggttcttcatgagcacataccccgtgaccagcaccagcagacccgtgtcttatgatggccggcagcggttcctgaacagcggcgatatggtggccccagtgaacaccatgctgcgcggattcagaagggccagatctgcctatccctatgacgtgcccgattatgccagcctgggcagcggctcccccaagaaaaaacgcaaggtggaagatcctaagaaaaagcggaaagtggacggcattggtagtgggagcaacggcagcagcggagaggaactgctgagcaagaactaccacctggaaaacgaggtggccagactgaagaaaggctctggctctggcggaagcggttctggcggatcaggatctggaagtggcggctctggaagcggaggttctggatctggcgaagaactgctgtctaagaattatcacggttcaggctccggccagcggggaagcaagcgcaccgccgatggttccgagttcgaaagccccaaaaaaaagcgcaaggtctga

SEQ ID NO: 308 - DNA, 7533 bp, synthetic construct
  misc_feature 1..7533: note = CDS of V20_KRAB-scFv-2a-D3a-D3l-dCas9-2xGCN4
  source 1..7533: mol_type = other DNA
atgcctgctgctaagagagtgaaactggatggatcccggacactggtgaccttcaaggatgtatttgtggacttcaccagggaggagtggaagctgctggacactgctcagcagatcgtgtacagaaatgtgatgctggagaactataagaacctggtttccttgggttatcagcttactaagccagatgtgatcctccggttggagaagggagaagagcccggaagcggaatgggccccgacatcgtgatgacccagagccccagcagcctgagcgccagcgtgggcgaccgcgtgaccatcacctgccgcagcagcaccggcgccgtgaccaccagcaactacgccagctgggtgcaggagaagcccggcaagctgttcaagggcctgatcggcggcaccaacaaccgcgcccccggcgtgcccagccgcttcagcggcagcctgatcggcgacaaggccaccctgaccatcagcagcctgcagcccgaggacttcgccacctacttctgcgccctgtggtacagcaaccactgggtgttcggccagggcaccaaggtggagctgaagcgcggcggcggcggcagcggcggcggcggcagcggcggcggcggcagcagcggcggcggcagcgaggtgaagctgctggagagcggcggcggcctggtgcagcccggcggcagcctgaagctgagctgcgccgtgagcggcttcagcctgaccgactacggcgtgaactgggtgcgccaggcccccggccgcggcctggagtggatcggcgtgatctggggcgacggcatcaccgactacaacagcgccctgaaggaccgcttcatcatcagcaaggacaacggcaagaacaccgtgtacctgcagatgagcaaggtgcgcagcgacgacaccgccctgtactactgcgtgaccggcctgttcgactactggggccagggcaccctggtgaccgtgagcagctacccatacgatgttccagattacgctggtggaggcggaggttctgggggaggaggtagtggcggtggtggttcaggaggcggcggaagcggaagcggagctactaacttcagcctgctgaagcaggctggagacgtggaggagaaccctggacctatgcctgctgctaagagagtgaaactggatggatccaaccatgaccaggaatttgaccccccaaaggtttacccacctgtgccagctgagaagaggaagcccatccgcgtgctgtctctctttgatgggattgctacagggctcctggtgctgaaggacctgggcatccaagtggaccgctacattgcctccgaggtgtgtgaggactccatcacggtgggcatggtgcggcaccagggaaagatcatgtacgtcggggacgtccgcagcgtcacacagaagcatatccaggagtggggcccattcgacctggtgattggaggcagtccctgcaatgacctctccattgtcaaccctgcccgcaagggactttatgagggtactggccgcctcttctttgagttctaccgcctcctgcatgatgcgcggcccaaggagggagatgatcgccccttcttctggctctttgagaatgtggtggccatgggcgttagtgacaagagggacatctcgcgatttcttgagtctaaccccgtgatgattgacgccaaagaagtgtctgctgcacacagggcccgttacttctggggtaaccttcctggcatgaacaggcctttggcatccactgtgaatgataagctggagctgcaagagtgtctggagcacggcagaatagccaagttcagcaaagtgaggaccattaccaccaggtcaaactctataaagcagggcaaagaccagcatttccccgtgttcatgaacgagaaggaggacatcctgtggtgcactgaaatggaaagggtgtttggcttccccgtccactacacagacgtctccaacatgagccgcttggcgaggcagagactgctgggccgatcgtggagcgtgccggtcatccgccacctcttcgctccgctgaaggaatattttgcttgtgtgtctagcggcaatagtaacgctaacagccgcgggccgagcttcagcagcggcctggtgccgttaagcttgcgcggcagccatatgttcgaaaccgtgcctgtgtggaggagacagccagtccgggtgctgtccctttttgaagacatcaagaaagagctgacgagtttgggctttttggaaagtggttctgacccgggacaactgaagcatgtggttgatgtcacagacacagtgaggaaggatgtggaggagtggggacccttcgatcttgtgtacggcgccacacctcccctgggccacacctgtgaccgtcctcccagctggtacctgttccagttccaccggctcctgcagtacgcacggcccaagccaggcagccccaggcccttcttctggatgttcgtggacaatctggtgctgaacaaggaagacctggacgtcgcatctcgcttcctggagatggagccagtcaccatcccagatgtccacggcggatccttgcagaatgctgtccgcgtgtggagcaacatcccagccataaggagcagcaggcactgggctctggtttcggaagaagaattgtccctgctggcccagaacaagcagagctcgaagctcgcggccaagtggcccaccaagctggtgaagaactgctttctccccctaagagaatatttcaagtatttttcaggagggccgagctctggcgcacccccaccaagtggagggtctcctgccgggtccccaacatctactgaagaaggcaccagcgaatccgcaacgcccgagtcaggccctggtacctccacagaaccatctgaaggtagtgcgcctggttccccagctggaagccctacttccaccgaagaaggcacgtcaaccgaaccaagtgaaggatctgcccctgggaccagcactgaaccatctgagccaaaaaagaagagaaaggtaatggacaagaagtacagcatcggcctggccatcggcaccaactctgtgggctgggccgtgatcaccgacgagtacaaggtgcccagcaagaaattcaaggtgctgggcaacaccgaccggcacagcatcaagaagaacctgatcggcgccctgctgttcgacagcggagaaacagccgaggccacccggctgaagagaaccgccagaagaagatacaccagacggaagaaccggatctgctatctgcaagagatcttcagcaacgagatggccaaggtggacgacagcttcttccacagactggaagagtccttcctggtggaagaggataagaagcacgagcggcaccccatcttcggcaacatcgtggacgaggtggcctaccacgagaagtaccccaccatctaccacctgagaaagaaactggtggacagcaccgacaaggccgacctgcggctgatctatctggccctggcccacatgatcaagttccggggccacttcctgatcgagggcgacctgaaccccgacaacagcgacgtggacaagctgttcatccagctggtgcagacctacaaccagctgttcgaggaaaaccccatcaacgccagcggcgtggacgccaaggccatcctgtctgccagactgagcaagagcagacggctggaaaatctgatcgcccagctgcccggcgagaagaagaatggcctgttcggcaacctgattgccctgagcctgggcctgacccccaacttcaagagcaacttcgacctggccgaggatgccaaactgcagctgagcaaggacacctacgacgacgacctggacaacctgctggcccagatcggcgaccagtacgccgacctgtttctggccgccaagaacctgtccgacgccatcctgctgagcgacatcctgagagtgaacaccgagatcaccaaggcccccctgagcgcctctatgatcaagagatacgacgagcaccaccaggacctgaccctgctgaaagctctcgtgcggcagcagctgcctgagaagtacaaagagattttcttcgaccagagcaagaacggctacgccggctacatcgatggcggagccagccaggaagagttctacaagttcatcaagcccatcctggaaaagatggacggcaccgaggaactgctcgtgaagctgaacagagaggacctgctgcggaagcagcggaccttcgacaacggcagcatcccccaccagatccacctgggagagctgcacgccattctgcggcggcaggaagatttttacccattcctgaaggacaaccgggaaaagatcgagaagatcctgaccttccgcatcccctactacgtgggccctctggccaggggaaacagcagattcgcctggatgaccagaaagagcgaggaaaccatcaccccctggaacttcgaggaagtggtggacaagggcgccagcgcccagagcttcatcgagcggatgaccaacttcgataagaacctgcccaacgagaaggtgctgcccaagcacagcctgctgtacgagtacttcaccgtgtacaacgagctgaccaaagtgaaatacgtgaccgagggaatgagaaagcccgccttcctgagcggcgagcagaaaaaagccatcgtggacctgctgttcaagaccaaccggaaagtgaccgtgaagcagctgaaagaggactacttcaagaaaatcgagtgcttcgactccgtggaaatctccggcgtggaagatcggttcaacgcctccctgggcacataccacgatctgctgaaaattatcaaggacaaggacttcctggacaatgaggaaaacgaggacattctggaagatatcgtgctgaccctgacactgtttgaggacagagagatgatcgaggaacggctgaaaacctatgcccacctgttcgacgacaaagtgatgaagcagctgaagcggcggagatacaccggctggggcaggctgagccggaagctgatcaacggcatccgggacaagcagtccggcaagacaatcctggatttcctgaagtccgacggcttcgccaacagaaacttcatgcagctgatccacgacgacagcctgacctttaaagaggacatccagaaagcccaggtgtccggccagggcgatagcctgcacgagcacattgccaatctggccggcagccccgccattaagaagggcatcctgcagacagtgaaggtggtggacgagctcgtgaaagtgatgggccggcacaagcccgagaacatcgtgatcgaaatggccagagagaaccagaccacccagaagggacagaagaacagccgcgagagaatgaagcggatcgaagagggcatcaaagagctgggcagccagatcctgaaagaacaccccgtggaaaacacccagctgcagaacgagaagctgtacctgtactacctgcagaatgggcgggatatgtacgtggaccaggaactggacatcaaccggctgtccgactacgatgtggacgctatcgtgcctcagagctttctgaaggacgactccatcgataacaaagtgctgactcggagcgacaagaaccggggcaagagcgacaacgtgccctccgaagaggtcgtgaagaagatgaagaactactggcgccagctgctgaatgccaagctgattacccagaggaagttcgacaatctgaccaaggccgagagaggcggcctgagcgaactggataaggccggcttcatcaagagacagctggtggaaacccggcagatcacaaagcacgtggcacagatcctggactcccggatgaacactaagtacgacgagaacgacaaactgatccgggaagtgaaagtgatcaccctgaagtccaagctggtgtccgatttccggaaggatttccagttttacaaagtgcgcgagatcaacaactaccaccacgcccacgacgcctacctgaacgccgtcgtgggaaccgccctgatcaaaaagtaccctaagctggaaagcgagttcgtgtacggcgactacaaggtgtacgacgtgcggaagatgatcgccaagagcgagcaggaaatcggcaaggctaccgccaagtacttcttctacagcaacatcatgaactttttcaagaccgagattaccctggccaacggcgagatccggaagcggcctctgatcgagacaaacggcgaaacaggcgagatcgtgtgggataagggccgggactttgccaccgtgcggaaagtgctgtctatgccccaagtgaatatcgtgaaaaagaccgaggtgcagacaggcggcttcagcaaagagtctatcctgcccaagaggaacagcgacaagctgatcgccagaaagaaggactgggaccctaagaagtacggcggcttcgacagccccaccgtggcctattctgtgctggtggtggccaaagtggaaaagggcaagtccaagaaactgaagagtgtgaaagagctgctggggatcaccatcatggaaagaagcagcttcgagaagaatcccatcgactttctggaagccaagggctacaaagaagtgaaaaaggacctgatcatcaagctgcctaagtactccctgttcgagctggaaaacggccggaagagaatgctggcctctgccggcgaactgcagaagggaaacgaactggccctgccctccaaatatgtgaacttcctgtacctggccagccactatgagaagctgaagggctcccccgaggataatgagcagaaacagctgtttgtggaacagcacaaacactacctggacgagatcatcgagcagatcagcgagttctccaagagagtgatcctggccgacgctaatctggacaaggtgctgagcgcctacaacaagcacagagacaagcctatcagagagcaggccgagaatatcatccacctgtttaccctgaccaatctgggagcccctgccgccttcaagtactttgacaccaccatcgaccggaagaggtacaccagcaccaaagaggtgctggacgccaccctgatccaccagagcatcaccggcctgtacgagacacggatcgacctgtctcagctgggaggcgacgcctatccctatgacgtgcccgattatgccagcctgggcagcggctcccccaagaaaaaacgcaaggtggaagatcctaagaaaaagcggaaagtggacggcattggtagtgggagcaacggcagcagcggagaggaactgctgagcaagaactaccacctggaaaacgaggtggccagactgaagaaaggctctggctctggcggaagcggttctggcggatcaggatctggaagtggcggctctggaagcggaggttctggatctggcgaagaactgctgtctaagaattatcacctcgagaatgaagtcgctcgtttgaagaaaggttcaggctccggccagcggggaagcaagcgcaccgccgatggttccgagttcgaaagccccaaaaaaaagcgcaaggtctga

SEQ ID NO: 309 - DNA, 8250 bp, synthetic construct
  misc_feature 1..8250: note = CDS of V21_hSIRT1-scFv-2a-D3a-D3l-dCas9-2xGCN4
  source 1..8250: mol_type = other DNA
atgcctgctgctaagagagtgaaactggatggatccacaattcttaaagatttattgccggaaacaatacctccacctgagttggatgatatgacactgtggcagattgttattaatatcctttcagaaccaccaaaaaggaaaaaaagaaaagatattaatacaattgaagatgctgtgaaattactgcaagagtgcaaaaaaattatagttctaactggagctggggtgtctgtttcatgtggaatacctgacttcaggtcaagggatggtatttatgctcgccttgctgtagacttcccagatcttccagatcctcaagcgatgtttgatattgaatatttcagaaaagatccaagaccattcttcaagtttgcaaaggaaatatatcctggacaattccagccatctctctgtcacaaattcatagccttgtcagataaggaaggaaaactacttcgcaactatacccagaacatagacacgctggaacaggttgcgggaatccaaaggataattcagtgtcatggttcctttgcaacagcatcttgcctgatttgtaaatacaaagttgactgtgaagctgtacgaggagatatttttaatcaggtagttcctcgatgtcctaggtgcccagctgatgaaccgcttgctatcatgaaaccagagattgtgttttttggtgaaaatttaccagaacagtttcatagagccatgaagtatgacaaagatgaagttgacctcctcattgttattgggtcttccctcaaagtaagaccagtagcactaattccaagttccataccccatgaagtgcctcagatattaattaatagagaacctttgcctcatctgcattttgatgtagagcttcttggagactgtgatgtcataattaatgaattgtgtcataggttaggtggtgaatatgccaaacttggaagcggaatgggccccgacatcgtgatgacccagagccccagcagcctgagcgccagcgtgggcgaccgcgtgaccatcacctgccgcagcagcaccggcgccgtgaccaccagcaactacgccagctgggtgcaggagaagcccggcaagctgttcaagggcctgatcggcggcaccaacaaccgcgcccccggcgtgcccagccgcttcagcggcagcctgatcggcgacaaggccaccctgaccatcagcagcctgcagcccgaggacttcgccacctacttctgcgccctgtggtacagcaaccactgggtgttcggccagggcaccaaggtggagctgaagcgcggcggcggcggcagcggcggcggcggcagcggcggcggcggcagcagcggcggcggcagcgaggtgaagctgctggagagcggcggcggcctggtgcagcccggcggcagcctgaagctgagctgcgccgtgagcggcttcagcctgaccgactacggcgtgaactgggtgcgccaggcccccggccgcggcctggagtggatcggcgtgatctggggcgacggcatcaccgactacaacagcgccctgaaggaccgcttcatcatcagcaaggacaacggcaagaacaccgtgtacctgcagatgagcaaggtgcgcagcgacgacaccgccctgtactactgcgtgaccggcctgttcgactactggggccagggcaccctggtgaccgtgagcagctacccatacgatgttccagattacgctggtggaggcggaggttctgggggaggaggtagtggcggtggtggttcaggaggcggcggaagcggaagcggagctactaacttcagcctgctgaagcaggctggagacgtggaggagaaccctggacctatgcctgctgctaagagagtgaaactggatggatccaaccatgaccaggaatttgaccccccaaaggtttacccacctgtgccagctgagaagaggaagcccatccgcgtgctgtctctctttgatgggattgctacagggctcctggtgctgaaggacctgggcatccaagtggaccgctacattgcctccgaggtgtgtgaggactccatcacggtgggcatggtgcggcaccagggaaagatcatgtacgtcggggacgtccgcagcgtcacacagaagcatatccaggagtggggcccattcgacctggtgattggaggcagtccctgcaatgacctctccattgtcaaccctgcccgcaagggactttatgagggtactggccgcctcttctttgagttctaccgcctcctgcatgatgcgcggcccaaggagggagatgatcgccccttcttctggctctttgagaatgtggtggccatgggcgttagtgacaagagggacatctcgcgatttcttgagtctaaccccgtgatgattgacgccaaagaagtgtctgctgcacacagggcccgttacttctggggtaaccttcctggcatgaacaggcctttggcatccactgtgaatgataagctggagctgcaagagtgtctggagcacggcagaatagccaagttcagcaaagtgaggaccattaccaccaggtcaaactctataaagcagggcaaagaccagcatttccccgtgttcatgaacgagaaggaggacatcctgtggtgcactgaaatggaaagggtgtttggcttccccgtccactacacagacgtctccaacatgagccgcttggcgaggcagagactgctgggccgatcgtggagcgtgccggtcatccgccacctcttcgctccgctgaaggaatattttgcttgtgtgtctagcggcaatagtaacgctaacagccgcgggccgagcttcagcagcggcctggtgccgttaagcttgcgcggcagccatatgttcgaaaccgtgcctgtgtggaggagacagccagtccgggtgctgtccctttttgaagacatcaagaaagagctgacgagtttgggctttttggaaagtggttctgacccgggacaactgaagcatgtggttgatgtcacagacacagtgaggaaggatgtggaggagtggggacccttcgatcttgtgtacggcgccacacctcccctgggccacacctgtgaccgtcctcccagctggtacctgttccagttccaccggctcctgcagtacgcacggcccaagccaggcagccccaggcccttcttctggatgttcgtggacaatctggtgctgaacaaggaagacctggacgtcgcatctcgcttcctggagatggagccagtcaccatcccagatgtccacggcggatccttgcagaatgctgtccgcgtgtggagcaacatcccagccataaggagcagcaggcactgggctctggtttcggaagaagaattgtccctgctggcccagaacaagcagagctcgaagctcgcggccaagtggcccaccaagctggtgaagaactgctttctccccctaagagaatatttcaagtatttttcaggagggccgagctctggcgcacccccaccaagtggagggtctcctgccgggtccccaacatctactgaagaaggcaccagcgaatccgcaacgcccgagtcaggccctggtacctccacagaaccatctgaaggtagtgcgcctggttccccagctggaagccctacttccaccgaagaaggcacgtcaaccgaaccaagtgaaggatctgcccctgggaccagcactgaaccatctgagccaaaaaagaagagaaaggtaatggacaagaagtacagcatcggcctggccatcggcaccaactctgtgggctgggccgtgatcaccgacgagtacaaggtgcccagcaagaaattcaaggtgctgggcaacaccgaccggcacagcatcaagaagaacctgatcggcgccctgctgttcgacagcggagaaacagccgaggccacccggctgaagagaaccgccagaagaagatacaccagacggaagaaccggatctgctatctgcaagagatcttcagcaacgagatggccaaggtggacgacagcttcttccacagactggaagagtccttcctggtggaagaggataagaagcacgagcggcaccccatcttcggcaacatcgtggacgaggtggcctaccacgagaagtaccccaccatctaccacctgagaaagaaactggtggacagcaccgacaaggccgacctgcggctgatctatctggccctggcccacatgatcaagttccggggccacttcctgatcgagggcgacctgaaccccgacaacagcgacgtggacaagctgttcatccagctggtgcagacctacaaccagctgttcgaggaaaaccccatcaacgccagcggcgtggacgccaaggccatcctgtctgccagactgagcaagagcagacggctggaaaatctgatcgcccagctgcccggcgagaagaagaatggcctgttcggcaacctgattgccctgagcctgggcctgacccccaacttcaagagcaacttcgacctggccgaggatgccaaactgcagctgagcaaggacacctacgacgacgacctggacaacctgctggcccagatcggcgaccagtacgccgacctgtttctggccgccaagaacctgtccgacgccatcctgctgagcgacatcctgagagtgaacaccgagatcaccaaggcccccctgagcgcctctatgatcaagagatacgacgagcaccaccaggacctgaccctgctgaaagctctcgtgcggcagcagctgcctgagaagtacaaagagattttcttcgaccagagcaagaacggctacgccggctacatcgatggcggagccagccaggaagagttctacaagttcatcaagcccatcctggaaaagatggacggcaccgaggaactgctcgtgaagctgaacagagaggacctgctgcggaagcagcggaccttcgacaacggcagcatcccccaccagatccacctgggagagctgcacgccattctgcggcggcaggaagatttttacccattcctgaaggacaaccgggaaaagatcgagaagatcctgaccttccgcatcccctactacgtgggccctctggccaggggaaacagcagattcgcctggatgaccagaaagagcgaggaaaccatcaccccctggaacttcgaggaagtggtggacaagggcgccagcgcccagagcttcatcgagcggatgaccaacttcgataagaacctgcccaacgagaaggtgctgcccaagcacagcctgctgtacgagtacttcaccgtgtacaacgagctgaccaaagtgaaatacgtgaccgagggaatgagaaagcccgccttcctgagcggcgagcagaaaaaagccatcgtggacctgctgttcaagaccaaccggaaagtgaccgtgaagcagctgaaagaggactacttcaagaaaatcgagtgcttcgactccgtggaaatctccggcgtggaagatcggttcaacgcctccctgggcacataccacgatctgctgaaaattatcaaggacaaggacttcctggacaatgaggaaaacgaggacattctggaagatatcgtgctgaccctgacactgtttgaggacagagagatgatcgaggaacggctgaaaacctatgcccacctgttcgacgacaaagtgatgaagcagctgaagcggcggagatacaccggctggggcaggctgagccggaagctgatcaacggcatccgggacaagcagtccggcaagacaatcctggatttcctgaagtccgacggcttcgccaacagaaacttcatgcagctgatccacgacgacagcctgacctttaaagaggacatccagaaagcccaggtgtccggccagggcgatagcctgcacgagcacattgccaatctggccggcagccccgccattaagaagggcatcctgcagacagtgaaggtggtggacgagctcgtgaaagtgatgggccggcacaagcccgagaacatcgtgatcgaaatggccagagagaaccagaccacccagaagggacagaagaacagccgcgagagaatgaagcggatcgaagagggcatcaaagagctgggcagccagatcctgaaagaacaccccgtggaaaacacccagctgcagaacgagaagctgtacctgtactacctgcagaatgggcgggatatgtacgtggaccaggaactggacatcaaccggctgtccgactacgatgtggacgctatcgtgcctcagagctttctgaaggacgactccatcgataacaaagtgctgactcggagcgacaagaaccggggcaagagcgacaacgtgccctccgaagaggtcgtgaagaagatgaagaactactggcgccagctgctgaatgccaagctgattacccagaggaagttcgacaatctgaccaaggccgagagaggcggcctgagcgaactggataaggccggcttcatcaagagacagctggtggaaacccggcagatcacaaagcacgtggcacagatcctggactcccggatgaacactaagtacgacgagaacgacaaactgatccgggaagtgaaagtgatcaccctgaagtccaagctggtgtccgatttccggaaggatttccagttttacaaagtgcgcgagatcaacaactaccaccacgcccacgacgcctacctgaacgccgtcgtgggaaccgccctgatcaaaaagtaccctaagctggaaagcgagttcgtgtacggcgactacaaggtgtacgacgtgcggaagatgatcgccaagagcgagcaggaaatcggcaaggctaccgccaagtacttcttctacagcaacatcatgaactttttcaagaccgagattaccctggccaacggcgagatccggaagcggcctctgatcgagacaaacggcgaaacaggcgagatcgtgtgggataagggccgggactttgccaccgtgcggaaagtgctgtctatgccccaagtgaatatcgtgaaaaagaccgaggtgcagacaggcggcttcagcaaagagtctatcctgcccaagaggaacagcgacaagctgatcgccagaaagaaggactgggaccctaagaagtacggcggcttcgacagccccaccgtggcctattctgtgctggtggtggccaaagtggaaaagggcaagtccaagaaactgaagagtgtgaaagagctgctggggatcaccatcatggaaagaagcagcttcgagaagaatcccatcgactttctggaagccaagggctacaaagaagtgaaaaaggacctgatcatcaagctgcctaagtactccctgttcgagctggaaaacggccggaagagaatgctggcctctgccggcgaactgcagaagggaaacgaactggccctgccctccaaatatgtgaacttcctgtacctggccagccactatgagaagctgaagggctcccccgaggataatgagcagaaacagctgtttgtggaacagcacaaacactacctggacgagatcatcgagcagatcagcgagttctccaagagagtgatcctggccgacgctaatctggacaaggtgctgagcgcctacaacaagcacagagacaagcctatcagagagcaggccgagaatatcatccacctgtttaccctgaccaatctgggagcccctgccgccttcaagtactttgacaccaccatcgaccggaagaggtacaccagcaccaaagaggtgctggacgccaccctgatccaccagagcatcaccggcctgtacgagacacggatcgacctgtctcagctgggaggcgacgcctatccctatgacgtgcccgattatgccagcctgggcagcggctcccccaagaaaaaacgcaaggtggaagatcctaagaaaaagcggaaagtggacggcattggtagtgggagcaacggcagcagcggagaggaactgctgagcaagaactaccacctggaaaacgaggtggccagactgaagaaaggctctggctctggcggaagcggttctggcggatcaggatctggaagtggcggctctggaagcggaggttctggatctggcgaagaactgctgtctaagaattatcacctcgagaatgaagtcgctcgtttgaagaaaggttcaggctccggccagcggggaagcaagcgcaccgccgatggttccgagttcgaaagccccaaaaaaaagcgcaaggtctga

SEQ ID NO: 310 - DNA, 7461 bp, synthetic construct
  misc_feature 1..7461: note = CDS of V22_D3a-D3l-scFv-2a-1xGCN4-dCas9-KRAB
  source 1..7461: mol_type = other DNA
atgcctgctgctaagagagtgaaactggatggatccaaccatgaccaggaatttgaccccccaaaggtttacccacctgtgccagctgagaagaggaagcccatccgcgtgctgtctctctttgatgggattgctacagggctcctggtgctgaaggacctgggcatccaagtggaccgctacattgcctccgaggtgtgtgaggactccatcacggtgggcatggtgcggcaccagggaaagatcatgtacgtcggggacgtccgcagcgtcacacagaagcatatccaggagtggggcccattcgacctggtgattggaggcagtccctgcaatgacctctccattgtcaaccctgcccgcaagggactttatgagggtactggccgcctcttctttgagttctaccgcctcctgcatgatgcgcggcccaaggagggagatgatcgccccttcttctggctctttgagaatgtggtggccatgggcgttagtgacaagagggacatctcgcgatttcttgagtctaaccccgtgatgattgacgccaaagaagtgtctgctgcacacagggcccgttacttctggggtaaccttcctggcatgaacaggcctttggcatccactgtgaatgataagctggagctgcaagagtgtctggagcacggcagaatagccaagttcagcaaagtgaggaccattaccaccaggtcaaactctataaagcagggcaaagaccagcatttccccgtgttcatgaacgagaaggaggacatcctgtggtgcactgaaatggaaagggtgtttggcttccccgtccactacacagacgtctccaacatgagccgcttggcgaggcagagactgctgggccgatcgtggagcgtgccggtcatccgccacctcttcgctccgctgaaggaatattttgcttgtgtgtctagcggcaatagtaacgctaacagccgcgggccgagcttcagcagcggcctggtgccgttaagcttgcgcggcagccatatgggccctatggagatatacaagacagtgtctgcatggaagagacagccagtgcgggtactgagcctcttcagaaacatcgacaaggtactaaagagtttgggcttcttggaaagcggttctggttctgggggaggaacgctgaagtacgtggaagatgtcacaaatgtcgtgaggagagacgtggagaaatggggcccctttgacctggtgtacggctcgacgcagcccctaggcagctcttgtgatcgctgtcccggctggtacatgttccagttccaccggatcctgcagtatgcgctgcctcgccaggagagtcagcggcccttcttctggatattcatggacaatctgctgctgactgaggatgaccaagagacaactacccgcttccttcagacagaggctgtgaccctccaggatgtccgtggcagagactaccagaatgctatgcgggtgtggagcaacattccagggctgaagagcaagcatgcgcccctgaccccaaaggaagaagagtatctgcaagcccaagtcagaagcaggagcaagctggacgccccgaaagttgacctcctggtgaagaactgccttctcccgctgagagagtacttcaagtatttttctcaaaactcacttcctcttggagggccgagctctggcgcacccccaccaagtggagggtctcctgccgggtccccaacatctactgaagaaggcaccagcgaatccgcaacgcccgagtcaggccctggtacctccacagaaccatctgaaggtagtgcgcctggttccccagctggaagccctacttccaccgaagaaggcacgtcaaccgaaccaagtgaaggatctgcccctgggaccagcactgaaccatctgagggccccgacatcgtgatgacccagagccccagcagcctgagcgccagcgtgggcgaccgcgtgaccatcacctgccgcagcagcaccggcgccgtgaccaccagcaactacgccagctgggtgcaggagaagcccggcaagctgttcaagggcctgatcggcggcaccaacaaccgcgcccccggcgtgcccagccgcttcagcggcagcctgatcggcgacaaggccaccctgaccatcagcagcctgcagcccgaggacttcgccacctacttctgcgccctgtggtacagcaaccactgggtgttcggccagggcaccaaggtggagctgaagcgcggcggcggcggcagcggcggcggcggcagcggcggcggcggcagcagcggcggcggcagcgaggtgaagctgctggagagcggcggcggcctggtgcagcccggcggcagcctgaagctgagctgcgccgtgagcggcttcagcctgaccgactacggcgtgaactgggtgcgccaggcccccggccgcggcctggagtggatcggcgtgatctggggcgacggcatcaccgactacaacagcgccctgaaggaccgcttcatcatcagcaaggacaacggcaagaacaccgtgtacctgcagatgagcaaggtgcgcagcgacgacaccgccctgtactactgcgtgaccggcctgttcgactactggggccagggcaccctggtgaccgtgagcagctacccatacgatgttccagattacgctggtggaggcggaggttctgggggaggaggtagtggcggtggtggttcaggaggcggcggaagcggaagcggagctactaacttcagcctgctgaagcaggctggagacgtggaggagaaccctggacctatgcctgctgctaagagagtgaaactggatggatccggctcaggcggatctggttcaggggaagaactcctctccaaaaactaccatctcgagaatgaggtcgcccgcctgaaaaaaggatcaggttccggtggttctggcagcggtggttcaggctcaggcagcggcggtagcggtagcggtggaagcggaagcggaccaaaaaagaagagaaaggtaatggacaagaagtacagcatcggcctggccatcggcaccaactctgtgggctgggccgtgatcaccgacgagtacaaggtgcccagcaagaaattcaaggtgctgggcaacaccgaccggcacagcatcaagaagaacctgatcggcgccctgctgttcgacagcggagaaacagccgaggccacccggctgaagagaaccgccagaagaagatacaccagacggaagaaccggatctgctatctgcaagagatcttcagcaacgagatggccaaggtggacgacagcttcttccacagactggaagagtccttcctggtggaagaggataagaagcacgagcggcaccccatcttcggcaacatcgtggacgaggtggcctaccacgagaagtaccccaccatctaccacctgagaaagaaactggtggacagcaccgacaaggccgacctgcggctgatctatctggccctggcccacatgatcaagttccggggccacttcctgatcgagggcgacctgaaccccgacaacagcgacgtggacaagctgttcatccagctggtgcagacctacaaccagctgttcgaggaaaaccccatcaacgccagcggcgtggacgccaaggccatcctgtctgccagactgagcaagagcagacggctggaaaatctgatcgcccagctgcccggcgagaagaagaatggcctgttcggcaacctgattgccctgagcctgggcctgacccccaacttcaagagcaacttcgacctggccgaggatgccaaactgcagctgagcaaggacacctacgacgacgacctggacaacctgctggcccagatcggcgaccagtacgccgacctgtttctggccgccaagaacctgtccgacgccatcctgctgagcgacatcctgagagtgaacaccgagatcaccaaggcccccctgagcgcctctatgatcaagagatacgacgagcaccaccaggacctgaccctgctgaaagctctcgtgcggcagcagctgcctgagaagtacaaagagattttcttcgaccagagcaagaacggctacgccggctacatcgatggcggagccagccaggaagagttctacaagttcatcaagcccatcctggaaaagatggacggcaccgaggaactgctcgtgaagctgaacagagaggacctgctgcggaagcagcggaccttcgacaacggcagcatcccccaccagatccacctgggagagctgcacgccattctgcggcggcaggaagatttttacccattcctgaaggacaaccgggaaaagatcgagaagatcctgaccttccgcatcccctactacgtgggccctctggccaggggaaacagcagattcgcctggatgaccagaaagagcgaggaaaccatcaccccctggaacttcgaggaagtggtggacaagggcgccagcgcccagagcttcatcgagcggatgaccaacttcgataagaacctgcccaacgagaaggtgctgcccaagcacagcctgctgtacgagtacttcaccgtgtacaacgagctgaccaaagtgaaatacgtgaccgagggaatgagaaagcccgccttcctgagcggcgagcagaaaaaagccatcgtggacctgctgttcaagaccaaccggaaagtgaccgtgaagcagctgaaagaggactacttcaagaaaatcgagtgcttcgactccgtggaaatctccggcgtggaagatcggttcaacgcctccctgggcacataccacgatctgctgaaaattatcaaggacaaggacttcctggacaatgaggaaaacgaggacattctggaagatatcgtgctgaccctgacactgtttgaggacagagagatgatcgaggaacggctgaaaacctatgcccacctgttcgacgacaaagtgatgaagcagctgaagcggcggagatacaccggctggggcaggctgagccggaagctgatcaacggcatccgggacaagcagtccggcaagacaatcctggatttcctgaagtccgacggcttcgccaacagaaacttcatgcagctgatccacgacgacagcctgacctttaaagaggacatccagaaagcccaggtgtccggccagggcgatagcctgcacgagcacattgccaatctggccggcagccccgccattaagaagggcatcctgcagacagtgaaggtggtggacgagctcgtgaaagtgatgggccggcacaagcccgagaacatcgtgatcgaaatggccagagagaaccagaccacccagaagggacagaagaacagccgcgagagaatgaagcggatcgaagagggcatcaaagagctgggcagccagatcctgaaagaacaccccgtggaaaacacccagctgcagaacgagaagctgtacctgtactacctgcagaatgggcgggatatgtacgtggaccaggaactggacatcaaccggctgtccgactacgatgtggacgctatcgtgcctcagagctttctgaaggacgactccatcgataacaaagtgctgactcggagcgacaagaaccggggcaagagcgacaacgtgccctccgaagaggtcgtgaagaagatgaagaactactggcgccagctgctgaatgccaagctgattacccagaggaagttcgacaatctgaccaaggccgagagaggcggcctgagcgaactggataaggccggcttcatcaagagacagctggtggaaacccggcagatcacaaagcacgtggcacagatcctggactcccggatgaacactaagtacgacgagaacgacaaactgatccgggaagtgaaagtgatcaccctgaagtccaagctggtgtccgatttccggaaggatttccagttttacaaagtgcgcgagatcaacaactaccaccacgcccacgacgcctacctgaacgccgtcgtgggaaccgccctgatcaaaaagtaccctaagctggaaagcgagttcgtgtacggcgactacaaggtgtacgacgtgcggaagatgatcgccaagagcgagcaggaaatcggcaaggctaccgccaagtacttcttctacagcaacatcatgaactttttcaagaccgagattaccctggccaacggcgagatccggaagcggcctctgatcgagacaaacggcgaaacaggcgagatcgtgtgggataagggccgggactttgccaccgtgcggaaagtgctgtctatgccccaagtgaatatcgtgaaaaagaccgaggtgcagacaggcggcttcagcaaagagtctatcctgcccaagaggaacagcgacaagctgatcgccagaaagaaggactgggaccctaagaagtacggcggcttcgacagccccaccgtggcctattctgtgctggtggtggccaaagtggaaaagggcaagtccaagaaactgaagagtgtgaaagagctgctggggatcaccatcatggaaagaagcagcttcgagaagaatcccatcgactttctggaagccaagggctacaaagaagtgaaaaaggacctgatcatcaagctgcctaagtactccctgttcgagctggaaaacggccggaagagaatgctggcctctgccggcgaactgcagaagggaaacgaactggccctgccctccaaatatgtgaacttcctgtacctggccagccactatgagaagctgaagggctcccccgaggataatgagcagaaacagctgtttgtggaacagcacaaacactacctggacgagatcatcgagcagatcagcgagttctccaagagagtgatcctggccgacgctaatctggacaaggtgctgagcgcctacaacaagcacagagacaagcctatcagagagcaggccgagaatatcatccacctgtttaccctgaccaatctgggagcccctgccgccttcaagtactttgacaccaccatcgaccggaagaggtacaccagcaccaaagaggtgctggacgccaccctgatccaccagagcatcaccggcctgtacgagacacggatcgacctgtctcagctgggaggcgacgcctatccctatgacgtgcccgattatgccagcctgggcagcggctcccccaagaaaaaacgcaaggtggaagatcctaagaaaaagcggaaagtggacggcagcggcagcgagacccccggtaccagcgagagcgccacccccgagagccggacactggtgaccttcaaggatgtatttgtggacttcaccagggaggagtggaagctgctggacactgctcagcagatcgtgtacagaaatgtgatgctggagaactataagaacctggtttccttgggttatcagcttactaagccagatgtgatcctccggttggagaagggagaagagccctga

SEQ ID NO: 311 - DNA, 7575 bp, synthetic construct
  misc_feature 1..7575: note = CDS of V23_D3a-D3l-scFv-2a-2xGCN4-dCas9-KRAB
  source 1..7575: mol_type = other DNA
atgcctgctgctaagagagtgaaactggatggatccaaccatgaccaggaatttgaccccccaaaggtttacccacctgtgccagctgagaagaggaagcccatccgcgtgctgtctctctttgatgggattgctacagggctcctggtgctgaaggacctgggcatccaagtggaccgctacattgcctccgaggtgtgtgaggactccatcacggtgggcatggtgcggcaccagggaaagatcatgtacgtcggggacgtccgcagcgtcacacagaagcatatccaggagtggggcccattcgacctggtgattggaggcagtccctgcaatgacctctccattgtcaaccctgcccgcaagggactttatgagggtactggccgcctcttctttgagttctaccgcctcctgcatgatgcgcggcccaaggagggagatgatcgccccttcttctggctctttgagaatgtggtggccatgggcgttagtgacaagagggacatctcgcgatttcttgagtctaaccccgtgatgattgacgccaaagaagtgtctgctgcacacagggcccgttacttctggggtaaccttcctggcatgaacaggcctttggcatccactgtgaatgataagctggagctgcaagagtgtctggagcacggcagaatagccaagttcagcaaagtgaggaccattaccaccaggtcaaactctataaagcagggcaaagaccagcatttccccgtgttcatgaacgagaaggaggacatcctgtggtgcactgaaatggaaagggtgtttggcttccccgtccactacacagacgtctccaacatgagccgcttggcgaggcagagactgctgggccgatcgtggagcgtgccggtcatccgccacctcttcgctccgctgaaggaatattttgcttgtgtgtctagcggcaatagtaacgctaacagccgcgggccgagcttcagcagcggcctggtgccgttaagcttgcgcggcagccatatgggccctatggagatatacaagacagtgtctgcatggaagagacagccagtgcgggtactgagcctcttcagaaacatcgacaaggtactaaagagtttgggcttcttggaaagcggttctggttctgggggaggaacgctgaagtacgtggaagatgtcacaaatgtcgtgaggagagacgtggagaaatggggcccctttgacctggtgtacggctcgacgcagcccctaggcagctcttgtgatcgctgtcccggctggtacatgttccagttccaccggatcctgcagtatgcgctgcctcgccaggagagtcagcggcccttcttctggatattcatggacaatctgctgctgactgaggatgaccaagagacaactacccgcttccttcagacagaggctgtgaccctccaggatgtccgtggcagagactaccagaatgctatgcgggtgtggagcaacattccagggctgaagagcaagcatgcgcccctgaccccaaaggaagaagagtatctgcaagcccaagtcagaagcaggagcaagctggacgccccgaaagttgacctcctggtgaagaactgccttctcccgctgagagagtacttcaagtatttttctcaaaactcacttcctcttggagggccgagctctggcgcacccccaccaagtggagggtctcctgccgggtccccaacatctactgaagaaggcaccagcgaatccgcaacgcccgagtcaggccctggtacctccacagaaccatctgaaggtagtgcgcctggttccccagctggaagccctacttccaccgaagaaggcacgtcaaccgaaccaagtgaaggatctgcccctgggaccagcactgaaccatctgagggccccgacatcgtgatgacccagagccccagcagcctgagcgccagcgtgggcgaccgcgtgaccatcacctgccgcagcagcaccggcgccgtgaccaccagcaactacgccagctgggtgcaggagaagcccggcaagctgttcaagggcctgatcggcggcaccaacaaccgcgcccccggcgtgcccagccgcttcagcggcagcctgatcggcgacaaggccaccctgaccatcagcagcctgcagcccgaggacttcgccacctacttctgcgccctgtggtacagcaaccactgggtgttcggccagggcaccaaggtggagctgaagcgcggcggcggcggcagcggcggcggcggcagcggcggcggcggcagcagcggcggcggcagcgaggtgaagctgctggagagcggcggcggcctggtgcagcccggcggcagcctgaagctgagctgcgccgtgagcggcttcagcctgaccgactacggcgtgaactgggtgcgccaggcccccggccgcggcctggagtggatcggcgtgatctggggcgacggcatcaccgactacaacagcgccctgaaggaccgcttcatcatcagcaaggacaacggcaagaacaccgtgtacctgcagatgagcaaggtgcgcagcgacgacaccgccctgtactactgcgtgaccggcctgttcgactactggggccagggcaccctggtgaccgtgagcagctacccatacgatgttccagattacgctggtggaggcggaggttctgggggaggaggtagtggcggtggtggttcaggaggcggcggaagcggaagcggagctactaacttcagcctgctgaagcaggctggagacgtggaggagaaccctggacctatgcctgctgctaagagagtgaaactggatggatccgaggaactgctgagcaagaactaccacctggaaaacgaggtggccagactgaagaaaggctctggctctggcggaagcggttctggcggatcaggatctggaagtggcggctctggaagcggaggttctggatctggcgaagaactgctgtctaagaattatcacctcgagaatgaggtcgcccgcctgaaaaaaggatcaggttccggtggttctggcagcggtggttcaggctcaggcagcggcggtagcggtagcggtggaagcggaagcggaccaaaaaagaagagaaaggtaatggacaagaagtacagcatcggcctggccatcggcaccaactctgtgggctgggccgtgatcaccgacgagtacaaggtgcccagcaagaaattcaaggtgctgggcaacaccgaccggcacagcatcaagaagaacctgatcggcgccctgctgttcgacagcggagaaacagccgaggccacccggctgaagagaaccgccagaagaagatacaccagacggaagaaccggatctgctatctgcaagagatcttcagcaacgagatggccaaggtggacgacagcttcttccacagactggaagagtccttcctggtggaagaggataagaagcacgagcggcaccccatcttcggcaacatcgtggacgaggtggcctaccacgagaagtaccccaccatctaccacctgagaaagaaactggtggacagcaccgacaaggccgacctgcggctgatctatctggccctggcccacatgatcaagttccggggccacttcctgatcgagggcgacctgaaccccgacaacagcgacgtggacaagctgttcatccagctggtgcagacctacaaccagctgttcgaggaaaaccccatcaacgccagcggcgtggacgccaaggccatcctgtctgccagactgagcaagagcagacggctggaaaatctgatcgcccagctgcccggcgagaagaagaatggcctgttcggcaacctgattgccctgagcctgggcctgacccccaacttcaagagcaacttcgacctggccgaggatgccaaactgcagctgagcaaggacacctacgacgacgacctggacaacctgctggcccagatcggcgaccagtacgccgacctgtttctggccgccaagaacctgtccgacgccatcctgctgagcgacatcctgagagtgaacaccgagatcaccaaggcccccctgagcgcctctatgatcaagagatacgacgagcaccaccaggacctgaccctgctgaaagctctcgtgcggcagcagctgcctgagaagtacaaagagattttcttcgaccagagcaagaacggctacgccggctacatcgatggcggagccagccaggaagagttctacaagttcatcaagcccatcctggaaaagatggacggcaccgaggaactgctcgtgaagctgaacagagaggacctgctgcggaagcagcggaccttcgacaacggcagcatcccccaccagatccacctgggagagctgcacgccattctgcggcggcaggaagatttttacccattcctgaaggacaaccgggaaaagatcgagaagatcctgaccttccgcatcccctactacgtgggccctctggccaggggaaacagcagattcgcctggatgaccagaaagagcgaggaaaccatcaccccctggaacttcgaggaagtggtggacaagggcgccagcgcccagagcttcatcgagcggatgaccaacttcgataagaacctgcccaacgagaaggtgctgcccaagcacagcctgctgtacgagtacttcaccgtgtacaacgagctgaccaaagtgaaatacgtgaccgagggaatgagaaagcccgccttcctgagcggcgagcagaaaaaagccatcgtggacctgctgttcaagaccaaccggaaagtgaccgtgaagcagctgaaagaggactacttcaagaaaatcgagtgcttcgactccgtggaaatctccggcgtggaagatcggttcaacgcctccctgggcacataccacgatctgctgaaaattatcaaggacaaggacttcctggacaatgaggaaaacgaggacattctggaagatatcgtgctgaccctgacactgtttgaggacagagagatgatcgaggaacggctgaaaacctatgcccacctgttcgacgacaaagtgatgaagcagctgaagcggcggagatacaccggctggggcaggctgagccggaagctgatcaacggcatccgggacaagcagtccggcaagacaatcctggatttcctgaagtccgacggcttcgccaacagaaacttcatgcagctgatccacgacgacagcctgacctttaaagaggacatccagaaagcccaggtgtccggccagggcgatagcctgcacgagcacattgccaatctggccggcagccccgccattaagaagggcatcctgcagacagtgaaggtggtggacgagctcgtgaaagtgatgggccggcacaagcccgagaacatcgtgatcgaaatggccagagagaaccagaccacccagaagggacagaagaacagccgcgagagaatgaagcggatcgaagagggcatcaaagagctgggcagccagatcctgaaagaacaccccgtggaaaacacccagctgcagaacgagaagctgtacctgtactacctgcagaatgggcgggatatgtacgtggaccaggaactggacatcaaccggctgtccgactacgatgtggacgctatcgtgcctcagagctttctgaaggacgactccatcgataacaaagtgctgactcggagcgacaagaaccggggcaagagcgacaacgtgccctccgaagaggtcgtgaagaagatgaagaactactggcgccagctgctgaatgccaagctgattacccagaggaagttcgacaatctgaccaaggccgagagaggcggcctgagcgaactggataaggccggcttcatcaagagacagctggtggaaacccggcagatcacaaagcacgtggcacagatcctggactcccggatgaacactaagtacgacgagaacgacaaactgatccgggaagtgaaagtgatcaccctgaagtccaagctggtgtccgatttccggaaggatttccagttttacaaagtgcgcgagatcaacaactaccaccacgcccacgacgcctacctgaacgccgtcgtgggaaccgccctgatcaaaaagtaccctaagctggaaagcgagttcgtgtacggcgactacaaggtgtacgacgtgcggaagatgatcgccaagagcgagcaggaaatcggcaaggctaccgccaagtacttcttctacagcaacatcatgaactttttcaagaccgagattaccctggccaacggcgagatccggaagcggcctctgatcgagacaaacggcgaaacaggcgagatcgtgtgggataagggccgggactttgccaccgtgcggaaagtgctgtctatgccccaagtgaatatcgtgaaaaagaccgaggtgcagacaggcggcttcagcaaagagtctatcctgcccaagaggaacagcgacaagctgatcgccagaaagaaggactgggaccctaagaagtacggcggcttcgacagccccaccgtggcctattctgtgctggtggtggccaaagtggaaaagggcaagtccaagaaactgaagagtgtgaaagagctgctggggatcaccatcatggaaagaagcagcttcgagaagaatcccatcgactttctggaagccaagggctacaaagaagtgaaaaaggacctgatcatcaagctgcctaagtactccctgttcgagctggaaaacggccggaagagaatgctggcctctgccggcgaactgcagaagggaaacgaactggccctgccctccaaatatgtgaacttcctgtacctggccagccactatgagaagctgaagggctcccccgaggataatgagcagaaacagctgtttgtggaacagcacaaacactacctggacgagatcatcgagcagatcagcgagttctccaagagagtgatcctggccgacgctaatctggacaaggtgctgagcgcctacaacaagcacagagacaagcctatcagagagcaggccgagaatatcatccacctgtttaccctgaccaatctgggagcccctgccgccttcaagtactttgacaccaccatcgaccggaagaggtacaccagcaccaaagaggtgctggacgccaccctgatccaccagagcatcaccggcctgtacgagacacggatcgacctgtctcagctgggaggcgacgcctatccctatgacgtgcccgattatgccagcctgggcagcggctcccccaagaaaaaacgcaaggtggaagatcctaagaaaaagcggaaagtggacggcagcggcagcgagacccccggtaccagcgagagcgccacccccgagagccggacactggtgaccttcaaggatgtatttgtggacttcaccagggaggagtggaagctgctggacactgctcagcagatcgtgtacagaaatgtgatgctggagaactataagaacctggtttccttgggttatcagcttactaagccagatgtgatcctccggttggagaagggagaagagccctga

SEQ ID NO: 312 - DNA, 7713 bp, synthetic construct
  misc_feature 1..7713: note = CDS of V24_D3a-D3l-scFv-2a-3xGCN4-dCas9-KRAB
  source 1..7713: mol_type = other DNA
atgcctgctgctaagagagtgaaactggatggatccaaccatgaccaggaatttgaccccccaaaggtttacccacctgtgccagctgagaagaggaagcccatccgcgtgctgtctctctttgatgggattgctacagggctcctggtgctgaaggacctgggcatccaagtggaccgctacattgcctccgaggtgtgtgaggactccatcacggtgggcatggtgcggcaccagggaaagatcatgtacgtcggggacgtccgcagcgtcacacagaagcatatccaggagtggggcccattcgacctggtgattggaggcagtccctgcaatgacctctccattgtcaaccctgcccgcaagggactttatgagggtactggccgcctcttctttgagttctaccgcctcctgcatgatgcgcggcccaaggagggagatgatcgccccttcttctggctctttgagaatgtggtggccatgggcgttagtgacaagagggacatctcgcgatttcttgagtctaaccccgtgatgattgacgccaaagaagtgtctgctgcacacagggcccgttacttctggggtaaccttcctggcatgaacaggcctttggcatccactgtgaatgataagctggagctgcaagagtgtctggagcacggcagaatagccaagttcagcaaagtgaggaccattaccaccaggtcaaactctataaagcagggcaaagaccagcatttccccgtgttcatgaacgagaaggaggacatcctgtggtgcactgaaatggaaagggtgtttggcttccccgtccactacacagacgtctccaacatgagccgcttggcgaggcagagactgctgggccgatcgtggagcgtgccggtcatccgccacctcttcgctccgctgaaggaatattttgcttgtgtgtctagcggcaatagtaacgctaacagccgcgggccgagcttcagcagcggcctggtgccgttaagcttgcgcggcagccatatgggccctatggagatatacaagacagtgtctgcatggaagagacagccagtgcgggtactgagcctcttcagaaacatcgacaaggtactaaagagtttgggcttcttggaaagcggttctggttctgggggaggaacgctgaagtacgtggaagatgtcacaaatgtcgtgaggagagacgtggagaaatggggcccctttgacctggtgtacggctcgacgcagcccctaggcagctcttgtgatcgctgtcccggctggtacatgttccagttccaccggatcctgcagtatgcgctgcctcgccaggagagtcagcggcccttcttctggatattcatggacaatctgctgctgactgaggatgaccaagagacaactacccgcttccttcagacagaggctgtgaccctccaggatgtccgtggcagagactaccagaatgctatgcgggtgtggagcaacattccagggctgaagagcaagcatgcgcccctgaccccaaaggaagaagagtatctgcaagcccaagtcagaagcaggagcaagctggacgccccgaaagttgacctcctggtgaagaactgccttctcccgctgagagagtacttcaagtatttttctcaaaactcacttcctcttggagggccgagctctggcgcacccccaccaagtggagggtctcctgccgggtccccaacatctactgaagaaggcaccagcgaatccgcaacgcccgagtcaggccctggtacctccacagaaccatctgaaggtagtgcgcctggttccccagctggaagccctacttccaccgaagaaggcacgtcaaccgaaccaagtgaaggatctgcccctgggaccagcactgaaccatctgagggccccgacatcgtgatgacccagagccccagcagcctgagcgccagcgtgggcgaccgcgtgaccatcacctgccgcagcagcaccggcgccgtgaccaccagcaactacgccagctgggtgcaggagaagcccggcaagctgttcaagggcctgatcggcggcaccaacaaccgcgcccccggcgtgcccagccgcttcagcggcagcctgatcggcgacaaggccaccctgaccatcagcagcctgcagcccgaggacttcgccacctacttctgcgccctgtggtacagcaaccactgggtgttcggccagggcaccaaggtggagctgaagcgcggcggcggcggcagcggcggcggcggcagcggcggcggcggcagcagcggcggcggcagcgaggtgaagctgctggagagcggcggcggcctggtgcagcccggcggcagcctgaagctgagctgcgccgtgagcggcttcagcctgaccgactacggcgtgaactgggtgcgccaggcccccggccgcggcctggagtggatcggcgtgatctggggcgacggcatcaccgactacaacagcgccctgaaggaccgcttcatcatcagcaaggacaacggcaagaacaccgtgtacctgcagatgagcaaggtgcgcagcgacgacaccgccctgtactactgcgtgaccggcctgttcgactactggggccagggcaccctggtgaccgtgagcagctacccatacgatgttccagattacgctggtggaggcggaggttctgggggaggaggtagtggcggtggtggttcaggaggcggcggaagcggaagcggagctactaacttcagcctgctgaagcaggctggagacgtggaggagaaccctggacctatgcctgctgctaagagagtgaaactggatggatccgaggaactgctgagcaagaactaccacctggaaaacgaggtggccagactgaagaaaggctctggctctggcggaagcggttctggcggatcaggatctggaagtggcggctctggaagcggaggttctggatctggcgaagaactgctgtctaagaattatcacctcgagaacgaagtggctcggctcaagaaaggcagtggcagcggaggaagtggatccggcggtagtggtagtggaagcggcggatccggctcaggcggatctggttcaggggaagaactcctctccaaaaactaccatctcgagaatgaggtcgcccgcctgaaaaaaggatcaggttccggtggttctggcagcggtggttcaggctcaggcagcggcggtagcggtagcggtggaagcggaagcggaccaaaaaagaagagaaaggtaatggacaagaagtacagcatcggcctggccatcggcaccaactctgtgggctgggccgtgatcaccgacgagtacaaggtgcccagcaagaaattcaaggtgctgggcaacaccgaccggcacagcatcaagaagaacctgatcggcgccctgctgttcgacagcggagaaacagccgaggccacccggctgaagagaaccgccagaagaagatacaccagacggaagaaccggatctgctatctgcaagagatcttcagcaacgagatggccaaggtggacgacagcttcttccacagactggaagagtccttcctggtggaagaggataagaagcacgagcggcaccccatcttcggcaacatcgtggacgaggtggcctaccacgagaagtaccccaccatctaccacctgagaaagaaactggtggacagcaccgacaaggccgacctgcggctgatctatctggccctggcccacatgatcaagttccggggccacttcctgatcgagggcgacctgaaccccgacaacagcgacgtggacaagctgttcatccagctggtgcagacctacaaccagctgttcgaggaaaaccccatcaacgccagcggcgtggacgccaaggccatcctgtctgccagactgagcaagagcagacggctggaaaatctgatcgcccagctgcccggcgagaagaagaatggcctgttcggcaacctgattgccctgagcctgggcctgacccccaacttcaagagcaacttcgacctggccgaggatgccaaactgcagctgagcaaggacacctacgacgacgacctggacaacctgctggcccagatcggcgaccagtacgccgacctgtttctggccgccaagaacctgtccgacgccatcctgctgagcgacatcctgagagtgaacaccgagatcaccaaggcccccctgagcgcctctatgatcaagagatacgacgagcaccaccaggacctgaccctgctgaaagctctcgtgcggcagcagctgcctgagaagtacaaagagattttcttcgaccagagcaagaacggctacgccggctacatcgatggcggagccagccaggaagagttctacaagttcatcaagcccatcctggaaaagatggacggcaccgaggaactgctcgtgaagctgaacagagaggacctgctgcggaagcagcggaccttcgacaacggcagcatcccccaccagatccacctgggagagctgcacgccattctgcggcggcaggaagatttttacccattcctgaaggacaaccgggaaaagatcgagaagatcctgaccttccgcatcccctactacgtgggccctctggccaggggaaacagcagattcgcctggatgaccagaaagagcgaggaaaccatcaccccctggaacttcgaggaagtggtggacaagggcgccagcgcccagagcttcatcgagcggatgaccaacttcgataagaacctgcccaacgagaaggtgctgcccaagcacagcctgctgtacgagtacttcaccgtgtacaacgagctgaccaaagtgaaatacgtgaccgagggaatgagaaagcccgccttcctgagcggcgagcagaaaaaagccatcgtggacctgctgttcaagaccaaccggaaagtgaccgtgaagcagctgaaagaggactacttcaagaaaatcgagtgcttcgactccgtggaaatctccggcgtggaagatcggttcaacgcctccctgggcacataccacgatctgctgaaaattatcaaggacaaggacttcctggacaatgaggaaaacgaggacattctggaagatatcgtgctgaccctgacactgtttgaggacagagagatgatcgaggaacggctgaaaacctatgcccacctgttcgacgacaaagtgatgaagcagctgaagcggcggagatacaccggctggggcaggctgagccggaagctgatcaacggcatccgggacaagcagtccggcaagacaatcctggatttcctgaagtccgacggcttcgccaacagaaacttcatgcagctgatccacgacgacagcctgacctttaaagaggacatccagaaagcccaggtgtccggccagggcgatagcctgcacgagcacattgccaatctggccggcagccccgccattaagaagggcatcctgcagacagtgaaggtggtggacgagctcgtgaaagtgatgggccggcacaagcccgagaacatcgtgatcgaaatggccagagagaaccagaccacccagaagggacagaagaacagccgcgagagaatgaagcggatcgaagagggcatcaaagagctgggcagccagatcctgaaagaacaccccgtggaaaacacccagctgcagaacgagaagctgtacctgtactacctgcagaatgggcgggatatgtacgtggaccaggaactggacatcaaccggctgtccgactacgatgtggacgctatcgtgcctcagagctttctgaaggacgactccatcgataacaaagtgctgactcggagcgacaagaaccggggcaagagcgacaacgtgccctccgaagaggtcgtgaagaagatgaagaactactggcgccagctgctgaatgccaagctgattacccagaggaagttcgacaatctgaccaaggccgagagaggcggcctgagcgaactggataaggccggcttcatcaagagacagctggtggaaacccggcagatcacaaagcacgtggcacagatcctggactcccggatgaacactaagtacgacgagaacgacaaactgatccgggaagtgaaagtgatcaccctgaagtccaagctggtgtccgatttccggaaggatttccagttttacaaagtgcgcgagatcaacaactaccaccacgcccacgacgcctacctgaacgccgtcgtgggaaccgccctgatcaaaaagtaccctaagctggaaagcgagttcgtgtacggcgactacaaggtgtacgacgtgcggaagatgatcgccaagagcgagcaggaaatcggcaaggctaccgccaagtacttcttctacagcaacatcatgaactttttcaagaccgagattaccctggccaacggcgagatccggaagcggcctctgatcgagacaaacggcgaaacaggcgagatcgtgtgggataagggccgggactttgccaccgtgcggaaagtgctgtctatgccccaagtgaatatcgtgaaaaagaccgaggtgcagacaggcggcttcagcaaagagtctatcctgcccaagaggaacagcgacaagctgatcgccagaaagaaggactgggaccctaagaagtacggcggcttcgacagccccaccgtggcctattctgtgctggtggtggccaaagtggaaaagggcaagtccaagaaactgaagagtgtgaaagagctgctggggatcaccatcatggaaagaagcagcttcgagaagaatcccatcgactttctggaagccaagggctacaaagaagtgaaaaaggacctgatcatcaagctgcctaagtactccctgttcgagctggaaaacggccggaagagaatgctggcctctgccggcgaactgcagaagggaaacgaactggccctgccctccaaatatgtgaacttcctgtacctggccagccactatgagaagctgaagggctcccccgaggataatgagcagaaacagctgtttgtggaacagcacaaacactacctggacgagatcatcgagcagatcagcgagttctccaagagagtgatcctggccgacgctaatctggacaaggtgctgagcgcctacaacaagcacagagacaagcctatcagagagcaggccgagaatatcatccacctgtttaccctgaccaatctgggagcccctgccgccttcaagtactttgacaccaccatcgaccggaagaggtacaccagcaccaaagaggtgctggacgccaccctgatccaccagagcatcaccggcctgtacgagacacggatcgacctgtctcagctgggaggcgacgcctatccctatgacgtgcccgattatgccagcctgggcagcggctcccccaagaaaaaacgcaaggtggaagatcctaagaaaaagcggaaagtggacggcagcggcagcgagacccccggtaccagcgagagcgccacccccgagagccggacactggtgaccttcaaggatgtatttgtggacttcaccagggaggagtggaagctgctggacactgctcagcagatcgtgtacagaaatgtgatgctggagaactataagaacctggtttccttgggttatcagcttactaagccagatgtgatcctccggttggagaagggagaagagccctga

SEQ ID NO: 313 - DNA, 7989 bp, synthetic construct
  misc_feature 1..7989: note = CDS of V25_D3a-D3l-scFv-2a-5xGCN4-dCas9-KRAB
  source 1..7989: mol_type = other DNA
atgcctgctgctaagagagtgaaactggatggatccaaccatgaccaggaatttgaccccccaaaggtttacccacctgtgccagctgagaagaggaagcccatccgcgtgctgtctctctttgatgggattgctacagggctcctggtgctgaaggacctgggcatccaagtggaccgctacattgcctccgaggtgtgtgaggactccatcacggtgggcatggtgcggcaccagggaaagatcatgtacgtcggggacgtccgcagcgtcacacagaagcatatccaggagtggggcccattcgacctggtgattggaggcagtccctgcaatgacctctccattgtcaaccctgcccgcaagggactttatgagggtactggccgcctcttctttgagttctaccgcctcctgcatgatgcgcggcccaaggagggagatgatcgccccttcttctggctctttgagaatgtggtggccatgggcgttagtgacaagagggacatctcgcgatttcttgagtctaaccccgtgatgattgacgccaaagaagtgtctgctgcacacagggcccgttacttctggggtaaccttcctggcatgaacaggcctttggcatccactgtgaatgataagctggagctgcaagagtgtctggagcacggcagaatagccaagttcagcaaagtgaggaccattaccaccaggtcaaactctataaagcagggcaaagaccagcatttccccgtgttcatgaacgagaaggaggacatcctgtggtgcactgaaatggaaagggtgtttggcttccccgtccactacacagacgtctccaacatgagccgcttggcgaggcagagactgctgggccgatcgtggagcgtgccggtcatccgccacctcttcgctccgctgaaggaatattttgcttgtgtgtctagcggcaatagtaacgctaacagccgcgggccgagcttcagcagcggcctggtgccgttaagcttgcgcggcagccatatgggccctatggagatatacaagacagtgtctgcatggaagagacagccagtgcgggtactgagcctcttcagaaacatcgacaaggtactaaagagtttgggcttcttggaaagcggttctggttctgggggaggaacgctgaagtacgtggaagatgtcacaaatgtcgtgaggagagacgtggagaaatggggcccctttgacctggtgtacggctcgacgcagcccctaggcagctcttgtgatcgctgtcccggctggtacatgttccagttccaccggatcctgcagtatgcgctgcctcgccaggagagtcagcggcccttcttctggatattcatggacaatctgctgctgactgaggatgaccaagagacaactacccgcttccttcagacagaggctgtgaccctccaggatgtccgtggcagagactaccagaatgctatgcgggtgtggagcaacattccagggctgaagagcaagcatgcgcccctgaccccaaaggaagaagagtatctgcaagcccaagtcagaagcaggagcaagctggacgccccgaaagttgacctcctggtgaagaactgccttctcccgctgagagagtacttcaagtatttttctcaaaactcacttcctcttggagggccgagctctggcgcacccccaccaagtggagggtctcctgccgggtccccaacatctactgaagaaggcaccagcgaatccgcaacgcccgagtcaggccctggtacctccacagaaccatctgaaggtagtgcgcctggttccccagctggaagccctacttccaccgaagaaggcacgtcaaccgaaccaagtgaaggatctgcccctgggaccagcactgaaccatctgagggccccgacatcgtgatgacccagagccccagcagcctgagcgccagcgtgggcgaccgcgtgaccatcacctgccgcagcagcaccggcgccgtgaccaccagcaactacgccagctgggtgcaggagaagcccggcaagctgttcaagggcctgatcggcggcaccaacaaccgcgcccccggcgtgcccagccgcttcagcggcagcctgatcggcgacaaggccaccctgaccatcagcagcctgcagcccgaggacttcgccacctacttctgcgccctgtggtacagcaaccactgggtgttcggccagggcaccaaggtggagctgaagcgcggcggcggcggcagcggcggcggcggcagcggcggcggcggcagcagcggcggcggcagcgaggtgaagctgctggagagcggcggcggcctggtgcagcccggcggcagcctgaagctgagctgcgccgtgagcggcttcagcctgaccgactacggcgtgaactgggtgcgccaggcccccggccgcggcctggagtggatcggcgtgatctggggcgacggcatcaccgactacaacagcgccctgaaggaccgcttcatcatcagcaaggacaacggcaagaacaccgtgtacctgcagatgagcaaggtgcgcagcgacgacaccgccctgtactactgcgtgaccggcctgttcgactactggggccagggcaccctggtgaccgtgagcagctacccatacgatgttccagattacgctggtggaggcggaggttctgggggaggaggtagtggcggtggtggttcaggaggcggcggaagcggaagcggagctactaacttcagcctgctgaagcaggctggagacgtggaggagaaccctggacctatgcctgctgctaagagagtgaaactggatggatccgaggaactgctgagcaagaactaccacctggaaaacgaggtggccagactgaagaaaggctctggctctggcggaagcggttctggcggatcaggatctggaagtggcggctctggaagcggaggttctggatctggcgaagaactgctgtctaagaattatcacctcgagaacgaggttgcacgcttgaagaaaggcagcggatcaggcggatctggcagcggtggatctggttctggatccggcggctccggtagtggtggaagtggctctggggaagaattgcttagcaagaattatcatcttgaaaatgaggttgccaggcttaaaaaaggcagtggctccggcggatccggaagcggaggcagcggatctggatctggtggttcaggatctggcggttctggtagcggggaagaactgttgagtaaaaactatcaccttgagaacgaggtcgcaaggttgaaaaaaggatccggctctggcggctccggaagtggcggatctggctccggtagcggaggatcaggatccggcggaagcggatcaggcgaggaactgctttccaaaaattaccacctcgagaatgaggtcgcccgcctgaaaaaaggatcaggttccggtggttctggcagcggtggttcaggctcaggcagcggcggtagcggtagcggtggaagcggaagcggaccaaaaaagaagagaaaggtaatggacaagaagtacagcatcggcctggccatcggcaccaactctgtgggctgggccgtgatcaccgacgagtacaaggtgcccagcaagaaattcaaggtgctgggcaacaccgaccggcacagcatcaagaagaacctgatcggcgccctgctgttcgacagcggagaaacagccgaggccacccggctgaagagaaccgccagaagaagatacaccagacggaagaaccggatctgctatctgcaagagatcttcagcaacgagatggccaaggtggacgacagcttcttccacagactggaagagtccttcctggtggaagaggataagaagcacgagcggcaccccatcttcggcaacatcgtggacgaggtggcctaccacgagaagtaccccaccatctaccacctgagaaagaaactggtggacagcaccgacaaggccgacctgcggctgatctatctggccctggcccacatgatcaagttccggggccacttcctgatcgagggcgacctgaaccccgacaacagcgacgtggacaagctgttcatccagctggtgcagacctacaaccagctgttcgaggaaaaccccatcaacgccagcggcgtggacgccaaggccatcctgtctgccagactgagcaagagcagacggctggaaaatctgatcgcccagctgcccggcgagaagaagaatggcctgttcggcaacctgattgccctgagcctgggcctgacccccaacttcaagagcaacttcgacctggccgaggatgccaaactgcagctgagcaaggacacctacgacgacgacctggacaacctgctggcccagatcggcgaccagtacgccgacctgtttctggccgccaagaacctgtccgacgccatcctgctgagcgacatcctgagagtgaacaccgagatcaccaaggcccccctgagcgcctctatgatcaagagatacgacgagcaccaccaggacctgaccctgctgaaagctctcgtgcggcagcagctgcctgagaagtacaaagagattttcttcgaccagagcaagaacggctacgccggctacatcgatggcggagccagccaggaagagttctacaagttcatcaagcccatcctggaaaagatggacggcaccgaggaactgctcgtgaagctgaacagagaggacctgctgcggaagcagcggaccttcgacaacggcagcatcccccaccagatccacctgggagagctgcacgccattctgcggcggcaggaagatttttacccattcctgaaggacaaccgggaaaagatcgagaagatcctgaccttccgcatcccctactacgtgggccctctggccaggggaaacagcagattcgcctggatgaccagaaagagcgaggaaaccatcaccccctggaacttcgaggaagtggtggacaagggcgccagcgcccagagcttcatcgagcggatgaccaacttcgataagaacctgcccaacgagaaggtgctgcccaagcacagcctgctgtacgagtacttcaccgtgtacaacgagctgaccaaagtgaaatacgtgaccgagggaatgagaaagcccgccttcctgagcggcgagcagaaaaaagccatcgtggacctgctgttcaagaccaaccggaaagtgaccgtgaagcagctgaaagaggactacttcaagaaaatcgagtgcttcgactccgtggaaatctccggcgtggaagatcggttcaacgcctccctgggcacataccacgatctgctgaaaattatcaaggacaaggacttcctggacaatgaggaaaacgaggacattctggaagatatcgtgctgaccctgacactgtttgaggacagagagatgatcgaggaacggctgaaaacctatgcccacctgttcgacgacaaagtgatgaagcagctgaagcggcggagatacaccggctggggcaggctgagccggaagctgatcaacggcatccgggacaagcagtccggcaagacaatcctggatttcctgaagtccgacggcttcgccaacagaaacttcatgcagctgatccacgacgacagcctgacctttaaagaggacatccagaaagcccaggtgtccggccagggcgatagcctgcacgagcacattgccaatctggccggcagccccgccattaagaagggcatcctgcagacagtgaaggtggtggacgagctcgtgaaagtgatgggccggcacaagcccgagaacatcgtgatcgaaatggccagagagaaccagaccacccagaagggacagaagaacagccgcgagagaatgaagcggatcgaagagggcatcaaagagctgggcagccagatcctgaaagaacaccccgtggaaaacacccagctgcagaacgagaagctgtacctgtactacctgcagaatgggcgggatatgtacgtggaccaggaactggacatcaaccggctgtccgactacgatgtggacgctatcgtgcctcagagctttctgaaggacgactccatcgataacaaagtgctgactcggagcgacaagaaccggggcaagagcgacaacgtgccctccgaagaggtcgtgaagaagatgaagaactactggcgccagctgctgaatgccaagctgattacccagaggaagttcgacaatctgaccaaggccgagagaggcggcctgagcgaactggataaggccggcttcatcaagagacagctggtggaaacccggcagatcacaaagcacgtggcacagatcctggactcccggatgaacactaagtacgacgagaacgacaaactgatccgggaagtgaaagtgatcaccctgaagtccaagctggtgtccgatttccggaaggatttccagttttacaaagtgcgcgagatcaacaactaccaccacgcccacgacgcctacctgaacgccgtcgtgggaaccgccctgatcaaaaagtaccctaagctggaaagcgagttcgtgtacggcgactacaaggtgtacgacgtgcggaagatgatcgccaagagcgagcaggaaatcggcaaggctaccgccaagtacttcttctacagcaacatcatgaactttttcaagaccgagattaccctggccaacggcgagatccggaagcggcctctgatcgagacaaacggcgaaacaggcgagatcgtgtgggataagggccgggactttgccaccgtgcggaaagtgctgtctatgccccaagtgaatatcgtgaaaaagaccgaggtgcagacaggcggcttcagcaaagagtctatcctgcccaagaggaacagcgacaagctgatcgccagaaagaaggactgggaccctaagaagtacggcggcttcgacagccccaccgtggcctattctgtgctggtggtggccaaagtggaaaagggcaagtccaagaaactgaagagtgtgaaagagctgctggggatcaccatcatggaaagaagcagcttcgagaagaatcccatcgactttctggaagccaagggctacaaagaagtgaaaaaggacctgatcatcaagctgcctaagtactccctgttcgagctggaaaacggccggaagagaatgctggcctctgccggcgaactgcagaagggaaacgaactggccctgccctccaaatatgtgaacttcctgtacctggccagccactatgagaagctgaagggctcccccgaggataatgagcagaaacagctgtttgtggaacagcacaaacactacctggacgagatcatcgagcagatcagcgagttctccaagagagtgatcctggccgacgctaatctggacaaggtgctgagcgcctacaacaagcacagagacaagcctatcagagagcaggccgagaatatcatccacctgtttaccctgaccaatctgggagcccctgccgccttcaagtactttgacaccaccatcgaccggaagaggtacaccagcaccaaagaggtgctggacgccaccctgatccaccagagcatcaccggcctgtacgagacacggatcgacctgtctcagctgggaggcgacgcctatccctatgacgtgcccgattatgccagcctgggcagcggctcccccaagaaaaaacgcaaggtggaagatcctaagaaaaagcggaaagtggacggcagcggcagcgagacccccggtaccagcgagagcgccacccccgagagccggacactggtgaccttcaaggatgtatttgtggacttcaccagggaggagtggaagctgctggacactgctcagcagatcgtgtacagaaatgtgatgctggagaactataagaacctggtttccttgggttatcagcttactaagccagatgtgatcctccggttggagaagggagaagagccctga

SEQ ID NO: 314 - DNA, 7827 bp, synthetic construct
  misc_feature 1..7827: note = CDS of V26_D3a-hD3L-scFv-2a-3xGCN4-dCas9-ZIM3
  source 1..7827: mol_type = other DNA
atgcctgctgctaagagagtgaaactggatggatccaaccatgaccaggaatttgaccccccaaaggtttacccacctgtgccagctgagaagaggaagcccatccgcgtgctgtctctctttgatgggattgctacagggctcctggtgctgaaggacctgggcatccaagtggaccgctacattgcctccgaggtgtgtgaggactccatcacggtgggcatggtgcggcaccagggaaagatcatgtacgtcggggacgtccgcagcgtcacacagaagcatatccaggagtggggcccattcgacctggtgattggaggcagtccctgcaatgacctctccattgtcaaccctgcccgcaagggactttatgagggtactggccgcctcttctttgagttctaccgcctcctgcatgatgcgcggcccaaggagggagatgatcgccccttcttctggctctttgagaatgtggtggccatgggcgttagtgacaagagggacatctcgcgatttcttgagtctaaccccgtgatgattgacgccaaagaagtgtctgctgcacacagggcccgttacttctggggtaaccttcctggcatgaacaggcctttggcatccactgtgaatgataagctggagctgcaagagtgtctggagcacggcagaatagccaagttcagcaaagtgaggaccattaccaccaggtcaaactctataaagcagggcaaagaccagcatttccccgtgttcatgaacgagaaggaggacatcctgtggtgcactgaaatggaaagggtgtttggcttccccgtccactacacagacgtctccaacatgagccgcttggcgaggcagagactgctgggccgatcgtggagcgtgccggtcatccgccacctcttcgctccgctgaaggaatattttgcttgtgtgtctagcggcaatagtaacgctaacagccgcgggccgagcttcagcagcggcctggtgccgttaagcttgcgcggcagccatatgttcgaaaccgtgcctgtgtggaggagacagccagtccgggtgctgtccctttttgaagacatcaagaaagagctgacgagtttgggctttttggaaagtggttctgacccgggacaactgaagcatgtggttgatgtcacagacacagtgaggaaggatgtggaggagtggggacccttcgatcttgtgtacggcgccacacctcccctgggccacacctgtgaccgtcctcccagctggtacctgttccagttccaccggctcctgcagtacgcacggcccaagccaggcagccccaggcccttcttctggatgttcgtggacaatctggtgctgaacaaggaagacctggacgtcgcatctcgcttcctggagatggagccagtcaccatcccagatgtccacggcggatccttgcagaatgctgtccgcgtgtggagcaacatcccagccataaggagcagcaggcactgggctctggtttcggaagaagaattgtccctgctggcccagaacaagcagagctcgaagctcgcggccaagtggcccaccaagctggtgaagaactgctttctccccctaagagaatatttcaagtatttttcaggagggccgagctctggcgcacccccaccaagtggagggtctcctgccgggtccccaacatctactgaagaaggcaccagcgaatccgcaacgcccgagtcaggccctggtacctccacagaaccatctgaaggtagtgcgcctggttccccagctggaagccctacttccaccgaagaaggcacgtcaaccgaaccaagtgaaggatctgcccctgggaccagcactgaaccatctgagccaaaaaagaagagaaaggtaccatctgagggccccgacatcgtgatgacccagagccccagcagcctgagcgccagcgtgggcgaccgcgtgaccatcacctgccgcagcagcaccggcgccgtgaccaccagcaactacgccagctgggtgcaggagaagcccggcaagctgttcaagggcctgatcggcggcaccaacaaccgcgcccccggcgtgcccagccgcttcagcggcagcctgatcggcgacaaggccaccctgaccatcagcagcctgcagcccgaggacttcgccacctacttctgcgccctgtggtacagcaaccactgggtgttcggccagggcaccaaggtggagctgaagcgcggcggcggcggcagcggcggcggcggcagcggcggcggcggcagcagcggcggcggcagcgaggtgaagctgctggagagcggcggcggcctggtgcagcccggcggcagcctgaagctgagctgcgccgtgagcggcttcagcctgaccgactacggcgtgaactgggtgcgccaggcccccggccgcggcctggagtggatcggcgtgatctggggcgacggcatcaccgactacaacagcgccctgaaggaccgcttcatcatcagcaaggacaacggcaagaacaccgtgtacctgcagatgagcaaggtgcgcagcgacgacaccgccctgtactactgcgtgaccggcctgttcgactactggggccagggcaccctggtgaccgtgagcagctacccatacgatgttccagattacgctggtggaggcggaggttctgggggaggaggtagtggcggtggtggttcaggaggcggcggaagcggaagcggagctactaacttcagcctgctgaagcaggctggagacgtggaggagaaccctggacctatgcctgctgctaagagagtgaaactggatggatccgaggaactgctgagcaagaactaccacctggaaaacgaggtggccagactgaagaaaggctctggctctggcggaagcggttctggcggatcaggatctggaagtggcggctctggaagcggaggttctggatctggcgaagaactgctgtctaagaattatcacctcgagaacgaagtggctcggctcaagaaaggcagtggcagcggaggaagtggatccggcggtagtggtagtggaagcggcggatccggctcaggcggatctggttcaggggaagaactcctctccaaaaactaccatctcgagaatgaggtcgcccgcctgaaaaaaggatcaggttccggtggttctggcagcggtggttcaggctcaggcagcggcggtagcggtagcggtggaagcggaagcggaccaaaaaagaagagaaaggtaatggacaagaagtacagcatcggcctggccatcggcaccaactctgtgggctgggccgtgatcaccgacgagtacaaggtgcccagcaagaaattcaaggtgctgggcaacaccgaccggcacagcatcaagaagaacctgatcggcgccctgctgttcgacagcggagaaacagccgaggccacccggctgaagagaaccgccagaagaagatacaccagacggaagaaccggatctgctatctgcaagagatcttcagcaacgagatggccaaggtggacgacagcttcttccacagactggaagagtccttcctggtggaagaggataagaagcacgagcggcaccccatcttcggcaacatcgtggacgaggtggcctaccacgagaagtaccccaccatctaccacctgagaaagaaactggtggacagcaccgacaaggccgacctgcggctgatctatctggccctggcccacatgatcaagttccggggccacttcctgatcgagggcgacctgaaccccgacaacagcgacgtggacaagctgttcatccagctggtgcagacctacaaccagctgttcgaggaaaaccccatcaacgccagcggcgtggacgccaaggccatcctgtctgccagactgagcaagagcagacggctggaaaatctgatcgcccagctgcccggcgagaagaagaatggcctgttcggcaacctgattgccctgagcctgggcctgacccccaacttcaagagcaacttcgacctggccgaggatgccaaactgcagctgagcaaggacacctacgacgacgacctggacaacctgctggcccagatcggcgaccagtacgccgacctgtttctggccgccaagaacctgtccgacgccatcctgctgagcgacatcctgagagtgaacaccgagatcaccaaggcccccctgagcgcctctatgatcaagagatacgacgagcaccaccaggacctgaccctgctgaaagctctcgtgcggcagcagctgcctgagaagtacaaagagattttcttcgaccagagcaagaacggctacgccggctacatcgatggcggagccagccaggaagagttctacaagttcatcaagcccatcctggaaaagatggacggcaccgaggaactgctcgtgaagctgaacagagaggacctgctgcggaagcagcggaccttcgacaacggcagcatcccccaccagatccacctgggagagctgcacgccattctgcggcggcaggaagatttttacccattcctgaaggacaaccgggaaaagatcgagaagatcctgaccttccgcatcccctactacgtgggccctctggccaggggaaacagcagattcgcctggatgaccagaaagagcgaggaaaccatcaccccctggaacttcgaggaagtggtggacaagggcgccagcgcccagagcttcatcgagcggatgaccaacttcgataagaacctgcccaacgagaaggtgctgcccaagcacagcctgctgtacgagtacttcaccgtgtacaacgagctgaccaaagtgaaatacgtgaccgagggaatgagaaagcccgccttcctgagcggcgagcagaaaaaagccatcgtggacctgctgttcaagaccaaccggaaagtgaccgtgaagcagctgaaagaggactacttcaagaaaatcgagtgcttcgactccgtggaaatctccggcgtggaagatcggttcaacgcctccctgggcacataccacgatctgctgaaaattatcaaggacaaggacttcctggacaatgaggaaaacgaggacattctggaagatatcgtgctgaccctgacactgtttgaggacagagagatgatcgaggaacggctgaaaacctatgcccacctgttcgacgacaaagtgatgaagcagctgaagcggcggagatacaccggctggggcaggctgagccggaagctgatcaacggcatccgggacaagcagtccggcaagacaatcctggatttcctgaagtccgacggcttcgccaacagaaacttcatgcagctgatccacgacgacagcctgacctttaaagaggacatccagaaagcccaggtgtccggccagggcgatagcctgcacgagcacattgccaatctggccggcagccccgccattaagaagggcatcctgcagacagtgaaggtggtggacgagctcgtgaaagtgatgggccggcacaagcccgagaacatcgtgatcgaaatggccagagagaaccagaccacccagaagggacagaagaacagccgcgagagaatgaagcggatcgaagagggcatcaaagagctgggcagccagatcctgaaagaacaccccgtggaaaacacccagctgcagaacgagaagctgtacctgtactacctgcagaatgggcgggatatgtacgtggaccaggaactggacatcaaccggctgtccgactacgatgtggacgctatcgtgcctcagagctttctgaaggacgactccatcgataacaaagtgctgactcggagcgacaagaaccggggcaagagcgacaacgtgccctccgaagaggtcgtgaagaagatgaagaactactggcgccagctgctgaatgccaagctgattacccagaggaagttcgacaatctgaccaaggccgagagaggcggcctgagcgaactggataaggccggcttcatcaagagacagctggtggaaacccggcagatcacaaagcacgtggcacagatcctggactcccggatgaacactaagtacgacgagaacgacaaactgatccgggaagtgaaagtgatcaccctgaagtccaagctggtgtccgatttccggaaggatttccagttttacaaagtgcgcgagatcaacaactaccaccacgcccacgacgcctacctgaacgccgtcgtgggaaccgccctgatcaaaaagtaccctaagctggaaagcgagttcgtgtacggcgactacaaggtgtacgacgtgcggaagatgatcgccaagagcgagcaggaaatcggcaaggctaccgccaagtacttcttctacagcaacatcatgaactttttcaagaccgagattaccctggccaacggcgagatccggaagcggcctctgatcgagacaaacggcgaaacaggcgagatcgtgtgggataagggccgggactttgccaccgtgcggaaagtgctgtctatgccccaagtgaatatcgtgaaaaagaccgaggtgcagacaggcggcttcagcaaagagtctatcctgcccaagaggaacagcgacaagctgatcgccagaaagaaggactgggaccctaagaagtacggcggcttcgacagccccaccgtggcctattctgtgctggtggtggccaaagtggaaaagggcaagtccaagaaactgaagagtgtgaaagagctgctggggatcaccatcatggaaagaagcagcttcgagaagaatcccatcgactttctggaagccaagggctacaaagaagtgaaaaaggacctgatcatcaagctgcctaagtactccctgttcgagctggaaaacggccggaagagaatgctggcctctgccggcgaactgcagaagggaaacgaactggccctgccctccaaatatgtgaacttcctgtacctggccagccactatgagaagctgaagggctcccccgaggataatgagcagaaacagctgtttgtggaacagcacaaacactacctggacgagatcatcgagcagatcagcgagttctccaagagagtgatcctggccgacgctaatctggacaaggtgctgagcgcctacaacaagcacagagacaagcctatcagagagcaggccgagaatatcatccacctgtttaccctgaccaatctgggagcccctgccgccttcaagtactttgacaccaccatcgaccggaagaggtacaccagcaccaaagaggtgctggacgccaccctgatccaccagagcatcaccggcctgtacgagacacggatcgacctgtctcagctgggaggcgacgcctatccctatgacgtgcccgattatgccagcctgggcagcggctcccccaagaaaaaacgcaaggtggaagatcctaagaaaaagcggaaagtggacggcagcggcagcgagacccccggtaccagcgagagcgccacccccgagagcatgaacaattcccagggaagagtgaccttcgaggatgtcactgtgaacttcacccagggggagtggcagcggctgaatcccgaacagagaaacttgtacagggatgtgatgctggagaattacagcaaccttgtctctgtgggacaaggggaaaccaccaaacccgatgtgatcttgaggttggaacaaggaaaggagccatggttggaggaagaggaagtgctgggaagtggccgtgcagaaaaaaatggggacattggagggcagatttggaagccaaaggatgtgaaagagagtctcctcgagtga

SEQ ID NO: 315 - DNA, 7827 bp, synthetic construct
  misc_feature 1..7827: note = CDS of V27_3xGCN4-dCas9-ZIM3-2a-D3a-hD3L-scFv
  source 1..7827: mol_type = other DNA
atgcctgctgctaagagagtgaaactggatggatccgaggaactgctgagcaagaactaccacctggaaaacgaggtggccagactgaagaaaggctctggctctggcggaagcggttctggcggatcaggatctggaagtggcggctctggaagcggaggttctggatctggcgaagaactgctgtctaagaattatcacctcgagaacgaagtggctcggctcaagaaaggcagtggcagcggaggaagtggatccggcggtagtggtagtggaagcggcggatccggctcaggcggatctggttcaggggaagaactcctctccaaaaactaccatctcgagaatgaggtcgcccgcctgaaaaaaggatcaggttccggtggttctggcagcggtggttcaggctcaggcagcggcggtagcggtagcggtggaagcggaagcggaccaaaaaagaagagaaaggtaatggacaagaagtacagcatcggcctggccatcggcaccaactctgtgggctgggccgtgatcaccgacgagtacaaggtgcccagcaagaaattcaaggtgctgggcaacaccgaccggcacagcatcaagaagaacctgatcggcgccctgctgttcgacagcggagaaacagccgaggccacccggctgaagagaaccgccagaagaagatacaccagacggaagaaccggatctgctatctgcaagagatcttcagcaacgagatggccaaggtggacgacagcttcttccacagactggaagagtccttcctggtggaagaggataagaagcacgagcggcaccccatcttcggcaacatcgtggacgaggtggcctaccacgagaagtaccccaccatctaccacctgagaaagaaactggtggacagcaccgacaaggccgacctgcggctgatctatctggccctggcccacatgatcaagttccggggccacttcctgatcgagggcgacctgaaccccgacaacagcgacgtggacaagctgttcatccagctggtgcagacctacaaccagctgttcgaggaaaaccccatcaacgccagcggcgtggacgccaaggccatcctgtctgccagactgagcaagagcagacggctggaaaatctgatcgcccagctgcccggcgagaagaagaatggcctgttcggcaacctgattgccctgagcctgggcctgacccccaacttcaagagcaacttcgacctggccgaggatgccaaactgcagctgagcaaggacacctacgacgacgacctggacaacctgctggcccagatcggcgaccagtacgccgacctgtttctggccgccaagaacctgtccgacgccatcctgctgagcgacatcctgagagtgaacaccgagatcaccaaggcccccctgagcgcctctatgatcaagagatacgacgagcaccaccaggacctgaccctgctgaaagctctcgtgcggcagcagctgcctgagaagtacaaagagattttcttcgaccagagcaagaacggctacgccggctacatcgatggcggagccagccaggaagagttctacaagttcatcaagcccatcctggaaaagatggacggcaccgaggaactgctcgtgaagctgaacagagaggacctgctgcggaagcagcggaccttcgacaacggcagcatcccccaccagatccacctgggagagctgcacgccattctgcggcggcaggaagatttttacccattcctgaaggacaaccgggaaaagatcgagaagatcctgaccttccgcatcccctactacgtgggccctctggccaggggaaacagcagattcgcctggatgaccagaaagagcgaggaaaccatcaccccctggaacttcgaggaagtggtggacaagggcgccagcgcccagagcttcatcgagcggatgaccaacttcgataagaacctgcccaacgagaaggtgctgcccaagcacagcctgctgtacgagtacttcaccgtgtacaacgagctgaccaaagtgaaatacgtgaccgagggaatgagaaagcccgccttcctgagcggcgagcagaaaaaagccatcgtggacctgctgttcaagaccaaccggaaagtgaccgtgaagcagctgaaagaggactacttcaagaaaatcgagtgcttcgactccgtggaaatctccggcgtggaagatcggttcaacgcctccctgggcacataccacgatctgctgaaaattatcaaggacaaggacttcctggacaatgaggaaaacgaggacattctggaagatatcgtgctgaccctgacactgtttgaggacagagagatgatcgaggaacggctgaaaacctatgcccacctgttcgacgacaaagtgatgaagcagctgaagcggcggagatacaccggctggggcaggctgagccggaagctgatcaacggcatccgggacaagcagtccggcaagacaatcctggatttcctgaagtccgacggcttcgccaacagaaacttcatgcagctgatccacgacgacagcctgacctttaaagaggacatccagaaagcccaggtgtccggccagggcgatagcctgcacgagcacattgccaatctggccggcagccccgccattaagaagggcatcctgcagacagtgaaggtggtggacgagctcgtgaaagtgatgggccggcacaagcccgagaacatcgtgatcgaaatggccagagagaaccagaccacccagaagggacagaagaacagccgcgagagaatgaagcggatcgaagagggcatcaaagagctgggcagccagatcctgaaagaacaccccgtggaaaacacccagctgcagaacgagaagctgtacctgtactacctgcagaatgggcgggatatgtacgtggaccaggaactggacatcaaccggctgtccgactacgatgtggacgctatcgtgcctcagagctttctgaaggacgactccatcgataacaaagtgctgactcggagcgacaagaaccggggcaagagcgacaacgtgccctccgaagaggtcgtgaagaagatgaagaactactggcgccagctgctgaatgccaagctgattacccagaggaagttcgacaatctgaccaaggccgagagaggcggcctgagcgaactggataaggccggcttcatcaagagacagctggtggaaacccggcagatcacaaagcacgtggcacagatcctggactcccggatgaacactaagtacgacgagaacgacaaactgatccgggaagtgaaagtgatcaccctgaagtccaagctggtgtccgatttccggaaggatttccagttttacaaagtgcgcgagatcaacaactaccaccacgcccacgacgcctacctgaacgccgtcgtgggaaccgccctgatcaaaaagtaccctaagctggaaagcgagttcgtgtacggcgactacaaggtgtacgacgtgcggaagatgatcgccaagagcgagcaggaaatcggcaaggctaccgccaagtacttcttctacagcaacatcatgaactttttcaagaccgagattaccctggccaacggcgagatccggaagcggcctctgatcgagacaaacggcgaaacaggcgagatcgtgtgggataagggccgggactttgccaccgtgcggaaagtgctgtctatgccccaagtgaatatcgtgaaaaagaccgaggtgcagacaggcggcttcagcaaagagtctatcctgcccaagaggaacagcgacaagctgatcgccagaaagaaggactgggaccctaagaagtacggcggcttcgacagccccaccgtggcctattctgtgctggtggtggccaaagtggaaaagggcaagtccaagaaactgaagagtgtgaaagagctgctggggatcaccatcatggaaagaagcagcttcgagaagaatcccatcgactttctggaagccaagggctacaaagaagtgaaaaaggacctgatcatcaagctgcctaagtactccctgttcgagctggaaaacggccggaagagaatgctggcctctgccggcgaactgcagaagggaaacgaactggccctgccctccaaatatgtgaacttcctgtacctggccagccactatgagaagctgaagggctcccccgaggataatgagcagaaacagctgtttgtggaacagcacaaacactacctggacgagatcatcgagcagatcagcgagttctccaagagagtgatcctggccgacgctaatctggacaaggtgctgagcgcctacaacaagcacagagacaagcctatcagagagcaggccgagaatatcatccacctgtttaccctgaccaatctgggagcccctgccgccttcaagtactttgacaccaccatcgaccggaagaggtacaccagcaccaaagaggtgctggacgccaccctgatccaccagagcatcaccggcctgtacgagacacggatcgacctgtctcagctgggaggcgacgcctatccctatgacgtgcccgattatgccagcctgggcagcggctcccccaagaaaaaacgcaaggtggaagatcctaagaaaaagcggaaagtggacggcagcggcagcgagacccccggtaccagcgagagcgccacccccgagagcatgaacaattcccagggaagagtgaccttcgaggatgtcactgtgaacttcacccagggggagtggcagcggctgaatcccgaacagagaaacttgtacagggatgtgatgctggagaattacagcaaccttgtctctgtgggacaaggggaaaccaccaaacccgatgtgatcttgaggttggaacaaggaaaggagccatggttggaggaagaggaagtgctgggaagtggccgtgcagaaaaaaatggggacattggagggcagatttggaagccaaaggatgtgaaagagagtctcctcgagggaagcggagctactaacttcagcctgctgaagcaggctggagacgtggaggagaaccctggacctatgcctgctgctaagagagtgaaactggatggatccaaccatgaccaggaatttgaccccccaaaggtttacccacctgtgccagctgagaagaggaagcccatccgcgtgctgtctctctttgatgggattgctacagggctcctggtgctgaaggacctgggcatccaagtggaccgctacattgcctccgaggtgtgtgaggactccatcacggtgggcatggtgcggcaccagggaaagatcatgtacgtcggggacgtccgcagcgtcacacagaagcatatccaggagtggggcccattcgacctggtgattggaggcagtccctgcaatgacctctccattgtcaaccctgcccgcaagggactttatgagggtactggccgcctcttctttgagttctaccgcctcctgcatgatgcgcggcccaaggagggagatgatcgccccttcttctggctctttgagaatgtggtggccatgggcgttagtgacaagagggacatctcgcgatttcttgagtctaaccccgtgatgattgacgccaaagaagtgtctgctgcacacagggcccgttacttctggggtaaccttcctggcatgaacaggcctttggcatccactgtgaatgataagctggagctgcaagagtgtctggagcacggcagaatagccaagttcagcaaagtgaggaccattaccaccaggtcaaactctataaagcagggcaaagaccagcatttccccgtgttcatgaacgagaaggaggacatcctgtggtgcactgaaatggaaagggtgtttggcttccccgtccactacacagacgtctccaacatgagccgcttggcgaggcagagactgctgggccgatcgtggagcgtgccggtcatccgccacctcttcgctccgctgaaggaatattttgcttgtgtgtctagcggcaatagtaacgctaacagccgcgggccgagcttcagcagcggcctggtgccgttaagcttgcgcggcagccatatgttcgaaaccgtgcctgtgtggaggagacagccagtccgggtgctgtccctttttgaagacatcaagaaagagctgacgagtttgggctttttggaaagtggttctgacccgggacaactgaagcatgtggttgatgtcacagacacagtgaggaaggatgtggaggagtggggacccttcgatcttgtgtacggcgccacacctcccctgggccacacctgtgaccgtcctcccagctggtacctgttccagttccaccggctcctgcagtacgcacggcccaagccaggcagccccaggcccttcttctggatgttcgtggacaatctggtgctgaacaaggaagacctggacgtcgcatctcgcttcctggagatggagccagtcaccatcccagatgtccacggcggatccttgcagaatgctgtccgcgtgtggagcaacatcccagccataaggagcagcaggcactgggctctggtttcggaagaagaattgtccctgctggcccagaacaagcagagctcgaagctcgcggccaagtggcccaccaagctggtgaagaactgctttctccccctaagagaatatttcaagtatttttcaggagggccgagctctggcgcacccccaccaagtggagggtctcctgccgggtccccaacatctactgaagaaggcaccagcgaatccgcaacgcccgagtcaggccctggtacctccacagaaccatctgaaggtagtgcgcctggttccccagctggaagccctacttccaccgaagaaggcacgtcaaccgaaccaagtgaaggatctgcccctgggaccagcactgaaccatctgagccaaaaaagaagagaaaggtaccatctgagggccccgacatcgtgatgacccagagccccagcagcctgagcgccagcgtgggcgaccgcgtgaccatcacctgccgcagcagcaccggcgccgtgaccaccagcaactacgccagctgggtgcaggagaagcccggcaagctgttcaagggcctgatcggcggcaccaacaaccgcgcccccggcgtgcccagccgcttcagcggcagcctgatcggcgacaaggccaccctgaccatcagcagcctgcagcccgaggacttcgccacctacttctgcgccctgtggtacagcaaccactgggtgttcggccagggcaccaaggtggagctgaagcgcggcggcggcggcagcggcggcggcggcagcggcggcggcggcagcagcggcggcggcagcgaggtgaagctgctggagagcggcggcggcctggtgcagcccggcggcagcctgaagctgagctgcgccgtgagcggcttcagcctgaccgactacggcgtgaactgggtgcgccaggcccccggccgcggcctggagtggatcggcgtgatctggggcgacggcatcaccgactacaacagcgccctgaaggaccgcttcatcatcagcaaggacaacggcaagaacaccgtgtacctgcagatgagcaaggtgcgcagcgacgacaccgccctgtactactgcgtgaccggcctgttcgactactggggccagggcaccctggtgaccgtgagcagctacccatacgatgttccagattacgctggtggaggcggaggttctgggggaggaggtagtggcggtggtggttcaggaggcggcggaagctga

SEQ ID NO: 316 - DNA, 7407 bp, synthetic construct
  misc_feature 1..7407: note = CDS of V28_3xGCN4-dCas12a-ZIM3-2a-D3a-hD3L-scFv
  source 1..7407: mol_type = other DNA
atgcctgctgctaagagagtgaaactggatggatccgaggaactgctgagcaagaactaccacctggaaaacgaggtggccagactgaagaaaggctctggctctggcggaagcggttctggcggatcaggatctggaagtggcggctctggaagcggaggttctggatctggcgaagaactgctgtctaagaattatcacctcgagaacgaagtggctcggctcaagaaaggcagtggcagcggaggaagtggatccggcggtagtggtagtggaagcggcggatccggctcaggcggatctggttcaggggaagaactcctctccaaaaactaccatctcgagaatgaggtcgcccgcctgaaaaaaggatcaggttccggtggttctggcagcggtggttcaggctcaggcagcggcggtagcggtagcggtggaagcggaagcggaccaaaaaagaagagaaaggtaatgtcaaagctggagaaattcaccaactgttatagcctgtctaagaccctgcgcttcaaggcaatcccagtgggcaagacacaagagaacattgacaacaaacggctcctggtggaggatgagaagagggctgaagattacaagggcgttaagaagctgctggataggtactatctgtcattcatcaacgatgtcctccacagtatcaagctgaagaatctgaacaattacatttctctgttccggaagaagacacggaccgagaaggagaacaaagagctggagaatctggagatcaacctgaggaaagaaatagctaaggctttcaaagggaacgagggttacaagtccctgttcaagaaagacattatcgagactattctgcctgagttcctggacgataaagatgagatcgccctcgtcaattccttcaatgggtttaccacagcctttaccggcttcttcgacaatagagagaatatgttctctgaagaggccaaatccactagcatcgcctttcgctgcataaacgagaacctgactaggtacatcagcaatatggacatctttgagaaagtcgatgccatattcgacaaacatgaggtgcaggagattaaggagaagatcctgaactcagattacgatgtcgaagatttcttcgagggagagttcttcaacttcgtgctcacacaagagggcattgatgtgtacaatgcaatcattggagggttcgtgacagagagtggcgagaagataaagggcctgaacgagtatatcaacctctacaaccagaaaaccaagcagaaactgcctaagttcaagccactgtacaaacaagtgctctcagatagggaaagcctgagcttctacggtgaagggtatacatcagatgaagaagtgctcgaagtgttccgcaacaccctcaataagaacagtgaaatcttctcttcaatcaagaagctggagaaactgttcaagaatttcgatgagtactcctctgccggaatctttgtgaagaatggccctgcaatatccactattagcaaagacatctttggcgagtggaacgttatcagggataagtggaatgccgagtacgatgatattcatctcaagaagaaagccgtggttacagagaaatacgaggatgatagacgcaagagctttaagaagattggtagcttctctctcgaacagctgcaggagtacgccgacgctgacctgtcagtcgtggagaaactcaaggagatcataatccagaaggtggatgaaatctacaaagtgtatggaagctctgagaaactcttcgatgcagactttgttctggagaagagtctgaagaagaacgacgcagtggttgctatcatgaaggacctgctggattctgttaagtctttcgagaattacattaaggcattctttggtgaagggaaggagacaaatagggacgagagcttctatggcgactttgttctggcctacgacatcctcctcaaggttgaccacatctatgacgctatacggaattacgttacccagaagccctatagcaaagacaagttcaagctgtatttccagaatccacagtttatgggtgggtgggataaagacaaagaaacagattacagggccactatcctgcggtacggcagcaaatactatctggctatcatggataagaagtacgccaaatgcctccagaagatcgacaaggacgacgtgaacggtaactacgagaagatcaattacaagctcctgccaggacctaacaagatgctgcccaaggtgttcttctccaagaaatggatggcctactataacccaagcgaggacattcagaagatatacaagaatgggacattcaagaagggcgatatgttcaacctcaacgactgccacaagctgattgatttcttcaaggatagcatttctcgctatcccaagtggtctaatgcatacgatttcaacttcagcgagactgagaagtacaaagacatcgctggcttctaccgggaggtggaagagcaaggctataaggtgtcattcgaatccgcttctaagaaggaagtggataagctcgtggaagagggtaagctgtacatgttccagatatacaacaaagacttcagcgataagagccacggcactccaaacctccatactatgtatttcaagctgctgtttgacgagaacaaccacggacagattaggctgtcaggaggcgcagaactcttcatgcgcagagcttcactgaagaaggaggaactcgttgtccacccagccaatagccctatagccaataagaatccagacaatcctaagaaaaccactactctgtcttacgatgtgtataaggataagagattctctgaagatcagtacgaactgcacatacccattgccattaacaagtgccctaagaacatcttcaagattaacacagaggttagagtgctcctgaaacacgacgataacccttatgttataggcattgctcgcggagagagaaacctgctgtacatcgtcgtggtggacggcaaaggcaacatcgtggaacagtacagtctcaatgaaatcattaacaatttcaacggaatccgcattaagaccgactaccattctctcctcgacaagaaggagaaagaaaggttcgaagcaagacagaattggacaagtatagagaatatcaaagaactgaaggctgggtacatctctcaggttgtgcacaagatatgtgagctggtggagaagtacgacgctgttatcgccctcgcggacctgaatagcggcttcaagaactccagggtgaaggtggagaagcaggtgtatcagaagttcgagaagatgctgatcgacaagctcaactatatggtggacaagaaatccaatccttgcgctactggtggagccctgaagggctatcaaatcaccaataagttcgaatctttcaagtctatgagcacccagaatggcttcatcttctacatacccgcatggctgacatccaagattgatccctctaccggatttgttaatctgctcaagactaagtacacctctattgctgactcaaagaagttcatatcatcatttgaccgcatcatgtacgtgccagaagaggacctgttcgagtttgccctggattacaagaatttctctcggactgacgccgactacatcaagaagtggaagctctactcttatggtaatcggattcgcatattccgcaatcccaagaagaataacgtgttcgattgggaggaagtttgcctcaccagcgcttacaaggagctgttcaataagtatgggattaactaccagcagggcgacataagagccctgctgtgcgaacaatctgataaggcattctattcctctttcatggcactgatgtcactgatgctgcaaatgcgcaattccatcaccggaagaacagacgtggcctttctgatctctcctgtcaagaactcagatggcatcttctacgattcccgcaactatgaagcacaggagaatgctatcctgcctaagaatgccgatgcaaatggagcctataacatcgccagaaaggtcctctgggccataggacaattcaagaaagctgaagatgagaagctggacaaggtgaagatcgccatttcaaacaaagagtggctcgaatatgctcagacctcagtgaagcatgcctatccctatgacgtgcccgattatgccagcctgggcagcggctcccccaagaaaaaacgcaaggtggaagatcctaagaaaaagcggaaagtggacggcagcggcagcgagacccccggtaccagcgagagcgccacccccgagagcatgaacaattcccagggaagagtgaccttcgaggatgtcactgtgaacttcacccagggggagtggcagcggctgaatcccgaacagagaaacttgtacagggatgtgatgctggagaattacagcaaccttgtctctgtgggacaaggggaaaccaccaaacccgatgtgatcttgaggttggaacaaggaaaggagccatggttggaggaagaggaagtgctgggaagtggccgtgcagaaaaaaatggggacattggagggcagatttggaagccaaaggatgtgaaagagagtctcctcgagggaagcggagctactaacttcagcctgctgaagcaggctggagacgtggaggagaaccctggacctatgcctgctgctaagagagtgaaactggatggatccaaccatgaccaggaatttgaccccccaaaggtttacccacctgtgccagctgagaagaggaagcccatccgcgtgctgtctctctttgatgggattgctacagggctcctggtgctgaaggacctgggcatccaagtggaccgctacattgcctccgaggtgtgtgaggactccatcacggtgggcatggtgcggcaccagggaaagatcatgtacgtcggggacgtccgcagcgtcacacagaagcatatccaggagtggggcccattcgacctggtgattggaggcagtccctgcaatgacctctccattgtcaaccctgcccgcaagggactttatgagggtactggccgcctcttctttgagttctaccgcctcctgcatgatgcgcggcccaaggagggagatgatcgccccttcttctggctctttgagaatgtggtggccatgggcgttagtgacaagagggacatctcgcgatttcttgagtctaaccccgtgatgattgacgccaaagaagtgtctgctgcacacagggcccgttacttctggggtaaccttcctggcatgaacaggcctttggcatccactgtgaatgataagctggagctgcaagagtgtctggagcacggcagaatagccaagttcagcaaagtgaggaccattaccaccaggtcaaactctataaagcagggcaaagaccagcatttccccgtgttcatgaacgagaaggaggacatcctgtggtgcactgaaatggaaagggtgtttggcttccccgtccactacacagacgtctccaacatgagccgcttggcgaggcagagactgctgggccgatcgtggagcgtgccggtcatccgccacctcttcgctccgctgaaggaatattttgcttgtgtgtctagcggcaatagtaacgctaacagccgcgggccgagcttcagcagcggcctggtgccgttaagcttgcgcggcagccatatgttcgaaaccgtgcctgtgtggaggagacagccagtccgggtgctgtccctttttgaagacatcaagaaagagctgacgagtttgggctttttggaaagtggttctgacccgggacaactgaagcatgtggttgatgtcacagacacagtgaggaaggatgtggaggagtggggacccttcgatcttgtgtacggcgccacacctcccctgggccacacctgtgaccgtcctcccagctggtacctgttccagttccaccggctcctgcagtacgcacggcccaagccaggcagccccaggcccttcttctggatgttcgtggacaatctggtgctgaacaaggaagacctggacgtcgcatctcgcttcctggagatggagccagtcaccatcccagatgtccacggcggatccttgcagaatgctgtccgcgtgtggagcaacatcccagccataaggagcagcaggcactgggctctggtttcggaagaagaattgtccctgctggcccagaacaagcagagctcgaagctcgcggccaagtggcccaccaagctggtgaagaactgctttctccccctaagagaatatttcaagtatttttcaggagggccgagctctggcgcacccccaccaagtggagggtctcctgccgggtccccaacatctactgaagaaggcaccagcgaatccgcaacgcccgagtcaggccctggtacctccacagaaccatctgaaggtagtgcgcctggttccccagctggaagccctacttccaccgaagaaggcacgtcaaccgaaccaagtgaaggatctgcccctgggaccagcactgaaccatctgagccaaaaaagaagagaaaggtaccatctgagggccccgacatcgtgatgacccagagccccagcagcctgagcgccagcgtgggcgaccgcgtgaccatcacctgccgcagcagcaccggcgccgtgaccaccagcaactacgccagctgggtgcaggagaagcccggcaagctgttcaagggcctgatcggcggcaccaacaaccgcgcccccggcgtgcccagccgcttcagcggcagcctgatcggcgacaaggccaccctgaccatcagcagcctgcagcccgaggacttcgccacctacttctgcgccctgtggtacagcaaccactgggtgttcggccagggcaccaaggtggagctgaagcgcggcggcggcggcagcggcggcggcggcagcggcggcggcggcagcagcggcggcggcagcgaggtgaagctgctggagagcggcggcggcctggtgcagcccggcggcagcctgaagctgagctgcgccgtgagcggcttcagcctgaccgactacggcgtgaactgggtgcgccaggcccccggccgcggcctggagtggatcggcgtgatctggggcgacggcatcaccgactacaacagcgccctgaaggaccgcttcatcatcagcaaggacaacggcaagaacaccgtgtacctgcagatgagcaaggtgcgcagcgacgacaccgccctgtactactgcgtgaccggcctgttcgactactggggccagggcaccctggtgaccgtgagcagctacccatacgatgttccagattacgctggtggaggcggaggttctgggggaggaggtagtggcggtggtggttcaggaggcggcggaagctga

SEQ ID NO: 317 - DNA, 6756 bp, synthetic construct
  misc_feature 1..6756: note = CDS of V29_3xGCN4-dCas12i-ZIM3-2a-D3a-hD3L-scFv
  source 1..6756: mol_type = other DNA
atgcctgctgctaagagagtgaaactggatggatccgaggaactgctgagcaagaactaccacctggaaaacgaggtggccagactgaagaaaggctctggctctggcggaagcggttctggcggatcaggatctggaagtggcggctctggaagcggaggttctggatctggcgaagaactgctgtctaagaattatcacctcgagaacgaagtggctcggctcaagaaaggcagtggcagcggaggaagtggatccggcggtagtggtagtggaagcggcggatccggctcaggcggatctggttcaggggaagaactcctctccaaaaactaccatctcgagaatgaggtcgcccgcctgaaaaaaggatcaggttccggtggttctggcagcggtggttcaggctcaggcagcggcggtagcggtagcggtggaagcggaagcggaccaaaaaagaagagaaaggtaatgggcatcaccatgagcgacaccaccttcagaccctacaagagcaagctgaaccccaacgagcggaagatgcctatggtggtggacaccatgaattggtgcgacaacgcctgcagcgtgttcttcgatctgttcgtgggcctgtacggcggcgtgaagatcggcgacgtgaccaatttcctgaccgagaagcaggacaccaccaccgatgccgatctgctgtgcgccatcaactggttcagagccatgcctgtgtctaaccccgatgccgttgtgggacctgagcagctggttgtgcggttcagagactacagcggccacaatccatctccaatggccagcatgtacctgagcgcccctgtgaaccctagatacacctgggtcgactgccggttcctgtaccagcagatgtgtcagaccctgggcgccaacctggatgtggacatctctaccctggtgcagaccggcctgctgcctatccagaaggatacacagctgaacgcctacagcttctgcagcaacgtgttcggcgagggcgtgaaagaagatcccagcgccaaagtgaccagctacacagccgctgccaatgctctgagcggcgccaccaatcctatcatcacctacgaggactaccggcagatcctgtccagcgccatcaccaacagacccagcagaaagggcgccaaggatattctggccgccgatctggatagcaccaagacaggtgttctgcccggcaactacgtgtcccagagaatcgccatgtaccaggcctctgccgcctctaaagctagaggcgtggtgctgcccaaccggctgagagtgaaagcctacctgcagaacctcgtgggactgaactacatctgcaccacctgggccgctcctatgctgagagccgtgggcgacatcaagagcaagaacagcaacaactaccgcttcgtgggcgagagactggaacggcagcaagagatcgataacctgctggccgtgtccaacatcagaagcgcccaggccatcctgcagcagttcagggccaatgagagcaaccagttctacatcaagaagcggcacatcggcaagggcctgcctagcctgtacgacatgtgggatctgatggacgagaaagagggcatcgacaactacatccagagcctgaagggcgacaagaccgagaggctgccaatcagagagctgctgcagatcatctaccctcacagaaagagcgtgtccgccgagctgtttctgtctgccgccgaactgaccgacgtggaagatagacagaaccggtgcatggtgcaccctacagtgcggggctctctggtcatcaacttcggcaagagcagcaccatcttcggcgctatcacccctcctgacacactgatcaagttccggggcgaaatggtgcctgctggacagacaggcatgatctggttcacaatgcacctggtggacggcggcaaatgggtcaagcaccacattccttgccacagcagccggtacttcgaggaaatctacgcctggaagaaggacctgcctacactgccctttccacggcggagcctgtatggctatgccatcggcaacaagatcagcgacacccggaagatcgacctgcggagaaagaaggccagcaagcagtacctgcggaccctggaaaacatgacccacaacgtggaatttgaccccaccacacagttcatggtggaccaagagctgaacgtgaccatcaccgccagagtgaagaaaatccctcctgtgcgggatgtgcccgtgggcagcagaattatgggcctgaacaagaaccagaccatccgggactgctacagcatctgggagagagtggaagccaacaccagcggcagctttcagcatcccgtggtccaggatgtgtggctgagactggtggccgatggccacgtgacctctacagtgaatggccccaacggccagatcgaccagatgagctactctggccccgatgtggccaactgcggcaactggatgcaagagcggagcaacttcatcaccagcgtggacgacgccgaccagtctatcatgaagcactttctgtggaacaaccgcgtgaagctgtatgcctggaactgcgtgtacgccggcacactgatgaaggccatctctaagcagatgaccaccgccaaccggaacctgttcagaaacgagatcctgagcttcgttggcggcagattcggctgcagactgggatctctggcccaggtttcactggacctgctgcggaggatgaagtccgtgatcagctgctacttcagccggaacaacgccttcaccatcgaggaaagaagcgccttcgacaaagaactgatggaactgttcgagagcctggacaacaagatgaacaacaagcggaaagagaaagtcaaccggacactcagcagcatcttccaggtggccaagcagcacaatgttgtgcggctggtggtcaccaagaacctgcagacccctgatgccaatgtgcggagcgtgatgaatcagagatccgtggattggtgcgctcggaagattgaagagaagatcgtggacctgggcaacgtgatcggaatctatgtggatctggtggaagccctggatctgagccatctggaccccttcatctatatcgccaagggcgacgtgggcaaagagtgccagtttgacgaggtggaaagcagctccctgctgccaattcacaccagcatgtttcgcgactggcacggcctggttaacaagggcagaaccaccacacctatctaccacagcgccctgaggagcttcgccagccactacggcctgagattcgatgacctggccagaatcaaggccgctgagctggccaaaatgctgccagaccagaaggtgttcatcccacacagaggcggacggttcttcatgagcacataccccgtgaccagcaccagcagacccgtgtcttatgatggccggcagcggttcctgaacagcggcgatatggtggccccagtgaacaccatgctgcgcggattcagaagggccagatctgcctatccctatgacgtgcccgattatgccagcctgggcagcggctcccccaagaaaaaacgcaaggtggaagatcctaagaaaaagcggaaagtggacggcagcggcagcgagacccccggtaccagcgagagcgccacccccgagagcatgaacaattcccagggaagagtgaccttcgaggatgtcactgtgaacttcacccagggggagtggcagcggctgaatcccgaacagagaaacttgtacagggatgtgatgctggagaattacagcaaccttgtctctgtgggacaaggggaaaccaccaaacccgatgtgatcttgaggttggaacaaggaaaggagccatggttggaggaagaggaagtgctgggaagtggccgtgcagaaaaaaatggggacattggagggcagatttggaagccaaaggatgtgaaagagagtctcctcgagggaagcggagctactaacttcagcctgctgaagcaggctggagacgtggaggagaaccctggacctatgcctgctgctaagagagtgaaactggatggatccaaccatgaccaggaatttgaccccccaaaggtttacccacctgtgccagctgagaagaggaagcccatccgcgtgctgtctctctttgatgggattgctacagggctcctggtgctgaaggacctgggcatccaagtggaccgctacattgcctccgaggtgtgtgaggactccatcacggtgggcatggtgcggcaccagggaaagatcatgtacgtcggggacgtccgcagcgtcacacagaagcatatccaggagtggggcccattcgacctggtgattggaggcagtccctgcaatgacctctccattgtcaaccctgcccgcaagggactttatgagggtactggccgcctcttctttgagttctaccgcctcctgcatgatgcgcggcccaaggagggagatgatcgccccttcttctggctctttgagaatgtggtggccatgggcgttagtgacaagagggacatctcgcgatttcttgagtctaaccccgtgatgattgacgccaaagaagtgtctgctgcacacagggcccgttacttctggggtaaccttcctggcatgaacaggcctttggcatccactgtgaatgataagctggagctgcaagagtgtctggagcacggcagaatagccaagttcagcaaagtgaggaccattaccaccaggtcaaactctataaagcagggcaaagaccagcatttccccgtgttcatgaacgagaaggaggacatcctgtggtgcactgaaatggaaagggtgtttggcttccccgtccactacacagacgtctccaacatgagccgcttggcgaggcagagactgctgggccgatcgtggagcgtgccggtcatccgccacctcttcgctccgctgaaggaatattttgcttgtgtgtctagcggcaatagtaacgctaacagccgcgggccgagcttcagcagcggcctggtgccgttaagcttgcgcggcagccatatgttcgaaaccgtgcctgtgtggaggagacagccagtccgggtgctgtccctttttgaagacatcaagaaagagctgacgagtttgggctttttggaaagtggttctgacccgggacaactgaagcatgtggttgatgtcacagacacagtgaggaaggatgtggaggagtggggacccttcgatcttgtgtacggcgccacacctcccctgggccacacctgtgaccgtcctcccagctggtacctgttccagttccaccggctcctgcagtacgcacggcccaagccaggcagccccaggcccttcttctggatgttcgtggacaatctggtgctgaacaaggaagacctggacgtcgcatctcgcttcctggagatggagccagtcaccatcccagatgtccacggcggatccttgcagaatgctgtccgcgtgtggagcaacatcccagccataaggagcagcaggcactgggctctggtttcggaagaagaattgtccctgctggcccagaacaagcagagctcgaagctcgcggccaagtggcccaccaagctggtgaagaactgctttctccccctaagagaatatttcaagtatttttcaggagggccgagctctggcgcacccccaccaagtggagggtctcctgccgggtccccaacatctactgaagaaggcaccagcgaatccgcaacgcccgagtcaggccctggtacctccacagaaccatctgaaggtagtgcgcctggttccccagctggaagccctacttccaccgaagaaggcacgtcaaccgaaccaagtgaaggatctgcccctgggaccagcactgaaccatctgagccaaaaaagaagagaaaggtaccatctgagggccccgacatcgtgatgacccagagccccagcagcctgagcgccagcgtgggcgaccgcgtgaccatcacctgccgcagcagcaccggcgccgtgaccaccagcaactacgccagctgggtgcaggagaagcccggcaagctgttcaagggcctgatcggcggcaccaacaaccgcgcccccggcgtgcccagccgcttcagcggcagcctgatcggcgacaaggccaccctgaccatcagcagcctgcagcccgaggacttcgccacctacttctgcgccctgtggtacagcaaccactgggtgttcggccagggcaccaaggtggagctgaagcgcggcggcggcggcagcggcggcggcggcagcggcggcggcggcagcagcggcggcggcagcgaggtgaagctgctggagagcggcggcggcctggtgcagcccggcggcagcctgaagctgagctgcgccgtgagcggcttcagcctgaccgactacggcgtgaactgggtgcgccaggcccccggccgcggcctggagtggatcggcgtgatctggggcgacggcatcaccgactacaacagcgccctgaaggaccgcttcatcatcagcaaggacaacggcaagaacaccgtgtacctgcagatgagcaaggtgcgcagcgacgacaccgccctgtactactgcgtgaccggcctgttcgactactggggccagggcaccctggtgaccgtgagcagctacccatacgatgttccagattacgctggtggaggcggaggttctgggggaggaggtagtggcggtggtggttcaggaggcggcggaagctga

SEQ ID NO: 318 - DNA, 8727 bp, synthetic construct
  misc_feature 1..8727: note = CDS of V30_10xGCN4-dCas9-ZIM3-2a-D3a-hD3L-scFv
  source 1..8727: mol_type = other DNA
atgcctgctgctaagagagtgaaactggatggatccgaggaactgctgagcaagaactaccacctggaaaacgaggtggccagactgaagaaaggctctggctctggcggaagcggttctggcggatcaggatctggaagtggcggctctggaagcggaggttctggatctggcgaagaactgctgtctaagaattatcacctcgagaacgaagtggctcggctcaagaaaggcagtggcagcggaggaagtggatccggcggtagtggtagtggaagcggcggatccggctcaggcggatctggttcaggggaagaactcctctccaaaaactaccatctcgagaatgaggtcgcccgcctgaaaaaaggatcaggttccggtggttctggcagcggtggttcaggctcaggcagcggcggtagcggtagcggtggaagcggaagcggagaagaacttctcagcaaaaattaccacttggagaatgaagttgcaagactcaaaaaaggttccggcagtggcggcagcggcagcggcggatctggtagtggatctggtggcagtggttcaggcggaagtggtagcggagaggaattgctctcaaagaactatcatttggagaacgaggttgcacgcttgaagaaaggcagcggatcaggcggatctggcagcggtggatctggttctggatccggcggctccggtagtggtggaagtggctctggggaagaattgcttagcaagaattatcatcttgaaaatgaggttgccaggcttaaaaaaggcagtggctccggcggatccggaagcggaggcagcggatctggatctggtggttcaggatctggcggttctggtagcggggaagaactgttgagtaaaaactatcaccttgagaacgaggtcgcaaggttgaaaaaaggatccggctctggcggctccggaagtggcggatctggctccggtagcggaggatcaggatccggcggaagcggatcaggcgaggaactgctttccaaaaattaccaccttgaaaacgaagtcgcccgcctcaagaaaggttctggcagcggaggctctggcagtggtggtagcggaagtggaagtggtggcagtggtagcggtggatctggaagcggcgaggaactcctgtcaaagaattaccatctcgaaaacgaggtcgcaaggctcaagaaaggctcaggatcaggcggctctggatccggcggttctggttccggctcaggtggaagtggatctggcggctcaggttccggcgaagaattgctttccaagaactaccatttggaaaatgaagtcgctcgtttgaagaaaggttcaggctccggcccaaaaaagaagagaaaggtaatggacaagaagtacagcatcggcctggccatcggcaccaactctgtgggctgggccgtgatcaccgacgagtacaaggtgcccagcaagaaattcaaggtgctgggcaacaccgaccggcacagcatcaagaagaacctgatcggcgccctgctgttcgacagcggagaaacagccgaggccacccggctgaagagaaccgccagaagaagatacaccagacggaagaaccggatctgctatctgcaagagatcttcagcaacgagatggccaaggtggacgacagcttcttccacagactggaagagtccttcctggtggaagaggataagaagcacgagcggcaccccatcttcggcaacatcgtggacgaggtggcctaccacgagaagtaccccaccatctaccacctgagaaagaaactggtggacagcaccgacaaggccgacctgcggctgatctatctggccctggcccacatgatcaagttccggggccacttcctgatcgagggcgacctgaaccccgacaacagcgacgtggacaagctgttcatccagctggtgcagacctacaaccagctgttcgaggaaaaccccatcaacgccagcggcgtggacgccaaggccatcctgtctgccagactgagcaagagcagacggctggaaaatctgatcgcccagctgcccggcgagaagaagaatggcctgttcggcaacctgattgccctgagcctgggcctgacccccaacttcaagagcaacttcgacctggccgaggatgccaaactgcagctgagcaaggacacctacgacgacgacctggacaacctgctggcccagatcggcgaccagtacgccgacctgtttctggccgccaagaacctgtccgacgccatcctgctgagcgacatcctgagagtgaacaccgagatcaccaaggcccccctgagcgcctctatgatcaagagatacgacgagcaccaccaggacctgaccctgctgaaagctctcgtgcggcagcagctgcctgagaagtacaaagagattttcttcgaccagagcaagaacggctacgccggctacatcgatggcggagccagccaggaagagttctacaagttcatcaagcccatcctggaaaagatggacggcaccgaggaactgctcgtgaagctgaacagagaggacctgctgcggaagcagcggaccttcgacaacggcagcatcccccaccagatccacctgggagagctgcacgccattctgcggcggcaggaagatttttacccattcctgaaggacaaccgggaaaagatcgagaagatcctgaccttccgcatcccctactacgtgggccctctggccaggggaaacagcagattcgcctggatgaccagaaagagcgaggaaaccatcaccccctggaacttcgaggaagtggtggacaagggcgccagcgcccagagcttcatcgagcggatgaccaacttcgataagaacctgcccaacgagaaggtgctgcccaagcacagcctgctgtacgagtacttcaccgtgtacaacgagctgaccaaagtgaaatacgtgaccgagggaatgagaaagcccgccttcctgagcggcgagcagaaaaaagccatcgtggacctgctgttcaagaccaaccggaaagtgaccgtgaagcagctgaaagaggactacttcaagaaaatcgagtgcttcgactccgtggaaatctccggcgtggaagatcggttcaacgcctccctgggcacataccacgatctgctgaaaattatcaaggacaaggacttcctggacaatgaggaaaacgaggacattctggaagatatcgtgctgaccctgacactgtttgaggacagagagatgatcgaggaacggctgaaaacctatgcccacctgttcgacgacaaagtgatgaagcagctgaagcggcggagatacaccggctggggcaggctgagccggaagctgatcaacggcatccgggacaagcagtccggcaagacaatcctggatttcctgaagtccgacggcttcgccaacagaaacttcatgcagctgatccacgacgacagcctgacctttaaagaggacatccagaaagcccaggtgtccggccagggcgatagcctgcacgagcacattgccaatctggccggcagccccgccattaagaagggcatcctgcagacagtgaaggtggtggacgagctcgtgaaagtgatgggccggcacaagcccgagaacatcgtgatcgaaatggccagagagaaccagaccacccagaagggacagaagaacagccgcgagagaatgaagcggatcgaagagggcatcaaagagctgggcagccagatcctgaaagaacaccccgtggaaaacacccagctgcagaacgagaagctgtacctgtactacctgcagaatgggcgggatatgtacgtggaccaggaactggacatcaaccggctgtccgactacgatgtggacgctatcgtgcctcagagctttctgaaggacgactccatcgataacaaagtgctgactcggagcgacaagaaccggggcaagagcgacaacgtgccctccgaagaggtcgtgaagaagatgaagaactactggcgccagctgctgaatgccaagctgattacccagaggaagttcgacaatctgaccaaggccgagagaggcggcctgagcgaactggataaggccggcttcatcaagagacagctggtggaaacccggcagatcacaaagcacgtggcacagatcctggactcccggatgaacactaagtacgacgagaacgacaaactgatccgggaagtgaaagtgatcaccctgaagtccaagctggtgtccgatttccggaaggatttccagttttacaaagtgcgcgagatcaacaactaccaccacgcccacgacgcctacctgaacgccgtcgtgggaaccgccctgatcaaaaagtaccctaagctggaaagcgagttcgtgtacggcgactacaaggtgtacgacgtgcggaagatgatcgccaagagcgagcaggaaatcggcaaggctaccgccaagtacttcttctacagcaacatcatgaactttttcaagaccgagattaccctggccaacggcgagatccggaagcggcctctgatcgagacaaacggcgaaacaggcgagatcgtgtgggataagggccgggactttgccaccgtgcggaaagtgctgtctatgccccaagtgaatatcgtgaaaaagaccgaggtgcagacaggcggcttcagcaaagagtctatcctgcccaagaggaacagcgacaagctgatcgccagaaagaaggactgggaccctaagaagtacggcggcttcgacagccccaccgtggcctattctgtgctggtggtggccaaagtggaaaagggcaagtccaagaaactgaagagtgtgaaagagctgctggggatcaccatcatggaaagaagcagcttcgagaagaatcccatcgactttctggaagccaagggctacaaagaagtgaaaaaggacctgatcatcaagctgcctaagtactccctgttcgagctggaaaacggccggaagagaatgctggcctctgccggcgaactgcagaagggaaacgaactggccctgccctccaaatatgtgaacttcctgtacctggccagccactatgagaagctgaagggctcccccgaggataatgagcagaaacagctgtttgtggaacagcacaaacactacctggacgagatcatcgagcagatcagcgagttctccaagagagtgatcctggccgacgctaatctggacaaggtgctgagcgcctacaacaagcacagagacaagcctatcagagagcaggccgagaatatcatccacctgtttaccctgaccaatctgggagcccctgccgccttcaagtactttgacaccaccatcgaccggaagaggtacaccagcaccaaagaggtgctggacgccaccctgatccaccagagcatcaccggcctgtacgagacacggatcgacctgtctcagctgggaggcgacgcctatccctatgacgtgcccgattatgccagcctgggcagcggctcccccaagaaaaaacgcaaggtggaagatcctaagaaaaagcggaaagtggacggcagcggcagcgagacccccggtaccagcgagagcgccacccccgagagcatgaacaattcccagggaagagtgaccttcgaggatgtcactgtgaacttcacccagggggagtggcagcggctgaatcccgaacagagaaacttgtacagggatgtgatgctggagaattacagcaaccttgtctctgtgggacaaggggaaaccaccaaacccgatgtgatcttgaggttggaacaaggaaaggagccatggttggaggaagaggaagtgctgggaagtggccgtgcagaaaaaaatggggacattggagggcagatttggaagccaaaggatgtgaaagagagtctcctcgagggaagcggagctactaacttcagcctgctgaagcaggctggagacgtggaggagaaccctggacctatgcctgctgctaagagagtgaaactggatggatccaaccatgaccaggaatttgaccccccaaaggtttacccacctgtgccagctgagaagaggaagcccatccgcgtgctgtctctctttgatgggattgctacagggctcctggtgctgaaggacctgggcatccaagtggaccgctacattgcctccgaggtgtgtgaggactccatcacggtgggcatggtgcggcaccagggaaagatcatgtacgtcggggacgtccgcagcgtcacacagaagcatatccaggagtggggcccattcgacctggtgattggaggcagtccctgcaatgacctctccattgtcaaccctgcccgcaagggactttatgagggtactggccgcctcttctttgagttctaccgcctcctgcatgatgcgcggcccaaggagggagatgatcgccccttcttctggctctttgagaatgtggtggccatgggcgttagtgacaagagggacatctcgcgatttcttgagtctaaccccgtgatgattgacgccaaagaagtgtctgctgcacacagggcccgttacttctggggtaaccttcctggcatgaacaggcctttggcatccactgtgaatgataagctggagctgcaagagtgtctggagcacggcagaatagccaagttcagcaaagtgaggaccattaccaccaggtcaaactctataaagcagggcaaagaccagcatttccccgtgttcatgaacgagaaggaggacatcctgtggtgcactgaaatggaaagggtgtttggcttccccgtccactacacagacgtctccaacatgagccgcttggcgaggcagagactgctgggccgatcgtggagcgtgccggtcatccgccacctcttcgctccgctgaaggaatattttgcttgtgtgtctagcggcaatagtaacgctaacagccgcgggccgagcttcagcagcggcctggtgccgttaagcttgcgcggcagccatatgttcgaaaccgtgcctgtgtggaggagacagccagtccgggtgctgtccctttttgaagacatcaagaaagagctgacgagtttgggctttttggaaagtggttctgacccgggacaactgaagcatgtggttgatgtcacagacacagtgaggaaggatgtggaggagtggggacccttcgatcttgtgtacggcgccacacctcccctgggccacacctgtgaccgtcctcccagctggtacctgttccagttccaccggctcctgcagtacgcacggcccaagccaggcagccccaggcccttcttctggatgttcgtggacaatctggtgctgaacaaggaagacctggacgtcgcatctcgcttcctggagatggagccagtcaccatcccagatgtccacggcggatccttgcagaatgctgtccgcgtgtggagcaacatcccagccataaggagcagcaggcactgggctctggtttcggaagaagaattgtccctgctggcccagaacaagcagagctcgaagctcgcggccaagtggcccaccaagctggtgaagaactgctttctccccctaagagaatatttcaagtatttttcaggagggccgagctctggcgcacccccaccaagtggagggtctcctgccgggtccccaacatctactgaagaaggcaccagcgaatccgcaacgcccgagtcaggccctggtacctccacagaaccatctgaaggtagtgcgcctggttccccagctggaagccctacttccaccgaagaaggcacgtcaaccgaaccaagtgaaggatctgcccctgggaccagcactgaaccatctgagccaaaaaagaagagaaaggtaccatctgagggccccgacatcgtgatgacccagagccccagcagcctgagcgccagcgtgggcgaccgcgtgaccatcacctgccgcagcagcaccggcgccgtgaccaccagcaactacgccagctgggtgcaggagaagcccggcaagctgttcaagggcctgatcggcggcaccaacaaccgcgcccccggcgtgcccagccgcttcagcggcagcctgatcggcgacaaggccaccctgaccatcagcagcctgcagcccgaggacttcgccacctacttctgcgccctgtggtacagcaaccactgggtgttcggccagggcaccaaggtggagctgaagcgcggcggcggcggcagcggcggcggcggcagcggcggcggcggcagcagcggcggcggcagcgaggtgaagctgctggagagcggcggcggcctggtgcagcccggcggcagcctgaagctgagctgcgccgtgagcggcttcagcctgaccgactacggcgtgaactgggtgcgccaggcccccggccgcggcctggagtggatcggcgtgatctggggcgacggcatcaccgactacaacagcgccctgaaggaccgcttcatcatcagcaaggacaacggcaagaacaccgtgtacctgcagatgagcaaggtgcgcagcgacgacaccgccctgtactactgcgtgaccggcctgttcgactactggggccagggcaccctggtgaccgtgagcagctacccatacgatgttccagattacgctggtggaggcggaggttctgggggaggaggtagtggcggtggtggttcaggaggcggcggaagctga

SEQ ID NO: 319 - DNA, 7461 bp, synthetic construct
  misc_feature 1..7461: note = CDS of V31_scFV-hD3L-D3a-2a-3xGCN4-dCas9-KRAB
  source 1..7461: mol_type = other DNA
atgcctgctgctaagagagtgaaactggatggatccggccccgacatcgtgatgacccagagccccagcagcctgagcgccagcgtgggcgaccgcgtgaccatcacctgccgcagcagcaccggcgccgtgaccaccagcaactacgccagctgggtgcaggagaagcccggcaagctgttcaagggcctgatcggcggcaccaacaaccgcgcccccggcgtgcccagccgcttcagcggcagcctgatcggcgacaaggccaccctgaccatcagcagcctgcagcccgaggacttcgccacctacttctgcgccctgtggtacagcaaccactgggtgttcggccagggcaccaaggtggagctgaagcgcggcggcggcggcagcggcggcggcggcagcggcggcggcggcagcagcggcggcggcagcgaggtgaagctgctggagagcggcggcggcctggtgcagcccggcggcagcctgaagctgagctgcgccgtgagcggcttcagcctgaccgactacggcgtgaactgggtgcgccaggcccccggccgcggcctggagtggatcggcgtgatctggggcgacggcatcaccgactacaacagcgccctgaaggaccgcttcatcatcagcaaggacaacggcaagaacaccgtgtacctgcagatgagcaaggtgcgcagcgacgacaccgccctgtactactgcgtgaccggcctgttcgactactggggccagggcaccctggtgaccgtgagcagctacccatacgatgttccagattacgctggtggaggcggaggttctgggggaggaggtagtggcggtggtggttcaggaggcggcggaagcatgttcgaaaccgtgcctgtgtggaggagacagccagtccgggtgctgtccctttttgaagacatcaagaaagagctgacgagtttgggctttttggaaagtggttctgacccgggacaactgaagcatgtggttgatgtcacagacacagtgaggaaggatgtggaggagtggggacccttcgatcttgtgtacggcgccacacctcccctgggccacacctgtgaccgtcctcccagctggtacctgttccagttccaccggctcctgcagtacgcacggcccaagccaggcagccccaggcccttcttctggatgttcgtggacaatctggtgctgaacaaggaagacctggacgtcgcatctcgcttcctggagatggagccagtcaccatcccagatgtccacggcggatccttgcagaatgctgtccgcgtgtggagcaacatcccagccataaggagcagcaggcactgggctctggtttcggaagaagaattgtccctgctggcccagaacaagcagagctcgaagctcgcggccaagtggcccaccaagctggtgaagaactgctttctccccctaagagaatatttcaagtatttttcaacagaactcacttcctctttatctagcggcaatagtaacgctaacagccgcgggccgagcttcagcagcggcctggtgccgttaagcttgcgcggcagccatatgaaccatgaccaggaatttgaccccccaaaggtttacccacctgtgccagctgagaagaggaagcccatccgcgtgctgtctctctttgatgggattgctacagggctcctggtgctgaaggacctgggcatccaagtggaccgctacattgcctccgaggtgtgtgaggactccatcacggtgggcatggtgcggcaccagggaaagatcatgtacgtcggggacgtccgcagcgtcacacagaagcatatccaggagtggggcccattcgacctggtgattggaggcagtccctgcaatgacctctccattgtcaaccctgcccgcaagggactttatgagggtactggccgcctcttctttgagttctaccgcctcctgcatgatgcgcggcccaaggagggagatgatcgccccttcttctggctctttgagaatgtggtggccatgggcgttagtgacaagagggacatctcgcgatttcttgagtctaaccccgtgatgattgacgccaaagaagtgtctgctgcacacagggcccgttacttctggggtaaccttcctggcatgaacaggcctttggcatccactgtgaatgataagctggagctgcaagagtgtctggagcacggcagaatagccaagttcagcaaagtgaggaccattaccaccaggtcaaactctataaagcagggcaaagaccagcatttccccgtcttcatgaacgagaaggaggacatcctgtggtgcactgaaatggaaagggtgtttggcttccccgtccactacacagacgtctccaacatgagccgcttggcgaggcagagactgctgggccgatcgtggagcgtgccggtcatccgccacctcttcgctccgctgaaggaatattttgcttgtgtgggaagcggagctactaacttcagcctgctgaagcaggctggagacgtggaggagaaccctggacctatgcctgctgctaagagagtgaaactggatggatccgaggaactgctgagcaagaactaccacctggaaaacgaggtggccagactgaagaaaggctctggctctggcggaagcggttctggcggatcaggatctggaagtggcggctctggaagcggaggttctggatctggcgaagaactgctgtctaagaattatcacctcgagaacgaagtggctcggctcaagaaaggcagtggcagcggaggaagtggatccggcggtagtggtagtggaagcggcggatccggctcaggcggatctggttcaggggaagaactcctctccaaaaactaccatctcgagaatgaggtcgcccgcctgaaaaaaggatcaggttccggtggttctggcagcggtggttcaggctcaggcagcggcggtagcggtagcggtggaagcggaagcggaccaaaaaagaagagaaaggtaatggacaagaagtacagcatcggcctggccatcggcaccaactctgtgggctgggccgtgatcaccgacgagtacaaggtgcccagcaagaaattcaaggtgctgggcaacaccgaccggcacagcatcaagaagaacctgatcggcgccctgctgttcgacagcggagaaacagccgaggccacccggctgaagagaaccgccagaagaagatacaccagacggaagaaccggatctgctatctgcaagagatcttcagcaacgagatggccaaggtggacgacagcttcttccacagactggaagagtccttcctggtggaagaggataagaagcacgagcggcaccccatcttcggcaacatcgtggacgaggtggcctaccacgagaagtaccccaccatctaccacctgagaaagaaactggtggacagcaccgacaaggccgacctgcggctgatctatctggccctggcccacatgatcaagttccggggccacttcctgatcgagggcgacctgaaccccgacaacagcgacgtggacaagctgttcatccagctggtgcagacctacaaccagctgttcgaggaaaaccccatcaacgccagcggcgtggacgccaaggccatcctgtctgccagactgagcaagagcagacggctggaaaatctgatcgcccagctgcccggcgagaagaagaatggcctgttcggcaacctgattgccctgagcctgggcctgacccccaacttcaagagcaacttcgacctggccgaggatgccaaactgcagctgagcaaggacacctacgacgacgacctggacaacctgctggcccagatcggcgaccagtacgccgacctgtttctggccgccaagaacctgtccgacgccatcctgctgagcgacatcctgagagtgaacaccgagatcaccaaggcccccctgagcgcctctatgatcaagagatacgacgagcaccaccaggacctgaccctgctgaaagctctcgtgcggcagcagctgcctgagaagtacaaagagattttcttcgaccagagcaagaacggctacgccggctacatcgatggcggagccagccaggaagagttctacaagttcatcaagcccatcctggaaaagatggacggcaccgaggaactgctcgtgaagctgaacagagaggacctgctgcggaagcagcggaccttcgacaacggcagcatcccccaccagatccacctgggagagctgcacgccattctgcggcggcaggaagatttttacccattcctgaaggacaaccgggaaaagatcgagaagatcctgaccttccgcatcccctactacgtgggccctctggccaggggaaacagcagattcgcctggatgaccagaaagagcgaggaaaccatcaccccctggaacttcgaggaagtggtggacaagggcgccagcgcccagagcttcatcgagcggatgaccaacttcgataagaacctgcccaacgagaaggtgctgcccaagcacagcctgctgtacgagtacttcaccgtgtacaacgagctgaccaaagtgaaatacgtgaccgagggaatgagaaagcccgccttcctgagcggcgagcagaaaaaagccatcgtggacctgctgttcaagaccaaccggaaagtgaccgtgaagcagctgaaagaggactacttcaagaaaatcgagtgcttcgactccgtggaaatctccggcgtggaagatcggttcaacgcctccctgggcacataccacgatctgctgaaaattatcaaggacaaggacttcctggacaatgaggaaaacgaggacattctggaagatatcgtgctgaccctgacactgtttgaggacagagagatgatcgaggaacggctgaaaacctatgcccacctgttcgacgacaaagtgatgaagcagctgaagcggcggagatacaccggctggggcaggctgagccggaagctgatcaacggcatccgggacaagcagtccggcaagacaatcctggatttcctgaagtccgacggcttcgccaacagaaacttcatgcagctgatccacgacgacagcctgacctttaaagaggacatccagaaagcccaggtgtccggccagggcgatagcctgcacgagcacattgccaatctggccggcagccccgccattaagaagggcatcctgcagacagtgaaggtggtggacgagctcgtgaaagtgatgggccggcacaagcccgagaacatcgtgatcgaaatggccagagagaaccagaccacccagaagggacagaagaacagccgcgagagaatgaagcggatcgaagagggcatcaaagagctgggcagccagatcctgaaagaacaccccgtggaaaacacccagctgcagaacgagaagctgtacctgtactacctgcagaatgggcgggatatgtacgtggaccaggaactggacatcaaccggctgtccgactacgatgtggacgctatcgtgcctcagagctttctgaaggacgactccatcgataacaaagtgctgactcggagcgacaagaaccggggcaagagcgacaacgtgccctccgaagaggtcgtgaagaagatgaagaactactggcgccagctgctgaatgccaagctgattacccagaggaagttcgacaatctgaccaaggccgagagaggcggcctgagcgaactggataaggccggcttcatcaagagacagctggtggaaacccggcagatcacaaagcacgtggcacagatcctggactcccggatgaacactaagtacgacgagaacgacaaactgatccgggaagtgaaagtgatcaccctgaagtccaagctggtgtccgatttccggaaggatttccagttttacaaagtgcgcgagatcaacaactaccaccacgcccacgacgcctacctgaacgccgtcgtgggaaccgccctgatcaaaaagtaccctaagctggaaagcgagttcgtgtacggcgactacaaggtgtacgacgtgcggaagatgatcgccaagagcgagcaggaaatcggcaaggctaccgccaagtacttcttctacagcaacatcatgaactttttcaagaccgagattaccctggccaacggcgagatccggaagcggcctctgatcgagacaaacggcgaaacaggcgagatcgtgtgggataagggccgggactttgccaccgtgcggaaagtgctgtctatgccccaagtgaatatcgtgaaaaagaccgaggtgcagacaggcggcttcagcaaagagtctatcctgcccaagaggaacagcgacaagctgatcgccagaaagaaggactgggaccctaagaagtacggcggcttcgacagccccaccgtggcctattctgtgctggtggtggccaaagtggaaaagggcaagtccaagaaactgaagagtgtgaaagagctgctggggatcaccatcatggaaagaagcagcttcgagaagaatcccatcgactttctggaagccaagggctacaaagaagtgaaaaaggacctgatcatcaagctgcctaagtactccctgttcgagctggaaaacggccggaagagaatgctggcctctgccggcgaactgcagaagggaaacgaactggccctgccctccaaatatgtgaacttcctgtacctggccagccactatgagaagctgaagggctcccccgaggataatgagcagaaacagctgtttgtggaacagcacaaacactacctggacgagatcatcgagcagatcagcgagttctccaagagagtgatcctggccgacgctaatctggacaaggtgctgagcgcctacaacaagcacagagacaagcctatcagagagcaggccgagaatatcatccacctgtttaccctgaccaatctgggagcccctgccgccttcaagtactttgacaccaccatcgaccggaagaggtacaccagcaccaaagaggtgctggacgccaccctgatccaccagagcatcaccggcctgtacgagacacggatcgacctgtctcagctgggaggcgacgcctatccctatgacgtgcccgattatgccagcctgggcagcggctcccccaagaaaaaacgcaaggtggaagatcctaagaaaaagcggaaagtggacggcagcggcagcgagacccccggtaccagcgagagcgccacccccgagagccggacactggtgaccttcaaggatgtatttgtggacttcaccagggaggagtggaagctgctggacactgctcagcagatcgtgtacagaaatgtgatgctggagaactataagaacctggtttccttgggttatcagcttactaagccagatgtgatcctccggttggagaagggagaagagccctga

SEQ ID NO: 320 - DNA, 7482 bp, synthetic construct
  misc_feature 1..7482: note = CDS of V32_1xGCN4-ZIM3-2a-D3a-hD3L-dCas9-scFv
  source 1..7482: mol_type = other DNA
atgcctgctgctaagagagtgaaactggatggatccgaggaactgctgagcaagaactaccacctggaaaacgaggtggccagactgaagaaaggctctggctctggcggaagcggttctggcggatcaggatctggaagtggcggctctggaagcggaggttctggatctggcatgaacaattcccagggaagagtgaccttcgaggacgtgaccgtgaacttcacccaaggcgagtggcagagactgaaccccgagcagagaaacctgtaccgggacgtgatgctggaaaactacagcaacctggtgtccgtcggccagggcgagacaacaaagcctgacgtgatcctgcggctggaacagggcaaagagccttggctggaagaggaagaggtgctcggatctggcagagccgagaagaatggcgatatcggcggacagatctggaagccaaaggatgtgaaagagagtctcggaagcggagctactaacttcagcctgctgaagcaggctggagacgtggaggagaaccctggacctatgcctgctgctaagagagtgaaactggatggatccaaccatgaccaggaatttgaccccccaaaggtttacccacctgtgccagctgagaagaggaagcccatccgcgtgctgtctctctttgatgggattgctacagggctcctggtgctgaaggacctgggcatccaagtggaccgctacattgcctccgaggtgtgtgaggactccatcacggtgggcatggtgcggcaccagggaaagatcatgtacgtcggggacgtccgcagcgtcacacagaagcatatccaggagtggggcccattcgacctggtgattggaggcagtccctgcaatgacctctccattgtcaaccctgcccgcaagggactttatgagggtactggccgcctcttctttgagttctaccgcctcctgcatgatgcgcggcccaaggagggagatgatcgccccttcttctggctctttgagaatgtggtggccatgggcgttagtgacaagagggacatctcgcgatttcttgagtctaaccccgtgatgattgacgccaaagaagtgtctgctgcacacagggcccgttacttctggggtaaccttcctggcatgaacaggcctttggcatccactgtgaatgataagctggagctgcaagagtgtctggagcacggcagaatagccaagttcagcaaagtgaggaccattaccaccaggtcaaactctataaagcagggcaaagaccagcatttccccgtgttcatgaacgagaaggaggacatcctgtggtgcactgaaatggaaagggtgtttggcttccccgtccactacacagacgtctccaacatgagccgcttggcgaggcagagactgctgggccgatcgtggagcgtgccggtcatccgccacctcttcgctccgctgaaggaatattttgcttgtgtgtctagcggcaatagtaacgctaacagccgcgggccgagcttcagcagcggcctggtgccgttaagcttgcgcggcagccatatgttcgaaaccgtgcctgtgtggaggagacagccagtccgggtgctgtccctttttgaagacatcaagaaagagctgacgagtttgggctttttggaaagtggttctgacccgggacaactgaagcatgtggttgatgtcacagacacagtgaggaaggatgtggaggagtggggacccttcgatcttgtgtacggcgccacacctcccctgggccacacctgtgaccgtcctcccagctggtacctgttccagttccaccggctcctgcagtacgcacggcccaagccaggcagccccaggcccttcttctggatgttcgtggacaatctggtgctgaacaaggaagacctggacgtcgcatctcgcttcctggagatggagccagtcaccatcccagatgtccacggcggatccttgcagaatgctgtccgcgtgtggagcaacatcccagccataaggagcagcaggcactgggctctggtttcggaagaagaattgtccctgctggcccagaacaagcagagctcgaagctcgcggccaagtggcccaccaagctggtgaagaactgctttctccccctaagagaatatttcaagtatttttcaggagggccgagctctggcgcacccccaccaagtggagggtctcctgccgggtccccaacatctactgaagaaggcaccagcgaatccgcaacgcccgagtcaggccctggtacctccacagaaccatctgaaggtagtgcgcctggttccccagctggaagccctacttccaccgaagaaggcacgtcaaccgaaccaagtgaaggatctgcccctgggaccagcactgaaccatctgagccaaaaaagaagagaaaggtaatggacaagaagtacagcatcggcctggccatcggcaccaactctgtgggctgggccgtgatcaccgacgagtacaaggtgcccagcaagaaattcaaggtgctgggcaacaccgaccggcacagcatcaagaagaacctgatcggcgccctgctgttcgacagcggagaaacagccgaggccacccggctgaagagaaccgccagaagaagatacaccagacggaagaaccggatctgctatctgcaagagatcttcagcaacgagatggccaaggtggacgacagcttcttccacagactggaagagtccttcctggtggaagaggataagaagcacgagcggcaccccatcttcggcaacatcgtggacgaggtggcctaccacgagaagtaccccaccatctaccacctgagaaagaaactggtggacagcaccgacaaggccgacctgcggctgatctatctggccctggcccacatgatcaagttccggggccacttcctgatcgagggcgacctgaaccccgacaacagcgacgtggacaagctgttcatccagctggtgcagacctacaaccagctgttcgaggaaaaccccatcaacgccagcggcgtggacgccaaggccatcctgtctgccagactgagcaagagcagacggctggaaaatctgatcgcccagctgcccggcgagaagaagaatggcctgttcggcaacctgattgccctgagcctgggcctgacccccaacttcaagagcaacttcgacctggccgaggatgccaaactgcagctgagcaaggacacctacgacgacgacctggacaacctgctggcccagatcggcgaccagtacgccgacctgtttctggccgccaagaacctgtccgacgccatcctgctgagcgacatcctgagagtgaacaccgagatcaccaaggcccccctgagcgcctctatgatcaagagatacgacgagcaccaccaggacctgaccctgctgaaagctctcgtgcggcagcagctgcctgagaagtacaaagagattttcttcgaccagagcaagaacggctacgccggctacatcgatggcggagccagccaggaagagttctacaagttcatcaagcccatcctggaaaagatggacggcaccgaggaactgctcgtgaagctgaacagagaggacctgctgcggaagcagcggaccttcgacaacggcagcatcccccaccagatccacctgggagagctgcacgccattctgcggcggcaggaagatttttacccattcctgaaggacaaccgggaaaagatcgagaagatcctgaccttccgcatcccctactacgtgggccctctggccaggggaaacagcagattcgcctggatgaccagaaagagcgaggaaaccatcaccccctggaacttcgaggaagtggtggacaagggcgccagcgcccagagcttcatcgagcggatgaccaacttcgataagaacctgcccaacgagaaggtgctgcccaagcacagcctgctgtacgagtacttcaccgtgtacaacgagctgaccaaagtgaaatacgtgaccgagggaatgagaaagcccgccttcctgagcggcgagcagaaaaaagccatcgtggacctgctgttcaagaccaaccggaaagtgaccgtgaagcagctgaaagaggactacttcaagaaaatcgagtgcttcgactccgtggaaatctccggcgtggaagatcggttcaacgcctccctgggcacataccacgatctgctgaaaattatcaaggacaaggacttcctggacaatgaggaaaacgaggacattctggaagatatcgtgctgaccctgacactgtttgaggacagagagatgatcgaggaacggctgaaaacctatgcccacctgttcgacgacaaagtgatgaagcagctgaagcggcggagatacaccggctggggcaggctgagccggaagctgatcaacggcatccgggacaagcagtccggcaagacaatcctggatttcctgaagtccgacggcttcgccaacagaaacttcatgcagctgatccacgacgacagcctgacctttaaagaggacatccagaaagcccaggtgtccggccagggcgatagcctgcacgagcacattgccaatctggccggcagccccgccattaagaagggcatcctgcagacagtgaaggtggtggacgagctcgtgaaagtgatgggccggcacaagcccgagaacatcgtgatcgaaatggccagagagaaccagaccacccagaagggacagaagaacagccgcgagagaatgaagcggatcgaagagggcatcaaagagctgggcagccagatcctgaaagaacaccccgtggaaaacacccagctgcagaacgagaagctgtacctgtactacctgcagaatgggcgggatatgtacgtggaccaggaactggacatcaaccggctgtccgactacgatgtggacgctatcgtgcctcagagctttctgaaggacgactccatcgataacaaagtgctgactcggagcgacaagaaccggggcaagagcgacaacgtgccctccgaagaggtcgtgaagaagatgaagaactactggcgccagctgctgaatgccaagctgattacccagaggaagttcgacaatctgaccaaggccgagagaggcggcctgagcgaactggataaggccggcttcatcaagagacagctggtggaaacccggcagatcacaaagcacgtggcacagatcctggactcccggatgaacactaagtacgacgagaacgacaaactgatccgggaagtgaaagtgatcaccctgaagtccaagctggtgtccgatttccggaaggatttccagttttacaaagtgcgcgagatcaacaactaccaccacgcccacgacgcctacctgaacgccgtcgtgggaaccgccctgatcaaaaagtaccctaagctggaaagcgagttcgtgtacggcgactacaaggtgtacgacgtgcggaagatgatcgccaagagcgagcaggaaatcggcaaggctaccgccaagtacttcttctacagcaacatcatgaactttttcaagaccgagattaccctggccaacggcgagatccggaagcggcctctgatcgagacaaacggcgaaacaggcgagatcgtgtgggataagggccgggactttgccaccgtgcggaaagtgctgtctatgccccaagtgaatatcgtgaaaaagaccgaggtgcagacaggcggcttcagcaaagagtctatcctgcccaagaggaacagcgacaagctgatcgccagaaagaaggactgggaccctaagaagtacggcggcttcgacagccccaccgtggcctattctgtgctggtggtggccaaagtggaaaagggcaagtccaagaaactgaagagtgtgaaagagctgctggggatcaccatcatggaaagaagcagcttcgagaagaatcccatcgactttctggaagccaagggctacaaagaagtgaaaaaggacctgatcatcaagctgcctaagtactccctgttcgagctggaaaacggccggaagagaatgctggcctctgccggcgaactgcagaagggaaacgaactggccctgccctccaaatatgtgaacttcctgtacctggccagccactatgagaagctgaagggctcccccgaggataatgagcagaaacagctgtttgtggaacagcacaaacactacctggacgagatcatcgagcagatcagcgagttctccaagagagtgatcctggccgacgctaatctggacaaggtgctgagcgcctacaacaagcacagagacaagcctatcagagagcaggccgagaatatcatccacctgtttaccctgaccaatctgggagcccctgccgccttcaagtactttgacaccaccatcgaccggaagaggtacaccagcaccaaagaggtgctggacgccaccctgatccaccagagcatcaccggcctgtacgagacacggatcgacctgtctcagctgggaggcgacgcctatccctatgacgtgcccgattatgccagcctgggcagcggctcccccaagaaaaaacgcaaggtggaagatcctaagaaaaagcggaaagtggacggcattggtagtgggagcggccccgacatcgtgatgacccagagccccagcagcctgagcgccagcgtgggcgaccgcgtgaccatcacctgccgcagcagcaccggcgccgtgaccaccagcaactacgccagctgggtgcaggagaagcccggcaagctgttcaagggcctgatcggcggcaccaacaaccgcgcccccggcgtgcccagccgcttcagcggcagcctgatcggcgacaaggccaccctgaccatcagcagcctgcagcccgaggacttcgccacctacttctgcgccctgtggtacagcaaccactgggtgttcggccagggcaccaaggtggagctgaagcgcggcggcggcggcagcggcggcggcggcagcggcggcggcggcagcagcggcggcggcagcgaggtgaagctgctggagagcggcggcggcctggtgcagcccggcggcagcctgaagctgagctgcgccgtgagcggcttcagcctgaccgactacggcgtgaactgggtgcgccaggcccccggccgcggcctggagtggatcggcgtgatctggggcgacggcatcaccgactacaacagcgccctgaaggaccgcttcatcatcagcaaggacaacggcaagaacaccgtgtacctgcagatgagcaaggtgcgcagcgacgacaccgccctgtactactgcgtgaccggcctgttcgactactggggccagggcaccctggtgaccgtgagcagctacccatacgatgttccagattacgctggtggaggcggaggttctgggggaggaggtagtggcggtggtggttcaggaggcggcggaagctag

SEQ ID NO: 321 - DNA, 7380 bp, synthetic construct
  misc_feature 1..7380: note = CDS of V33_KRAB-1xGCN4-2a-D3a-hD3l-dCas9-scFv
  source 1..7380: mol_type = other DNA
atgcctgctgctaagagagtgaaactggatggatcccggacactggtgaccttcaaggatgtatttgtggacttcaccagggaggagtggaagctgctggacactgctcagcagatcgtgtacagaaatgtgatgctggagaactataagaacctggtttccttgggttatcagcttactaagccagatgtgatcctccggttggagaagggagaagagcccggaagcggaatggaggaactgctgagcaagaactaccacctggaaaacgaggtggccagactgaagaaaggctctggctctggcggaagcggttctggcggatcaggatctggaagtggcggctctggaagcggaggttctggatctggcggaagcggagctactaacttcagcctgctgaagcaggctggagacgtggaggagaaccctggacctatgcctgctgctaagagagtgaaactggatggatccaaccatgaccaggaatttgaccccccaaaggtttacccacctgtgccagctgagaagaggaagcccatccgcgtgctgtctctctttgatgggattgctacagggctcctggtgctgaaggacctgggcatccaagtggaccgctacattgcctccgaggtgtgtgaggactccatcacggtgggcatggtgcggcaccagggaaagatcatgtacgtcggggacgtccgcagcgtcacacagaagcatatccaggagtggggcccattcgacctggtgattggaggcagtccctgcaatgacctctccattgtcaaccctgcccgcaagggactttatgagggtactggccgcctcttctttgagttctaccgcctcctgcatgatgcgcggcccaaggagggagatgatcgccccttcttctggctctttgagaatgtggtggccatgggcgttagtgacaagagggacatctcgcgatttcttgagtctaaccccgtgatgattgacgccaaagaagtgtctgctgcacacagggcccgttacttctggggtaaccttcctggcatgaacaggcctttggcatccactgtgaatgataagctggagctgcaagagtgtctggagcacggcagaatagccaagttcagcaaagtgaggaccattaccaccaggtcaaactctataaagcagggcaaagaccagcatttccccgtgttcatgaacgagaaggaggacatcctgtggtgcactgaaatggaaagggtgtttggcttccccgtccactacacagacgtctccaacatgagccgcttggcgaggcagagactgctgggccgatcgtggagcgtgccggtcatccgccacctcttcgctccgctgaaggaatattttgcttgtgtgtctagcggcaatagtaacgctaacagccgcgggccgagcttcagcagcggcctggtgccgttaagcttgcgcggcagccatatgttcgaaaccgtgcctgtgtggaggagacagccagtccgggtgctgtccctttttgaagacatcaagaaagagctgacgagtttgggctttttggaaagtggttctgacccgggacaactgaagcatgtggttgatgtcacagacacagtgaggaaggatgtggaggagtggggacccttcgatcttgtgtacggcgccacacctcccctgggccacacctgtgaccgtcctcccagctggtacctgttccagttccaccggctcctgcagtacgcacggcccaagccaggcagccccaggcccttcttctggatgttcgtggacaatctggtgctgaacaaggaagacctggacgtcgcatctcgcttcctggagatggagccagtcaccatcccagatgtccacggcggatccttgcagaatgctgtccgcgtgtggagcaacatcccagccataaggagcagcaggcactgggctctggtttcggaagaagaattgtccctgctggcccagaacaagcagagctcgaagctcgcggccaagtggcccaccaagctggtgaagaactgctttctccccctaagagaatatttcaagtatttttcaggagggccgagctctggcgcacccccaccaagtggagggtctcctgccgggtccccaacatctactgaagaaggcaccagcgaatccgcaacgcccgagtcaggccctggtacctccacagaaccatctgaaggtagtgcgcctggttccccagctggaagccctacttccaccgaagaaggcacgtcaaccgaaccaagtgaaggatctgcccctgggaccagcactgaaccatctgagccaaaaaagaagagaaaggtaatggacaagaagtacagcatcggcctggccatcggcaccaactctgtgggctgggccgtgatcaccgacgagtacaaggtgcccagcaagaaattcaaggtgctgggcaacaccgaccggcacagcatcaagaagaacctgatcggcgccctgctgttcgacagcggagaaacagccgaggccacccggctgaagagaaccgccagaagaagatacaccagacggaagaaccggatctgctatctgcaagagatcttcagcaacgagatggccaaggtggacgacagcttcttccacagactggaagagtccttcctggtggaagaggataagaagcacgagcggcaccccatcttcggcaacatcgtggacgaggtggcctaccacgagaagtaccccaccatctaccacctgagaaagaaactggtggacagcaccgacaaggccgacctgcggctgatctatctggccctggcccacatgatcaagttccggggccacttcctgatcgagggcgacctgaaccccgacaacagcgacgtggacaagctgttcatccagctggtgcagacctacaaccagctgttcgaggaaaaccccatcaacgccagcggcgtggacgccaaggccatcctgtctgccagactgagcaagagcagacggctggaaaatctgatcgcccagctgcccggcgagaagaagaatggcctgttcggcaacctgattgccctgagcctgggcctgacccccaacttcaagagcaacttcgacctggccgaggatgccaaactgcagctgagcaaggacacctacgacgacgacctggacaacctgctggcccagatcggcgaccagtacgccgacctgtttctggccgccaagaacctgtccgacgccatcctgctgagcgacatcctgagagtgaacaccgagatcaccaaggcccccctgagcgcctctatgatcaagagatacgacgagcaccaccaggacctgaccctgctgaaagctctcgtgcggcagcagctgcctgagaagtacaaagagattttcttcgaccagagcaagaacggctacgccggctacatcgatggcggagccagccaggaagagttctacaagttcatcaagcccatcctggaaaagatggacggcaccgaggaactgctcgtgaagctgaacagagaggacctgctgcggaagcagcggaccttcgacaacggcagcatcccccaccagatccacctgggagagctgcacgccattctgcggcggcaggaagatttttacccattcctgaaggacaaccgggaaaagatcgagaagatcctgaccttccgcatcccctactacgtgggccctctggccaggggaaacagcagattcgcctggatgaccagaaagagcgaggaaaccatcaccccctggaacttcgaggaagtggtggacaagggcgccagcgcccagagcttcatcgagcggatgaccaacttcgataagaacctgcccaacgagaaggtgctgcccaagcacagcctgctgtacgagtacttcaccgtgtacaacgagctgaccaaagtgaaatacgtgaccgagggaatgagaaagcccgccttcctgagcggcgagcagaaaaaagccatcgtggacctgctgttcaagaccaaccggaaagtgaccgtgaagcagctgaaagaggactacttcaagaaaatcgagtgcttcgactccgtggaaatctccggcgtggaagatcggttcaacgcctccctgggcacataccacgatctgctgaaaattatcaaggacaaggacttcctggacaatgaggaaaacgaggacattctggaagatatcgtgctgaccctgacactgtttgaggacagagagatgatcgaggaacggctgaaaacctatgcccacctgttcgacgacaaagtgatgaagcagctgaagcggcggagatacaccggctggggcaggctgagccggaagctgatcaacggcatccgggacaagcagtccggcaagacaatcctggatttcctgaagtccgacggcttcgccaacagaaacttcatgcagctgatccacgacgacagcctgacctttaaagaggacatccagaaagcccaggtgtccggccagggcgatagcctgcacgagcacattgccaatctggccggcagccccgccattaagaagggcatcctgcagacagtgaaggtggtggacgagctcgtgaaagtgatgggccggcacaagcccgagaacatcgtgatcgaaatggccagagagaaccagaccacccagaagggacagaagaacagccgcgagagaatgaagcggatcgaagagggcatcaaagagctgggcagccagatcctgaaagaacaccccgtggaaaacacccagctgcagaacgagaagctgtacctgtactacctgcagaatgggcgggatatgtacgtggaccaggaactggacatcaaccggctgtccgactacgatgtggacgctatcgtgcctcagagctttctgaaggacgactccatcgataacaaagtgctgactcggagcgacaagaaccggggcaagagcgacaacgtgccctccgaagaggtcgtgaagaagatgaagaactactggcgccagctgctgaatgccaagctgattacccagaggaagttcgacaatctgaccaaggccgagagaggcggcctgagcgaactggataaggccggcttcatcaagagacagctggtggaaacccggcagatcacaaagcacgtggcacagatcctggactcccggatgaacactaagtacgacgagaacgacaaactgatccgggaagtgaaagtgatcaccctgaagtccaagctggtgtccgatttccggaaggatttccagttttacaaagtgcgcgagatcaacaactaccaccacgcccacgacgcctacctgaacgccgtcgtgggaaccgccctgatcaaaaagtaccctaagctggaaagcgagttcgtgtacggcgactacaaggtgtacgacgtgcggaagatgatcgccaagagcgagcaggaaatcggcaaggctaccgccaagtacttcttctacagcaacatcatgaactttttcaagaccgagattaccctggccaacggcgagatccggaagcggcctctgatcgagacaaacggcgaaacaggcgagatcgtgtgggataagggccgggactttgccaccgtgcggaaagtgctgtctatgccccaagtgaatatcgtgaaaaagaccgaggtgcagacaggcggcttcagcaaagagtctatcctgcccaagaggaacagcgacaagctgatcgccagaaagaaggactgggaccctaagaagtacggcggcttcgacagccccaccgtggcctattctgtgctggtggtggccaaagtggaaaagggcaagtccaagaaactgaagagtgtgaaagagctgctggggatcaccatcatggaaagaagcagcttcgagaagaatcccatcgactttctggaagccaagggctacaaagaagtgaaaaaggacctgatcatcaagctgcctaagtactccctgttcgagctggaaaacggccggaagagaatgctggcctctgccggcgaactgcagaagggaaacgaactggccctgccctccaaatatgtgaacttcctgtacctggccagccactatgagaagctgaagggctcccccgaggataatgagcagaaacagctgtttgtggaacagcacaaacactacctggacgagatcatcgagcagatcagcgagttctccaagagagtgatcctggccgacgctaatctggacaaggtgctgagcgcctacaacaagcacagagacaagcctatcagagagcaggccgagaatatcatccacctgtttaccctgaccaatctgggagcccctgccgccttcaagtactttgacaccaccatcgaccggaagaggtacaccagcaccaaagaggtgctggacgccaccctgatccaccagagcatcaccggcctgtacgagacacggatcgacctgtctcagctgggaggcgacgcctatccctatgacgtgcccgattatgccagcctgggcagcggctcccccaagaaaaaacgcaaggtggaagatcctaagaaaaagcggaaagtggacggcattggtagtgggagcggccccgacatcgtgatgacccagagccccagcagcctgagcgccagcgtgggcgaccgcgtgaccatcacctgccgcagcagcaccggcgccgtgaccaccagcaactacgccagctgggtgcaggagaagcccggcaagctgttcaagggcctgatcggcggcaccaacaaccgcgcccccggcgtgcccagccgcttcagcggcagcctgatcggcgacaaggccaccctgaccatcagcagcctgcagcccgaggacttcgccacctacttctgcgccctgtggtacagcaaccactgggtgttcggccagggcaccaaggtggagctgaagcgcggcggcggcggcagcggcggcggcggcagcggcggcggcggcagcagcggcggcggcagcgaggtgaagctgctggagagcggcggcggcctggtgcagcccggcggcagcctgaagctgagctgcgccgtgagcggcttcagcctgaccgactacggcgtgaactgggtgcgccaggcccccggccgcggcctggagtggatcggcgtgatctggggcgacggcatcaccgactacaacagcgccctgaaggaccgcttcatcatcagcaaggacaacggcaagaacaccgtgtacctgcagatgagcaaggtgcgcagcgacgacaccgccctgtactactgcgtgaccggcctgttcgactactggggccagggcaccctggtgaccgtgagcagctacccatacgatgttccagattacgctggtggaggcggaggttctgggggaggaggtagtggcggtggtggttcaggaggcggcggaagctag

SEQ ID NO: 322 - DNA, 7401 bp, synthetic construct
  misc_feature 1..7401: note = CDS of V34_D3a-D3l-1xGCN4-2a-scFv-dCas9-KRAB
  source 1..7401: mol_type = other DNA
atgcctgctgctaagagagtgaaactggatggatccaaccatgaccaggaatttgaccccccaaaggtttacccacctgtgccagctgagaagaggaagcccatccgcgtgctgtctctctttgatgggattgctacagggctcctggtgctgaaggacctgggcatccaagtggaccgctacattgcctccgaggtgtgtgaggactccatcacggtgggcatggtgcggcaccagggaaagatcatgtacgtcggggacgtccgcagcgtcacacagaagcatatccaggagtggggcccattcgacctggtgattggaggcagtccctgcaatgacctctccattgtcaaccctgcccgcaagggactttatgagggtactggccgcctcttctttgagttctaccgcctcctgcatgatgcgcggcccaaggagggagatgatcgccccttcttctggctctttgagaatgtggtggccatgggcgttagtgacaagagggacatctcgcgatttcttgagtctaaccccgtgatgattgacgccaaagaagtgtctgctgcacacagggcccgttacttctggggtaaccttcctggcatgaacaggcctttggcatccactgtgaatgataagctggagctgcaagagtgtctggagcacggcagaatagccaagttcagcaaagtgaggaccattaccaccaggtcaaactctataaagcagggcaaagaccagcatttccccgtgttcatgaacgagaaggaggacatcctgtggtgcactgaaatggaaagggtgtttggcttccccgtccactacacagacgtctccaacatgagccgcttggcgaggcagagactgctgggccgatcgtggagcgtgccggtcatccgccacctcttcgctccgctgaaggaatattttgcttgtgtgtctagcggcaatagtaacgctaacagccgcgggccgagcttcagcagcggcctggtgccgttaagcttgcgcggcagccatatgggccctatggagatatacaagacagtgtctgcatggaagagacagccagtgcgggtactgagcctcttcagaaacatcgacaaggtactaaagagtttgggcttcttggaaagcggttctggttctgggggaggaacgctgaagtacgtggaagatgtcacaaatgtcgtgaggagagacgtggagaaatggggcccctttgacctggtgtacggctcgacgcagcccctaggcagctcttgtgatcgctgtcccggctggtacatgttccagttccaccggatcctgcagtatgcgctgcctcgccaggagagtcagcggcccttcttctggatattcatggacaatctgctgctgactgaggatgaccaagagacaactacccgcttccttcagacagaggctgtgaccctccaggatgtccgtggcagagactaccagaatgctatgcgggtgtggagcaacattccagggctgaagagcaagcatgcgcccctgaccccaaaggaagaagagtatctgcaagcccaagtcagaagcaggagcaagctggacgccccgaaagttgacctcctggtgaagaactgccttctcccgctgagagagtacttcaagtatttttctcaaaactcacttcctcttggagggccgagctctggcgcacccccaccaagtggagggtctcctgccgggtccccaacatctactgaagaaggcaccagcgaatccgcaacgggcagtggcagcggaggaagtggatccggcggtagtggtagtggaagcggcggatccggctcaggcggatctggttcaggggaagaactcctctccaaaaactaccatctcgagaatgaggtcgcccgcctgaaaaaaggatcaggttccggtggttctggcagcggtggttcaggctcaggcagcggcggtagcggtagcggtggaagcggaagcggaccaaaaaagaagagaaaggtaggaagcggagctactaacttcagcctgctgaagcaggctggagacgtggaggagaaccctggacctatgcctgctgctaagagagtgaaactggatggatccggccccgacatcgtgatgacccagagccccagcagcctgagcgccagcgtgggcgaccgcgtgaccatcacctgccgcagcagcaccggcgccgtgaccaccagcaactacgccagctgggtgcaggagaagcccggcaagctgttcaagggcctgatcggcggcaccaacaaccgcgcccccggcgtgcccagccgcttcagcggcagcctgatcggcgacaaggccaccctgaccatcagcagcctgcagcccgaggacttcgccacctacttctgcgccctgtggtacagcaaccactgggtgttcggccagggcaccaaggtggagctgaagcgcggcggcggcggcagcggcggcggcggcagcggcggcggcggcagcagcggcggcggcagcgaggtgaagctgctggagagcggcggcggcctggtgcagcccggcggcagcctgaagctgagctgcgccgtgagcggcttcagcctgaccgactacggcgtgaactgggtgcgccaggcccccggccgcggcctggagtggatcggcgtgatctggggcgacggcatcaccgactacaacagcgccctgaaggaccgcttcatcatcagcaaggacaacggcaagaacaccgtgtacctgcagatgagcaaggtgcgcagcgacgacaccgccctgtactactgcgtgaccggcctgttcgactactggggccagggcaccctggtgaccgtgagcagctacccatacgatgttccagattacgctggtggaggcggaggttctgggggaggaggtagtggcggtggtggttcaggaggcggcggaagcggaagcggaccaaaaaagaagagaaaggtaatggacaagaagtacagcatcggcctggccatcggcaccaactctgtgggctgggccgtgatcaccgacgagtacaaggtgcccagcaagaaattcaaggtgctgggcaacaccgaccggcacagcatcaagaagaacctgatcggcgccctgctgttcgacagcggagaaacagccgaggccacccggctgaagagaaccgccagaagaagatacaccagacggaagaaccggatctgctatctgcaagagatcttcagcaacgagatggccaaggtggacgacagcttcttccacagactggaagagtccttcctggtggaagaggataagaagcacgagcggcaccccatcttcggcaacatcgtggacgaggtggcctaccacgagaagtaccccaccatctaccacctgagaaagaaactggtggacagcaccgacaaggccgacctgcggctgatctatctggccctggcccacatgatcaagttccggggccacttcctgatcgagggcgacctgaaccccgacaacagcgacgtggacaagctgttcatccagctggtgcagacctacaaccagctgttcgaggaaaaccccatcaacgccagcggcgtggacgccaaggccatcctgtctgccagactgagcaagagcagacggctggaaaatctgatcgcccagctgcccggcgagaagaagaatggcctgttcggcaacctgattgccctgagcctgggcctgacccccaacttcaagagcaacttcgacctggccgaggatgccaaactgcagctgagcaaggacacctacgacgacgacctggacaacctgctggcccagatcggcgaccagtacgccgacctgtttctggccgccaagaacctgtccgacgccatcctgctgagcgacatcctgagagtgaacaccgagatcaccaaggcccccctgagcgcctctatgatcaagagatacgacgagcaccaccaggacctgaccctgctgaaagctctcgtgcggcagcagctgcctgagaagtacaaagagattttcttcgaccagagcaagaacggctacgccggctacatcgatggcggagccagccaggaagagttctacaagttcatcaagcccatcctggaaaagatggacggcaccgaggaactgctcgtgaagctgaacagagaggacctgctgcggaagcagcggaccttcgacaacggcagcatcccccaccagatccacctgggagagctgcacgccattctgcggcggcaggaagatttttacccattcctgaaggacaaccgggaaaagatcgagaagatcctgaccttccgcatcccctactacgtgggccctctggccaggggaaacagcagattcgcctggatgaccagaaagagcgaggaaaccatcaccccctggaacttcgaggaagtggtggacaagggcgccagcgcccagagcttcatcgagcggatgaccaacttcgataagaacctgcccaacgagaaggtgctgcccaagcacagcctgctgtacgagtacttcaccgtgtacaacgagctgaccaaagtgaaatacgtgaccgagggaatgagaaagcccgccttcctgagcggcgagcagaaaaaagccatcgtggacctgctgttcaagaccaaccggaaagtgaccgtgaagcagctgaaagaggactacttcaagaaaatcgagtgcttcgactccgtggaaatctccggcgtggaagatcggttcaacgcctccctgggcacataccacgatctgctgaaaattatcaaggacaaggacttcctggacaatgaggaaaacgaggacattctggaagatatcgtgctgaccctgacactgtttgaggacagagagatgatcgaggaacggctgaaaacctatgcccacctgttcgacgacaaagtgatgaagcagctgaagcggcggagatacaccggctggggcaggctgagccggaagctgatcaacggcatccgggacaagcagtccggcaagacaatcctggatttcctgaagtccgacggcttcgccaacagaaacttcatgcagctgatccacgacgacagcctgacctttaaagaggacatccagaaagcccaggtgtccggccagggcgatagcctgcacgagcacattgccaatctggccggcagccccgccattaagaagggcatcctgcagacagtgaaggtggtggacgagctcgtgaaagtgatgggccggcacaagcccgagaacatcgtgatcgaaatggccagagagaaccagaccacccagaagggacagaagaacagccgcgagagaatgaagcggatcgaagagggcatcaaagagctgggcagccagatcctgaaagaacaccccgtggaaaacacccagctgcagaacgagaagctgtacctgtactacctgcagaatgggcgggatatgtacgtggaccaggaactggacatcaaccggctgtccgactacgatgtggacgctatcgtgcctcagagctttctgaaggacgactccatcgataacaaagtgctgactcggagcgacaagaaccggggcaagagcgacaacgtgccctccgaagaggtcgtgaagaagatgaagaactactggcgccagctgctgaatgccaagctgattacccagaggaagttcgacaatctgaccaaggccgagagaggcggcctgagcgaactggataaggccggcttcatcaagagacagctggtggaaacccggcagatcacaaagcacgtggcacagatcctggactcccggatgaacactaagtacgacgagaacgacaaactgatccgggaagtgaaagtgatcaccctgaagtccaagctggtgtccgatttccggaaggatttccagttttacaaagtgcgcgagatcaacaactaccaccacgcccacgacgcctacctgaacgccgtcgtgggaaccgccctgatcaaaaagtaccctaagctggaaagcgagttcgtgtacggcgactacaaggtgtacgacgtgcggaagatgatcgccaagagcgagcaggaaatcggcaaggctaccgccaagtacttcttctacagcaacatcatgaactttttcaagaccgagattaccctggccaacggcgagatccggaagcggcctctgatcgagacaaacggcgaaacaggcgagatcgtgtgggataagggccgggactttgccaccgtgcggaaagtgctgtctatgccccaagtgaatatcgtgaaaaagaccgaggtgcagacaggcggcttcagcaaagagtctatcctgcccaagaggaacagcgacaagctgatcgccagaaagaaggactgggaccctaagaagtacggcggcttcgacagccccaccgtggcctattctgtgctggtggtggccaaagtggaaaagggcaagtccaagaaactgaagagtgtgaaagagctgctggggatcaccatcatggaaagaagcagcttcgagaagaatcccatcgactttctggaagccaagggctacaaagaagtgaaaaaggacctgatcatcaagctgcctaagtactccctgttcgagctggaaaacggccggaagagaatgctggcctctgccggcgaactgcagaagggaaacgaactggccctgccctccaaatatgtgaacttcctgtacctggccagccactatgagaagctgaagggctcccccgaggataatgagcagaaacagctgtttgtggaacagcacaaacactacctggacgagatcatcgagcagatcagcgagttctccaagagagtgatcctggccgacgctaatctggacaaggtgctgagcgcctacaacaagcacagagacaagcctatcagagagcaggccgagaatatcatccacctgtttaccctgaccaatctgggagcccctgccgccttcaagtactttgacaccaccatcgaccggaagaggtacaccagcaccaaagaggtgctggacgccaccctgatccaccagagcatcaccggcctgtacgagacacggatcgacctgtctcagctgggaggcgacgcctatccctatgacgtgcccgattatgccagcctgggcagcggctcccccaagaaaaaacgcaaggtggaagatcctaagaaaaagcggaaagtggacggcagcggcagcgagacccccggtaccagcgagagcgccacccccgagagccggacactggtgaccttcaaggatgtatttgtggacttcaccagggaggagtggaagctgctggacactgctcagcagatcgtgtacagaaatgtgatgctggagaactataagaacctggtttccttgggttatcagcttactaagccagatgtgatcctccggttggagaagggagaagagccctga

SEQ ID NO: 323 - DNA, 7563 bp, synthetic construct
  misc_feature 1..7563: note = CDS of V35_scFv-dCas9-KRAB-2a-1xGCN4-D3l-D3a
  source 1..7563: mol_type = other DNA
atgcctgctgctaagagagtgaaactggatggatccggccccgacatcgtgatgacccagagccccagcagcctgagcgccagcgtgggcgaccgcgtgaccatcacctgccgcagcagcaccggcgccgtgaccaccagcaactacgccagctgggtgcaggagaagcccggcaagctgttcaagggcctgatcggcggcaccaacaaccgcgcccccggcgtgcccagccgcttcagcggcagcctgatcggcgacaaggccaccctgaccatcagcagcctgcagcccgaggacttcgccacctacttctgcgccctgtggtacagcaaccactgggtgttcggccagggcaccaaggtggagctgaagcgcggcggcggcggcagcggcggcggcggcagcggcggcggcggcagcagcggcggcggcagcgaggtgaagctgctggagagcggcggcggcctggtgcagcccggcggcagcctgaagctgagctgcgccgtgagcggcttcagcctgaccgactacggcgtgaactgggtgcgccaggcccccggccgcggcctggagtggatcggcgtgatctggggcgacggcatcaccgactacaacagcgccctgaaggaccgcttcatcatcagcaaggacaacggcaagaacaccgtgtacctgcagatgagcaaggtgcgcagcgacgacaccgccctgtactactgcgtgaccggcctgttcgactactggggccagggcaccctggtgaccgtgagcagctacccatacgatgttccagattacgctggtggaggcggaggttctgggggaggaggtagtggcggtggtggttcaggaggcggcggaagcggaagcggaccaaaaaagaagagaaaggtaatggacaagaagtacagcatcggcctggccatcggcaccaactctgtgggctgggccgtgatcaccgacgagtacaaggtgcccagcaagaaattcaaggtgctgggcaacaccgaccggcacagcatcaagaagaacctgatcggcgccctgctgttcgacagcggagaaacagccgaggccacccggctgaagagaaccgccagaagaagatacaccagacggaagaaccggatctgctatctgcaagagatcttcagcaacgagatggccaaggtggacgacagcttcttccacagactggaagagtccttcctggtggaagaggataagaagcacgagcggcaccccatcttcggcaacatcgtggacgaggtggcctaccacgagaagtaccccaccatctaccacctgagaaagaaactggtggacagcaccgacaaggccgacctgcggctgatctatctggccctggcccacatgatcaagttccggggccacttcctgatcgagggcgacctgaaccccgacaacagcgacgtggacaagctgttcatccagctggtgcagacctacaaccagctgttcgaggaaaaccccatcaacgccagcggcgtggacgccaaggccatcctgtctgccagactgagcaagagcagacggctggaaaatctgatcgcccagctgcccggcgagaagaagaatggcctgttcggcaacctgattgccctgagcctgggcctgacccccaacttcaagagcaacttcgacctggccgaggatgccaaactgcagctgagcaaggacacctacgacgacgacctggacaacctgctggcccagatcggcgaccagtacgccgacctgtttctggccgccaagaacctgtccgacgccatcctgctgagcgacatcctgagagtgaacaccgagatcaccaaggcccccctgagcgcctctatgatcaagagatacgacgagcaccaccaggacctgaccctgctgaaagctctcgtgcggcagcagctgcctgagaagtacaaagagattttcttcgaccagagcaagaacggctacgccggctacatcgatggcggagccagccaggaagagttctacaagttcatcaagcccatcctggaaaagatggacggcaccgaggaactgctcgtgaagctgaacagagaggacctgctgcggaagcagcggaccttcgacaacggcagcatcccccaccagatccacctgggagagctgcacgccattctgcggcggcaggaagatttttacccattcctgaaggacaaccgggaaaagatcgagaagatcctgaccttccgcatcccctactacgtgggccctctggccaggggaaacagcagattcgcctggatgaccagaaagagcgaggaaaccatcaccccctggaacttcgaggaagtggtggacaagggcgccagcgcccagagcttcatcgagcggatgaccaacttcgataagaacctgcccaacgagaaggtgctgcccaagcacagcctgctgtacgagtacttcaccgtgtacaacgagctgaccaaagtgaaatacgtgaccgagggaatgagaaagcccgccttcctgagcggcgagcagaaaaaagccatcgtggacctgctgttcaagaccaaccggaaagtgaccgtgaagcagctgaaagaggactacttcaagaaaatcgagtgcttcgactccgtggaaatctccggcgtggaagatcggttcaacgcctccctgggcacataccacgatctgctgaaaattatcaaggacaaggacttcctggacaatgaggaaaacgaggacattctggaagatatcgtgctgaccctgacactgtttgaggacagagagatgatcgaggaacggctgaaaacctatgcccacctgttcgacgacaaagtgatgaagcagctgaagcggcggagatacaccggctggggcaggctgagccggaagctgatcaacggcatccgggacaagcagtccggcaagacaatcctggatttcctgaagtccgacggcttcgccaacagaaacttcatgcagctgatccacgacgacagcctgacctttaaagaggacatccagaaagcccaggtgtccggccagggcgatagcctgcacgagcacattgccaatctggccggcagccccgccattaagaagggcatcctgcagacagtgaaggtggtggacgagctcgtgaaagtgatgggccggcacaagcccgagaacatcgtgatcgaaatggccagagagaaccagaccacccagaagggacagaagaacagccgcgagagaatgaagcggatcgaagagggcatcaaagagctgggcagccagatcctgaaagaacaccccgtggaaaacacccagctgcagaacgagaagctgtacctgtactacctgcagaatgggcgggatatgtacgtggaccaggaactggacatcaaccggctgtccgactacgatgtggacgctatcgtgcctcagagctttctgaaggacgactccatcgataacaaagtgctgactcggagcgacaagaaccggggcaagagcgacaacgtgccctccgaagaggtcgtgaagaagatgaagaactactggcgccagctgctgaatgccaagctgattacccagaggaagttcgacaatctgaccaaggccgagagaggcggcctgagcgaactggataaggccggcttcatcaagagacagctggtggaaacccggcagatcacaaagcacgtggcacagatcctggactcccggatgaacactaagtacgacgagaacgacaaactgatccgggaagtgaaagtgatcaccctgaagtccaagctggtgtccgatttccggaaggatttccagttttacaaagtgcgcgagatcaacaactaccaccacgcccacgacgcctacctgaacgccgtcgtgggaaccgccctgatcaaaaagtaccctaagctggaaagcgagttcgtgtacggcgactacaaggtgtacgacgtgcggaagatgatcgccaagagcgagcaggaaatcggcaaggctaccgccaagtacttcttctacagcaacatcatgaactttttcaagaccgagattaccctggccaacggcgagatccggaagcggcctctgatcgagacaaacggcgaaacaggcgagatcgtgtgggataagggccgggactttgccaccgtgcggaaagtgctgtctatgccccaagtgaatatcgtgaaaaagaccgaggtgcagacaggcggcttcagcaaagagtctatcctgcccaagaggaacagcgacaagctgatcgccagaaagaaggactgggaccctaagaagtacggcggcttcgacagccccaccgtggcctattctgtgctggtggtggccaaagtggaaaagggcaagtccaagaaactgaagagtgtgaaagagctgctggggatcaccatcatggaaagaagcagcttcgagaagaatcccatcgactttctggaagccaagggctacaaagaagtgaaaaaggacctgatcatcaagctgcctaagtactccctgttcgagctggaaaacggccggaagagaatgctggcctctgccggcgaactgcagaagggaaacgaactggccctgccctccaaatatgtgaacttcctgtacctggccagccactatgagaagctgaagggctcccccgaggataatgagcagaaacagctgtttgtggaacagcacaaacactacctggacgagatcatcgagcagatcagcgagttctccaagagagtgatcctggccgacgctaatctggacaaggtgctgagcgcctacaacaagcacagagacaagcctatcagagagcaggccgagaatatcatccacctgtttaccctgaccaatctgggagcccctgccgccttcaagtactttgacaccaccatcgaccggaagaggtacaccagcaccaaagaggtgctggacgccaccctgatccaccagagcatcaccggcctgtacgagacacggatcgacctgtctcagctgggaggcgacgcctatccctatgacgtgcccgattatgccagcctgggcagcggctcccccaagaaaaaacgcaaggtggaagatcctaagaaaaagcggaaagtggacggcagcggcagcgagacccccggtaccagcgagagcgccacccccgagagccggacactggtgaccttcaaggatgtatttgtggacttcaccagggaggagtggaagctgctggacactgctcagcagatcgtgtacagaaatgtgatgctggagaactataagaacctggtttccttgggttatcagcttactaagccagatgtgatcctccggttggagaagggagaagagcccggaagcggagctactaacttcagcctgctgaagcaggctggagacgtggaggagaaccctggacctatgcctgctgctaagagagtgaaactggatggatccggctcaggcggatctggttcaggggaagaactcctctccaaaaactaccatctcgagaatgaggtcgcccgcctgaaaaaaggatcaggttccggtggttctggcagcggtggttcaggctcaggcagcggcggtagcggtagcggtggaagcggaagcggaacccccggtaccagcgagggcggccctagcagcggcgcccctccccctagcggcggcagccctgccggatcccctacaagcaccgaagaaggcacaagcgagtccgctacccctgagtccggccctggcacctccacagagcctagcgagggatccgctcctggatcccctgccggaagccctacctccaccgaggagggcacaagcaccgagccttccgagggcagcgcccccggaacaagcaccgaacctagcgagagcgccacccccgagagcatgttcgaaaccgtgcctgtgtggaggagacagccagtccgggtgctgtccctttttgaagacatcaagaaagagctgacgagtttgggctttttggaaagtggttctgacccgggacaactgaagcatgtggttgatgtcacagacacagtgaggaaggatgtggaggagtggggacccttcgatcttgtgtacggcgccacacctcccctgggccacacctgtgaccgtcctcccagctggtacctgttccagttccaccggctcctgcagtacgcacggcccaagccaggcagccccaggcccttcttctggatgttcgtggacaatctggtgctgaacaaggaagacctggacgtcgcatctcgcttcctggagatggagccagtcaccatcccagatgtccacggcggatccttgcagaatgctgtccgcgtgtggagcaacatcccagccataaggagcagcaggcactgggctctggtttcggaagaagaattgtccctgctggcccagaacaagcagagctcgaagctcgcggccaagtggcccaccaagctggtgaagaactgctttctccccctaagagaatatttcaagtatttttcaacagaactcacttcctctttatctagcggcaatagtaacgctaacagccgcgggccgagcttcagcagcggcctggtgccgttaagcttgcgcggcagccatatgaaccatgaccaggaatttgaccccccaaaggtttacccacctgtgccagctgagaagaggaagcccatccgcgtgctgtctctctttgatgggattgctacagggctcctggtgctgaaggacctgggcatccaagtggaccgctacattgcctccgaggtgtgtgaggactccatcacggtgggcatggtgcggcaccagggaaagatcatgtacgtcggggacgtccgcagcgtcacacagaagcatatccaggagtggggcccattcgacctggtgattggaggcagtccctgcaatgacctctccattgtcaaccctgcccgcaagggactttatgagggtactggccgcctcttctttgagttctaccgcctcctgcatgatgcgcggcccaaggagggagatgatcgccccttcttctggctctttgagaatgtggtggccatgggcgttagtgacaagagggacatctcgcgatttcttgagtctaaccccgtgatgattgacgccaaagaagtgtctgctgcacacagggcccgttacttctggggtaaccttcctggcatgaacaggcctttggcatccactgtgaatgataagctggagctgcaagagtgtctggagcacggcagaatagccaagttcagcaaagtgaggaccattaccaccaggtcaaactctataaagcagggcaaagaccagcatttccccgtcttcatgaacgagaaggaggacatcctgtggtgcactgaaatggaaagggtgtttggcttccccgtccactacacagacgtctccaacatgagccgcttggcgaggcagagactgctgggccgatcgtggagcgtgccggtcatccgccacctcttcgctccgctgaaggaatattttgcttgtgtgctcgaggctactaacttcagcctgctgaagcaggctggagacgtggaggagaaccctggacctatgcattaa

SEQ ID NO: 324 - DNA, 7959 bp, synthetic construct
  misc_feature 1..7959: note = CDS of V36_scFv-dCas9-HP1a-2a-1xGCN4-D3l-D3a
  source 1..7959: mol_type = other DNA
atgcctgctgctaagagagtgaaactggatggatccggccccgacatcgtgatgacccagagccccagcagcctgagcgccagcgtgggcgaccgcgtgaccatcacctgccgcagcagcaccggcgccgtgaccaccagcaactacgccagctgggtgcaggagaagcccggcaagctgttcaagggcctgatcggcggcaccaacaaccgcgcccccggcgtgcccagccgcttcagcggcagcctgatcggcgacaaggccaccctgaccatcagcagcctgcagcccgaggacttcgccacctacttctgcgccctgtggtacagcaaccactgggtgttcggccagggcaccaaggtggagctgaagcgcggcggcggcggcagcggcggcggcggcagcggcggcggcggcagcagcggcggcggcagcgaggtgaagctgctggagagcggcggcggcctggtgcagcccggcggcagcctgaagctgagctgcgccgtgagcggcttcagcctgaccgactacggcgtgaactgggtgcgccaggcccccggccgcggcctggagtggatcggcgtgatctggggcgacggcatcaccgactacaacagcgccctgaaggaccgcttcatcatcagcaaggacaacggcaagaacaccgtgtacctgcagatgagcaaggtgcgcagcgacgacaccgccctgtactactgcgtgaccggcctgttcgactactggggccagggcaccctggtgaccgtgagcagctacccatacgatgttccagattacgctggtggaggcggaggttctgggggaggaggtagtggcggtggtggttcaggaggcggcggaagcggaagcggaccaaaaaagaagagaaaggtaatggacaagaagtacagcatcggcctggccatcggcaccaactctgtgggctgggccgtgatcaccgacgagtacaaggtgcccagcaagaaattcaaggtgctgggcaacaccgaccggcacagcatcaagaagaacctgatcggcgccctgctgttcgacagcggagaaacagccgaggccacccggctgaagagaaccgccagaagaagatacaccagacggaagaaccggatctgctatctgcaagagatcttcagcaacgagatggccaaggtggacgacagcttcttccacagactggaagagtccttcctggtggaagaggataagaagcacgagcggcaccccatcttcggcaacatcgtggacgaggtggcctaccacgagaagtaccccaccatctaccacctgagaaagaaactggtggacagcaccgacaaggccgacctgcggctgatctatctggccctggcccacatgatcaagttccggggccacttcctgatcgagggcgacctgaaccccgacaacagcgacgtggacaagctgttcatccagctggtgcagacctacaaccagctgttcgaggaaaaccccatcaacgccagcggcgtggacgccaaggccatcctgtctgccagactgagcaagagcagacggctggaaaatctgatcgcccagctgcccggcgagaagaagaatggcctgttcggcaacctgattgccctgagcctgggcctgacccccaacttcaagagcaacttcgacctggccgaggatgccaaactgcagctgagcaaggacacctacgacgacgacctggacaacctgctggcccagatcggcgaccagtacgccgacctgtttctggccgccaagaacctgtccgacgccatcctgctgagcgacatcctgagagtgaacaccgagatcaccaaggcccccctgagcgcctctatgatcaagagatacgacgagcaccaccaggacctgaccctgctgaaagctctcgtgcggcagcagctgcctgagaagtacaaagagattttcttcgaccagagcaagaacggctacgccggctacatcgatggcggagccagccaggaagagttctacaagttcatcaagcccatcctggaaaagatggacggcaccgaggaactgctcgtgaagctgaacagagaggacctgctgcggaagcagcggaccttcgacaacggcagcatcccccaccagatccacctgggagagctgcacgccattctgcggcggcaggaagatttttacccattcctgaaggacaaccgggaaaagatcgagaagatcctgaccttccgcatcccctactacgtgggccctctggccaggggaaacagcagattcgcctggatgaccagaaagagcgaggaaaccatcaccccctggaacttcgaggaagtggtggacaagggcgccagcgcccagagcttcatcgagcggatgaccaacttcgataagaacctgcccaacgagaaggtgctgcccaagcacagcctgctgtacgagtacttcaccgtgtacaacgagctgaccaaagtgaaatacgtgaccgagggaatgagaaagcccgccttcctgagcggcgagcagaaaaaagccatcgtggacctgctgttcaagaccaaccggaaagtgaccgtgaagcagctgaaagaggactacttcaagaaaatcgagtgcttcgactccgtggaaatctccggcgtggaagatcggttcaacgcctccctgggcacataccacgatctgctgaaaattatcaaggacaaggacttcctggacaatgaggaaaacgaggacattctggaagatatcgtgctgaccctgacactgtttgaggacagagagatgatcgaggaacggctgaaaacctatgcccacctgttcgacgacaaagtgatgaagcagctgaagcggcggagatacaccggctggggcaggctgagccggaagctgatcaacggcatccgggacaagcagtccggcaagacaatcctggatttcctgaagtccgacggcttcgccaacagaaacttcatgcagctgatccacgacgacagcctgacctttaaagaggacatccagaaagcccaggtgtccggccagggcgatagcctgcacgagcacattgccaatctggccggcagccccgccattaagaagggcatcctgcagacagtgaaggtggtggacgagctcgtgaaagtgatgggccggcacaagcccgagaacatcgtgatcgaaatggccagagagaaccagaccacccagaagggacagaagaacagccgcgagagaatgaagcggatcgaagagggcatcaaagagctgggcagccagatcctgaaagaacaccccgtggaaaacacccagctgcagaacgagaagctgtacctgtactacctgcagaatgggcgggatatgtacgtggaccaggaactggacatcaaccggctgtccgactacgatgtggacgctatcgtgcctcagagctttctgaaggacgactccatcgataacaaagtgctgactcggagcgacaagaaccggggcaagagcgacaacgtgccctccgaagaggtcgtgaagaagatgaagaactactggcgccagctgctgaatgccaagctgattacccagaggaagttcgacaatctgaccaaggccgagagaggcggcctgagcgaactggataaggccggcttcatcaagagacagctggtggaaacccggcagatcacaaagcacgtggcacagatcctggactcccggatgaacactaagtacgacgagaacgacaaactgatccgggaagtgaaagtgatcaccctgaagtccaagctggtgtccgatttccggaaggatttccagttttacaaagtgcgcgagatcaacaactaccaccacgcccacgacgcctacctgaacgccgtcgtgggaaccgccctgatcaaaaagtaccctaagctggaaagcgagttcgtgtacggcgactacaaggtgtacgacgtgcggaagatgatcgccaagagcgagcaggaaatcggcaaggctaccgccaagtacttcttctacagcaacatcatgaactttttcaagaccgagattaccctggccaacggcgagatccggaagcggcctctgatcgagacaaacggcgaaacaggcgagatcgtgtgggataagggccgggactttgccaccgtgcggaaagtgctgtctatgccccaagtgaatatcgtgaaaaagaccgaggtgcagacaggcggcttcagcaaagagtctatcctgcccaagaggaacagcgacaagctgatcgccagaaagaaggactgggaccctaagaagtacggcggcttcgacagccccaccgtggcctattctgtgctggtggtggccaaagtggaaaagggcaagtccaagaaactgaagagtgtgaaagagctgctggggatcaccatcatggaaagaagcagcttcgagaagaatcccatcgactttctggaagccaagggctacaaagaagtgaaaaaggacctgatcatcaagctgcctaagtactccctgttcgagctggaaaacggccggaagagaatgctggcctctgccggcgaactgcagaagggaaacgaactggccctgccctccaaatatgtgaacttcctgtacctggccagccactatgagaagctgaagggctcccccgaggataatgagcagaaacagctgtttgtggaacagcacaaacactacctggacgagatcatcgagcagatcagcgagttctccaagagagtgatcctggccgacgctaatctggacaaggtgctgagcgcctacaacaagcacagagacaagcctatcagagagcaggccgagaatatcatccacctgtttaccctgaccaatctgggagcccctgccgccttcaagtactttgacaccaccatcgaccggaagaggtacaccagcaccaaagaggtgctggacgccaccctgatccaccagagcatcaccggcctgtacgagacacggatcgacctgtctcagctgggaggcgacgcctatccctatgacgtgcccgattatgccagcctgggcagcggctcccccaagaaaaaacgcaaggtggaagatcctaagaaaaagcggaaagtggacggcagcggcagcgagacccccggtaccagcgagagcgccacccccgagagccggacactcggaaagaaaaccaagcggacagctgacagttcttcttcagaggatgaggaggagtatgttgtggagaaggtgctagacaggcgcgtggttaagggacaagtggaatatctactgaagtggaaaggcttttctgaggagcacaatacttgggaacctgagaaaaacttggattgccctgagctaatttctgaatttatgaaaaagtataagaagatgaaggagggtgaaaataataaacccagggagaagtcagaaagtaacaagaggaaatccaatttctcaaacagtgccgatgacatcaaatctaaaaaaaagagagagcagagcaatgatatcgctcggggctttgagagaggactggaaccagaaaagatcattggggcaacagattcctgtggtgatttaatgttcctaatgaaatggaaagacacagatgaagctgacctggttcttgcaaaagaagctaatgtgaaatgtccacaaattgtgatagcattttatgaagagagactgacatggcatgcatatcctgaggatgcggaaaacaaagagaaagaaacagcaaagagcgagggcagcggcgctactaacttcagcctgctgaagcaggctggagacgtggaggagaaccctggacctatgcctgctgctaagagagtgaaactggatggatccggctcaggcggatctggttcaggggaagaactcctctccaaaaactaccatctcgagaatgaggtcgcccgcctgaaaaaaggatcaggttccggtggttctggcagcggtggttcaggctcaggcagcggcggtagcggtagcggtggaagcggaagcggaacccccggtaccagcgagggcggccctagcagcggcgcccctccccctagcggcggcagccctgccggatcccctacaagcaccgaagaaggcacaagcgagtccgctacccctgagtccggccctggcacctccacagagcctagcgagggatccgctcctggatcccctgccggaagccctacctccaccgaggagggcacaagcaccgagccttccgagggcagcgcccccggaacaagcaccgaacctagcgagagcgccacccccgagagcatgttcgaaaccgtgcctgtgtggaggagacagccagtccgggtgctgtccctttttgaagacatcaagaaagagctgacgagtttgggctttttggaaagtggttctgacccgggacaactgaagcatgtggttgatgtcacagacacagtgaggaaggatgtggaggagtggggacccttcgatcttgtgtacggcgccacacctcccctgggccacacctgtgaccgtcctcccagctggtacctgttccagttccaccggctcctgcagtacgcacggcccaagccaggcagccccaggcccttcttctggatgttcgtggacaatctggtgctgaacaaggaagacctggacgtcgcatctcgcttcctggagatggagccagtcaccatcccagatgtccacggcggatccttgcagaatgctgtccgcgtgtggagcaacatcccagccataaggagcagcaggcactgggctctggtttcggaagaagaattgtccctgctggcccagaacaagcagagctcgaagctcgcggccaagtggcccaccaagctggtgaagaactgctttctccccctaagagaatatttcaagtatttttcaacagaactcacttcctctttatctagcggcaatagtaacgctaacagccgcgggccgagcttcagcagcggcctggtgccgttaagcttgcgcggcagccatatgaaccatgaccaggaatttgaccccccaaaggtttacccacctgtgccagctgagaagaggaagcccatccgcgtgctgtctctctttgatgggattgctacagggctcctggtgctgaaggacctgggcatccaagtggaccgctacattgcctccgaggtgtgtgaggactccatcacggtgggcatggtgcggcaccagggaaagatcatgtacgtcggggacgtccgcagcgtcacacagaagcatatccaggagtggggcccattcgacctggtgattggaggcagtccctgcaatgacctctccattgtcaaccctgcccgcaagggactttatgagggtactggccgcctcttctttgagttctaccgcctcctgcatgatgcgcggcccaaggagggagatgatcgccccttcttctggctctttgagaatgtggtggccatgggcgttagtgacaagagggacatctcgcgatttcttgagtctaaccccgtgatgattgacgccaaagaagtgtctgctgcacacagggcccgttacttctggggtaaccttcctggcatgaacaggcctttggcatccactgtgaatgataagctggagctgcaagagtgtctggagcacggcagaatagccaagttcagcaaagtgaggaccattaccaccaggtcaaactctataaagcagggcaaagaccagcatttccccgtcttcatgaacgagaaggaggacatcctgtggtgcactgaaatggaaagggtgtttggcttccccgtccactacacagacgtctccaacatgagccgcttggcgaggcagagactgctgggccgatcgtggagcgtgccggtcatccgccacctcttcgctccgctgaaggaatattttgcttgtgtgctcgaggctactaacttcagcctgctgaagcaggctggagacgtggaggagaaccctggacctatgcattaa

SEQ ID NO: 325 - DNA, 7713 bp, synthetic construct
  misc_feature 1..7713: note = CDS of V37_GFP1-10-KRAB-2a-D3a-D3l-dCas9-7xGFP11
  source 1..7713: mol_type = other DNA
atgtccaagggagaggagctgttcaccggagtggtgccaatcctggtggagctggacggcgatgtgaacggccacaagttttctgtgcgcggagagggagagggcgacgcaaccatcggcaagctgacactgaagttcatctgcaccacaggcaagctgcccgtgccttggccaaccctggtgaccacactgacatacggcgtgcagtgtttctctaggtatccagaccacatgaagagacacgatttctttaagagcgccatgccagagggatacgtgcaggagcggaccatctccttcaaggacgatggcaagtataagacccgcgccgtggtgaagtttgagggcgatacactggtgaacaggatcgagctgaagggcaccgacttcaaggaggatggcaatatcctgggccacaagctggagtacaactttaatagccacaacgtgtatatcacagccgacaagcagaagaacggcatcaaggccaacttcaccgtgaggcacaatgtggaggacggctccgtgcagctggccgatcactaccagcagaacacacctatcggcgacggacccgtgctgctgcctgataatcactatctgtccacccagacagtgctgtctaaggacccaaacgagaagttggatccaggtggaggtggaagcggtcggacactggtgaccttcaaggatgtatttgtggacttcaccagggaggagtggaagctgctggacactgctcagcagatcgtgtacagaaatgtgatgctggagaactataagaacctggtttccttgggttatcagcttactaagccagatgtgatcctccggttggagaagggagaagagcccggaagcggaaagcgcaccgccgatggttccgagttcgaaagccccaaaaaaaagcgcaaggtcggaagcggagctactaacttcagcctgctgaagcaggctggagacgtggaggagaaccctggacctcctgctgctaagagagtgaaactggatggatccaaccatgaccaggaatttgaccccccaaaggtttacccacctgtgccagctgagaagaggaagcccatccgcgtgctgtctctctttgatgggattgctacagggctcctggtgctgaaggacctgggcatccaagtggaccgctacattgcctccgaggtgtgtgaggactccatcacggtgggcatggtgcggcaccagggaaagatcatgtacgtcggggacgtccgcagcgtcacacagaagcatatccaggagtggggcccattcgacctggtgattggaggcagtccctgcaatgacctctccattgtcaaccctgcccgcaagggactttatgagggtactggccgcctcttctttgagttctaccgcctcctgcatgatgcgcggcccaaggagggagatgatcgccccttcttctggctctttgagaatgtggtggccatgggcgttagtgacaagagggacatctcgcgatttcttgagtctaaccccgtgatgattgacgccaaagaagtgtctgctgcacacagggcccgttacttctggggtaaccttcctggcatgaacaggcctttggcatccactgtgaatgataagctggagctgcaagagtgtctggagcacggcagaatagccaagttcagcaaagtgaggaccattaccaccaggtcaaactctataaagcagggcaaagaccagcatttccccgtgttcatgaacgagaaggaggacatcctgtggtgcactgaaatggaaagggtgtttggcttccccgtccactacacagacgtctccaacatgagccgcttggcgaggcagagactgctgggccgatcgtggagcgtgccggtcatccgccacctcttcgctccgctgaaggaatattttgcttgtgtgtctagcggcaatagtaacgctaacagccgcgggccgagcttcagcagcggcctggtgccgttaagcttgcgcggcagccatatgggccctatggagatatacaagacagtgtctgcatggaagagacagccagtgcgggtactgagcctcttcagaaacatcgacaaggtactaaagagtttgggcttcttggaaagcggttctggttctgggggaggaacgctgaagtacgtggaagatgtcacaaatgtcgtgaggagagacgtggagaaatggggcccctttgacctggtgtacggctcgacgcagcccctaggcagctcttgtgatcgctgtcccggctggtacatgttccagttccaccggatcctgcagtatgcgctgcctcgccaggagagtcagcggcccttcttctggatattcatggacaatctgctgctgactgaggatgaccaagagacaactacccgcttccttcagacagaggctgtgaccctccaggatgtccgtggcagagactaccagaatgctatgcgggtgtggagcaacattccagggctgaagagcaagcatgcgcccctgaccccaaaggaagaagagtatctgcaagcccaagtcagaagcaggagcaagctggacgccccgaaagttgacctcctggtgaagaactgccttctcccgctgagagagtacttcaagtatttttctcaaaactcacttcctcttggagggccgagctctggcgcacccccaccaagtggagggtctcctgccgggtccccaacatctactgaagaaggcaccagcgaatccgcaacgcccgagtcaggccctggtacctccacagaaccatctgaaggtagtgcgcctggttccccagctggaagccctacttccaccgaagaaggcacgtcaaccgaaccaagtgaaggatctgcccctgggaccagcactgaaccatctgagccaaaaaagaagagaaaggtaatggacaagaagtacagcatcggcctggccatcggcaccaactctgtgggctgggccgtgatcaccgacgagtacaaggtgcccagcaagaaattcaaggtgctgggcaacaccgaccggcacagcatcaagaagaacctgatcggcgccctgctgttcgacagcggagaaacagccgaggccacccggctgaagagaaccgccagaagaagatacaccagacggaagaaccggatctgctatctgcaagagatcttcagcaacgagatggccaaggtggacgacagcttcttccacagactggaagagtccttcctggtggaagaggataagaagcacgagcggcaccccatcttcggcaacatcgtggacgaggtggcctaccacgagaagtaccccaccatctaccacctgagaaagaaactggtggacagcaccgacaaggccgacctgcggctgatctatctggccctggcccacatgatcaagttccggggccacttcctgatcgagggcgacctgaaccccgacaacagcgacgtggacaagctgttcatccagctggtgcagacctacaaccagctgttcgaggaaaaccccatcaacgccagcggcgtggacgccaaggccatcctgtctgccagactgagcaagagcagacggctggaaaatctgatcgcccagctgcccggcgagaagaagaatggcctgttcggcaacctgattgccctgagcctgggcctgacccccaacttcaagagcaacttcgacctggccgaggatgccaaactgcagctgagcaaggacacctacgacgacgacctggacaacctgctggcccagatcggcgaccagtacgccgacctgtttctggccgccaagaacctgtccgacgccatcctgctgagcgacatcctgagagtgaacaccgagatcaccaaggcccccctgagcgcctctatgatcaagagatacgacgagcaccaccaggacctgaccctgctgaaagctctcgtgcggcagcagctgcctgagaagtacaaagagattttcttcgaccagagcaagaacggctacgccggctacatcgatggcggagccagccaggaagagttctacaagttcatcaagcccatcctggaaaagatggacggcaccgaggaactgctcgtgaagctgaacagagaggacctgctgcggaagcagcggaccttcgacaacggcagcatcccccaccagatccacctgggagagctgcacgccattctgcggcggcaggaagatttttacccattcctgaaggacaaccgggaaaagatcgagaagatcctgaccttccgcatcccctactacgtgggccctctggccaggggaaacagcagattcgcctggatgaccagaaagagcgaggaaaccatcaccccctggaacttcgaggaagtggtggacaagggcgccagcgcccagagcttcatcgagcggatgaccaacttcgataagaacctgcccaacgagaaggtgctgcccaagcacagcctgctgtacgagtacttcaccgtgtacaacgagctgaccaaagtgaaatacgtgaccgagggaatgagaaagcccgccttcctgagcggcgagcagaaaaaagccatcgtggacctgctgttcaagaccaaccggaaagtgaccgtgaagcagctgaaagaggactacttcaagaaaatcgagtgcttcgactccgtggaaatctccggcgtggaagatcggttcaacgcctccctgggcacataccacgatctgctgaaaattatcaaggacaaggacttcctggacaatgaggaaaacgaggacattctggaagatatcgtgctgaccctgacactgtttgaggacagagagatgatcgaggaacggctgaaaacctatgcccacctgttcgacgacaaagtgatgaagcagctgaagcggcggagatacaccggctggggcaggctgagccggaagctgatcaacggcatccgggacaagcagtccggcaagacaatcctggatttcctgaagtccgacggcttcgccaacagaaacttcatgcagctgatccacgacgacagcctgacctttaaagaggacatccagaaagcccaggtgtccggccagggcgatagcctgcacgagcacattgccaatctggccggcagccccgccattaagaagggcatcctgcagacagtgaaggtggtggacgagctcgtgaaagtgatgggccggcacaagcccgagaacatcgtgatcgaaatggccagagagaaccagaccacccagaagggacagaagaacagccgcgagagaatgaagcggatcgaagagggcatcaaagagctgggcagccagatcctgaaagaacaccccgtggaaaacacccagctgcagaacgagaagctgtacctgtactacctgcagaatgggcgggatatgtacgtggaccaggaactggacatcaaccggctgtccgactacgatgtggacgctatcgtgcctcagagctttctgaaggacgactccatcgataacaaagtgctgactcggagcgacaagaaccggggcaagagcgacaacgtgccctccgaagaggtcgtgaagaagatgaagaactactggcgccagctgctgaatgccaagctgattacccagaggaagttcgacaatctgaccaaggccgagagaggcggcctgagcgaactggataaggccggcttcatcaagagacagctggtggaaacccggcagatcacaaagcacgtggcacagatcctggactcccggatgaacactaagtacgacgagaacgacaaactgatccgggaagtgaaagtgatcaccctgaagtccaagctggtgtccgatttccggaaggatttccagttttacaaagtgcgcgagatcaacaactaccaccacgcccacgacgcctacctgaacgccgtcgtgggaaccgccctgatcaaaaagtaccctaagctggaaagcgagttcgtgtacggcgactacaaggtgtacgacgtgcggaagatgatcgccaagagcgagcaggaaatcggcaaggctaccgccaagtacttcttctacagcaacatcatgaactttttcaagaccgagattaccctggccaacggcgagatccggaagcggcctctgatcgagacaaacggcgaaacaggcgagatcgtgtgggataagggccgggactttgccaccgtgcggaaagtgctgtctatgccccaagtgaatatcgtgaaaaagaccgaggtgcagacaggcggcttcagcaaagagtctatcctgcccaagaggaacagcgacaagctgatcgccagaaagaaggactgggaccctaagaagtacggcggcttcgacagccccaccgtggcctattctgtgctggtggtggccaaagtggaaaagggcaagtccaagaaactgaagagtgtgaaagagctgctggggatcaccatcatggaaagaagcagcttcgagaagaatcccatcgactttctggaagccaagggctacaaagaagtgaaaaaggacctgatcatcaagctgcctaagtactccctgttcgagctggaaaacggccggaagagaatgctggcctctgccggcgaactgcagaagggaaacgaactggccctgccctccaaatatgtgaacttcctgtacctggccagccactatgagaagctgaagggctcccccgaggataatgagcagaaacagctgtttgtggaacagcacaaacactacctggacgagatcatcgagcagatcagcgagttctccaagagagtgatcctggccgacgctaatctggacaaggtgctgagcgcctacaacaagcacagagacaagcctatcagagagcaggccgagaatatcatccacctgtttaccctgaccaatctgggagcccctgccgccttcaagtactttgacaccaccatcgaccggaagaggtacaccagcaccaaagaggtgctggacgccaccctgatccaccagagcatcaccggcctgtacgagacacggatcgacctgtctcagctgggaggcgacgcctatccctatgacgtgcccgattatgccagcctgggcagcggctcccccaagaaaaaacgcaaggtggaagatcctaagaaaaagcggaaagtggacggcagcggcagcgagacccccggtaccagcgagagcgccacccccgagagcggtagtgggagcaacggcagcagcggatccatgcgtgaccacatggtccttcatgagtatgtaaatgctgctgggattacaggtggctctggaggtagagatcatatggttctccacgaatacgttaacgccgcaggcatcactggcggtagtggaggacgcgaccatatggtactacatgaatatgtcaatgcagccggaataaccggagggtccggaggccgggatcacatggtgctgcatgagtatgtgaacgcggcgggtataactggtgggtcgggcggacgagaccatatggtgcttcacgaatacgtaaacgcagctggcattactggcggatcaggtggcagggatcacatggtactccatgagtacgtgaacgctgctggaatcacaggcggtagcggcggtcgggaccatatggtcctgcacgaatatgtcaatgctgccggtatcaccgcggccgcaaggtcaggctccggccagcggggaagcaagcgcaccgccgatggttccgagttcgaaagccccaaaaaaaagcgcaaggtctga

SEQ ID NO: 326 - DNA, 7335 bp, synthetic construct
  misc_feature 1..7335: note = CDS of V38_GFP1-10-KRAB-2a-D3a-D3l-dCas9-1xGFP11
  source 1..7335: mol_type = other DNA
atgtccaagggagaggagctgttcaccggagtggtgccaatcctggtggagctggacggcgatgtgaacggccacaagttttctgtgcgcggagagggagagggcgacgcaaccatcggcaagctgacactgaagttcatctgcaccacaggcaagctgcccgtgccttggccaaccctggtgaccacactgacatacggcgtgcagtgtttctctaggtatccagaccacatgaagagacacgatttctttaagagcgccatgccagagggatacgtgcaggagcggaccatctccttcaaggacgatggcaagtataagacccgcgccgtggtgaagtttgagggcgatacactggtgaacaggatcgagctgaagggcaccgacttcaaggaggatggcaatatcctgggccacaagctggagtacaactttaatagccacaacgtgtatatcacagccgacaagcagaagaacggcatcaaggccaacttcaccgtgaggcacaatgtggaggacggctccgtgcagctggccgatcactaccagcagaacacacctatcggcgacggacccgtgctgctgcctgataatcactatctgtccacccagacagtgctgtctaaggacccaaacgagaagttggatccaggtggaggtggaagcggtcggacactggtgaccttcaaggatgtatttgtggacttcaccagggaggagtggaagctgctggacactgctcagcagatcgtgtacagaaatgtgatgctggagaactataagaacctggtttccttgggttatcagcttactaagccagatgtgatcctccggttggagaagggagaagagcccggaagcggaaagcgcaccgccgatggttccgagttcgaaagccccaaaaaaaagcgcaaggtcggaagcggagctactaacttcagcctgctgaagcaggctggagacgtggaggagaaccctggacctcctgctgctaagagagtgaaactggatggatccaaccatgaccaggaatttgaccccccaaaggtttacccacctgtgccagctgagaagaggaagcccatccgcgtgctgtctctctttgatgggattgctacagggctcctggtgctgaaggacctgggcatccaagtggaccgctacattgcctccgaggtgtgtgaggactccatcacggtgggcatggtgcggcaccagggaaagatcatgtacgtcggggacgtccgcagcgtcacacagaagcatatccaggagtggggcccattcgacctggtgattggaggcagtccctgcaatgacctctccattgtcaaccctgcccgcaagggactttatgagggtactggccgcctcttctttgagttctaccgcctcctgcatgatgcgcggcccaaggagggagatgatcgccccttcttctggctctttgagaatgtggtggccatgggcgttagtgacaagagggacatctcgcgatttcttgagtctaaccccgtgatgattgacgccaaagaagtgtctgctgcacacagggcccgttacttctggggtaaccttcctggcatgaacaggcctttggcatccactgtgaatgataagctggagctgcaagagtgtctggagcacggcagaatagccaagttcagcaaagtgaggaccattaccaccaggtcaaactctataaagcagggcaaagaccagcatttccccgtgttcatgaacgagaaggaggacatcctgtggtgcactgaaatggaaagggtgtttggcttccccgtccactacacagacgtctccaacatgagccgcttggcgaggcagagactgctgggccgatcgtggagcgtgccggtcatccgccacctcttcgctccgctgaaggaatattttgcttgtgtgtctagcggcaatagtaacgctaacagccgcgggccgagcttcagcagcggcctggtgccgttaagcttgcgcggcagccatatgggccctatggagatatacaagacagtgtctgcatggaagagacagccagtgcgggtactgagcctcttcagaaacatcgacaaggtactaaagagtttgggcttcttggaaagcggttctggttctgggggaggaacgctgaagtacgtggaagatgtcacaaatgtcgtgaggagagacgtggagaaatggggcccctttgacctggtgtacggctcgacgcagcccctaggcagctcttgtgatcgctgtcccggctggtacatgttccagttccaccggatcctgcagtatgcgctgcctcgccaggagagtcagcggcccttcttctggatattcatggacaatctgctgctgactgaggatgaccaagagacaactacccgcttccttcagacagaggctgtgaccctccaggatgtccgtggcagagactaccagaatgctatgcgggtgtggagcaacattccagggctgaagagcaagcatgcgcccctgaccccaaaggaagaagagtatctgcaagcccaagtcagaagcaggagcaagctggacgccccgaaagttgacctcctggtgaagaactgccttctcccgctgagagagtacttcaagtatttttctcaaaactcacttcctcttggagggccgagctctggcgcacccccaccaagtggagggtctcctgccgggtccccaacatctactgaagaaggcaccagcgaatccgcaacgcccgagtcaggccctggtacctccacagaaccatctgaaggtagtgcgcctggttccccagctggaagccctacttccaccgaagaaggcacgtcaaccgaaccaagtgaaggatctgcccctgggaccagcactgaaccatctgagccaaaaaagaagagaaaggtaatggacaagaagtacagcatcggcctggccatcggcaccaactctgtgggctgggccgtgatcaccgacgagtacaaggtgcccagcaagaaattcaaggtgctgggcaacaccgaccggcacagcatcaagaagaacctgatcggcgccctgctgttcgacagcggagaaacagccgaggccacccggctgaagagaaccgccagaagaagatacaccagacggaagaaccggatctgctatctgcaagagatcttcagcaacgagatggccaaggtggacgacagcttcttccacagactggaagagtccttcctggtggaagaggataagaagcacgagcggcaccccatcttcggcaacatcgtggacgaggtggcctaccacgagaagtaccccaccatctaccacctgagaaagaaactggtggacagcaccgacaaggccgacctgcggctgatctatctggccctggcccacatgatcaagttccggggccacttcctgatcgagggcgacctgaaccccgacaacagcgacgtggacaagctgttcatccagctggtgcagacctacaaccagctgttcgaggaaaaccccatcaacgccagcggcgtggacgccaaggccatcctgtctgccagactgagcaagagcagacggctggaaaatctgatcgcccagctgcccggcgagaagaagaatggcctgttcggcaacctgattgccctgagcctgggcctgacccccaacttcaagagcaacttcgacctggccgaggatgccaaactgcagctgagcaaggacacctacgacgacgacctggacaacctgctggcccagatcggcgaccagtacgccgacctgtttctggccgccaagaacctgtccgacgccatcctgctgagcgacatcctgagagtgaacaccgagatcaccaaggcccccctgagcgcctctatgatcaagagatacgacgagcaccaccaggacctgaccctgctgaaagctctcgtgcggcagcagctgcctgagaagtacaaagagattttcttcgaccagagcaagaacggctacgccggctacatcgatggcggagccagccaggaagagttctacaagttcatcaagcccatcctggaaaagatggacggcaccgaggaactgctcgtgaagctgaacagagaggacctgctgcggaagcagcggaccttcgacaacggcagcatcccccaccagatccacctgggagagctgcacgccattctgcggcggcaggaagatttttacccattcctgaaggacaaccgggaaaagatcgagaagatcctgaccttccgcatcccctactacgtgggccctctggccaggggaaacagcagattcgcctggatgaccagaaagagcgaggaaaccatcaccccctggaacttcgaggaagtggtggacaagggcgccagcgcccagagcttcatcgagcggatgaccaacttcgataagaacctgcccaacgagaaggtgctgcccaagcacagcctgctgtacgagtacttcaccgtgtacaacgagctgaccaaagtgaaatacgtgaccgagggaatgagaaagcccgccttcctgagcggcgagcagaaaaaagccatcgtggacctgctgttcaagaccaaccggaaagtgaccgtgaagcagctgaaagaggactacttcaagaaaatcgagtgcttcgactccgtggaaatctccggcgtggaagatcggttcaacgcctccctgggcacataccacgatctgctgaaaattatcaaggacaaggacttcctggacaatgaggaaaacgaggacattctggaagatatcgtgctgaccctgacactgtttgaggacagagagatgatcgaggaacggctgaaaacctatgcccacctgttcgacgacaaagtgatgaagcagctgaagcggcggagatacaccggctggggcaggctgagccggaagctgatcaacggcatccgggacaagcagtccggcaagacaatcctggatttcctgaagtccgacggcttcgccaacagaaacttcatgcagctgatccacgacgacagcctgacctttaaagaggacatccagaaagcccaggtgtccggccagggcgatagcctgcacgagcacattgccaatctggccggcagccccgccattaagaagggcatcctgcagacagtgaaggtggtggacgagctcgtgaaagtgatgggccggcacaagcccgagaacatcgtgatcgaaatggccagagagaaccagaccacccagaagggacagaagaacagccgcgagagaatgaagcggatcgaagagggcatcaaagagctgggcagccagatcctgaaagaacaccccgtggaaaacacccagctgcagaacgagaagctgtacctgtactacctgcagaatgggcgggatatgtacgtggaccaggaactggacatcaaccggctgtccgactacgatgtggacgctatcgtgcctcagagctttctgaaggacgactccatcgataacaaagtgctgactcggagcgacaagaaccggggcaagagcgacaacgtgccctccgaagaggtcgtgaagaagatgaagaactactggcgccagctgctgaatgccaagctgattacccagaggaagttcgacaatctgaccaaggccgagagaggcggcctgagcgaactggataaggccggcttcatcaagagacagctggtggaaacccggcagatcacaaagcacgtggcacagatcctggactcccggatgaacactaagtacgacgagaacgacaaactgatccgggaagtgaaagtgatcaccctgaagtccaagctggtgtccgatttccggaaggatttccagttttacaaagtgcgcgagatcaacaactaccaccacgcccacgacgcctacctgaacgccgtcgtgggaaccgccctgatcaaaaagtaccctaagctggaaagcgagttcgtgtacggcgactacaaggtgtacgacgtgcggaagatgatcgccaagagcgagcaggaaatcggcaaggctaccgccaagtacttcttctacagcaacatcatgaactttttcaagaccgagattaccctggccaacggcgagatccggaagcggcctctgatcgagacaaacggcgaaacaggcgagatcgtgtgggataagggccgggactttgccaccgtgcggaaagtgctgtctatgccccaagtgaatatcgtgaaaaagaccgaggtgcagacaggcggcttcagcaaagagtctatcctgcccaagaggaacagcgacaagctgatcgccagaaagaaggactgggaccctaagaagtacggcggcttcgacagccccaccgtggcctattctgtgctggtggtggccaaagtggaaaagggcaagtccaagaaactgaagagtgtgaaagagctgctggggatcaccatcatggaaagaagcagcttcgagaagaatcccatcgactttctggaagccaagggctacaaagaagtgaaaaaggacctgatcatcaagctgcctaagtactccctgttcgagctggaaaacggccggaagagaatgctggcctctgccggcgaactgcagaagggaaacgaactggccctgccctccaaatatgtgaacttcctgtacctggccagccactatgagaagctgaagggctcccccgaggataatgagcagaaacagctgtttgtggaacagcacaaacactacctggacgagatcatcgagcagatcagcgagttctccaagagagtgatcctggccgacgctaatctggacaaggtgctgagcgcctacaacaagcacagagacaagcctatcagagagcaggccgagaatatcatccacctgtttaccctgaccaatctgggagcccctgccgccttcaagtactttgacaccaccatcgaccggaagaggtacaccagcaccaaagaggtgctggacgccaccctgatccaccagagcatcaccggcctgtacgagacacggatcgacctgtctcagctgggaggcgacgcctatccctatgacgtgcccgattatgccagcctgggcagcggctcccccaagaaaaaacgcaaggtggaagatcctaagaaaaagcggaaagtggacggcagcggcagcgagacccccggtaccagcgagagcgccacccccgagagcggtagtgggagcaacggcagcagcggatccatgcgtgaccacatggtccttcatgagtatgtaaatgctgctgggattacagcggccgcaaggtcaggctccggccagcggggaagcaagcgcaccgccgatggttccgagttcgaaagccccaaaaaaaagcgcaaggtctga

SEQ ID NO: 327 - DNA, 7353 bp, synthetic construct
  misc_feature 1..7353: note = CDS of V39_GFP1-10-ZIM3-2a-D3a-hD3L-dCas9-1xGFP11
  source 1..7353: mol_type = other DNA
atgtccaagggagaggagctgttcaccggagtggtgccaatcctggtggagctggacggcgatgtgaacggccacaagttttctgtgcgcggagagggagagggcgacgcaaccatcggcaagctgacactgaagttcatctgcaccacaggcaagctgcccgtgccttggccaaccctggtgaccacactgacatacggcgtgcagtgtttctctaggtatccagaccacatgaagagacacgatttctttaagagcgccatgccagagggatacgtgcaggagcggaccatctccttcaaggacgatggcaagtataagacccgcgccgtggtgaagtttgagggcgatacactggtgaacaggatcgagctgaagggcaccgacttcaaggaggatggcaatatcctgggccacaagctggagtacaactttaatagccacaacgtgtatatcacagccgacaagcagaagaacggcatcaaggccaacttcaccgtgaggcacaatgtggaggacggctccgtgcagctggccgatcactaccagcagaacacacctatcggcgacggacccgtgctgctgcctgataatcactatctgtccacccagacagtgctgtctaaggacccaaacgagaagttggatccaggtggaggtggaagcggtatgaacaattcccagggaagagtgaccttcgaggacgtgaccgtgaacttcacccaaggcgagtggcagagactgaaccccgagcagagaaacctgtaccgggacgtgatgctggaaaactacagcaacctggtgtccgtcggccagggcgagacaacaaagcctgacgtgatcctgcggctggaacagggcaaagagccttggctggaagaggaagaggtgctcggatctggcagagccgagaagaatggcgatatcggcggacagatctggaagccaaaggatgtgaaagagagtctcggaagcggagctactaacttcagcctgctgaagcaggctggagacgtggaggagaaccctggacctatgcctgctgctaagagagtgaaactggatggatccaaccatgaccaggaatttgaccccccaaaggtttacccacctgtgccagctgagaagaggaagcccatccgcgtgctgtctctctttgatgggattgctacagggctcctggtgctgaaggacctgggcatccaagtggaccgctacattgcctccgaggtgtgtgaggactccatcacggtgggcatggtgcggcaccagggaaagatcatgtacgtcggggacgtccgcagcgtcacacagaagcatatccaggagtggggcccattcgacctggtgattggaggcagtccctgcaatgacctctccattgtcaaccctgcccgcaagggactttatgagggtactggccgcctcttctttgagttctaccgcctcctgcatgatgcgcggcccaaggagggagatgatcgccccttcttctggctctttgagaatgtggtggccatgggcgttagtgacaagagggacatctcgcgatttcttgagtctaaccccgtgatgattgacgccaaagaagtgtctgctgcacacagggcccgttacttctggggtaaccttcctggcatgaacaggcctttggcatccactgtgaatgataagctggagctgcaagagtgtctggagcacggcagaatagccaagttcagcaaagtgaggaccattaccaccaggtcaaactctataaagcagggcaaagaccagcatttccccgtgttcatgaacgagaaggaggacatcctgtggtgcactgaaatggaaagggtgtttggcttccccgtccactacacagacgtctccaacatgagccgcttggcgaggcagagactgctgggccgatcgtggagcgtgccggtcatccgccacctcttcgctccgctgaaggaatattttgcttgtgtgtctagcggcaatagtaacgctaacagccgcgggccgagcttcagcagcggcctggtgccgttaagcttgcgcggcagccatatgttcgaaaccgtgcctgtgtggaggagacagccagtccgggtgctgtccctttttgaagacatcaagaaagagctgacgagtttgggctttttggaaagtggttctgacccgggacaactgaagcatgtggttgatgtcacagacacagtgaggaaggatgtggaggagtggggacccttcgatcttgtgtacggcgccacacctcccctgggccacacctgtgaccgtcctcccagctggtacctgttccagttccaccggctcctgcagtacgcacggcccaagccaggcagccccaggcccttcttctggatgttcgtggacaatctggtgctgaacaaggaagacctggacgtcgcatctcgcttcctggagatggagccagtcaccatcccagatgtccacggcggatccttgcagaatgctgtccgcgtgtggagcaacatcccagccataaggagcagcaggcactgggctctggtttcggaagaagaattgtccctgctggcccagaacaagcagagctcgaagctcgcggccaagtggcccaccaagctggtgaagaactgctttctccccctaagagaatatttcaagtatttttcaggagggccgagctctggcgcacccccaccaagtggagggtctcctgccgggtccccaacatctactgaagaaggcaccagcgaatccgcaacgcccgagtcaggccctggtacctccacagaaccatctgaaggtagtgcgcctggttccccagctggaagccctacttccaccgaagaaggcacgtcaaccgaaccaagtgaaggatctgcccctgggaccagcactgaaccatctgagccaaaaaagaagagaaaggtaatggacaagaagtacagcatcggcctggccatcggcaccaactctgtgggctgggccgtgatcaccgacgagtacaaggtgcccagcaagaaattcaaggtgctgggcaacaccgaccggcacagcatcaagaagaacctgatcggcgccctgctgttcgacagcggagaaacagccgaggccacccggctgaagagaaccgccagaagaagatacaccagacggaagaaccggatctgctatctgcaagagatcttcagcaacgagatggccaaggtggacgacagcttcttccacagactggaagagtccttcctggtggaagaggataagaagcacgagcggcaccccatcttcggcaacatcgtggacgaggtggcctaccacgagaagtaccccaccatctaccacctgagaaagaaactggtggacagcaccgacaaggccgacctgcggctgatctatctggccctggcccacatgatcaagttccggggccacttcctgatcgagggcgacctgaaccccgacaacagcgacgtggacaagctgttcatccagctggtgcagacctacaaccagctgttcgaggaaaaccccatcaacgccagcggcgtggacgccaaggccatcctgtctgccagactgagcaagagcagacggctggaaaatctgatcgcccagctgcccggcgagaagaagaatggcctgttcggcaacctgattgccctgagcctgggcctgacccccaacttcaagagcaacttcgacctggccgaggatgccaaactgcagctgagcaaggacacctacgacgacgacctggacaacctgctggcccagatcggcgaccagtacgccgacctgtttctggccgccaagaacctgtccgacgccatcctgctgagcgacatcctgagagtgaacaccgagatcaccaaggcccccctgagcgcctctatgatcaagagatacgacgagcaccaccaggacctgaccctgctgaaagctctcgtgcggcagcagctgcctgagaagtacaaagagattttcttcgaccagagcaagaacggctacgccggctacatcgatggcggagccagccaggaagagttctacaagttcatcaagcccatcctggaaaagatggacggcaccgaggaactgctcgtgaagctgaacagagaggacctgctgcggaagcagcggaccttcgacaacggcagcatcccccaccagatccacctgggagagctgcacgccattctgcggcggcaggaagatttttacccattcctgaaggacaaccgggaaaagatcgagaagatcctgaccttccgcatcccctactacgtgggccctctggccaggggaaacagcagattcgcctggatgaccagaaagagcgaggaaaccatcaccccctggaacttcgaggaagtggtggacaagggcgccagcgcccagagcttcatcgagcggatgaccaacttcgataagaacctgcccaacgagaaggtgctgcccaagcacagcctgctgtacgagtacttcaccgtgtacaacgagctgaccaaagtgaaatacgtgaccgagggaatgagaaagcccgccttcctgagcggcgagcagaaaaaagccatcgtggacctgctgttcaagaccaaccggaaagtgaccgtgaagcagctgaaagaggactacttcaagaaaatcgagtgcttcgactccgtggaaatctccggcgtggaagatcggttcaacgcctccctgggcacataccacgatctgctgaaaattatcaaggacaaggacttcctggacaatgaggaaaacgaggacattctggaagatatcgtgctgaccctgacactgtttgaggacagagagatgatcgaggaacggctgaaaacctatgcccacctgttcgacgacaaagtgatgaagcagctgaagcggcggagatacaccggctggggcaggctgagccggaagctgatcaacggcatccgggacaagcagtccggcaagacaatcctggatttcctgaagtccgacggcttcgccaacagaaacttcatgcagctgatccacgacgacagcctgacctttaaagaggacatccagaaagcccaggtgtccggccagggcgatagcctgcacgagcacattgccaatctggccggcagccccgccattaagaagggcatcctgcagacagtgaaggtggtggacgagctcgtgaaagtgatgggccggcacaagcccgagaacatcgtgatcgaaatggccagagagaaccagaccacccagaagggacagaagaacagccgcgagagaatgaagcggatcgaagagggcatcaaagagctgggcagccagatcctgaaagaacaccccgtggaaaacacccagctgcagaacgagaagctgtacctgtactacctgcagaatgggcgggatatgtacgtggaccaggaactggacatcaaccggctgtccgactacgatgtggacgctatcgtgcctcagagctttctgaaggacgactccatcgataacaaagtgctgactcggagcgacaagaaccggggcaagagcgacaacgtgccctccgaagaggtcgtgaagaagatgaagaactactggcgccagctgctgaatgccaagctgattacccagaggaagttcgacaatctgaccaaggccgagagaggcggcctgagcgaactggataaggccggcttcatcaagagacagctggtggaaacccggcagatcacaaagcacgtggcacagatcctggactcccggatgaacactaagtacgacgagaacgacaaactgatccgggaagtgaaagtgatcaccctgaagtccaagctggtgtccgatttccggaaggatttccagttttacaaagtgcgcgagatcaacaactaccaccacgcccacgacgcctacctgaacgccgtcgtgggaaccgccctgatcaaaaagtaccctaagctggaaagcgagttcgtgtacggcgactacaaggtgtacgacgtgcggaagatgatcgccaagagcgagcaggaaatcggcaaggctaccgccaagtacttcttctacagcaacatcatgaactttttcaagaccgagattaccctggccaacggcgagatccggaagcggcctctgatcgagacaaacggcgaaacaggcgagatcgtgtgggataagggccgggactttgccaccgtgcggaaagtgctgtctatgccccaagtgaatatcgtgaaaaagaccgaggtgcagacaggcggcttcagcaaagagtctatcctgcccaagaggaacagcgacaagctgatcgccagaaagaaggactgggaccctaagaagtacggcggcttcgacagccccaccgtggcctattctgtgctggtggtggccaaagtggaaaagggcaagtccaagaaactgaagagtgtgaaagagctgctggggatcaccatcatggaaagaagcagcttcgagaagaatcccatcgactttctggaagccaagggctacaaagaagtgaaaaaggacctgatcatcaagctgcctaagtactccctgttcgagctggaaaacggccggaagagaatgctggcctctgccggcgaactgcagaagggaaacgaactggccctgccctccaaatatgtgaacttcctgtacctggccagccactatgagaagctgaagggctcccccgaggataatgagcagaaacagctgtttgtggaacagcacaaacactacctggacgagatcatcgagcagatcagcgagttctccaagagagtgatcctggccgacgctaatctggacaaggtgctgagcgcctacaacaagcacagagacaagcctatcagagagcaggccgagaatatcatccacctgtttaccctgaccaatctgggagcccctgccgccttcaagtactttgacaccaccatcgaccggaagaggtacaccagcaccaaagaggtgctggacgccaccctgatccaccagagcatcaccggcctgtacgagacacggatcgacctgtctcagctgggaggcgacgcctatccctatgacgtgcccgattatgccagcctgggcagcggctcccccaagaaaaaacgcaaggtggaagatcctaagaaaaagcggaaagtggacggcagcggcagcgagacccccggtaccagcgagagcgccacccccgagagcggtagtgggagcaacggcagcagcggatccatgcgtgaccacatggtccttcatgagtatgtaaatgctgctgggattacagcggccgcaaggtcaggctccggccagcggggaagcaagcgcaccgccgatggttccgagttcgaaagccccaaaaaaaagcgcaaggtctga

SEQ ID NO: 328 - DNA, 8499 bp, synthetic construct
  misc_feature 1..8499: note = CDS of V40_GFP1-10-HDAC1-2a-D3a-hD3L-dCas9-1xGFP11
  source 1..8499: mol_type = other DNA
atgtccaagggagaggagctgttcaccggagtggtgccaatcctggtggagctggacggcgatgtgaacggccacaagttttctgtgcgcggagagggagagggcgacgcaaccatcggcaagctgacactgaagttcatctgcaccacaggcaagctgcccgtgccttggccaaccctggtgaccacactgacatacggcgtgcagtgtttctctaggtatccagaccacatgaagagacacgatttctttaagagcgccatgccagagggatacgtgcaggagcggaccatctccttcaaggacgatggcaagtataagacccgcgccgtggtgaagtttgagggcgatacactggtgaacaggatcgagctgaagggcaccgacttcaaggaggatggcaatatcctgggccacaagctggagtacaactttaatagccacaacgtgtatatcacagccgacaagcagaagaacggcatcaaggccaacttcaccgtgaggcacaatgtggaggacggctccgtgcagctggccgatcactaccagcagaacacacctatcggcgacggacccgtgctgctgcctgataatcactatctgtccacccagacagtgctgtctaaggacccaaacgagaagttggatccaggtggaggtggaagcggtatggcgcagacgcagggcacccggaggaaagtctgttactactacgacggggatgttggaaattactattatggacaaggccacccaatgaagcctcaccgaatccgcatgactcataatttgctgctcaactatggtctctaccgaaaaatggaaatctatcgccctcacaaagccaatgctgaggagatgaccaagtaccacagcgatgactacattaaattcttgcgctccatccgtccagataacatgtcggagtacagcaagcagatgcagagattcaacgttggtgaggactgtccagtattcgatggcctgtttgagttctgtcagttgtctactggtggttctgtggcaagtgctgtgaaacttaataagcagcagacggacatcgctgtgaattgggctgggggcctgcaccatgcaaagaagtccgaggcatctggcttctgttacgtcaatgatatcgtcttggccatcctggaactgctaaagtatcaccagagggtgctgtacattgacattgatattcaccatggtgacggcgtggaagaggccttctacaccacggaccgggtcatgactgtgtcctttcataagtatggagagtacttcccaggaactggggacctacgggatatcggggctggcaaaggcaagtattatgctgttaactacccgctccgagacgggattgatgacgagtcctatgaggccattttcaagccggtcatgtccaaagtaatggagatgttccagcctagtgcggtggtcttacagtgtggctcagactccctatctggggatcggttaggttgcttcaatctaactatcaaaggacacgccaagtgtgtggaatttgtcaagagctttaacctgcctatgctgatgctgggaggcggtggttacaccattcgtaacgttgcccggtgctggacatatgagacagctgtggccctggatacggagatccctaatgagcttccatacaatgactactttgaatactttggaccagatttcaagctccacatcagtccttccaatatgactaaccagaacacgaatgagtacctggagaagatcaaacagcgactgtttgagaaccttagaatgctgccgcacgcacctggggtccaaatgcaggcgattcctgaggacgccatccctgaggagagtggcgatgaggacgaagacgaccctgacaagcgcatctcgatctgctcctctgacaaacgaattgcctgtgaggaagagttctccgattctgaagaggagggagaggggggccgcaagaactcttccaacttcaaaaaagccaagagagtcaaaacagaggatgaaaaagagaaagacccagaggagaagaaagaagtcaccgaagaggagaaaaccaaggaggagaagccagaagccaaaggggtcaaggaggaggtcaagttggccggaagcggagctactaacttcagcctgctgaagcaggctggagacgtggaggagaaccctggacctatgcctgctgctaagagagtgaaactggatggatccaaccatgaccaggaatttgaccccccaaaggtttacccacctgtgccagctgagaagaggaagcccatccgcgtgctgtctctctttgatgggattgctacagggctcctggtgctgaaggacctgggcatccaagtggaccgctacattgcctccgaggtgtgtgaggactccatcacggtgggcatggtgcggcaccagggaaagatcatgtacgtcggggacgtccgcagcgtcacacagaagcatatccaggagtggggcccattcgacctggtgattggaggcagtccctgcaatgacctctccattgtcaaccctgcccgcaagggactttatgagggtactggccgcctcttctttgagttctaccgcctcctgcatgatgcgcggcccaaggagggagatgatcgccccttcttctggctctttgagaatgtggtggccatgggcgttagtgacaagagggacatctcgcgatttcttgagtctaaccccgtgatgattgacgccaaagaagtgtctgctgcacacagggcccgttacttctggggtaaccttcctggcatgaacaggcctttggcatccactgtgaatgataagctggagctgcaagagtgtctggagcacggcagaatagccaagttcagcaaagtgaggaccattaccaccaggtcaaactctataaagcagggcaaagaccagcatttccccgtgttcatgaacgagaaggaggacatcctgtggtgcactgaaatggaaagggtgtttggcttccccgtccactacacagacgtctccaacatgagccgcttggcgaggcagagactgctgggccgatcgtggagcgtgccggtcatccgccacctcttcgctccgctgaaggaatattttgcttgtgtgtctagcggcaatagtaacgctaacagccgcgggccgagcttcagcagcggcctggtgccgttaagcttgcgcggcagccatatgttcgaaaccgtgcctgtgtggaggagacagccagtccgggtgctgtccctttttgaagacatcaagaaagagctgacgagtttgggctttttggaaagtggttctgacccgggacaactgaagcatgtggttgatgtcacagacacagtgaggaaggatgtggaggagtggggacccttcgatcttgtgtacggcgccacacctcccctgggccacacctgtgaccgtcctcccagctggtacctgttccagttccaccggctcctgcagtacgcacggcccaagccaggcagccccaggcccttcttctggatgttcgtggacaatctggtgctgaacaaggaagacctggacgtcgcatctcgcttcctggagatggagccagtcaccatcccagatgtccacggcggatccttgcagaatgctgtccgcgtgtggagcaacatcccagccataaggagcagcaggcactgggctctggtttcggaagaagaattgtccctgctggcccagaacaagcagagctcgaagctcgcggccaagtggcccaccaagctggtgaagaactgctttctccccctaagagaatatttcaagtatttttcaggagggccgagctctggcgcacccccaccaagtggagggtctcctgccgggtccccaacatctactgaagaaggcaccagcgaatccgcaacgcccgagtcaggccctggtacctccacagaaccatctgaaggtagtgcgcctggttccccagctggaagccctacttccaccgaagaaggcacgtcaaccgaaccaagtgaaggatctgcccctgggaccagcactgaaccatctgagccaaaaaagaagagaaaggtaatggacaagaagtacagcatcggcctggccatcggcaccaactctgtgggctgggccgtgatcaccgacgagtacaaggtgcccagcaagaaattcaaggtgctgggcaacaccgaccggcacagcatcaagaagaacctgatcggcgccctgctgttcgacagcggagaaacagccgaggccacccggctgaagagaaccgccagaagaagatacaccagacggaagaaccggatctgctatctgcaagagatcttcagcaacgagatggccaaggtggacgacagcttcttccacagactggaagagtccttcctggtggaagaggataagaagcacgagcggcaccccatcttcggcaacatcgtggacgaggtggcctaccacgagaagtaccccaccatctaccacctgagaaagaaactggtggacagcaccgacaaggccgacctgcggctgatctatctggccctggcccacatgatcaagttccggggccacttcctgatcgagggcgacctgaaccccgacaacagcgacgtggacaagctgttcatccagctggtgcagacctacaaccagctgttcgaggaaaaccccatcaacgccagcggcgtggacgccaaggccatcctgtctgccagactgagcaagagcagacggctggaaaatctgatcgcccagctgcccggcgagaagaagaatggcctgttcggcaacctgattgccctgagcctgggcctgacccccaacttcaagagcaacttcgacctggccgaggatgccaaactgcagctgagcaaggacacctacgacgacgacctggacaacctgctggcccagatcggcgaccagtacgccgacctgtttctggccgccaagaacctgtccgacgccatcctgctgagcgacatcctgagagtgaacaccgagatcaccaaggcccccctgagcgcctctatgatcaagagatacgacgagcaccaccaggacctgaccctgctgaaagctctcgtgcggcagcagctgcctgagaagtacaaagagattttcttcgaccagagcaagaacggctacgccggctacatcgatggcggagccagccaggaagagttctacaagttcatcaagcccatcctggaaaagatggacggcaccgaggaactgctcgtgaagctgaacagagaggacctgctgcggaagcagcggaccttcgacaacggcagcatcccccaccagatccacctgggagagctgcacgccattctgcggcggcaggaagatttttacccattcctgaaggacaaccgggaaaagatcgagaagatcctgaccttccgcatcccctactacgtgggccctctggccaggggaaacagcagattcgcctggatgaccagaaagagcgaggaaaccatcaccccctggaacttcgaggaagtggtggacaagggcgccagcgcccagagcttcatcgagcggatgaccaacttcgataagaacctgcccaacgagaaggtgctgcccaagcacagcctgctgtacgagtacttcaccgtgtacaacgagctgaccaaagtgaaatacgtgaccgagggaatgagaaagcccgccttcctgagcggcgagcagaaaaaagccatcgtggacctgctgttcaagaccaaccggaaagtgaccgtgaagcagctgaaagaggactacttcaagaaaatcgagtgcttcgactccgtggaaatctccggcgtggaagatcggttcaacgcctccctgggcacataccacgatctgctgaaaattatcaaggacaaggacttcctggacaatgaggaaaacgaggacattctggaagatatcgtgctgaccctgacactgtttgaggacagagagatgatcgaggaacggctgaaaacctatgcccacctgttcgacgacaaagtgatgaagcagctgaagcggcggagatacaccggctggggcaggctgagccggaagctgatcaacggcatccgggacaagcagtccggcaagacaatcctggatttcctgaagtccgacggcttcgccaacagaaacttcatgcagctgatccacgacgacagcctgacctttaaagaggacatccagaaagcccaggtgtccggccagggcgatagcctgcacgagcacattgccaatctggccggcagccccgccattaagaagggcatcctgcagacagtgaaggtggtggacgagctcgtgaaagtgatgggccggcacaagcccgagaacatcgtgatcgaaatggccagagagaaccagaccacccagaagggacagaagaacagccgcgagagaatgaagcggatcgaagagggcatcaaagagctgggcagccagatcctgaaagaacaccccgtggaaaacacccagctgcagaacgagaagctgtacctgtactacctgcagaatgggcgggatatgtacgtggaccaggaactggacatcaaccggctgtccgactacgatgtggacgctatcgtgcctcagagctttctgaaggacgactccatcgataacaaagtgctgactcggagcgacaagaaccggggcaagagcgacaacgtgccctccgaagaggtcgtgaagaagatgaagaactactggcgccagctgctgaatgccaagctgattacccagaggaagttcgacaatctgaccaaggccgagagaggcggcctgagcgaactggataaggccggcttcatcaagagacagctggtggaaacccggcagatcacaaagcacgtggcacagatcctggactcccggatgaacactaagtacgacgagaacgacaaactgatccgggaagtgaaagtgatcaccctgaagtccaagctggtgtccgatttccggaaggatttccagttttacaaagtgcgcgagatcaacaactaccaccacgcccacgacgcctacctgaacgccgtcgtgggaaccgccctgatcaaaaagtaccctaagctggaaagcgagttcgtgtacggcgactacaaggtgtacgacgtgcggaagatgatcgccaagagcgagcaggaaatcggcaaggctaccgccaagtacttcttctacagcaacatcatgaactttttcaagaccgagattaccctggccaacggcgagatccggaagcggcctctgatcgagacaaacggcgaaacaggcgagatcgtgtgggataagggccgggactttgccaccgtgcggaaagtgctgtctatgccccaagtgaatatcgtgaaaaagaccgaggtgcagacaggcggcttcagcaaagagtctatcctgcccaagaggaacagcgacaagctgatcgccagaaagaaggactgggaccctaagaagtacggcggcttcgacagccccaccgtggcctattctgtgctggtggtggccaaagtggaaaagggcaagtccaagaaactgaagagtgtgaaagagctgctggggatcaccatcatggaaagaagcagcttcgagaagaatcccatcgactttctggaagccaagggctacaaagaagtgaaaaaggacctgatcatcaagctgcctaagtactccctgttcgagctggaaaacggccggaagagaatgctggcctctgccggcgaactgcagaagggaaacgaactggccctgccctccaaatatgtgaacttcctgtacctggccagccactatgagaagctgaagggctcccccgaggataatgagcagaaacagctgtttgtggaacagcacaaacactacctggacgagatcatcgagcagatcagcgagttctccaagagagtgatcctggccgacgctaatctggacaaggtgctgagcgcctacaacaagcacagagacaagcctatcagagagcaggccgagaatatcatccacctgtttaccctgaccaatctgggagcccctgccgccttcaagtactttgacaccaccatcgaccggaagaggtacaccagcaccaaagaggtgctggacgccaccctgatccaccagagcatcaccggcctgtacgagacacggatcgacctgtctcagctgggaggcgacgcctatccctatgacgtgcccgattatgccagcctgggcagcggctcccccaagaaaaaacgcaaggtggaagatcctaagaaaaagcggaaagtggacggcagcggcagcgagacccccggtaccagcgagagcgccacccccgagagcggtagtgggagcaacggcagcagcggatccatgcgtgaccacatggtccttcatgagtatgtaaatgctgctgggattacagcggccgcaaggtcaggctccggccagcggggaagcaagcgcaccgccgatggttccgagttcgaaagccccaaaaaaaagcgcaaggtctga

SEQ ID NO: 329 - DNA, 6933 bp, synthetic construct
  misc_feature 1..6933: note = CDS of V41_GFP1-10-ZIM3-2a-D3a-hD3L-dCas12a-1xGFP11
  source 1..6933: mol_type = other DNA
atgtccaagggagaggagctgttcaccggagtggtgccaatcctggtggagctggacggcgatgtgaacggccacaagttttctgtgcgcggagagggagagggcgacgcaaccatcggcaagctgacactgaagttcatctgcaccacaggcaagctgcccgtgccttggccaaccctggtgaccacactgacatacggcgtgcagtgtttctctaggtatccagaccacatgaagagacacgatttctttaagagcgccatgccagagggatacgtgcaggagcggaccatctccttcaaggacgatggcaagtataagacccgcgccgtggtgaagtttgagggcgatacactggtgaacaggatcgagctgaagggcaccgacttcaaggaggatggcaatatcctgggccacaagctggagtacaactttaatagccacaacgtgtatatcacagccgacaagcagaagaacggcatcaaggccaacttcaccgtgaggcacaatgtggaggacggctccgtgcagctggccgatcactaccagcagaacacacctatcggcgacggacccgtgctgctgcctgataatcactatctgtccacccagacagtgctgtctaaggacccaaacgagaagttggatccaggtggaggtggaagcggtatgaacaattcccagggaagagtgaccttcgaggacgtgaccgtgaacttcacccaaggcgagtggcagagactgaaccccgagcagagaaacctgtaccgggacgtgatgctggaaaactacagcaacctggtgtccgtcggccagggcgagacaacaaagcctgacgtgatcctgcggctggaacagggcaaagagccttggctggaagaggaagaggtgctcggatctggcagagccgagaagaatggcgatatcggcggacagatctggaagccaaaggatgtgaaagagagtctcggaagcggagctactaacttcagcctgctgaagcaggctggagacgtggaggagaaccctggacctatgcctgctgctaagagagtgaaactggatggatccaaccatgaccaggaatttgaccccccaaaggtttacccacctgtgccagctgagaagaggaagcccatccgcgtgctgtctctctttgatgggattgctacagggctcctggtgctgaaggacctgggcatccaagtggaccgctacattgcctccgaggtgtgtgaggactccatcacggtgggcatggtgcggcaccagggaaagatcatgtacgtcggggacgtccgcagcgtcacacagaagcatatccaggagtggggcccattcgacctggtgattggaggcagtccctgcaatgacctctccattgtcaaccctgcccgcaagggactttatgagggtactggccgcctcttctttgagttctaccgcctcctgcatgatgcgcggcccaaggagggagatgatcgccccttcttctggctctttgagaatgtggtggccatgggcgttagtgacaagagggacatctcgcgatttcttgagtctaaccccgtgatgattgacgccaaagaagtgtctgctgcacacagggcccgttacttctggggtaaccttcctggcatgaacaggcctttggcatccactgtgaatgataagctggagctgcaagagtgtctggagcacggcagaatagccaagttcagcaaagtgaggaccattaccaccaggtcaaactctataaagcagggcaaagaccagcatttccccgtgttcatgaacgagaaggaggacatcctgtggtgcactgaaatggaaagggtgtttggcttccccgtccactacacagacgtctccaacatgagccgcttggcgaggcagagactgctgggccgatcgtggagcgtgccggtcatccgccacctcttcgctccgctgaaggaatattttgcttgtgtgtctagcggcaatagtaacgctaacagccgcgggccgagcttcagcagcggcctggtgccgttaagcttgcgcggcagccatatgttcgaaaccgtgcctgtgtggaggagacagccagtccgggtgctgtccctttttgaagacatcaagaaagagctgacgagtttgggctttttggaaagtggttctgacccgggacaactgaagcatgtggttgatgtcacagacacagtgaggaaggatgtggaggagtggggacccttcgatcttgtgtacggcgccacacctcccctgggccacacctgtgaccgtcctcccagctggtacctgttccagttccaccggctcctgcagtacgcacggcccaagccaggcagccccaggcccttcttctggatgttcgtggacaatctggtgctgaacaaggaagacctggacgtcgcatctcgcttcctggagatggagccagtcaccatcccagatgtccacggcggatccttgcagaatgctgtccgcgtgtggagcaacatcccagccataaggagcagcaggcactgggctctggtttcggaagaagaattgtccctgctggcccagaacaagcagagctcgaagctcgcggccaagtggcccaccaagctggtgaagaactgctttctccccctaagagaatatttcaagtatttttcaggagggccgagctctggcgcacccccaccaagtggagggtctcctgccgggtccccaacatctactgaagaaggcaccagcgaatccgcaacgcccgagtcaggccctggtacctccacagaaccatctgaaggtagtgcgcctggttccccagctggaagccctacttccaccgaagaaggcacgtcaaccgaaccaagtgaaggatctgcccctgggaccagcactgaaccatctgagccaaaaaagaagagaaaggtaatgtcaaagctggagaaattcaccaactgttatagcctgtctaagaccctgcgcttcaaggcaatcccagtgggcaagacacaagagaacattgacaacaaacggctcctggtggaggatgagaagagggctgaagattacaagggcgttaagaagctgctggataggtactatctgtcattcatcaacgatgtcctccacagtatcaagctgaagaatctgaacaattacatttctctgttccggaagaagacacggaccgagaaggagaacaaagagctggagaatctggagatcaacctgaggaaagaaatagctaaggctttcaaagggaacgagggttacaagtccctgttcaagaaagacattatcgagactattctgcctgagttcctggacgataaagatgagatcgccctcgtcaattccttcaatgggtttaccacagcctttaccggcttcttcgacaatagagagaatatgttctctgaagaggccaaatccactagcatcgcctttcgctgcataaacgagaacctgactaggtacatcagcaatatggacatctttgagaaagtcgatgccatattcgacaaacatgaggtgcaggagattaaggagaagatcctgaactcagattacgatgtcgaagatttcttcgagggagagttcttcaacttcgtgctcacacaagagggcattgatgtgtacaatgcaatcattggagggttcgtgacagagagtggcgagaagataaagggcctgaacgagtatatcaacctctacaaccagaaaaccaagcagaaactgcctaagttcaagccactgtacaaacaagtgctctcagatagggaaagcctgagcttctacggtgaagggtatacatcagatgaagaagtgctcgaagtgttccgcaacaccctcaataagaacagtgaaatcttctcttcaatcaagaagctggagaaactgttcaagaatttcgatgagtactcctctgccggaatctttgtgaagaatggccctgcaatatccactattagcaaagacatctttggcgagtggaacgttatcagggataagtggaatgccgagtacgatgatattcatctcaagaagaaagccgtggttacagagaaatacgaggatgatagacgcaagagctttaagaagattggtagcttctctctcgaacagctgcaggagtacgccgacgctgacctgtcagtcgtggagaaactcaaggagatcataatccagaaggtggatgaaatctacaaagtgtatggaagctctgagaaactcttcgatgcagactttgttctggagaagagtctgaagaagaacgacgcagtggttgctatcatgaaggacctgctggattctgttaagtctttcgagaattacattaaggcattctttggtgaagggaaggagacaaatagggacgagagcttctatggcgactttgttctggcctacgacatcctcctcaaggttgaccacatctatgacgctatacggaattacgttacccagaagccctatagcaaagacaagttcaagctgtatttccagaatccacagtttatgggtgggtgggataaagacaaagaaacagattacagggccactatcctgcggtacggcagcaaatactatctggctatcatggataagaagtacgccaaatgcctccagaagatcgacaaggacgacgtgaacggtaactacgagaagatcaattacaagctcctgccaggacctaacaagatgctgcccaaggtgttcttctccaagaaatggatggcctactataacccaagcgaggacattcagaagatatacaagaatgggacattcaagaagggcgatatgttcaacctcaacgactgccacaagctgattgatttcttcaaggatagcatttctcgctatcccaagtggtctaatgcatacgatttcaacttcagcgagactgagaagtacaaagacatcgctggcttctaccgggaggtggaagagcaaggctataaggtgtcattcgaatccgcttctaagaaggaagtggataagctcgtggaagagggtaagctgtacatgttccagatatacaacaaagacttcagcgataagagccacggcactccaaacctccatactatgtatttcaagctgctgtttgacgagaacaaccacggacagattaggctgtcaggaggcgcagaactcttcatgcgcagagcttcactgaagaaggaggaactcgttgtccacccagccaatagccctatagccaataagaatccagacaatcctaagaaaaccactactctgtcttacgatgtgtataaggataagagattctctgaagatcagtacgaactgcacatacccattgccattaacaagtgccctaagaacatcttcaagattaacacagaggttagagtgctcctgaaacacgacgataacccttatgttataggcattgctcgcggagagagaaacctgctgtacatcgtcgtggtggacggcaaaggcaacatcgtggaacagtacagtctcaatgaaatcattaacaatttcaacggaatccgcattaagaccgactaccattctctcctcgacaagaaggagaaagaaaggttcgaagcaagacagaattggacaagtatagagaatatcaaagaactgaaggctgggtacatctctcaggttgtgcacaagatatgtgagctggtggagaagtacgacgctgttatcgccctcgcggacctgaatagcggcttcaagaactccagggtgaaggtggagaagcaggtgtatcagaagttcgagaagatgctgatcgacaagctcaactatatggtggacaagaaatccaatccttgcgctactggtggagccctgaagggctatcaaatcaccaataagttcgaatctttcaagtctatgagcacccagaatggcttcatcttctacatacccgcatggctgacatccaagattgatccctctaccggatttgttaatctgctcaagactaagtacacctctattgctgactcaaagaagttcatatcatcatttgaccgcatcatgtacgtgccagaagaggacctgttcgagtttgccctggattacaagaatttctctcggactgacgccgactacatcaagaagtggaagctctactcttatggtaatcggattcgcatattccgcaatcccaagaagaataacgtgttcgattgggaggaagtttgcctcaccagcgcttacaaggagctgttcaataagtatgggattaactaccagcagggcgacataagagccctgctgtgcgaacaatctgataaggcattctattcctctttcatggcactgatgtcactgatgctgcaaatgcgcaattccatcaccggaagaacagacgtggcctttctgatctctcctgtcaagaactcagatggcatcttctacgattcccgcaactatgaagcacaggagaatgctatcctgcctaagaatgccgatgcaaatggagcctataacatcgccagaaaggtcctctgggccataggacaattcaagaaagctgaagatgagaagctggacaaggtgaagatcgccatttcaaacaaagagtggctcgaatatgctcagacctcagtgaagcatgcctatccctatgacgtgcccgattatgccagcctgggcagcggctcccccaagaaaaaacgcaaggtggaagatcctaagaaaaagcggaaagtggacggcagcggcagcgagacccccggtaccagcgagagcgccacccccgagagcggtagtgggagcaacggcagcagcggatccatgcgtgaccacatggtccttcatgagtatgtaaatgctgctgggattacagcggccgcaaggtcaggctccggccagcggggaagcaagcgcaccgccgatggttccgagttcgaaagccccaaaaaaaagcgcaaggtctga

SEQ ID NO: 330 - DNA, 6282 bp, synthetic construct
  misc_feature 1..6282: note = CDS of V42_GFP1-10-ZIM3-2a-D3a-hD3L-dCas12i-1xGFP11
  source 1..6282: mol_type = other DNA
atgtccaagggagaggagctgttcaccggagtggtgccaatcctggtggagctggacggcgatgtgaacggccacaagttttctgtgcgcggagagggagagggcgacgcaaccatcggcaagctgacactgaagttcatctgcaccacaggcaagctgcccgtgccttggccaaccctggtgaccacactgacatacggcgtgcagtgtttctctaggtatccagaccacatgaagagacacgatttctttaagagcgccatgccagagggatacgtgcaggagcggaccatctccttcaaggacgatggcaagtataagacccgcgccgtggtgaagtttgagggcgatacactggtgaacaggatcgagctgaagggcaccgacttcaaggaggatggcaatatcctgggccacaagctggagtacaactttaatagccacaacgtgtatatcacagccgacaagcagaagaacggcatcaaggccaacttcaccgtgaggcacaatgtggaggacggctccgtgcagctggccgatcactaccagcagaacacacctatcggcgacggacccgtgctgctgcctgataatcactatctgtccacccagacagtgctgtctaaggacccaaacgagaagttggatccaggtggaggtggaagcggtatgaacaattcccagggaagagtgaccttcgaggacgtgaccgtgaacttcacccaaggcgagtggcagagactgaaccccgagcagagaaacctgtaccgggacgtgatgctggaaaactacagcaacctggtgtccgtcggccagggcgagacaacaaagcctgacgtgatcctgcggctggaacagggcaaagagccttggctggaagaggaagaggtgctcggatctggcagagccgagaagaatggcgatatcggcggacagatctggaagccaaaggatgtgaaagagagtctcggaagcggagctactaacttcagcctgctgaagcaggctggagacgtggaggagaaccctggacctatgcctgctgctaagagagtgaaactggatggatccaaccatgaccaggaatttgaccccccaaaggtttacccacctgtgccagctgagaagaggaagcccatccgcgtgctgtctctctttgatgggattgctacagggctcctggtgctgaaggacctgggcatccaagtggaccgctacattgcctccgaggtgtgtgaggactccatcacggtgggcatggtgcggcaccagggaaagatcatgtacgtcggggacgtccgcagcgtcacacagaagcatatccaggagtggggcccattcgacctggtgattggaggcagtccctgcaatgacctctccattgtcaaccctgcccgcaagggactttatgagggtactggccgcctcttctttgagttctaccgcctcctgcatgatgcgcggcccaaggagggagatgatcgccccttcttctggctctttgagaatgtggtggccatgggcgttagtgacaagagggacatctcgcgatttcttgagtctaaccccgtgatgattgacgccaaagaagtgtctgctgcacacagggcccgttacttctggggtaaccttcctggcatgaacaggcctttggcatccactgtgaatgataagctggagctgcaagagtgtctggagcacggcagaatagccaagttcagcaaagtgaggaccattaccaccaggtcaaactctataaagcagggcaaagaccagcatttccccgtgttcatgaacgagaaggaggacatcctgtggtgcactgaaatggaaagggtgtttggcttccccgtccactacacagacgtctccaacatgagccgcttggcgaggcagagactgctgggccgatcgtggagcgtgccggtcatccgccacctcttcgctccgctgaaggaatattttgcttgtgtgtctagcggcaatagtaacgctaacagccgcgggccgagcttcagcagcggcctggtgccgttaagcttgcgcggcagccatatgttcgaaaccgtgcctgtgtggaggagacagccagtccgggtgctgtccctttttgaagacatcaagaaagagctgacgagtttgggctttttggaaagtggttctgacccgggacaactgaagcatgtggttgatgtcacagacacagtgaggaaggatgtggaggagtggggacccttcgatcttgtgtacggcgccacacctcccctgggccacacctgtgaccgtcctcccagctggtacctgttccagttccaccggctcctgcagtacgcacggcccaagccaggcagccccaggcccttcttctggatgttcgtggacaatctggtgctgaacaaggaagacctggacgtcgcatctcgcttcctggagatggagccagtcaccatcccagatgtccacggcggatccttgcagaatgctgtccgcgtgtggagcaacatcccagccataaggagcagcaggcactgggctctggtttcggaagaagaattgtccctgctggcccagaacaagcagagctcgaagctcgcggccaagtggcccaccaagctggtgaagaactgctttctccccctaagagaatatttcaagtatttttcaggagggccgagctctggcgcacccccaccaagtggagggtctcctgccgggtccccaacatctactgaagaaggcaccagcgaatccgcaacgcccgagtcaggccctggtacctccacagaaccatctgaaggtagtgcgcctggttccccagctggaagccctacttccaccgaagaaggcacgtcaaccgaaccaagtgaaggatctgcccctgggaccagcactgaaccatctgagccaaaaaagaagagaaaggtaatgggcatcaccatgagcgacaccaccttcagaccctacaagagcaagctgaaccccaacgagcggaagatgcctatggtggtggacaccatgaattggtgcgacaacgcctgcagcgtgttcttcgatctgttcgtgggcctgtacggcggcgtgaagatcggcgacgtgaccaatttcctgaccgagaagcaggacaccaccaccgatgccgatctgctgtgcgccatcaactggttcagagccatgcctgtgtctaaccccgatgccgttgtgggacctgagcagctggttgtgcggttcagagactacagcggccacaatccatctccaatggccagcatgtacctgagcgcccctgtgaaccctagatacacctgggtcgactgccggttcctgtaccagcagatgtgtcagaccctgggcgccaacctggatgtggacatctctaccctggtgcagaccggcctgctgcctatccagaaggatacacagctgaacgcctacagcttctgcagcaacgtgttcggcgagggcgtgaaagaagatcccagcgccaaagtgaccagctacacagccgctgccaatgctctgagcggcgccaccaatcctatcatcacctacgaggactaccggcagatcctgtccagcgccatcaccaacagacccagcagaaagggcgccaaggatattctggccgccgatctggatagcaccaagacaggtgttctgcccggcaactacgtgtcccagagaatcgccatgtaccaggcctctgccgcctctaaagctagaggcgtggtgctgcccaaccggctgagagtgaaagcctacctgcagaacctcgtgggactgaactacatctgcaccacctgggccgctcctatgctgagagccgtgggcgacatcaagagcaagaacagcaacaactaccgcttcgtgggcgagagactggaacggcagcaagagatcgataacctgctggccgtgtccaacatcagaagcgcccaggccatcctgcagcagttcagggccaatgagagcaaccagttctacatcaagaagcggcacatcggcaagggcctgcctagcctgtacgacatgtgggatctgatggacgagaaagagggcatcgacaactacatccagagcctgaagggcgacaagaccgagaggctgccaatcagagagctgctgcagatcatctaccctcacagaaagagcgtgtccgccgagctgtttctgtctgccgccgaactgaccgacgtggaagatagacagaaccggtgcatggtgcaccctacagtgcggggctctctggtcatcaacttcggcaagagcagcaccatcttcggcgctatcacccctcctgacacactgatcaagttccggggcgaaatggtgcctgctggacagacaggcatgatctggttcacaatgcacctggtggacggcggcaaatgggtcaagcaccacattccttgccacagcagccggtacttcgaggaaatctacgcctggaagaaggacctgcctacactgccctttccacggcggagcctgtatggctatgccatcggcaacaagatcagcgacacccggaagatcgacctgcggagaaagaaggccagcaagcagtacctgcggaccctggaaaacatgacccacaacgtggaatttgaccccaccacacagttcatggtggaccaagagctgaacgtgaccatcaccgccagagtgaagaaaatccctcctgtgcgggatgtgcccgtgggcagcagaattatgggcctgaacaagaaccagaccatccgggactgctacagcatctgggagagagtggaagccaacaccagcggcagctttcagcatcccgtggtccaggatgtgtggctgagactggtggccgatggccacgtgacctctacagtgaatggccccaacggccagatcgaccagatgagctactctggccccgatgtggccaactgcggcaactggatgcaagagcggagcaacttcatcaccagcgtggacgacgccgaccagtctatcatgaagcactttctgtggaacaaccgcgtgaagctgtatgcctggaactgcgtgtacgccggcacactgatgaaggccatctctaagcagatgaccaccgccaaccggaacctgttcagaaacgagatcctgagcttcgttggcggcagattcggctgcagactgggatctctggcccaggtttcactggacctgctgcggaggatgaagtccgtgatcagctgctacttcagccggaacaacgccttcaccatcgaggaaagaagcgccttcgacaaagaactgatggaactgttcgagagcctggacaacaagatgaacaacaagcggaaagagaaagtcaaccggacactcagcagcatcttccaggtggccaagcagcacaatgttgtgcggctggtggtcaccaagaacctgcagacccctgatgccaatgtgcggagcgtgatgaatcagagatccgtggattggtgcgctcggaagattgaagagaagatcgtggacctgggcaacgtgatcggaatctatgtggatctggtggaagccctggatctgagccatctggaccccttcatctatatcgccaagggcgacgtgggcaaagagtgccagtttgacgaggtggaaagcagctccctgctgccaattcacaccagcatgtttcgcgactggcacggcctggttaacaagggcagaaccaccacacctatctaccacagcgccctgaggagcttcgccagccactacggcctgagattcgatgacctggccagaatcaaggccgctgagctggccaaaatgctgccagaccagaaggtgttcatcccacacagaggcggacggttcttcatgagcacataccccgtgaccagcaccagcagacccgtgtcttatgatggccggcagcggttcctgaacagcggcgatatggtggccccagtgaacaccatgctgcgcggattcagaagggccagatctgcctatccctatgacgtgcccgattatgccagcctgggcagcggctcccccaagaaaaaacgcaaggtggaagatcctaagaaaaagcggaaagtggacggcagcggcagcgagacccccggtaccagcgagagcgccacccccgagagcggtagtgggagcaacggcagcagcggatccatgcgtgaccacatggtccttcatgagtatgtaaatgctgctgggattacagcggccgcaaggtcaggctccggccagcggggaagcaagcgcaccgccgatggttccgagttcgaaagccccaaaaaaaagcgcaaggtctga

SEQ ID NO: 331 - DNA, 7176 bp, synthetic construct
  misc_feature 1..7176: note = CDS of V43_D3a-D3l-GFP1-10-2a-1xGFP11-dCas9-KRAB
  source 1..7176: mol_type = other DNA
atgcctgctgctaagagagtgaaactggatggatccaaccatgaccaggaatttgaccccccaaaggtttacccacctgtgccagctgagaagaggaagcccatccgcgtgctgtctctctttgatgggattgctacagggctcctggtgctgaaggacctgggcatccaagtggaccgctacattgcctccgaggtgtgtgaggactccatcacggtgggcatggtgcggcaccagggaaagatcatgtacgtcggggacgtccgcagcgtcacacagaagcatatccaggagtggggcccattcgacctggtgattggaggcagtccctgcaatgacctctccattgtcaaccctgcccgcaagggactttatgagggtactggccgcctcttctttgagttctaccgcctcctgcatgatgcgcggcccaaggagggagatgatcgccccttcttctggctctttgagaatgtggtggccatgggcgttagtgacaagagggacatctcgcgatttcttgagtctaaccccgtgatgattgacgccaaagaagtgtctgctgcacacagggcccgttacttctggggtaaccttcctggcatgaacaggcctttggcatccactgtgaatgataagctggagctgcaagagtgtctggagcacggcagaatagccaagttcagcaaagtgaggaccattaccaccaggtcaaactctataaagcagggcaaagaccagcatttccccgtgttcatgaacgagaaggaggacatcctgtggtgcactgaaatggaaagggtgtttggcttccccgtccactacacagacgtctccaacatgagccgcttggcgaggcagagactgctgggccgatcgtggagcgtgccggtcatccgccacctcttcgctccgctgaaggaatattttgcttgtgtgtctagcggcaatagtaacgctaacagccgcgggccgagcttcagcagcggcctggtgccgttaagcttgcgcggcagccatatgggccctatggagatatacaagacagtgtctgcatggaagagacagccagtgcgggtactgagcctcttcagaaacatcgacaaggtactaaagagtttgggcttcttggaaagcggttctggttctgggggaggaacgctgaagtacgtggaagatgtcacaaatgtcgtgaggagagacgtggagaaatggggcccctttgacctggtgtacggctcgacgcagcccctaggcagctcttgtgatcgctgtcccggctggtacatgttccagttccaccggatcctgcagtatgcgctgcctcgccaggagagtcagcggcccttcttctggatattcatggacaatctgctgctgactgaggatgaccaagagacaactacccgcttccttcagacagaggctgtgaccctccaggatgtccgtggcagagactaccagaatgctatgcgggtgtggagcaacattccagggctgaagagcaagcatgcgcccctgaccccaaaggaagaagagtatctgcaagcccaagtcagaagcaggagcaagctggacgccccgaaagttgacctcctggtgaagaactgccttctcccgctgagagagtacttcaagtatttttctcaaaactcacttcctcttggagggccgagctctggcgcacccccaccaagtggagggtctcctgccgggtccccaacatctactgaagaaggcaccagcgaatccgcaacgatgtccaagggagaggagctgttcaccggagtggtgccaatcctggtggagctggacggcgatgtgaacggccacaagttttctgtgcgcggagagggagagggcgacgcaaccatcggcaagctgacactgaagttcatctgcaccacaggcaagctgcccgtgccttggccaaccctggtgaccacactgacatacggcgtgcagtgtttctctaggtatccagaccacatgaagagacacgatttctttaagagcgccatgccagagggatacgtgcaggagcggaccatctccttcaaggacgatggcaagtataagacccgcgccgtggtgaagtttgagggcgatacactggtgaacaggatcgagctgaagggcaccgacttcaaggaggatggcaatatcctgggccacaagctggagtacaactttaatagccacaacgtgtatatcacagccgacaagcagaagaacggcatcaaggccaacttcaccgtgaggcacaatgtggaggacggctccgtgcagctggccgatcactaccagcagaacacacctatcggcgacggacccgtgctgctgcctgataatcactatctgtccacccagacagtgctgtctaaggacccaaacgagaagttggatccaggtggaggtggaagcggaagcggagctactaacttcagcctgctgaagcaggctggagacgtggaggagaaccctggacctatgcctgctgctaagagagtgaaactggatggatccggccccgacatcgtgatcggtagcggcggtcgggaccatatggtcctgcacgaatatgtcaatgctgccggtatcaccgcggccgcaaggtcaggctccggccagcggggaagcaagcgcaccgccgatggttccgagttcgaaagccccaaaaaaaagcgcaaggtcggcggaagcggaagcggaccaaaaaagaagagaaaggtaatggacaagaagtacagcatcggcctggccatcggcaccaactctgtgggctgggccgtgatcaccgacgagtacaaggtgcccagcaagaaattcaaggtgctgggcaacaccgaccggcacagcatcaagaagaacctgatcggcgccctgctgttcgacagcggagaaacagccgaggccacccggctgaagagaaccgccagaagaagatacaccagacggaagaaccggatctgctatctgcaagagatcttcagcaacgagatggccaaggtggacgacagcttcttccacagactggaagagtccttcctggtggaagaggataagaagcacgagcggcaccccatcttcggcaacatcgtggacgaggtggcctaccacgagaagtaccccaccatctaccacctgagaaagaaactggtggacagcaccgacaaggccgacctgcggctgatctatctggccctggcccacatgatcaagttccggggccacttcctgatcgagggcgacctgaaccccgacaacagcgacgtggacaagctgttcatccagctggtgcagacctacaaccagctgttcgaggaaaaccccatcaacgccagcggcgtggacgccaaggccatcctgtctgccagactgagcaagagcagacggctggaaaatctgatcgcccagctgcccggcgagaagaagaatggcctgttcggcaacctgattgccctgagcctgggcctgacccccaacttcaagagcaacttcgacctggccgaggatgccaaactgcagctgagcaaggacacctacgacgacgacctggacaacctgctggcccagatcggcgaccagtacgccgacctgtttctggccgccaagaacctgtccgacgccatcctgctgagcgacatcctgagagtgaacaccgagatcaccaaggcccccctgagcgcctctatgatcaagagatacgacgagcaccaccaggacctgaccctgctgaaagctctcgtgcggcagcagctgcctgagaagtacaaagagattttcttcgaccagagcaagaacggctacgccggctacatcgatggcggagccagccaggaagagttctacaagttcatcaagcccatcctggaaaagatggacggcaccgaggaactgctcgtgaagctgaacagagaggacctgctgcggaagcagcggaccttcgacaacggcagcatcccccaccagatccacctgggagagctgcacgccattctgcggcggcaggaagatttttacccattcctgaaggacaaccgggaaaagatcgagaagatcctgaccttccgcatcccctactacgtgggccctctggccaggggaaacagcagattcgcctggatgaccagaaagagcgaggaaaccatcaccccctggaacttcgaggaagtggtggacaagggcgccagcgcccagagcttcatcgagcggatgaccaacttcgataagaacctgcccaacgagaaggtgctgcccaagcacagcctgctgtacgagtacttcaccgtgtacaacgagctgaccaaagtgaaatacgtgaccgagggaatgagaaagcccgccttcctgagcggcgagcagaaaaaagccatcgtggacctgctgttcaagaccaaccggaaagtgaccgtgaagcagctgaaagaggactacttcaagaaaatcgagtgcttcgactccgtggaaatctccggcgtggaagatcggttcaacgcctccctgggcacataccacgatctgctgaaaattatcaaggacaaggacttcctggacaatgaggaaaacgaggacattctggaagatatcgtgctgaccctgacactgtttgaggacagagagatgatcgaggaacggctgaaaacctatgcccacctgttcgacgacaaagtgatgaagcagctgaagcggcggagatacaccggctggggcaggctgagccggaagctgatcaacggcatccgggacaagcagtccggcaagacaatcctggatttcctgaagtccgacggcttcgccaacagaaacttcatgcagctgatccacgacgacagcctgacctttaaagaggacatccagaaagcccaggtgtccggccagggcgatagcctgcacgagcacattgccaatctggccggcagccccgccattaagaagggcatcctgcagacagtgaaggtggtggacgagctcgtgaaagtgatgggccggcacaagcccgagaacatcgtgatcgaaatggccagagagaaccagaccacccagaagggacagaagaacagccgcgagagaatgaagcggatcgaagagggcatcaaagagctgggcagccagatcctgaaagaacaccccgtggaaaacacccagctgcagaacgagaagctgtacctgtactacctgcagaatgggcgggatatgtacgtggaccaggaactggacatcaaccggctgtccgactacgatgtggacgctatcgtgcctcagagctttctgaaggacgactccatcgataacaaagtgctgactcggagcgacaagaaccggggcaagagcgacaacgtgccctccgaagaggtcgtgaagaagatgaagaactactggcgccagctgctgaatgccaagctgattacccagaggaagttcgacaatctgaccaaggccgagagaggcggcctgagcgaactggataaggccggcttcatcaagagacagctggtggaaacccggcagatcacaaagcacgtggcacagatcctggactcccggatgaacactaagtacgacgagaacgacaaactgatccgggaagtgaaagtgatcaccctgaagtccaagctggtgtccgatttccggaaggatttccagttttacaaagtgcgcgagatcaacaactaccaccacgcccacgacgcctacctgaacgccgtcgtgggaaccgccctgatcaaaaagtaccctaagctggaaagcgagttcgtgtacggcgactacaaggtgtacgacgtgcggaagatgatcgccaagagcgagcaggaaatcggcaaggctaccgccaagtacttcttctacagcaacatcatgaactttttcaagaccgagattaccctggccaacggcgagatccggaagcggcctctgatcgagacaaacggcgaaacaggcgagatcgtgtgggataagggccgggactttgccaccgtgcggaaagtgctgtctatgccccaagtgaatatcgtgaaaaagaccgaggtgcagacaggcggcttcagcaaagagtctatcctgcccaagaggaacagcgacaagctgatcgccagaaagaaggactgggaccctaagaagtacggcggcttcgacagccccaccgtggcctattctgtgctggtggtggccaaagtggaaaagggcaagtccaagaaactgaagagtgtgaaagagctgctggggatcaccatcatggaaagaagcagcttcgagaagaatcccatcgactttctggaagccaagggctacaaagaagtgaaaaaggacctgatcatcaagctgcctaagtactccctgttcgagctggaaaacggccggaagagaatgctggcctctgccggcgaactgcagaagggaaacgaactggccctgccctccaaatatgtgaacttcctgtacctggccagccactatgagaagctgaagggctcccccgaggataatgagcagaaacagctgtttgtggaacagcacaaacactacctggacgagatcatcgagcagatcagcgagttctccaagagagtgatcctggccgacgctaatctggacaaggtgctgagcgcctacaacaagcacagagacaagcctatcagagagcaggccgagaatatcatccacctgtttaccctgaccaatctgggagcccctgccgccttcaagtactttgacaccaccatcgaccggaagaggtacaccagcaccaaagaggtgctggacgccaccctgatccaccagagcatcaccggcctgtacgagacacggatcgacctgtctcagctgggaggcgacgcctatccctatgacgtgcccgattatgccagcctgggcagcggctcccccaagaaaaaacgcaaggtggaagatcctaagaaaaagcggaaagtggacggcagcggcagcgagacccccggtaccagcgagagcgccacccccgagagccggacactggtgaccttcaaggatgtatttgtggacttcaccagggaggagtggaagctgctggacactgctcagcagatcgtgtacagaaatgtgatgctggagaactataagaacctggtttccttgggttatcagcttactaagccagatgtgatcctccggttggagaagggagaagagccctga

SEQ ID NO: 332 - DNA, 7764 bp, synthetic construct
  misc_feature 1..7764: note = CDS of V44_7xGFP11-dCas9-ZIM3-2a-D3a-hD3L-GFP1-10
  source 1..7764: mol_type = other DNA
atgcctgctgctaagagagtgaaactggatggatccatgcgtgaccacatggtccttcatgagtatgtaaatgctgctgggattacaggtggctctggaggtagagatcatatggttctccacgaatacgttaacgccgcaggcatcactggcggtagtggaggacgcgaccatatggtactacatgaatatgtcaatgcagccggaataaccggagggtccggaggccgggatcacatggtgctgcatgagtatgtgaacgcggcgggtataactggtgggtcgggcggacgagaccatatggtgcttcacgaatacgtaaacgcagctggcattactggcggatcaggtggcagggatcacatggtactccatgagtacgtgaacgctgctggaatcacaggcggtagcggcggtcgggaccatatggtcctgcacgaatatgtcaatgctgccggtatcaccgcggccgcaaggtcaggctccggccagcggggaagcaagcgcaccgccgatggttccgagttcgaaagccccaaaaaaaagcgcaaggtcggcggaagcggaagcggaccaaaaaagaagagaaaggtaatggacaagaagtacagcatcggcctggccatcggcaccaactctgtgggctgggccgtgatcaccgacgagtacaaggtgcccagcaagaaattcaaggtgctgggcaacaccgaccggcacagcatcaagaagaacctgatcggcgccctgctgttcgacagcggagaaacagccgaggccacccggctgaagagaaccgccagaagaagatacaccagacggaagaaccggatctgctatctgcaagagatcttcagcaacgagatggccaaggtggacgacagcttcttccacagactggaagagtccttcctggtggaagaggataagaagcacgagcggcaccccatcttcggcaacatcgtggacgaggtggcctaccacgagaagtaccccaccatctaccacctgagaaagaaactggtggacagcaccgacaaggccgacctgcggctgatctatctggccctggcccacatgatcaagttccggggccacttcctgatcgagggcgacctgaaccccgacaacagcgacgtggacaagctgttcatccagctggtgcagacctacaaccagctgttcgaggaaaaccccatcaacgccagcggcgtggacgccaaggccatcctgtctgccagactgagcaagagcagacggctggaaaatctgatcgcccagctgcccggcgagaagaagaatggcctgttcggcaacctgattgccctgagcctgggcctgacccccaacttcaagagcaacttcgacctggccgaggatgccaaactgcagctgagcaaggacacctacgacgacgacctggacaacctgctggcccagatcggcgaccagtacgccgacctgtttctggccgccaagaacctgtccgacgccatcctgctgagcgacatcctgagagtgaacaccgagatcaccaaggcccccctgagcgcctctatgatcaagagatacgacgagcaccaccaggacctgaccctgctgaaagctctcgtgcggcagcagctgcctgagaagtacaaagagattttcttcgaccagagcaagaacggctacgccggctacatcgatggcggagccagccaggaagagttctacaagttcatcaagcccatcctggaaaagatggacggcaccgaggaactgctcgtgaagctgaacagagaggacctgctgcggaagcagcggaccttcgacaacggcagcatcccccaccagatccacctgggagagctgcacgccattctgcggcggcaggaagatttttacccattcctgaaggacaaccgggaaaagatcgagaagatcctgaccttccgcatcccctactacgtgggccctctggccaggggaaacagcagattcgcctggatgaccagaaagagcgaggaaaccatcaccccctggaacttcgaggaagtggtggacaagggcgccagcgcccagagcttcatcgagcggatgaccaacttcgataagaacctgcccaacgagaaggtgctgcccaagcacagcctgctgtacgagtacttcaccgtgtacaacgagctgaccaaagtgaaatacgtgaccgagggaatgagaaagcccgccttcctgagcggcgagcagaaaaaagccatcgtggacctgctgttcaagaccaaccggaaagtgaccgtgaagcagctgaaagaggactacttcaagaaaatcgagtgcttcgactccgtggaaatctccggcgtggaagatcggttcaacgcctccctgggcacataccacgatctgctgaaaattatcaaggacaaggacttcctggacaatgaggaaaacgaggacattctggaagatatcgtgctgaccctgacactgtttgaggacagagagatgatcgaggaacggctgaaaacctatgcccacctgttcgacgacaaagtgatgaagcagctgaagcggcggagatacaccggctggggcaggctgagccggaagctgatcaacggcatccgggacaagcagtccggcaagacaatcctggatttcctgaagtccgacggcttcgccaacagaaacttcatgcagctgatccacgacgacagcctgacctttaaagaggacatccagaaagcccaggtgtccggccagggcgatagcctgcacgagcacattgccaatctggccggcagccccgccattaagaagggcatcctgcagacagtgaaggtggtggacgagctcgtgaaagtgatgggccggcacaagcccgagaacatcgtgatcgaaatggccagagagaaccagaccacccagaagggacagaagaacagccgcgagagaatgaagcggatcgaagagggcatcaaagagctgggcagccagatcctgaaagaacaccccgtggaaaacacccagctgcagaacgagaagctgtacctgtactacctgcagaatgggcgggatatgtacgtggaccaggaactggacatcaaccggctgtccgactacgatgtggacgctatcgtgcctcagagctttctgaaggacgactccatcgataacaaagtgctgactcggagcgacaagaaccggggcaagagcgacaacgtgccctccgaagaggtcgtgaagaagatgaagaactactggcgccagctgctgaatgccaagctgattacccagaggaagttcgacaatctgaccaaggccgagagaggcggcctgagcgaactggataaggccggcttcatcaagagacagctggtggaaacccggcagatcacaaagcacgtggcacagatcctggactcccggatgaacactaagtacgacgagaacgacaaactgatccgggaagtgaaagtgatcaccctgaagtccaagctggtgtccgatttccggaaggatttccagttttacaaagtgcgcgagatcaacaactaccaccacgcccacgacgcctacctgaacgccgtcgtgggaaccgccctgatcaaaaagtaccctaagctggaaagcgagttcgtgtacggcgactacaaggtgtacgacgtgcggaagatgatcgccaagagcgagcaggaaatcggcaaggctaccgccaagtacttcttctacagcaacatcatgaactttttcaagaccgagattaccctggccaacggcgagatccggaagcggcctctgatcgagacaaacggcgaaacaggcgagatcgtgtgggataagggccgggactttgccaccgtgcggaaagtgctgtctatgccccaagtgaatatcgtgaaaaagaccgaggtgcagacaggcggcttcagcaaagagtctatcctgcccaagaggaacagcgacaagctgatcgccagaaagaaggactgggaccctaagaagtacggcggcttcgacagccccaccgtggcctattctgtgctggtggtggccaaagtggaaaagggcaagtccaagaaactgaagagtgtgaaagagctgctggggatcaccatcatggaaagaagcagcttcgagaagaatcccatcgactttctggaagccaagggctacaaagaagtgaaaaaggacctgatcatcaagctgcctaagtactccctgttcgagctggaaaacggccggaagagaatgctggcctctgccggcgaactgcagaagggaaacgaactggccctgccctccaaatatgtgaacttcctgtacctggccagccactatgagaagctgaagggctcccccgaggataatgagcagaaacagctgtttgtggaacagcacaaacactacctggacgagatcatcgagcagatcagcgagttctccaagagagtgatcctggccgacgctaatctggacaaggtgctgagcgcctacaacaagcacagagacaagcctatcagagagcaggccgagaatatcatccacctgtttaccctgaccaatctgggagcccctgccgccttcaagtactttgacaccaccatcgaccggaagaggtacaccagcaccaaagaggtgctggacgccaccctgatccaccagagcatcaccggcctgtacgagacacggatcgacctgtctcagctgggaggcgacgcctatccctatgacgtgcccgattatgccagcctgggcagcggctcccccaagaaaaaacgcaaggtggaagatcctaagaaaaagcggaaagtggacggcagcggcagcgagacccccggtaccagcgagagcgccacccccgagagcatgaacaattcccagggaagagtgaccttcgaggatgtcactgtgaacttcacccagggggagtggcagcggctgaatcccgaacagagaaacttgtacagggatgtgatgctggagaattacagcaaccttgtctctgtgggacaaggggaaaccaccaaacccgatgtgatcttgaggttggaacaaggaaaggagccatggttggaggaagaggaagtgctgggaagtggccgtgcagaaaaaaatggggacattggagggcagatttggaagccaaaggatgtgaaagagagtctcctcgagggaagcggagctactaacttcagcctgctgaagcaggctggagacgtggaggagaaccctggacctatgcctgctgctaagagagtgaaactggatggatccaaccatgaccaggaatttgaccccccaaaggtttacccacctgtgccagctgagaagaggaagcccatccgcgtgctgtctctctttgatgggattgctacagggctcctggtgctgaaggacctgggcatccaagtggaccgctacattgcctccgaggtgtgtgaggactccatcacggtgggcatggtgcggcaccagggaaagatcatgtacgtcggggacgtccgcagcgtcacacagaagcatatccaggagtggggcccattcgacctggtgattggaggcagtccctgcaatgacctctccattgtcaaccctgcccgcaagggactttatgagggtactggccgcctcttctttgagttctaccgcctcctgcatgatgcgcggcccaaggagggagatgatcgccccttcttctggctctttgagaatgtggtggccatgggcgttagtgacaagagggacatctcgcgatttcttgagtctaaccccgtgatgattgacgccaaagaagtgtctgctgcacacagggcccgttacttctggggtaaccttcctggcatgaacaggcctttggcatccactgtgaatgataagctggagctgcaagagtgtctggagcacggcagaatagccaagttcagcaaagtgaggaccattaccaccaggtcaaactctataaagcagggcaaagaccagcatttccccgtgttcatgaacgagaaggaggacatcctgtggtgcactgaaatggaaagggtgtttggcttccccgtccactacacagacgtctccaacatgagccgcttggcgaggcagagactgctgggccgatcgtggagcgtgccggtcatccgccacctcttcgctccgctgaaggaatattttgcttgtgtgtctagcggcaatagtaacgctaacagccgcgggccgagcttcagcagcggcctggtgccgttaagcttgcgcggcagccatatgttcgaaaccgtgcctgtgtggaggagacagccagtccgggtgctgtccctttttgaagacatcaagaaagagctgacgagtttgggctttttggaaagtggttctgacccgggacaactgaagcatgtggttgatgtcacagacacagtgaggaaggatgtggaggagtggggacccttcgatcttgtgtacggcgccacacctcccctgggccacacctgtgaccgtcctcccagctggtacctgttccagttccaccggctcctgcagtacgcacggcccaagccaggcagccccaggcccttcttctggatgttcgtggacaatctggtgctgaacaaggaagacctggacgtcgcatctcgcttcctggagatggagccagtcaccatcccagatgtccacggcggatccttgcagaatgctgtccgcgtgtggagcaacatcccagccataaggagcagcaggcactgggctctggtttcggaagaagaattgtccctgctggcccagaacaagcagagctcgaagctcgcggccaagtggcccaccaagctggtgaagaactgctttctccccctaagagaatatttcaagtatttttcaggagggccgagctctggcgcacccccaccaagtggagggtctcctgccgggtccccaacatctactgaagaaggcaccagcgaatccgcaacgcccgagtcaggccctggtacctccacagaaccatctgaaggtagtgcgcctggttccccagctggaagccctacttccaccgaagaaggcacgtcaaccgaaccaagtgaaggatctgcccctgggaccagcactgaaccatctgagccaaaaaagaagagaaaggtaccatctgagatgtccaagggagaggagctgttcaccggagtggtgccaatcctggtggagctggacggcgatgtgaacggccacaagttttctgtgcgcggagagggagagggcgacgcaaccatcggcaagctgacactgaagttcatctgcaccacaggcaagctgcccgtgccttggccaaccctggtgaccacactgacatacggcgtgcagtgtttctctaggtatccagaccacatgaagagacacgatttctttaagagcgccatgccagagggatacgtgcaggagcggaccatctccttcaaggacgatggcaagtataagacccgcgccgtggtgaagtttgagggcgatacactggtgaacaggatcgagctgaagggcaccgacttcaaggaggatggcaatatcctgggccacaagctggagtacaactttaatagccacaacgtgtatatcacagccgacaagcagaagaacggcatcaaggccaacttcaccgtgaggcacaatgtggaggacggctccgtgcagctggccgatcactaccagcagaacacacctatcggcgacggacccgtgctgctgcctgataatcactatctgtccacccagacagtgctgtctaaggacccaaacgagaagtga

SEQ ID NO: 333 - DNA, 7167 bp, synthetic construct
  misc_feature 1..7167: note = CDS of V45_D3a-D3l-1xGFP11-2a-GFP1-10-dCas9-KRAB
  source 1..7167: mol_type = other DNA
atgcctgctgctaagagagtgaaactggatggatccaaccatgaccaggaatttgaccccccaaaggtttacccacctgtgccagctgagaagaggaagcccatccgcgtgctgtctctctttgatgggattgctacagggctcctggtgctgaaggacctgggcatccaagtggaccgctacattgcctccgaggtgtgtgaggactccatcacggtgggcatggtgcggcaccagggaaagatcatgtacgtcggggacgtccgcagcgtcacacagaagcatatccaggagtggggcccattcgacctggtgattggaggcagtccctgcaatgacctctccattgtcaaccctgcccgcaagggactttatgagggtactggccgcctcttctttgagttctaccgcctcctgcatgatgcgcggcccaaggagggagatgatcgccccttcttctggctctttgagaatgtggtggccatgggcgttagtgacaagagggacatctcgcgatttcttgagtctaaccccgtgatgattgacgccaaagaagtgtctgctgcacacagggcccgttacttctggggtaaccttcctggcatgaacaggcctttggcatccactgtgaatgataagctggagctgcaagagtgtctggagcacggcagaatagccaagttcagcaaagtgaggaccattaccaccaggtcaaactctataaagcagggcaaagaccagcatttccccgtgttcatgaacgagaaggaggacatcctgtggtgcactgaaatggaaagggtgtttggcttccccgtccactacacagacgtctccaacatgagccgcttggcgaggcagagactgctgggccgatcgtggagcgtgccggtcatccgccacctcttcgctccgctgaaggaatattttgcttgtgtgtctagcggcaatagtaacgctaacagccgcgggccgagcttcagcagcggcctggtgccgttaagcttgcgcggcagccatatgggccctatggagatatacaagacagtgtctgcatggaagagacagccagtgcgggtactgagcctcttcagaaacatcgacaaggtactaaagagtttgggcttcttggaaagcggttctggttctgggggaggaacgctgaagtacgtggaagatgtcacaaatgtcgtgaggagagacgtggagaaatggggcccctttgacctggtgtacggctcgacgcagcccctaggcagctcttgtgatcgctgtcccggctggtacatgttccagttccaccggatcctgcagtatgcgctgcctcgccaggagagtcagcggcccttcttctggatattcatggacaatctgctgctgactgaggatgaccaagagacaactacccgcttccttcagacagaggctgtgaccctccaggatgtccgtggcagagactaccagaatgctatgcgggtgtggagcaacattccagggctgaagagcaagcatgcgcccctgaccccaaaggaagaagagtatctgcaagcccaagtcagaagcaggagcaagctggacgccccgaaagttgacctcctggtgaagaactgccttctcccgctgagagagtacttcaagtatttttctcaaaactcacttcctcttggagggccgagctctggcgcacccccaccaagtggagggtctcctgccgggtccccaacatctactgaagaaggcaccagcgaatccgcaacgggcggtagcggcggtcgggaccatatggtcctgcacgaatatgtcaatgctgccggtatcaccgcggccgcaaggtcaggctccggccagcggggaagcaagcgcaccgccgatggttccgagttcgaaagccccaaaaaaaagcgcaaggtcggaagcggagctactaacttcagcctgctgaagcaggctggagacgtggaggagaaccctggacctatgcctgctgctaagagagtgaaactggatggatccggccccgacatcgtgatgtccaagggagaggagctgttcaccggagtggtgccaatcctggtggagctggacggcgatgtgaacggccacaagttttctgtgcgcggagagggagagggcgacgcaaccatcggcaagctgacactgaagttcatctgcaccacaggcaagctgcccgtgccttggccaaccctggtgaccacactgacatacggcgtgcagtgtttctctaggtatccagaccacatgaagagacacgatttctttaagagcgccatgccagagggatacgtgcaggagcggaccatctccttcaaggacgatggcaagtataagacccgcgccgtggtgaagtttgagggcgatacactggtgaacaggatcgagctgaagggcaccgacttcaaggaggatggcaatatcctgggccacaagctggagtacaactttaatagccacaacgtgtatatcacagccgacaagcagaagaacggcatcaaggccaacttcaccgtgaggcacaatgtggaggacggctccgtgcagctggccgatcactaccagcagaacacacctatcggcgacggacccgtgctgctgcctgataatcactatctgtccacccagacagtgctgtctaaggacccaaacgagaagttggatccaggtggaggcggaagcggaagcggaccaaaaaagaagagaaaggtaatggacaagaagtacagcatcggcctggccatcggcaccaactctgtgggctgggccgtgatcaccgacgagtacaaggtgcccagcaagaaattcaaggtgctgggcaacaccgaccggcacagcatcaagaagaacctgatcggcgccctgctgttcgacagcggagaaacagccgaggccacccggctgaagagaaccgccagaagaagatacaccagacggaagaaccggatctgctatctgcaagagatcttcagcaacgagatggccaaggtggacgacagcttcttccacagactggaagagtccttcctggtggaagaggataagaagcacgagcggcaccccatcttcggcaacatcgtggacgaggtggcctaccacgagaagtaccccaccatctaccacctgagaaagaaactggtggacagcaccgacaaggccgacctgcggctgatctatctggccctggcccacatgatcaagttccggggccacttcctgatcgagggcgacctgaaccccgacaacagcgacgtggacaagctgttcatccagctggtgcagacctacaaccagctgttcgaggaaaaccccatcaacgccagcggcgtggacgccaaggccatcctgtctgccagactgagcaagagcagacggctggaaaatctgatcgcccagctgcccggcgagaagaagaatggcctgttcggcaacctgattgccctgagcctgggcctgacccccaacttcaagagcaacttcgacctggccgaggatgccaaactgcagctgagcaaggacacctacgacgacgacctggacaacctgctggcccagatcggcgaccagtacgccgacctgtttctggccgccaagaacctgtccgacgccatcctgctgagcgacatcctgagagtgaacaccgagatcaccaaggcccccctgagcgcctctatgatcaagagatacgacgagcaccaccaggacctgaccctgctgaaagctctcgtgcggcagcagctgcctgagaagtacaaagagattttcttcgaccagagcaagaacggctacgccggctacatcgatggcggagccagccaggaagagttctacaagttcatcaagcccatcctggaaaagatggacggcaccgaggaactgctcgtgaagctgaacagagaggacctgctgcggaagcagcggaccttcgacaacggcagcatcccccaccagatccacctgggagagctgcacgccattctgcggcggcaggaagatttttacccattcctgaaggacaaccgggaaaagatcgagaagatcctgaccttccgcatcccctactacgtgggccctctggccaggggaaacagcagattcgcctggatgaccagaaagagcgaggaaaccatcaccccctggaacttcgaggaagtggtggacaagggcgccagcgcccagagcttcatcgagcggatgaccaacttcgataagaacctgcccaacgagaaggtgctgcccaagcacagcctgctgtacgagtacttcaccgtgtacaacgagctgaccaaagtgaaatacgtgaccgagggaatgagaaagcccgccttcctgagcggcgagcagaaaaaagccatcgtggacctgctgttcaagaccaaccggaaagtgaccgtgaagcagctgaaagaggactacttcaagaaaatcgagtgcttcgactccgtggaaatctccggcgtggaagatcggttcaacgcctccctgggcacataccacgatctgctgaaaattatcaaggacaaggacttcctggacaatgaggaaaacgaggacattctggaagatatcgtgctgaccctgacactgtttgaggacagagagatgatcgaggaacggctgaaaacctatgcccacctgttcgacgacaaagtgatgaagcagctgaagcggcggagatacaccggctggggcaggctgagccggaagctgatcaacggcatccgggacaagcagtccggcaagacaatcctggatttcctgaagtccgacggcttcgccaacagaaacttcatgcagctgatccacgacgacagcctgacctttaaagaggacatccagaaagcccaggtgtccggccagggcgatagcctgcacgagcacattgccaatctggccggcagccccgccattaagaagggcatcctgcagacagtgaaggtggtggacgagctcgtgaaagtgatgggccggcacaagcccgagaacatcgtgatcgaaatggccagagagaaccagaccacccagaagggacagaagaacagccgcgagagaatgaagcggatcgaagagggcatcaaagagctgggcagccagatcctgaaagaacaccccgtggaaaacacccagctgcagaacgagaagctgtacctgtactacctgcagaatgggcgggatatgtacgtggaccaggaactggacatcaaccggctgtccgactacgatgtggacgctatcgtgcctcagagctttctgaaggacgactccatcgataacaaagtgctgactcggagcgacaagaaccggggcaagagcgacaacgtgccctccgaagaggtcgtgaagaagatgaagaactactggcgccagctgctgaatgccaagctgattacccagaggaagttcgacaatctgaccaaggccgagagaggcggcctgagcgaactggataaggccggcttcatcaagagacagctggtggaaacccggcagatcacaaagcacgtggcacagatcctggactcccggatgaacactaagtacgacgagaacgacaaactgatccgggaagtgaaagtgatcaccctgaagtccaagctggtgtccgatttccggaaggatttccagttttacaaagtgcgcgagatcaacaactaccaccacgcccacgacgcctacctgaacgccgtcgtgggaaccgccctgatcaaaaagtaccctaagctggaaagcgagttcgtgtacggcgactacaaggtgtacgacgtgcggaagatgatcgccaagagcgagcaggaaatcggcaaggctaccgccaagtacttcttctacagcaacatcatgaactttttcaagaccgagattaccctggccaacggcgagatccggaagcggcctctgatcgagacaaacggcgaaacaggcgagatcgtgtgggataagggccgggactttgccaccgtgcggaaagtgctgtctatgccccaagtgaatatcgtgaaaaagaccgaggtgcagacaggcggcttcagcaaagagtctatcctgcccaagaggaacagcgacaagctgatcgccagaaagaaggactgggaccctaagaagtacggcggcttcgacagccccaccgtggcctattctgtgctggtggtggccaaagtggaaaagggcaagtccaagaaactgaagagtgtgaaagagctgctggggatcaccatcatggaaagaagcagcttcgagaagaatcccatcgactttctggaagccaagggctacaaagaagtgaaaaaggacctgatcatcaagctgcctaagtactccctgttcgagctggaaaacggccggaagagaatgctggcctctgccggcgaactgcagaagggaaacgaactggccctgccctccaaatatgtgaacttcctgtacctggccagccactatgagaagctgaagggctcccccgaggataatgagcagaaacagctgtttgtggaacagcacaaacactacctggacgagatcatcgagcagatcagcgagttctccaagagagtgatcctggccgacgctaatctggacaaggtgctgagcgcctacaacaagcacagagacaagcctatcagagagcaggccgagaatatcatccacctgtttaccctgaccaatctgggagcccctgccgccttcaagtactttgacaccaccatcgaccggaagaggtacaccagcaccaaagaggtgctggacgccaccctgatccaccagagcatcaccggcctgtacgagacacggatcgacctgtctcagctgggaggcgacgcctatccctatgacgtgcccgattatgccagcctgggcagcggctcccccaagaaaaaacgcaaggtggaagatcctaagaaaaagcggaaagtggacggcagcggcagcgagacccccggtaccagcgagagcgccacccccgagagccggacactggtgaccttcaaggatgtatttgtggacttcaccagggaggagtggaagctgctggacactgctcagcagatcgtgtacagaaatgtgatgctggagaactataagaacctggtttccttgggttatcagcttactaagccagatgtgatcctccggttggagaagggagaagagccctga

SEQ ID NO: 334 - DNA, 7968 bp, synthetic construct
  misc_feature 1..7968: note = CDS of V46_10xGFP11-dCas9-ZIM3-2a-D3a-hD3L-GFP1-10
  source 1..7968: mol_type = other DNA
atgcctgctgctaagagagtgaaactggatggatccatgcgtgaccacatggtccttcatgagtatgtaaatgctgctgggattacaggtggctctggaggtagagatcatatggttctccacgaatacgttaacgccgcaggcatcactggcggtagtggaggacgcgaccatatggtactacatgaatatgtcaatgcagccggaataaccggagggtccggaggccgggatcacatggtgctgcatgagtatgtgaacgcggcgggtataactggtgggtcgggcggacgagaccatatggtgcttcacgaatacgtaaacgcagctggcattactggcggatcaggtggcagggatcacatggtactccatgagtacgtgaacgctgctggaatcacaggcggtagcggcggtcgggaccatatggtcctgcacgaatatgtcaatgctgccggtatcaccgcggccgcaggtggctctggaggtagagatcatatggttctccacgaatacgttaacgccgcaggcatcactggcggtagtggaggacgcgaccatatggtactacatgaatatgtcaatgcagccggaataaccggagggtccggaggccgggatcacatggtgctgcatgagtatgtgaacgcggcgggtataactggtgggtcgggcggaaggtcaggctccggccagcggggaagcaagcgcaccgccgatggttccgagttcgaaagccccaaaaaaaagcgcaaggtcggcggaagcggaagcggaccaaaaaagaagagaaaggtaatggacaagaagtacagcatcggcctggccatcggcaccaactctgtgggctgggccgtgatcaccgacgagtacaaggtgcccagcaagaaattcaaggtgctgggcaacaccgaccggcacagcatcaagaagaacctgatcggcgccctgctgttcgacagcggagaaacagccgaggccacccggctgaagagaaccgccagaagaagatacaccagacggaagaaccggatctgctatctgcaagagatcttcagcaacgagatggccaaggtggacgacagcttcttccacagactggaagagtccttcctggtggaagaggataagaagcacgagcggcaccccatcttcggcaacatcgtggacgaggtggcctaccacgagaagtaccccaccatctaccacctgagaaagaaactggtggacagcaccgacaaggccgacctgcggctgatctatctggccctggcccacatgatcaagttccggggccacttcctgatcgagggcgacctgaaccccgacaacagcgacgtggacaagctgttcatccagctggtgcagacctacaaccagctgttcgaggaaaaccccatcaacgccagcggcgtggacgccaaggccatcctgtctgccagactgagcaagagcagacggctggaaaatctgatcgcccagctgcccggcgagaagaagaatggcctgttcggcaacctgattgccctgagcctgggcctgacccccaacttcaagagcaacttcgacctggccgaggatgccaaactgcagctgagcaaggacacctacgacgacgacctggacaacctgctggcccagatcggcgaccagtacgccgacctgtttctggccgccaagaacctgtccgacgccatcctgctgagcgacatcctgagagtgaacaccgagatcaccaaggcccccctgagcgcctctatgatcaagagatacgacgagcaccaccaggacctgaccctgctgaaagctctcgtgcggcagcagctgcctgagaagtacaaagagattttcttcgaccagagcaagaacggctacgccggctacatcgatggcggagccagccaggaagagttctacaagttcatcaagcccatcctggaaaagatggacggcaccgaggaactgctcgtgaagctgaacagagaggacctgctgcggaagcagcggaccttcgacaacggcagcatcccccaccagatccacctgggagagctgcacgccattctgcggcggcaggaagatttttacccattcctgaaggacaaccgggaaaagatcgagaagatcctgaccttccgcatcccctactacgtgggccctctggccaggggaaacagcagattcgcctggatgaccagaaagagcgaggaaaccatcaccccctggaacttcgaggaagtggtggacaagggcgccagcgcccagagcttcatcgagcggatgaccaacttcgataagaacctgcccaacgagaaggtgctgcccaagcacagcctgctgtacgagtacttcaccgtgtacaacgagctgaccaaagtgaaatacgtgaccgagggaatgagaaagcccgccttcctgagcggcgagcagaaaaaagccatcgtggacctgctgttcaagaccaaccggaaagtgaccgtgaagcagctgaaagaggactacttcaagaaaatcgagtgcttcgactccgtggaaatctccggcgtggaagatcggttcaacgcctccctgggcacataccacgatctgctgaaaattatcaaggacaaggacttcctggacaatgaggaaaacgaggacattctggaagatatcgtgctgaccctgacactgtttgaggacagagagatgatcgaggaacggctgaaaacctatgcccacctgttcgacgacaaagtgatgaagcagctgaagcggcggagatacaccggctggggcaggctgagccggaagctgatcaacggcatccgggacaagcagtccggcaagacaatcctggatttcctgaagtccgacggcttcgccaacagaaacttcatgcagctgatccacgacgacagcctgacctttaaagaggacatccagaaagcccaggtgtccggccagggcgatagcctgcacgagcacattgccaatctggccggcagccccgccattaagaagggcatcctgcagacagtgaaggtggtggacgagctcgtgaaagtgatgggccggcacaagcccgagaacatcgtgatcgaaatggccagagagaaccagaccacccagaagggacagaagaacagccgcgagagaatgaagcggatcgaagagggcatcaaagagctgggcagccagatcctgaaagaacaccccgtggaaaacacccagctgcagaacgagaagctgtacctgtactacctgcagaatgggcgggatatgtacgtggaccaggaactggacatcaaccggctgtccgactacgatgtggacgctatcgtgcctcagagctttctgaaggacgactccatcgataacaaagtgctgactcggagcgacaagaaccggggcaagagcgacaacgtgccctccgaagaggtcgtgaagaagatgaagaactactggcgccagctgctgaatgccaagctgattacccagaggaagttcgacaatctgaccaaggccgagagaggcggcctgagcgaactggataaggccggcttcatcaagagacagctggtggaaacccggcagatcacaaagcacgtggcacagatcctggactcccggatgaacactaagtacgacgagaacgacaaactgatccgggaagtgaaagtgatcaccctgaagtccaagctggtgtccgatttccggaaggatttccagttttacaaagtgcgcgagatcaacaactaccaccacgcccacgacgcctacctgaacgccgtcgtgggaaccgccctgatcaaaaagtaccctaagctggaaagcgagttcgtgtacggcgactacaaggtgtacgacgtgcggaagatgatcgccaagagcgagcaggaaatcggcaaggctaccgccaagtacttcttctacagcaacatcatgaactttttcaagaccgagattaccctggccaacggcgagatccggaagcggcctctgatcgagacaaacggcgaaacaggcgagatcgtgtgggataagggccgggactttgccaccgtgcggaaagtgctgtctatgccccaagtgaatatcgtgaaaaagaccgaggtgcagacaggcggcttcagcaaagagtctatcctgcccaagaggaacagcgacaagctgatcgccagaaagaaggactgggaccctaagaagtacggcggcttcgacagccccaccgtggcctattctgtgctggtggtggccaaagtggaaaagggcaagtccaagaaactgaagagtgtgaaagagctgctggggatcaccatcatggaaagaagcagcttcgagaagaatcccatcgactttctggaagccaagggctacaaagaagtgaaaaaggacctgatcatcaagctgcctaagtactccctgttcgagctggaaaacggccggaagagaatgctggcctctgccggcgaactgcagaagggaaacgaactggccctgccctccaaatatgtgaacttcctgtacctggccagccactatgagaagctgaagggctcccccgaggataatgagcagaaacagctgtttgtggaacagcacaaacactacctggacgagatcatcgagcagatcagcgagttctccaagagagtgatcctggccgacgctaatctggacaaggtgctgagcgcctacaacaagcacagagacaagcctatcagagagcaggccgagaatatcatccacctgtttaccctgaccaatctgggagcccctgccgccttcaagtactttgacaccaccatcgaccggaagaggtacaccagcaccaaagaggtgctggacgccaccctgatccaccagagcatcaccggcctgtacgagacacggatcgacctgtctcagctgggaggcgacgcctatccctatgacgtgcccgattatgccagcctgggcagcggctcccccaagaaaaaacgcaaggtggaagatcctaagaaaaagcggaaagtggacggcagcggcagcgagacccccggtaccagcgagagcgccacccccgagagcatgaacaattcccagggaagagtgaccttcgaggatgtcactgtgaacttcacccagggggagtggcagcggctgaatcccgaacagagaaacttgtacagggatgtgatgctggagaattacagcaaccttgtctctgtgggacaaggggaaaccaccaaacccgatgtgatcttgaggttggaacaaggaaaggagccatggttggaggaagaggaagtgctgggaagtggccgtgcagaaaaaaatggggacattggagggcagatttggaagccaaaggatgtgaaagagagtctcctcgagggaagcggagctactaacttcagcctgctgaagcaggctggagacgtggaggagaaccctggacctatgcctgctgctaagagagtgaaactggatggatccaaccatgaccaggaatttgaccccccaaaggtttacccacctgtgccagctgagaagaggaagcccatccgcgtgctgtctctctttgatgggattgctacagggctcctggtgctgaaggacctgggcatccaagtggaccgctacattgcctccgaggtgtgtgaggactccatcacggtgggcatggtgcggcaccagggaaagatcatgtacgtcggggacgtccgcagcgtcacacagaagcatatccaggagtggggcccattcgacctggtgattggaggcagtccctgcaatgacctctccattgtcaaccctgcccgcaagggactttatgagggtactggccgcctcttctttgagttctaccgcctcctgcatgatgcgcggcccaaggagggagatgatcgccccttcttctggctctttgagaatgtggtggccatgggcgttagtgacaagagggacatctcgcgatttcttgagtctaaccccgtgatgattgacgccaaagaagtgtctgctgcacacagggcccgttacttctggggtaaccttcctggcatgaacaggcctttggcatccactgtgaatgataagctggagctgcaagagtgtctggagcacggcagaatagccaagttcagcaaagtgaggaccattaccaccaggtcaaactctataaagcagggcaaagaccagcatttccccgtgttcatgaacgagaaggaggacatcctgtggtgcactgaaatggaaagggtgtttggcttccccgtccactacacagacgtctccaacatgagccgcttggcgaggcagagactgctgggccgatcgtggagcgtgccggtcatccgccacctcttcgctccgctgaaggaatattttgcttgtgtgtctagcggcaatagtaacgctaacagccgcgggccgagcttcagcagcggcctggtgccgttaagcttgcgcggcagccatatgttcgaaaccgtgcctgtgtggaggagacagccagtccgggtgctgtccctttttgaagacatcaagaaagagctgacgagtttgggctttttggaaagtggttctgacccgggacaactgaagcatgtggttgatgtcacagacacagtgaggaaggatgtggaggagtggggacccttcgatcttgtgtacggcgccacacctcccctgggccacacctgtgaccgtcctcccagctggtacctgttccagttccaccggctcctgcagtacgcacggcccaagccaggcagccccaggcccttcttctggatgttcgtggacaatctggtgctgaacaaggaagacctggacgtcgcatctcgcttcctggagatggagccagtcaccatcccagatgtccacggcggatccttgcagaatgctgtccgcgtgtggagcaacatcccagccataaggagcagcaggcactgggctctggtttcggaagaagaattgtccctgctggcccagaacaagcagagctcgaagctcgcggccaagtggcccaccaagctggtgaagaactgctttctccccctaagagaatatttcaagtatttttcaggagggccgagctctggcgcacccccaccaagtggagggtctcctgccgggtccccaacatctactgaagaaggcaccagcgaatccgcaacgcccgagtcaggccctggtacctccacagaaccatctgaaggtagtgcgcctggttccccagctggaagccctacttccaccgaagaaggcacgtcaaccgaaccaagtgaaggatctgcccctgggaccagcactgaaccatctgagccaaaaaagaagagaaaggtaccatctgagatgtccaagggagaggagctgttcaccggagtggtgccaatcctggtggagctggacggcgatgtgaacggccacaagttttctgtgcgcggagagggagagggcgacgcaaccatcggcaagctgacactgaagttcatctgcaccacaggcaagctgcccgtgccttggccaaccctggtgaccacactgacatacggcgtgcagtgtttctctaggtatccagaccacatgaagagacacgatttctttaagagcgccatgccagagggatacgtgcaggagcggaccatctccttcaaggacgatggcaagtataagacccgcgccgtggtgaagtttgagggcgatacactggtgaacaggatcgagctgaagggcaccgacttcaaggaggatggcaatatcctgggccacaagctggagtacaactttaatagccacaacgtgtatatcacagccgacaagcagaagaacggcatcaaggccaacttcaccgtgaggcacaatgtggaggacggctccgtgcagctggccgatcactaccagcagaacacacctatcggcgacggacccgtgctgctgcctgataatcactatctgtccacccagacagtgctgtctaaggacccaaacgagaagtga

SEQ ID NO: 335 - DNA, 7638 bp, synthetic construct
  misc_feature 1..7638: note = CDS of V47_scFv-ZIM3-2a-D3a-hD3L-dCas9-1xGCN4
  source 1..7638: mol_type = other DNA
atggtgcctgccgccaagagagtgaagctggacggaagcggccctgacatcgtgatgacacagagcccttctagcctgagcgccagcgtgggagacagagtgaccatcacctgtagaagcagcacaggcgccgtgaccaccagcaattatgccagctgggtgcaagagaagcccggcaagctgttcaagggactgatcggcggcaccaacaatagagcacctggcgtgccaagcagattcagcggctctctgatcggagacaaggccacactgaccataagcagcctgcagcctgaggacttcgccacctacttttgcgccctgtggtacagcaaccactgggtgttcggccagggcaccaaggtggaactgaaaagaggcggcggaggatctggcggaggtggaagcggaggcggaggttctagtggtggtggcagcgaagtgaaactgctggaaagtggtggcggcctggttcagcctggcggatctctgaaactgagctgtgccgtgtccggcttcagcctgacagattacggcgtgaactgggtccgacaggcccctggaagaggactggaatggatcggagtgatctggggcgacggcatcaccgactacaatagcgccctgaaggaccggttcatcatcagcaaggacaacggcaagaacaccgtgtacctgcagatgagcaaagtgcggagcgacgacacagccctgtactactgtgtgaccggcctgttcgattactggggccagggaacactggtcaccgtgtctagctacccctacgacgtgccagattatgctggtggcggtggtggtagtggtggcggaggaagcggcggaggcggttctggtggcggcggttctcttgatcctggcggtggcggcagcggcatgaacaattctcagggcagagtgacattcgaggacgtgaccgtgaacttcacccaaggcgagtggcagagactgaaccccgagcagagaaacctgtaccgggacgtgatgctggaaaactactccaacctggtgtccgttggccagggcgaaaccaccaagcctgacgtgatcctgagactggaacagggcaaagagccctggctcgaagaggaagaggtgctcggatctggcagagccgagaagaatggcgatattggcggacagatctggaagcccaaggacgtgaaagagagccttggcagcggcgccaccaatttcagcctgctgaaacaggctggcgacgtggaagagaaccccggacctatgcctgccgccaagagagtgaagctggacggcagcaaccacgaccaagagttcgaccctcctaaggtgtaccctcctgtgccagccgagaagcggaagcctatcagagtgctgagcctgttcgacggaatcgccacaggactgctggtgctgaaggatctgggaatccaggtggaccggtatatcgccagcgaagtgtgcgaggacagcatcacagttggcatggttcgacaccagggcaagattatgtacgtgggcgacgtgcggagcgtgacccagaaacacattcaagagtggggccccttcgacctggttatcggcggcagcccttgcaacgatctgagcatcgtgaaccccgccagaaagggcctgtatgaaggcaccggcagactgttcttcgagttctacagactgctgcacgacgccagacctaaagagggcgacgacagaccattcttctggctgttcgagaacgtggtggctatgggcgtgtccgacaagcgggacatcagccggtttctggaaagcaaccccgtgatgatcgacgccaaagaggtgtccgctgctcaccgggccagatacttttggggcaatctgcccggcatgaacagacctctggccagcaccgtgaacgacaagctggaactgcaagagtgcctggaacacggccggatcgccaagtttagcaaagtgcggaccatcaccaccaggtccaacagcatcaagcagggcaaagaccagcacttccccgtgttcatgaatgagaaagaggacatcctgtggtgcaccgagatggaaagagtgttcggcttccctgtgcactacaccgacgtgtccaacatgagcagactggccagacagaggctgctgggcagatcttggagcgtgccagtgatcagacacctgttcgcccctctgaaagaatacttcgcctgcgtgtccagcggcaacagcaacgccaatagcagaggccctagcttcagctctggactggtgcctttgagcctgagaggcagccacatgttcgagacagtgcctgtgtggcggagacagcccgttagagtgctgtccctgtttgaggacatcaagaaagagctgaccagcctgggcttcctggaaagcggatctgatcctggccagctgaagcacgtggtggacgtgaccgataccgtgcggaaggatgtggaagaatggggcccttttgatctggtgtacggcgccacacctcctctgggccacacatgtgatagacctccaagctggtatctgttccagttccaccggctgctgcagtacgctagacccaagcctggaagccccaggcctttcttttggatgttcgtggacaacctggtcctgaacaaagaggacctggacgtcgccagccggttcctcgaaatggaacctgtgacaatccccgacgtgcacggcggatctctgcagaatgctgtcagagtgtggtctaacatccccgccatcagaagcagcagacactgggcccttgtgtccgaggaagaactgtctctgctggcccagaacaagcagagcagcaagctggccgccaagtggcctacaaagctggtcaagaactgcttcctgcctctgcgcgagtacttcaagtatttcagcggcggacctagctctggcgcccctccacctagcggaggatctccagcaggatctcctaccagcaccgaggaaggcacaagcgagtctgccacacctgagtctggccctggcacatctacagagcctagcgagggatctgcccctggatctcctgctggcagccctacatctaccgaagagggaaccagcacagagccttccgaaggttctgctcctggcacaagcaccgagccaagcgagcctaagaagaagagaaaagtcggcagcgacaagaagtacagcatcggcctggccatcggcaccaactctgtgggctgggccgtgatcaccgacgagtacaaggtgcccagcaagaaattcaaggtgctgggcaacaccgaccggcacagcatcaagaagaacctgatcggcgccctgctgttcgacagcggagaaacagccgaggccacccggctgaagagaaccgccagaagaagatacaccagacggaagaaccggatctgctatctgcaagagatcttcagcaacgagatggccaaggtggacgacagcttcttccacagactggaagagtccttcctggtggaagaggataagaagcacgagcggcaccccatcttcggcaacatcgtggacgaggtggcctaccacgagaagtaccccaccatctaccacctgagaaagaaactggtggacagcaccgacaaggccgacctgcggctgatctatctggccctggcccacatgatcaagttccggggccacttcctgatcgagggcgacctgaaccccgacaacagcgacgtggacaagctgttcatccagctggtgcagacctacaaccagctgttcgaggaaaaccccatcaacgccagcggcgtggacgccaaggccatcctgtctgccagactgagcaagagcagacggctggaaaatctgatcgcccagctgcccggcgagaagaagaatggcctgttcggcaacctgattgccctgagcctgggcctgacccccaacttcaagagcaacttcgacctggccgaggatgccaaactgcagctgagcaaggacacctacgacgacgacctggacaacctgctggcccagatcggcgaccagtacgccgacctgtttctggccgccaagaacctgtccgacgccatcctgctgagcgacatcctgagagtgaacaccgagatcaccaaggcccccctgagcgcctctatgatcaagagatacgacgagcaccaccaggacctgaccctgctgaaagctctcgtgcggcagcagctgcctgagaagtacaaagagattttcttcgaccagagcaagaacggctacgccggctacatcgatggcggagccagccaggaagagttctacaagttcatcaagcccatcctggaaaagatggacggcaccgaggaactgctcgtgaagctgaacagagaggacctgctgcggaagcagcggaccttcgacaacggcagcatcccccaccagatccacctgggagagctgcacgccattctgcggcggcaggaagatttttacccattcctgaaggacaaccgggaaaagatcgagaagatcctgaccttccgcatcccctactacgtgggccctctggccaggggaaacagcagattcgcctggatgaccagaaagagcgaggaaaccatcaccccctggaacttcgaggaagtggtggacaagggcgccagcgcccagagcttcatcgagcggatgaccaacttcgataagaacctgcccaacgagaaggtgctgcccaagcacagcctgctgtacgagtacttcaccgtgtacaacgagctgaccaaagtgaaatacgtgaccgagggaatgagaaagcccgccttcctgagcggcgagcagaaaaaagccatcgtggacctgctgttcaagaccaaccggaaagtgaccgtgaagcagctgaaagaggactacttcaagaaaatcgagtgcttcgactccgtggaaatctccggcgtggaagatcggttcaacgcctccctgggcacataccacgatctgctgaaaattatcaaggacaaggacttcctggacaatgaggaaaacgaggacattctggaagatatcgtgctgaccctgacactgtttgaggacagagagatgatcgaggaacggctgaaaacctatgcccacctgttcgacgacaaagtgatgaagcagctgaagcggcggagatacaccggctggggcaggctgagccggaagctgatcaacggcatccgggacaagcagtccggcaagacaatcctggatttcctgaagtccgacggcttcgccaacagaaacttcatgcagctgatccacgacgacagcctgacctttaaagaggacatccagaaagcccaggtgtccggccagggcgatagcctgcacgagcacattgccaatctggccggcagccccgccattaagaagggcatcctgcagacagtgaaggtggtggacgagctcgtgaaagtgatgggccggcacaagcccgagaacatcgtgatcgaaatggccagagagaaccagaccacccagaagggacagaagaacagccgcgagagaatgaagcggatcgaagagggcatcaaagagctgggcagccagatcctgaaagaacaccccgtggaaaacacccagctgcagaacgagaagctgtacctgtactacctgcagaatgggcgggatatgtacgtggaccaggaactggacatcaaccggctgtccgactacgatgtggacgctatcgtgcctcagagctttctgaaggacgactccatcgataacaaagtgctgactcggagcgacaagaaccggggcaagagcgacaacgtgccctccgaagaggtcgtgaagaagatgaagaactactggcgccagctgctgaatgccaagctgattacccagaggaagttcgacaatctgaccaaggccgagagaggcggcctgagcgaactggataaggccggcttcatcaagagacagctggtggaaacccggcagatcacaaagcacgtggcacagatcctggactcccggatgaacactaagtacgacgagaacgacaaactgatccgggaagtgaaagtgatcaccctgaagtccaagctggtgtccgatttccggaaggatttccagttttacaaagtgcgcgagatcaacaactaccaccacgcccacgacgcctacctgaacgccgtcgtgggaaccgccctgatcaaaaagtaccctaagctggaaagcgagttcgtgtacggcgactacaaggtgtacgacgtgcggaagatgatcgccaagagcgagcaggaaatcggcaaggctaccgccaagtacttcttctacagcaacatcatgaactttttcaagaccgagattaccctggccaacggcgagatccggaagcggcctctgatcgagacaaacggcgaaacaggcgagatcgtgtgggataagggccgggactttgccaccgtgcggaaagtgctgtctatgccccaagtgaatatcgtgaaaaagaccgaggtgcagacaggcggcttcagcaaagagtctatcctgcccaagaggaacagcgacaagctgatcgccagaaagaaggactgggaccctaagaagtacggcggcttcgacagccccaccgtggcctattctgtgctggtggtggccaaagtggaaaagggcaagtccaagaaactgaagagtgtgaaagagctgctggggatcaccatcatggaaagaagcagcttcgagaagaatcccatcgactttctggaagccaagggctacaaagaagtgaaaaaggacctgatcatcaagctgcctaagtactccctgttcgagctggaaaacggccggaagagaatgctggcctctgccggcgaactgcagaagggaaacgaactggccctgccctccaaatatgtgaacttcctgtacctggccagccactatgagaagctgaagggctcccccgaggataatgagcagaaacagctgtttgtggaacagcacaaacactacctggacgagatcatcgagcagatcagcgagttctccaagagagtgatcctggccgacgctaatctggacaaggtgctgagcgcctacaacaagcacagagacaagcctatcagagagcaggccgagaatatcatccacctgtttaccctgaccaatctgggagcccctgccgccttcaagtactttgacaccaccatcgaccggaagaggtacaccagcaccaaagaggtgctggacgccaccctgatccaccagagcatcaccggcctgtacgagacacggatcgacctgtctcagctgggaggcgacgcctatccctatgacgtgcccgattatgccagcctgggcagcggctcccccaagaaaaaacgcaaggtggaagatcctaagaaaaagcggaaagtggacggcatcggctccggctctaatggatctagcggagaggaactcctgtccaagaactaccaccttgagaacgaagtggcccgactcaagaaaggctctggtagcggaggctcaggttccggcggatcaggcagtggttctggcggttccggctcaggcggtagtggcagtggcgaagaacttctgagcaaaaactaccacggctctggctccggacagcggggctctaaaagaacagccgacggcagcgagtttgagagccctaaaaagaaaagaaaagtgtga

SEQ ID NO: 336 - DNA, 20 bp, synthetic construct
  misc_feature 1..20: note = sg1(sgPtp1b-1)
  source 1..20: mol_type = other DNA
ggagatggagaaggagttcg

SEQ ID NO: 337 - DNA, 20 bp, synthetic construct
  misc_feature 1..20: note = sg2(sgPtp1b-2)
  source 1..20: mol_type = other DNA
tgactggtcctcccgtacag

SEQ ID NO: 338 - protein, 7 aa, synthetic construct
  REGION 1..7: note = NLS-1
PKKKRKV

SEQ ID NO: 339 - protein, 18 aa, synthetic construct
  REGION 1..18: note = NLS-2
KRTADGSEFESPKKKRKV

SEQ ID NO: 340 - protein, 9 aa, synthetic construct
  REGION 1..9: note = NLS-3
PAAKRVKLD

SEQ ID NO: 341 - DNA, 20 bp, synthetic construct
  misc_feature 1..20: note = sg1(PCSK9)
  source 1..20: mol_type = other DNA
aacctgatcctttagtaccg

SEQ ID NO: 342 - DNA, 20 bp, synthetic construct
  misc_feature 1..20: note = sg2(PCSK9)
  source 1..20: mol_type = other DNA
ggccccggtactaaaggatc

SEQ ID NO: 343 - protein, 796 aa, synthetic construct
  REGION 1..796: note = TALE HPT8
VDLRTLGYSQQQQEKIKPKVRSTVAQHHEALVGHGFTHAHIVALSQHPAALGTVAVKYQDMIAALPEATHEAIVGVGKQWSGARALEALLTVAGELRGPPLQLDTGQLLKIAKRGGVTAVEAVHAWRNALTGAPLNLTPDQVVAIASNGGGKQALETVQRLLPVLCQDHGLTPDQVVAIASHDGGKQALETVQRLLPVLCQDHGLTPDQVVAIASNIGGKQALETVQRLLPVLCQDHGLTPDQVVAIASNNGGKQALETVQRLLPVLCQDHGLTPDQVVAIASNGGGKQALETVQRLLPVLCQDHGLTPDQVVAIASNGGGKQALETVQRLLPVLCQDHGLTPDQVVAIASHDGGKQALETVQRLLPVLCQDHGLTPDQVVAIASNIGGKQALETVQRLLPVLCQDHGLTPDQVVAIASNNGGKQALETVQRLLPVLCQDHGLTPDQVVAIASNNGGKQALETVQRLLPVLCQDHGLTPDQVVAIASNNGGKQALETVQRLLPVLCQDHGLTPDQVVAIASNGGGKQALETVQRLLPVLCQDHGLTPDQVVAIASHDGGKQALETVQRLLPVLCQDHGLTPDQVVAIASNGGGKQALETVQRLLPVLCQDHGLTPDQVVAIASNNGGKQALETVQRLLPVLCQDHGLTPDQVVAIASNIGGKQALETVQRLLPVLCQDHGLTPDQVVAIASNNGGKQALETVQRLLPVLCQDHGLTPDQVVAIASHDGGKQALESIVAQLSRPDPALAALTNDHLVALACLGGRPAMDAVKKGLPHAPELIRRVNRRIGERTSHRV

SEQ ID NO: 344 - protein, 796 aa, synthetic construct
  REGION 1..796: note = TALE HPT12
VDLRTLGYSQQQQEKIKPKVRSTVAQHHEALVGHGFTHAHIVALSQHPAALGTVAVKYQDMIAALPEATHEAIVGVGKQWSGARALEALLTVAGELRGPPLQLDTGQLLKIAKRGGVTAVEAVHAWRNALTGAPLNLTPDQVVAIASNNGGKQALETVQRLLPVLCQDHGLTPDQVVAIASNNGGKQALETVQRLLPVLCQDHGLTPDQVVAIASNIGGKQALETVQRLLPVLCQDHGLTPDQVVAIASNNGGKQALETVQRLLPVLCQDHGLTPDQVVAIASNNGGKQALETVQRLLPVLCQDHGLTPDQVVAIASNIGGKQALETVQRLLPVLCQDHGLTPDQVVAIASNNGGKQALETVQRLLPVLCQDHGLTPDQVVAIASNGGGKQALETVQRLLPVLCQDHGLTPDQVVAIASNNGGKQALETVQRLLPVLCQDHGLTPDQVVAIASNIGGKQALETVQRLLPVLCQDHGLTPDQVVAIASNNGGKQALETVQRLLPVLCQDHGLTPDQVVAIASHDGGKQALETVQRLLPVLCQDHGLTPDQVVAIASHDGGKQALETVQRLLPVLCQDHGLTPDQVVAIASNIGGKQALETVQRLLPVLCQDHGLTPDQVVAIASNNGGKQALETVQRLLPVLCQDHGLTPDQVVAIASNNGGKQALETVQRLLPVLCQDHGLTPDQVVAIASHDGGKQALETVQRLLPVLCQDHGLTPDQVVAIASNIGGKQALESIVAQLSRPDPALAALTNDHLVALACLGGRPAMDAVKKGLPHAPELIRRVNRRIGERTSHRV

SEQ ID NO: 345 - protein, 1973 aa, synthetic construct
  REGION 1..1973: note = V48_scFv-ZIM3-P2A-D3a-hD3L-XTEN80-TALE HPT8-1xGCN4
  SITE 1973: note = misc_feature - Xaa =
MPAAKRVKLDGSGPDIVMTQSPSSLSASVGDRVTITCRSSTGAVTTSNYASWVQEKPGKLFKGLIGGTNNRAPGVPSRFSGSLIGDKATLTISSLQPEDFATYFCALWYSNHWVFGQGTKVELKRGGGGSGGGGSGGGGSSGGGSEVKLLESGGGLVQPGGSLKLSCAVSGFSLTDYGVNWVRQAPGRGLEWIGVIWGDGITDYNSALKDRFIISKDNGKNTVYLQMSKVRSDDTALYYCVTGLFDYWGQGTLVTVSSYPYDVPDYAGGGGGSGGGGSGGGGSGGGGSLDPGGGGSGMNNSQGRVTFEDVTVNFTQGEWQRLNPEQRNLYRDVMLENYSNLVSVGQGETTKPDVILRLEQGKEPWLEEEEVLGSGRAEKNGDIGGQIWKPKDVKESLGSGATNFSLLKQAGDVEENPGPMPAAKRVKLDGSNHDQEFDPPKVYPPVPAEKRKPIRVLSLFDGIATGLLVLKDLGIQVDRYIASEVCEDSITVGMVRHQGKIMYVGDVRSVTQKHIQEWGPFDLVIGGSPCNDLSIVNPARKGLYEGTGRLFFEFYRLLHDARPKEGDDRPFFWLFENVVAMGVSDKRDISRFLESNPVMIDAKEVSAAHRARYFWGNLPGMNRPLASTVNDKLELQECLEHGRIAKFSKVRTITTRSNSIKQGKDQHFPVFMNEKEDILWCTEMERVFGFPVHYTDVSNMSRLARQRLLGRSWSVPVIRHLFAPLKEYFACVSSGNSNANSRGPSFSSGLVPLSLRGSHMFETVPVWRRQPVRVLSLFEDIKKELTSLGFLESGSDPGQLKHVVDVTDTVRKDVEEWGPFDLVYGATPPLGHTCDRPPSWYLFQFHRLLQYARPKPGSPRPFFWMFVDNLVLNKEDLDVASRFLEMEPVTIPDVHGGSLQNAVRVWSNIPAIRSSRHWALVSEEELSLLAQNKQSSKLAAKWPTKLVKNCFLPLREYFKYFSGGPSSGAPPPSGGSPAGSPTSTEEGTSESATPESGPGTSTEPSEGSAPGSPAGSPTSTEEGTSTEPSEGSAPGTSTEPSEPKKKRKVMVDLRTLGYSQQQQEKIKPKVRSTVAQHHEALVGHGFTHAHIVALSQHPAALGTVAVKYQDMIAALPEATHEAIVGVGKQWSGARALEALLTVAGELRGPPLQLDTGQLLKIAKRGGVTAVEAVHAWRNALTGAPLNLTPDQVVAIASNGGGKQALETVQRLLPVLCQDHGLTPDQVVAIASHDGGKQALETVQRLLPVLCQDHGLTPDQVVAIASNIGGKQALETVQRLLPVLCQDHGLTPDQVVAIASNNGGKQALETVQRLLPVLCQDHGLTPDQVVAIASNGGGKQALETVQRLLPVLCQDHGLTPDQVVAIASNGGGKQALETVQRLLPVLCQDHGLTPDQVVAIASHDGGKQALETVQRLLPVLCQDHGLTPDQVVAIASNIGGKQALETVQRLLPVLCQDHGLTPDQVVAIASNNGGKQALETVQRLLPVLCQDHGLTPDQVVAIASNNGGKQALETVQRLLPVLCQDHGLTPDQVVAIASNNGGKQALETVQRLLPVLCQDHGLTPDQVVAIASNGGGKQALETVQRLLPVLCQDHGLTPDQVVAIASHDGGKQALETVQRLLPVLCQDHGLTPDQVVAIASNGGGKQALETVQRLLPVLCQDHGLTPDQVVAIASNNGGKQALETVQRLLPVLCQDHGLTPDQVVAIASNIGGKQALETVQRLLPVLCQDHGLTPDQVVAIASNNGGKQALETVQRLLPVLCQDHGLTPDQVVAIASHDGGKQALESIVAQLSRPDPALAALTNDHLVALACLGGRPAMDAVKKGLPHAPELIRRVNRRIGERTSHRVAYPYDVPDYASLGSGSPKKKRKVEDPKKKRKVDGIGSGSNGSSGEELLSKNYHLENEVARLKKGSGSGGSGSGGSGSGSGGSGSGGSGSGEELLSKNYHGSGSGQRGSKRTADGSEFESPKKKRKVX

SEQ ID NO: 346 - protein, 1973 aa, synthetic construct
  REGION 1..1973: note = V49_scFv-ZIM3-P2A-D3a-hD3L-XTEN80-TALE HPT12-1xGCN4
  SITE 1973: note = misc_feature - Xaa =
MPAAKRVKLDGSGPDIVMTQSPSSLSASVGDRVTITCRSSTGAVTTSNYASWVQEKPGKLFKGLIGGTNNRAPGVPSRFSGSLIGDKATLTISSLQPEDFATYFCALWYSNHWVFGQGTKVELKRGGGGSGGGGSGGGGSSGGGSEVKLLESGGGLVQPGGSLKLSCAVSGFSLTDYGVNWVRQAPGRGLEWIGVIWGDGITDYNSALKDRFIISKDNGKNTVYLQMSKVRSDDTALYYCVTGLFDYWGQGTLVTVSSYPYDVPDYAGGGGGSGGGGSGGGGSGGGGSLDPGGGGSGMNNSQGRVTFEDVTVNFTQGEWQRLNPEQRNLYRDVMLENYSNLVSVGQGETTKPDVILRLEQGKEPWLEEEEVLGSGRAEKNGDIGGQIWKPKDVKESLGSGATNFSLLKQAGDVEENPGPMPAAKRVKLDGSNHDQEFDPPKVYPPVPAEKRKPIRVLSLFDGIATGLLVLKDLGIQVDRYIASEVCEDSITVGMVRHQGKIMYVGDVRSVTQKHIQEWGPFDLVIGGSPCNDLSIVNPARKGLYEGTGRLFFEFYRLLHDARPKEGDDRPFFWLFENVVAMGVSDKRDISRFLESNPVMIDAKEVSAAHRARYFWGNLPGMNRPLASTVNDKLELQECLEHGRIAKFSKVRTITTRSNSIKQGKDQHFPVFMNEKEDILWCTEMERVFGFPVHYTDVSNMSRLARQRLLGRSWSVPVIRHLFAPLKEYFACVSSGNSNANSRGPSFSSGLVPLSLRGSHMFETVPVWRRQPVRVLSLFEDIKKELTSLGFLESGSDPGQLKHVVDVTDTVRKDVEEWGPFDLVYGATPPLGHTCDRPPSWYLFQFHRLLQYARPKPGSPRPFFWMFVDNLVLNKEDLDVASRFLEMEPVTIPDVHGGSLQNAVRVWSNIPAIRSSRHWALVSEEELSLLAQNKQSSKLAAKWPTKLVKNCFLPLREYFKYFSGGPSSGAPPPSGGSPAGSPTSTEEGTSESATPESGPGTSTEPSEGSAPGSPAGSPTSTEEGTSTEPSEGSAPGTSTEPSEPKKKRKVMVDLRTLGYSQQQQEKIKPKVRSTVAQHHEALVGHGFTHAHIVALSQHPAALGTVAVKYQDMIAALPEATHEAIVGVGKQWSGARALEALLTVAGELRGPPLQLDTGQLLKIAKRGGVTAVEAVHAWRNALTGAPLNLTPDQVVAIASNNGGKQALETVQRLLPVLCQDHGLTPDQVVAIASNNGGKQALETVQRLLPVLCQDHGLTPDQVVAIASNIGGKQALETVQRLLPVLCQDHGLTPDQVVAIASNNGGKQALETVQRLLPVLCQDHGLTPDQVVAIASNNGGKQALETVQRLLPVLCQDHGLTPDQVVAIASNIGGKQALETVQRLLPVLCQDHGLTPDQVVAIASNNGGKQALETVQRLLPVLCQDHGLTPDQVVAIASNGGGKQALETVQRLLPVLCQDHGLTPDQVVAIASNNGGKQALETVQRLLPVLCQDHGLTPDQVVAIASNIGGKQALETVQRLLPVLCQDHGLTPDQVVAIASNNGGKQALETVQRLLPVLCQDHGLTPDQVVAIASHDGGKQALETVQRLLPVLCQDHGLTPDQVVAIASHDGGKQALETVQRLLPVLCQDHGLTPDQVVAIASNIGGKQALETVQRLLPVLCQDHGLTPDQVVAIASNNGGKQALETVQRLLPVLCQDHGLTPDQVVAIASNNGGKQALETVQRLLPVLCQDHGLTPDQVVAIASHDGGKQALETVQRLLPVLCQDHGLTPDQVVAIASNIGGKQALESIVAQLSRPDPALAALTNDHLVALACLGGRPAMDAVKKGLPHAPELIRRVNRRIGERTSHRVAYPYDVPDYASLGSGSPKKKRKVEDPKKKRKVDGIGSGSNGSSGEELLSKNYHLENEVARLKKGSGSGGSGSGGSGSGSGGSGSGGSGSGEELLSKNYHGSGSGQRGSKRTADGSEFESPKKKRKVX

SEQ ID NO: 347 - protein, 2038 aa, synthetic construct
  REGION 1..2038: note = V50_3xGCN4-TALE HPT8-ZIM3-P2A-D3a-hD3L-XTEN80-scFv
  SITE 2038: note = misc_feature - Xaa =
MPAAKRVKLDGSEELLSKNYHLENEVARLKKGSGSGGSGSGGSGSGSGGSGSGGSGSGEELLSKNYHLENEVARLKKGSGSGGSGSGGSGSGSGGSGSGGSGSGEELLSKNYHLENEVARLKKGSGSGGSGSGGSGSGSGGSGSGGSGSGPKKKRKVMVDLRTLGYSQQQQEKIKPKVRSTVAQHHEALVGHGFTHAHIVALSQHPAALGTVAVKYQDMIAALPEATHEAIVGVGKQWSGARALEALLTVAGELRGPPLQLDTGQLLKIAKRGGVTAVEAVHAWRNALTGAPLNLTPDQVVAIASNGGGKQALETVQRLLPVLCQDHGLTPDQVVAIASHDGGKQALETVQRLLPVLCQDHGLTPDQVVAIASNIGGKQALETVQRLLPVLCQDHGLTPDQVVAIASNNGGKQALETVQRLLPVLCQDHGLTPDQVVAIASNGGGKQALETVQRLLPVLCQDHGLTPDQVVAIASNGGGKQALETVQRLLPVLCQDHGLTPDQVVAIASHDGGKQALETVQRLLPVLCQDHGLTPDQVVAIASNIGGKQALETVQRLLPVLCQDHGLTPDQVVAIASNNGGKQALETVQRLLPVLCQDHGLTPDQVVAIASNNGGKQALETVQRLLPVLCQDHGLTPDQVVAIASNNGGKQALETVQRLLPVLCQDHGLTPDQVVAIASNGGGKQALETVQRLLPVLCQDHGLTPDQVVAIASHDGGKQALETVQRLLPVLCQDHGLTPDQVVAIASNGGGKQALETVQRLLPVLCQDHGLTPDQVVAIASNNGGKQALETVQRLLPVLCQDHGLTPDQVVAIASNIGGKQALETVQRLLPVLCQDHGLTPDQVVAIASNNGGKQALETVQRLLPVLCQDHGLTPDQVVAIASHDGGKQALESIVAQLSRPDPALAALTNDHLVALACLGGRPAMDAVKKGLPHAPELIRRVNRRIGERTSHRVAYPYDVPDYASLGSGSPKKKRKVEDPKKKRKVDGSGSETPGTSESATPESMNNSQGRVTFEDVTVNFTQGEWQRLNPEQRNLYRDVMLENYSNLVSVGQGETTKPDVILRLEQGKEPWLEEEEVLGSGRAEKNGDIGGQIWKPKDVKESLLEGSGATNFSLLKQAGDVEENPGPMPAAKRVKLDGSNHDQEFDPPKVYPPVPAEKRKPIRVLSLFDGIATGLLVLKDLGIQVDRYIASEVCEDSITVGMVRHQGKIMYVGDVRSVTQKHIQEWGPFDLVIGGSPCNDLSIVNPARKGLYEGTGRLFFEFYRLLHDARPKEGDDRPFFWLFENVVAMGVSDKRDISRFLESNPVMIDAKEVSAAHRARYFWGNLPGMNRPLASTVNDKLELQECLEHGRIAKFSKVRTITTRSNSIKQGKDQHFPVFMNEKEDILWCTEMERVFGFPVHYTDVSNMSRLARQRLLGRSWSVPVIRHLFAPLKEYFACVSSGNSNANSRGPSFSSGLVPLSLRGSHMFETVPVWRRQPVRVLSLFEDIKKELTSLGFLESGSDPGQLKHVVDVTDTVRKDVEEWGPFDLVYGATPPLGHTCDRPPSWYLFQFHRLLQYARPKPGSPRPFFWMFVDNLVLNKEDLDVASRFLEMEPVTIPDVHGGSLQNAVRVWSNIPAIRSSRHWALVSEEELSLLAQNKQSSKLAAKWPTKLVKNCFLPLREYFKYFSGGPSSGAPPPSGGSPAGSPTSTEEGTSESATPESGPGTSTEPSEGSAPGSPAGSPTSTEEGTSTEPSEGSAPGTSTEPSEPKKKRKVPSEGPDIVMTQSPSSLSASVGDRVTITCRSSTGAVTTSNYASWVQEKPGKLFKGLIGGTNNRAPGVPSRFSGSLIGDKATLTISSLQPEDFATYFCALWYSNHWVFGQGTKVELKRGGGGSGGGGSGGGGSSGGGSEVKLLESGGGLVQPGGSLKLSCAVSGFSLTDYGVNWVRQAPGRGLEWIGVIWGDGITDYNSALKDRFIISKDNGKNTVYLQMSKVRSDDTALYYCVTGLFDYWGQGTLVTVSSYPYDVPDYAGGGGGSGGGGSGGGGSGGGGSX

SEQ ID NO: 348 - protein, 2038 aa, synthetic construct
  REGION 1..2038: note = V51_3xGCN4-TALE HPT12-ZIM3-P2A-D3a-hD3L-XTEN80-scFv
  SITE 2038: note = misc_feature - Xaa =
MPAAKRVKLDGSEELLSKNYHLENEVARLKKGSGSGGSGSGGSGSGSGGSGSGGSGSGEELLSKNYHLENEVARLKKGSGSGGSGSGGSGSGSGGSGSGGSGSGEELLSKNYHLENEVARLKKGSGSGGSGSGGSGSGSGGSGSGGSGSGPKKKRKVMVDLRTLGYSQQQQEKIKPKVRSTVAQHHEALVGHGFTHAHIVALSQHPAALGTVAVKYQDMIAALPEATHEAIVGVGKQWSGARALEALLTVAGELRGPPLQLDTGQLLKIAKRGGVTAVEAVHAWRNALTGAPLNLTPDQVVAIASNNGGKQALETVQRLLPVLCQDHGLTPDQVVAIASNNGGKQALETVQRLLPVLCQDHGLTPDQVVAIASNIGGKQALETVQRLLPVLCQDHGLTPDQVVAIASNNGGKQALETVQRLLPVLCQDHGLTPDQVVAIASNNGGKQALETVQRLLPVLCQDHGLTPDQVVAIASNIGGKQALETVQRLLPVLCQDHGLTPDQVVAIASNNGGKQALETVQRLLPVLCQDHGLTPDQVVAIASNGGGKQALETVQRLLPVLCQDHGLTPDQVVAIASNNGGKQALETVQRLLPVLCQDHGLTPDQVVAIASNIGGKQALETVQRLLPVLCQDHGLTPDQVVAIASNNGGKQALETVQRLLPVLCQDHGLTPDQVVAIASHDGGKQALETVQRLLPVLCQDHGLTPDQVVAIASHDGGKQALETVQRLLPVLCQDHGLTPDQVVAIASNIGGKQALETVQRLLPVLCQDHGLTPDQVVAIASNNGGKQALETVQRLLPVLCQDHGLTPDQVVAIASNNGGKQALETVQRLLPVLCQDHGLTPDQVVAIASHDGGKQALETVQRLLPVLCQDHGLTPDQVVAIASNIGGKQALESIVAQLSRPDPALAALTNDHLVALACLGGRPAMDAVKKGLPHAPELIRRVNRRIGERTSHRVAYPYDVPDYASLGSGSPKKKRKVEDPKKKRKVDGSGSETPGTSESATPESMNNSQGRVTFEDVTVNFTQGEWQRLNPEQRNLYRDVMLENYSNLVSVGQGETTKPDVILRLEQGKEPWLEEEEVLGSGRAEKNGDIGGQIWKPKDVKESLLEGSGATNFSLLKQAGDVEENPGPMPAAKRVKLDGSNHDQEFDPPKVYPPVPAEKRKPIRVLSLFDGIATGLLVLKDLGIQVDRYIASEVCEDSITVGMVRHQGKIMYVGDVRSVTQKHIQEWGPFDLVIGGSPCNDLSIVNPARKGLYEGTGRLFFEFYRLLHDARPKEGDDRPFFWLFENVVAMGVSDKRDISRFLESNPVMIDAKEVSAAHRARYFWGNLPGMNRPLASTVNDKLELQECLEHGRIAKFSKVRTITTRSNSIKQGKDQHFPVFMNEKEDILWCTEMERVFGFPVHYTDVSNMSRLARQRLLGRSWSVPVIRHLFAPLKEYFACVSSGNSNANSRGPSFSSGLVPLSLRGSHMFETVPVWRRQPVRVLSLFEDIKKELTSLGFLESGSDPGQLKHVVDVTDTVRKDVEEWGPFDLVYGATPPLGHTCDRPPSWYLFQFHRLLQYARPKPGSPRPFFWMFVDNLVLNKEDLDVASRFLEMEPVTIPDVHGGSLQNAVRVWSNIPAIRSSRHWALVSEEELSLLAQNKQSSKLAAKWPTKLVKNCFLPLREYFKYFSGGPSSGAPPPSGGSPAGSPTSTEEGTSESATPESGPGTSTEPSEGSAPGSPAGSPTSTEEGTSTEPSEGSAPGTSTEPSEPKKKRKVPSEGPDIVMTQSPSSLSASVGDRVTITCRSSTGAVTTSNYASWVQEKPGKLFKGLIGGTNNRAPGVPSRFSGSLIGDKATLTISSLQPEDFATYFCALWYSNHWVFGQGTKVELKRGGGGSGGGGSGGGGSSGGGSEVKLLESGGGLVQPGGSLKLSCAVSGFSLTDYGVNWVRQAPGRGLEWIGVIWGDGITDYNSALKDRFIISKDNGKNTVYLQMSKVRSDDTALYYCVTGLFDYWGQGTLVTVSSYPYDVPDYAGGGGGSGGGGSGGGGSGGGGSX

SEQ ID NO: 349 - DNA, 9387 bp, synthetic construct
  misc_feature 1..9387: note = DNA of V48_scFv-ZIM3-P2A-D3a-hD3L-XTEN80-TALE HPT8-1xGCN4
  source 1..9387: mol_type = other DNA
tcatatatactttagattgatttaaaacttcatttttaatttaaaaggatctaggtgaagatcctttttgataatctcatgaccaaaatcccttaacgtgagttttcgttccactgagcgtcagaccccgtagaaaagatcaaaggatcttcttgagatcctttttttctgcgcgtaatctgctgcttgcaaacaaaaaaaccaccgctaccagcggtggtttgtttgccggatcaagagctaccaactctttttccgaaggtaactggcttcagcagagcgcagataccaaatactgttcttctagtgtagccgtagttaggccaccacttcaagaactctgtagcaccgcctacatacctcgctctgctaatcctgttaccagtggctgctgccagtggcgataagtcgtgtcttaccgggttggactcaagacgatagttaccggataaggcgcagcggtcgggctgaacggggggttcgtgcacacagcccagcttggagcgaacgacctacaccgaactgagatacctacagcgtgagctatgagaaagcgccacgcttcccgaagggagaaaggcggacaggtatccggtaagcggcagggtcggaacaggagagcgcacgagggagcttccagggggaaacgcctggtatctttatagtcctgtcgggtttcgccacctctgacttgagcgtcgatttttgtgatgctcgtcaggggggcggagcctatggaaaaacgccagcaacgcggcctttttacggttcctggccttttgctggccttttgctcacatgttctttcctgcgttatcccctgattctgtggataaccgtattaccgcctttgagtgagctgataccgctcgccgcagccgaacgaccgagcgcagcgagtcagtgagcgaggaagcggaagagcgcccaatacgcaaaccgcctctccccgcgcgttggccgattcattaatgcagctggcacgacaggtttcccgactggaaagcgggcagtgagcgcaacgcaattaatgtgagttagctcactcattaggcaccccaggctttacactttatgcttccggctcgtatgttgtgtggaattgtgagcggataacaatttcacacaggaaacagctatgaccatgattacgcctctagaaagctttaatacgactcactataaggactcactatttgttttcgcgcccagttgcaaaaagtgtcgacatttgcttctgacacaactgtgttcactagcaacctcaaacagacaccgccaccatgcctgctgctaagagagtgaaactggatggatccggccccgacatcgtgatgacccagagccccagcagcctgagcgccagcgtgggcgaccgcgtgaccatcacctgccgcagcagcaccggcgccgtgaccaccagcaactacgccagctgggtgcaggagaagcccggcaagctgttcaagggcctgatcggcggcaccaacaaccgcgcccccggcgtgcccagccgcttcagcggcagcctgatcggcgacaaggccaccctgaccatcagcagcctgcagcccgaggacttcgccacctacttctgcgccctgtggtacagcaaccactgggtgttcggccagggcaccaaggtggagctgaagcgcggcggcggcggcagcggcggcggcggcagcggcggcggcggcagcagcggcggcggcagcgaggtgaagctgctggagagcggcggcggcctggtgcagcccggcggcagcctgaagctgagctgcgccgtgagcggcttcagcctgaccgactacggcgtgaactgggtgcgccaggcccccggccgcggcctggagtggatcggcgtgatctggggcgacggcatcaccgactacaacagcgccctgaaggaccgcttcatcatcagcaaggacaacggcaagaacaccgtgtacctgcagatgagcaaggtgcgcagcgacgacaccgccctgtactactgcgtgaccggcctgttcgactactggggccagggcaccctggtgaccgtgagcagctacccatacgatgttccagattacgctggtggaggcggaggttctgggggaggaggtagtggcggtggtggttcaggaggcggcggaagcttggatccaggtggaggtggaagcggtatgaacaattcccagggaagagtgaccttcgaggacgtgaccgtgaacttcacccaaggcgagtggcagagactgaaccccgagcagagaaacctgtaccgggacgtgatgctggaaaactacagcaacctggtgtccgtcggccagggcgagacaacaaagcctgacgtgatcctgcggctggaacagggcaaagagccttggctggaagaggaagaggtgctcggatctggcagagccgagaagaatggcgatatcggcggacagatctggaagccaaaggatgtgaaagagagtctcggaagcggagctactaacttcagcctgctgaagcaggctggagacgtggaggagaaccctggacctatgcctgctgctaagagagtgaaactggatggatccaaccatgaccaggaatttgaccccccaaaggtttacccacctgtgccagctgagaagaggaagcccatccgcgtgctgtctctctttgatgggattgctacagggctcctggtgctgaaggacctgggcatccaagtggaccgctacattgcctccgaggtgtgtgaggactccatcacggtgggcatggtgcggcaccagggaaagatcatgtacgtcggggacgtccgcagcgtcacacagaagcatatccaggagtggggcccattcgacctggtgattggaggcagtccctgcaatgacctctccattgtcaaccctgcccgcaagggactttatgagggtactggccgcctcttctttgagttctaccgcctcctgcatgatgcgcggcccaaggagggagatgatcgccccttcttctggctctttgagaatgtggtggccatgggcgttagtgacaagagggacatctcgcgatttcttgagtctaaccccgtgatgattgacgccaaagaagtgtctgctgcacacagggcccgttacttctggggtaaccttcctggcatgaacaggcctttggcatccactgtgaatgataagctggagctgcaagagtgtctggagcacggcagaatagccaagttcagcaaagtgaggaccattaccaccaggtcaaactctataaagcagggcaaagaccagcatttccccgtgttcatgaacgagaaggaggacatcctgtggtgcactgaaatggaaagggtgtttggcttccccgtccactacacagacgtctccaacatgagccgcttggcgaggcagagactgctgggccgatcgtggagcgtgccggtcatccgccacctcttcgctccgctgaaggaatattttgcttgtgtgtctagcggcaatagtaacgctaacagccgcgggccgagcttcagcagcggcctggtgccgttaagcttgcgcggcagccatatgttcgaaaccgtgcctgtgtggaggagacagccagtccgggtgctgtccctttttgaagacatcaagaaagagctgacgagtttgggctttttggaaagtggttctgacccgggacaactgaagcatgtggttgatgtcacagacacagtgaggaaggatgtggaggagtggggacccttcgatcttgtgtacggcgccacacctcccctgggccacacctgtgaccgtcctcccagctggtacctgttccagttccaccggctcctgcagtacgcacggcccaagccaggcagccccaggcccttcttctggatgttcgtggacaatctggtgctgaacaaggaagacctggacgtcgcatctcgcttcctggagatggagccagtcaccatcccagatgtccacggcggatccttgcagaatgctgtccgcgtgtggagcaacatcccagccataaggagcagcaggcactgggctctggtttcggaagaagaattgtccctgctggcccagaacaagcagagctcgaagctcgcggccaagtggcccaccaagctggtgaagaactgctttctccccctaagagaatatttcaagtatttttcaggagggccgagctctggcgcacccccaccaagtggagggtctcctgccgggtccccaacatctactgaagaaggcaccagcgaatccgcaacgcccgagtcaggccctggtacctccacagaaccatctgaaggtagtgcgcctggttccccagctggaagccctacttccaccgaagaaggcacgtcaaccgaaccaagtgaaggatctgcccctgggaccagcactgaaccatctgagccaaaaaagaagagaaaggtaatggtggatctacgcacgctcggctacagccagcagcaacaggagaagatcaaaccgaaggttcgttcgacagtggcgcagcaccacgaggcactggtcggccatgggtttacacacgcgcacatcgttgcgctcagccaacacccggcagcgttagggaccgtcgctgtcaagtatcaggacatgatcgcagcgttgccagaggcgacacacgaagcgatcgttggcgtcggcaaacagtggtccggcgcacgcgctctggaggccttgctcacggtggcgggagagttgagaggtccaccgttacagttggacacaggccaacttctcaagattgcaaaacgtggcggcgtgaccgcagtggaggcagtgcatgcatggcgcaatgcactgacgggtgcccccctgaacctgaccccggaccaagtggtggctatcgccagcaacggtggcggcaagcaagcgctcgaaacggtgcagcggctgttgccggtgctgtgccaggaccatggcctgactccggaccaagtggtggctatcgccagccacgatggcggcaagcaagcgctcgaaacggtgcagcggctgttgccggtgctgtgccaggaccatggcctgaccccggaccaagtggtggctatcgccagcaacattggcggcaagcaagcgctcgaaacggtgcagcggctgttgccggtgctgtgccaggaccatggcctgaccccggaccaagtggtggctatcgccagcaacaatggcggcaagcaagcgctcgaaacggtgcagcggctgttgccggtgctgtgccaggaccatggcctgaccccggaccaagtggtggctatcgccagcaacggtggcggcaagcaagcgctcgaaacggtgcagcggctgttgccggtgctgtgccaggaccatggcctgaccccggaccaagtggtggctatcgccagcaacggtggcggcaagcaagcgctcgaaacggtgcagcggctgttgccggtgctgtgccaggaccatggcctgactccggaccaagtggtggctatcgccagccacgatggcggcaagcaagcgctcgaaacggtgcagcggctgttgccggtgctgtgccaggaccatggcctgaccccggaccaagtggtggctatcgccagcaacattggcggcaagcaagcgctcgaaacggtgcagcggctgttgccggtgctgtgccaggaccatggcctgaccccggaccaagtggtggctatcgccagcaacaatggcggcaagcaagcgctcgaaacggtgcagcggctgttgccggtgctgtgccaggaccatggcctgaccccggaccaagtggtggctatcgccagcaacaatggcggcaagcaagcgctcgaaacggtgcagcggctgttgccggtgctgtgccaggaccatggcctgaccccggaccaagtggtggctatcgccagcaacaatggcggcaagcaagcgctcgaaacggtgcagcggctgttgccggtgctgtgccaggaccatggcctgaccccggaccaagtggtggctatcgccagcaacggtggcggcaagcaagcgctcgaaacggtgcagcggctgttgccggtgctgtgccaggaccatggcctgactccggaccaagtggtggctatcgccagccacgatggcggcaagcaagcgctcgaaacggtgcagcggctgttgccggtgctgtgccaggaccatggcctgaccccggaccaagtggtggctatcgccagcaacggtggcggcaagcaagcgctcgaaacggtgcagcggctgttgccggtgctgtgccaggaccatggcctgaccccggaccaagtggtggctatcgccagcaacaatggcggcaagcaagcgctcgaaacggtgcagcggctgttgccggtgctgtgccaggaccatggcctgaccccggaccaagtggtggctatcgccagcaacattggcggcaagcaagcgctcgaaacggtgcagcggctgttgccggtgctgtgccaggaccatggcctgaccccggaccaagtggtggctatcgccagcaacaatggcggcaagcaagcgctcgaaacggtgcagcggctgttgccggtgctgtgccaggaccatggcctgaccccggaccaagtggtggctatcgccagccacgatggcggcaagcaagcgctcgaaagcattgtggcccagctgagccggcctgatccggcgttggccgcgttgaccaacgaccacctcgtcgccttggcctgcctcggcggacgtcctgccatggatgcagtgaaaaagggattgccgcacgcgccggaattgatcagaagagtcaatcgccgtattggcgaacgcacgtcccatcgcgttgcctatccctatgacgtgcccgattatgccagcctgggcagcggctcccccaagaaaaaacgcaaggtggaagatcctaagaaaaagcggaaagtggacggcattggtagtgggagcaacggcagcagcggagaggaactgctgagcaagaactaccacctggaaaacgaggtggccagactgaagaaaggctctggctctggcggaagcggttctggcggatcaggatctggaagtggcggctctggaagcggaggttctggatctggcgaagaactgctgtctaagaattatcacggttcaggctccggccagcggggaagcaagcgcaccgccgatggttccgagttcgaaagccccaaaaaaaagcgcaaggtctgagatcccaagcacgcagcaatgcagctcaaaacgcttagcctagccacacccccacgggaaacagcagtgattaacctttagcaataaacgaaagtttaactaagctatactaaccccagggttggtcaatttcgtgccagccacaccctggtactgcatgcacgcaatgctagctgcccctttcccgtcctgggcaccccgagtctcccccgaccccgggtcccaggtatgctcccacctccacctgccccactcaccacctctgctagttccagacacctccgagacgaggaaaaaaaaaaaaaaaaaaaaaaaaaaaaaaaaaaaaaaaaaaaaaaaaaaaaaaaaaaaaaaaaaaaaaaaaaaaaaaaaaaaaaaaaaaaaaaaaaaaaaaaaaaaaaaaaaaaaaaaaaaaaaaaaaaaaaaaaaaaaaaaaaaaaaaaaaaaaaaaaaaaaaaaaaaaaaaaaaaaaaaaaaaaaaaaaaaaaaaaaaaaaaaaaaaaaaaaaaaaaaaaaaaaaaaaaaaaaaaaaaaaaaaaaaaaaaaaaaaaaaaaaaaaaaaaaaaaaaaaaaaaaaaaaaaaaaaaaaaaaaaaaaaaaaaaaaaaaaaaaaaaaaaaaaaaaaaaaaaaaaaaaaaaaaaaaaaaaaaaaaaaaaaaaaaaaaaaaaaaaaaaaaaaaaaaaaaccgtcttcaagctttctagaaattcactggccgtcgttttacaacgtcgtgactgggaaaaccctggcgttacccaacttaatcgccttgcagcacatccccctttcgccagctggcgtaatagcgaagaggcccgcaccgatcgcccttcccaacagttgcgcagcctgaatggcgaatggcgcctgatgcggtattttctccttacgcatctgtgcggtatttcacaccgcatatggtgcactctcagtacaatctgctctgatgccgcatagttaagccagccccgacacccgccaacacccgctgacgcgccctgacgggcttgtctgctcccggcatccgcttacagacaagctgtgaccgtctccgggagctgcatgtgtcagaggttttcaccgtcatcaccgaaacgcgcgagacgaaagggcctcgtgatacgcctatttttataggttaatgtcatgataataatggtttcttagacgtcaggtggcacttttcggggaaatgtgcgcggaacccctatttgtttatttttctaaatacattcaaatatgtatccgctcatgagacaataaccctgataaatgcttcaataatattgaaaaaggaagagtatgagtattcaacatttccgtgtcgcccttattcccttttttgcggcattttgccttcctgtttttgctcacccagaaacgctggtgaaagtaaaagatgctgaagatcagttgggtgcacgagtgggttacatcgaactggatctcaacagcggtaagatccttgagagttttcgccccgaagaacgttttccaatgatgagcacttttaaagttctgctatgtggcgcggtattatcccgtattgacgccgggcaagagcaactcggtcgccgcatacactattctcagaatgacttggttgagtactcaccagtcacagaaaagcatcttacggatggcatgacagtaagagaattatgcagtgctgccataaccatgagtgataacactgcggccaacttacttctgacaacgatcggaggaccgaaggagctaaccgcttttttgcacaacatgggggatcatgtaactcgccttgatcgttgggaaccggagctgaatgaagccataccaaacgacgagcgtgacaccacgatgcctgtagcaatggcaacaacgttgcgcaaactattaactggcgaactacttactctagcttcccggcaacaattaatagactggatggaggcggataaagttgcaggaccacttctgcgctcggcccttccggctggctggtttattgctgataaatctggagccggtgagcgtgggtctcgcggtatcattgcagcactggggccagatggtaagccctcccgtatcgtagttatctacacgacggggagtcaggcaactatggatgaacgaaatagacagatcgctgagataggtgcctcactgattaagcattggtaactgtcagaccaagtttac

SEQ ID NO: 350 - DNA, 9387 bp, synthetic construct
  misc_feature 1..9387: note = DNA of V49_scFv-ZIM3-P2A-D3a-hD3L-XTEN80-TALE HPT12-1xGCN4
  source 1..9387: mol_type = other DNA
tcatatatactttagattgatttaaaacttcatttttaatttaaaaggatctaggtgaagatcctttttgataatctcatgaccaaaatcccttaacgtgagttttcgttccactgagcgtcagaccccgtagaaaagatcaaaggatcttcttgagatcctttttttctgcgcgtaatctgctgcttgcaaacaaaaaaaccaccgctaccagcggtggtttgtttgccggatcaagagctaccaactctttttccgaaggtaactggcttcagcagagcgcagataccaaatactgttcttctagtgtagccgtagttaggccaccacttcaagaactctgtagcaccgcctacatacctcgctctgctaatcctgttaccagtggctgctgccagtggcgataagtcgtgtcttaccgggttggactcaagacgatagttaccggataaggcgcagcggtcgggctgaacggggggttcgtgcacacagcccagcttggagcgaacgacctacaccgaactgagatacctacagcgtgagctatgagaaagcgccacgcttcccgaagggagaaaggcggacaggtatccggtaagcggcagggtcggaacaggagagcgcacgagggagcttccagggggaaacgcctggtatctttatagtcctgtcgggtttcgccacctctgacttgagcgtcgatttttgtgatgctcgtcaggggggcggagcctatggaaaaacgccagcaacgcggcctttttacggttcctggccttttgctggccttttgctcacatgttctttcctgcgttatcccctgattctgtggataaccgtattaccgcctttgagtgagctgataccgctcgccgcagccgaacgaccgagcgcagcgagtcagtgagcgaggaagcggaagagcgcccaatacgcaaaccgcctctccccgcgcgttggccgattcattaatgcagctggcacgacaggtttcccgactggaaagcgggcagtgagcgcaacgcaattaatgtgagttagctcactcattaggcaccccaggctttacactttatgcttccggctcgtatgttgtgtggaattgtgagcggataacaatttcacacaggaaacagctatgaccatgattacgcctctagaaagctttaatacgactcactataaggactcactatttgttttcgcgcccagttgcaaaaagtgtcgacatttgcttctgacacaactgtgttcactagcaacctcaaacagacaccgccaccatgcctgctgctaagagagtgaaactggatggatccggccccgacatcgtgatgacccagagccccagcagcctgagcgccagcgtgggcgaccgcgtgaccatcacctgccgcagcagcaccggcgccgtgaccaccagcaactacgccagctgggtgcaggagaagcccggcaagctgttcaagggcctgatcggcggcaccaacaaccgcgcccccggcgtgcccagccgcttcagcggcagcctgatcggcgacaaggccaccctgaccatcagcagcctgcagcccgaggacttcgccacctacttctgcgccctgtggtacagcaaccactgggtgttcggccagggcaccaaggtggagctgaagcgcggcggcggcggcagcggcggcggcggcagcggcggcggcggcagcagcggcggcggcagcgaggtgaagctgctggagagcggcggcggcctggtgcagcccggcggcagcctgaagctgagctgcgccgtgagcggcttcagcctgaccgactacggcgtgaactgggtgcgccaggcccccggccgcggcctggagtggatcggcgtgatctggggcgacggcatcaccgactacaacagcgccctgaaggaccgcttcatcatcagcaaggacaacggcaagaacaccgtgtacctgcagatgagcaaggtgcgcagcgacgacaccgccctgtactactgcgtgaccggcctgttcgactactggggccagggcaccctggtgaccgtgagcagctacccatacgatgttccagattacgctggtggaggcggaggttctgggggaggaggtagtggcggtggtggttcaggaggcggcggaagcttggatccaggtggaggtggaagcggtatgaacaattcccagggaagagtgaccttcgaggacgtgaccgtgaacttcacccaaggcgagtggcagagactgaaccccgagcagagaaacctgtaccgggacgtgatgctggaaaactacagcaacctggtgtccgtcggccagggcgagacaacaaagcctgacgtgatcctgcggctggaacagggcaaagagccttggctggaagaggaagaggtgctcggatctggcagagccgagaagaatggcgatatcggcggacagatctggaagccaaaggatgtgaaagagagtctcggaagcggagctactaacttcagcctgctgaagcaggctggagacgtggaggagaaccctggacctatgcctgctgctaagagagtgaaactggatggatccaaccatgaccaggaatttgaccccccaaaggtttacccacctgtgccagctgagaagaggaagcccatccgcgtgctgtctctctttgatgggattgctacagggctcctggtgctgaaggacctgggcatccaagtggaccgctacattgcctccgaggtgtgtgaggactccatcacggtgggcatggtgcggcaccagggaaagatcatgtacgtcggggacgtccgcagcgtcacacagaagcatatccaggagtggggcccattcgacctggtgattggaggcagtccctgcaatgacctctccattgtcaaccctgcccgcaagggactttatgagggtactggccgcctcttctttgagttctaccgcctcctgcatgatgcgcggcccaaggagggagatgatcgccccttcttctggctctttgagaatgtggtggccatgggcgttagtgacaagagggacatctcgcgatttcttgagtctaaccccgtgatgattgacgccaaagaagtgtctgctgcacacagggcccgttacttctggggtaaccttcctggcatgaacaggcctttggcatccactgtgaatgataagctggagctgcaagagtgtctggagcacggcagaatagccaagttcagcaaagtgaggaccattaccaccaggtcaaactctataaagcagggcaaagaccagcatttccccgtgttcatgaacgagaaggaggacatcctgtggtgcactgaaatggaaagggtgtttggcttccccgtccactacacagacgtctccaacatgagccgcttggcgaggcagagactgctgggccgatcgtggagcgtgccggtcatccgccacctcttcgctccgctgaaggaatattttgcttgtgtgtctagcggcaatagtaacgctaacagccgcgggccgagcttcagcagcggcctggtgccgttaagcttgcgcggcagccatatgttcgaaaccgtgcctgtgtggaggagacagccagtccgggtgctgtccctttttgaagacatcaagaaagagctgacgagtttgggctttttggaaagtggttctgacccgggacaactgaagcatgtggttgatgtcacagacacagtgaggaaggatgtggaggagtggggacccttcgatcttgtgtacggcgccacacctcccctgggccacacctgtgaccgtcctcccagctggtacctgttccagttccaccggctcctgcagtacgcacggcccaagccaggcagccccaggcccttcttctggatgttcgtggacaatctggtgctgaacaaggaagacctggacgtcgcatctcgcttcctggagatggagccagtcaccatcccagatgtccacggcggatccttgcagaatgctgtccgcgtgtggagcaacatcccagccataaggagcagcaggcactgggctctggtttcggaagaagaattgtccctgctggcccagaacaagcagagctcgaagctcgcggccaagtggcccaccaagctggtgaagaactgctttctccccctaagagaatatttcaagtatttttcaggagggccgagctctggcgcacccccaccaagtggagggtctcctgccgggtccccaacatctactgaagaaggcaccagcgaatccgcaacgcccgagtcaggccctggtacctccacagaaccatctgaaggtagtgcgcctggttccccagctggaagccctacttccaccgaagaaggcacgtcaaccgaaccaagtgaaggatctgcccctgggaccagcactgaaccatctgagccaaaaaagaagagaaaggtaatggtggatctacgcacgctcggctacagccagcagcaacaggagaagatcaaaccgaaggttcgttcgacagtggcgcagcaccacgaggcactggtcggccatgggtttacacacgcgcacatcgttgcgctcagccaacacccggcagcgttagggaccgtcgctgtcaagtatcaggacatgatcgcagcgttgccagaggcgacacacgaagcgatcgttggcgtcggcaaacagtggtccggcgcacgcgctctggaggccttgctcacggtggcgggagagttgagaggtccaccgttacagttggacacaggccaacttctcaagattgcaaaacgtggcggcgtgaccgcagtggaggcagtgcatgcatggcgcaatgcactgacgggtgcccccctgaacctgaccccggaccaagtggtggctatcgccagcaacaatggcggcaagcaagcgctcgaaacggtgcagcggctgttgccggtgctgtgccaggaccatggcctgaccccggaccaagtggtggctatcgccagcaacaatggcggcaagcaagcgctcgaaacggtgcagcggctgttgccggtgctgtgccaggaccatggcctgaccccggaccaagtggtggctatcgccagcaacattggcggcaagcaagcgctcgaaacggtgcagcggctgttgccggtgctgtgccaggaccatggcctgaccccggaccaagtggtggctatcgccagcaacaatggcggcaagcaagcgctcgaaacggtgcagcggctgttgccggtgctgtgccaggaccatggcctgaccccggaccaagtggtggctatcgccagcaacaatggcggcaagcaagcgctcgaaacggtgcagcggctgttgccggtgctgtgccaggaccatggcctgaccccggaccaagtggtggctatcgccagcaacattggcggcaagcaagcgctcgaaacggtgcagcggctgttgccggtgctgtgccaggaccatggcctgaccccggaccaagtggtggctatcgccagcaacaatggcggcaagcaagcgctcgaaacggtgcagcggctgttgccggtgctgtgccaggaccatggcctgaccccggaccaagtggtggctatcgccagcaacggtggcggcaagcaagcgctcgaaacggtgcagcggctgttgccggtgctgtgccaggaccatggcctgaccccggaccaagtggtggctatcgccagcaacaatggcggcaagcaagcgctcgaaacggtgcagcggctgttgccggtgctgtgccaggaccatggcctgaccccggaccaagtggtggctatcgccagcaacattggcggcaagcaagcgctcgaaacggtgcagcggctgttgccggtgctgtgccaggaccatggcctgaccccggaccaagtggtggctatcgccagcaacaatggcggcaagcaagcgctcgaaacggtgcagcggctgttgccggtgctgtgccaggaccatggcctgactccggaccaagtggtggctatcgccagccacgatggcggcaagcaagcgctcgaaacggtgcagcggctgttgccggtgctgtgccaggaccatggcctgactccggaccaagtggtggctatcgccagccacgatggcggcaagcaagcgctcgaaacggtgcagcggctgttgccggtgctgtgccaggaccatggcctgaccccggaccaagtggtggctatcgccagcaacattggcggcaagcaagcgctcgaaacggtgcagcggctgttgccggtgctgtgccaggaccatggcctgaccccggaccaagtggtggctatcgccagcaacaatggcggcaagcaagcgctcgaaacggtgcagcggctgttgccggtgctgtgccaggaccatggcctgaccccggaccaagtggtggctatcgccagcaacaatggcggcaagcaagcgctcgaaacggtgcagcggctgttgccggtgctgtgccaggaccatggcctgactccggaccaagtggtggctatcgccagccacgatggcggcaagcaagcgctcgaaacggtgcagcggctgttgccggtgctgtgccaggaccatggcctgaccccggaccaagtggtggctatcgccagcaacattggcggcaagcaagcgctcgaaagcattgtggcccagctgagccggcctgatccggcgttggccgcgttgaccaacgaccacctcgtcgccttggcctgcctcggcggacgtcctgccatggatgcagtgaaaaagggattgccgcacgcgccggaattgatcagaagagtcaatcgccgtattggcgaacgcacgtcccatcgcgttgcctatccctatgacgtgcccgattatgccagcctgggcagcggctcccccaagaaaaaacgcaaggtggaagatcctaagaaaaagcggaaagtggacggcattggtagtgggagcaacggcagcagcggagaggaactgctgagcaagaactaccacctggaaaacgaggtggccagactgaagaaaggctctggctctggcggaagcggttctggcggatcaggatctggaagtggcggctctggaagcggaggttctggatctggcgaagaactgctgtctaagaattatcacggttcaggctccggccagcggggaagcaagcgcaccgccgatggttccgagttcgaaagccccaaaaaaaagcgcaaggtctgagatcccaagcacgcagcaatgcagctcaaaacgcttagcctagccacacccccacgggaaacagcagtgattaacctttagcaataaacgaaagtttaactaagctatactaaccccagggttggtcaatttcgtgccagccacaccctggtactgcatgcacgcaatgctagctgcccctttcccgtcctgggcaccccgagtctcccccgaccccgggtcccaggtatgctcccacctccacctgccccactcaccacctctgctagttccagacacctccgagacgaggaaaaaaaaaaaaaaaaaaaaaaaaaaaaaaaaaaaaaaaaaaaaaaaaaaaaaaaaaaaaaaaaaaaaaaaaaaaaaaaaaaaaaaaaaaaaaaaaaaaaaaaaaaaaaaaaaaaaaaaaaaaaaaaaaaaaaaaaaaaaaaaaaaaaaaaaaaaaaaaaaaaaaaaaaaaaaaaaaaaaaaaaaaaaaaaaaaaaaaaaaaaaaaaaaaaaaaaaaaaaaaaaaaaaaaaaaaaaaaaaaaaaaaaaaaaaaaaaaaaaaaaaaaaaaaaaaaaaaaaaaaaaaaaaaaaaaaaaaaaaaaaaaaaaaaaaaaaaaaaaaaaaaaaaaaaaaaaaaaaaaaaaaaaaaaaaaaaaaaaaaaaaaaaaaaaaaaaaaaaaaaaaaaaaaaaaaaccgtcttcaagctttctagaaattcactggccgtcgttttacaacgtcgtgactgggaaaaccctggcgttacccaacttaatcgccttgcagcacatccccctttcgccagctggcgtaatagcgaagaggcccgcaccgatcgcccttcccaacagttgcgcagcctgaatggcgaatggcgcctgatgcggtattttctccttacgcatctgtgcggtatttcacaccgcatatggtgcactctcagtacaatctgctctgatgccgcatagttaagccagccccgacacccgccaacacccgctgacgcgccctgacgggcttgtctgctcccggcatccgcttacagacaagctgtgaccgtctccgggagctgcatgtgtcagaggttttcaccgtcatcaccgaaacgcgcgagacgaaagggcctcgtgatacgcctatttttataggttaatgtcatgataataatggtttcttagacgtcaggtggcacttttcggggaaatgtgcgcggaacccctatttgtttatttttctaaatacattcaaatatgtatccgctcatgagacaataaccctgataaatgcttcaataatattgaaaaaggaagagtatgagtattcaacatttccgtgtcgcccttattcccttttttgcggcattttgccttcctgtttttgctcacccagaaacgctggtgaaagtaaaagatgctgaagatcagttgggtgcacgagtgggttacatcgaactggatctcaacagcggtaagatccttgagagttttcgccccgaagaacgttttccaatgatgagcacttttaaagttctgctatgtggcgcggtattatcccgtattgacgccgggcaagagcaactcggtcgccgcatacactattctcagaatgacttggttgagtactcaccagtcacagaaaagcatcttacggatggcatgacagtaagagaattatgcagtgctgccataaccatgagtgataacactgcggccaacttacttctgacaacgatcggaggaccgaaggagctaaccgcttttttgcacaacatgggggatcatgtaactcgccttgatcgttgggaaccggagctgaatgaagccataccaaacgacgagcgtgacaccacgatgcctgtagcaatggcaacaacgttgcgcaaactattaactggcgaactacttactctagcttcccggcaacaattaatagactggatggaggcggataaagttgcaggaccacttctgcgctcggcccttccggctggctggtttattgctgataaatctggagccggtgagcgtgggtctcgcggtatcattgcagcactggggccagatggtaagccctcccgtatcgtagttatctacacgacggggagtcaggcaactatggatgaacgaaatagacagatcgctgagataggtgcctcactgattaagcattggtaactgtcagaccaagtttac

SEQ ID NO: 351 - DNA, 9588 bp, synthetic construct
  misc_feature 1..9588: note = DNA of V50_3xGCN4-TALE HPT8-ZIM3-P2A-D3a-hD3L-XTEN80-scFv
  source 1..9588: mol_type = other DNA
tgagataggtgcctcactgattaagcattggtaactgtcagaccaagtttactcatatatactttagattgatttaaaacttcatttttaatttaaaaggatctaggtgaagatcctttttgataatctcatgaccaaaatcccttaacgtgagttttcgttccactgagcgtcagaccccgtagaaaagatcaaaggatcttcttgagatcctttttttctgcgcgtaatctgctgcttgcaaacaaaaaaaccaccgctaccagcggtggtttgtttgccggatcaagagctaccaactctttttccgaaggtaactggcttcagcagagcgcagataccaaatactgttcttctagtgtagccgtagttaggccaccacttcaagaactctgtagcaccgcctacatacctcgctctgctaatcctgttaccagtggctgctgccagtggcgataagtcgtgtcttaccgggttggactcaagacgatagttaccggataaggcgcagcggtcgggctgaacggggggttcgtgcacacagcccagcttggagcgaacgacctacaccgaactgagatacctacagcgtgagctatgagaaagcgccacgcttcccgaagggagaaaggcggacaggtatccggtaagcggcagggtcggaacaggagagcgcacgagggagcttccagggggaaacgcctggtatctttatagtcctgtcgggtttcgccacctctgacttgagcgtcgatttttgtgatgctcgtcaggggggcggagcctatggaaaaacgccagcaacgcggcctttttacggttcctggccttttgctggccttttgctcacatgttctttcctgcgttatcccctgattctgtggataaccgtattaccgcctttgagtgagctgataccgctcgccgcagccgaacgaccgagcgcagcgagtcagtgagcgaggaagcggaagagcgcccaatacgcaaaccgcctctccccgcgcgttggccgattcattaatgcagctggcacgacaggtttcccgactggaaagcgggcagtgagcgcaacgcaattaatgtgagttagctcactcattaggcaccccaggctttacactttatgcttccggctcgtatgttgtgtggaattgtgagcggataacaatttcacacaggaaacagctatgaccatgattacgcctctagaaagctttaatacgactcactataaggactcactatttgttttcgcgcccagttgcaaaaagtgtcgacatttgcttctgacacaactgtgttcactagcaacctcaaacagacaccgccaccatgcctgctgctaagagagtgaaactggatggatccgaggaactgctgagcaagaactaccacctggaaaacgaggtggccagactgaagaaaggctctggctctggcggaagcggttctggcggatcaggatctggaagtggcggctctggaagcggaggttctggatctggcgaagaactgctgtctaagaattatcacctcgagaacgaagtggctcggctcaagaaaggcagtggcagcggaggaagtggatccggcggtagtggtagtggaagcggcggatccggctcaggcggatctggttcaggggaagaactcctctccaaaaactaccatctcgagaatgaggtcgcccgcctgaaaaaaggatcaggttccggtggttctggcagcggtggttcaggctcaggcagcggcggtagcggtagcggtggaagcggaagcggaccaaaaaagaagagaaaggtaatggtggatctacgcacgctcggctacagccagcagcaacaggagaagatcaaaccgaaggttcgttcgacagtggcgcagcaccacgaggcactggtcggccatgggtttacacacgcgcacatcgttgcgctcagccaacacccggcagcgttagggaccgtcgctgtcaagtatcaggacatgatcgcagcgttgccagaggcgacacacgaagcgatcgttggcgtcggcaaacagtggtccggcgcacgcgctctggaggccttgctcacggtggcgggagagttgagaggtccaccgttacagttggacacaggccaacttctcaagattgcaaaacgtggcggcgtgaccgcagtggaggcagtgcatgcatggcgcaatgcactgacgggtgcccccctgaacctgaccccggaccaagtggtggctatcgccagcaacggtggcggcaagcaagcgctcgaaacggtgcagcggctgttgccggtgctgtgccaggaccatggcctgactccggaccaagtggtggctatcgccagccacgatggcggcaagcaagcgctcgaaacggtgcagcggctgttgccggtgctgtgccaggaccatggcctgaccccggaccaagtggtggctatcgccagcaacattggcggcaagcaagcgctcgaaacggtgcagcggctgttgccggtgctgtgccaggaccatggcctgaccccggaccaagtggtggctatcgccagcaacaatggcggcaagcaagcgctcgaaacggtgcagcggctgttgccggtgctgtgccaggaccatggcctgaccccggaccaagtggtggctatcgccagcaacggtggcggcaagcaagcgctcgaaacggtgcagcggctgttgccggtgctgtgccaggaccatggcctgaccccggaccaagtggtggctatcgccagcaacggtggcggcaagcaagcgctcgaaacggtgcagcggctgttgccggtgctgtgccaggaccatggcctgactccggaccaagtggtggctatcgccagccacgatggcggcaagcaagcgctcgaaacggtgcagcggctgttgccggtgctgtgccaggaccatggcctgaccccggaccaagtggtggctatcgccagcaacattggcggcaagcaagcgctcgaaacggtgcagcggctgttgccggtgctgtgccaggaccatggcctgaccccggaccaagtggtggctatcgccagcaacaatggcggcaagcaagcgctcgaaacggtgcagcggctgttgccggtgctgtgccaggaccatggcctgaccccggaccaagtggtggctatcgccagcaacaatggcggcaagcaagcgctcgaaacggtgcagcggctgttgccggtgctgtgccaggaccatggcctgaccccggaccaagtggtggctatcgccagcaacaatggcggcaagcaagcgctcgaaacggtgcagcggctgttgccggtgctgtgccaggaccatggcctgaccccggaccaagtggtggctatcgccagcaacggtggcggcaagcaagcgctcgaaacggtgcagcggctgttgccggtgctgtgccaggaccatggcctgactccggaccaagtggtggctatcgccagccacgatggcggcaagcaagcgctcgaaacggtgcagcggctgttgccggtgctgtgccaggaccatggcctgaccccggaccaagtggtggctatcgccagcaacggtggcggcaagcaagcgctcgaaacggtgcagcggctgttgccggtgctgtgccaggaccatggcctgaccccggaccaagtggtggctatcgccagcaacaatggcggcaagcaagcgctcgaaacggtgcagcggctgttgccggtgctgtgccaggaccatggcctgaccccggaccaagtggtggctatcgccagcaacattggcggcaagcaagcgctcgaaacggtgcagcggctgttgccggtgctgtgccaggaccatggcctgaccccggaccaagtggtggctatcgccagcaacaatggcggcaagcaagcgctcgaaacggtgcagcggctgttgccggtgctgtgccaggaccatggcctgaccccggaccaagtggtggctatcgccagccacgatggcggcaagcaagcgctcgaaagcattgtggcccagctgagccggcctgatccggcgttggccgcgttgaccaacgaccacctcgtcgccttggcctgcctcggcggacgtcctgccatggatgcagtgaaaaagggattgccgcacgcgccggaattgatcagaagagtcaatcgccgtattggcgaacgcacgtcccatcgcgttgcctatccctatgacgtgcccgattatgccagcctgggcagcggctcccccaagaaaaaacgcaaggtggaagatcctaagaaaaagcggaaagtggacggcagcggcagcgagacccccggtaccagcgagagcgccacccccgagagcatgaacaattcccagggaagagtgaccttcgaggatgtcactgtgaacttcacccagggggagtggcagcggctgaatcccgaacagagaaacttgtacagggatgtgatgctggagaattacagcaaccttgtctctgtgggacaaggggaaaccaccaaacccgatgtgatcttgaggttggaacaaggaaaggagccatggttggaggaagaggaagtgctgggaagtggccgtgcagaaaaaaatggggacattggagggcagatttggaagccaaaggatgtgaaagagagtctcctcgagggaagcggagctactaacttcagcctgctgaagcaggctggagacgtggaggagaaccctggacctatgcctgctgctaagagagtgaaactggatggatccaaccatgaccaggaatttgaccccccaaaggtttacccacctgtgccagctgagaagaggaagcccatccgcgtgctgtctctctttgatgggattgctacagggctcctggtgctgaaggacctgggcatccaagtggaccgctacattgcctccgaggtgtgtgaggactccatcacggtgggcatggtgcggcaccagggaaagatcatgtacgtcggggacgtccgcagcgtcacacagaagcatatccaggagtggggcccattcgacctggtgattggaggcagtccctgcaatgacctctccattgtcaaccctgcccgcaagggactttatgagggtactggccgcctcttctttgagttctaccgcctcctgcatgatgcgcggcccaaggagggagatgatcgccccttcttctggctctttgagaatgtggtggccatgggcgttagtgacaagagggacatctcgcgatttcttgagtctaaccccgtgatgattgacgccaaagaagtgtctgctgcacacagggcccgttacttctggggtaaccttcctggcatgaacaggcctttggcatccactgtgaatgataagctggagctgcaagagtgtctggagcacggcagaatagccaagttcagcaaagtgaggaccattaccaccaggtcaaactctataaagcagggcaaagaccagcatttccccgtgttcatgaacgagaaggaggacatcctgtggtgcactgaaatggaaagggtgtttggcttccccgtccactacacagacgtctccaacatgagccgcttggcgaggcagagactgctgggccgatcgtggagcgtgccggtcatccgccacctcttcgctccgctgaaggaatattttgcttgtgtgtctagcggcaatagtaacgctaacagccgcgggccgagcttcagcagcggcctggtgccgttaagcttgcgcggcagccatatgttcgaaaccgtgcctgtgtggaggagacagccagtccgggtgctgtccctttttgaagacatcaagaaagagctgacgagtttgggctttttggaaagtggttctgacccgggacaactgaagcatgtggttgatgtcacagacacagtgaggaaggatgtggaggagtggggacccttcgatcttgtgtacggcgccacacctcccctgggccacacctgtgaccgtcctcccagctggtacctgttccagttccaccggctcctgcagtacgcacggcccaagccaggcagccccaggcccttcttctggatgttcgtggacaatctggtgctgaacaaggaagacctggacgtcgcatctcgcttcctggagatggagccagtcaccatcccagatgtccacggcggatccttgcagaatgctgtccgcgtgtggagcaacatcccagccataaggagcagcaggcactgggctctggtttcggaagaagaattgtccctgctggcccagaacaagcagagctcgaagctcgcggccaagtggcccaccaagctggtgaagaactgctttctccccctaagagaatatttcaagtatttttcaggagggccgagctctggcgcacccccaccaagtggagggtctcctgccgggtccccaacatctactgaagaaggcaccagcgaatccgcaacgcccgagtcaggccctggtacctccacagaaccatctgaaggtagtgcgcctggttccccagctggaagccctacttccaccgaagaaggcacgtcaaccgaaccaagtgaaggatctgcccctgggaccagcactgaaccatctgagccaaaaaagaagagaaaggtaccatctgagggccccgacatcgtgatgacccagagccccagcagcctgagcgccagcgtgggcgaccgcgtgaccatcacctgccgcagcagcaccggcgccgtgaccaccagcaactacgccagctgggtgcaggagaagcccggcaagctgttcaagggcctgatcggcggcaccaacaaccgcgcccccggcgtgcccagccgcttcagcggcagcctgatcggcgacaaggccaccctgaccatcagcagcctgcagcccgaggacttcgccacctacttctgcgccctgtggtacagcaaccactgggtgttcggccagggcaccaaggtggagctgaagcgcggcggcggcggcagcggcggcggcggcagcggcggcggcggcagcagcggcggcggcagcgaggtgaagctgctggagagcggcggcggcctggtgcagcccggcggcagcctgaagctgagctgcgccgtgagcggcttcagcctgaccgactacggcgtgaactgggtgcgccaggcccccggccgcggcctggagtggatcggcgtgatctggggcgacggcatcaccgactacaacagcgccctgaaggaccgcttcatcatcagcaaggacaacggcaagaacaccgtgtacctgcagatgagcaaggtgcgcagcgacgacaccgccctgtactactgcgtgaccggcctgttcgactactggggccagggcaccctggtgaccgtgagcagctacccatacgatgttccagattacgctggtggaggcggaggttctgggggaggaggtagtggcggtggtggttcaggaggcggcggaagctgataataggatcccaagcacgcagcaatgcagctcaaaacgcttagcctagccacacccccacgggaaacagcagtgattaacctttagcaataaacgaaagtttaactaagctatactaaccccagggttggtcaatttcgtgccagccacaccctggtactgcatgcacgcaatgctagctgcccctttcccgtcctgggcaccccgagtctcccccgaccccgggtcccaggtatgctcccacctccacctgccccactcaccacctctgctagttccagacacctccgagacgaggaaaaaaaaaaaaaaaaaaaaaaaaaaaaaaaaaaaaaaaaaaaaaaaaaaaaaaaaaaaaaaaaaaaaaaaaaaaaaaaaaaaaaaaaaaaaaaaaaaaaaaaaaaaaaaaaaaaaaaaaaaaaaaaaaaaaaaaaaaaaaaaaaaaaaaaaaaaaaaaaaaaaaaaaaaaaaaaaaaaaaaaaaaaaaaaaaaaaaaaaaaaaaaaaaaaaaaaaaaaaaaaaaaaaaaaaaaaaaaaaaaaaaaaaaaaaaaaaaaaaaaaaaaaaaaaaaaaaaaaaaaaaaaaaaaaaaaaaaaaaaaaaaaaaaaaaaaaaaaaaaaaaaaaaaaaaaaaaaaaaaaaaaaaaaaaaaaaaaaaaaaaaaaaaaaaaaaaaaaaaaaaaaaaaaaaaaaccgtcttcaagctttctagaaattcactggccgtcgttttacaacgtcgtgactgggaaaaccctggcgttacccaacttaatcgccttgcagcacatccccctttcgccagctggcgtaatagcgaagaggcccgcaccgatcgcccttcccaacagttgcgcagcctgaatggcgaatggcgcctgatgcggtattttctccttacgcatctgtgcggtatttcacaccgcatatggtgcactctcagtacaatctgctctgatgccgcatagttaagccagccccgacacccgccaacacccgctgacgcgccctgacgggcttgtctgctcccggcatccgcttacagacaagctgtgaccgtctccgggagctgcatgtgtcagaggttttcaccgtcatcaccgaaacgcgcgagacgaaagggcctcgtgatacgcctatttttataggttaatgtcatgataataatggtttcttagacgtcaggtggcacttttcggggaaatgtgcgcggaacccctatttgtttatttttctaaatacattcaaatatgtatccgctcatgagacaataaccctgataaatgcttcaataatattgaaaaaggaagagtatgagtattcaacatttccgtgtcgcccttattcccttttttgcggcattttgccttcctgtttttgctcacccagaaacgctggtgaaagtaaaagatgctgaagatcagttgggtgcacgagtgggttacatcgaactggatctcaacagcggtaagatccttgagagttttcgccccgaagaacgttttccaatgatgagcacttttaaagttctgctatgtggcgcggtattatcccgtattgacgccgggcaagagcaactcggtcgccgcatacactattctcagaatgacttggttgagtactcaccagtcacagaaaagcatcttacggatggcatgacagtaagagaattatgcagtgctgccataaccatgagtgataacactgcggccaacttacttctgacaacgatcggaggaccgaaggagctaaccgcttttttgcacaacatgggggatcatgtaactcgccttgatcgttgggaaccggagctgaatgaagccataccaaacgacgagcgtgacaccacgatgcctgtagcaatggcaacaacgttgcgcaaactattaactggcgaactacttactctagcttcccggcaacaattaatagactggatggaggcggataaagttgcaggaccacttctgcgctcggcccttccggctggctggtttattgctgataaatctggagccggtgagcgtgggtctcgcggtatcattgcagcactggggccagatggtaagccctcccgtatcgtagttatctacacgacggggagtcaggcaactatggatgaacgaaatagacagatcgc

SEQ ID NO: 352 - DNA, 9588 bp, synthetic construct
  misc_feature 1..9588: note = DNA of V51_3xGCN4-TALE HPT12-ZIM3-P2A-D3a-hD3L-XTEN80-scFv
  source 1..9588: mol_type = other DNA
tgagataggtgcctcactgattaagcattggtaactgtcagaccaagtttactcatatatactttagattgatttaaaacttcatttttaatttaaaaggatctaggtgaagatcctttttgataatctcatgaccaaaatcccttaacgtgagttttcgttccactgagcgtcagaccccgtagaaaagatcaaaggatcttcttgagatcctttttttctgcgcgtaatctgctgcttgcaaacaaaaaaaccaccgctaccagcggtggtttgtttgccggatcaagagctaccaactctttttccgaaggtaactggcttcagcagagcgcagataccaaatactgttcttctagtgtagccgtagttaggccaccacttcaagaactctgtagcaccgcctacatacctcgctctgctaatcctgttaccagtggctgctgccagtggcgataagtcgtgtcttaccgggttggactcaagacgatagttaccggataaggcgcagcggtcgggctgaacggggggttcgtgcacacagcccagcttggagcgaacgacctacaccgaactgagatacctacagcgtgagctatgagaaagcgccacgcttcccgaagggagaaaggcggacaggtatccggtaagcggcagggtcggaacaggagagcgcacgagggagcttccagggggaaacgcctggtatctttatagtcctgtcgggtttcgccacctctgacttgagcgtcgatttttgtgatgctcgtcaggggggcggagcctatggaaaaacgccagcaacgcggcctttttacggttcctggccttttgctggccttttgctcacatgttctttcctgcgttatcccctgattctgtggataaccgtattaccgcctttgagtgagctgataccgctcgccgcagccgaacgaccgagcgcagcgagtcagtgagcgaggaagcggaagagcgcccaatacgcaaaccgcctctccccgcgcgttggccgattcattaatgcagctggcacgacaggtttcccgactggaaagcgggcagtgagcgcaacgcaattaatgtgagttagctcactcattaggcaccccaggctttacactttatgcttccggctcgtatgttgtgtggaattgtgagcggataacaatttcacacaggaaacagctatgaccatgattacgcctctagaaagctttaatacgactcactataaggactcactatttgttttcgcgcccagttgcaaaaagtgtcgacatttgcttctgacacaactgtgttcactagcaacctcaaacagacaccgccaccatgcctgctgctaagagagtgaaactggatggatccgaggaactgctgagcaagaactaccacctggaaaacgaggtggccagactgaagaaaggctctggctctggcggaagcggttctggcggatcaggatctggaagtggcggctctggaagcggaggttctggatctggcgaagaactgctgtctaagaattatcacctcgagaacgaagtggctcggctcaagaaaggcagtggcagcggaggaagtggatccggcggtagtggtagtggaagcggcggatccggctcaggcggatctggttcaggggaagaactcctctccaaaaactaccatctcgagaatgaggtcgcccgcctgaaaaaaggatcaggttccggtggttctggcagcggtggttcaggctcaggcagcggcggtagcggtagcggtggaagcggaagcggaccaaaaaagaagagaaaggtaatggtggatctacgcacgctcggctacagccagcagcaacaggagaagatcaaaccgaaggttcgttcgacagtggcgcagcaccacgaggcactggtcggccatgggtttacacacgcgcacatcgttgcgctcagccaacacccggcagcgttagggaccgtcgctgtcaagtatcaggacatgatcgcagcgttgccagaggcgacacacgaagcgatcgttggcgtcggcaaacagtggtccggcgcacgcgctctggaggccttgctcacggtggcgggagagttgagaggtccaccgttacagttggacacaggccaacttctcaagattgcaaaacgtggcggcgtgaccgcagtggaggcagtgcatgcatggcgcaatgcactgacgggtgcccccctgaacctgaccccggaccaagtggtggctatcgccagcaacaatggcggcaagcaagcgctcgaaacggtgcagcggctgttgccggtgctgtgccaggaccatggcctgaccccggaccaagtggtggctatcgccagcaacaatggcggcaagcaagcgctcgaaacggtgcagcggctgttgccggtgctgtgccaggaccatggcctgaccccggaccaagtggtggctatcgccagcaacattggcggcaagcaagcgctcgaaacggtgcagcggctgttgccggtgctgtgccaggaccatggcctgaccccggaccaagtggtggctatcgccagcaacaatggcggcaagcaagcgctcgaaacggtgcagcggctgttgccggtgctgtgccaggaccatggcctgaccccggaccaagtggtggctatcgccagcaacaatggcggcaagcaagcgctcgaaacggtgcagcggctgttgccggtgctgtgccaggaccatggcctgaccccggaccaagtggtggctatcgccagcaacattggcggcaagcaagcgctcgaaacggtgcagcggctgttgccggtgctgtgccaggaccatggcctgaccccggaccaagtggtggctatcgccagcaacaatggcggcaagcaagcgctcgaaacggtgcagcggctgttgccggtgctgtgccaggaccatggcctgaccccggaccaagtggtggctatcgccagcaacggtggcggcaagcaagcgctcgaaacggtgcagcggctgttgccggtgctgtgccaggaccatggcctgaccccggaccaagtggtggctatcgccagcaacaatggcggcaagcaagcgctcgaaacggtgcagcggctgttgccggtgctgtgccaggaccatggcctgaccccggaccaagtggtggctatcgccagcaacattggcggcaagcaagcgctcgaaacggtgcagcggctgttgccggtgctgtgccaggaccatggcctgaccccggaccaagtggtggctatcgccagcaacaatggcggcaagcaagcgctcgaaacggtgcagcggctgttgccggtgctgtgccaggaccatggcctgactccggaccaagtggtggctatcgccagccacgatggcggcaagcaagcgctcgaaacggtgcagcggctgttgccggtgctgtgccaggaccatggcctgactccggaccaagtggtggctatcgccagccacgatggcggcaagcaagcgctcgaaacggtgcagcggctgttgccggtgctgtgccaggaccatggcctgaccccggaccaagtggtggctatcgccagcaacattggcggcaagcaagcgctcgaaacggtgcagcggctgttgccggtgctgtgccaggaccatggcctgaccccggaccaagtggtggctatcgccagcaacaatggcggcaagcaagcgctcgaaacggtgcagcggctgttgccggtgctgtgccaggaccatggcctgaccccggaccaagtggtggctatcgccagcaacaatggcggcaagcaagcgctcgaaacggtgcagcggctgttgccggtgctgtgccaggaccatggcctgactccggaccaagtggtggctatcgccagccacgatggcggcaagcaagcgctcgaaacggtgcagcggctgttgccggtgctgtgccaggaccatggcctgaccccggaccaagtggtggctatcgccagcaacattggcggcaagcaagcgctcgaaagcattgtggcccagctgagccggcctgatccggcgttggccgcgttgaccaacgaccacctcgtcgccttggcctgcctcggcggacgtcctgccatggatgcagtgaaaaagggattgccgcacgcgccggaattgatcagaagagtcaatcgccgtattggcgaacgcacgtcccatcgcgttgcctatccctatgacgtgcccgattatgccagcctgggcagcggctcccccaagaaaaaacgcaaggtggaagatcctaagaaaaagcggaaagtggacggcagcggcagcgagacccccggtaccagcgagagcgccacccccgagagcatgaacaattcccagggaagagtgaccttcgaggatgtcactgtgaacttcacccagggggagtggcagcggctgaatcccgaacagagaaacttgtacagggatgtgatgctggagaattacagcaaccttgtctctgtgggacaaggggaaaccaccaaacccgatgtgatcttgaggttggaacaaggaaaggagccatggttggaggaagaggaagtgctgggaagtggccgtgcagaaaaaaatggggacattggagggcagatttggaagccaaaggatgtgaaagagagtctcctcgagggaagcggagctactaacttcagcctgctgaagcaggctggagacgtggaggagaaccctggacctatgcctgctgctaagagagtgaaactggatggatccaaccatgaccaggaatttgaccccccaaaggtttacccacctgtgccagctgagaagaggaagcccatccgcgtgctgtctctctttgatgggattgctacagggctcctggtgctgaaggacctgggcatccaagtggaccgctacattgcctccgaggtgtgtgaggactccatcacggtgggcatggtgcggcaccagggaaagatcatgtacgtcggggacgtccgcagcgtcacacagaagcatatccaggagtggggcccattcgacctggtgattggaggcagtccctgcaatgacctctccattgtcaaccctgcccgcaagggactttatgagggtactggccgcctcttctttgagttctaccgcctcctgcatgatgcgcggcccaaggagggagatgatcgccccttcttctggctctttgagaatgtggtggccatgggcgttagtgacaagagggacatctcgcgatttcttgagtctaaccccgtgatgattgacgccaaagaagtgtctgctgcacacagggcccgttacttctggggtaaccttcctggcatgaacaggcctttggcatccactgtgaatgataagctggagctgcaagagtgtctggagcacggcagaatagccaagttcagcaaagtgaggaccattaccaccaggtcaaactctataaagcagggcaaagaccagcatttccccgtgttcatgaacgagaaggaggacatcctgtggtgcactgaaatggaaagggtgtttggcttccccgtccactacacagacgtctccaacatgagccgcttggcgaggcagagactgctgggccgatcgtggagcgtgccggtcatccgccacctcttcgctccgctgaaggaatattttgcttgtgtgtctagcggcaatagtaacgctaacagccgcgggccgagcttcagcagcggcctggtgccgttaagcttgcgcggcagccatatgttcgaaaccgtgcctgtgtggaggagacagccagtccgggtgctgtccctttttgaagacatcaagaaagagctgacgagtttgggctttttggaaagtggttctgacccgggacaactgaagcatgtggttgatgtcacagacacagtgaggaaggatgtggaggagtggggacccttcgatcttgtgtacggcgccacacctcccctgggccacacctgtgaccgtcctcccagctggtacctgttccagttccaccggctcctgcagtacgcacggcccaagccaggcagccccaggcccttcttctggatgttcgtggacaatctggtgctgaacaaggaagacctggacgtcgcatctcgcttcctggagatggagccagtcaccatcccagatgtccacggcggatccttgcagaatgctgtccgcgtgtggagcaacatcccagccataaggagcagcaggcactgggctctggtttcggaagaagaattgtccctgctggcccagaacaagcagagctcgaagctcgcggccaagtggcccaccaagctggtgaagaactgctttctccccctaagagaatatttcaagtatttttcaggagggccgagctctggcgcacccccaccaagtggagggtctcctgccgggtccccaacatctactgaagaaggcaccagcgaatccgcaacgcccgagtcaggccctggtacctccacagaaccatctgaaggtagtgcgcctggttccccagctggaagccctacttccaccgaagaaggcacgtcaaccgaaccaagtgaaggatctgcccctgggaccagcactgaaccatctgagccaaaaaagaagagaaaggtaccatctgagggccccgacatcgtgatgacccagagccccagcagcctgagcgccagcgtgggcgaccgcgtgaccatcacctgccgcagcagcaccggcgccgtgaccaccagcaactacgccagctgggtgcaggagaagcccggcaagctgttcaagggcctgatcggcggcaccaacaaccgcgcccccggcgtgcccagccgcttcagcggcagcctgatcggcgacaaggccaccctgaccatcagcagcctgcagcccgaggacttcgccacctacttctgcgccctgtggtacagcaaccactgggtgttcggccagggcaccaaggtggagctgaagcgcggcggcggcggcagcggcggcggcggcagcggcggcggcggcagcagcggcggcggcagcgaggtgaagctgctggagagcggcggcggcctggtgcagcccggcggcagcctgaagctgagctgcgccgtgagcggcttcagcctgaccgactacggcgtgaactgggtgcgccaggcccccggccgcggcctggagtggatcggcgtgatctggggcgacggcatcaccgactacaacagcgccctgaaggaccgcttcatcatcagcaaggacaacggcaagaacaccgtgtacctgcagatgagcaaggtgcgcagcgacgacaccgccctgtactactgcgtgaccggcctgttcgactactggggccagggcaccctggtgaccgtgagcagctacccatacgatgttccagattacgctggtggaggcggaggttctgggggaggaggtagtggcggtggtggttcaggaggcggcggaagctgataataggatcccaagcacgcagcaatgcagctcaaaacgcttagcctagccacacccccacgggaaacagcagtgattaacctttagcaataaacgaaagtttaactaagctatactaaccccagggttggtcaatttcgtgccagccacaccctggtactgcatgcacgcaatgctagctgcccctttcccgtcctgggcaccccgagtctcccccgaccccgggtcccaggtatgctcccacctccacctgccccactcaccacctctgctagttccagacacctccgagacgaggaaaaaaaaaaaaaaaaaaaaaaaaaaaaaaaaaaaaaaaaaaaaaaaaaaaaaaaaaaaaaaaaaaaaaaaaaaaaaaaaaaaaaaaaaaaaaaaaaaaaaaaaaaaaaaaaaaaaaaaaaaaaaaaaaaaaaaaaaaaaaaaaaaaaaaaaaaaaaaaaaaaaaaaaaaaaaaaaaaaaaaaaaaaaaaaaaaaaaaaaaaaaaaaaaaaaaaaaaaaaaaaaaaaaaaaaaaaaaaaaaaaaaaaaaaaaaaaaaaaaaaaaaaaaaaaaaaaaaaaaaaaaaaaaaaaaaaaaaaaaaaaaaaaaaaaaaaaaaaaaaaaaaaaaaaaaaaaaaaaaaaaaaaaaaaaaaaaaaaaaaaaaaaaaaaaaaaaaaaaaaaaaaaaaaaaaaaccgtcttcaagctttctagaaattcactggccgtcgttttacaacgtcgtgactgggaaaaccctggcgttacccaacttaatcgccttgcagcacatccccctttcgccagctggcgtaatagcgaagaggcccgcaccgatcgcccttcccaacagttgcgcagcctgaatggcgaatggcgcctgatgcggtattttctccttacgcatctgtgcggtatttcacaccgcatatggtgcactctcagtacaatctgctctgatgccgcatagttaagccagccccgacacccgccaacacccgctgacgcgccctgacgggcttgtctgctcccggcatccgcttacagacaagctgtgaccgtctccgggagctgcatgtgtcagaggttttcaccgtcatcaccgaaacgcgcgagacgaaagggcctcgtgatacgcctatttttataggttaatgtcatgataataatggtttcttagacgtcaggtggcacttttcggggaaatgtgcgcggaacccctatttgtttatttttctaaatacattcaaatatgtatccgctcatgagacaataaccctgataaatgcttcaataatattgaaaaaggaagagtatgagtattcaacatttccgtgtcgcccttattcccttttttgcggcattttgccttcctgtttttgctcacccagaaacgctggtgaaagtaaaagatgctgaagatcagttgggtgcacgagtgggttacatcgaactggatctcaacagcggtaagatccttgagagttttcgccccgaagaacgttttccaatgatgagcacttttaaagttctgctatgtggcgcggtattatcccgtattgacgccgggcaagagcaactcggtcgccgcatacactattctcagaatgacttggttgagtactcaccagtcacagaaaagcatcttacggatggcatgacagtaagagaattatgcagtgctgccataaccatgagtgataacactgcggccaacttacttctgacaacgatcggaggaccgaaggagctaaccgcttttttgcacaacatgggggatcatgtaactcgccttgatcgttgggaaccggagctgaatgaagccataccaaacgacgagcgtgacaccacgatgcctgtagcaatggcaacaacgttgcgcaaactattaactggcgaactacttactctagcttcccggcaacaattaatagactggatggaggcggataaagttgcaggaccacttctgcgctcggcccttccggctggctggtttattgctgataaatctggagccggtgagcgtgggtctcgcggtatcattgcagcactggggccagatggtaagccctcccgtatcgtagttatctacacgacggggagtcaggcaactatggatgaacgaaatagacagatcgc

SEQ ID NO: 353 - RNA, 6436 nt, synthetic construct
  misc_feature 1..6436: note = mRNA of V48_scFv-ZIM3-P2A-D3a-hD3L-XTEN80-TALE HPT8-1xGCN4
  source 1..6436: mol_type = other RNA
aggactcactatttgttttcgcgcccagttgcaaaaagtgtcgacatttgcttctgacacaactgtgttcactagcaacctcaaacagacaccgccaccatgcctgctgctaagagagtgaaactggatggatccggccccgacatcgtgatgacccagagccccagcagcctgagcgccagcgtgggcgaccgcgtgaccatcacctgccgcagcagcaccggcgccgtgaccaccagcaactacgccagctgggtgcaggagaagcccggcaagctgttcaagggcctgatcggcggcaccaacaaccgcgcccccggcgtgcccagccgcttcagcggcagcctgatcggcgacaaggccaccctgaccatcagcagcctgcagcccgaggacttcgccacctacttctgcgccctgtggtacagcaaccactgggtgttcggccagggcaccaaggtggagctgaagcgcggcggcggcggcagcggcggcggcggcagcggcggcggcggcagcagcggcggcggcagcgaggtgaagctgctggagagcggcggcggcctggtgcagcccggcggcagcctgaagctgagctgcgccgtgagcggcttcagcctgaccgactacggcgtgaactgggtgcgccaggcccccggccgcggcctggagtggatcggcgtgatctggggcgacggcatcaccgactacaacagcgccctgaaggaccgcttcatcatcagcaaggacaacggcaagaacaccgtgtacctgcagatgagcaaggtgcgcagcgacgacaccgccctgtactactgcgtgaccggcctgttcgactactggggccagggcaccctggtgaccgtgagcagctacccatacgatgttccagattacgctggtggaggcggaggttctgggggaggaggtagtggcggtggtggttcaggaggcggcggaagcttggatccaggtggaggtggaagcggtatgaacaattcccagggaagagtgaccttcgaggacgtgaccgtgaacttcacccaaggcgagtggcagagactgaaccccgagcagagaaacctgtaccgggacgtgatgctggaaaactacagcaacctggtgtccgtcggccagggcgagacaacaaagcctgacgtgatcctgcggctggaacagggcaaagagccttggctggaagaggaagaggtgctcggatctggcagagccgagaagaatggcgatatcggcggacagatctggaagccaaaggatgtgaaagagagtctcggaagcggagctactaacttcagcctgctgaagcaggctggagacgtggaggagaaccctggacctatgcctgctgctaagagagtgaaactggatggatccaaccatgaccaggaatttgaccccccaaaggtttacccacctgtgccagctgagaagaggaagcccatccgcgtgctgtctctctttgatgggattgctacagggctcctggtgctgaaggacctgggcatccaagtggaccgctacattgcctccgaggtgtgtgaggactccatcacggtgggcatggtgcggcaccagggaaagatcatgtacgtcggggacgtccgcagcgtcacacagaagcatatccaggagtggggcccattcgacctggtgattggaggcagtccctgcaatgacctctccattgtcaaccctgcccgcaagggactttatgagggtactggccgcctcttctttgagttctaccgcctcctgcatgatgcgcggcccaaggagggagatgatcgccccttcttctggctctttgagaatgtggtggccatgggcgttagtgacaagagggacatctcgcgatttcttgagtctaaccccgtgatgattgacgccaaagaagtgtctgctgcacacagggcccgttacttctggggtaaccttcctggcatgaacaggcctttggcatccactgtgaatgataagctggagctgcaagagtgtctggagcacggcagaatagccaagttcagcaaagtgaggaccattaccaccaggtcaaactctataaagcagggcaaagaccagcatttccccgtgttcatgaacgagaaggaggacatcctgtggtgcactgaaatggaaagggtgtttggcttccccgtccactacacagacgtctccaacatgagccgcttggcgaggcagagactgctgggccgatcgtggagcgtgccggtcatccgccacctcttcgctccgctgaaggaatattttgcttgtgtgtctagcggcaatagtaacgctaacagccgcgggccgagcttcagcagcggcctggtgccgttaagcttgcgcggcagccatatgttcgaaaccgtgcctgtgtggaggagacagccagtccgggtgctgtccctttttgaagacatcaagaaagagctgacgagtttgggctttttggaaagtggttctgacccgggacaactgaagcatgtggttgatgtcacagacacagtgaggaaggatgtggaggagtggggacccttcgatcttgtgtacggcgccacacctcccctgggccacacctgtgaccgtcctcccagctggtacctgttccagttccaccggctcctgcagtacgcacggcccaagccaggcagccccaggcccttcttctggatgttcgtggacaatctggtgctgaacaaggaagacctggacgtcgcatctcgcttcctggagatggagccagtcaccatcccagatgtccacggcggatccttgcagaatgctgtccgcgtgtggagcaacatcccagccataaggagcagcaggcactgggctctggtttcggaagaagaattgtccctgctggcccagaacaagcagagctcgaagctcgcggccaagtggcccaccaagctggtgaagaactgctttctccccctaagagaatatttcaagtatttttcaggagggccgagctctggcgcacccccaccaagtggagggtctcctgccgggtccccaacatctactgaagaaggcaccagcgaatccgcaacgcccgagtcaggccctggtacctccacagaaccatctgaaggtagtgcgcctggttccccagctggaagccctacttccaccgaagaaggcacgtcaaccgaaccaagtgaaggatctgcccctgggaccagcactgaaccatctgagccaaaaaagaagagaaaggtaatggtggatctacgcacgctcggctacagccagcagcaacaggagaagatcaaaccgaaggttcgttcgacagtggcgcagcaccacgaggcactggtcggccatgggtttacacacgcgcacatcgttgcgctcagccaacacccggcagcgttagggaccgtcgctgtcaagtatcaggacatgatcgcagcgttgccagaggcgacacacgaagcgatcgttggcgtcggcaaacagtggtccggcgcacgcgctctggaggccttgctcacggtggcgggagagttgagaggtccaccgttacagttggacacaggccaacttctcaagattgcaaaacgtggcggcgtgaccgcagtggaggcagtgcatgcatggcgcaatgcactgacgggtgcccccctgaacctgaccccggaccaagtggtggctatcgccagcaacggtggcggcaagcaagcgctcgaaacggtgcagcggctgttgccggtgctgtgccaggaccatggcctgactccggaccaagtggtggctatcgccagccacgatggcggcaagcaagcgctcgaaacggtgcagcggctgttgccggtgctgtgccaggaccatggcctgaccccggaccaagtggtggctatcgccagcaacattggcggcaagcaagcgctcgaaacggtgcagcggctgttgccggtgctgtgccaggaccatggcctgaccccggaccaagtggtggctatcgccagcaacaatggcggcaagcaagcgctcgaaacggtgcagcggctgttgccggtgctgtgccaggaccatggcctgaccccggaccaagtggtggctatcgccagcaacggtggcggcaagcaagcgctcgaaacggtgcagcggctgttgccggtgctgtgccaggaccatggcctgaccccggaccaagtggtggctatcgccagcaacggtggcggcaagcaagcgctcgaaacggtgcagcggctgttgccggtgctgtgccaggaccatggcctgactccggaccaagtggtggctatcgccagccacgatggcggcaagcaagcgctcgaaacggtgcagcggctgttgccggtgctgtgccaggaccatggcctgaccccggaccaagtggtggctatcgccagcaacattggcggcaagcaagcgctcgaaacggtgcagcggctgttgccggtgctgtgccaggaccatggcctgaccccggaccaagtggtggctatcgccagcaacaatggcggcaagcaagcgctcgaaacggtgcagcggctgttgccggtgctgtgccaggaccatggcctgaccccggaccaagtggtggctatcgccagcaacaatggcggcaagcaagcgctcgaaacggtgcagcggctgttgccggtgctgtgccaggaccatggcctgaccccggaccaagtggtggctatcgccagcaacaatggcggcaagcaagcgctcgaaacggtgcagcggctgttgccggtgctgtgccaggaccatggcctgaccccggaccaagtggtggctatcgccagcaacggtggcggcaagcaagcgctcgaaacggtgcagcggctgttgccggtgctgtgccaggaccatggcctgactccggaccaagtggtggctatcgccagccacgatggcggcaagcaagcgctcgaaacggtgcagcggctgttgccggtgctgtgccaggaccatggcctgaccccggaccaagtggtggctatcgccagcaacggtggcggcaagcaagcgctcgaaacggtgcagcggctgttgccggtgctgtgccaggaccatggcctgaccccggaccaagtggtggctatcgccagcaacaatggcggcaagcaagcgctcgaaacggtgcagcggctgttgccggtgctgtgccaggaccatggcctgaccccggaccaagtggtggctatcgccagcaacattggcggcaagcaagcgctcgaaacggtgcagcggctgttgccggtgctgtgccaggaccatggcctgaccccggaccaagtggtggctatcgccagcaacaatggcggcaagcaagcgctcgaaacggtgcagcggctgttgccggtgctgtgccaggaccatggcctgaccccggaccaagtggtggctatcgccagccacgatggcggcaagcaagcgctcgaaagcattgtggcccagctgagccggcctgatccggcgttggccgcgttgaccaacgaccacctcgtcgccttggcctgcctcggcggacgtcctgccatggatgcagtgaaaaagggattgccgcacgcgccggaattgatcagaagagtcaatcgccgtattggcgaacgcacgtcccatcgcgttgcctatccctatgacgtgcccgattatgccagcctgggcagcggctcccccaagaaaaaacgcaaggtggaagatcctaagaaaaagcggaaagtggacggcattggtagtgggagcaacggcagcagcggagaggaactgctgagcaagaactaccacctggaaaacgaggtggccagactgaagaaaggctctggctctggcggaagcggttctggcggatcaggatctggaagtggcggctctggaagcggaggttctggatctggcgaagaactgctgtctaagaattatcacggttcaggctccggccagcggggaagcaagcgcaccgccgatggttccgagttcgaaagccccaaaaaaaagcgcaaggtctgataataggatcccaagcacgcagcaatgcagctcaaaacgcttagcctagccacacccccacgggaaacagcagtgattaacctttagcaataaacgaaagtttaactaagctatactaaccccagggttggtcaatttcgtgccagccacaccctggtactgcatgcacgcaatgctagctgcccctttcccgtcctgggcaccccgagtctcccccgaccccgggtcccaggtatgctcccacctccacctgccccactcaccacctctgctagttccagacacctccgagacgaggaaaaaaaaaaaaaaaaaaaaaaaaaaaaaaaaaaaaaaaaaaaaaaaaaaaaaaaaaaaaaaaaaaaaaaaaaaaaaaaaaaaaaaaaaaaaaaaaaaaaaaaaaaaaaaaaaaaaaaaa

SEQ ID NO: 354 - RNA, 6436 nt, synthetic construct
  misc_feature 1..6436: note = mRNA of V49_scFv-ZIM3-P2A-D3a-hD3L-XTEN80-TALE HPT12-1xGCN4
  source 1..6436: mol_type = other RNA
aggactcactatttgttttcgcgcccagttgcaaaaagtgtcgacatttgcttctgacacaactgtgttcactagcaacctcaaacagacaccgccaccatgcctgctgctaagagagtgaaactggatggatccggccccgacatcgtgatgacccagagccccagcagcctgagcgccagcgtgggcgaccgcgtgaccatcacctgccgcagcagcaccggcgccgtgaccaccagcaactacgccagctgggtgcaggagaagcccggcaagctgttcaagggcctgatcggcggcaccaacaaccgcgcccccggcgtgcccagccgcttcagcggcagcctgatcggcgacaaggccaccctgaccatcagcagcctgcagcccgaggacttcgccacctacttctgcgccctgtggtacagcaaccactgggtgttcggccagggcaccaaggtggagctgaagcgcggcggcggcggcagcggcggcggcggcagcggcggcggcggcagcagcggcggcggcagcgaggtgaagctgctggagagcggcggcggcctggtgcagcccggcggcagcctgaagctgagctgcgccgtgagcggcttcagcctgaccgactacggcgtgaactgggtgcgccaggcccccggccgcggcctggagtggatcggcgtgatctggggcgacggcatcaccgactacaacagcgccctgaaggaccgcttcatcatcagcaaggacaacggcaagaacaccgtgtacctgcagatgagcaaggtgcgcagcgacgacaccgccctgtactactgcgtgaccggcctgttcgactactggggccagggcaccctggtgaccgtgagcagctacccatacgatgttccagattacgctggtggaggcggaggttctgggggaggaggtagtggcggtggtggttcaggaggcggcggaagcttggatccaggtggaggtggaagcggtatgaacaattcccagggaagagtgaccttcgaggacgtgaccgtgaacttcacccaaggcgagtggcagagactgaaccccgagcagagaaacctgtaccgggacgtgatgctggaaaactacagcaacctggtgtccgtcggccagggcgagacaacaaagcctgacgtgatcctgcggctggaacagggcaaagagccttggctggaagaggaagaggtgctcggatctggcagagccgagaagaatggcgatatcggcggacagatctggaagccaaaggatgtgaaagagagtctcggaagcggagctactaacttcagcctgctgaagcaggctggagacgtggaggagaaccctggacctatgcctgctgctaagagagtgaaactggatggatccaaccatgaccaggaatttgaccccccaaaggtttacccacctgtgccagctgagaagaggaagcccatccgcgtgctgtctctctttgatgggattgctacagggctcctggtgctgaaggacctgggcatccaagtggaccgctacattgcctccgaggtgtgtgaggactccatcacggtgggcatggtgcggcaccagggaaagatcatgtacgtcggggacgtccgcagcgtcacacagaagcatatccaggagtggggcccattcgacctggtgattggaggcagtccctgcaatgacctctccattgtcaaccctgcccgcaagggactttatgagggtactggccgcctcttctttgagttctaccgcctcctgcatgatgcgcggcccaaggagggagatgatcgccccttcttctggctctttgagaatgtggtggccatgggcgttagtgacaagagggacatctcgcgatttcttgagtctaaccccgtgatgattgacgccaaagaagtgtctgctgcacacagggcccgttacttctggggtaaccttcctggcatgaacaggcctttggcatccactgtgaatgataagctggagctgcaagagtgtctggagcacggcagaatagccaagttcagcaaagtgaggaccattaccaccaggtcaaactctataaagcagggcaaagaccagcatttccccgtgttcatgaacgagaaggaggacatcctgtggtgcactgaaatggaaagggtgtttggcttccccgtccactacacagacgtctccaacatgagccgcttggcgaggcagagactgctgggccgatcgtggagcgtgccggtcatccgccacctcttcgctccgctgaaggaatattttgcttgtgtgtctagcggcaatagtaacgctaacagccgcgggccgagcttcagcagcggcctggtgccgttaagcttgcgcggcagccatatgttcgaaaccgtgcctgtgtggaggagacagccagtccgggtgctgtccctttttgaagacatcaagaaagagctgacgagtttgggctttttggaaagtggttctgacccgggacaactgaagcatgtggttgatgtcacagacacagtgaggaaggatgtggaggagtggggacccttcgatcttgtgtacggcgccacacctcccctgggccacacctgtgaccgtcctcccagctggtacctgttccagttccaccggctcctgcagtacgcacggcccaagccaggcagccccaggcccttcttctggatgttcgtggacaatctggtgctgaacaaggaagacctggacgtcgcatctcgcttcctggagatggagccagtcaccatcccagatgtccacggcggatccttgcagaatgctgtccgcgtgtggagcaacatcccagccataaggagcagcaggcactgggctctggtttcggaagaagaattgtccctgctggcccagaacaagcagagctcgaagctcgcggccaagtggcccaccaagctggtgaagaactgctttctccccctaagagaatatttcaagtatttttcaggagggccgagctctggcgcacccccaccaagtggagggtctcctgccgggtccccaacatctactgaagaaggcaccagcgaatccgcaacgcccgagtcaggccctggtacctccacagaaccatctgaaggtagtgcgcctggttccccagctggaagccctacttccaccgaagaaggcacgtcaaccgaaccaagtgaaggatctgcccctgggaccagcactgaaccatctgagccaaaaaagaagagaaaggtaatggtggatctacgcacgctcggctacagccagcagcaacaggagaagatcaaaccgaaggttcgttcgacagtggcgcagcaccacgaggcactggtcggccatgggtttacacacgcgcacatcgttgcgctcagccaacacccggcagcgttagggaccgtcgctgtcaagtatcaggacatgatcgcagcgttgccagaggcgacacacgaagcgatcgttggcgtcggcaaacagtggtccggcgcacgcgctctggaggccttgctcacggtggcgggagagttgagaggtccaccgttacagttggacacaggccaacttctcaagattgcaaaacgtggcggcgtgaccgcagtggaggcagtgcatgcatggcgcaatgcactgacgggtgcccccctgaacctgaccccggaccaagtggtggctatcgccagcaacaatggcggcaagcaagcgctcgaaacggtgcagcggctgttgccggtgctgtgccaggaccatggcctgaccccggaccaagtggtggctatcgccagcaacaatggcggcaagcaagcgctcgaaacggtgcagcggctgttgccggtgctgtgccaggaccatggcctgaccccggaccaagtggtggctatcgccagcaacattggcggcaagcaagcgctcgaaacggtgcagcggctgttgccggtgctgtgccaggaccatggcctgaccccggaccaagtggtggctatcgccagcaacaatggcggcaagcaagcgctcgaaacggtgcagcggctgttgccggtgctgtgccaggaccatggcctgaccccggaccaagtggtggctatcgccagcaacaatggcggcaagcaagcgctcgaaacggtgcagcggctgttgccggtgctgtgccaggaccatggcctgaccccggaccaagtggtggctatcgccagcaacattggcggcaagcaagcgctcgaaacggtgcagcggctgttgccggtgctgtgccaggaccatggcctgaccccggaccaagtggtggctatcgccagcaacaatggcggcaagcaagcgctcgaaacggtgcagcggctgttgccggtgctgtgccaggaccatggcctgaccccggaccaagtggtggctatcgccagcaacggtggcggcaagcaagcgctcgaaacggtgcagcggctgttgccggtgctgtgccaggaccatggcctgaccccggaccaagtggtggctatcgccagcaacaatggcggcaagcaagcgctcgaaacggtgcagcggctgttgccggtgctgtgccaggaccatggcctgaccccggaccaagtggtggctatcgccagcaacattggcggcaagcaagcgctcgaaacggtgcagcggctgttgccggtgctgtgccaggaccatggcctgaccccggaccaagtggtggctatcgccagcaacaatggcggcaagcaagcgctcgaaacggtgcagcggctgttgccggtgctgtgccaggaccatggcctgactccggaccaagtggtggctatcgccagccacgatggcggcaagcaagcgctcgaaacggtgcagcggctgttgccggtgctgtgccaggaccatggcctgactccggaccaagtggtggctatcgccagccacgatggcggcaagcaagcgctcgaaacggtgcagcggctgttgccggtgctgtgccaggaccatggcctgaccccggaccaagtggtggctatcgccagcaacattggcggcaagcaagcgctcgaaacggtgcagcggctgttgccggtgctgtgccaggaccatggcctgaccccggaccaagtggtggctatcgccagcaacaatggcggcaagcaagcgctcgaaacggtgcagcggctgttgccggtgctgtgccaggaccatggcctgaccccggaccaagtggtggctatcgccagcaacaatggcggcaagcaagcgctcgaaacggtgcagcggctgttgccggtgctgtgccaggaccatggcctgactccggaccaagtggtggctatcgccagccacgatggcggcaagcaagcgctcgaaacggtgcagcggctgttgccggtgctgtgccaggaccatggcctgaccccggaccaagtggtggctatcgccagcaacattggcggcaagcaagcgctcgaaagcattgtggcccagctgagccggcctgatccggcgttggccgcgttgaccaacgaccacctcgtcgccttggcctgcctcggcggacgtcctgccatggatgcagtgaaaaagggattgccgcacgcgccggaattgatcagaagagtcaatcgccgtattggcgaacgcacgtcccatcgcgttgcctatccctatgacgtgcccgattatgccagcctgggcagcggctcccccaagaaaaaacgcaaggtggaagatcctaagaaaaagcggaaagtggacggcattggtagtgggagcaacggcagcagcggagaggaactgctgagcaagaactaccacctggaaaacgaggtggccagactgaagaaaggctctggctctggcggaagcggttctggcggatcaggatctggaagtggcggctctggaagcggaggttctggatctggcgaagaactgctgtctaagaattatcacggttcaggctccggccagcggggaagcaagcgcaccgccgatggttccgagttcgaaagccccaaaaaaaagcgcaaggtctgataataggatcccaagcacgcagcaatgcagctcaaaacgcttagcctagccacacccccacgggaaacagcagtgattaacctttagcaataaacgaaagtttaactaagctatactaaccccagggttggtcaatttcgtgccagccacaccctggtactgcatgcacgcaatgctagctgcccctttcccgtcctgggcaccccgagtctcccccgaccccgggtcccaggtatgctcccacctccacctgccccactcaccacctctgctagttccagacacctccgagacgaggaaaaaaaaaaaaaaaaaaaaaaaaaaaaaaaaaaaaaaaaaaaaaaaaaaaaaaaaaaaaaaaaaaaaaaaaaaaaaaaaaaaaaaaaaaaaaaaaaaaaaaaaaaaaaaaaaaaaaaaa

SEQ ID NO: 355 - RNA, 6631 nt, synthetic construct
  misc_feature 1..6631: note = mRNA of V50_3xGCN4-TALE HPT8-ZIM3-P2A-D3a-hD3L-XTEN80-scFv
  source 1..6631: mol_type = other RNA
aggactcactatttgttttcgcgcccagttgcaaaaagtgtcgacatttgcttctgacacaactgtgttcactagcaacctcaaacagacaccgccaccatgcctgctgctaagagagtgaaactggatggatccgaggaactgctgagcaagaactaccacctggaaaacgaggtggccagactgaagaaaggctctggctctggcggaagcggttctggcggatcaggatctggaagtggcggctctggaagcggaggttctggatctggcgaagaactgctgtctaagaattatcacctcgagaacgaagtggctcggctcaagaaaggcagtggcagcggaggaagtggatccggcggtagtggtagtggaagcggcggatccggctcaggcggatctggttcaggggaagaactcctctccaaaaactaccatctcgagaatgaggtcgcccgcctgaaaaaaggatcaggttccggtggttctggcagcggtggttcaggctcaggcagcggcggtagcggtagcggtggaagcggaagcggaccaaaaaagaagagaaaggtaatggtggatctacgcacgctcggctacagccagcagcaacaggagaagatcaaaccgaaggttcgttcgacagtggcgcagcaccacgaggcactggtcggccatgggtttacacacgcgcacatcgttgcgctcagccaacacccggcagcgttagggaccgtcgctgtcaagtatcaggacatgatcgcagcgttgccagaggcgacacacgaagcgatcgttggcgtcggcaaacagtggtccggcgcacgcgctctggaggccttgctcacggtggcgggagagttgagaggtccaccgttacagttggacacaggccaacttctcaagattgcaaaacgtggcggcgtgaccgcagtggaggcagtgcatgcatggcgcaatgcactgacgggtgcccccctgaacctgaccccggaccaagtggtggctatcgccagcaacggtggcggcaagcaagcgctcgaaacggtgcagcggctgttgccggtgctgtgccaggaccatggcctgactccggaccaagtggtggctatcgccagccacgatggcggcaagcaagcgctcgaaacggtgcagcggctgttgccggtgctgtgccaggaccatggcctgaccccggaccaagtggtggctatcgccagcaacattggcggcaagcaagcgctcgaaacggtgcagcggctgttgccggtgctgtgccaggaccatggcctgaccccggaccaagtggtggctatcgccagcaacaatggcggcaagcaagcgctcgaaacggtgcagcggctgttgccggtgctgtgccaggaccatggcctgaccccggaccaagtggtggctatcgccagcaacggtggcggcaagcaagcgctcgaaacggtgcagcggctgttgccggtgctgtgccaggaccatggcctgaccccggaccaagtggtggctatcgccagcaacggtggcggcaagcaagcgctcgaaacggtgcagcggctgttgccggtgctgtgccaggaccatggcctgactccggaccaagtggtggctatcgccagccacgatggcggcaagcaagcgctcgaaacggtgcagcggctgttgccggtgctgtgccaggaccatggcctgaccccggaccaagtggtggctatcgccagcaacattggcggcaagcaagcgctcgaaacggtgcagcggctgttgccggtgctgtgccaggaccatggcctgaccccggaccaagtggtggctatcgccagcaacaatggcggcaagcaagcgctcgaaacggtgcagcggctgttgccggtgctgtgccaggaccatggcctgaccccggaccaagtggtggctatcgccagcaacaatggcggcaagcaagcgctcgaaacggtgcagcggctgttgccggtgctgtgccaggaccatggcctgaccccggaccaagtggtggctatcgccagcaacaatggcggcaagcaagcgctcgaaacggtgcagcggctgttgccggtgctgtgccaggaccatggcctgaccccggaccaagtggtggctatcgccagcaacggtggcggcaagcaagcgctcgaaacggtgcagcggctgttgccggtgctgtgccaggaccatggcctgactccggaccaagtggtggctatcgccagccacgatggcggcaagcaagcgctcgaaacggtgcagcggctgttgccggtgctgtgccaggaccatggcctgaccccggaccaagtggtggctatcgccagcaacggtggcggcaagcaagcgctcgaaacggtgcagcggctgttgccggtgctgtgccaggaccatggcctgaccccggaccaagtggtggctatcgccagcaacaatggcggcaagcaagcgctcgaaacggtgcagcggctgttgccggtgctgtgccaggaccatggcctgaccccggaccaagtggtggctatcgccagcaacattggcggcaagcaagcgctcgaaacggtgcagcggctgttgccggtgctgtgccaggaccatggcctgaccccggaccaagtggtggctatcgccagcaacaatggcggcaagcaagcgctcgaaacggtgcagcggctgttgccggtgctgtgccaggaccatggcctgaccccggaccaagtggtggctatcgccagccacgatggcggcaagcaagcgctcgaaagcattgtggcccagctgagccggcctgatccggcgttggccgcgttgaccaacgaccacctcgtcgccttggcctgcctcggcggacgtcctgccatggatgcagtgaaaaagggattgccgcacgcgccggaattgatcagaagagtcaatcgccgtattggcgaacgcacgtcccatcgcgttgcctatccctatgacgtgcccgattatgccagcctgggcagcggctcccccaagaaaaaacgcaaggtggaagatcctaagaaaaagcggaaagtggacggcagcggcagcgagacccccggtaccagcgagagcgccacccccgagagcatgaacaattcccagggaagagtgaccttcgaggatgtcactgtgaacttcacccagggggagtggcagcggctgaatcccgaacagagaaacttgtacagggatgtgatgctggagaattacagcaaccttgtctctgtgggacaaggggaaaccaccaaacccgatgtgatcttgaggttggaacaaggaaaggagccatggttggaggaagaggaagtgctgggaagtggccgtgcagaaaaaaatggggacattggagggcagatttggaagccaaaggatgtgaaagagagtctcctcgagggaagcggagctactaacttcagcctgctgaagcaggctggagacgtggaggagaaccctggacctatgcctgctgctaagagagtgaaactggatggatccaaccatgaccaggaatttgaccccccaaaggtttacccacctgtgccagctgagaagaggaagcccatccgcgtgctgtctctctttgatgggattgctacagggctcctggtgctgaaggacctgggcatccaagtggaccgctacattgcctccgaggtgtgtgaggactccatcacggtgggcatggtgcggcaccagggaaagatcatgtacgtcggggacgtccgcagcgtcacacagaagcatatccaggagtggggcccattcgacctggtgattggaggcagtccctgcaatgacctctccattgtcaaccctgcccgcaagggactttatgagggtactggccgcctcttctttgagttctaccgcctcctgcatgatgcgcggcccaaggagggagatgatcgccccttcttctggctctttgagaatgtggtggccatgggcgttagtgacaagagggacatctcgcgatttcttgagtctaaccccgtgatgattgacgccaaagaagtgtctgctgcacacagggcccgttacttctggggtaaccttcctggcatgaacaggcctttggcatccactgtgaatgataagctggagctgcaagagtgtctggagcacggcagaatagccaagttcagcaaagtgaggaccattaccaccaggtcaaactctataaagcagggcaaagaccagcatttccccgtgttcatgaacgagaaggaggacatcctgtggtgcactgaaatggaaagggtgtttggcttccccgtccactacacagacgtctccaacatgagccgcttggcgaggcagagactgctgggccgatcgtggagcgtgccggtcatccgccacctcttcgctccgctgaaggaatattttgcttgtgtgtctagcggcaatagtaacgctaacagccgcgggccgagcttcagcagcggcctggtgccgttaagcttgcgcggcagccatatgttcgaaaccgtgcctgtgtggaggagacagccagtccgggtgctgtccctttttgaagacatcaagaaagagctgacgagtttgggctttttggaaagtggttctgacccgggacaactgaagcatgtggttgatgtcacagacacagtgaggaaggatgtggaggagtggggacccttcgatcttgtgtacggcgccacacctcccctgggccacacctgtgaccgtcctcccagctggtacctgttccagttccaccggctcctgcagtacgcacggcccaagccaggcagccccaggcccttcttctggatgttcgtggacaatctggtgctgaacaaggaagacctggacgtcgcatctcgcttcctggagatggagccagtcaccatcccagatgtccacggcggatccttgcagaatgctgtccgcgtgtggagcaacatcccagccataaggagcagcaggcactgggctctggtttcggaagaagaattgtccctgctggcccagaacaagcagagctcgaagctcgcggccaagtggcccaccaagctggtgaagaactgctttctccccctaagagaatatttcaagtatttttcaggagggccgagctctggcgcacccccaccaagtggagggtctcctgccgggtccccaacatctactgaagaaggcaccagcgaatccgcaacgcccgagtcaggccctggtacctccacagaaccatctgaaggtagtgcgcctggttccccagctggaagccctacttccaccgaagaaggcacgtcaaccgaaccaagtgaaggatctgcccctgggaccagcactgaaccatctgagccaaaaaagaagagaaaggtaccatctgagggccccgacatcgtgatgacccagagccccagcagcctgagcgccagcgtgggcgaccgcgtgaccatcacctgccgcagcagcaccggcgccgtgaccaccagcaactacgccagctgggtgcaggagaagcccggcaagctgttcaagggcctgatcggcggcaccaacaaccgcgcccccggcgtgcccagccgcttcagcggcagcctgatcggcgacaaggccaccctgaccatcagcagcctgcagcccgaggacttcgccacctacttctgcgccctgtggtacagcaaccactgggtgttcggccagggcaccaaggtggagctgaagcgcggcggcggcggcagcggcggcggcggcagcggcggcggcggcagcagcggcggcggcagcgaggtgaagctgctggagagcggcggcggcctggtgcagcccggcggcagcctgaagctgagctgcgccgtgagcggcttcagcctgaccgactacggcgtgaactgggtgcgccaggcccccggccgcggcctggagtggatcggcgtgatctggggcgacggcatcaccgactacaacagcgccctgaaggaccgcttcatcatcagcaaggacaacggcaagaacaccgtgtacctgcagatgagcaaggtgcgcagcgacgacaccgccctgtactactgcgtgaccggcctgttcgactactggggccagggcaccctggtgaccgtgagcagctacccatacgatgttccagattacgctggtggaggcggaggttctgggggaggaggtagtggcggtggtggttcaggaggcggcggaagctgataataggatcccaagcacgcagcaatgcagctcaaaacgcttagcctagccacacccccacgggaaacagcagtgattaacctttagcaataaacgaaagtttaactaagctatactaaccccagggttggtcaatttcgtgccagccacaccctggtactgcatgcacgcaatgctagctgcccctttcccgtcctgggcaccccgagtctcccccgaccccgggtcccaggtatgctcccacctccacctgccccactcaccacctctgctagttccagacacctccgagacgaggaaaaaaaaaaaaaaaaaaaaaaaaaaaaaaaaaaaaaaaaaaaaaaaaaaaaaaaaaaaaaaaaaaaaaaaaaaaaaaaaaaaaaaaaaaaaaaaaaaaaaaaaaaaaaaaaaaaaaaaa

SEQ ID NO: 356 - RNA, 6631 nt, synthetic construct
  misc_feature 1..6631: note = mRNA of V51_3xGCN4-TALE HPT12-ZIM3-P2A-D3a-hD3L-XTEN80-scFv
  source 1..6631: mol_type = other RNA
aggactcactatttgttttcgcgcccagttgcaaaaagtgtcgacatttgcttctgacacaactgtgttcactagcaacctcaaacagacaccgccaccatgcctgctgctaagagagtgaaactggatggatccgaggaactgctgagcaagaactaccacctggaaaacgaggtggccagactgaagaaaggctctggctctggcggaagcggttctggcggatcaggatctggaagtggcggctctggaagcggaggttctggatctggcgaagaactgctgtctaagaattatcacctcgagaacgaagtggctcggctcaagaaaggcagtggcagcggaggaagtggatccggcggtagtggtagtggaagcggcggatccggctcaggcggatctggttcaggggaagaactcctctccaaaaactaccatctcgagaatgaggtcgcccgcctgaaaaaaggatcaggttccggtggttctggcagcggtggttcaggctcaggcagcggcggtagcggtagcggtggaagcggaagcggaccaaaaaagaagagaaaggtaatggtggatctacgcacgctcggctacagccagcagcaacaggagaagatcaaaccgaaggttcgttcgacagtggcgcagcaccacgaggcactggtcggccatgggtttacacacgcgcacatcgttgcgctcagccaacacccggcagcgttagggaccgtcgctgtcaagtatcaggacatgatcgcagcgttgccagaggcgacacacgaagcgatcgttggcgtcggcaaacagtggtccggcgcacgcgctctggaggccttgctcacggtggcgggagagttgagaggtccaccgttacagttggacacaggccaacttctcaagattgcaaaacgtggcggcgtgaccgcagtggaggcagtgcatgcatggcgcaatgcactgacgggtgcccccctgaacctgaccccggaccaagtggtggctatcgccagcaacaatggcggcaagcaagcgctcgaaacggtgcagcggctgttgccggtgctgtgccaggaccatggcctgaccccggaccaagtggtggctatcgccagcaacaatggcggcaagcaagcgctcgaaacggtgcagcggctgttgccggtgctgtgccaggaccatggcctgaccccggaccaagtggtggctatcgccagcaacattggcggcaagcaagcgctcgaaacggtgcagcggctgttgccggtgctgtgccaggaccatggcctgaccccggaccaagtggtggctatcgccagcaacaatggcggcaagcaagcgctcgaaacggtgcagcggctgttgccggtgctgtgccaggaccatggcctgaccccggaccaagtggtggctatcgccagcaacaatggcggcaagcaagcgctcgaaacggtgcagcggctgttgccggtgctgtgccaggaccatggcctgaccccggaccaagtggtggctatcgccagcaacattggcggcaagcaagcgctcgaaacggtgcagcggctgttgccggtgctgtgccaggaccatggcctgaccccggaccaagtggtggctatcgccagcaacaatggcggcaagcaagcgctcgaaacggtgcagcggctgttgccggtgctgtgccaggaccatggcctgaccccggaccaagtggtggctatcgccagcaacggtggcggcaagcaagcgctcgaaacggtgcagcggctgttgccggtgctgtgccaggaccatggcctgaccccggaccaagtggtggctatcgccagcaacaatggcggcaagcaagcgctcgaaacggtgcagcggctgttgccggtgctgtgccaggaccatggcctgaccccggaccaagtggtggctatcgccagcaacattggcggcaagcaagcgctcgaaacggtgcagcggctgttgccggtgctgtgccaggaccatggcctgaccccggaccaagtggtggctatcgccagcaacaatggcggcaagcaagcgctcgaaacggtgcagcggctgttgccggtgctgtgccaggaccatggcctgactccggaccaagtggtggctatcgccagccacgatggcggcaagcaagcgctcgaaacggtgcagcggctgttgccggtgctgtgccaggaccatggcctgactccggaccaagtggtggctatcgccagccacgatggcggcaagcaagcgctcgaaacggtgcagcggctgttgccggtgctgtgccaggaccatggcctgaccccggaccaagtggtggctatcgccagcaacattggcggcaagcaagcgctcgaaacggtgcagcggctgttgccggtgctgtgccaggaccatggcctgaccccggaccaagtggtggctatcgccagcaacaatggcggcaagcaagcgctcgaaacggtgcagcggctgttgccggtgctgtgccaggaccatggcctgaccccggaccaagtggtggctatcgccagcaacaatggcggcaagcaagcgctcgaaacggtgcagcggctgttgccggtgctgtgccaggaccatggcctgactccggaccaagtggtggctatcgccagccacgatggcggcaagcaagcgctcgaaacggtgcagcggctgttgccggtgctgtgccaggaccatggcctgaccccggaccaagtggtggctatcgccagcaacattggcggcaagcaagcgctcgaaagcattgtggcccagctgagccggcctgatccggcgttggccgcgttgaccaacgaccacctcgtcgccttggcctgcctcggcggacgtcctgccatggatgcagtgaaaaagggattgccgcacgcgccggaattgatcagaagagtcaatcgccgtattggcgaacgcacgtcccatcgcgttgcctatccctatgacgtgcccgattatgccagcctgggcagcggctcccccaagaaaaaacgcaaggtggaagatcctaagaaaaagcggaaagtggacggcagcggcagcgagacccccggtaccagcgagagcgccacccccgagagcatgaacaattcccagggaagagtgaccttcgaggatgtcactgtgaacttcacccagggggagtggcagcggctgaatcccgaacagagaaacttgtacagggatgtgatgctggagaattacagcaaccttgtctctgtgggacaaggggaaaccaccaaacccgatgtgatcttgaggttggaacaaggaaaggagccatggttggaggaagaggaagtgctgggaagtggccgtgcagaaaaaaatggggacattggagggcagatttggaagccaaaggatgtgaaagagagtctcctcgagggaagcggagctactaacttcagcctgctgaagcaggctggagacgtggaggagaaccctggacctatgcctgctgctaagagagtgaaactggatggatccaaccatgaccaggaatttgaccccccaaaggtttacccacctgtgccagctgagaagaggaagcccatccgcgtgctgtctctctttgatgggattgctacagggctcctggtgctgaaggacctgggcatccaagtggaccgctacattgcctccgaggtgtgtgaggactccatcacggtgggcatggtgcggcaccagggaaagatcatgtacgtcggggacgtccgcagcgtcacacagaagcatatccaggagtggggcccattcgacctggtgattggaggcagtccctgcaatgacctctccattgtcaaccctgcccgcaagggactttatgagggtactggccgcctcttctttgagttctaccgcctcctgcatgatgcgcggcccaaggagggagatgatcgccccttcttctggctctttgagaatgtggtggccatgggcgttagtgacaagagggacatctcgcgatttcttgagtctaaccccgtgatgattgacgccaaagaagtgtctgctgcacacagggcccgttacttctggggtaaccttcctggcatgaacaggcctttggcatccactgtgaatgataagctggagctgcaagagtgtctggagcacggcagaatagccaagttcagcaaagtgaggaccattaccaccaggtcaaactctataaagcagggcaaagaccagcatttccccgtgttcatgaacgagaaggaggacatcctgtggtgcactgaaatggaaagggtgtttggcttccccgtccactacacagacgtctccaacatgagccgcttggcgaggcagagactgctgggccgatcgtggagcgtgccggtcatccgccacctcttcgctccgctgaaggaatattttgcttgtgtgtctagcggcaatagtaacgctaacagccgcgggccgagcttcagcagcggcctggtgccgttaagcttgcgcggcagccatatgttcgaaaccgtgcctgtgtggaggagacagccagtccgggtgctgtccctttttgaagacatcaagaaagagctgacgagtttgggctttttggaaagtggttctgacccgggacaactgaagcatgtggttgatgtcacagacacagtgaggaaggatgtggaggagtggggacccttcgatcttgtgtacggcgccacacctcccctgggccacacctgtgaccgtcctcccagctggtacctgttccagttccaccggctcctgcagtacgcacggcccaagccaggcagccccaggcccttcttctggatgttcgtggacaatctggtgctgaacaaggaagacctggacgtcgcatctcgcttcctggagatggagccagtcaccatcccagatgtccacggcggatccttgcagaatgctgtccgcgtgtggagcaacatcccagccataaggagcagcaggcactgggctctggtttcggaagaagaattgtccctgctggcccagaacaagcagagctcgaagctcgcggccaagtggcccaccaagctggtgaagaactgctttctccccctaagagaatatttcaagtatttttcaggagggccgagctctggcgcacccccaccaagtggagggtctcctgccgggtccccaacatctactgaagaaggcaccagcgaatccgcaacgcccgagtcaggccctggtacctccacagaaccatctgaaggtagtgcgcctggttccccagctggaagccctacttccaccgaagaaggcacgtcaaccgaaccaagtgaaggatctgcccctgggaccagcactgaaccatctgagccaaaaaagaagagaaaggtaccatctgagggccccgacatcgtgatgacccagagccccagcagcctgagcgccagcgtgggcgaccgcgtgaccatcacctgccgcagcagcaccggcgccgtgaccaccagcaactacgccagctgggtgcaggagaagcccggcaagctgttcaagggcctgatcggcggcaccaacaaccgcgcccccggcgtgcccagccgcttcagcggcagcctgatcggcgacaaggccaccctgaccatcagcagcctgcagcccgaggacttcgccacctacttctgcgccctgtggtacagcaaccactgggtgttcggccagggcaccaaggtggagctgaagcgcggcggcggcggcagcggcggcggcggcagcggcggcggcggcagcagcggcggcggcagcgaggtgaagctgctggagagcggcggcggcctggtgcagcccggcggcagcctgaagctgagctgcgccgtgagcggcttcagcctgaccgactacggcgtgaactgggtgcgccaggcccccggccgcggcctggagtggatcggcgtgatctggggcgacggcatcaccgactacaacagcgccctgaaggaccgcttcatcatcagcaaggacaacggcaagaacaccgtgtacctgcagatgagcaaggtgcgcagcgacgacaccgccctgtactactgcgtgaccggcctgttcgactactggggccagggcaccctggtgaccgtgagcagctacccatacgatgttccagattacgctggtggaggcggaggttctgggggaggaggtagtggcggtggtggttcaggaggcggcggaagctgataataggatcccaagcacgcagcaatgcagctcaaaacgcttagcctagccacacccccacgggaaacagcagtgattaacctttagcaataaacgaaagtttaactaagctatactaaccccagggttggtcaatttcgtgccagccacaccctggtactgcatgcacgcaatgctagctgcccctttcccgtcctgggcaccccgagtctcccccgaccccgggtcccaggtatgctcccacctccacctgccccactcaccacctctgctagttccagacacctccgagacgaggaaaaaaaaaaaaaaaaaaaaaaaaaaaaaaaaaaaaaaaaaaaaaaaaaaaaaaaaaaaaaaaaaaaaaaaaaaaaaaaaaaaaaaaaaaaaaaaaaaaaaaaaaaaaaaaaaaaaaaaa

SEQ ID NO: 357 - DNA, 5919 bp, synthetic construct
  misc_feature 1..5919: note = CDS of V48_scFv-ZIM3-P2A-D3a-hD3L-XTEN80-TALE HPT8-1xGCN4
  source 1..5919: mol_type = other DNA
atgcctgctgctaagagagtgaaactggatggatccggccccgacatcgtgatgacccagagccccagcagcctgagcgccagcgtgggcgaccgcgtgaccatcacctgccgcagcagcaccggcgccgtgaccaccagcaactacgccagctgggtgcaggagaagcccggcaagctgttcaagggcctgatcggcggcaccaacaaccgcgcccccggcgtgcccagccgcttcagcggcagcctgatcggcgacaaggccaccctgaccatcagcagcctgcagcccgaggacttcgccacctacttctgcgccctgtggtacagcaaccactgggtgttcggccagggcaccaaggtggagctgaagcgcggcggcggcggcagcggcggcggcggcagcggcggcggcggcagcagcggcggcggcagcgaggtgaagctgctggagagcggcggcggcctggtgcagcccggcggcagcctgaagctgagctgcgccgtgagcggcttcagcctgaccgactacggcgtgaactgggtgcgccaggcccccggccgcggcctggagtggatcggcgtgatctggggcgacggcatcaccgactacaacagcgccctgaaggaccgcttcatcatcagcaaggacaacggcaagaacaccgtgtacctgcagatgagcaaggtgcgcagcgacgacaccgccctgtactactgcgtgaccggcctgttcgactactggggccagggcaccctggtgaccgtgagcagctacccatacgatgttccagattacgctggtggaggcggaggttctgggggaggaggtagtggcggtggtggttcaggaggcggcggaagcttggatccaggtggaggtggaagcggtatgaacaattcccagggaagagtgaccttcgaggacgtgaccgtgaacttcacccaaggcgagtggcagagactgaaccccgagcagagaaacctgtaccgggacgtgatgctggaaaactacagcaacctggtgtccgtcggccagggcgagacaacaaagcctgacgtgatcctgcggctggaacagggcaaagagccttggctggaagaggaagaggtgctcggatctggcagagccgagaagaatggcgatatcggcggacagatctggaagccaaaggatgtgaaagagagtctcggaagcggagctactaacttcagcctgctgaagcaggctggagacgtggaggagaaccctggacctatgcctgctgctaagagagtgaaactggatggatccaaccatgaccaggaatttgaccccccaaaggtttacccacctgtgccagctgagaagaggaagcccatccgcgtgctgtctctctttgatgggattgctacagggctcctggtgctgaaggacctgggcatccaagtggaccgctacattgcctccgaggtgtgtgaggactccatcacggtgggcatggtgcggcaccagggaaagatcatgtacgtcggggacgtccgcagcgtcacacagaagcatatccaggagtggggcccattcgacctggtgattggaggcagtccctgcaatgacctctccattgtcaaccctgcccgcaagggactttatgagggtactggccgcctcttctttgagttctaccgcctcctgcatgatgcgcggcccaaggagggagatgatcgccccttcttctggctctttgagaatgtggtggccatgggcgttagtgacaagagggacatctcgcgatttcttgagtctaaccccgtgatgattgacgccaaagaagtgtctgctgcacacagggcccgttacttctggggtaaccttcctggcatgaacaggcctttggcatccactgtgaatgataagctggagctgcaagagtgtctggagcacggcagaatagccaagttcagcaaagtgaggaccattaccaccaggtcaaactctataaagcagggcaaagaccagcatttccccgtgttcatgaacgagaaggaggacatcctgtggtgcactgaaatggaaagggtgtttggcttccccgtccactacacagacgtctccaacatgagccgcttggcgaggcagagactgctgggccgatcgtggagcgtgccggtcatccgccacctcttcgctccgctgaaggaatattttgcttgtgtgtctagcggcaatagtaacgctaacagccgcgggccgagcttcagcagcggcctggtgccgttaagcttgcgcggcagccatatgttcgaaaccgtgcctgtgtggaggagacagccagtccgggtgctgtccctttttgaagacatcaagaaagagctgacgagtttgggctttttggaaagtggttctgacccgggacaactgaagcatgtggttgatgtcacagacacagtgaggaaggatgtggaggagtggggacccttcgatcttgtgtacggcgccacacctcccctgggccacacctgtgaccgtcctcccagctggtacctgttccagttccaccggctcctgcagtacgcacggcccaagccaggcagccccaggcccttcttctggatgttcgtggacaatctggtgctgaacaaggaagacctggacgtcgcatctcgcttcctggagatggagccagtcaccatcccagatgtccacggcggatccttgcagaatgctgtccgcgtgtggagcaacatcccagccataaggagcagcaggcactgggctctggtttcggaagaagaattgtccctgctggcccagaacaagcagagctcgaagctcgcggccaagtggcccaccaagctggtgaagaactgctttctccccctaagagaatatttcaagtatttttcaggagggccgagctctggcgcacccccaccaagtggagggtctcctgccgggtccccaacatctactgaagaaggcaccagcgaatccgcaacgcccgagtcaggccctggtacctccacagaaccatctgaaggtagtgcgcctggttccccagctggaagccctacttccaccgaagaaggcacgtcaaccgaaccaagtgaaggatctgcccctgggaccagcactgaaccatctgagccaaaaaagaagagaaaggtaatggtggatctacgcacgctcggctacagccagcagcaacaggagaagatcaaaccgaaggttcgttcgacagtggcgcagcaccacgaggcactggtcggccatgggtttacacacgcgcacatcgttgcgctcagccaacacccggcagcgttagggaccgtcgctgtcaagtatcaggacatgatcgcagcgttgccagaggcgacacacgaagcgatcgttggcgtcggcaaacagtggtccggcgcacgcgctctggaggccttgctcacggtggcgggagagttgagaggtccaccgttacagttggacacaggccaacttctcaagattgcaaaacgtggcggcgtgaccgcagtggaggcagtgcatgcatggcgcaatgcactgacgggtgcccccctgaacctgaccccggaccaagtggtggctatcgccagcaacggtggcggcaagcaagcgctcgaaacggtgcagcggctgttgccggtgctgtgccaggaccatggcctgactccggaccaagtggtggctatcgccagccacgatggcggcaagcaagcgctcgaaacggtgcagcggctgttgccggtgctgtgccaggaccatggcctgaccccggaccaagtggtggctatcgccagcaacattggcggcaagcaagcgctcgaaacggtgcagcggctgttgccggtgctgtgccaggaccatggcctgaccccggaccaagtggtggctatcgccagcaacaatggcggcaagcaagcgctcgaaacggtgcagcggctgttgccggtgctgtgccaggaccatggcctgaccccggaccaagtggtggctatcgccagcaacggtggcggcaagcaagcgctcgaaacggtgcagcggctgttgccggtgctgtgccaggaccatggcctgaccccggaccaagtggtggctatcgccagcaacggtggcggcaagcaagcgctcgaaacggtgcagcggctgttgccggtgctgtgccaggaccatggcctgactccggaccaagtggtggctatcgccagccacgatggcggcaagcaagcgctcgaaacggtgcagcggctgttgccggtgctgtgccaggaccatggcctgaccccggaccaagtggtggctatcgccagcaacattggcggcaagcaagcgctcgaaacggtgcagcggctgttgccggtgctgtgccaggaccatggcctgaccccggaccaagtggtggctatcgccagcaacaatggcggcaagcaagcgctcgaaacggtgcagcggctgttgccggtgctgtgccaggaccatggcctgaccccggaccaagtggtggctatcgccagcaacaatggcggcaagcaagcgctcgaaacggtgcagcggctgttgccggtgctgtgccaggaccatggcctgaccccggaccaagtggtggctatcgccagcaacaatggcggcaagcaagcgctcgaaacggtgcagcggctgttgccggtgctgtgccaggaccatggcctgaccccggaccaagtggtggctatcgccagcaacggtggcggcaagcaagcgctcgaaacggtgcagcggctgttgccggtgctgtgccaggaccatggcctgactccggaccaagtggtggctatcgccagccacgatggcggcaagcaagcgctcgaaacggtgcagcggctgttgccggtgctgtgccaggaccatggcctgaccccggaccaagtggtggctatcgccagcaacggtggcggcaagcaagcgctcgaaacggtgcagcggctgttgccggtgctgtgccaggaccatggcctgaccccggaccaagtggtggctatcgccagcaacaatggcggcaagcaagcgctcgaaacggtgcagcggctgttgccggtgctgtgccaggaccatggcctgaccccggaccaagtggtggctatcgccagcaacattggcggcaagcaagcgctcgaaacggtgcagcggctgttgccggtgctgtgccaggaccatggcctgaccccggaccaagtggtggctatcgccagcaacaatggcggcaagcaagcgctcgaaacggtgcagcggctgttgccggtgctgtgccaggaccatggcctgaccccggaccaagtggtggctatcgccagccacgatggcggcaagcaagcgctcgaaagcattgtggcccagctgagccggcctgatccggcgttggccgcgttgaccaacgaccacctcgtcgccttggcctgcctcggcggacgtcctgccatggatgcagtgaaaaagggattgccgcacgcgccggaattgatcagaagagtcaatcgccgtattggcgaacgcacgtcccatcgcgttgcctatccctatgacgtgcccgattatgccagcctgggcagcggctcccccaagaaaaaacgcaaggtggaagatcctaagaaaaagcggaaagtggacggcattggtagtgggagcaacggcagcagcggagaggaactgctgagcaagaactaccacctggaaaacgaggtggccagactgaagaaaggctctggctctggcggaagcggttctggcggatcaggatctggaagtggcggctctggaagcggaggttctggatctggcgaagaactgctgtctaagaattatcacggttcaggctccggccagcggggaagcaagcgcaccgccgatggttccgagttcgaaagccccaaaaaaaagcgcaaggtctga

SEQ ID NO: 358 - DNA, 5919 bp, synthetic construct
  misc_feature 1..5919: note = CDS of V49_scFv-ZIM3-P2A-D3a-hD3L-XTEN80-TALE HPT12-1xGCN4
  source 1..5919: mol_type = other DNA
atgcctgctgctaagagagtgaaactggatggatccggccccgacatcgtgatgacccagagccccagcagcctgagcgccagcgtgggcgaccgcgtgaccatcacctgccgcagcagcaccggcgccgtgaccaccagcaactacgccagctgggtgcaggagaagcccggcaagctgttcaagggcctgatcggcggcaccaacaaccgcgcccccggcgtgcccagccgcttcagcggcagcctgatcggcgacaaggccaccctgaccatcagcagcctgcagcccgaggacttcgccacctacttctgcgccctgtggtacagcaaccactgggtgttcggccagggcaccaaggtggagctgaagcgcggcggcggcggcagcggcggcggcggcagcggcggcggcggcagcagcggcggcggcagcgaggtgaagctgctggagagcggcggcggcctggtgcagcccggcggcagcctgaagctgagctgcgccgtgagcggcttcagcctgaccgactacggcgtgaactgggtgcgccaggcccccggccgcggcctggagtggatcggcgtgatctggggcgacggcatcaccgactacaacagcgccctgaaggaccgcttcatcatcagcaaggacaacggcaagaacaccgtgtacctgcagatgagcaaggtgcgcagcgacgacaccgccctgtactactgcgtgaccggcctgttcgactactggggccagggcaccctggtgaccgtgagcagctacccatacgatgttccagattacgctggtggaggcggaggttctgggggaggaggtagtggcggtggtggttcaggaggcggcggaagcttggatccaggtggaggtggaagcggtatgaacaattcccagggaagagtgaccttcgaggacgtgaccgtgaacttcacccaaggcgagtggcagagactgaaccccgagcagagaaacctgtaccgggacgtgatgctggaaaactacagcaacctggtgtccgtcggccagggcgagacaacaaagcctgacgtgatcctgcggctggaacagggcaaagagccttggctggaagaggaagaggtgctcggatctggcagagccgagaagaatggcgatatcggcggacagatctggaagccaaaggatgtgaaagagagtctcggaagcggagctactaacttcagcctgctgaagcaggctggagacgtggaggagaaccctggacctatgcctgctgctaagagagtgaaactggatggatccaaccatgaccaggaatttgaccccccaaaggtttacccacctgtgccagctgagaagaggaagcccatccgcgtgctgtctctctttgatgggattgctacagggctcctggtgctgaaggacctgggcatccaagtggaccgctacattgcctccgaggtgtgtgaggactccatcacggtgggcatggtgcggcaccagggaaagatcatgtacgtcggggacgtccgcagcgtcacacagaagcatatccaggagtggggcccattcgacctggtgattggaggcagtccctgcaatgacctctccattgtcaaccctgcccgcaagggactttatgagggtactggccgcctcttctttgagttctaccgcctcctgcatgatgcgcggcccaaggagggagatgatcgccccttcttctggctctttgagaatgtggtggccatgggcgttagtgacaagagggacatctcgcgatttcttgagtctaaccccgtgatgattgacgccaaagaagtgtctgctgcacacagggcccgttacttctggggtaaccttcctggcatgaacaggcctttggcatccactgtgaatgataagctggagctgcaagagtgtctggagcacggcagaatagccaagttcagcaaagtgaggaccattaccaccaggtcaaactctataaagcagggcaaagaccagcatttccccgtgttcatgaacgagaaggaggacatcctgtggtgcactgaaatggaaagggtgtttggcttccccgtccactacacagacgtctccaacatgagccgcttggcgaggcagagactgctgggccgatcgtggagcgtgccggtcatccgccacctcttcgctccgctgaaggaatattttgcttgtgtgtctagcggcaatagtaacgctaacagccgcgggccgagcttcagcagcggcctggtgccgttaagcttgcgcggcagccatatgttcgaaaccgtgcctgtgtggaggagacagccagtccgggtgctgtccctttttgaagacatcaagaaagagctgacgagtttgggctttttggaaagtggttctgacccgggacaactgaagcatgtggttgatgtcacagacacagtgaggaaggatgtggaggagtggggacccttcgatcttgtgtacggcgccacacctcccctgggccacacctgtgaccgtcctcccagctggtacctgttccagttccaccggctcctgcagtacgcacggcccaagccaggcagccccaggcccttcttctggatgttcgtggacaatctggtgctgaacaaggaagacctggacgtcgcatctcgcttcctggagatggagccagtcaccatcccagatgtccacggcggatccttgcagaatgctgtccgcgtgtggagcaacatcccagccataaggagcagcaggcactgggctctggtttcggaagaagaattgtccctgctggcccagaacaagcagagctcgaagctcgcggccaagtggcccaccaagctggtgaagaactgctttctccccctaagagaatatttcaagtatttttcaggagggccgagctctggcgcacccccaccaagtggagggtctcctgccgggtccccaacatctactgaagaaggcaccagcgaatccgcaacgcccgagtcaggccctggtacctccacagaaccatctgaaggtagtgcgcctggttccccagctggaagccctacttccaccgaagaaggcacgtcaaccgaaccaagtgaaggatctgcccctgggaccagcactgaaccatctgagccaaaaaagaagagaaaggtaatggtggatctacgcacgctcggctacagccagcagcaacaggagaagatcaaaccgaaggttcgttcgacagtggcgcagcaccacgaggcactggtcggccatgggtttacacacgcgcacatcgttgcgctcagccaacacccggcagcgttagggaccgtcgctgtcaagtatcaggacatgatcgcagcgttgccagaggcgacacacgaagcgatcgttggcgtcggcaaacagtggtccggcgcacgcgctctggaggccttgctcacggtggcgggagagttgagaggtccaccgttacagttggacacaggccaacttctcaagattgcaaaacgtggcggcgtgaccgcagtggaggcagtgcatgcatggcgcaatgcactgacgggtgcccccctgaacctgaccccggaccaagtggtggctatcgccagcaacaatggcggcaagcaagcgctcgaaacggtgcagcggctgttgccggtgctgtgccaggaccatggcctgaccccggaccaagtggtggctatcgccagcaacaatggcggcaagcaagcgctcgaaacggtgcagcggctgttgccggtgctgtgccaggaccatggcctgaccccggaccaagtggtggctatcgccagcaacattggcggcaagcaagcgctcgaaacggtgcagcggctgttgccggtgctgtgccaggaccatggcctgaccccggaccaagtggtggctatcgccagcaacaatggcggcaagcaagcgctcgaaacggtgcagcggctgttgccggtgctgtgccaggaccatggcctgaccccggaccaagtggtggctatcgccagcaacaatggcggcaagcaagcgctcgaaacggtgcagcggctgttgccggtgctgtgccaggaccatggcctgaccccggaccaagtggtggctatcgccagcaacattggcggcaagcaagcgctcgaaacggtgcagcggctgttgccggtgctgtgccaggaccatggcctgaccccggaccaagtggtggctatcgccagcaacaatggcggcaagcaagcgctcgaaacggtgcagcggctgttgccggtgctgtgccaggaccatggcctgaccccggaccaagtggtggctatcgccagcaacggtggcggcaagcaagcgctcgaaacggtgcagcggctgttgccggtgctgtgccaggaccatggcctgaccccggaccaagtggtggctatcgccagcaacaatggcggcaagcaagcgctcgaaacggtgcagcggctgttgccggtgctgtgccaggaccatggcctgaccccggaccaagtggtggctatcgccagcaacattggcggcaagcaagcgctcgaaacggtgcagcggctgttgccggtgctgtgccaggaccatggcctgaccccggaccaagtggtggctatcgccagcaacaatggcggcaagcaagcgctcgaaacggtgcagcggctgttgccggtgctgtgccaggaccatggcctgactccggaccaagtggtggctatcgccagccacgatggcggcaagcaagcgctcgaaacggtgcagcggctgttgccggtgctgtgccaggaccatggcctgactccggaccaagtggtggctatcgccagccacgatggcggcaagcaagcgctcgaaacggtgcagcggctgttgccggtgctgtgccaggaccatggcctgaccccggaccaagtggtggctatcgccagcaacattggcggcaagcaagcgctcgaaacggtgcagcggctgttgccggtgctgtgccaggaccatggcctgaccccggaccaagtggtggctatcgccagcaacaatggcggcaagcaagcgctcgaaacggtgcagcggctgttgccggtgctgtgccaggaccatggcctgaccccggaccaagtggtggctatcgccagcaacaatggcggcaagcaagcgctcgaaacggtgcagcggctgttgccggtgctgtgccaggaccatggcctgactccggaccaagtggtggctatcgccagccacgatggcggcaagcaagcgctcgaaacggtgcagcggctgttgccggtgctgtgccaggaccatggcctgaccccggaccaagtggtggctatcgccagcaacattggcggcaagcaagcgctcgaaagcattgtggcccagctgagccggcctgatccggcgttggccgcgttgaccaacgaccacctcgtcgccttggcctgcctcggcggacgtcctgccatggatgcagtgaaaaagggattgccgcacgcgccggaattgatcagaagagtcaatcgccgtattggcgaacgcacgtcccatcgcgttgcctatccctatgacgtgcccgattatgccagcctgggcagcggctcccccaagaaaaaacgcaaggtggaagatcctaagaaaaagcggaaagtggacggcattggtagtgggagcaacggcagcagcggagaggaactgctgagcaagaactaccacctggaaaacgaggtggccagactgaagaaaggctctggctctggcggaagcggttctggcggatcaggatctggaagtggcggctctggaagcggaggttctggatctggcgaagaactgctgtctaagaattatcacggttcaggctccggccagcggggaagcaagcgcaccgccgatggttccgagttcgaaagccccaaaaaaaagcgcaaggtctga

SEQ ID NO: 359 - DNA, 6114 bp, synthetic construct
  misc_feature 1..6114: note = CDS of V50_3xGCN4-TALE HPT8-ZIM3-P2A-D3a-hD3L-XTEN80-scFv
  source 1..6114: mol_type = other DNA
atgcctgctgctaagagagtgaaactggatggatccgaggaactgctgagcaagaactaccacctggaaaacgaggtggccagactgaagaaaggctctggctctggcggaagcggttctggcggatcaggatctggaagtggcggctctggaagcggaggttctggatctggcgaagaactgctgtctaagaattatcacctcgagaacgaagtggctcggctcaagaaaggcagtggcagcggaggaagtggatccggcggtagtggtagtggaagcggcggatccggctcaggcggatctggttcaggggaagaactcctctccaaaaactaccatctcgagaatgaggtcgcccgcctgaaaaaaggatcaggttccggtggttctggcagcggtggttcaggctcaggcagcggcggtagcggtagcggtggaagcggaagcggaccaaaaaagaagagaaaggtaatggtggatctacgcacgctcggctacagccagcagcaacaggagaagatcaaaccgaaggttcgttcgacagtggcgcagcaccacgaggcactggtcggccatgggtttacacacgcgcacatcgttgcgctcagccaacacccggcagcgttagggaccgtcgctgtcaagtatcaggacatgatcgcagcgttgccagaggcgacacacgaagcgatcgttggcgtcggcaaacagtggtccggcgcacgcgctctggaggccttgctcacggtggcgggagagttgagaggtccaccgttacagttggacacaggccaacttctcaagattgcaaaacgtggcggcgtgaccgcagtggaggcagtgcatgcatggcgcaatgcactgacgggtgcccccctgaacctgaccccggaccaagtggtggctatcgccagcaacggtggcggcaagcaagcgctcgaaacggtgcagcggctgttgccggtgctgtgccaggaccatggcctgactccggaccaagtggtggctatcgccagccacgatggcggcaagcaagcgctcgaaacggtgcagcggctgttgccggtgctgtgccaggaccatggcctgaccccggaccaagtggtggctatcgccagcaacattggcggcaagcaagcgctcgaaacggtgcagcggctgttgccggtgctgtgccaggaccatggcctgaccccggaccaagtggtggctatcgccagcaacaatggcggcaagcaagcgctcgaaacggtgcagcggctgttgccggtgctgtgccaggaccatggcctgaccccggaccaagtggtggctatcgccagcaacggtggcggcaagcaagcgctcgaaacggtgcagcggctgttgccggtgctgtgccaggaccatggcctgaccccggaccaagtggtggctatcgccagcaacggtggcggcaagcaagcgctcgaaacggtgcagcggctgttgccggtgctgtgccaggaccatggcctgactccggaccaagtggtggctatcgccagccacgatggcggcaagcaagcgctcgaaacggtgcagcggctgttgccggtgctgtgccaggaccatggcctgaccccggaccaagtggtggctatcgccagcaacattggcggcaagcaagcgctcgaaacggtgcagcggctgttgccggtgctgtgccaggaccatggcctgaccccggaccaagtggtggctatcgccagcaacaatggcggcaagcaagcgctcgaaacggtgcagcggctgttgccggtgctgtgccaggaccatggcctgaccccggaccaagtggtggctatcgccagcaacaatggcggcaagcaagcgctcgaaacggtgcagcggctgttgccggtgctgtgccaggaccatggcctgaccccggaccaagtggtggctatcgccagcaacaatggcggcaagcaagcgctcgaaacggtgcagcggctgttgccggtgctgtgccaggaccatggcctgaccccggaccaagtggtggctatcgccagcaacggtggcggcaagcaagcgctcgaaacggtgcagcggctgttgccggtgctgtgccaggaccatggcctgactccggaccaagtggtggctatcgccagccacgatggcggcaagcaagcgctcgaaacggtgcagcggctgttgccggtgctgtgccaggaccatggcctgaccccggaccaagtggtggctatcgccagcaacggtggcggcaagcaagcgctcgaaacggtgcagcggctgttgccggtgctgtgccaggaccatggcctgaccccggaccaagtggtggctatcgccagcaacaatggcggcaagcaagcgctcgaaacggtgcagcggctgttgccggtgctgtgccaggaccatggcctgaccccggaccaagtggtggctatcgccagcaacattggcggcaagcaagcgctcgaaacggtgcagcggctgttgccggtgctgtgccaggaccatggcctgaccccggaccaagtggtggctatcgccagcaacaatggcggcaagcaagcgctcgaaacggtgcagcggctgttgccggtgctgtgccaggaccatggcctgaccccggaccaagtggtggctatcgccagccacgatggcggcaagcaagcgctcgaaagcattgtggcccagctgagccggcctgatccggcgttggccgcgttgaccaacgaccacctcgtcgccttggcctgcctcggcggacgtcctgccatggatgcagtgaaaaagggattgccgcacgcgccggaattgatcagaagagtcaatcgccgtattggcgaacgcacgtcccatcgcgttgcctatccctatgacgtgcccgattatgccagcctgggcagcggctcccccaagaaaaaacgcaaggtggaagatcctaagaaaaagcggaaagtggacggcagcggcagcgagacccccggtaccagcgagagcgccacccccgagagcatgaacaattcccagggaagagtgaccttcgaggatgtcactgtgaacttcacccagggggagtggcagcggctgaatcccgaacagagaaacttgtacagggatgtgatgctggagaattacagcaaccttgtctctgtgggacaaggggaaaccaccaaacccgatgtgatcttgaggttggaacaaggaaaggagccatggttggaggaagaggaagtgctgggaagtggccgtgcagaaaaaaatggggacattggagggcagatttggaagccaaaggatgtgaaagagagtctcctcgagggaagcggagctactaacttcagcctgctgaagcaggctggagacgtggaggagaaccctggacctatgcctgctgctaagagagtgaaactggatggatccaaccatgaccaggaatttgaccccccaaaggtttacccacctgtgccagctgagaagaggaagcccatccgcgtgctgtctctctttgatgggattgctacagggctcctggtgctgaaggacctgggcatccaagtggaccgctacattgcctccgaggtgtgtgaggactccatcacggtgggcatggtgcggcaccagggaaagatcatgtacgtcggggacgtccgcagcgtcacacagaagcatatccaggagtggggcccattcgacctggtgattggaggcagtccctgcaatgacctctccattgtcaaccctgcccgcaagggactttatgagggtactggccgcctcttctttgagttctaccgcctcctgcatgatgcgcggcccaaggagggagatgatcgccccttcttctggctctttgagaatgtggtggccatgggcgttagtgacaagagggacatctcgcgatttcttgagtctaaccccgtgatgattgacgccaaagaagtgtctgctgcacacagggcccgttacttctggggtaaccttcctggcatgaacaggcctttggcatccactgtgaatgataagctggagctgcaagagtgtctggagcacggcagaatagccaagttcagcaaagtgaggaccattaccaccaggtcaaactctataaagcagggcaaagaccagcatttccccgtgttcatgaacgagaaggaggacatcctgtggtgcactgaaatggaaagggtgtttggcttccccgtccactacacagacgtctccaacatgagccgcttggcgaggcagagactgctgggccgatcgtggagcgtgccggtcatccgccacctcttcgctccgctgaaggaatattttgcttgtgtgtctagcggcaatagtaacgctaacagccgcgggccgagcttcagcagcggcctggtgccgttaagcttgcgcggcagccatatgttcgaaaccgtgcctgtgtggaggagacagccagtccgggtgctgtccctttttgaagacatcaagaaagagctgacgagtttgggctttttggaaagtggttctgacccgggacaactgaagcatgtggttgatgtcacagacacagtgaggaaggatgtggaggagtggggacccttcgatcttgtgtacggcgccacacctcccctgggccacacctgtgaccgtcctcccagctggtacctgttccagttccaccggctcctgcagtacgcacggcccaagccaggcagccccaggcccttcttctggatgttcgtggacaatctggtgctgaacaaggaagacctggacgtcgcatctcgcttcctggagatggagccagtcaccatcccagatgtccacggcggatccttgcagaatgctgtccgcgtgtggagcaacatcccagccataaggagcagcaggcactgggctctggtttcggaagaagaattgtccctgctggcccagaacaagcagagctcgaagctcgcggccaagtggcccaccaagctggtgaagaactgctttctccccctaagagaatatttcaagtatttttcaggagggccgagctctggcgcacccccaccaagtggagggtctcctgccgggtccccaacatctactgaagaaggcaccagcgaatccgcaacgcccgagtcaggccctggtacctccacagaaccatctgaaggtagtgcgcctggttccccagctggaagccctacttccaccgaagaaggcacgtcaaccgaaccaagtgaaggatctgcccctgggaccagcactgaaccatctgagccaaaaaagaagagaaaggtaccatctgagggccccgacatcgtgatgacccagagccccagcagcctgagcgccagcgtgggcgaccgcgtgaccatcacctgccgcagcagcaccggcgccgtgaccaccagcaactacgccagctgggtgcaggagaagcccggcaagctgttcaagggcctgatcggcggcaccaacaaccgcgcccccggcgtgcccagccgcttcagcggcagcctgatcggcgacaaggccaccctgaccatcagcagcctgcagcccgaggacttcgccacctacttctgcgccctgtggtacagcaaccactgggtgttcggccagggcaccaaggtggagctgaagcgcggcggcggcggcagcggcggcggcggcagcggcggcggcggcagcagcggcggcggcagcgaggtgaagctgctggagagcggcggcggcctggtgcagcccggcggcagcctgaagctgagctgcgccgtgagcggcttcagcctgaccgactacggcgtgaactgggtgcgccaggcccccggccgcggcctggagtggatcggcgtgatctggggcgacggcatcaccgactacaacagcgccctgaaggaccgcttcatcatcagcaaggacaacggcaagaacaccgtgtacctgcagatgagcaaggtgcgcagcgacgacaccgccctgtactactgcgtgaccggcctgttcgactactggggccagggcaccctggtgaccgtgagcagctacccatacgatgttccagattacgctggtggaggcggaggttctgggggaggaggtagtggcggtggtggttcaggaggcggcggaagctga

SEQ ID NO: 360 - DNA, 6114 bp, synthetic construct
  misc_feature 1..6114: note = CDS of V51_3xGCN4-TALE HPT12-ZIM3-P2A-D3a-hD3L-XTEN80-scFv
  source 1..6114: mol_type = other DNA
atgcctgctgctaagagagtgaaactggatggatccgaggaactgctgagcaagaactaccacctggaaaacgaggtggccagactgaagaaaggctctggctctggcggaagcggttctggcggatcaggatctggaagtggcggctctggaagcggaggttctggatctggcgaagaactgctgtctaagaattatcacctcgagaacgaagtggctcggctcaagaaaggcagtggcagcggaggaagtggatccggcggtagtggtagtggaagcggcggatccggctcaggcggatctggttcaggggaagaactcctctccaaaaactaccatctcgagaatgaggtcgcccgcctgaaaaaaggatcaggttccggtggttctggcagcggtggttcaggctcaggcagcggcggtagcggtagcggtggaagcggaagcggaccaaaaaagaagagaaaggtaatggtggatctacgcacgctcggctacagccagcagcaacaggagaagatcaaaccgaaggttcgttcgacagtggcgcagcaccacgaggcactggtcggccatgggtttacacacgcgcacatcgttgcgctcagccaacacccggcagcgttagggaccgtcgctgtcaagtatcaggacatgatcgcagcgttgccagaggcgacacacgaagcgatcgttggcgtcggcaaacagtggtccggcgcacgcgctctggaggccttgctcacggtggcgggagagttgagaggtccaccgttacagttggacacaggccaacttctcaagattgcaaaacgtggcggcgtgaccgcagtggaggcagtgcatgcatggcgcaatgcactgacgggtgcccccctgaacctgaccccggaccaagtggtggctatcgccagcaacaatggcggcaagcaagcgctcgaaacggtgcagcggctgttgccggtgctgtgccaggaccatggcctgaccccggaccaagtggtggctatcgccagcaacaatggcggcaagcaagcgctcgaaacggtgcagcggctgttgccggtgctgtgccaggaccatggcctgaccccggaccaagtggtggctatcgccagcaacattggcggcaagcaagcgctcgaaacggtgcagcggctgttgccggtgctgtgccaggaccatggcctgaccccggaccaagtggtggctatcgccagcaacaatggcggcaagcaagcgctcgaaacggtgcagcggctgttgccggtgctgtgccaggaccatggcctgaccccggaccaagtggtggctatcgccagcaacaatggcggcaagcaagcgctcgaaacggtgcagcggctgttgccggtgctgtgccaggaccatggcctgaccccggaccaagtggtggctatcgccagcaacattggcggcaagcaagcgctcgaaacggtgcagcggctgttgccggtgctgtgccaggaccatggcctgaccccggaccaagtggtggctatcgccagcaacaatggcggcaagcaagcgctcgaaacggtgcagcggctgttgccggtgctgtgccaggaccatggcctgaccccggaccaagtggtggctatcgccagcaacggtggcggcaagcaagcgctcgaaacggtgcagcggctgttgccggtgctgtgccaggaccatggcctgaccccggaccaagtggtggctatcgccagcaacaatggcggcaagcaagcgctcgaaacggtgcagcggctgttgccggtgctgtgccaggaccatggcctgaccccggaccaagtggtggctatcgccagcaacattggcggcaagcaagcgctcgaaacggtgcagcggctgttgccggtgctgtgccaggaccatggcctgaccccggaccaagtggtggctatcgccagcaacaatggcggcaagcaagcgctcgaaacggtgcagcggctgttgccggtgctgtgccaggaccatggcctgactccggaccaagtggtggctatcgccagccacgatggcggcaagcaagcgctcgaaacggtgcagcggctgttgccggtgctgtgccaggaccatggcctgactccggaccaagtggtggctatcgccagccacgatggcggcaagcaagcgctcgaaacggtgcagcggctgttgccggtgctgtgccaggaccatggcctgaccccggaccaagtggtggctatcgccagcaacattggcggcaagcaagcgctcgaaacggtgcagcggctgttgccggtgctgtgccaggaccatggcctgaccccggaccaagtggtggctatcgccagcaacaatggcggcaagcaagcgctcgaaacggtgcagcggctgttgccggtgctgtgccaggaccatggcctgaccccggaccaagtggtggctatcgccagcaacaatggcggcaagcaagcgctcgaaacggtgcagcggctgttgccggtgctgtgccaggaccatggcctgactccggaccaagtggtggctatcgccagccacgatggcggcaagcaagcgctcgaaacggtgcagcggctgttgccggtgctgtgccaggaccatggcctgaccccggaccaagtggtggctatcgccagcaacattggcggcaagcaagcgctcgaaagcattgtggcccagctgagccggcctgatccggcgttggccgcgttgaccaacgaccacctcgtcgccttggcctgcctcggcggacgtcctgccatggatgcagtgaaaaagggattgccgcacgcgccggaattgatcagaagagtcaatcgccgtattggcgaacgcacgtcccatcgcgttgcctatccctatgacgtgcccgattatgccagcctgggcagcggctcccccaagaaaaaacgcaaggtggaagatcctaagaaaaagcggaaagtggacggcagcggcagcgagacccccggtaccagcgagagcgccacccccgagagcatgaacaattcccagggaagagtgaccttcgaggatgtcactgtgaacttcacccagggggagtggcagcggctgaatcccgaacagagaaacttgtacagggatgtgatgctggagaattacagcaaccttgtctctgtgggacaaggggaaaccaccaaacccgatgtgatcttgaggttggaacaaggaaaggagccatggttggaggaagaggaagtgctgggaagtggccgtgcagaaaaaaatggggacattggagggcagatttggaagccaaaggatgtgaaagagagtctcctcgagggaagcggagctactaacttcagcctgctgaagcaggctggagacgtggaggagaaccctggacctatgcctgctgctaagagagtgaaactggatggatccaaccatgaccaggaatttgaccccccaaaggtttacccacctgtgccagctgagaagaggaagcccatccgcgtgctgtctctctttgatgggattgctacagggctcctggtgctgaaggacctgggcatccaagtggaccgctacattgcctccgaggtgtgtgaggactccatcacggtgggcatggtgcggcaccagggaaagatcatgtacgtcggggacgtccgcagcgtcacacagaagcatatccaggagtggggcccattcgacctggtgattggaggcagtccctgcaatgacctctccattgtcaaccctgcccgcaagggactttatgagggtactggccgcctcttctttgagttctaccgcctcctgcatgatgcgcggcccaaggagggagatgatcgccccttcttctggctctttgagaatgtggtggccatgggcgttagtgacaagagggacatctcgcgatttcttgagtctaaccccgtgatgattgacgccaaagaagtgtctgctgcacacagggcccgttacttctggggtaaccttcctggcatgaacaggcctttggcatccactgtgaatgataagctggagctgcaagagtgtctggagcacggcagaatagccaagttcagcaaagtgaggaccattaccaccaggtcaaactctataaagcagggcaaagaccagcatttccccgtgttcatgaacgagaaggaggacatcctgtggtgcactgaaatggaaagggtgtttggcttccccgtccactacacagacgtctccaacatgagccgcttggcgaggcagagactgctgggccgatcgtggagcgtgccggtcatccgccacctcttcgctccgctgaaggaatattttgcttgtgtgtctagcggcaatagtaacgctaacagccgcgggccgagcttcagcagcggcctggtgccgttaagcttgcgcggcagccatatgttcgaaaccgtgcctgtgtggaggagacagccagtccgggtgctgtccctttttgaagacatcaagaaagagctgacgagtttgggctttttggaaagtggttctgacccgggacaactgaagcatgtggttgatgtcacagacacagtgaggaaggatgtggaggagtggggacccttcgatcttgtgtacggcgccacacctcccctgggccacacctgtgaccgtcctcccagctggtacctgttccagttccaccggctcctgcagtacgcacggcccaagccaggcagccccaggcccttcttctggatgttcgtggacaatctggtgctgaacaaggaagacctggacgtcgcatctcgcttcctggagatggagccagtcaccatcccagatgtccacggcggatccttgcagaatgctgtccgcgtgtggagcaacatcccagccataaggagcagcaggcactgggctctggtttcggaagaagaattgtccctgctggcccagaacaagcagagctcgaagctcgcggccaagtggcccaccaagctggtgaagaactgctttctccccctaagagaatatttcaagtatttttcaggagggccgagctctggcgcacccccaccaagtggagggtctcctgccgggtccccaacatctactgaagaaggcaccagcgaatccgcaacgcccgagtcaggccctggtacctccacagaaccatctgaaggtagtgcgcctggttccccagctggaagccctacttccaccgaagaaggcacgtcaaccgaaccaagtgaaggatctgcccctgggaccagcactgaaccatctgagccaaaaaagaagagaaaggtaccatctgagggccccgacatcgtgatgacccagagccccagcagcctgagcgccagcgtgggcgaccgcgtgaccatcacctgccgcagcagcaccggcgccgtgaccaccagcaactacgccagctgggtgcaggagaagcccggcaagctgttcaagggcctgatcggcggcaccaacaaccgcgcccccggcgtgcccagccgcttcagcggcagcctgatcggcgacaaggccaccctgaccatcagcagcctgcagcccgaggacttcgccacctacttctgcgccctgtggtacagcaaccactgggtgttcggccagggcaccaaggtggagctgaagcgcggcggcggcggcagcggcggcggcggcagcggcggcggcggcagcagcggcggcggcagcgaggtgaagctgctggagagcggcggcggcctggtgcagcccggcggcagcctgaagctgagctgcgccgtgagcggcttcagcctgaccgactacggcgtgaactgggtgcgccaggcccccggccgcggcctggagtggatcggcgtgatctggggcgacggcatcaccgactacaacagcgccctgaaggaccgcttcatcatcagcaaggacaacggcaagaacaccgtgtacctgcagatgagcaaggtgcgcagcgacgacaccgccctgtactactgcgtgaccggcctgttcgactactggggccagggcaccctggtgaccgtgagcagctacccatacgatgttccagattacgctggtggaggcggaggttctgggggaggaggtagtggcggtggtggttcaggaggcggcggaagctga

SEQ ID NO: 361 - protein, 1554 aa, synthetic construct
  REGION 1..1554: note = (from V48)_D3a-hD3L-TALE HPT8-1xGCN4
  SITE 1554: note = misc_feature - Xaa =
MPAAKRVKLDGSNHDQEFDPPKVYPPVPAEKRKPIRVLSLFDGIATGLLVLKDLGIQVDRYIASEVCEDSITVGMVRHQGKIMYVGDVRSVTQKHIQEWGPFDLVIGGSPCNDLSIVNPARKGLYEGTGRLFFEFYRLLHDARPKEGDDRPFFWLFENVVAMGVSDKRDISRFLESNPVMIDAKEVSAAHRARYFWGNLPGMNRPLASTVNDKLELQECLEHGRIAKFSKVRTITTRSNSIKQGKDQHFPVFMNEKEDILWCTEMERVFGFPVHYTDVSNMSRLARQRLLGRSWSVPVIRHLFAPLKEYFACVSSGNSNANSRGPSFSSGLVPLSLRGSHMFETVPVWRRQPVRVLSLFEDIKKELTSLGFLESGSDPGQLKHVVDVTDTVRKDVEEWGPFDLVYGATPPLGHTCDRPPSWYLFQFHRLLQYARPKPGSPRPFFWMFVDNLVLNKEDLDVASRFLEMEPVTIPDVHGGSLQNAVRVWSNIPAIRSSRHWALVSEEELSLLAQNKQSSKLAAKWPTKLVKNCFLPLREYFKYFSGGPSSGAPPPSGGSPAGSPTSTEEGTSESATPESGPGTSTEPSEGSAPGSPAGSPTSTEEGTSTEPSEGSAPGTSTEPSEPKKKRKVMVDLRTLGYSQQQQEKIKPKVRSTVAQHHEALVGHGFTHAHIVALSQHPAALGTVAVKYQDMIAALPEATHEAIVGVGKQWSGARALEALLTVAGELRGPPLQLDTGQLLKIAKRGGVTAVEAVHAWRNALTGAPLNLTPDQVVAIASNGGGKQALETVQRLLPVLCQDHGLTPDQVVAIASHDGGKQALETVQRLLPVLCQDHGLTPDQVVAIASNIGGKQALETVQRLLPVLCQDHGLTPDQVVAIASNNGGKQALETVQRLLPVLCQDHGLTPDQVVAIASNGGGKQALETVQRLLPVLCQDHGLTPDQVVAIASNGGGKQALETVQRLLPVLCQDHGLTPDQVVAIASHDGGKQALETVQRLLPVLCQDHGLTPDQVVAIASNIGGKQALETVQRLLPVLCQDHGLTPDQVVAIASNNGGKQALETVQRLLPVLCQDHGLTPDQVVAIASNNGGKQALETVQRLLPVLCQDHGLTPDQVVAIASNNGGKQALETVQRLLPVLCQDHGLTPDQVVAIASNGGGKQALETVQRLLPVLCQDHGLTPDQVVAIASHDGGKQALETVQRLLPVLCQDHGLTPDQVVAIASNGGGKQALETVQRLLPVLCQDHGLTPDQVVAIASNNGGKQALETVQRLLPVLCQDHGLTPDQVVAIASNIGGKQALETVQRLLPVLCQDHGLTPDQVVAIASNNGGKQALETVQRLLPVLCQDHGLTPDQVVAIASHDGGKQALESIVAQLSRPDPALAALTNDHLVALACLGGRPAMDAVKKGLPHAPELIRRVNRRIGERTSHRVAYPYDVPDYASLGSGSPKKKRKVEDPKKKRKVDGIGSGSNGSSGEELLSKNYHLENEVARLKKGSGSGGSGSGGSGSGSGGSGSGGSGSGEELLSKNYHGSGSGQRGSKRTADGSEFESPKKKRKVX

SEQ ID NO: 362 - protein, 1554 aa, synthetic construct
  REGION 1..1554: note = (from V49)_D3a-hD3L-TALE HPT12-1xGCN4
  SITE 1554: note = misc_feature - Xaa =
MPAAKRVKLDGSNHDQEFDPPKVYPPVPAEKRKPIRVLSLFDGIATGLLVLKDLGIQVDRYIASEVCEDSITVGMVRHQGKIMYVGDVRSVTQKHIQEWGPFDLVIGGSPCNDLSIVNPARKGLYEGTGRLFFEFYRLLHDARPKEGDDRPFFWLFENVVAMGVSDKRDISRFLESNPVMIDAKEVSAAHRARYFWGNLPGMNRPLASTVNDKLELQECLEHGRIAKFSKVRTITTRSNSIKQGKDQHFPVFMNEKEDILWCTEMERVFGFPVHYTDVSNMSRLARQRLLGRSWSVPVIRHLFAPLKEYFACVSSGNSNANSRGPSFSSGLVPLSLRGSHMFETVPVWRRQPVRVLSLFEDIKKELTSLGFLESGSDPGQLKHVVDVTDTVRKDVEEWGPFDLVYGATPPLGHTCDRPPSWYLFQFHRLLQYARPKPGSPRPFFWMFVDNLVLNKEDLDVASRFLEMEPVTIPDVHGGSLQNAVRVWSNIPAIRSSRHWALVSEEELSLLAQNKQSSKLAAKWPTKLVKNCFLPLREYFKYFSGGPSSGAPPPSGGSPAGSPTSTEEGTSESATPESGPGTSTEPSEGSAPGSPAGSPTSTEEGTSTEPSEGSAPGTSTEPSEPKKKRKVMVDLRTLGYSQQQQEKIKPKVRSTVAQHHEALVGHGFTHAHIVALSQHPAALGTVAVKYQDMIAALPEATHEAIVGVGKQWSGARALEALLTVAGELRGPPLQLDTGQLLKIAKRGGVTAVEAVHAWRNALTGAPLNLTPDQVVAIASNNGGKQALETVQRLLPVLCQDHGLTPDQVVAIASNNGGKQALETVQRLLPVLCQDHGLTPDQVVAIASNIGGKQALETVQRLLPVLCQDHGLTPDQVVAIASNNGGKQALETVQRLLPVLCQDHGLTPDQVVAIASNNGGKQALETVQRLLPVLCQDHGLTPDQVVAIASNIGGKQALETVQRLLPVLCQDHGLTPDQVVAIASNNGGKQALETVQRLLPVLCQDHGLTPDQVVAIASNGGGKQALETVQRLLPVLCQDHGLTPDQVVAIASNNGGKQALETVQRLLPVLCQDHGLTPDQVVAIASNIGGKQALETVQRLLPVLCQDHGLTPDQVVAIASNNGGKQALETVQRLLPVLCQDHGLTPDQVVAIASHDGGKQALETVQRLLPVLCQDHGLTPDQVVAIASHDGGKQALETVQRLLPVLCQDHGLTPDQVVAIASNIGGKQALETVQRLLPVLCQDHGLTPDQVVAIASNNGGKQALETVQRLLPVLCQDHGLTPDQVVAIASNNGGKQALETVQRLLPVLCQDHGLTPDQVVAIASHDGGKQALETVQRLLPVLCQDHGLTPDQVVAIASNIGGKQALESIVAQLSRPDPALAALTNDHLVALACLGGRPAMDAVKKGLPHAPELIRRVNRRIGERTSHRVAYPYDVPDYASLGSGSPKKKRKVEDPKKKRKVDGIGSGSNGSSGEELLSKNYHLENEVARLKKGSGSGGSGSGGSGSGSGGSGSGGSGSGEELLSKNYHGSGSGQRGSKRTADGSEFESPKKKRKVX

SEQ ID NO: 363 - protein, 1104 aa, synthetic construct
  REGION 1..1104: note = (from V50)_3xGCN4-TALE HPT8-ZIM3
MPAAKRVKLDGSEELLSKNYHLENEVARLKKGSGSGGSGSGGSGSGSGGSGSGGSGSGEELLSKNYHLENEVARLKKGSGSGGSGSGGSGSGSGGSGSGGSGSGEELLSKNYHLENEVARLKKGSGSGGSGSGGSGSGSGGSGSGGSGSGPKKKRKVMVDLRTLGYSQQQQEKIKPKVRSTVAQHHEALVGHGFTHAHIVALSQHPAALGTVAVKYQDMIAALPEATHEAIVGVGKQWSGARALEALLTVAGELRGPPLQLDTGQLLKIAKRGGVTAVEAVHAWRNALTGAPLNLTPDQVVAIASNGGGKQALETVQRLLPVLCQDHGLTPDQVVAIASHDGGKQALETVQRLLPVLCQDHGLTPDQVVAIASNIGGKQALETVQRLLPVLCQDHGLTPDQVVAIASNNGGKQALETVQRLLPVLCQDHGLTPDQVVAIASNGGGKQALETVQRLLPVLCQDHGLTPDQVVAIASNGGGKQALETVQRLLPVLCQDHGLTPDQVVAIASHDGGKQALETVQRLLPVLCQDHGLTPDQVVAIASNIGGKQALETVQRLLPVLCQDHGLTPDQVVAIASNNGGKQALETVQRLLPVLCQDHGLTPDQVVAIASNNGGKQALETVQRLLPVLCQDHGLTPDQVVAIASNNGGKQALETVQRLLPVLCQDHGLTPDQVVAIASNGGGKQALETVQRLLPVLCQDHGLTPDQVVAIASHDGGKQALETVQRLLPVLCQDHGLTPDQVVAIASNGGGKQALETVQRLLPVLCQDHGLTPDQVVAIASNNGGKQALETVQRLLPVLCQDHGLTPDQVVAIASNIGGKQALETVQRLLPVLCQDHGLTPDQVVAIASNNGGKQALETVQRLLPVLCQDHGLTPDQVVAIASHDGGKQALESIVAQLSRPDPALAALTNDHLVALACLGGRPAMDAVKKGLPHAPELIRRVNRRIGERTSHRVAYPYDVPDYASLGSGSPKKKRKVEDPKKKRKVDGSGSETPGTSESATPESMNNSQGRVTFEDVTVNFTQGEWQRLNPEQRNLYRDVMLENYSNLVSVGQGETTKPDVILRLEQGKEPWLEEEEVLGSGRAEKNGDIGGQIWKPKDVKESL

SEQ ID NO: 364 - protein, 1104 aa, synthetic construct
  REGION 1..1104: note = (from V51)_3xGCN4-TALE HPT12-ZIM3
MPAAKRVKLDGSEELLSKNYHLENEVARLKKGSGSGGSGSGGSGSGSGGSGSGGSGSGEELLSKNYHLENEVARLKKGSGSGGSGSGGSGSGSGGSGSGGSGSGEELLSKNYHLENEVARLKKGSGSGGSGSGGSGSGSGGSGSGGSGSGPKKKRKVMVDLRTLGYSQQQQEKIKPKVRSTVAQHHEALVGHGFTHAHIVALSQHPAALGTVAVKYQDMIAALPEATHEAIVGVGKQWSGARALEALLTVAGELRGPPLQLDTGQLLKIAKRGGVTAVEAVHAWRNALTGAPLNLTPDQVVAIASNNGGKQALETVQRLLPVLCQDHGLTPDQVVAIASNNGGKQALETVQRLLPVLCQDHGLTPDQVVAIASNIGGKQALETVQRLLPVLCQDHGLTPDQVVAIASNNGGKQALETVQRLLPVLCQDHGLTPDQVVAIASNNGGKQALETVQRLLPVLCQDHGLTPDQVVAIASNIGGKQALETVQRLLPVLCQDHGLTPDQVVAIASNNGGKQALETVQRLLPVLCQDHGLTPDQVVAIASNGGGKQALETVQRLLPVLCQDHGLTPDQVVAIASNNGGKQALETVQRLLPVLCQDHGLTPDQVVAIASNIGGKQALETVQRLLPVLCQDHGLTPDQVVAIASNNGGKQALETVQRLLPVLCQDHGLTPDQVVAIASHDGGKQALETVQRLLPVLCQDHGLTPDQVVAIASHDGGKQALETVQRLLPVLCQDHGLTPDQVVAIASNIGGKQALETVQRLLPVLCQDHGLTPDQVVAIASNNGGKQALETVQRLLPVLCQDHGLTPDQVVAIASNNGGKQALETVQRLLPVLCQDHGLTPDQVVAIASHDGGKQALETVQRLLPVLCQDHGLTPDQVVAIASNIGGKQALESIVAQLSRPDPALAALTNDHLVALACLGGRPAMDAVKKGLPHAPELIRRVNRRIGERTSHRVAYPYDVPDYASLGSGSPKKKRKVEDPKKKRKVDGSGSETPGTSESATPESMNNSQGRVTFEDVTVNFTQGEWQRLNPEQRNLYRDVMLENYSNLVSVGQGETTKPDVILRLEQGKEPWLEEEEVLGSGRAEKNGDIGGQIWKPKDVKESL

SEQ ID NO: 365 - DNA, 20 bp, synthetic construct
  misc_feature 1..20: note = NT gRNA
  source 1..20: mol_type = other DNA
ctgaaggtgtctggcagagc